European Patent Application EP 4 141 103 A1, published March 1, 2023. Title: NOUVEL AGENT DE BIOSTIMULATION ET SES UTILISATIONS. Applicant: AGRO INDUSTRIE RECHERCHES ET DEVELOPPEMENTS (A.R.D.). Application EP. The sequence listing filed with the application follows.

SEQUENCE LISTING (78 sequences)

SEQ ID NO: 1 - DNA, 1168789 bp, Chitinophaga pinensis
  source 1..1168789: mol_type = genomic DNA
ttgctaaagcaagctgacattaactatttattctcttaaaaaacacctgatcatcataatgattattaggccatcttttggctaaaacaaagaagctgtctcaattaattatgagacagcttcttttaatataaagtcaatattatgctaaccagttattttttctgctgcgcaagatagctaacgagcgatgcaagttcctcgtatgataatgcgttggcaaggccggttggcatcatcgatgttttcatttccttacgggtcaggatatcggccgttttaacggtgaatacctggccggtgatatctctcatgactaccctggcggaagtttcttccgtaacaaatcccatataagacttgttgcctttcgccgtgatcatcaccgtggcaaatccctgtgaaatagatgcgttaggtttgagaatggattccgtgatctgctcccggttcatgatggatccgatctgtcccataaaaggacctttcattgtttctcctttattgatactgtggcaggccacacaaccctggatggtaaacaattgctttcccctggccggatctccttttaatttattgatggccagcaacacatcttcgatagatgacttacctacctgaccttttttactttttatcttttccaggtctactttaggttctttcaccggagccgctatcacttttttctctgctgcgaaagcaggaatatccatcctgttgcgcgcatcgagatccctgaaaaacgctttgccggtggggcttgttttcagcgattcttttttaaggaatttttcgatagccggtgatgcttcccaggttactgctttgtagtaggggccatgcgagtcgggcctggttccccaccaccatgatgcatcataggtatcttcttttttgtagaggcgtgctaaggtggtgatgatctgccgttttagtttcgcatctttcgacagctcgtaagcatttatcaggccgtccactgccttcggatcatgcatgtatcgtagcgcccacaaggcaagcgtggcattttcggtgttgatggctgctacggtggcatctacggcgtgcagatttacaagggcccgaactgccaggtgaggcagtacgatagctgcattaggcgtagcatgcggtccttcgatatctttaacaggtgcaacaaatgaggcaggcactttggtttgcagcaaagcgctggcagtttcaatgcgacctaaacgtccaagtcctattattgcagcagcctgtacgcgcggagacggatctttaagtccttccaggaaaggttcagtggcaacatctttcaggagacctttccggtcggccaaagcgcgcaatgcatgttccctcatggtggcatcttttgttaaggctgttaaagcggggatgccttctgcgccggcaatttgtgcgtatgtataaagaccggccacacgtgcaaataacggcaactgcacatctgaagcgattcccagcgctgcggcaatggcgtctttaccggcgcgtgcgattaattcctgggaggcattcaaacgggctaccgcgctggccgatttaagcaaccgggccaattcttcaacagaggctttggccacgtcagggaatggctggtaagtccagttgtttggtaccgcgcggattacataacctttctccggactgccggaatagcctgcgccatcccatgcggaaaggtaaagccggccggagccgtcaacatccagatctgtaatctgaggcaatcctataaactcctcttctttttgggtgaaggtcgggccatcgggcgttacgcggtgaatatacagcatgctccggccccaatctgccatcatgggaacgttattgtatttctccggccagcttggttccgccatgtataaagcgcctgtgcctgagccaccgccaaggtctgcaagcgctggtaatatttcgtctgtaaaatgctgaaacaataccgggtatccatattccccggattggatatggtgggaaaaccgcacattccatccaccgccgtcattggtattttctcttgtaaaaatattcatgtaggggtcaatggccacgtcatacacattgcgtgtaccatgggtaaatatctccatttccgtaccgtcggggcgtacccgtacgataccaccaccaagcatggtcagtttcttaccggaacggtctgttgcatcatgaaatccaaaatcacctaccgcaatatagatccagccatcaatacccatccggataccgttagtggcatgatccgttccccgctcctggatgtatttggtattactgaggttttcgatcagtggctggggaggtccgtctgcttttccgtccccgtctttatcttcaaaaacaaccagcgccattcctgacgctttaccggtttctttggaaaatgtggtatgcaatacaaaaacccggctgccctgcacaatgatgccacgcgggttatccaccgttgcaaattcaatatgctggtccattttaccgtcgttgtccttatcaataagcttaagaatccggcctttgcccgggtcctttcctaatgaaccgatcatatccactcctacaaacacttcgcctgttggcgccactgcaaggcaggcggggctgggcgttatatccggaccggaaaatcttgtaatagttaattcaggtggattgggagcagtggtttgagcgtctccaataaattgatttgagccaataaatactgcaagagaatagatcaggccgagagaaattttcgtcatttgtgttcgctgtattaataagatagtattgttcagtgctttgccaaaagcaaaggtcaatatagaaaaaataaactttcaggccggaattatttggcgaacggcaccaggtgctgttgaatgcgatgctatttcccctctgtcagcttcaatacatattccatctgtgtatcgcggttttgcataaaatcgctgaaggaaggccacacggtataatcgggaataatccctctaccttccggctgatccggttttacaggtgcgtcctgctccacataaacaatagagaatttcgtttttatttttgagtgcggcagttcgtatatcatggatgcatggccgttgtggacataataaccaccaacagtttccacccccacaatggtcacattgcgggcataggcttttacgagagaagccaggtgggaggccgccgatgccacgttttcatcaatcagtaaatataactttcctttgaaaccaggactcttagggtggtataccgggttgtacttcgggttttgcatattcctgccgttgtgcagtgccgggaaataatctttcagaaacgcttttccggcaactttgcccgccgaatccagtctttccgcggtggacacgccccaaaagtattcttcatacggaattccattatcaaagatggtatatgccaatgtattctctttgaagcttgtatccgtgaggtacatcatcggttgttcaaaagtaggatcactgccgccgggattaccgcggatatccaggatgaggtgcgggatactgttgtggctaagcgcctggaatacgctgtcgagaaacgccacatataccgggaaagccggatcagccgcgtcgctggccatggagaatatccgcaggctcagtaaacctgttgaagggtttaccatcttaaaactatatttgggctgcacattataatcgatcaggctgtcgaccggcgcgctatgacgccgtattaagtttgctttttgttcttccagcgataccgccggtactgtaacggtttgctgccgggtagtgcccggagctgtaaaccggatggcgaagctatcattaatgccatactcatacaggtaacgcaaaccatagctcctgttcacgctgcccgattgcttttgtgtctggataaatccatcggaggtcatgtacttgtaaaaggattgcatcaggtctttgtctgcaacgccgttgatactcattatccttgatcctaccggaatatcgggcgtttcgctattgaagatcatattgccgtcaatatacttcagggcaaaaggaaagaagccacgctgccggttgaaatacccgaccagggcggcatccggctctgtataattatgacagcttccttcaaaatcggtgagctgcaaaatgatcttataaaaagccacagtggacataggttgacgcacctggcggaaggcccattggtagatgctgtcgacttgcttcggggtgcggtagcgatacaaaccagagttggcttttttacggatatcgagaaacacctgcaggtcctgcttcatttcaccgggattgagctgccggttgtagatggagaggctgtcgatagattggttggccctggatagatgtttggttgattgtgcccatccctggtgcaccagcagtagcaaaaacagtacttttctcatttggtttttaagatatcaggggcgaatctacaaaaacctgttccatttcgcgcggacagcctggcctattactggaaaaatccactgtacaaaaacaaccgtgatccaaggctgacagccagcgttcttttcccggggcaaacatttgtaaaccgtttgctggacccattcacggcgggatcggcagaccagatcggggctgcgcaatccacgcaaaccggcttctgggtgaggaaatatctcgatgccaaagatgtgtcccgcaatatgccggcaccttaaattttatgatcatccgttacgcagagatcttactgagttatgtagaagccttagtagaatcgggcgactggcaaaacccggatgtattgctgtatctcaacaagatccgcaaccgcgcaggaatgccaaatgtaaatacggcggtgtataacaccgctgaaaaaatgcgtgaattataccgccgggaaagaaaagtggagctggcatttgaaggtacccgcctgtttgacatacgccgctggaagataggagaagaaagttctgaaagggcccgcgatgggtgctatcaatcctaatacaagtcagccggtaattgtagagaacaggatatttgaccgggagcgtgattacctgtggccgattcccctggtggagattaatgggaatccggcgatgaagcagaatccgaagtggtaatttgattagaccgacctttctaccaggttgttttttatcccgatgccaaaggcgctctactaactgagcgcctttcttataataattatagtcaaaattcgaatttttctcatttttatgctatacaatgaatttattttactatatttgagataatttctcataaatagacaattctatgttattagagttttccgttactaattatctttcctttaaagaaaagactacattaaacctttcagctacagctattaaggaacatgttgcgtcaaatattttcacctccggacgccataacttgcttaaaggggctgttatctatggtgctaatgccagtggcaaaagtaattttgtaaaagccatgtctactatgaggcgacttgtattacaatcatttgaacaatcttctacagatgagttggatattacgcctttcctgttaaacactgaaacagaaaatgctccctcctcttttgaagttgtatttcttattggcgaaagtaaatatcgttatggctttgaggtggataaccgcagtgtattatctgaatggctttttgatgccccgaaacaagccgaaaggcctttgtttatcagggaaaaagatggtattgaagtaatgccaagggttttcccggaagggagagatctggaagaaagaacaagggacaatgcactattcctatcagtggtagatcagtttaatggcaagattgccaagcaaataatgcgttggtttcatgattttatcaccatttccggattaagtcatgagcgatataaaggcgtaacatttgatttgcttgaaaacaaacacacccagcatcttttacttgatttctataaaaaagttgacctgggatttgatgacattaccatttccaaagccccttttgatccgagagaactgcccaatgacctgcctgaaaaccttctgaaacagttaattaccgatcttgaagagtcttacagaatagatattaaaaccgttcacaaaaaatacaatgcaaaaaataaggtggtcggcaatgttgaatttgatatgcgtagccaggagtcttctggtagcaataaactgttcaatatctcaggccccatctttgatgtactaaatgatggtggaacacttgtagtggacgagttagatgccagcttgcaccctttattaacgctggcaattaccagactttttaactccgccgaatttaacaagaacaacgcacagctgatatttgctacacatgataccaatctgctgaattatggtaactaccgtagagatcagatttattttgtagaaaaaaataaatacggagcttctgaaatgtattcactcgtggaatataaagaagaaggaaaaaccattcgtaaagaccgctcttttgagaaggattatatagagggccggtatggtgctattccgtttattggcaacctttcaaatgtaattacggaatggcaagaaaaataaagattccaaatgaacatttaaagcgtttcaaaagagaggaacaaaagcgcaaaattaatgtaagaaataaacgcagatattacctgatagtttgcgaaggtgaaaaaactgaacctaattattttcagggccttaaagaggatttgcctaaaggtgtactaacctggtgtcaaatagatattgaaggtactggcagaaatacccagtcgctcgttgatgaagcactgcgcctaaaaaagtggtatgagcaggagtataacagacctattgataaactttgggttgtttttgacagggacagcttttctgcaaatgatttcaataatgctgttcaacgatgtcagaacacaaaacctgtaataggatgtgcctggactaacgaggcttttgaactatggtatctgctgcattttcattactataatcacagtatgagcagaaaagactaccagaatgctattgaagataatttaaaacctatactgggaggaggatatagttatcaaaagaatagcagggatatgtatgatctcttgaaagaacatggaagtttagaagccgcaacaaggaacgctaaacggttgacagaaagttatgcaaaacgagaagattatgcgaatcataatccttgtacaatggtatggcagctggtagaggaattattgaatctgtagccgacctgcgaatcctgtatcctatacctgactttgctctcaaatacagcgcattccctctgaaaccggatagaactgcaatagcaacaggcgtttacctacagaagccgtgcaggaaaggtggacttgatcaggagatgtgattgggatgaatttgatcttcgcgaaaggtattttaggaaagaggatgatgtgatttttactgatacgatgaccttcttactcccccaaagcggccggacgcacacttacgggcataacaacgcacagaaaggcagtttcctttgcagggaaatatatgctgatggaagtggtgatgataattaccgcgctgcgtagtctacagcatagttaatgccatgactatggcgtaactcattcccgttgccgcgcagataccggcaacgttgttttttttgtggcaggcagcgggtgataaggcagcactctttttacatgaggtatcttgtttactttaacgggttgcttctttctggcagcaggcgccattaccgcaatgatgtcagcggccttgctccggcggttttcaatagcagcgccatgttcatatgcttttacctgtaaagtgaccagcaatgtacctttcccgggaacggtggcggccagttcagcgccgttgaaaggccggctcaaatcaattatgatggccgaatcaatacaccctgttacctgccgttgcgcgaagttaatacgaacagccaccaccgtaatttccaggtgcgttgctttggcgggcggccacaactgctgtgctggtatatgcagcattccgccggatgtgataactggttggtgcgaaaagaactggtccacgccggtatacgggttaaaccggaagcctttcagctccgtgaggcaatcctttgttgcggtgatcagcgctttgtttaagcggttcaccagcgtgccgcagggatttatttccaggcgaggaacgatggcctgccggatcagtttccctttcctgctggcaacaccaaagtcacgtgatgctctccgtgtagcggtagtttgccgtactgcatccggcatgctgcggaggaagtaggttccatttctccggtatcctatgacgttgcccaatttaccggtgaattggagcaaccctgtttgttttgccataaggggttaacatttttactgaaaatacgaaattattttcaatgaaatcagcagcaaaatcatcacttttttaacttctcaatggtcaatcccatttcagccagcctgtggccaaggttggacaggatatggtcttgctccgttggaaatctctctgctatctttttatacactggcaataatcttttatccttcactccggatagtgcctgcaatgcagcatgcaccacattatttgaaggatcatttaacccattgataaaaacatccaggtaggcagccttctttttaactttccctaaagtataaaaagctgttttccggatatcttcattgctgtgggttgtcatcggaacaattaaatgcgcgtagtccactttcatttcttccaacaggtaggtgcaaaaccggaatatttcctcatcatggatgttcaggatatttttttcgatgacttcctgccattccctacttttatcttttgcgtaccaccagataaatttagcaacggataagagatcaatatcgctgtaggccaccaggtgaggctttgccagcgggtagctgaactttgtgagcgcctgcagccagtcgcgtttgtactcttcttctgcctcccggtattccttttccagtattgcagcaaccgccggttcaacgcttcgtttgcacactatgccggtgatgcagttcagccgggttgttttatctgaagcagcatggtatttttccagcagagaagttacacttcctcccatggcatagccaaaccacgaaacaccatctgccagcaggtcttcagaaattatttcatccagccagcgttcataccaatcgaggaaattattttcaaaagtgaatcttggtttttgcctgtctatatcaatgtttactaccttaccggcatgttccccgtttaacaccaggccatgaataaaggcgcatccctgtgatccgatgggtagaataccagtgtaaatattttgtatggcggcatcgtatgcttcatctgaaagatcctccctttcggtttcctttatgagattattccattcgtcgtctgatataccggggtaaatttttacgggttcacttaaatattcttcaggattacttgtcaggtcatccgcacctttcttcagcgggtaaatgccatagtacggacctgcagctgagccggcctgggatactcctccatgtcccacataaagcaggaatgccctgaaacttccgggtaaagaaatgttgtgttctttttcaaaacccgaaagttgagcttcctccagcggtggatggatggtgtatttatggtagctggcgccgaatactttcagctgtttatctttttgctttgctgcttttaatttggtgctgatccgttctatttgttccttaaactgatgcatgggggttattttaaattaattaaaattaattttttttccccacaaacttttacttcttctcccgctgataagtaagcactactaccccgccatccagtatttttgtatcagaaagatgcaggccaccgggaagttttccgtctttaaagaaacgtttcccacttcccatgatgacgggatgtacaaagaatttgtattcatcaatcagatcggctttgataagcgcgtctaccaggatggcgcttccttctacctggatttccttgccgggttgttgtttcagccgggtgatttcttctatgacattgttttttatgatcgtggtattttcccacgcggctgtttccagcgtttcagatactacgtatttggctacactgtttagttttgcggagatgcccatttcgttgtttttcatctgcgaccaataaggcgccagcatttcatatgttttacggccaaagaggatggcatcgcaggcgtgaataccttcgctgatcagctcctgccgggcggggctgtcgtagggcataaaccattctcccattgtttctgcatcgaagataccgtcgagtgtgatccattcggaaatgactaactttctcatgttattttgtttttgttttttgatgatgattgtttacaggtacaaaataacagcacctttcccccttatgatagaagaaacccgacaaaatgaaaaagatggattaaccggggaagttgttcgcctgttttacatactccaggggagagtaatgggtaaagtctttaaacgcgcggatcaggtgactttgatctgcatagccgttttccagtgccacgtcgatcatgtctgaaaagttattctgactaagctggcggaaggcggcgttgaactggcagatcctgctgtacatttttggcgtaagaccaatatgttgttcaaacaaccgttgcagtgtgcgttctgtggtatatacttctttctgaagatcgttcattaacagggtacccttatttttctgaataaggcgggtggcaaaagaaatggtttcatttacccggatcttttttgaccgcaccaatgtgagtacataattattcatcagttccaggcggccgtttaaagagggcgtattgagcagctgttctttcaggctcatttccctggcgggatcatcatagctcaggtctataccctgatctgtgagttctttggcattgtatccaaaaagggagggcaacataaagggatacaggaaataggcaatcacggttatttcacctgccgtgtaaagccggatggggcgggtattctgaccgtacaataccaggtgatgacttttttttgtggtgctcagcatccttgccgggtctgttaactggaaagtaatactgggatacccgttggcgatgaggggaagaaccgcttcatagaacatactgttattttcaagcaccacgatgttgcttacataatcagctatagcaggaggaggcgtaagtgtttgtactttcattcccgggaaagatataggctaatttaggaaaaaacaatggttgttattcgaccttttctctccggagcctgaattccagtccgtctaccacgtctccttccatgcgcagcctgatggtaagcggcagcttcgcaggagtggcggtcatgccgagtttttgcaactgcagcgggtctattcttaccgtataggttccgggcggcaatcccatataattgaaatagccatctgcttccgtttgggtacgggccaccagtgtggaatcatttctgtaaaaaccgatggacaggcggcctattccctttgttacattttgttcttccaggatcactttaccggatacttcgcccataatcaccaccggcacttccaccagtttcatctggttgggatctattgctacactgatagcgggtttctttatctgccaggcaacattctcaaaactgttctttcccagttcgataaaatagtattcgtagggctccatatttacgatgcggatggtggtgtcgtgttgattctggagaatccggccgccgttacaatttgttttgaggccgtaggctttgggctcaccgggatcgcggcggtcattggcgttgagatccaggaagggcagcagtactacgcctcctgttcccacgctggtgcggttgctgaatcctgcgaatttggctttatcatcgtataccaggctgccgcgtgcagattctaccagggtagtcatgttagttcctttccaggcagaaaacccgatttgtgagaaagcgaaatcataacgcaaaccgatgcccacatttgtgatattacttttatagttacgttcataggatacgttcatgtaaccatgtctgaaaagatatttacccagctcgcatcttaccgccatcaggctgttgctgttgtattcatattgtacctggggagtaattaaaatttctcccggcaaccggtaggtgagcgcgaggttggtatatacaaacggcggttcaggttttataaagatggcataggtattcacgttaacgcctacacggaaaactgccccggacaccagccattcagcggtcgtatattttgtttccggtaagatgatctggttgagtgtgacgcggttgaagaaagagaatttttttgccaggaagggctttgagataatcagctttctttcttccacaaaattataaataatggcctgctgacctttcttatacctcgtataaaacagttcgaactgtaagttggagggcattcgatacgtgagtataccgcgtccccgtactccgtaggtataatcgcccgccagcaaaagattggacgccacacgggcagaagccatcacaaaaggcatggcctttccggtgggtatagacgacaggtactccatgcctccgcccactgttacattccggctgaggccatagttcatttgcacccttgaaaagatactccggtgtccatcttccaccataccggcgctggcagtatattcaaattcatgcaatggcaggaagttaaaagggatgctgatattttcctctctcgaccgttcctctccccaggggccataaaagcggagccgcaccacagagttaccatatacaagtggcacctggaaagtaaagaagccggctgcatctgcagttgtataatccaccagggcgttgttcacatataactccacggtccatccgggatctgtaaaatcgctcagggtataggaaccataagagcgcctgtaggaagtgggggtatttgtaaactgcacgcctaccaccggatcaaagatagatgccgtggatggcgtgaatattttacctgcaatgatctgccgaagggcgctgtgatcattattcacatagcgccaccggtagtattgctgccgttgatcaaacggcttgatcagggcgctgtcgtggctataaggcagctgctgctctgcgtagttattgtaattaagtgatacgctggtttcaccgcccagaacaacgccccccatagcaaggtttaaccaggtattaccggcgccgccttcagggcgttgtgtagctaccaccgaccaatcggccatcccgatactgaacatctgcctgcgggggccgatgatggtatctgctttcagttctccttttaaccggctgatattccggcgcatcatttcctgccgcatttccctgatagcaggcagctcctgcctggtttccagtttaacagagagcgagcggaaactaaatttacactgtagtccgaacacgcttgcaaacataccggttttcaggtaaagcgcggtttctgtgctcaccatatcatctttattcaacggcacgattttatcctggtagtgaatcacattgttttttttatctaccaggaacggggcgttttcattgataaagaaaccatatatagaatccatatggggtgaggccgtgtttcttatcttcagaaaattaaaaatatcggtgatagataagtaggcagaatcattgttgataacggcgggaatttcggcccctcctattccctgcactaccacgaaaacagaagtttcataaaaaacaggttccggctctatggctatggctttcaacggagctgcaaacagtatagcgcaaaagatcatccacaccggcgttacccggaatatgctgcgcaggcagcggaggatgatatttttgcttcctgttgtcatatccgttattcctggataaacgtgacgttaaatacgccgctgtacgagcccgatggattggatggcgggctgcccacggtgagcgttccgccgatcctcaccaggtttcttgccggtggtgtagcagttgtaataaatgagcttcctgtgctggcggcgcccacatgtaaagtgatggtaccaccgttgctcccggtgaggatgacatcgggtccgtttaatatggaaatgagtgtacccctgtttgcttctatttcaaaaatggcgggtgaaaacggataccccaggttggcctgcactacgctgccagttacggcgcgcgagccatcgggatagatgatcactgttccgccggataatccctggaagaaggcgccgaagatgagaccctgcgcggggtttacatataccgcaatagggcgcggaggcggctcctgcgcagatgcggccgcatatcccaacagcaccaggatacctgctactaataaccggtagccgaactgcctgagaagatccatatcttttatcatcctggtgaaaaacatctcaaaaaaattattactgattacttataaatacttttttagacactactttatcatctgtataaaatgaaacaatgtacattccgctgctatactgcttccctattacatgttgcccgttgccagtaacatcctgccgccacaatacctgcccgagcagattagagatggtgatgcggcatttttcaccgggtactttatcgaagtagccatacagtaccctgccaatgctataagccctgaacacgggttctgatgaaggcgaggtggtagttccgttgtgccggaatacgagcgaaaagcggttttcataagtacctgcatccaggtataccctgtactttgcgtactgctgcaattcctcggttttgccggttacggcatcctgcaggtaaatatgcaagcgctgcggcatgcgtgcaatttccgctgtattgaatgttatccatcctgccctttctgttttgaggcccagtggtattacatcggtactgtcggggaactgcggccatgcgttaatagagagccgggcgctgtcggccgacaatgcgtaaatgttaggcactgccggatcggtattcatcagttttaatgcatccattgttttttcgaaagatgcagatgcatcggcatcaaaataaaccactacgggatcagctgtcagcccatcgtcggcgaaggctgcgcccaacctgagtattggtgttgtaagtgaaacccggtgatacaccggtgagaggttattggttcttgcattattgtttaccgacaaggtacctgttaccggaaaagccccattggtcacatgcacaaaaaatccctgcatggaagcgatcatgttggtggcgatgccatcgctggatacgccgttgatgtaagagctgtaggtaccggtatactgatcggctgtacctccgttaaaatagtacacggcattgtcaatattggtgcggctccatcccgcggcaatgtcccaatcgaccggagaaggatacggatttcctaccaggttgaacccctgcgtatagggttgattgttattggtcagcatgggcgcggtaacggtttggttattcactacgccggtgatatccagggttgccggcgtattggaagtccccatttgcgcggtatatccctgcataggtgtaagcacaccggcggggctggtatacgccacccatccggaggaggtacggttttccacatagcggtaaaacgatgggaaggcagcgttaagattaatatcatctgccagttcatttacggtggccgcctggaaaggagagctgatgtatttatatccgaatgcggtgggcaggtatctttggatggtaacattaccggttacctgtccggcgccgctgccatcgatcagcgctgtttgcgtggcggtagacagcagtgtaagaaagccgccggtgttcagttgtccgctggttactttgaggatgccgctgatattcagtgtaccattcagcgttacaccgggtgtgttattgatggtcaggtgcagcaatgtattcgaagtaaaggcagctgcaggaattacctgtgcagcggccccatttaattctatggtaccggcagtagccgtgaaggcgccgctgttagaaataacacctcctatctggagtgtggcgccgcttacggttaccgaggcgcccgtttgtatcgttacattattggccacggctacaccggagttgataagcggatagttcaccaggccggttggaatagtaacattagtagtgctcaccggtatggcggcggaggaccagttgccggtaatataccagttggtgctcactgcgccggtccatatagcgccggtggccagctctcctactaccaggtcgcccaatgcggttaacccggttgcctgtatggaagccggttgcggggaactcacggcggccagcgaccaggaagttccgttataccttgctactttaaaattggtggtaacagcacctgcgtctacatccgccgctacccagttgagtgttacagaaacggtggtaaaggtggcgccgctgttggtaaaagcccagtacctgtttactttccggcttacatttaagccggaggtcagcaggtttggatggctggcagcgaatacacccgccagtacatcgccggcggcgcttacgttggcgtataacgttgttgccggtgtatagttaaggctgtcgcccagttcataagtgcgggtaatattggtaccggcagcaacatttttttgcaggcggccgtatacccatccggtattttgtgcggcgccgctgaccgttccggtagcggtaacaattacggcgttggtggcgccggtacggatctttcctgccataaatgtaagcgcaccgtttatggtagcatttgtggacagggtcaccagcccggtggctttatttactttaacatgattaaaagcaccggtagaagaaatgttctggttagcggcgccattaaaataaatagtagaaccggtgttggtaaatgttccgccggtcatgctccagtttcccctgagtgtatccgtaaaacttcccggcacaaacgtgccgttgctgagtgtaaaatcattcaggatggttaatggtgcagtagcggttttggtacctgtggccgagatggtgaggttaccatatggtgtaaccgcagcaacagtttgcgtgctgcctgcatattccacggtgctgagtgtatccagctggtaaatatcaaaagccgggaggctgtaaatgcctcttacgatgaggcgtgcgctgtcatcgatcgacattttgccgccgttggtggcatcctgggtaatggtggagtcgccggtatcgagggtgccgccggtgatgtccagtgtggtcatattcctgagacttctggcaagtgtggtggtggcggcagcatctttatgtacctgcaactgtgcgaggtcaaaggggctgccggtaccgccgataacagatggtccagtgccggtcatggcgggcatgcctgtggatgcatccagcgatccgttgatggtaaagttgtgctctatattaaaatcggcatccgaggtaacggcgccattgatcacgaggttataaaaggtagttccttcgctgccggttaatacgccggcgggggaagtcatggtaaaagtagaagtgccaccgttcagggtgccattactttcgagatcgcctgcaaccgtgaagttgttactgcccgcattaaaaatggcgttgccattaatgtgaaggtccccgctgatattccagctggtagcaggcgtaacaccggctgtattggcgatggtcacatctgtaagtgtggtgggcgagcctgaaacggtgagcgctgcgctgccgccgaatattacggagccggtactggaaaatgcagtacctctgagggtaatgttctgtgctgcaaaaggattaaaataaagcgtaccggtgctggttaccgtaccgttgttggtaaagctgccacggatagtatgcgtggaaattccgccgttgaaagtggcgccgttgctgatattaaaggccaccagtacggtccatcccacgcttggattgatgccggcggtgttgttcacattcagggtggcgaaggtaggggcactggtagaatttaataccggtgaaacgttaccattaaagttgatcacgccgcttgaattggaaacaatggcatttaagaagcggatggtttgcagggaggtgccggtaaaggtggtcacgccgttgctgatcagtgatccgctgttggtgaggtcgccgtttatggtggcagagccactgccaccgtcgtacgaaccgccggcaactatctgcaataaatcattgtaagtgatatcgctgccggctactgcgtagctgccataaacggtaagcctgctgaacgtagtatttccggtaattgttttgccgctgccgttaagtgttacggtccctgtaccgccattaaaagtgccgctgttggtccagttgccatagaggttgacagtaaatgtgccggcgctgaaggtggcgccgctgccgatcagcaaatcgccgtttatggtggtattggcggcgagggttttagtgccgctgccgctgagggtaagatgtccgtaggcaatatttcctgccacagtttgcgctcctgccctgtagtagttaacggtgctggtgatgccgggcaggtactgagagtagtttgccggaaaattacctgcgccgccgacattcacggtggcgccgtttgcgatggttaacgatcctcccggagaactacggttagccgtaaacgttgccagatccagtgtaccgccggtcaccgacaggttgccgttggtagttacattaccggtgagcgtggcagttcctcctgatttattaatcacaaagttattaaaggccgtagcagaaatattttgtgcgttgccaccggtgaaattaacggtgccggttccgggagtaaacgtgccgctgttactccagttgccgtttaaggtgactgtggcagctcctccgttcatagtagcgccggcactgatggccacatttcctgtgatggtggtggctgcgttgatgctcaggtcaccgctggtaacggtgaggttgccgtttaccgtggcggcgctgttgatttgcgcactaccggccgtttttgctatactgagatgattataggttagtccggctaccgactgaatggaggagccattataaactacagtaccgctgccggcagtaaacgtaccactgctgtagttaaagctgttgcctatattcaatgcgccggtaccggagaaggcaatgcccgcaccacccgactgggtaacagacccggtagtggtaacgttaccatttccgatgtttaattgtatgttatgaccggcagtgccatcgctcaggataatgttcccatttaccgtgagattttgatcattcacattaatagtgtgggtagcattagccgaccataagccagtgatattaccctgtgttaccagcgatccaccggcggccaatgtaatcgtggctgcctgtgcgctgccgaaggaaatgcttttcacactggcgctgttgctgatgactggttggttagtgaaagcgatggtgcctatttcagcgatatcattcacgccgggtggccgggaagggctgccctgtgctatagtccagttggcggcagtgttccagtcgctgctcaccgagccgttccatctcaccacattagatgccgccgccaacgtgtatcggcccgtaaatgcagccagcaggcctgtttgctccacataattgctggtggtgttgctgcctgaatttccgtataaagaccagcccgagccagtgttgcgccagatgctgagactggcttccgcgttaccgttcagttctgcatcttcatagtgaaaacgcaggagcgtagctgccagcgtgatgccgctggcggtaacgttatactcccggtttatggccgcgccggaagggaaatcggctactccctgcggggtgacggtcatcgtaacagacgcggatgtagtaacacccgtaagtgtgaatgtattattagggctttcaaaagcataggcggtacccaatacaaaagtgtgggaatgctggatgctgcccagtatgataccgttgcctgttctgttgcctgtaatggtaactgtattggcgccggtgatcattgttccgctggtcatgttcagcgtggttactgaaatattatttaacagggttacctggttaacggcgctggttttattgagggtaaggatattaaaagtagtggcgccgctcacggaagtattggcagcgccgctcagtgttacggtactggtggcaggcgtgaaagtaccgttgttgatccagtttcccaggacagtgatggattgactggaggcattgaaggttgtagccgatgcgatggtaaaatcgctgttgaccaccacagcgccacccagtgttttggtgttgccattacttacgatgagcttattataagtaccggcagccagtgtttgggcgccggttccattaaagtttaccgtattgggaacagtggaggttacgttgagcgttcctgccgtaatggtgtatacattggctattcccagcaccgcgttggccgatagctgcaatgctgttccgttgagggtaacgttgaacaggttggcggtaccattcagggagctgctgcctgtaaaagtagcggtgccggcactggcggtgaaagtgccggaaacatccaggacgttgccgatggaaaaactggaggaggaggtgatacttcctgttattgccaatgttcccaaagtgatggtacctgcgcctgacaatgttttccctgcaccactcatggctacgctgccggtagtgttattcaggctgccgcttacagacaggttaccggtgatagtgatcgcatctgctgagcttacggaaccggagacggtaaggttttcaaacgtaaggcccgtaccactgattgttttggttgcgccggtcattgtaacggtaccacctgtaagatgcgtgaaggtgcccggggctgtgctgctaaaatttccggagactgtaatggcagtaccggcagccgcggtaatattggtggcagcgacggtgaggttattgaaattatgtgtgcctgttccgctgatagaagcacctcctcccgccaataccactgttcctgtaccgccgctgaaaacaccattatttacccaattggaagaggtggcggtggtgaagcttcctccgttgaaggtagtagctgcgccaatatttacattaccgctcaccgtgatgttggaagcagcggtaaagctcacggaggtaccgctgccaatggtcgaggtaaggtttcctgatatgggaagtgccgtagcaggcatggttttaatagctgccccgctgccggcagacagggtaagatttccatagggctgtaccgctaccgactgattggtaccattgtattccaccgtactggtaaggccaagtgaaacggtagcatagttaaccgggaaggtgttcacaccaccgatcttcaggatagcattgttgactacggttaaaccgccaccggccactgtagtgcccctgttggcggtaaaggtggacaggtcgagtgtgccggcaagcacttctattttcccggctgttgcagtagtcgcattcagtgcgtttagatttcctcccagtgtttttatgccggtgccgctgatgcggagggtggaataggtaagggtgttcctgacggtttgatttaccagcgtaccgctataatccacaatactgccggcggcaagggttactgtacctgtgaggccatagttccctccgatagctgccgcttttacgtgtaagatgccaccggcggctacggaggtggtggcggccccggaaataagcacgggagtggccacatctgccggaacgaatgtgccgttcaccgcaaaggtaccggagacggtcatgttcacattttgcgtagtggtactacccacgccgatggtgagtttcctgaaagtggtaaccgaggcgccgcctatagactgtgtggttcctgcaaaggttactttggcattggtactcgaagtgctgtaagtgcctgagttggtccagttaccttttaaagtaagggtaacgccgcgctgggaaatagtgctgccggaaccaattaccaggtcgcccgccacggtgaggctttgggaaatggttaataccgcattagtgcctgcgcctacggtaagtgatttacaactggcgctgtagctgatcacggggtaaaatatcccggtaaacgcggcatcgccaatgatagcgtccacattggcattgggtacaccggcggtccagttggcgctgttagaccaggagctgctgaatgttcctttccatcttgtttgcgccgataacataaccgggaagagcagtaacagtatcagcaggcctctgccgcaggcggacatgggtatacgggggacgccggaaagaagagccctgattatcctgatgtaaaactgatgaacgaaccaatgtacaatcacttccataggagcgttatttgatggagactttctcccggctaccgtaactgcaactcggcctgggccagttgttctgttgaagcttttgatttggtgatatatgctacccgtaatttgccggtatggtaattaataccgggtttgttttcaagtggaagatgaagataacgctgtgtgtttggtgtgtatacagccagccccctggcgactcctacctgtgttatttttccctgtggcgacacataatccactgtgagatcaccgtacacggaagagttacccagccggttgaataatacattcaggcccgggtcttttgcgaggtcaacagagaggtctgacaactgcacgctggcggcggtttcccccacccgtataattaccgggatggtgataccaaaaacgggggtgagctttacattgatgccggtgctgtctttaggcggatcatcttcaccgatgggtttttcatccggtaccgcccggaaataaagatgcgaacggtattcaccgggttccagctgactggccccggttaactgcagttttattgcctgtgcttcattggggcctagtaccacgctccggggaaagaagcgcaggtatttactggcgaactgttgccctgaatcaggttcgttgatctgttgaaaggtgccgttcttattcatcctgatttcaacaaatgaaataagatacctggcggtatcttttcctgagttcgcaagattcagttcttctgcacgtttcgtgccttcaaaaacgacccgtacaggggttacgagcaggttgccctgtgcgcatgtttcctgtattgccatgcaaaaacatatcatacatatgattacaaaatagtaaggatatctaacgacggaattattcggtggcaccgatacattcatgggttcatgctttggaataagcgtgtagctgcgcgcttcgcagctacacaggatatgattaaggttgttgtaaagcgtgggcggttatgtgttataaccggttgatcagttgtaattaacagttacatcaaagggggtagctgaaacatatgttccggcagcctgtgcggcacttacattcagggtagcgcccacattaagtgtttgtgtaccggcagtaagtgtaccaactcctgaagggtcactggtgaaatttgtaaccgtcatcgtattggatccactggtgatagtaagcgcagtagaaggcaatgtaatgctgtaggaataactgccggtacctgttacagtaaaggaagcggctgtaatagttcctgtagcagtggtgggcagtgtaacaccgcccgtagcgctgcgaacgcctgcgggagtaagcacaaccgttcctccagtggttgactgtactgcaacgttaccaaaattcatatccacatctttcacaatgctgatgggggtcacaatagtagcggtagcagtagcggaagcggtttcctgcgcgaatgcgttggttgtaagggctgcaaatacgagcgtaacggcggaaataagactagttcttttcattctcggctgttttaatgatgagggaatgtatttgaagattgttttaggatacagaacagtaaaatgactaacgtaccgatcacaagctacagatgtcaaacagggctaaggctttcataatccagtcattataatcacgacaatttctactatgaagataatacaaaatatttagaaccgtttactccgagctgattctttatccaatatttacgtattaatttttcatgtggtttgctcagtccgtcattcagcggcttccttattacgattttcatataacgccgatctgtatctcttcgccagcaaacctgtggccagcgccggatcgattgcagctactattacgcccggtttaccatattccccgtgtgctatgcaggtaccatcggggccaataatggagctggccgagtcggggtatgtaaatgcataattagcgctggcgaagtagatggtattttccaatgcgcgcatcatcatggctttctcgtagtaggggttattgatatggccccattcggtgagtagttcaccggtagtattgctgccggtgcaatgcgggtgaaatactattttagcatcttgccgcgctgcccaccggacggattcgggataacggaatccttcatgacagatcgtgataccaaactttacaccattcacttcaaagatactgcgtgcggtaccgggtatccagatattatcttctgtgggatctaactggtttttggtctggtatcccaatacttcaccggtggctgcaatcacaaaggccacattcagcaatgcttctccctgatgccagtccatgggcataataacggcgatggaattttcagcggcgagtttacccactttttccagcgcctcctgcaggttccggggagaacgttcttcttccggaaaacccatacccggatagccgggaatataggactccgggaaacagataatttccgcctgttgttttgctgcctctcctatcagtttttcagcccataacaaaccgtcgctgatagatgttggaggtggtggagcagccaatgctattttcataagatgcagattatgacaacaaagttattcagaattattaaagaagaggctgactttaaatgaccggtacccgataaaattccggatttgtaaaaagtaattccggattccgtaaacgaaaattaagggaagcgatcaatctttggggttgaattatacctgttaaataatgaatataagaaccgcaaagcgttggtttctgtggcataaatggaccagcctcgtttgcactgtttttttactgatgctgtgtttaactggtctcccgctgatctttcatgaggagctggatggactgctggagaaacaggtagcagctgaaataccggagggcacgcgtaaactaagcctggactcccttgccgtacttgccggccagcaataccccgcagaaaaaatacggtatattttctgggacgagaaagatgaaaacaagatcttatttgacctcgctgccaaacccgatgctcctcctgaaggaagcaggtatgtagcgctcaacatgtataccggcgccgtgctgggcaagccaactactgatggattaatggacgttatattgaagatccacatcaatatgtttcttggtattggcgggaaattatttctgggactgatgggcatcttattcattattgccattgtttccggcgtagtactttatgggcgtatcatgaaaaagtacgacttcgggatggtgcggaaatataaatcgaaccgcctgaaatggctggatacccataacctgattggaattgttacgctcacctgggccagcgtggtagggcttaccggtgtgatcaacacgttgtcggatgtaatccttggcctgtggcaacaggggcagttaaaagagatggtggcgccctacgcccaacagcaaccgcttaccggcaagctgagttcactggacggtgcaatggcggtagcgcgaaaagcagcgccgcatatggagccgcgcatcgtcacttatcccggtaccttgttttccagcaaacatcactacgctgtatttatgcggggcaataccgccctcacctcaaggttactgatgcctgcactgatagatgccaaaaccggcgcgcttaccgatgcccggcgcatgccctggtttgtaaacaccctgtttttatcggagcccctgcatttcggcgattatggcgggatgcctttaaaggtcatctgggcattatttgacctggctaccatcattgtattaattaccggcctttacctgtggtttgcacgcagaaaggctgccaacctgcaatggagcaggctaaccgaaaaaactgtataccaggatgaagaatagcgcttttttcagattatggggaaaaccgctgctgatggcattgctgtcgatagccggattaattacagcgctgatgggcgacggttactgggatgtattttcctggatagcgctggccatacctgttatcatcattgtgcgcaactattattttacggggaagcagggttaagcacctgataccttcgttattacgataaaaaaaaatcggccaaccagattgactggttggccgattttttcaatgctattttgatgattacttcaatgtgatcgtgcttacggtagatacttcccctgtttttactgctacggcagcaacggtagtatcttttaagataccattaccggcaatagccacattataggtacctgcgcttaagcctgaaattacataggcgccggttaatgcgtccggtaatgcggaagccacggtatcagtgttctgaatagcatatacgcctttcacctgcagtaatggtaacgcaattcctttgatagtaccgctggttgctgctgtataagtacggatcactggtttcaggatgtacttattgcttccggtggtaacgatagagcgaccggcatcaaaatcgatccagaggcggtattcgatgtcggctaccaggtcggcatgcacattcagttttaaacctgattgctgagcagaaggcgtttccagcgggtgggataccccattcaataccacgctgttgttggcgcccaatatcaaccggatctgtgaaattttaccggcgggtaattcttttgatgccagtaaggtgtctaatccatttctgaaatcaagcaggttatacacgccgggacgtgccaggggaacagatacccaacctgcacccgtttctgctgcatcagctgatgcatttacctggatatcctggatatcgatgttcacttcatcgtaaatagccggatcatctgtcaggtacactgtgagcttcgactttccgctgttggaagtagattcgtctttgctgcacgcactaaagaatagcatggatgcggaaaccaccattaacgtggcgaagaattggtttttcatgattcaagaattgaataacagttttcggttaaaatttgaatttgagttgataaagttgacaacagatagtgacagatttcgcgtttgagttgtaagtataatcccgggaagacaaaaactgtaccggaaacagccataccggtggatgagcgttttcctgtcaacagaacggccaggcaaattgcctggccgttctgttgatatatgcataaacagtatttcttatcccttctttctcaccagctttgcttctttggtgtccattccatagaggtcattgaacaacaatttgaaggtgcctaacgactgggcgcggaaagtaatttcagggccaaaggcatagagcatgccggcgcccacgggggcagaaaatgcggccacgccatctttcaggtatgtttgtccccatgcccagccgctatgcagcggtttatctgtggaaaaccaggcaatgggtttaattcctttatcagcggcatctgtatccaggcggaacacgggactgttatcgaagttcacatctccaacagcgggaaggccccatgcggcggggtgtgtgctatcgaaagacacctgcaggatgcttccgggtacaaaatactttgtaccgggtaatggtttttccttgccggctttatctgtttcgaccaaggcattgtgcaccggcaggccgagatgataggccaggttggtgctgctgccgatcgtgatcacggttccgccttcttccaggaatgtttttatctgcggaatagatttctctttcgtgatcttccctaacaaatgccggtattgttccgggatatctgcgggcgaaggatctttgggggcatagccatacctgttgggctctgctcctgataccggtggaatagcacgggtagcgaagatgatggcatcgtatttactgcggagattaccggtatcgatatcctgcgggtatattacctcgaaagggaaatgatactgctccatgatccaccgcatccagccggagggcatagagccgccgtaagtgtcccataatgcaatgcgcatgggcgccatactcactgttccggccgggcgtttgctgataccggtggttttaagtccgagggtattggcggattgttgcaggatctcttttgctttgccatctgcaggcacataaaagctacccgcaacggctttatcgttgccggctactcctttggtaagacggtatactttcacgcctgctttcataaggtcatttaccgcgatgaaggcgttgttttcccgcgcactcaggaggtagccgccggcagtagccagcgctgctttgggaggtgattgtaaagcgccatagggcaactttataaagggtccgtcgaagctatccaggatcctgtcgaactgcacgcccatttgaaacgccagtgtccatccggcagcatcataaggccggatgggaggaccaccaggatactgaaaatcgtttgggtggtcctgtggttcaaacatatccaatacatgcgggcggaaggcctggtttgtttttacgatgtaggagccggcagggtattgtttaccggctactgtgaacggtgcatctgccttctgtacctgtatgccggctttaatgagggcattgataaatttcacagcggtggggaaatcggcctggtcggcggggaggatgtatccgcggggatcccttccggcaggatctttaaacaccgcatcataatacttcatcgggatattgcttcccctgcgcatccatccatacggatcgctgccatcgtttttgtcggtggagtccacgttatcctttttaaaagcagcggtaatggcttcggagcgtttgggtgataatgtccacgaatcctggttgcctttatcgatagcattcttccccattttgtaaatattgaaaagcacttcatcacgttgtcttgctgcgtaatcgagcaccgcgtagttgagcgataccgagtaatcaatcgagcgtttgaagcgccagtcgttttgcggtgttaccgggttcggggtagcgccgttagggatcagtcgttgcggcactaccggaattttttccggtgtagggttgccgataatttccgtaagcagcccgatcatgttatgatactgcgtggttgtgcgtaagccgccattgtaccaggtagagaagctggagccattgaggcgggtgtagccgggtttatcttccgcattgaggcggttatacatcgctgcgccgagtgcatcgatgccagtgatcatcagcgggtcaaagaaataattgaaagggtcgcggtaaggagggcctgcgagtacggatccttccggcccgcgttggtggtgattgtacataatttgcggcatccattccaggaacaactggcgtcccatgttcacgctttccttcatattcatgatgtagaaatcgcggttattatcgtgcccgatgtacttctggtatagtacgggcagttgatcaaccgtacgtttcagtgtatcgggattccgcatgtaccagttggacaccagctcctggccgtcggggttggcgtgtgtcatgaggatgatcacattgtcgagaatgcgcatggtttccgggtctttccggctactcagttcccaggtggtttcaatgagctggtgagtgcctactacttccgtggcgtgcaagccgccatctatccataccactgcttttccttccgcggccagttcccgtgcctgttcagtggagatgccttctgcgcgtgcgagctgttgtgatatctttttatatttttccagcagtttaaggtttgcgggagaagagatgatcagcatgtactgatcgcggccttcttctgttttaccgatgtccaccagctgtacgcggttcgacgtggcagccagtttcttaaaatacgcggctgtttgcgtgtagttagccagctgataatcgtccccgatgttaaaaccaaaatgatctttcggggaaggaatattttgtgccatcgcggttgtgcaatacaatccaacagcggtgagcgtgacaagcagtttatttctcataacatttactgattgagttatttacgataatccagtgcgggttttctgtcgcccagcattgcttcatatttgaacccggttccctgtcttttatccagttcttcttttgccactttcagggtttccgggcttttgaataaatcgtatgcggtgagcgccatggttttggcggccaccatcatgccttttatgccgatgctgctgccggcggcggctacgttctgccagctgtgaccagaagatccgggcacaaaggtggccgttacaatgccggctgtaggagctacccagcttacatccgccacatcggaagaggcgctgccgccttcgcggatcattgcaaaaggactcacgcgggaagtgaccgtatcaggattgggagtgttatctttttccacgaagctggcctgaatcttttttgcaaactccttttcttccggggtatagctgaaaccgcccacctggtggagatttttatccattatttgcgacagggtaatattgggcaacatgttatacacccctcctattacctcataatccatgcgggtaccggttcccagcgcagcgccttccgcgcactttaccagccgttcccacacgcttttcaccactttcatttccgggtgccttacatagtaatatacttctgcaaatgcaggtactacgttgggagcgtcgccacctttggtgatcacatagtgaatgcgggtggtagaaggaatatgctcccgcatcatgttcaccatataatccattgcttccacgccatcgagggcggaacggcctttttcaggagaggccgccgcatgagccgccgtgccataaaacctgaactttgcgttcttattggccagccagggcgacactgcagcagaattctggttaccaggatgccaatgcagcactgcatttacatctttaaataacccctcccttaccatgtacactttcccggagccgccttcttccgcaggacaaccatataaccggatcgttccttttgcaccgctggattgcagccagtttttcacactgatggccgccgccacggaggcggttccaaaaagattatgaccgcaaccatgtccggggccgccgtctttcaccgggtgtttttcaggaacggcttcctgtgacagaccgggtaacgcgtcgtattccgccagtatggcgattattggttcgccgctgccatagctggcttcaaaagcggtgggaataccggcgatacccgcttttacggtgaagccctgttgctgtaaagttgtttgcagcagtgccgcacttttttcttccaggtaacccggttccgcatagctccagatcttttttgcaatggaatcgtaactggcggtatgctgatcaagatacgtgatcatggctgctttatctttctgttgttgcgctgccgcggaaaaagcgaaaccgcacattatgctgctcaaaatgatttgctgcctcataaaattatttatacaattggttaaacagtaatttgaaggtactgtgagattggccccggaacgtgatttccggaccaaaggcatacagtttgcctttgcctaccggcgccacaaatgctgcaatgccatttttgaggtactgctgaccccaggcccatccgctgtgtaatggtttatcgtctgaaaaccacatcagttttttaatgctggcggtatccccggtggcactcagtttaaaaacggggctgcgctcaaaatacacatcatttcttgccgccatgccgaaggtttccgcaacggtagtatctatatccgccagcaggagactgcccggaatatagtatttggtaccgctgagtggtttccattcatttttgctgttcttttccaccagtgcattctgtaccggcagttgcaggtgataggccaggttggtactgctgccaatggtaacaatacggccgccgtcttccaggaatttcttcagccggggaatggaggtatccgcggtaattttccccagccagccgcggtattgcgttggcagttcagctggtttaggtggtttggtttcaaatccgttgcgtgtctttttaggtttgccggtatcgggtatggcgccggtagcaaaaatgatcatgtcgtatttgctgcggagctttccactgtcaatagcggaggtataaacggattcataagagaagtgatactgttccatcagccagctgatccagccggcgggaatagatccgccgtagttgttccagatgccgatgcgcatgggcgctactgctttcaagccggcaggtttgctttcactaacggtaacgggtataccaaatgaggccgcatctcttgcgagcagttcatgcgctttagcagaggaagggatgtagaagctacctgcctctttaacgccaacgggcacacgaaatactttcacgcctgctttcagcagatcgttcactacgatgaaagcattgttgatgcgggcatcaatgaggtaacctttgcccatggccacttcctgctttggcggggattgcaggctgccgtatggcagtttttcaaacggaccactgaaggcttcgggaatacgatcaaactgtacacccatctggaaggccagcgtccatccggcggcatcgtagggccggataggcggaccaccttcatattgaaaatcgttcggatggtcctgtggttcgaacatgtctattacatgcgggcgaaaagcctggctggtttttacaatgtatgagccggcaggatattgttttcctgccactgtaaaaccagccgtggctttctgcaccgctatgcctgattgaatgagggcattgataaacttcacggcggtggggaaatccggctgatctgccgggatgatgtagccgcgggcatcccggcgtccggggtctttcagcacagcatcgtagtatttcaccgccacggtatcctcccggccgaaggagaattcgccaccaccttctccttctgtaccgggttcggattttttattgttcttattggcaatttttatgctgtcgatatagctcgggtagaacgtccagttgtcacggtttcctctcgcaatagcgttggcgcccatgcggtagatattgaacagcagttcgctgcgatagcgggaggcgtagtcgagtacggcatagttgagcgatacggaataatcgatcgattgccggaagtgccaccgctgcggtgttaccgggttgggggtagcaccattggggatgagccgttccggtaccaggggtacattttccggtgtggggctgcctattatttccgtcaggattcctacgatattatgaaagtagggcgtagtgcgcaagccgccgttccaccaggtggagaactgtgagccggcgcgctgggtatagccgggttttccttccacgttgagccggttgttcatagcagcgcctacagcgtctatactcgttacgatcagcggatcgaacacatggttgaagggatcgcggtatggcgggccggccagcacggagcccgcggggccgcgctggtggtgattgtacatgatttgcgggagccactctacaaacagctggcggctgatgttctggctctcttttatgttcatcatgtagaagtcgcggttattatcgtgtcctacatacttttcgtatagccgtggtatgttagtagctcttttgctggtatcgggttcgcgcatgtaccagtcagacaccagttcctgcccgtcggggttggcatgtgttaagaggatgatatcgttgtccaggatattcatggtttccggatctgtacggcttaccagctgccacatggtttctataagctggtgggtgcctactacttcggtagcatgcaatccgccgtcgatccagatgatggacttcccctctgcggccagttcgcgggcttgctggtcggtaagaccttccgcgtgtgccagttgctgtgagatggttttataccgttccagccgctttatattttccggggaagaaacgatgagcatatactggtgacggccttcttctgtaagcccgatatccaccagttttgtacggggagaagccgacagctttttaaagtaggcggccgtttgtgtatagttggccagtttataatcatctcctatattaaaaccaaagtgttctttgggagatggtacctgctgtgcccatgcgccggctgcggcagtcagcaacaggagtagcaggccgtaaaatttcctattcatacgggttatcagtttcagttgatcaaaacgggttctctattgttttttaaacctcacacctacgcggcagtcgccgggttcgcctcttgcttcatcgcagatattgttgaagaaggtgacgatcctgcggccatcggccaggttgaggataaatttgaacaaaaagtaatcgtttacgcccacatttgaaagacttacatgattcagtgttgccaattgcgctgctgtaaaggaatacgttttcgggaaggtggtcacggtttcatataaatgatcgttggtgcctactatgctgggcaacggaaactgtgcgatgttcgtatattggttaccgggagaagagatcactaacggataagcaggtacgctggtttcggctttattatagctggtatacacttcaatagaagtaacggtttctttcccgaatccttcccagctgagggcaaaggcaaactgctgactggccacgtccggatctttcaggttaaagaaagctactttgcctgcctgccgcgttggcagggctgttttggtagtatctatcgtaactaccggcacggcggtataggtatatccctcccattcgtacttcacctttttacaggaaaatgcaaccgatgaaataagcagtatggcaactataaaatgtttcataattataattttagtcccgtaaaattttttacttatttatcccagaaaaccggtgttgtttgttgcgctacctgcaagcggccggcgtcatcccctaaactggtattggcggtaagctctgtttctgaataatataggcgcaacgggaaggtattgagcggcgacagcggcgtgcgcagcgttggtaaaccggtacggcgatagtcgttatacgcttccatgccattgccgtattccgcgatgtatttctgtgtcatcaccagttccagtttaccggcattgctggcggcgtcatatttcaccagcaggcctgcggcaaagtcggcgatggtggtggtggttaatgcaacgccgccattcgcggcggcataggtgctcacgctgttgagatgtgcggtgataccgtctttaaacgcctgccgggcatcgtcgccggtgttgagcgtaagggctgcttctgcacggatgaacttcaccatggcgttggtgatcataggcatgatgcctgcgccggtgccatctgtagggcctactactttgagggcgccggtggcattggtattggtaaggaattgattggtgacgggcatattatttaccggtgcattgtcgtacaaaccgccggcgggatagataccgaaggtagagcgccggttcagatcggccggtgcggcggtaccatcgccggggttgcggccatagtagccgttgctgttggccgaattatttaatcctgccgtggcgttctggcgaatgatgtagtagcgcaaccggggatcgtcgttgttaaagagcaggtcgatcagcgactggctcatataaaacgttttgctgccctggtattccgaccggtgccagggatgcctgttgttgggattttgcccgggcccgaagcggaaggtaaagtccgatgcgttggtattggtggcgccaccaatcagcgtggccggatcggcgatcagcgcctgtatagcggtagcggatcgtgcaggattcaccaagcggatctggttatacagctttagcttgagcgagttggccatcatgagccaggagcttttaagcccgctgtacaggagatcggatgtagcgggaaccagtgtggtggcagaaattttcccggcatcaacagctgcttcgtcgatcatcttcaaaagatcttcataaatatccgcacctttttcaaacggcgggctcaccgtttcctggcctttttgtgattgtgaataaggaatatctccccacatatccaccatcaggcttacgaggtatgccttctccagtttggcgatggccacgtagccccattgttcctgtgccgtgcccgtttttataatagcctccaggtcgttcagcgtttgtgtgtaaaacccgtcccatgagtcgttgaagctggtgccctgttgctgcagcctgctcaggccggaggagaaaacggtgtactgcataaaagtggcggtgccgctgttcagctggtacatgttggctgccattgatacttctgtagccggcagcaataacgataactgggcagtggtgggattgtttggatctgtattgatatctacaaattttttacaaccggtaactgtgaaaacacctgccagtgctattgtatatgcaatatatttaagtgccatcatcatatcaggttttatgatcagaaagaacatttcaggtttacaccaaagcgacgggtggtgggtactgccaggttatcgtatccctgcgagttaccaacgccgagcgaactgacttccgggtcgaagttggtatacttcgggaagttgggagcgctgtaccagaggtttctgccggtaacagaaatgaaggcagacccgaaaggtgttttacctaaaaagcttttgggaagttcatatcccagcgccacttcccgcaggcggaataccgtggcatcgaataccgatccttcattgataccgccgttgcctgggcccatactgctgctgaagaagtgatcttcaaaagacagcgccacgttattcgggatcttattgcctttgtcgtccagcagtggcgtttgtgtattgatatcacccagcacgcccggcgacacgatagtgaattcgcggttttccatgtcgcgggtaacgccgcgcgacagcatctccgctacggtgcgggagtacagttgtccgccttgtttccaatcgaacaggatattcagtgagaagctgcggaagcggaaagtattggtaatgcctaccatgaaatcgggattgggattaccgattgctttgagtgcgccggagatcagtggtttgcctgtgttgggatctatgagcacattgccttcctcgtcgcgtgcataggctgttccctggataaggccgtatggttggcctacaacgtgcacgctgctggtaccgttggtgccgccatagctgaagcgttcatatcctcccaggtcgcggatgatgttcctgttgcgggtaaagttggccgagatatcccagttgaggccattattggattgcaagggcactaccgttaaacctagctccacgcctttgttggtggcttcacccaggttaaggatctgggtagtatagccggaagagggtgcagcagtaacctcgaagatctgcgaggtacttttcttattgtaccaggtaaagtcgacgcctatacgattatgaaagaactgcagttctgttcccagttccagttccgtaataaactccggtttcaggttagcgttggtgagcaggttggcctgagtaaccacgttatatacgctgccacctgccggcgtaaagggcagtcctacgtttgcgggcgtagtgctggcgccgaggatcgggttgatctggtaaaagttttgtgtctgataaggagaggcttcgttacctaccttggtgtaacctgctcttactttaccgaagttcagtactccttttgggaggtgcagcgcttctgtgaataccagtgatccgtttacaccgccgtagaaatagcttttgttattggcgggcagtgtagaggaaatatcgttgcgtccaacaaagttgagggaggcaaagtttttataatcaaaggtgatgtctgtaaagaaggcgtagtagcgttgtttcaggatgttcctgttattgatcagctgtatcggtgttactgagctggtgttgttcatgtctatcaggtcggccacgatgatattatccccgtaaaatgctttcctgtctgtaagccgctggttcacattgttaccaacgattgcccgcagcgatatatctgatgtaagaggtttggtggcggttaccagcagggtgttatccagttcctggcggtaaatattatctgatgtgatgcttccgttgggataggaagagctgcctttaccgcgtacgctcattcgcctgtcggtgtatgcgttaaagccgatggtattctgcacattcagccagggcagcggatcgaaacccagtacgaggttaccgtagtacctgtccacgtcgctggtagaaggactgtgtttcactgaccagtagggattatcaattcccgtatagtcgtatacgttactaccatccagcgggttctcgtaagggtagttagtgagatcgtagctggttggtacgtacatgagggtagacatgatagagcctgtgaggccgcctaccggtggtgttttttgccgggtggtgacgtagttgatagcgccgctggcatagaatttattttccagccggatgtttccgccgatgttgacagaggtacgggttatttcattgccgggtactacgcctttattttttgtgttggagaagcctgcgttgaagtttcctttttcgctaccggaagagatggtgatggcattttcgtatacgctaccctggcggaagaaatttttcgcattgtccttcgcatacgatttgtagggcacctggatgggcgttacgccatctgcttcgtagaactgcgggaacacggcggaagagaactgccgcgtgagctgatgcggaacggtagcgcgtgtgggcaggatgctttccactccttcaaagggctggccccaggaagcgtataccccttgccggtagtcgttgttggtaccttgtccgtatttggtttgataatcgggcaggccggacacctgttccacggaatagccggtgttgtaagtaatttctgtgcctttcctgcttttctttttacctgctttcgtggtgatgatgatagcgccgttagcggctcttgatccatacaatgcggcggcggcggcgcctttcagcaccgtcatggtctggatattattcggatcgaggtcgaatgcgcggttggtaacgcctgcgccgcctacggtggtcgcgcctacgttggcgaagctggagttatcgaagggaacgccgtctaccacaaacagcggctggttgttgccattgagtgaggagttaccgcggatggtgatattggtaccacctccggctacgccgccggcagattgtacattcacaccggctactttcccggtaagggctcttacggggtccggttctgatttctgtgccagtttatccgaggtgatggtgcttacggagtagcctagactgtttttctggcgggcaattccggcagctgttactacgaagtcctgcaattgttttacggcggctttcagtcgtacgataccggcgtcagcggcttttacttcggtgatgctgtatccgatggcggtaactactagcgtggcgccttctttgactttcagggtgaaggtgccgtcgcctgccgaggtaacgccattgccggtacctttttccatgacggtagcgccggggaagggatcgcctgtttcattcagtatttttcctttcactacaatatccgccagtgcgatggaggtcatcatatccgggctggcggtacgtttagcggcggcgtcattatctgtaagaatgatatagtcgtcgttcactacaaaacctatttcgaggcggccgaggagccggtcgagcaccttaccgagtgcttcctggtcggcccttgcggatactttcctgtcgagcgcgatgtggctggagctatatacaaatttcacttctgctttgctgtggatctggttcagcacacctttcaggctcatatcatctgcctgcagcgatattttcctgtcgagaactccctgggcgtgtgccgcagcgggatgcgtaataccatagagtaatacgcctgccatcaggttggccgccgttactttcttgcatttggacaggaaggcatttgtctttaaatttatgagcatagaccttgtactttgttagatttcggaaagaatttgacaaaggaattcccttaccgcgctgtcacgcggtgataaacagggctatttatcataagctggcggggctgtcacccctccggcttttttagttggaaatgatgttagccatgatgttagatttttgtgtttgactcggtttgattgtggttgataacaggttcatttttcactttttttgtttgagtaaaatagttttgccgttgatcccgaagtccaggttgagtgcctggctgatcatctccattgtctgttgtaaagactggtcagtaaaatctgccgtgattagatttgtgttgattactgcgtcctgcagttgtatgtttatctcaaatttattttctatccgttgtaaaacctgttgcatggtggcatcgttgaatgccatgttatattctgtgccttttgtgatatcgctgatgggcggcgttccttcttcctctttccgtatagccgttcctgttgtggcatatattgcctgttgttccgggtacaatacgacgggagccgattgcggcgcgctgagtgcaatttttcccgtaagcagggtcacctgtgtttctttgcctgtttcccggatattgaaactggtacccagcacggtggtggtgagtgtgccgcacttcaccaggaacggatgccgcgggtctttcgcaatttcaaagagggcttcgccctgcaatgttacttcgcggttaccggcgccaaaacctgccgggtaaattaatttactgtttcctttgagccaaacgatagagccatcggacaggatatgttttttagttttgccgggagtactttgcagcgacaccaggcgatgcggcgctactatgttcaacatttcctttttgaatatagcgccggcgataatgatacccgcgatgcaggcagccgctttccagtagcggaacagcggtgttattatgcctggttgccggtattgattgatgcgctttaccaggtgatggtatcctgctattctggctgcttccttttctgcttcgggcatcgcatcaaatgcgtgttcgtcgcctattgcatccagccactgctccagctgttgcgcttccgcagcttccagcgtgccatttagatatttctcgattaaatttttaagatcctggttgttcatcagtttttcacacttgtatttaatcaggcagttaatagtgtcacctatagataagtacactttgaaaagcgtaacacctacgtcttttaaaaaaaatttaaaaataaaagaccgggtaggccatattactgttgcagggctgtattcagcaccaggatgatgaggcacaggtgatgccccagcaccattctaagctgccggagcgctttggtaagatggttttccactgttttgtgagagatgttcagtgtattagcgatgtcggtaacagaaaggtgttgatggcggctcatcctgaatacctgctggcatttttccgggagccgtgatacttctttctccatggtatttttcagatcggtagccgcgatactttcctcgttggaattatcggatcgctgttcaggtaattgcgcaaactggtggatataggttttgcggatacggtctgatttgagatagttgagtagctggtactttaccgcggtaaatagatacgcggagagcgtgtgtgtgagttgcagttcttcatgttttttccagagggaaaaaaatacttcctggataatttcttctgctatttctttacttttcagcctgttgtaaacatatccgtataaacggggccagtattcgttgtagatagcctcatatgcacccatatcaccttccttcagtaaggctaatatgtgagattcatctgattgattatatttttttataatgttcaatatttccgtttattcagatgttataaacataaacaaacgaaaaaaataccaattatcataataataggatgataatttatgttggaacacttaaataaattgattttttataggtaacgtgttaagtaacatgataaaatggcctggaataaaaaagaaaaggccgccttgttacgggacgacctttcctgcctatgagtggttggttaaatattatcttctcttcctgtaaagcagcagtgtagtagcaaaaatcagcagtgatacgggtattacgccaaagaaaaatatccgcatggtcaggatcccctgatcatcgctgtcgattacatcttttgatctgatggcgccggtatttacggggaaatcgccgtaggtaaaccagcggaataattctgtgatcagcgactggttccatacggagggtttgcgccgcgccagctcgccggtgctcataaaatcggcatcgccggtaacaatgatgcgttgggttttgcccgccacttctctttcggcggcaatggccagtgcctggttattttttgccagcagcagcggtaccgagtggaaaccgtgctgttgtgcatactgaagattcacagcgcccggcatggataccaccgcactatcacccttgaatgcggcgagctttggagagatcttcccggcatcgtctgaaaaacgggcgaggataaagtcgggtgcatagtccctgctttcctcctgtaccggcgctgcgccgggttgcacgcccagttgttgcagtaagggttgcaatatttcctgtgatcctggttctgtgatcacgaacaggtttctgccgctggcaatatattggtccagttttgcctgtgctgccggcgggagggctgttttcggatcagcaattaccagcactgaagtggcggcaggaatttcttcactggtaagatttacggtatctacattaaatccctggttaatcaacgcccccctgaaggtgagttcatttacaaacatcctgaatgcggcatcacctgcttttgtgatgcttctttcgccgttgcctgcaacaaacgtaaccacgggtatttcagcaggtgttacgatacgtttcagcgcagcggtaaattcctgttcgccgggatatatcatgatatcgttgtaataccggagaaaagttttcttatcgccatattgcaggagccttaccagccggttttcttcaggcccgagatccaccattttccggatctgtgcaggtggaattactttcttgtaatccaggtcctggatatctgctactttttttgcgatggcggcatcgctttctccggggtaatttttatagagatttttgttgttggcgaagtcgtagtaatacacatattccatttgcaggttgggcataaaccggcggtagggtgtgagtattctttcatccgcgcttttcttctccggtgcgccgaggtagtaattatcgtcgaggatattcacataggtggtaattttcagcgacttgtccatcgcctttaccaattcgcggctttgcaggccgagtgtatgggttttggtagccgtcatatccacatacccggtgaaggacgggcgggagctgatatacccggtaaggaagcaaagcgctatcagtccgaggtaccttacggtacgtatccacggcgactttgcctcccgctggtcttgcagccgcatgccggtaatggccaggaaaaagccgattacaaggaagaagtaaaaggcgtcttctgtgctgatcagtccataaataaattgttcggttctacctgaaatagacataaaataggtgatatgccgcactgcatcattgccctggaacaggccaccgataaagttgagaccggccagcactgccaatgtgctgatagctgccaccacctggtaggtagtaagcgaggacatgaacagcccgatagctgcataggcgcagatgagcaggtacaatcccagtgcgccggaggccagcagtttccagtcgatatgctcaataaaaaacgaaccggagattccatacaggcaaatgataaccagcaatagtgcgccgtatcccatcatggctacatactttcccagtacgatgtcccttactttaatgggagacgacaataataatttaatggaaccgctgtgtgtttcccggctgatgaggcccatcgttaacagtggaatatagaagtacagggtatttttcacgccggggtaaaatccttcctgctgaccggtgaagatcatggaagtaacatcggtgaagtgatgtcccatacgttgtgcgcgtcctatcatctggatatagtgaaggaagtcgattcctatttgtaccgggaatacaattaagataagccaggctaccggcgagtgaaacaggaggctcagctcctggcgggctattctgataattattttcattactgtatggcaggtttagattttttattggataactgtgcgaaaatggcgtccagggagcttttctccagtgttatttctttgaggcgccattttttctgcacactcatttccacgatattttcagcgatatcggtggcgggctcaaatcttacgcgaatcgttttttctgtcaggaactccacgtctttaatgcctttgatggctctcagttccttttcttccggagggttttcgagggtggtgatgaggctgtccggttctatataattgttgaaagattccatggtgtctttaaacaccattctgccgccctctatcataataatatcctggcaggtagcctgtatttccgagagaatatgtgaagagaagatcacggcgcgatctgtggctatttctttgatcagctggcgtacttccaggatctggttgggatccaggccattggtgggttcatccagcactaccagcagtggcgtgtgaatgagggcctgcgcgatgcctacccgctggcggtagccaccggagaggttgccgatgagccttttgctgaaatgcgccacaccgcatctttccttcacggtatctaccgctgcttttatacggcgtttatctatcaggcggaggtgggcgcaaaaggttaggtattcatccactgtttgttcgaggtagagcggtgcattttgcggcaggaagccaatccttttctttgcttcttccgggtcggccctcatatcgatgccttcaatgagcacctggccgcgggtttgacttaacactccgcaaagaatgttcatagtagtggatttgccggcgccattggagccaagcaaccctacaatgcctttcttgttgatttcgaaactgacatctttcactgcccagtctttactgtaacggtgtgatagtccttcaattttaacgatgttgtcttgcatgtgtgatttaattagtcaataggaggttaatgacgccggcaggttaccggcgtcacaaatggaacagggaggacaggaatgacttatggattcagcggccagtccgggttgaatacagtagcattgggccacagctggcgcaggtaattattactgccgggcagcaactcatacgttttgccttctgcggtatgctttattattttctgaaaacgggtttctttgttcaggcgtttcaggtcgatgacccgcatcccggtgaatgccatttcccttcttctttcttccaaaacaaaccgtaatactttctcaccatcattactgaagtctgccggtgtaaaggctttataggcggccggtgtaatccggttgagtcttaatttattgatatctgcgagggcagcagttaaattgttttcacgggcaaagcattctgcgcgggtcaggtacatttccggcacattgagatagttgctatagaaatctccgcggaggaagatcttcacctggtacctggacatgtaattaaacggtggcgcgggaggccagccatcagcatagtataatgtccagcgtttatcgtcgttggtaaagagtgcacttaattccggggaggcgcaaacatccatgcccaatccgaatggccgcaggaagtgccgtgccacgatggtttccgggttaagctgcgcgtcggggatgttggtccatccgagcggcgcaccgggaacatttggaaacggcccggggatcgtgatcttataatcattcatgttggccagctcactttgcagcgacaacgccaggtcagcatttttgcgggcattggcgtaatcgcccataaagagataggttctggccagtaaggcgtatccgcctgctttacctgccctgaactttgtgagcttatgatttagcggcaggtcggcgatggcggcgttggcatcgctgagtacctggtcgtatacttcttttaccgtgttccttttgaattttgcgttgatgtctgcaatcagtgcaatgggaataccgttctgcgtggcggcggtggctgcatcataatgctgtgcgtatacatttaccagctgcaggtgctccattgcgcggcccagcaaggcttccgcgcgaacactttttttgttggcgtctgtaccttccgttgcatccatgatattgttgatgatgctgttgtagtagaagatccttttatagccttcactccacatgaaatcgttggcaccttgttcaaatggagctgggttgaatgtataaattttccggccatgtagctgttgcttcgtgaacaggttgccaggttctccttccggcaggaaagcatcgtctgagagcaggtcccagaagtaatcaccgaagttcactacggtgccggagttcagcatattttcgtaatcggctactgttaccgggataaatttatcctttggttttatatccaggaactttgtgcaaccggataagatcagtatgccggagatgatataaagatgtaattttttcatgtttcctggttttaaaaggtgatatctattcctgccatgtaagtggacattaccggtaatgttctgtttgcgtactggctggcgatttcataagcttcaggatcaattccaacggagttgttgtaccagtggaaaggattttgtacctgcagtgttaatttggcggaagataattttttgacacgggacaatgcggacgcaaaattataagagagcgcgatatcccttactttgatataatctgccttgagcacattttgatcggaggcataccagatgagcgtataatagttgccgccattacctttgagatcgggtgccggtaacatgccgggtttattttcatcgcccggtttgcgccagaagttcatcaccctgctgtctacgttgctgcgggggaaaccatagtcgataacaggcaccacatctctcatcacatttcctccgttggcaatgatcatgatacttagtgtgagttgctgataagtgaaggtgttggtaaaaccagtcgtgtatttcggtcttaatgtgccgctgtatacaaggccgtttatatccgtcatgttggccacaatggtgccggactgatcataattctttaccacttttcctgcggcatcgtataccgtcatggaaccgttggccggatcaagccctgccgatctgaaactgaaaacggcatccatcgggtagccaatgcgatttacgccgtagccaccggtaaggccgtatacattttcatccctggtatttatttctgtcatcttgtttttgttgaaactcagtgccagggtgctgctccaggtgaaatgtttcttgtttatattgagggtgttgagtgccagctcaatacctttattatttaagctgccgtagttaatcaatgcgctgggaaatgcgttggtgggatcgatggccttttctcccagcaggtcggtggttttacggatgtagtaatctattgatcccgacacccggttatttaatacggcgaagtcgacaccgatattggtagtagctgttttctcccatcttaatgatttatttggcggatagatgatatccgttgcggtggcattggcttcagaaaagaaggtagatcttgcctggaggtaggggcctaccgttctggctacgtttccgccgaggccgtaagtagagcggatgctcaggctgtttaaccagctgatatctttcatgaaatcttcttcagacattctccagctggcgccaacagaccagagcggcaggtagcggtagcgggggtcggtaccaaagaggttggagttatctacccgtacgcttccggtaacgttatacttcccgttgtacgtatagccggcattaccataggccgagatgtacctgtcttctccataataaaagttattattttcgttatacttcatggagaaggtgctgcccagggattctgttcctttcagattaccgagagcaatttcatttaccggcaggtattgcaggttattatcgttatagcccattttaaacacggaggtcgacgtttgtgatactgccctgcgttccacaccggctaaggccgacacgtgatgttttgtgctgatatttttgtcgaagttcagttgcgcgcgggcggtataggattttgaattgccacgtgtttcgtatagttgtccgccatcaggtacattcttcaccaactccccgtcgatgacctgcgcagcgtcgttgatcatatttttggtgtagtaagagtcgggagaataatatgatttattgtagctgctaccgcgttctgtctggtatttcagatccagtgtaaggccgctgataattttaacggtgaatccgccctgcagcctgaagtaatttgaccaataggaaagatctgatttatacagttcatccagcggattgaatgtttcatcatacagcccgaggtttttcaggcggtctatttcatagggtgactttaatttagtgaacggggcggagctgccatcgggatttttcagtacttcataaggcatattccggtaaaaggattcggggctttcgcggagatacttcccgttgcggatattggtattggcgcctacttctgcgtccagccatttaaacactttcactttatctttcatgcccacgttaatatcttcattgccggtacggaaaccgtagtccctgttacctgtataattcatcatgatattatactggtggatttcgtttccgccgctggcggagaagctgtggcgttgtttgacacggttacgcatgaacaggttttccagctggctttgcccgttggcgttccttaaattattgagggtattgtcgagatcagttttgctgatgagattttgctcgtaattatagagtgcttccattgcttttggctggcctgcacgtttgatgacatcgttataaccaggatgccagctattgaacagttcctgttgcagatccaccatctgggaggaattgagcaggtgcatataacctgcgtcagggatgcctgttataaacacggtgctgttgaagttgaccgtgagtttcctgttgctgccataccttgtggtaatggagatcacgccattggctgccctggttccgtagatcgaagcggcggcggcatctttcattactgttacgttcactacatcagcggggttgatatagttaaggtctccttcgaatggaaaaccgtccaccacatataacgggttttggttgccgtataaggtggaaagtccgcggatattaacggcgccgttctgcataaagaggccgggcacagtgccttccaggcggtccataatattggtttccatcctggcgccgagtgttttttctgtaatcacgctgaatgatccggtggcgcgttcttttgggattgattgatagccggtgttggccgtaacatttaatgctgacaaggtagccgagatgacagacaaaacgatgttaccgatattcccggttcgcagcataccgggagttactgtcacctctttggttttatatcctataaagctgatgcgaagtacatccccggcagataccggcaaggtgaagttgccttctgagttggtaatagcgggttgactggcgccaggcacctgcaccgtagccccgatgaggggaatgccggtgctgtcggtaacatgccctgttaccggtgattctttctccagcatggcgatattcgaggcagcaggaagcttgctgtacagcatgatggtgttgcctgctattttatagttgaatggttggtccttcatcaccagttccaggaagctgatcaggggcatattctgcactgatactgatacggcgccggcctgtttcagcagttcagatttaccccacaccacgaaacccgtttgttttttgatggcggcaaaaagtttttccattgggacggctcgtccggaaaaggtgacagattgcgaaaatgtgttggctgatacatgtaagcaaatggtaagaaggagaacactggtaaatctcataatccggagcattttggttgggagccggcacggcaagtcccaacggctccaataagcagttttttgcatagatttgcaacgtttggttgttaaaaatggaggtctcgaaacctgatttaagtcagccagcaactttccggaagtgttggtcgcacttccggctttttttgccggtcaacctgttttagttgatattcattactggcatagtgtttcagttttatggtatccgggataaataatatacgttaaggcattacgatcagccggcggccctcttccagccggaaatgcacatccgaccgttccagccccgcgagcacatcagagagttgcagggttctgctcatctcaccaaaaaagtgaacatcgggcacatttccttcatacactacttccaggttgtaccagcgttccagctggcgcatcatttcccgcaggcccactccttcgaggttaaacaggccgtttttccaggcgatggccttttccacatttgcgttccgcgttacttttataccagcatcgcctgtctgtagctgatctcctggttttaacaccacgctgccagcggtttgattggtaagggatatactgactgctccttccaccagcgtagtatagctattcttttcattcgtgtatgcgtttacgttaaaaccggtaccgagtacctggatgtccattttccggagcacattcaccctgaagggttgtgctgcgttgccggcaacttcgaaataggcttccccggagagttccactctcctttcctttcctttgaaggctacaggaaactgcagggagctggcggcattgagccatactttggtgccatccggcagtaccacctggaattgccgtcctttgggtgtggtgatggtattgtattccatttcgcctgcacccggggcttcctgcgtgtattggaggccgttacttttcaggactatggtagttccgttctgatgggtgatgataccgtttcccatgctgtcgagcaccatctgtgagccatccgccagcgtaaggatggcgccatttttcccgggagctatgtccggcagcgtgtttccggcgataacagcaaccggttgccggcgatgatagtggctgataaaccaggcagctgccccaaacagtaacactacagcggccgcccatccccatttgtggaggaaatgtacacggtgaagcggtttggtaaccgggtcgtttgatagtttatccgatgacaggatctggtcagccacctgcatccagtgttgctggttgtaggccggcaaggcggttgaatgatgttccttcagccagccttccacgtcgtcgatggaagcgccggtttcgtcccggtcaacccaaccggttaattcgtccagttcttcctctgtggcagtgtgtgttgccagacgatcgagtaaatatgccagtcggtggtgatgttccatttatgaaggtgatacaggtaaatgaaagtgatgtatgtccccttatctataccagacaattgagcggggaattggtaccgaaaaaaagtgaagttttttttcagagggactgtttattcagatgagtatatctatcaatatggcgaggagcagcgggtagccggccttttgcagggaggagcggatatttttcaacgccattaccagcaggtttttcaccgtgctgatggcgagatccatatgttgtgcgatttcactgctggagagtccctgttcacggctaaggcggtagatttgttgctgcttctccggtaattgctgcacagccttgttcaccaggcccagcaactgccggaattcaatcatgtctgccaccggcaggtccttacccgagctgtctttttcatagccaacggtatgcattactttatcgcggatggtttggcgacggacatagttcacggccaggaaaaaacagatttttttaatccaggcgcctggttgtgccacttccgtgagttggtcgcgggctacccatattttgagaaaggtatcctgtaccaggtcgtctgccactgtcactgatccggtaatacgtgctgccatcgcctgcaggcgtggtgcataaatttcaaaaagactcctgaacgcagattcgtcgccggccgctatccgcttataaaggtcaggagcatcaatagaatggccctcgctcattgacaaccttgcttgcgtgaaataacaaatgtgacggcaaggtagaataataatgtaaaattccatagcacccggggaaatgtgctgatggacgtattttattaacgggaaagcatataagctaccagcgccatggcagtgatacctgctacatcattccaacggaaaggggatgtctggcgatagttgtttaaatgatggtgagatggataggcctcgtatatcaggctcctgctgttgctgctgtctttgacagcgggcaggtattgctgccatgaccactgtttatggttggcagtctgcccaaaggaattggttttcggggccggcagcagcaacatttctttcttgccggtgatcgcgctgctgtcctgcgcaggtgcggttaaagtaacgcccacggccaaaccggcggtgagcatgattgcccggaaataacttttcaattgatctggtagtagcatggtaatagtcctcctgtattcaggacgcatggaattcgccgttcccctatgcgcggggtattttttttccggcaaaataaagagccttcgtattgcagggcaatacaaaggctctttatttttatagagataaattacgcctggttgttttgcaccggaaaaagcgtgcgcagcgcgggaatacgtaaaaagaggcttacccataccaggataccgaacaccaccgggaaataatagggttcgttgatcctggacatgatggctacagcgccgccgaggtaagcggtgaccagtatcgcacccagtatagccgtacggggaatggcatacaaaatagtggcgatgagcaatataatgccgataccctgtacctgttctgccggccagcccagctttacgctgccttccatggaagtgatgttcttaattactttcatgatggcgtctaccaggagaaagagtacacaaagaacggtgattacccaaccggtaatattagctgctttagaaggagctttcttattcagataaattgtttgcgcttccatataagttgtttttttgtttttgtttgatttgattgacaatacaaacttaccggcatttgtgcgcattcctgctggggaaatacgacattcttactggttgattgcgacaattcaggaacatcttacctttgcgtcatggattatttcaaaaagcagcttgatttattaaaaacagagcgggaagaagacaggaaatcatacaaacaaatgacggaatccacgtctgtagcagatcgcagggcaaacggacttacctggtaccctattgctatcaggggatcagagatgagccggggagattatctgactgtggaagtggagcgcaccactcaccaggacctgccgcatcagctgcgttttggcgcttctgccgtattattttccaatcatgatccaaagcaggatcatcttgaaggcactatcacttaccagggcgggaacaggctgaagatcaccctgcgcaccgacgagctgccggaatgggccagtgatggtaaactgggcatcgacgtactttttgatgataacagttatgacgaaatgcaaaacgccctgaaacaggcggatgcattgcaggataaagtacccgaaggacggctgataaaaatactgaccggggaaaagaaacccgtgtttcatccggatattactccttatgtaaatcccgcgctgaatgcctcccagcaatcggccgttaataaaatactttccgccggcgacctggccattgtacacggtccgcccggcactggcaaaaccactaccctggtacaggccattaaagtgctgatcaaacaggagcaacaacagatacttgtggtggcgcctagtaataccgcagtggatctgctcagcgaaaagctatcggatgaaggactgaatgtgttgcgggtgggcaacccggcgcgcgtatcagagcggctgatgtcgctcacgctcgacagcaaaatatctgagcatgccagtatcaaagaaatcaagcgcctgaaaaagcaggcgaatgagttccgcgacatggcccacaaatacaagcgtaactttggcaaagcagaaagggatcagcggaaagccttgtttgacgaggcccgcaagatcatgaaagaagtaggcaatacagagcaatatattattgacgacctgatctccaaggcacaggtgattacggccaccctggtgggcgccaatcattataccgtgaaaaatttaaagtaccatacggttgtaatagatgaagccgggcaggcactggaacctgcctgctggatccccatcctgaaagcgcaaaaggtaatccttgccggagaccattgccagctgtcgcccaccgtaaaatcggaggaagccgcccgtaaaggtctcagcactaccctgctggaaaaatgcaccgccctgcaccccgaaagcgtaacgctgctggaagaacagtaccgtatgcacgccactatcatgggatactcttccagtatcttttatgaggataaattaagggcccatgcctctgttgccggacacctgctgttttccgaagataacccgctcagctttgtagacactgccggttgcggttttgatgaaaagctggatggcaccagtaccaccaacccggaagaagctgtttttttatttaaacatcttacccggctggtaactgcgctgggggaacattaccagccgaaagactttcccacggtggcggttatatctccctataaacaacaaatacaattattaaaagagcagctgcatcactccccgttgttgcagccctatgcagacaaaatatctgtgaacaccatcgatagtttccagggacaggagcgcgatattgtgtatatcagcatgacgcgcagcaacaccgaaaataaaataggcttcttatcagacatccggcggatgaatgtagcgatgaccagggcccgcaagaagctggtggtgataggcgacagcggcaccctttcccagcttgggttttatgcggatttcatcacttatgcggagcataaaaacgcctaccagagcgcatgggagtttatggatgtgtaacgctggttgtcattaccttttccaatacctcaaaaaaagccggttgctgttcaaacatcgggaagtgacccgaagcctggatccaatgcagtacgatatccgggcggatgatcttcagttcgtaggtatagaaagccaggggatcctggcggctgccgatcacggtgaccggccctttatattgcggcaggtttttactgagatcaaaatgggtcctttgcaggtctgataccattaacccctgcatacggacattgggttttgccacataaatcttcgccatgaggctgtcgatgtccgctttgttgtaaatgtatgccaaccgtatggtgcggttatacagcgcactgtctgcgccagttgccctccctccttctatctttttgctcagggaatccatcagcgccaggtcggatacacccaggcgtgcccgcaggttgttcatatgcgtggtcatgaaatcggcggagaacttatagtagccaggatttgccagcaccagggcgcgcaccttttccgggtgggcagctgcgtaactcatggccagcatagcgccccaggagtggccgtaaataacggttttgctgatcccttctttctgcagcaaccgctgaatgtcttccacggcggctttgaggttaatagtagtagaatcgaatggtacggggatggataagccggtgccccgttgttccagtaagatggccttgtaatgcttccccagctcaatcgccacttcttcctgctgcaaacaggagttgccagggccgccagacaacactataacagggcttcccttcccataagtatgataataaagccagccgttggggtatttcagtgagtccagttgctgtgcatggatgggcaggcaatacagcaacgtggttaacaataacaacagtttcataagacggtttttccctattaaaataggtgatttcaggcatataatgtgcctgttcccctgaaagccgctgcagtaaaggacaaataattccttgccgggagcctgaaaaagcgtaactttgcccgtttttcgggataagataaatggtagcctgctcataatgatcagcctgtttattttttgaataaatacattatgagtaaaatagttgattacaggaagttactgggtgttaccaaaactactgaagtaaaagaattgaaaacgatctacaggaatttaatgaaggagtggcatcccgataaatttgaaggcctggcagaagaacagaaactggaagcagaagcaaagagtaaagaattgattgaggcttatcactttttagtaagcatagcacctgaaacaattgctgctgctttaccacagtacaccgccaccatttctgcttctaccctggtggatttctcctaccagaaacaaacacttcagcttcactttgaagatggcagcagttatgaatacctcgacgttccgaaaacattatatataaagctgatcaactctgatacgccgggcaggttctgccgcaggcatatttaccacgaatttgtataccgtaaagtgagcaaggcggttgaagcatagcatacctgttagtatgctttgttttaaagaataaactatatttgcgccatgcgttcatggatcacaaagatatcgttgatgctggcagtaatggttattactgcgcacaacgttatgtttcatgaccatcagcatatcatttcatcgtccggacacttcgtccacgatgatgatgatgatgaccacgatcatgatatgcagcattcgctggcgctgaacctgattgatcacagcttcacttctccctcttccagccacctgcaacacgaagtgcccgttttaacgctggcgcctgcacctgacctggtttctcttccggaggttatctgctttctgatatcgaaaaccagctatcagcaaaagcaggaatttccacctccgctgcaaagcctttcattttcggcattaagagcaccccctattttccttgcataacttcaccggaattttgtttataagacggttgtattaatgctattgcgtttaatgcattcaatctgataaatctgtctactgggaataccggcaccggtggctgctttccaaccttccctgcattttatttttagtacttatgcccgctcaacggggcggaatgagtatgccaattattcgatatgctgaataagatcattgaattttcaatccggaacaaattgattgtaggcttatttatactcggtcttatcggctatggtatttatgaagtcaccaggctgcctatagatgcggtacctgatattacagacaaccaggtacaggtaataaccgtaacaccttcattaggtgcgccggacgttgagcggctgatatcgtttcctatagaacaggcaaaccgcagtatacccggactggcaaagatcaggagcttttccaggtttgggttatctgtagtgacccttgtttttaatgagggcgtggatgtttactgggcaagacaacaggttaccgagcggctccaggaagtgcaaagccagatacccggcggaataggtgttcccaagctggcgccggttacaactggtttaggagagatttaccagtatacgatacggcctaaaaagggctatgaagaccggtatacggcaatggagctccgcactatccaggactggattgttcgccggcaactgttgggcgttaccggcgttgcggatgtgagcagctttggcggctacctgaaacaatacgaaatagcggtagaaccggccaaactgaagtcttacggactttccatcaatgatgtattcaaagcactcgaaacaaataaccagaacaccggtggagcctacattgaaaaagagccaacggtactttttattcgcagtgagggcctggtcggctcagaagacgatatcaggaaaattgtcgttaaaaataccggtaacggcacgccgttgctggtaagggatattggtgaagtgcggttaggctatgccacccggtacggcgctttgacctataatggcgaacgtgaggtatcaggtgcggtagtaatgatgctgaaaggagccaacagtaatgaggtgatcaaaaagatcaaagcgcgtgtagaccagatccagaaaacacttccggaaggagtgatgatcgaccccttcctggatagaacaaaaatggtcaataacgccattggcactgttgagaaaaatctcatggaaggcgcattgatcgtggtatttgtactggtgttgttcctgggtaacttcagggccggcttacttgtagcttctgttattccgctggcgatgctgatagcggtaattatgatgaacacctttggcgtaagcggtaacctgatgagcctcggtgcgctggatttcgggttgattgtagatggcaccctgattatagtagaagcctgtatgttcagactgcatcattacaacaaaccctttatcacgcaaacggaaatggacgacctggtgttggaaacatcaggcaggatgcgaaatgcagcggttttcggagagctgattatcctgatcgtatatcttcccatatttgccctcgccggtgtggagggtaaaatgtttaagcccatggcgcagacagtagccttcgcgctatttggcgctttcctgctttccctgacctatgtacccatgatgagcgcactggttttaagtaaaaaaattcccgctaaactttcctggtccgacaggatgatggaaaaactggaagtccgctaccagcgcctgttaaacaaggtactgaacatacccaaaacagtaattggaacggcggcaggtttattagctattgctttatttgttctttcgcagctgggaggcgaatttataccccggttggaagagggggattttgcggtagaaacccgcgtacttaccggcagtagcctgaaaacctctactactgcggtgtcgcagggtgcgaaaattttgctggcgaagtttccagaagtggagaaggtggtggggaaaaccggtagcagcgagattcctactgaccctatgccgattgatgccagcgacctgatggtaattttgaaagataaaaaggaatggacttctgcaaaaacctttgatgaattaacagagaaaatgtcaaaggaactggaagccatacccggcgttactttcggattccaataccctgtacagatgcgctttaatgaattaatgacaggcgcccgtcaggatgttgtctgtaaaatttatggcgaggacctggacagcctggctcaatatgccacccgcctcggggcagtggtcaataccgtgaaaggtgctaccgatctgtatgtggaagccatcaccgggatgccgcagattgttattaaatataacagggacgctattgcgcaatatggccttaacatcaatgatataaacagaatagtaaataccgccttcgcggggcaaagcagcgggcttgtttatgaaggagaaaaacgtttcgacctggtagtaaggctgagtggtcagcagcggcaaaaccttactgatgtgcagcatttactaattcctacccaacagggttcacagatacccttatacctggtagcaaaagtagctatagaggaagggcccaatcagatacagcgcgaagatgcccagcgccggatcattgtaggattcaatgtgcgtggccgtgatgtgcagactgtagtagaagaactgcagcaaaaggtatccggtaaaataaaattaccaccgggttactacgttacctatggtggcgcatttgaaaacctggaagctgcgaaaaagcgtttaggcattgccgtacccgtttccctgctgcttatcctgctgatgttatattttgctttcaacagtatcaggcaagggttgctgatttattctgctattcctttatctgcaataggaggcatttttgcccttgcattgcggggaatgccgttcagtatttcagccggcattggtttcattgcattatttggtgtggccgtattgaatggtattgtgctcattgcagaatttaaccggttacataaagaaggactgaacgatgtccgggaaattgtgttaaaaggaacgagggtacgtttacggccggtattgatgacggcatccgtggcatctttgggcttcctgccgatggcactgagcaatggcgccggcgccgaggtgcaacggccattggctactgtggttatcgggggactgatcctggcaacgttcctgaccctgtttgtacttccaattctttacatcatttttgaaaagaagcatctgatgaagcaacccaagcatttaccgggcgctgcactcttattattaccattccttttgctggcagcacctaacgcacgggcacaacaaccgatctcccttaatgcagcgctggataccgctatgaagaataacctgtctgtccggaaccaacagctgaatgcagactatctgaaaaaattaaaaggagcgggatgggatgccaaccaggcggttgttaccggtgaatatggtaaaatcaacagcgcttacaatgataaccggtttaccatttcacagaccatcaaattcccaaccatatacagcaggcaaaaactgttgctgaatgaagaatggaaagaaggactgctgaatgtttccgttaaacaatctgaattaaaaaagcaggtcacttcggtgtactaccagctcctgttcctgcgcaataaaaaagaactgcttcagtatacggatagtatctatgcgcttttcctggaaaaggcggcaatacgttttaaaacgggagaaagtaacatactcgaaaaaacgaccgccgaaacccagcgtggacaaatcgctttgcaggcgggccagttacagcaggactatgccatcctgcaagcgcggctgaaagtgctgctcaacacgactactgatgtagaacctgatgatacaccgcttaaaatgccgcttcccggtggtattgatagcacggagcttaaaaagcatccctacctccaactgctggagcaacaggagcaaacaagtttttccaggtacaaactggaaaaatccaggctgttacccgacttactgctgggatacaataacatgaccatgcgtggtatgggagcggatgataaagaatattcgggagacacccggttccagtccgcccagataggcgttggtattccgctattctttggtgcgcagaaagcaaaaatcggcgctcagaaaataaaccaggaactggcaaaaagcacttaccaggcaggattacaggaattgcaattaagatataccgaagctgaaaagcaatatagtaaaatgatgcaggcggtttcctactatgaacaaagtgggctaaagaatgcggataccatcattgctaccgcaaatctgcaattcgtaaacggggaaatcaattacctggaatgggtgatgctgaacaaccaggctttcagtctccggaatgaatacctcgatgctgtaaataaccttaaccagtctatcattgaatccaattctttattgaacaggtaaatataaaattcatgaaacaatacatcatcatattagctacatcctgtttactggcagcctgtaacaacaaaccgaaagaggaggaaaaagcaccggccggcgataaaggaaatctcattgaactgacggatgcccagcaaaaaaatgcgggcatcgaaaccgggcacctggagaaaaggcgtattgctgctgcaatccgggtaaacgggcagattgacgtacctccgcagaatatggttagcatcagtttcccgttaggaggctttttaaaatccaccaccttgcttcccggtatgcatgttaccaaaggagaagtaatcggcgttatggaggatcaacaatttattcagctgcagcaggattatctcacttcaaaagcgaaattggcgtacctggaaaaagagtatgcccgtcagcgtgaacttaaccagagcaaagctaccagcgataaattatttgagcaaaccgaagcggagtataaaagccagcgtgtactgaacagatctgttgcagaaaaattgcaactgattggtattaatgcctccaggcttgatgagaacggcatttccagaagtgttaatcttcattctcccatcaatggttttgtgtcaaaggtaaatgtgaacataggcaagtatgtaaatccttcagatgttttatttgaaatagtaaatccggcggatattcaccttgcgttgaccgtttttgagaaagacatcaataaactggctatcggtcaaacggtggtggcttttaccaacagcaatcccgaaaaaaagtacgattgtaagatcatactgataggccaggatcttacggcagacaggagtgtgcaggtacattgccactttgagcaatacgacaaatcactgatcccgggaacttttatgaatgctgatatagagtcagccaatgatagtacctggtcgctgccggcggatgcagtggtacgttttgaaaacaaagagtatgttttttgccggaaggataaaaatgtatttgagatgatacctgtaaaaacaggcaacagcgagaatggatatgtggaaataatattgaatggcaatacacccgcagtcaacagtgaatatgtgataaaaggcgcttattctcttttaatgaaaatgaagaatacggcagatgaataagttgctgaagattgatggtgtttacttcttcaataaattttttttatagacagaagggcttttgcctgtatgtactttaaaaacccgcgtgaaatggctctggtctgaaaacccggtaagatatgctatttcggtaagtgaatgcgacgtggtggaaagcagctgtatcgctttgtctatccggagttttctgatataatcaccaaaggaaaggtcatcaaaatattttgaaaattcccgtgataaataggcgggatgtacctgtaaagtttctgaaattcccttcagactcagattcaggttggtatctatctggtcctggatgatctctttcagctcctttgcccagtgaggtacctttttactgtctttttcatgttgcaggaaatttttaaagatgtccagcagctgactttcaaatggttgctgcgtgtgctttacatgttgcaggtattttgcccagctgtatagcgaatcgtataacaacattcctttttccagcagttgatagtcgtctggttcatcatgcgccataccagcggagatagcccataaaccggcagcttgcggcgccaggttatggcggtcggtatcagcaccgcgaacaattggcgccagcgcgtgaatggccggatcttcaaggtggtgtttttttatgatgtagtcaaatgtgcataagtcgtcatagtgtgtgtattccacaccggctatatcaaaaggaatggcgttcagctcagcggcctttgacaatacttcattgaacggcacgtatataaattcagccgcctggtctacaaatctttttataagccagggacaagccagtctgtctattttcgggcgctcgcgggtgatccatttcatacctgataattaattatgatagttacgtgtagaacaatttagttccccgtaggccggaagctgggggtgcttacattactttctataaatgccttacggtattccctgggagattttccctggtaaattttaaactgcctgttaaagtaagagatattatcaaacccacaggcatagcatatttcagatatgccatttccggtgcctatcagcagttttgtagcatgactgatccttatctcgtttacaaactgtgagaatgttttcgtggttctttttttaaagtagcggcaaaatgcagcttcattcatacaggcaagagaggcagcagatttgctatctacatgatcagcataattttccagtacatacttaaatattggttccagttttttcgaatctgcatccttataacgtgtctttccctgatcatctgtcagtagttgaacactttccctgccttgcagtgataattcatccaggatctgtaaaaggatgatcaggtttttcatctgctgatttgcctgaaactggaaaaacagggtattcacaacaggcgatatcttattaaattttataccgtattcagataactgcatcagttcctttatctttctcaattccagtttttcaaaaaaatcctttcctataaaatcttctgtaaactgcactataatagcgtgcgctatttcgtcggcaccaacaggtgagctattattgcaaaagcaatggaccaaacccggaccgaacatataaatttctccttcattgtaattcatcaccttgtttcccgcatacattctgcctgcactttttacaatcaggatcagctcgtgcccatgatgaaaatgaaatgtattggtgaaccggggctgacagaattcttttattacaaaactggcatcttccggggtagatatgtgtcggtaagaaactttcataatgtctttatctttagtacactatttattttctaaagcaaaaaaatcagaaatatggtaaatatagtattgatatcttgcaaatgaagtacttttatttcaatggaagtctgaataagtttgtgaaacaatgaattcttaaaaaacgttccggttatgaaaccaacaggcttatgccttacagatgccacatgattcgacgtagctattatctgcagcatacattaatccacttttatatatcaatgcgttatggaactagggatacacaactggatgcggtctgaaacgatagaaactaccatcaggagagtttctgcgctgcgatataccaggcttgaaattgccggcacccccgaacattatgatacgaaaagtttaagagaactgatgaagacgcatggtttgtcttgctggggagctgtaacgctgatgctgggtgaccgcaacctgcttgccagggatgaggcgcaacgtgcaaaatcagtacagtatgtaaaggatgtaatcaccatggtaaaggaactggatggtcacatggtggctgttgtaccttgcaccgttggaaaaattgtaccggacggaaggcccgatgaagagtggaattgggctgttggtgcgttgaaggaaatttacgcctatagcgaggctgcaggcatccggataggcattgagcctatcaacaggtttgaaacctatttcatcaacagggctgatcaggcattggctttagcagccgccgtagggcctaattgcggtgtttgcctggataccttccacatgaatatcgaagaatcggatttgtttgaggccatcagaagggctaaggggaaactggttggttttcatgtggcagacaacaacaggatggcgccgggaatggggcatctcaattggcaaaagattgtagatacgttgagggaaataaattatgatgaggtgctttccgtggaattttgcgcttcgctggatcgcacgccagccaatccttacccggattcgattgacgaaaaccctgaaaacttatctgctgagcaggcgaagttcctggtggaccacggcagtgcttctgttacagaagcgttttataccatgctgactacccaatcatttaatactttatcaaaacttatttaaagaagtcaactgctaacagatgaaaatagctaatgtagaggcattttggttgcgctgtcctgttcctaaagaaaaacaacatacttcagactatggattactggccaattttgacatgacgcttgttgtgataactacagaggacggtcttcagggatttggagaagccaaagcagcggttggatcttcaggcgtgtgtgcttccatcgtgaattgcattgaaaatgagttgaagccagctttactgggtaaggatgttaaagacatttccaggttatgggaggagatgtataatggcacacgggatcattatgccttgctgagaggccggaaattccctatcctggggagaaggggccttactatatctgccatgagcggcattgataccgccttgtgggatttgaaaggcaaaatgctcaatgttccggtgatggatttgctcggtggcgcctgcagggatcagatgccggcatatgcaagtggtggctgggcagatgcagacaatattggcacacaattgaaaggatacatagataaaggctttaagagtgttaagatgcgtgttggcgtgatggatcagaccgtacaaaacagcattgaaagggtaaaagctgcgagagccgctatcggtcctgatattaaactgatggccgacgcacacggcaccttcagtgttccggaggcgaaacagttttgccggggagtagcagattgtaacttgtactggtttgaagaacctatcagtcctgataacaaaagggggactgcagaagtaagggcttccacgcatattcctatcgcagcaggtgaaagtgaatataccagttttgacatacaggcacttttggaaataagggccattgatgtaatacagccggatgcggccatcattggcggcatttcggaagcggtgcgggtttcgcacctcgccagtgtgcatcaactggagctggcgccgcattgctggggttctgccttttcttttatggcagggctgaatgtagcatttgcatcgccttccgcaaccatcattgagttctccgttggaggaaacccgatgatgtatgacctggtgaaggaacagattaccgttacaaatggctccatccaggcgcccaccgcacctggattaggggtaacgccggactgggattttgtacggcagtataaacaaaaagtttagaagtggtatttgtaaatatttatttatggccaaagcacttaaaattaatcacgtaacactgattgtggacaacctggaaaaagcaggtcaattctatcagcatgaattgggcctggagccgcttgccgccttccggtttgattaccctgttatgtttttcaagttcaatgatgagcagcaattgcatatctccgaatgggaagacaaaacctcttttcgcggacatgtatgtgtgcaggtagatgatttcagcagtctttttttccgcatgaaagcactgaatataattgatattcatccgtggggaaaggtaagaaagctgcctgacggggctatgcagatgtttgtgcgcgatcctgccggcaacctggtggaaatatcttccataccaggagttgaagtggactcgcgaatattcactgatgaactttatgaagaagggttgtatgtttcaaacagaaatgacttcagaggataccggtctgatgatgccaccttatatcacaacaaatgagaaaaaacgtactgttgcttgaaaccattgcagaggaagcgttagccgttcttcagaaaaatgtgaatgtattcacaggatacgacgaacctagcttacaggaggttttgaacaaagaggacattcatgccatcattacaagagggaaaggcctgatcactcaaccactcatggatgccttcccgcatttacaggtagtggccaggtgtggcgttgggttggataatgtagatgtagctgcagcaacagtaaaaaagatcaaggtaattaatgcaccgggcagtaatgccgccactattgcggaacataccctgagcctgatgctgatgctgatgcgtaatatgtatgaatcggtttcccaggtgaaacaaaacaactggagctggcgcaattcatatgcaggagatgagttgaacggcaaaaccctgggtgtgctgggaatggggaacataggaaaacgtgttgcccggcttggagaagctttcgggatggaggtcgtgtactggagtaaatctgttcaggatctgccttataaatacctggtcatggaagatgtattacggcagtcagatgttgttagccttcatcttccactcaataacgaaacaggtaagatcataggagaagaacaactgcgtttaatgaaacggggttctttactgatcaacactgcaagaggcgcgcttatcgaccatccggcgttattgcaggcattaaattccggggtgatttcgggttttgctgcggatgtattaccggatgagccaccagttgagagcgttgatatagtgcgtcacccgcgggccatcatcacgccgcataccggcagtcttacctcggccacctaccggcagatatgcctgcttaccatcaataatgtagtagccgtgcttaccggtggggagccggagccagacagcatatataaccgcaaggcgttgttttgaaatatatcgtattcaaacggtcatcataatctctgttcaaatgaaaaaattttgcgtttgtttattgttcatggtaagcaccggtataacatctgccggcttgctctttgcacaatcttccaaagagataaaaaagccgctggttgttttcgtgaccggtgatcatgagtacagcagcgaagaaaccatgcctttagtcgccgccgcgctggagaaagattacggcatgaaaacgatcgttctcaaagcatctcccgattataacagtgaagaaaatattccgggcctcgaggcattgaaacatgcagacctggccgttttctttttgcgctggcgcaggcttccgcctgagcaacttgcctatatcgacgcttacctgaaatccggcaagcctgttatgggtttccgtaccaccacgcatgcattccattttccggagggacatgccagtgagaaatggaacgcctttggagaatttgcattaaatgcacctcccggatggggcggcgccgccaaacatacccattatggacatgagagcagcacggatgtacgcatcattcctgagcaggccggcaatcctatcctgacaggcgttgcaaagaattttcatgtgcgttcatggctgtaccgtgttttacccgattatcctgtgaaagggtctacctggttactgatgggaaaggccgtaaatcctgataaagaagcgattcaaaacccggttgcctggaccggcaccaacgcttttggcggacgtgtttttatgacaaccttaggtcaccctgaagatttcagccaggaaccctttcagcgcctggtgatcaacgccattcactatgagctgggccttaaaattccacgaaaatggaaaggtaaaatgaatatccaggtgccctaccgtgaggcgaaatagtatttcacgtttcctgatgctgctaaactttttaaagatgtccaaactattaaaaattggcatttacgcgccttttattcccatagtattggcgataatgatactgcatgcctgtaaatcgcaggcgcctgctccgctcactatttccgatacctcccatatatccctgattggtaacaacctgggatccaggatgattaattatgataattttgaaacggaactgtatctccgttacccggaatataaactgcacgtccgcaacatgtgcgatggtggggaaacacccggattccggccacatgccggcagaaattctccatgggcatttcccggtgcagagaaattccatccggagctcgccggccaggttcaaacaatagaaggcccgagcgaaggacgctttgaaacacccgatcaatggctcaccaggcacaaaacagatgtgatcattgccttcttcggttacaatgaatcatttgaggggaaagaagggctggacagtaataaagcagagctggatgcatttataaagtggacgttgaagcagaaatacaatggcgcctcagcgccgcaactggccattgtttcacccattgctttcgaaaatctttccggcaaatatgacttaccggatggccggaaggaaaatgaaaaccttgccttgtatacccaggccatgaaggaagtggctgcccgcaataacgtattatttgttgacgcattcacaccttcccaaaaatggtataaggatgcgaaagagcctttgaccatcgacggttctcaactgaatgaagaaggttataaaaagctgggacttttgctggcagaccagatttttggaaaggtagccccagccgcaacagctaacaggcagctggtgcacgatgccgtgatggaaaaaaactggatgtggctaaatgattacaaaatccccaacggcgtacatgtgtatggtcgccggtatgatccttacgggccggataattaccctgcagaaatagaaaagatccgcgagatgacagcgatcagggacaccgcggtttggctggctgctgctaaaggaacgaaaatggatattgcagctgcagataaaaacaccaaagtattgcccgccgttaaaaccaactataaccccgctaaaaatggcagtctccggtatctcagcggagaggaagcggtagcaaagctgaaagtgccgccaggatataagattgagctatttgcctcagaagagcagtttaaagaccttgccaagccaatgcagatgtcatttgacaataagggcaggctgtgggtagccgtgatgccgagctatccccactataagccgggcgatgccaaacccaatgataaaattattatccttgaagataccaacaacgacggcaaagccgataaagaaacggtatttgcagacagcctgcacctgcccatcggttttgagatagcagcagaaggcgtgtatgttgcccagggaactaaccttaaattgctgacagatacagacggcgacgataaagcggataaaacagaaatcctgctcagtggttttgatgatcacgatacacatcacagcagtcatgcgtttactgccgatccttcaggagcgatctattcgggagaaggcgtgtttcttcatacacatatagaaacttcctacggaactattcgtgcgtctaacggcggcttttacaggtatgacccgcgtcgcaggaaactggaacgtactgcacaactttccattccaaacccctggggtattgcgttcgacgactggggacagcccttctttgcagaaacctccagtccggatgtacgctggatgctgccaggcaccgtactgcccaggtacggccaggctacacataaatcgatccagctgatagaagataaacataaagtacggcccacatcaggacttgaatttgtgtccagccgccactttcccgatgaagtgcagggcgacttcctgatcaataataccataggatttctcggaacaaaagaacatacgctgcaggatgatggaacaggctacaaaagccgtcatcgcaccgacctgctcgtgagcggggatcccaatttccggccggtagacctggagtttgcgcccgacggatcattgtacgtgatcgactggcataacatcctgatcgggcacatgcagcataatgcacgggatcctttgagggatcattcccatgggagagtgtaccgcattacttatccctcgaggcccctggtgaaaccggcaaatatagcgggagcctccatagaagaattgctggacaaccttaaactaccggaatacaggacccgctacagaacccgccgcgaactgagaggacgggatgtttccgccgtactgtccaaactgcaaacctgggtttcccagctgaataaaaacgatccgcgatatgagcatcatttgctcgaaggactttgggtgagctggggtatggataaagtagaccagccgcttttaaaacaggtactaaaagcccgcgattatcatgcaagagccgcagccgtgcaggtactgcgttatacaggacaccaggttcctgaccaggcagatttgctgatgcaggccgccagcgacgaaaatagccgtgtacgcctgatggcaattgtggccgcctcatggatcggtaaagaaaaggggcttcccattttggcagcagccaagaaaatgccactggatgaatggatgatccatgcgtatgaaaccgccgtagcccacttaaacggggagaatgtgaaaaagggaaaagagaaagatgataataccaacctgaaaggcgctgagctggccctgtttaaccagggaaagaaaatttattccatagaaggatattgtaaaacatgtcaccaggcggacggcaaaggccttcctgattctggcttccctcctcttgccggttccaggtgggtaacgggaagtgatgaacggctcatcaagctggtgatgaaaggactcttaggtccgatagaagtaaataataaaacgtattccggccaggttcctatgacgcctttcggcgggttactgaaagatgatgaggttgctgccgtgctaacctacgtcaggaattcgttcggtaacaaaggatcagctgtttctcccgaaaaagtaaaacaggtaaggaagcgcatagaaagtaaaaaggatttttattcttcagaacaactgctcaaagaacatccaatggaaaagagataataaaacacccgtccgtttaccctgtttcagcgtttaggcactgttgttaatttactatgtcacttagtgaaaatatcacaaggaagtatcatttcgtatacttaatattgttaggattactatcaatctaatttgtcaaccgatttaaaaaaccagttactctattttctttttaacagtgaaagatacctgatatgagctgtagctcccactggtattaactgttagctttttcacggatatgaaaaaccattcagcatagaacgatcatcgacaagccatactcatttgcctgaaaaaaacttataagatcattcaaccaaaacacaacgcattttctgcgaaagctttacgctgcccttaaattctgctacttaaaaaaatgtatccggaacaacggatacgatcaaattaacctgataactttttaattatgaaacagttttccacggtgactttcaacatgccggcgttacgccagaaaatcatttatgccgcctttgttttattcatgggagtagtcacgcagctccatgcgaaagatccggtaacaggtaattattcacctgcattcctcatggatgtgcgtggtaaggttttggaagagaatggcgttggcgtgccgggagtaagtattaaagtaaagaatgttaataaggccacgactaccgacggcgacgggaacttcagcattaaaggcgttaatgaagatgcagtgctgattgtttcttatatcggctatgttacccaggaagtgaaggttactgcggacatggtgattaagcttgttccgcaggttaaaaagatagatgaggtagtggtggtaggttatggaacgaccaaaaaatcagatctgaccggggcggttggtactgttaaagccgaaacgttacaggaacgtccggcctcctcgttaaaccaaagcctatccggccgtgtatcgggggtgaatgtttcttccaactccggtagacctggtgggagaaccaacgttcgcatccgcggatcaagctctctgagcgtttccaataacccattgtatgtaatagatggtgtgatactgaacccggtgggtttgaggaatggcagtacgccgattgactatatcaatcctaacgatattgcttctattgaagtactgaaggatgcttcttccaccgcgatctatggggccaggggagccaatggcgttatccttgttaccacgaaaagaggcacttccgccggtggaagaatcacgtatgatccggatttcagtattggtgtgctgcctaaaaaactggaactgctcaatgcaaaagagttcctggcggtggaggatctggcttatgccaacgcgcaaaaatatgatcccgttggatgggcaacgggaacaaaatacaccgatcccaaaaccaaacgcacgaatcccaaattatttgattcacagggaaacccgctgtacgacaccgactggcaggacgaagcatttcaaaaagcttttacgcagaaccatcaacttggatttaccgatggtgatgaaaaaagaagcataggcgctttcctgaactatcgcagccaggatggattggcgcggggttcctggcaggatcggtatgccggccgtgtggtatacgacagccagataaaagactggttaaagatcggtggtaccatgagctatacggatcagcgggaaaaacaggtggatcaactcgatggaggcggtattaccatgatgcgccaggtattggaagcgctgcctattatcccggtaaaatatgcagacgggtcgtgggcgagcaacagggactatccgggcatggagggcggcgataatcctttaagggtatccgccgacaggatctccatactgcatacccaaacgcttcttggcaatatgtatacaaacattcacctggcggaagggctggaattgaaatcgacgattggtgtcaacatcattaaccaacgggaagattatttcgccgccaagggaatgcaatacatttcagacaacggaaatgcttttattaataacaacaggtacaactcctggcagtttgagaactaccttacctacaacaggcagtttgcaaaagtacatgctttaaatgcgatggcaggggtgtcctggcagcatatcgaccgtttcgaaaaccaggcaagtacagagggcttcaccgattcgtactacaaatattacaatcttggtgcaggatccagcccccagcctccttcttccgtgggaactgccaatggcttgaattcttattttggccgtgtaaattatggtttccgcaataagtatttagtcactttcaccggccgtttggatggatcttccaaattcggaagtgataaccagtttgcattctttccttctgccgctctcgcctggagggtaacagaagaagatttcatgaagagtattgctgctatatccaatttaaaagtgcgtgccagttacggagctaccggcaactctgaaatccctgcctacagggcgctcgcgggcatgggaaattacagtgtgattttcaacggggcacgtaattccggcgttggtattgaccgtatcgccaatcctggtttgcagtgggaaaaaacaaagcaggtcgacttcggtcttgaactcggtttattttccaacaggctgaatctcgaactggacttataccgcagaaaagtagatggtatgttgctggatgcgccgttaccatataccagcgggcgtgataaaattttctccaatgttggcagtatggaaaacaagggtgttgagtttgccatcaattctattaatattcaaaacgataatttttcctggaataccaccttcaacatttctgtcaataaaaacagggtacttgctttggccaatggtgatatatcttccggcaacgggatcatcagggtgggtgaaccggttggttctttctttggaagaatgcatctcggcacctggggcagcaaggaagctgacgaagcaaagaaatataatatgctgcccggcgacgtaaaatataaggatatcaataatgatggtatcatcaatgatttagacaggaccatcatcggtaaaggcatacccgacggatatggtaccttcctgaacacctttcagtataaatcatggtcgctgactgtagacctgcagtttatgtatggcaacgatgtattagacaggagcatacattctgctgaagatagacaaggcattgccaatagttataaaaccgtgcttaatgcatggacggaaaccaatcaaaatacgcctattgcacagatacgccctattaacgcctattacaccaccaataacgacagccataaggttaccgacggatcgtttatccgtggccgtaatttgttactggcttatgtatttccggcaaacaccgtttctgctttaaagcttagccgcctgagagtatatgcatccgtacagaattttttcctggtcacaaaatataaaggatacgatcctgaagtttccaactccagctctcctttcgatcagggtttgaacttgtacgattatccgaagccacgggtatttatgctgggtcttaatgtgggattataatacagaataaactttaaacgaaaaattatgaaagcaacaataataagatacggactgctggtattaacaaccggtacactatggataagcggttgccggaaatttttagatgaaacggatcccagcaactatacagaagatacttattttacaaagcccgaacacgcaagaagttctgtaaacgccatttacgccagtttacgggaaccgatgtccggtgagtttggcggcggcccctggaccatgacagaatttgccaccgggcaggccggtactgatcttgggcaggctgttaacagctactttgtaaaagacctccacaataccgccgataatgcttatggagagaattactggagaaactattacaaaggcatcagcaatgctaatttatctatcgccaaaataccaggtatttctatggatgcagcagaagccaaaagcctgctgggcgaagctcactttttacgggcctggtattatttcaacctggtgcaaatgtttggcaatattcctttaattacggagcccgttgatttgaaatccgatcagttaagacccatgcaggccgctccggaagatgtttataaattaattgtagatgatttgacaacagcggaaaatgccgggttaccctggaaggacgccagcggaaaagtatcgctgggagctgtaaaatcattgctggcaaaggtgtatctgacaatggccggctaccctttacaaaaaggagctacctactttgacctggcagcaaaaaaagcagcagaagtattggattcaaaacaatttaaactatttgacacctatggtgatttgcataatcctgcaaagaaaaacatagaggaaaatatttttatgatccagtataaaacacaggtcattcccgggtcctggcaaccgctcattattccttacaacaaaaatatttctgcctattctgctgaaacaggcggtatttatgcaacggccgactttgtaagatcctatgatgccgctgatctgcgcgccaaggaaggtcagttcttttttaccgaattcaccaaccaggacaaccggaacctgaaggtagaccttggcggatattttatctacaagctttttgacgtgacggcgcaaacaactaccgccaacagcgatcttaactggtcgttgatccgctatgccgatatcctgctcgtgtatgctgaagctgctaacgaagtaagcggtccgggtgcaaaagtgtacgatgcggttaaccaggtaagggcgagggctacattacaggcgttggcgggattgtctaaggaccaattacgggaagccatctggcgggaacgctggtacgagttgtgctttgaaaacattacctggtttgatatggtacgcctccgcaaagcattcaacctcactactaaaggctttgataattatgtaggacataaattctcttatggaccggttttaacggaaagagaattgttattcccaataccaagtacggagttaagaaataaccccaacctggtacctaccaaaggatattaatatcggatagttgattacaccggtaaggcactgaagaggtatgccctctctagtgccttaccggttttagtatcaatcctctttgttatctttattaaaaattcatgagacatgatactgcaatatttaacacaggaattcgaacatgaagtaaataacacacgtaaattattacaagccattccagaagatgacctcggttacaaaccctctgaaacttcctggacgatgggtgagctggcacagcacattgccaccatttaccactggtactccggcacattcacgcaggacgtgtatgatttggctaaggatcgcccggaacggggcgacacgaacgatatcaaagctaccctggcgttttttgaaagtaatgttgagaaagccaggactgcaataaaatcgcttaccgaagaaaaattgcaggacaactggaccatgaaagcaggagaacgggtaattctgggtccggtgccgaggggaatcgtagcacggggatttctttttaatcatatctatcatcatcgtggagaaatgattgtttacctgcgtgccacaggaaacaaggtaccgggtttatacggccctacttatgaagaaagcaaaaaaagctgaaccatatcaaaggaggcttgaaaatcatggatgttcaagcctcctttgatgtagtgttaatttgtttactccttttctattgctgatctccagcgtataaacgcccttagtcaggtgactgttacttagctacattatcatcccttgatttaacaataaaatcttacaaaatccagcaataaaattctaacttaaatactcatttgaaaacctaatattaaattttaacccatgagaaaagccatctttcttagctttctgtccgcactttttttattacagagcaatgcaactcccacgtccggcagaaatgatgacatcagcagcgcccattgtattgttcccggaaaatccagcaaaatcctgacggaatttagtgtccgaataacactggtagacatttatggcgcgccggttacaggcggcaccgggttacgcggttactgggcaaaaaatgtagccactggtgtgtactattatcccggcggccaggaagacgaggataaatttgaaaacctgccggccggcacgtatacctttggtgcgtacccgggcaactgggaaggggctgtatcctctactgttacactcagcagcgatgctgttggacccgatggctatattgttgtaccgttaacctactgggtggaataatttaaccagctcattataaagaagggttgtaaatctttcgatctgcaacccttttttataagcgcctgtttcaggctatcgtatatttccataacctgacaatttaatcagttgcttcacatctttaatacagatatttttcccctgcgtcgttaaaataccggtggctttaaattcggataaaaacctggtgatgttttcgttgccggtacctaccatgttggccaggtcactacgggaaagattgatcaggatatcgtttccggaaggagtttcttctttgaatttctcccgtaaaatgattaatactatagccagtcgttctttaacagaccgctgtgcaaatacggaaacgctgtttgccagtacagtatattcatgactgagcgttttcagtaacctgcgtggcaatacatccgaccggtttaaggtagccataaaatcttctttgggaataaaagaaaggaggcattcttccagggcagccgcagcatcagggtaacgctctcctgctaaaattgcatggtatccgattaattctcctttattggcgacgtatattatctgttcttttcctttatggtctacgtgatactttttaatctttcccttttttataaagaaaatacctgacgccactgttccttccctgaatattacatcccctttacggtatcgctgttcctccatgtgggaacagagttccgcgtactcatcttccgggagatcagttaaaatggattgagatttgaaattccatttatcaataggaaacaggccagctagactcataaaaacgacctttgatttatccgtgataagcaaatatcatcaaaggtacccttacggtatgaaaatgtcaactaattcccgtccacggggcattgttcttatgcgacgcacccatttaaacaagcggatccggaaaacgtcgtaaaatacagcaatagcgaggatggcagccggtaaataaaaggtgaaatactggtatctgaggaacacgtatcctcctgctattccaccagccaggaaaaaggcgatgatgacaagccgcagtgtgaccttcttttttacatgatccacatttttaccatgagcagctgccagcgtatacaggtcgattcccaggtcggtgaacatgcctgtaagatgtgtagttctgacaacataaccggagatggtggataccaaagcattctgcattcccattgcgaaaagcaaactgccggcgaagagttctgttttgataatagactgatcaaatgagcttccgaagcttcccacctgcaggagaataatgatctcaatcacgatacacgccacgttaccccatcgtttgtttttaccggctttcccggttaagaagcttgagaaaaaagccccggcaagaaaaaggatcagccataagcctaccatccttgcggcgcgcagatcgccggttgccagtttgtgagccagcaatgcggcatgcccggtaacattagtggttagcacagcgaaggcaaaaaaaccggccgcatttacgatacctgctgtaaaacatagcaacactgccaattgcaggttgtgcttataatttctctttcttccaatatggcgtagcatttattatctccgtaatttttcaggaagacaccatggttcttcccctgcaaccaacaaagttactggcaggtggattccgtttaactgatatttttcaagataatgattgcaaaaagtcacttttacccggaacattacccccaccccatttgttaatccgggtactgaattgctcatcttcaatcattcacccatgcaaaatgccaattccaaacaggatcaatggcctgtgctgacctataacgactggaaagataccttagcgacagtacacctgtggacgcagatcgtgggaaaaatccgcctccggaaaatgccgtggttaaaccactcgtggcatgtgaccttgtatgtaagtccggatggactcagcaccggaagcgtgccgtaccaacatggcatattccagatcgactttaacttcatgcagcaccagctggtcatcatcaccagtaccggcaaaaaagaaatagtggaactgcggcccagaacggtggccgacttttaccatgcgttatttgaaaaactgaaggagctggatattgatgtgactatttacacagttcccagtgaaatagcggaggcgattccgtttgagaaagatgaggttcaccagtcgtacgaccgccaaaaaatggaggacttctggcaggccctggtgaaaatccacaacatcttcacccgattcaggacacgtttcaccggcaaatgcagccccgtccacttcttctggggcgcattcgacctggcggtaacccggttctcgggaagggatgcgccgcctcaccagggtgaagcccccaatatgccggcagcggtaatgcgggaggcttactccaaagaggtaagctcctgtggattctggcctggcagtgaacagtatccgcatgctgttttttacgcttactgttacccggttccccctgctttcagcgaacaacctgttcaacctgccggcgctttttacagccaggagatgggggaatttatgttgccttatgaagtagtacaacaggcaacagatccggaggaaacgttgctcgcgttcatgcagtcgacctatgaggcagcggctaacacagggcattgggaccgcgcagcactggaatgcgatctttcccgtttggaggttgcctatgggtgttacaaatagactccactatttttttgcaaaaatatttggtaaaaagttttagctgcttatctttgcaacccctgacacaatatcagttgcccagatggcgaaattggtagacgcactgtgttcaggtcgcagcgcctgcaagggtgtgctggttcgaatccagttctgggcacgaaagtggacaaatcaagattactcctggtttgtccatttttatttttaggaagacccgtgtccagcgcgtatattagctttactgcttcattcagtcgggcggttcgataatggcttccatcaaaaacgagtttttagagggaaatcgaaccacacttccttttacaattgaattattctcctgtcgcattaacttccaattaacgcttataattctttcgttatctagttttcaggttattcatctaacgtgagaatctggcattcctcaatactggattgctaataaattaagcacaatggcaaaaggaagaagcgtaacgtcaatcgaagagtccttattcaaagagctttcgcagcttattgagcaaagtcaacgacaagtattttcacatgctaacagtactcttacaatacttttctggcagattggccagcgcatcaacaatgaaatccttaaaaataaacgggcggcgtatgccaaacagattgtgtcgacgctgtcgacacaattgaggagtcaatacgggagaaactttgagacttacaaccctattttatttgtatcaatgtcgaatttcctcaagcgaaaaaataagaagggacataaacttatcccactgctttattcagtgcaatgatcgccgctttgaaatgttcccgggtaatcacgaactggaaattaacctttctcaatgctactccaacgcttaatatattgatatctgcgttggccagtgcagcagtagctttggctaacaatcccggctgatccatattagaacccagcaaacataccattgctataggttccaaagtcacatgttcatatttttccttcagttccttcagcagctgctgtttcaaatcactttcccaaataacgatactaatgctgttggcgctggtagccttaaaagtatagctgacaccgtaacgggcaaatacctgcatgatgtcgagatcgcttcctacggcgcctaccattagcggatcatagatgtcgatgagcaattgctggtctgagccggtgatgacctctaccctcttatgttcagaaatataatttttagtgatcagcgtgcccggatgttcaggttcaaaggtgtttttgatgcgcaggttaatacgcgatatttccagtggctttgcagctttaggatgaatagcctccatccctacatcggccagttgatctgcaatatcgtaattggtatagccaaccggtttcacgttttctatgcctaccaatccgggatctgcggttgacaggtggtattctttgtggataatagcttcctcaggccggagtagttctgctattctgctgaaagttacttcggaataaccgcggtcaaattctctcatgatcccttctgtccctttcacgtaccctgttgcaatacacaggcagcttttaagatcgagacgctcaaattcttccctgatacgttcatcaatggttagtgaacgtccatcccccaggccgctcaggtctgccagcgctacgttaagccctttgttccgcaggatatttgtcagcataaaagccgagtgactttctcctacggaagccaggatctcacgaacagccagcaggatgccttcattaaggtaccccgaggccaacatagtgtttgcgctgtccagatatgtcagcacccggttaataatgccgtccgtcacttcgttggcttgtgctatgttcagcccaagcggttggtaataggcattcaactctttaaggtgaagccttacagattcaagtgcctgatggtaatcatttccagtggcgaattgatgataggctccaggggcttttgtttttttattctccagcagcaggtttgtcacgccggaaaaagcagaaacaataaagacacgattgtataacctatcgccggtacggccataataaatgatattgtcgattacatctttcagggcactcattgacgtgccaccgattttttccacagttaacatgctgcgaagctatataatttattaatggaataaaagctatcaaaaacttcataagggtaagctacccggaggaaacgggtattattccggcaaaggcgtatttgaaaattcatcgttgaaatgtttaggtactccctacgttcctcacaaccagaaatttagtaccttaacagatgtcaacggtaatgccactgtaaaccggcacgttatgaagcgattgtctctggtctgtttcctgctgatctgtatattcacctgtgcaccagctgtttttgcgggtgacacagcgtcttactatacccaacaactcgataaccgcaacggtctttccaacagcgcagttaattccctgttcctggattccgataagctgctgtgggccgccacctgggacgggctgaatatgtatgatggcaccgctttccatgtatttaattacagcaaagacaacccgctgcacagcatcggcaataacgtggtgctgcaggtaacggaagacggccagcggcgcatctggctcagcaccatcgaaggggtatcgcgatacgataaacaaaccgggaaattttataattacttttacggccgccaacaacgcagccgcatcagcgagcaggaataccggctgatcgccgataccgccggacagctttactgcctgagccggcaggaaggacttacccgctacaatgccgccaccgattcttttgtggtatgccccctcccggctggcaataaccgtatcagcaaagccgtattcgacagcgctaaccacctgtgggtactccgcggcgatggcagcctggagatatatgccgactggcaggcacaatggcccttattacagcgctataccaatgtgcaggccttgttctccgttaacggcaggatctttttcaccaccgccgcgcacgagctgatggcagtatcgggcggtacccaccaggcacaactgcaggcgctgcttccgcatgccgtaaacgccatgactatctacaaccagcattacctgctggcatgggtaacacaaggctttggagagtatgatgcccagttccggcccacgcatcttttgcccgaagccacgcggcagctgcaggacatgaaaatcatatcctgggccagcggcaataacgaacaggtgttatggtgcggaacagatggcaatggcatcatcaaaatatacccgcaaacaaaatacttcggcaccgtaaacaaaattaccggcggcgccgcttttaataaaccgatacgcgccttctgtgccaatggcaacgatctttgggtgggcaccaaaggcagtggcatcatctgtttgtccaacttcacccggcaacccgccgctacgcaccaacagctattttcggcagaactggaagataattccgtttttgcgctttgccgtggcatggatagtatcatctttattggcaccgatggcaaaggtcttgctatttatgaccagttgcataaacgcttcatcaactggcaacaggtacgcggcagcaataaattgccgttgtttggctctgtatatgccatactgccggatgccgatagctccctatggctgggcaccagcgggtacgggctggtacatctgcgtattcagcggcagggtggcgatatcgccgtaacggcatttcaacaatatacttttaatggcagcaacagcggccctgccaatgatatcatttattcactggctcccggccctgctaactcgctatggataggctgccgctacggcggacttaacctgttcaataaaaagcttcaacaattccaggtatttaaggcctttagttacgaaggcagcttatcacataacgatgtgctggcgctttaccgcgataccaaacagcggttatggataggtaccagctatgggttgaactgtattgcagaagcagatatcagtaaaccgcgaccggcatttacccgctataataccggcaacggcctgcctaataataccattcatgctattacacaggacaacgacggcctgatctgggtaagtaccaataaagggctggcgcgcatcaatcccgctactgcggaaatatctcatttccaggaggccgatggattacaaagcaacgagtttagtgatggggccgtttggaaagatccagcgggacggctgtacttcggtggcgtatatggcttcaattattttataccggctaatatacaggaacgccgtgtatatcctaacctgctggtatcaggattgcaactggccggcaaaacaaatgaaaccggcctggaggtattgcaacccggggaatataataccgccgcctatacgctggcaaggcgggataacttttttgaattgcagggaaaagccgtcagttttcttcatgcagaaaaatgtgaatacgcctggctgttggaaggctacgataaaacctggcagtacaccggtggcaatggcaggatcgcttacagcaatgtacctcccggccggtatgtgctgaaagtaaaatggagtaacggggaaggcgtatggacgccgcccagcgtactgttcacccttaccattcaacaatatttctggcttacgtggcctgcgttcctattgtacctggtactgctgggcagcgcgggtactgctttctggctgtaccggaaaaataaactggccatgaagcatcagctggaaatggaacacctgctgcgtaaaaaagaagaagaagtacacgaagaacaactccgcttttttaccaacattgcccacgaactgcaaacaccgctcacgctgatcgttggtgcggcagaacgcagccgggaacaacccggcgacacgtatcaccaggcgcttgtacatcagcatgcctccaggcttacctacctggtgcaacagttgctcgaattccgcagggccgaagccggttttctgaaaaactattattccgcgcttaatatttccgcgctgctggaaaatattgcggccttgtttaaacctatgtgccagcaaaaagccctgcgttttgacactcatattgcaccggctatgattgctgcgatggataaagacaaattggaaaaaatcctgtttaacctgctgagcaatgcctgtaaatataccaaccgggaagaatccatcctgcttcgcgcccaacaaacgaacgactgcctgcacctctatgtgtataattccggtagtcacatctccaacgaacaactggataacttgtttacccgttttttcagtaccgctactgccacacatggcacattcggaacgggcatcgggctggcttttacccagcaaatggtacacctgctcaatggcagcatccgtgcggcaaatgaaaataacggcgtggccttttatgtacagctcccgctttcagaaacgggcaacacttacctgcagcaacaggaggcgcctgccaatcctgttccctcctacctgttgcaatccattactgccgacctgttaccccaggcggcgccggtgattgatcccaacaaactgtcccgcatccgaagcgtacaggaggcgggtaaaaaaagtattttgttagtggaagatgaatacgccatccggcagctattaaaagacctgcttgccggtcagtatattatatatgaagccggtaatgggaatgaagcactggagctgatccggcaaaccctgcccgacctgatcatcagcgatatcatgatgcccgatatgaacggcctggaactctgcgacaaagtaaagaataccgccagtacctgtcatattccttttattatcctgtcggcccgcagcgccatcgaccagcaaacagaaggctacgaagcaggtgcagatgcctatcttcccaaacccttctatgctgatcacttacaggtgagggtacgtaagctgctggaataccgccaacgcctgcacgaaatcttccggagggatcatccgttcggccaactggaagaaaccgatatgccggataccgacaaacagttcctgcaggaactggtacaggtaatagaaaaccggatggatgaagaaggattaaatgccgaagcattggaaaagcatttgctcctcagcaaaatgcaattataccggaagctgaaaacacttaccaatatgacaccggcagaattcatccgttacatccggttaaaacaagctgcccaactcctggtaaaaacccgttttaccgtggccgaaatattctataaaacaggttttaataaccagtcttatttcttccgtgagtttaaaaagatgtaccactgttcccctaatgaataccgcgaacaacaaaccatggtatagtttggcccacaagacaagtaagcaaccaaccacttgattatcaatatataccaattataaattctcccaattgtacagttatttgtaactatagtacagtcgcttcccgctccttacacctatctttagctcatccaaatcaatcaaaaatattccggcgtatgaaaaaacaggtgatgcacggcctgtaaattccattcaaatccaacgttaaatacatttctcaaaccggttcttccagggggacggaaccattaaattcttacgaatgaaaaactggacacaattaatgtcagctatgatactgctgctgcttggcggggcaacttatgcccaggtgaaagtaagcggccgtgttagcgacgagcagggtggcgccctccccggcgtcaccgtagtacagcccaataccaaaaacggcgctgtttcaggggtggatggcagctataccattaccatcagcggcggcggtcctgctacgctgcagttttcctttatgggatttctgaccaaaacaatcccgtactccggcagcggcgccctcgatgtaaccctgcaaaaagacgaagtggccttgaaagatgtggtggtaatcggttatggtacgcaacggcgaagccaggtgaccggcgccatctcctccatagatggaaaaagccttgctaaaacgcaggcggtcgacctcagcacagcgttgcagggacaggcctccggtgtttccgttacctcgcctaccggcgcacccggcaccgaagccgtcgtacgcatcaggggtattggctccctcagccagagcagcaacccgctttatattattgacggagtgcctatgaacagcgggctgaacaccatttcacccaacgacattgcctccattgaagtgctgaaagatgcggcagcggcagccatttatggttcgcgcgcagccaatggtgtgatactcgtgaccactaaaacaggacaagccggtaaaaacgaaatcaatatcgacatcgcctatggcattgccaatgccagcgggttacccgatatgctgagtaccagccagtttatagaattacaaaacgaggcttttgccaacgatggctcttccacccgcaaccaggacgatgccgccaaattgcccaataccaactggctgaacgccattttccggcaggcgctcacccagcgttataacctggctttctccggcggctcggataaaacccgctattacctggccggcaacgtagtaaaccaggatggtactatcgtaaactccaatttcaaacggtacgggctccgctccaatgtaagcagcgaagtaaaaagctggctgcgggtaggtgaaaacctgaaccttacctacgaccgtacccaggaaataggcgcttccggcgatggcgcccgcccaggcagcttaccaggcgtagtacgctatgcgcttatcaggcccaatgcgcttccactctatgatgataagaccggtttttataccgacctgccgccggcggatctctataaaaatcctttgctctatggtgatggaaaaaatccactggccattgctgattaccgtacccgcaccatgagcaaataccgcctgttgggtaacgtgtttgcagaagcccgctttctgaatgattttaaactccgcagtgatctgggtaccgatttttatgtggcggaacaacagcagtacagcgggcaaatacccggcgatcgtacgctgatgcaggataaagacaaagggctcgataaattccgtaaccgctatactacgtataactggaccaatgtactcagctacaatcacctgttcaatgaaaaacacaatgtgggcgtaacactgggttccgaatatatttcttccaaggtagactacctcgcagcatcccgtaatggctacgacaatcgcgccgatgcttccgccagcctgcgttacctcgactacggttccgggcagcaatttaacagcggcaacctggaagaatgggcgctgatgtcttacttcggcagggttacctacgcatatgataacaaatacatgctgaatgtgaacatgcggacggatgcttcctcccggtttggcgccgacaaccgctggggttactttccctctttctctgccggctggaacattgcccatgaaagtttcatgaaagatgtgacctggctgaatgaccttaaaatccgcggaggatggggacagctgggcaaccaggatatcggcctttatccatttgccaccatttactccaccagcaataatattttacaggtaatcagccgtggtaaccccgatgtgaaatgggaaaccactacccaatccaacatcggtgtggacgcaggtttcctgaaaggcgcactgaccctcagcgtggattatttcaacaaacaatcttcagacattctcatacagctgccctcttcctacaccaatggcgatgctacgccaccctatgtaaacggcgctaaaatgagcaacaaaggactggaaattaccgccgtctataaacagtcgttgcagaaagatctctctcttaatatagccgccaacgttaccaccctgcgcaacaaggtagtgtcgttgtacaaaggccgtgaacagatcttttccgccggctccggtcgcgtaatcctgcgggaaggccagcctatcagctctttctatggttacaaaacaaatggtttattccagaacgatcaggacgtagcgcagtatacaaacagcaaaggcgaactgtatcagcccaatgccaaacccggtgatatccgttttgttgattacaataacgacggaaaaattgatgatgcagaccgcactattatcggcaatcctaatcccaagctgctgtacagcctgaatgccggtatcaattacaaacagtttgacctcaccctgttctttaacggggtacagggcaaccagatctataatgaagtagataacatcatcaacagtttcgacggacggggatttaataacaaggaagatttctacaatgatcgctggcatggagaaggcaccagcaacaaaacacccagggccaccttccttgacccaaataacaaccgccgcacctccgaccgctatgtggaaaatggcagctacctgcggcttaaaaacgcgatgctgggttataccttgtcgccttccctgttgcaacgcatcggttttaccaatgcacgcatctatgtaagcgctcaaaacctgtttaccattaccaagtatggcggcatggatccggagttgtataccaacgagaacctcgccaactatgctgatatggcggtgggtattgacatgggtacttatccgccttcccgcacctacacttttggtttgcaattcggtttctaggaatgccattttattaaaatcaacacaccatgaaaaaattagttgttattatatcaattgccgttagtatagtaagctgcaccaagcagctggaaaaattcccgcagggaaagctcacaggcggcaatgtttttacagaggccaatgattttgtaatggctactgatgctgcatatctgcccattaccaaccgtttccgcggcgactggggctgggatgatggtagcagcataccgcgcgattgggtaataggcgatctgatgagtgatgatgcggtgaaaggcggcggtagtttgggcgaccaggaagacatgcggcggatgcagacctttggcatcttcccggaaaataataatgtgctgggcatctggcgttttaactataaaggggtggacgcctgtaacacgctgctggcgcaggacggcgccggcgttcccggcctggatccggcgttgctgaaacggatgaaaggcgaagcctattttctgcgcgctttttattacttccggctggtggtcaactttggcgatatccctttgctggtgcctgaaaaaaatatgaccgataataccgtgcgcacacccgtggcacaggtgtatgaacagatagaaagtgatctggcacaagccttcggtatgttacccgccacctatgatgctgataactaccaacgggctactaccggcgccgcgcacgccctgctggccaaaacttacctgtaccggcagcgctggcaggattgcttaaaccagattgcggaagtggaaaaaggtaattaccagttgctggatcattatgaagataattttaacggtgttggagaaaaggcaggtgagatcatctttgctgcccgtcatgatgccggcaaaacaccttcccagggatctgtactaaatgctgtattcgcaccacagggcaaaggctggggctttgaaattcctaccaaagaccttgtaaatgcttttgaaaccggtgatccccgcagggccgccacccttttccaggcaggcgataaatacctcgatggcagcaactacgatccggcctggtcgccggtaacgggtttcaatgtgcgcaagtttatgagcaatgtaaaccccatcgatgatggcggagtagactttgcgtatatccgtttgggtgatgtaatactgtggaaagccgaatgtcatgctaacctcggtgcattccccgatgcacgcgccgacctggaaagaataagggcccgggcacgcaagtatgcagccaacccggctactgccctgccgcctgttaccgccaatgataaaacagcgctcctttccgccatccaacatgaaagacgcgtggaacttgccatggaaggccatcgttattatgacctggtaagatggaacctggcgcagaccatactggccaaagccccggatgccgatcccctgaaaggatacaaggactatggcaatggctggcaatcttttaataagctgttgcctatcccgcaaagagaagcagacctgctgaaacttaatcaaaacaccggctactaatatgaaccaggttaccgctaaccgctttatcgaaaatccattgctgaaaccgtcggatgtacggcccagcaggccaggcctggaagtagcctgtttgctgaacccgggcgtttttgagtacgacaataaaatatggctgatcatccgcgtagcagaaaggccgcaacaacagcatgatatcatttcatttcctgtactgctcaatggcggaatagaaatcagggaaatctttaaaaatgatccgcacctggatgctaccgacccgcggatactccgttataaaggcgacgactacctcaccacgctttcccatttgcggctgttttgcagcgaagacggcattcacttccacgagcctgaaggttatcctcagctgcatggagaaggaccgctggaagcatttggtgtggaagactgcagggtaacaaaaatagaagacacctattatctcaccttcaccgcagtatcatcaaatggtgtgggagtaggcatgcgcactacccgcgattggaaaacattttcagatcaatgcatgatcatacctccgcataataaggactgtgcattatttgatgaaaaaataaacggcaggtactatgccctgcaccggcccagcagcgtggatcttggcggcaactacatctggctggcacaatcgccggatggggtgcattggggaaagcaccaatgcttaataaggacccgcccgggttactgggacagtgcaagggtaggcgccggtgcgtctcccattaaaacaacagacggatggctggaaatttatcacggcgccaatgaaaagcaccagtacgggctgggcgccgttttgctggaccttaacgatccatccaaagtgctggcacgcagcgatgatcctattatgatacccgaagccccttacgagcttaccggctttttcgggcaggtggtttttacaaacgggcatattgtgaaaggcaatgaagtcaccatctattacggcgctgccgacgaagtagtatgcgctgcaaggttttctatcggggaaatactttcatccttaaaaagataacaacttatgctcaaaaacctttctgcagaaataaaacatttcaaccagcagccgcaaaacttccgtatactggtgctcaccaatatgatttatgcactcgtactgccggtgatcgacatatttgtggcggcttatgtgatgcgtaactctaacgaccctacgaaagtggtgatctatcagctcaccatttacaccggtatcccacttactttcttattaaatggttttttgctgagccgtttcaacattaaaacattgtattcggccggtatgctgctgagcggcgtatccatgatcgtgatgatgtcgctcaaaacgctggacctcaccggtattggaattgcgggtattattatgggcatgtcgtttggcttctattgggccaatcgcgactacctggcgttatccatcaccaatgatcaaaaccgcaattattactatggtcttgaaacgttcttttatactatcatcgccgtagtagtgcctatctgtatcggctggtttatagagtccggcggtgaaatcaatgtcaacaatgcctaccgcattattaccgggctggtatttatcatcaccatccttgcttcggtagtatgcttcagggggcagttccacaacccggacgaaaaaacgttcctgtacctgcgcttccacccctactggcgcaaactgctgatgctggcatctttgaaggggttagcacagggttacctggtaacggcgccggctatgctgatcatgttgctgttgggaaaagaaggggcattaggcaccgcccaatcggtgggcgccatcattgccgcggtgctgatgtatattattggcagggcggcgaaaccggaacaccggatcaccatttttgcaggaggactcatatgttttgcgctggcggctattttcaacggcgccttttataacgccacgggcgtggtaatcttcatgctattccttttgctggcaaaaccgctgctcgacatggcctatttccctattcaattcaacgtgattgatattctttccaaaaaagaaaaacgtaacgtatacgcctatatccttaatcatgaagtaggcctgtatgccggtcgcttcctgggcgccggtacctttattttcctggcttactacttctccaccgaagtggcgctgcggtatgccatcattatcattgccatactgcaactactttccattgcggtaggcaaaagtattatcaaagaaggaaaagcgctgatcaaagaaactactgaaaaaaccactgtagtcgtataaattttataagcatggtaaaattaacaacaacggggttcgtactctgcctgctatggatggcctgtaaaacaactacgccgtcgccggtagtgcagcaacacctgccccgcctggactccatggccgatatgccgcagcccctacagatcatagactggtatgccctggcccggcagttcgacagcaccgcttacaactttaacaccacgggtccacattggccactggtgtggtgggatagcagccggcacaattttgatcagccggtagtagggctttatactgcgatggacgatcagcgccagggtcccctgcatcacaagggaatcttccatgaagcgctggctaccatgggcgccacgctgggtgctacattggtgggtgttgacaaaagccggcaacagggtattaactatgtggcgatgctaaaaaattatttcaaccgtgaaacaggctgggatattatgatgaataatacctgcccggaagtagccttactcggcggtggttatgggcgcgattggtggtatgatgtatatcccaacgttcttttttatggcatctatgatcattatcccaacatgccgggatttgatacgctggcgcatcgcattgcggaaaagttctgcgcggcagattcggtactgaacggcaactatgatcattcctttttcgactatgcacaaatgcagccaaaagataaccagatctgtaaacaacaggacgccgctgccggtcatgcttacgtattatatgccgcctacaaaaagtttggcgacccacgctacctgcagcacgccataaaggccctgcaaacgctggaacagcagccacacaataccaactatgaagtgctgatgccttttggcgcttatatggcagcaagactaaatgcagaacagggccaacacttcaatgtgcaaaaatttatggaatggacatttaacggcgaccctcaatgccgccagggatggggcgtgctgacaggcaactggaatggcattgacatatcaggtattgtgggcagcacaacagacaggggcggttacggctttctcatgaatacttttgatgccgcgtggccactcgtagccatggtacgctatgatccttcctatgccgccgccgtaggcaaatggatgctgaatgccagcaatgccgcccgcttcttctatacccagtacatgcccgatgagcatgaaactatcccggaaaaagctgctatcacaaaaggtgtgattggctatgaaggcattatccatacttcctcttaccctgaatatgcacacctcaaagcgccggtagcacagggcgatggcccgcaatgggccaaaggaaatcccgatgtatcgcaattcagcgtatacggcagcgggcatgcaggaatcttcggcagtattatccgtaccaccacggtaccaggtatattacaactgaatttgctggccacagattttttcagggagaaagcttacccgtcctatctttactataatccctacgcggaagaaaaaacagtcaccataaatgtgggtgatcagccggtggatatttataatacgattacccggcagtttattgcccgcaaagtgaaacaggcttacaacctggtgttaccggggcgcagcccggcagtactggtatttacgccgcccggcgggaaagtaagtaaagtgggaaaccggttgctggtaaacgaagtaacggtcagcttttaattaaaatacactggccaaacagtttaaacactgtctggccggttttcttccaataacctgctattttccgctatagctttgcgcccagctgttcatataatcttcgagcacattcaacggcatatctccgtatccgagcagggcatcatggaattctttcaggctgaatttaccgcccagctttgctgcaaatttatctctcagcgctttgatctttagttccccggtcttgtaagacagtgcctgtcccggcatagccatatagcgttccacttcggcggtggcaaccggttcactgatagattcatgctgcatcatatagacgatagcttcctcgcgggtcattttaccggtatgaatagccacatctgttaccagtctcaccgcccggtgaatttccatattcaatgcgcccatcttctggtaaagatctgtgtagcaacccaattgttctccgagtgattcacagtataatgcccatccctcaaagtaggcatagaaagccggttgcctgcggaatgccggtatatcactattttcctgctgggatgatatctgaaaatgatgaccgggtactgcctcatggataaaggtggcttccatgccctggaaggtaacgttgatttttgttgcatcgggaaccggcacataaaagacagctggtatattttcctgcaggttccccttgatataaaaggggccgccctgtgaggcttcgcggtaagcttccacccttttgatcacaaaaggagttttaggctggtgaccaaataatgcagtcaaccctggctgcactttttcatcgatatgacggtatgcttccagcacctgttccggcgttttgaaaggcatgaagcgcgcatccgttctcaggtaatgaaaaaaatcagctaaagaacctttaaatcccacctttgtttttatgacttccatttccccggtaatacgcgctacttctgttaatccggtctggtacaccttttccggggtaagacctggagaggtggtatacatgcgcagataataccggtatatcctgtttccacctggaagaaaagacaagcctgcatgatcctgtgcggcgggtagataggtatctttcaggtaggtggccagtttccggtaagcggggatcatgctggcggtaatcacctggtgatataatgtagtgatccgttgttgttccgccgctgtaaatgaggccggaaactgcgacaggggtttataaaagatatttttagcggtgtccctttccgccagttcttccatctgcgggatcatttttactaccagcgctttagggagtacgatacctgcacggatacctttattaaagtttgcgatggcggtgtctgtccaggccatgaacgccgtcatgcgttttgaccagttctcataatcctttaccgtgttaaaaggttgtgcgccacctcccgatccgaattgtgccagttccagtggtgtagatataaactggttcatcggcatatattccaggtgcagttgcaatgattcctggccggtgttgaggatatatttcaggatgtcataggagatcctgtccggcgtatttaatgcggtgcggttaacctgtttcaatgcctcgaggtatttcccgtagaactttccggcaacagccaccttgggaccggcgccatattccggcaggaggtcgtcgtaacggtgatcacctgctgatgtagcttctgtggggaacagttgctggcgttcattatagtagttatcaaatagctggtgcagcttttcattgcgctgttgggctccggcgacggtaacatttaatatgctcactattaccaggatgaaccaccttacttttcttttttcagacatgactgctttgtttaccgggcaaagctagtaggcatggggagtaaaaaattgtataaaattagcctgttgtcagatgctcctgtattgcttaggaagcaaacccgttacatgccggaacgttttggtaaaatgcgcctggtctgtaaaaccacactcataggcaatttccgtaagcgaatagttgcccttttttattaaaggaaatgcccgttctattttaatgcgccgcaggtattcacctgctgagcagccgaaatacctggggaaatattttgaaatggtcacaggatgaagttccaggtgggttgccagcagggaaagcgacagtggctgattccaataatcattcatgactgtttttatcttcttcgtccattcggggaaatatgcctctccttctttaccgggatgcaccaggttaatgcatagctggtctatcgccatcggcgagtctgcatcatccaggtaatgttctttcataatcctgataagcccggtggtattaagctggttgctatcttcaaacatcagggatgccgatggaagtgataatccgaaggtgttgaaaaatgcggcatccagttcaagattaaatatgcgtgtgccggggcggtagtcaacattctggtgtacgatgccaggataataatacagtcccttaccggcgtattgtatatcggaattaccgttccggatctctttgcttccacctgccagtatatgagaaaaatgcggattagcgtgatagtgataggcggaactcatatcaggcacaaaagcggtttcactggtaataatagcaccgaatgtccgttcctttatttttgcgccaacgtacatccctttttcatactgaactggcttatgcataattacattattttaaatttacgcagtatcaacctgaaatcttggctgatattgtccttccgtcaaagctacggtttccatccatagcgcttttaacagatcggtgcttgccattaactcctgtgcccctgtaccagcatgccccaatattttactgagtgtttcttctacattaaaaggcgaccggttaaaagctgttattagccgcatggctcttttgtcgcccagcggatacgtttcatttattgcgaacaaggcgtgggtaagataattggcaattcttgtaaaacaaccaacggtattataagtatccgctgcagccgcaaaagcataacattgtattaatgtaaactccgccagccagagacagtcggatagaatggtttgtttcagcttagcgggataagtagtaacctgatctttaagcttcctgataatgttttctggatcaaataaaggcttacaaacctgtgtttcacctaagtaaatcactgatctgaatccgtaaggcggttgctgatcaaagttatgatgccagataccattggcggcatccgtaatggtttgttgtacctggtcgatattgcgatagagcagatctacctttccggcagctgttgtgatccatgccccgccattcacccagggcccccattcataaaaaccggtaaccagtggcaaaccctgtatggaaaaactattggcgattcttctgatactttctgtatcaaaaggatgtttctcaaagtagtacagcccgatatccaggtctgatttttcatgggcttgtcctgccgcctgtgagcctcccagcacaatagccactatgcccggaacatctttaaatgctgaagttattgcatccagtattatccttttttcatccggatcagatttcatctcctttacatttttcttcgataaaatatatcctctgcagcagttcggatcttctgatagccgaatgtaaataaaactattataagttatagccgtaactgacatttaactgatctcttcctttttcagtggcctcaatattaaccggagcgactgatcttttgtaaagtaagcgatcagccagttataaagtgttttgacacggttgccgtaactgatcagaaaggtgaggtgaatgaaaagccagataaaccaggcaataaaacctttgaagtggagtttgggtttggggatgtctgccacggccttattccggccgatgatagccatattacctttatcgtaataacggaacggcttacggttctcctgctttgcgagcgccaggaaattctctgcgaggtggctaccctgctgtatagccacctgcgccagctgcggatgcccgttgggaaaagcagggtcggtggtttgtatacacatatcgcctattgcaaaaatatccttcatgccctttatctcattgaactcgtctacgatcagtctttttccgcgaccataacattccgccgggatgccttccgttacagttgccgttactcctgccgcccatactaccgttttggtggcaatggtttctccgttggaaaagatcacggtatcatccacataatcttttacctgcatacccagttttatttccacacccattttaacgagggcatcgtaggcgtcccgctgcgactggtcactcatggcggccagtactttggagatgccgtctaccaggtaaatatgcgattcaaatcctttccccgctatttcgggatagtctttcggcaccacttcctttttcaattccgccagcaggccggatacttccactccggtagggccgccccctactacaacgatggtgagcagcctggttctttcttccggatcggtggtaagcgctgccttttccattacctgcaggaaatggttgcgcagttcgagggcatcgttcactgttttcaccggcttcgcatgccgctgtacgctttccatgccaaaataattggtagacgtgccaaaagccagtaccaggtaatcgtatttcaattcagtggtagagagtattacttttttttcttccggtattactttctgaaattcaccgatcacaaaacgtgcgtttttgtttttgcgcaacagtttcctgaacggataactaatatcagtaggatctaaaaagcccattgacacctggtaaaccagcgggggaaaatagttatagttgttacggtctaccagtgtaacggtatattcctctttgcgggccagtttcctgaccaggttaacgcctgcaaatccaccaccaatgataacgatatgtttcataatatgaccttttatctgtgttgttaaaacagccaaaaggccattttgttgctgtatggtccgcaacaacaaccaggccaccggaagaaatgccataaaaatcgtccgttcatttaccggagcagacacacctgtcgacacaactccccatcctttggataaatttcacgttataataagctgcgagatggacaagaataggaactgagccatgaaccgtttcccttctccacaaaatatattttttattttataccaaatggtatatttttgctttgtcaaaagaaagagggatatgaacaaggcagagaaaacaaaacagtttattgtggagatgacggcccctgtttttaatgagaagggctacaccggcacttctttgaatgatatgacgaatgctacagggctgacaaaaggaagtatttacggcaatttcgctaacaaagatgaagtggccctggcatgcttcgactacaacctgaagaaagtaaacaccattatccggcaggaaatggacaaaaaaacaaccagcagggataagctgatggtgtatgtgcatatatatgagaacttcctgaaacacccgttccctgccggcggatgccctattctcaatacagcagtggaagcagacgacacgcatcctttattgaaacaaaaagccgcagatgccatcctttcctggaagggcgttattacagggctgatcgaaaaaggaaaagccgaaggggagttcagtgaagacgtaaatgccgaacaaactgcactcaccatgatcgctaccattgagggttgcattatgattgccaaattaaccggtaagataaactaccgtaatactattatgcagtcggttggaaaaatgatagacacactataacacttttttttctttataaatataccgattggtataaaaaacaaacacatgaaaacaacaggaaatactgtacttattaccggcggcagcgcaggtatcggactggaaatagccaggcaattatcacaacagggcaaccaggtaatcatcaccggcagggacgccgcccgcctggaaaaggccacgcaacaactgccgggcgtgaaaggcatcgtgagcgatgtaaccagcgatgaagcagtgacccagctggcagccaccctgcacaaggaatatccgtctttaaatatcctggtcaacaatgcaggccgtgcatttgcctatgagttgtcggacaacgcggatgccgccggaaaagcagcggaagaaatggatactaatttcttttcggtgatccgcctcaccgaaaaattgctgccattactcagtcggcagccggaagccgccattgtaaatgtaacctccattgttgcctttgcaccgggcgtacgggtacccacttattccgctaccaaagctgcgctccggtcctacacccaatccatgcgggtcacctttcctaagctgcacatctttgaactgatgcctcccctggtaaataccgatttttcacaggagataggcggcattaacgggatccctccttcacaggtggctgctgatcttgtaactgcactcggaaaaaatgaatatgaaatccgtgtgggcaataccgaattgatctaccagttatcactcagcaatcctgcagccgcactagccgctgtaaacggcggtggcgaataaaaaaatttatataataatataccaaccggtatattaaatagcagcaatgaaacggacagtactgatcctggtggtgattacagcggccatcatggagttgatagacacctctatcgtaaacgtagccttatcgcatatgagtggcaacctcggcgccacgctggaagacacttcctgggtcattactgcctacgccattgccaacgtgatcatcattcccatcacgggctttctcgccgcgaaactgggccggcgtaattattatatcggctccatcgtcgccttcaccttcttttcactgatgtgcgggcaggccaccaacatctggatgctggtagtattccgtttcctgcagggcatcggcggcggcgcgctgctatccgtatcgcaggtgatcatctttgaactgtttcccaaagaaaaacaaaatgtagccagcgcactttttggcgtaggcgtgtttattggtcccacgataggccccaccctcggcggttatatcaccgaattttattcctggccctggatcttttatatcaacgtacccataggtattacagtggcaacactctgctatatactcctcaaagaacccgctaatgtgcctgcggccaagcggatcgactggaccggtatcctcctgctggccgttggcgtgagcgcattgcaaaccgtactggaaagaggggaaaccgacgactggtttgaagcgccctatatcacctggctttccgtgatcgccactttcgccatcctggtatttgtgtggtgggaactgcggatcaaagacccggtggtaaacctgcgggtgctgaaaagcaggaacctgagcattgccgcgatattgacatttgtttccggcatgggcattttcagctctgtttttcttacgccggtatttgcacagcgactgcttaatttcacaccgctgcaaacaggtatgctcctgctgcccggcgcctgcttagccataggtgggctcattatttctgcgaggctgctacagcgcggtgtttcgccggtgtttcttattgtagcgggaatgggattatttattctattcagctggcagatgtcggcattgaaccaggacgccggcgccgccactattactacttctctcatctggcggggcgtaggactggcactggtaacggttccccttaccaccctggccgtatcctcactgacgccggcagatattccgcagggcgccgctttaaataatatgatgcggcaactgggcggctccttcggcatcgccatggtgaacacctacctcgccaaccggaacgcccagcaccggtcggatctagtgagcaacctcactaccgataaccctgaggtgaccaaccggttaagcagctacgcgcacttctttctcagcaaaggcgctaccgcaacagatgcccatcataaagcattgaaactcctggatagctccgtgataaaacaaagcaccctgctaagtttcagcgacgcctttttactggtaggcattatattcctggcagcgcttcctttgctgttaatggcttccactaaaaagaaaacagcccatgtaattgtgatggatcattaacacaggccaattaatttgataaaactgaccgaaaaatccaaaaaaaataaaatcagaaaaataagcttaatcaacctaatcctgctccagacaatttccgcgccgaaggcgcgcccggcagggtaccacgatttttttgtactttgcgatatcggtcacaccacttgattcgtctgtttaacggcgatagggtgatatttacttttaaggggaactggatctaacggatgaataatgacactgtacatgaaactgcacttttccaccaaattgccgggggggatgaatctgcatttgaagcattattccacctctatgtgccgaagatcaggccggtaattgcccgtattatacaggtagaagggccggagaaagacatcatacaggaaatattcctgggcatatggctgagccgggagaagctgacagaggtagtggttccccataactggatcttcaaaatggtgtatcaccgctgctacagctggttgcagaagcagggcgtacggaataaggccagccagatcattacccgcgaaagcactgaccactccaatcttaccgaagaaaatattgctttttctgaaaccgcgctgctggtaaagcaggctatcctgcaattgccgccgcaggcgcaaaagatctacctactcagccgggagaaggatcttaaagtcgccgaaattgccagtgaattacagctctccccccaaaccattaaaaattccctggtccgttccctcaaatctatccgggaatacctgaccagccagggcatcaccctcccgctattcctgcttgggtggggtgttttatatttttcttaacttttttttgaaagacataggtactctttggctgctgacggtacgtatatgcagggggctttctgtaattgggtagtccccgtatatgtcaactgaattccgaatgctttaaaacgaggccgttgtccacatcagaaagactaacatacttattggaacaggtacggctgcgtcgtgccaccaccggggagtacagggaactgttacaactgatcagtgaagatgagtcgggggaaataatccgccagctggatgcgtttcatgcgaactggccaatggaagctgctgcccatgcggatcacgaccgcgactactggcagcaggccgtcaaagaaatactggccgccgataagcttgcgcagcagccggaaatgctgccctcaaccccgaaccgggtctatttcctgcaacgctactggtgggctgctgcctgtatcgttgtgctggcaacgggcgcttattatctttcaaagcaagcccctcccacggctgtagtggctacttcccccgtaaaggatattgcaccgggcggcaacagggcggtacttacgctttcagatggtacccaaatccccctcgacagtgcaggcaatggcgtattggcgcaacagggcaatacccggatcaccaagctgaataacgggcaactggcttacaatggctccggcagttcggaggataaagtattatataataccatgagtacccctttgggtggacaataccagcttattttgcccgatggtaccggcgtatggctgaatgccgcctcttccatcagttatcccactgcctttaccggcaacgaaagaagtgtaaccgttaccggtgaagtgtactttgaagtggtgaaaaatgaaaagatgcctttccgcgtaaaggcaggcaatacgaccatcgacgtactgggtacgcattttaatattaacgcatataaagacgaagccagcatcaatactaccttagtacagggatctgtgcgggtaagtgtacaacagcaacagcaaatgctgaaacccgggcagcaggccagggtggcggcaaagggggagtctatccaggtgctggaccatgcggatctatccgaggtgctggcctggaaagccggatttttctcctttaatgatgcggatcttccggctgtaatgcggcagctgtcgcgctggtacaatgtagaagtaacatatgaaggcaagattcctcagcgtgtattcaccggggaaataggccggaacctcaccttatcgcaggtgttaaaaggacttacaaaaacaagaattaaatatagaattgagaatggtaaccggatcgttatccaaccatagttatgaacaatgaacaatgaaaattgggaacaatgaaaaacaccaggctatcgccattggcattccatgcgcattgaataaaaaccggggctgagattggcgtcctaccccggccgtcgttcaatttaatcaacaaacaagtcggtaaacattatttattaattcaaccaaacattgcaaaagtatgcaacttaaggctatttgtaattccggtacccgcagatattggaaatttgcggggctctcaaccaaaacactgttagttatgaagctaacttcttttatgctgctccttgctgccttgcaggtaagcgctaagggcagcgcccaaacggtgacttattccgccaaggcggtgagtctccagaaagtgctgaacgttattaaagcacaaacggggtatgttttcttttacgataaagaggatctgaaaaacagtaatcctgtttcggtagacataaaaaacgcatcgccgcaagccgcgatggaagcagtattgcgccagcagccgttgagctttgaaatccagggcaataccatcttcattacaaaaaatgaaaaaccggcagcaacaccggtaacggccccacctgccgccaacatcacaggaaaggtgacagatgaaaccggggcagggcttccgggtgtatccatcgttatcaagggcacccagaaaggcgttgtttccggaccggatggcaccttccagctggccaacgtaccggacaacgcggtactggtggtaaccagcatcgggtacatcacccaggaaatcaaggtagccggaaaaacacagatcaatatttcaatggcgccggatgtaagtgcgctgaaacaatttgtggtagtaggttatggcacgcagaaaaaggcgaacctcaccggggccgttacttctatcaccacagagcaactgactaacaggccggtaacaagcctgggtaacgcattgcagggtacgatgccaggtatcaccgtcacagccgccaagagcggacaaccgggcagtgatgcaggacaaatccgtatccggggtattggtacgctaaacaatgccgacccggtaattgtggtagacggagtagttaccaacctgagtagtcttaataatattaaccccgacgatattgccaccttatcggtactgaaagatgcggcatctgccgctatctatggttcccgtgcagccaacggcgttattctcattaccaccaaacaaggcaggaaaggtcccccacaggttacctataccgggtatgtgggtaaacaacaagccaccggcttaccggactttttaccttcctggcaagctgccactttatataaccaggcactgagcaatgaaggaaaagcagcacgctggaccgatgcagaaatccagaaattcaaagatggctctgatccttttaactatcctaacaccgactggctcgacctgttttaccagggcagcggtttacaacagaaccactatgtaggtgtttccggcggcagcgaccatacacaatatgctttctctttaggtgtatttgatcagaatggcctcatggaaaaaacaaatgccaaacgttacaccagcagattgaatattacatctgagatcaacgataaaataaaagtaatcggcaatatcgcctttacttcttccggcagaaatgagcccagcaatccttacaccggcgattttacgcagctggtaagacagatcaaccgcatctcccctaccattccttataaatatgaaaatggccactacggctatatttcagatggcagcccgatggcgtggctggaagggaacagcctgaataaatacaataattatgacctgataggtaatgtaggcgtagactgggaaattgtgaaaggactgcattttaaaccctcccttgcttatgtgatgaagatcgctcataacaagaagttcattgctgaccagcaatattatgatgctgccggtaatgaaactttttaccaggggcccagctacgtaaccgacgaaaacaccttcggcaatacggttacacagcaggcattgctggactacaccaaatctttcagtaaacataacttcaaaatactgggtggctattcccaggagctcaccaagttcagctttgatgacggctaccggaaaggcttcctgaataaccagttaaccgatattaatcttggttctaccgacggacagaaagccaccggttactcttatgaactggcgcttcagtcttattttggcaggttaaactacgactacgacggtaagtacctgtttgaagcgaatctgcggtatgatggttcttcccgcttttctcccgccaacaggtggggtttatttccctccttttccgctggctggaatttagacagggaagacttcttcacaccactgaagaaatatgtttccaatcttaaaataagaggttcatggggacagctgggtaaccagtacattaccggtaaagatgatgtcaattacccaagctatccgtactacccgtatattgccactatcaacggaagccagaactatacttttggtggtaccgcggctgctattgccgctggtgtagcgccggttaatggtgccaacgaaaacatcaaatgggaaagcaccaccgccacaggcgtgggtattgatgcgggattcctggacgggaaactgaatttcactgccgactattttcataaacgcacttccgacatcctgttatcagtaccggttggcgccgtatacggcctgaatgcgccggttcaaaacgcaggttctgtcatcaacaaaggttgggagtttgcactgagctatgccagcaacgcaggtgatttcaagtacaatgctgccgtaaacgcggcctttatcaacaacgaagtaaccgatcttcacggaacagggccgattatcgacggctatacctttaaacaggtgggttatccgatcaactccctgtatggatatgaagcagatggcattttccaatcggccgatgaagtgaccaaagcgccttatcaatccaacagaacggctgccggtgatctgagatacaaagacaaggacggcaatgatactattaacagcgccgataaagtatacctcggcaactacttcccgaaagtaacctttggcctgaacctgggcggtacctggaaaaatatagacctgaatatcttcctgcagggcgctgctggcgtaaaaacatacatcgacgccggtaaactgggcagtgtaagttcttctgctggtaaacctacttccgctttactggatacctggacaccggaaaacacttcagccgcgctaccacgcatctggaatggctatacgcagaatgatcccggcggcacgccgtcttccttctgggtgaaagacggatcttacctgcgccttaaaaacctgcaggtaggttatacactgccggaaagaatagtaaaacggataggcatcaacaaagtacgtttctactacagcgggcaaaacatcctcaccttcgacggcctgtataactggatagatccggaagcatctattacgagcagtatctattactacccgcaggtgaaagtgcacacgtttggcgtaaatgttagtttttaacgaaaagcaatcaacatcatgaaaaggaacattctctatataatatttttctctgctgcactgctatctgcgtgcaataaagatttcctcgacaggcagccactggatgcctataacaacgacgttctctggaaaacgcagaacgatgcaaccgctgcactcaatggctgttataaagaatgggaaattgactataccatcctttatatggacgctgtgagcgataatatgtacagccagtattactgggaaggctatacggattatggcaatggcaacattacgcctgccaataccagtgcctccaagcgctggagttataccaccattcagaaatgcaactggttcctggaaaacatcgacaaaacaccgatcgacgaaaccttaaaaacgcagtttaaaagtgaagcccgttttctgagagcttatcagtacttcacgctgtcacagctttatggtgatgtaccgctggtcaaaaacactattaccagtgaagaagctaataccatttcccgcacagccgctaccgaagtacgcaaatttgtactggacgaattggaagcgattgcgcctaccctcccggcaagctacagtggtagcgacgttggacgtattactcagggcgcggctatttccctgaaggccaggctggaattgtatgataaaaactacgccgcctgtatcgttgattgtaaaaagatcatggccctgggttatgaactctttccaaactatcagaacctgtttcgtatacagaacgaaaacaataaagaagtgatcctcgatgtgcagtataaagagaatgactattccaatgccgacatcggcgtaatgccttcttcctcctttggtggctggggctcgctggatcccactcaggcgctggtagacgcttacgaaatgaaaaacggcaaacttattactgatccaacatccggctattccgaaaatgatccgtacaataacagggatccacgcttaacagctacaatcgtatgtcccggccagttgtatgaaggtaaatactacaactctattcaaaatacctccggtgattattataatggggataacaattctaaaacagcttacatcccgaaaaaattcacgtctaacctgtccgactatacggatatgtggaacaccgggctgaatatgatcgtaatccgctacgcagaaatactgctcacttatgccgaagcacaaattgaatcaggcattattgacaataccgtgtatgatgcaatagatgccatcagaaagcgcgctggcatgccagtggtagacagaaccgtgtataacaccgttgataaaatgcgtacgctcgtaagacgcgaacgcagggtggaactggcactggaaggcttacgctggtacgatattcaacgctggaagataggcactgccgttagatccggcaccgtatacggcgcacgactgggtactgtagatcctgccaacggcaagcttaccctcagcggagatcacgtcaccgttgagcagcgcacctttgtggaaaacagggattacctctggccggtaccgcaaacagaaagagatatcaacaaaaacctgacacaaaacccaggctactaatacaactgtaacaatcaaaaaaaatcccgcgagttgaaagatgagcgggatttttttatgcttaaaaagtattcacatgtatcgtttcattaccggcctgctggtttattttatttgtccttttaccttatgcgcccagcaaagcagaaccgttcttaacttcaatacccactgggcctttcaaagaggcgatatcaccggggcggagcaggcaacatttaatgacaagaattgggcgggcatcagcattccgcacgtaatgcgtattgaaaaaaagcacaacggcggcaatgccgtgtaccagggcatcggctggtacaggagatattttaaagtacctccctctttccgcaataaaaggatcactgtttgttttgaaggcgtgcaaaccactgcggatgtgtatctcaatggtaaaaaaatagcgacccatacaggtggttacatgggctttgtagtggacatcagcgcgtatgtggattttgaaaaaaacaatgtgctggcagtgagggtatccaataaagataacccgcagatcccccccggaaagccgcagtcgaagctcgacttcaattactttggcggcatctatagaaatgtgtcactgacggttaccggcaaagtatttatctcccatccactggaagctaacaaggtagccggtggcggcatatttatcacctatccttccgttggcaaaaacgctgcagctgttgcggtaaaaaccaatatcgtgaatgcttccggtaaaccggtacataccacgctgaaaacgacattgattgataccagtggcatgccggtagcaacagcagccattgaacagcccattcctgcacaggcagatacagatatccggcaatcgctgacggtgaccgctcctcatttatggcatccggatcatccttacctgtatcgcctggtatctgttgtttatgaagacaatgcaccagtggatagcctgatcacctatacgggtatacgaaacatcgctttcgctgccgacggtttttatatcaatggaacgaaattatacctgcgcggcgccaacaggcaccaggcgtacgaatacaccggtgatgccgccacagacaacctgcaataccgggatgcccttcaactgaaaaagggcgggttcaatgccgtgcgggccgcccattatcccgcatcgcccgcattcctggatgcatgcgacaaaacaggtttactggtgattgagtgtgagccaggatggcaatttttttccaaagattccctcttcgttgaaaacacttaccacgacatccgggagatgatccgccgcgaccgcaaccacccatctgttttcctgtgggaaacttccctgaatgaatcacccaccagcgaagcatggatggaaaaagccgtacaaaccgcacgggctgaaatgcctggcaaccaactgtttgtagccgatgattttaacgcacgcagcaaagaccattacaacgtttcctacaaagtggtaaatgaagatggcaccgaccctatgccatcacgcccgtttattacccgtgagtggggagatagctggatggccgatgctgaaaaagaaaacagcctgcgcgccagcaggatgtacacagagaaaggattgatcaaccaatgtattttacggcaaaatgcgttgaatggtgaaacatccgaagcgttgggcggctattgggatcatggcggactggatgccaatccaagaattggtggctactttgtatggagctacaatgattacacccgtggctccgatcccatcaccgctttcagcggcgttaccgatcttgaccgctatgaaaagttcagttactaccagctacaggcaatgcaggatgcccgcaatcctgcatatggcccaatggtatacattggcagctataataaccagccagcactggatagttccatcatgatattctctaactgtgatgccgtacaactttaccggaacaacaaattctgcggcgaaataacaaggacgcaaaatgcccgtaccgctccttttgtagcggccaaaggcggtagcccttactttgttttccacaccgggaaatacgagcatggagagttgaaagccatcggtatcctgaatgaaaaagccatctgcacgcatattgtaaaaacacccggcgcgcctcatcacctggaaattgaaattcctgccggcgctgccacttccaccgccgacggcttttctatgacgccgttttatgtgaaggtatgcgaccggaacggcacacttgtatctaatcaaaccgccgggcaatcctatactgttcagatcagtgtatcaggacaaggcaccctcataggcggaaatattccggctgcgggtattgccttgcagaaaacggaaggcggcattgcctatggcgttatccgccacactgctacagcaggaaacatatatatcaacgtaaagagcgccggcatggcttcaggcagtaaggtgattaaaaccaccgcaacaccctatgaatatgtaaaagacggtatccaccggccatggatacacgaagataaaaaaacaatgactgcctattatacggatactattgccgccaaacagctccgggaaattaaactcgccggcaaggccagttttgttcagcctgcggatgaaagtcttaacgcggttattgacggcaacaccgccacaggatggatatccggcgcaggaagtgttcctgtcagcattaccctggatctgaaaaatgaataccagctgagcggcagccgcgtagtatgggggaaagacagcgactggtacacttacagtatcgcggtatctgccaatggcagcgactggataagtgtaaagagcacggaacgggtatccgggcaaaattatcagccggtgcttttccatcgcacagcggtaagatatgtccgttatcttattaccggtatccagccagaaagcagcaggatagcggtaaaagaaatacagctgtacgggacgatgtaaccgctcatccgccttccgctacccgtttgcgtcttgccagctccgcttcgctggggttatcccctacaaacgagcccggtttgatttctcctcccggttcatagctggcaatgatcactcctttcggggagctttttacgtccattaatttccagtccaccggttgggtcccttcccggaataaccgtttgccttcaccgatggttaacgggagggtccatacggtgagtgtgtccaccaaaccattcgccagtaaagtttgtaccagtttgctgctgccgtgcaccagcaggtcgggaccttcctgttgtttgagctgcctgagcccggccactacatcgccggtgatcagcgtggagttttcccagctcagatccattggtttgccggacactgcatacttatggatactattaaacttgtcggcgatactatgatcctgtataaaaggccagtaagccgcaaatatctcatatgttcgtcttcctaacaacagatcaaaagactgagacatgagtgcgttcatgatcccatttgtgaagtcgtcggaataaggcgtcatccagccgccccatctgaagccattactgcggtcctcttcgggggctccgggcgcctgcataacgccgtccatagacataaaagtgatgacgataatctttctcatagtaatctttgttatttgattcaaagatactttcagtaagaatggccggggctgtgtaaatacgactttatgaagggtgaattgcgacaatctgccggaatcatcactatttacaacatcaataaatgtttaagataaagcctcaggtgttgcagcgcgtgggtgatctggttttccacgcttcttttggagatatttaaccgttctgcgatttcctggttgctgagctgttcttccctgcttaacaggaatatttctttactgcgttttggtaaattgctgagggacgcgtgcagttgctggcggaaagactgttcctggattttttcttctgcggtattcccgatagccgccatatgttcttctgcttccactacctggaacgctttccgtgttttcagcacccggtatacatgatagcgggtggcggaaataatatagttacggaaatgaacgatatgcagttcttctcttttaagccataaggtgagaaatatatcatgcacaattgtttcgctcgcttccggatcgtttaacaggttattggcggtttgatacatctttccccaatagcggttaaataacaggttataggctgttttttcaccgtctctgactgcaagccataaatcagcatctgctgtgttagcatcccacctaatcatgtcacaaaaattgacaaaataaaattacctgcatgttaaattaagatgaactatataggaattgatcctggttgattgtctgtgtaacacccgttggcgcttccttccccgacaaaatactcttttttttaaaaagtaggtgtgtaagggaaaataattgtctctatagaataaatgaatcgcctgtgctgacaaaagaagaataccttgatctgtacgaaaggtccctgaacggggattgcagccctgaagagctgatccggctgcagcagtatgaggatgacttttgtttttccgatgacgctgattccgacgaagtattaaaagaaaagatatacaacaggctctctgcaagtatttcgcgggaagagaacgtaaagcggctattcccctggaaagcagtagcagcggcagcagcagtattgctgatggtagcgtcgggcttcctgtattttaacggccgcctgcagcagcggaataagccattggcagtgatagctgaaaaaacacctgtaataaaacgagatattacacctgctaccaataaggctgtgcttattctaagcgatggcacggaggtagagctgaacaaggccacagaagggcaaatagcagcgcaaggcaataccacggtgaataaatccggtaacgggcaactggtttaccagctgaccgataaaccgccaacaacttccctggcggtatttaataccctggccatcccacgtggcgggcaatacaacctgacattgccggatggcagcaaaatatggctgaatgccgccagtaaactgcgcttccctacccagtttacaggaaaggaaagaatggtggagctggagggagaagcctattttgaagtagcgcataaccagcagcaaccctttgtggtgaaagttaaaggcatgcaggtagaagtattgggtactcattttaacgtaatggcatatgcagatgaagccagtataaacactacgttactggaaggaaaagtaaggttacgcaacgaaggaacagcggcggtcatactgaatcccggccaggaaggggtatttaccgggagcaaaggttttaaggtgaacaaagcagatatagaacaggtaatgtcgtggaagaatggctattttatttttaatgatgaagacctgacatccatcatgcgtaaaatttcacgttggtacaacgtggatattgaatatagcagtggcacaaaaaaattatcttttgcgggtagtatctcgcgctttaaaaatgttacagaagtattaaatatgctggcattaacaggaacagtacaatttaaaatagaagcaggaaaaatcactgtcattaattaacctatcgtccacaactatcggccaggtcaataattcgtaaactaaactttatttatgaagcgtaatgctcatgccttgaaaaaggcaggtctactgtcatgggagacactcaggttagtcaagctctccttctctcttgtcattttcctttcgctgcaggtaagcgctgttacctatgcacaaagggtgaatctttctgagaaacaaaccccgttaagggaagtgtttaaagaaataaaaaaacaaaccggttataatttcctgctcaatacggaaatgctggcagacgcccggccggtaacccttaccctggtgaatgctacgctggaagaagcattgaacaagtgcttcgaagggcagcctttcacctacaccattaacaacaacaccattgtggtaaaaagaaaggccatgccggttgtggcggcccaggaaataaccggtactgttaccgatgaaaaaggtgttccggttcccggcgccaggatactgaatcaatccaccaataaaggcgctatcaccaacgataagggggagttcaggatcgcggtgaatcctggtgaaaagctatccataaaaatgctgggatatgaagaaattattattacggcagatagtaaacaagactaccacatccgcctgaagccatctacggtgggcctggatgcggtagtggtggtaggctatggcacacagaaaaaagccaaccttaccggtgcggtgagtatggtgagcagcgacgacttcaaaggccggccggctacctccgctgtttcagcgctgcaaggtcaaatgacgggtgttaccgtgatcaatgccacggctattcccggcggctccgatgaaaatacgatccgtatccgtggtataggcacgctcaatgatgccggcccgctggtggtggtagacggtattcccggcggcaaccttaatatcctgaaccccgacgatatagaaacggtgtctgtgcttaaagatgcagcctcctcttctatttacggggtacgtggcgccaacggcgttattcttgtgaccacaaaaaaaggtaaaagcggcaagccgtctttaacgtatgccaattactttggcgtacaaacgcctactgcgttacctactttcctgggttctgcggattatatgacgctgctaaatgaagccaaggtaaacgccggcaacaatcctacttatacacaggaacagattgacatcgccaaaaacggcagcgacctgaattattacgccaataccaactggctgaaagaaatgtacaagtccggcgcaccacagcaaaatcatatgctgaacctttccggcggcgctaataatattaactactacctgtcttacggcttcctgaaacagggcggccttatcaccggcgataactacaacgccaaaagacataatgtgcgtttaagacttaataccacgttgttcgacattcttcaactggatgccaacattgggtatatcgaccggaaccagaccggttccagtgctgatgtaagcggttcaggcgggcctattcaatctgcccaccagatctctccgctggtaccggtaagatttaccaccggcggatggggatatctcggcggatccgtgaatcccgttgcacttgtaaccgatggcggtaccaatgacttctcctcacaggaaattaccggtaacatccaggcgacgctgaatattacaaaagactttcgtttaaggggacagtatggcctggtgaaaagtaattctttcagacagatctttacaaaaaccattaactactacagtccggaagataattcactgatttaccagaccaataatcccaacaagattgacaaccgcgattatacttctttgtaccagaccgtgatcgggatggcagaatatgaaaagacctttgcaggaaagcattacgtgaaagcgcttgctgcggcttcttctgaagaaacggtgagccgtaatttcacagccagcagaaccaacctgcctacgcaggatctcggcagcatcaacctcggcacactcaatccgcttaacggttcagatggcagccagaatgcattgcaatctatctttggccgcgtgaactacgcttacagcgacaaatacctgctggaaggtaacttccgttacgatgggtctacccggtttgccgcagacctccgctggaactggttcttctccggatctgcaggatgggtgttttcaaaagagtccttcttcaaatcactggaaggcattatcaattttggtaagatcagggcctcctatggtacgcagggtaatgacaaagtgcaggatgatttcggatatctttcttccatcagttctgtcgcgacgatgccaatcggcaatgtgctgacccttggttacaggcaaaccggtattcccaacccgttgctcacctgggagtccatgaccaaacaggatatcggcctggatctcaccttcctgaacaaccggttaagcctcacggcggactactacatcaacaacaccaacgatattttgctgagagtaccgttgccggatgtacttggcatgaatggaagctatccgtaccagaatgccggtaaagtgcgcaataaaggatgggagctgatggtaggctggcaggacaggatcggtgatgtgagctatggtgtgagcggcaacttgtctgatgtaaaaaatgaagtaatgagtttaggtaatgcgccggccactatcgccgaccagatcagaacagtaggtcagccgattgatgccttctatggttttgtggccgaccgtatttcgcagatctccgattactcttatgatgccgctaccaacaaatacacgccgctgttcccttatgatgccagttatcctatgatgcccggcgatatcatctacaaagatttaaacaacgataaaaagatcaccgccgcagacgaccgccaggtgataggcagcgctatccccaggtatacgtatggctttaaaggaaatgttgcttataaaggtgttgatttcagcttctttttacagggagtaggtaaagcagatggatggattaccagtgctgcccgtcatgcttttattaacgatggttccaatccgcaaccgattcacctggaccggtggacgcctcagaatcccggcgccagctacccacggcttgcctatggttactcgtataaccagcgcttatcaactttctggctcgaaaatgcttcctatctccggttaaaaaatatccaggtaggatatacgcttccggcgcacattaccgagaagctgcggatagaccgcttccggctttatttctctgccgacaacctgtttactgcttccgacttcttttatggatatgatccggaaacaccagtgagcagtggtggtttttatccccaggtgaaaacatttgtatttggtttaaacatcaactttaaataattatgaaaaagatattgctatatacctgcgtgttattagcggtaacatctacgggttgccggaaaggattccttgaccggactccgttggatgccatatctgatgaaacgtactggacaacagaagagcagctgacattagcgttgaacgggctttatgccaatgtgaaaaataataacacggtggcgatggaccagatgggagacaacagtattaattcttccaccggagatacctaccgtatttttggcagcggcaacttcggtcctgacctgtcggcggtagatgcagaatggcgcagtcagtacaccggtatccgccagtgtaatgtattccttgccaattatgagcgcgccaccagcgtatcacaggaaataaaaaaccagatggccggcgaagccaaaactatccgggcatacatgtacatgaacctggtatcttacttcggcgatcttccgctggtgaccaaaccgctgaatattgatgaactgtatggtccgcgtaataaacgtaaagagatcatcgactttatattatctgaacttgaagaagctgccggcctgatgaaaaaagagcggcaggttggtcccacactgggacgcttcagcaaaggtaccgcgctggccttcaaagcccgcatggccctgtacgacagccgctgggatgtagcagaaaaagccgccaaagatgtaatggatctcaacgtatattccctttacagcacgggtaagcctgcacaggactattacgacctgttcacctacaaaggtaagctcagcgccggcgtgaataaagaaaccattgccgcccgcctcaatctcacggatgtaagcatgcataacatcagccgtgaatcgcaggtgcctgaccaggcctcccggtacaatcccaccaaagcattggtggatgcgtatctttgcagtgatggcttaaccatcgataaatcgccgctgtacaaggaagatacttatgctaacatttttgagaatcgcgatccgcgcatgaagcaaaccattcttgcaccgggtgctacctggggtggtagaaaagatggcaaccccgccaataccaatcccgctatttttacggcgccgaaatttgtgtctgataaactgggatgcgttaccatcactggttattattataccaaatacgtggaagtaagcaccgtatcgcaggtaagcaaagaccagaacgatatacacgtgatgcgcctggcggaggtgctgttaacctatgcagaggcgaagatggaacagggtacccttacacagggcgatatagatctgaccattaataaactccgcgaccgggtgggcatgaaaaggatgctcctcacagagctggccgccaacgggcaggacctgcgcacggaaatccggagggaacgcaggattgaactggcgcgcgaaggacaacgctggtatgatattatccgctggaaacagggcagcctgctgggtgctgatgtgaagggtatgaagaaatcactggcagcagtgccatcacaggtaagcaacatcgcagcagatgccaacggttatattattgtaatgaccggcaggcagtttgtagatccgaaacactacctcttccctgttccgctgacgcagatacaacgtaaccctgcactcggtccacaaaatcccggttgggaataatgctaaataagataaacatgatgaaaatatctctgaaaatattatctgcgctcctgctatgcgcctgtttctataaagcatcagcaagcgataccctgcgtgtgatgacttacaatattcatcactgcaatcctccgacaaaaagtaaaacaggggaaattgaagtagatgccattgcccatgttatcaacagccggcaccccgacctggtggcgctacaggaagtggatgtaaacacaaaacgttccggcggtattgaccaggctgcacaactggctgccaaaaccggtatgcaggtgtactttgccaaagccattgatcatgatggcggcgaatatggcgtggctattttatctaaacttcctttaaccggtacacaaaccattcacctgccggaaaccgcgaatcctgccagtgaagaccgtgtagtggcattggccggtattactttacgcagcggcaaaaagtttattttcgcctgcacgcatatggatgtgagcaatgcagcggtaagagatgaacaggcaggtgagatcaataaaattgctaccgccaaagccattcctttcctgcttgccggcgatcttaactgcgtaccggaaagtgcatcttaccagctactgctgaaaaaatttaccccttcctgtaccggttgcgggttcaccatcccggtgaacaaccccaacagggtgattgaccacattatgtggacaaacgccccgggctttacggtaaaaagcagcagtgtagtaaatgagccgtatccctcggatcatttaccggtgatagcggagattgttatcaaatagtatattcaggccgcacaagtcgcaggatttgtgcggccctattattcgcggttaacatgcagcatcccgtttaacgtcaccaggtttttaatggcatccccgatagtgttgttaaaataaacatacacctccttcccttctttgatccacgcgcggatctcctttgcccgttgcgccaggtaatcatctgtatacccacccttataatcgccggcgggtccatgaaaccgcaggtatacgaaatcagcccttgcattaagtcgttcattccttgattttggaatatcatgcagcacgatgctgcattcatattcatctgccagctcatacacttccccgatgtaccaggagctgtgcctgaactccagcgctactttccagccatccgggggattaatgccttgtactatatccagcagttgttctacctggccatattgctccaccgttacaccgggtggaaactgtattaacaggcatcctttcttcgctccggcctcattgatcacttccataaaacgaatcacatccgcttcctggaatgccagctgcttcacatgggtgatgtcgcgccataacttgaaggtgaaaacaaaatcatccggtactgagtccgcccacttttttaccgttgcggcctggggtactttgtagaaggagctgttgatttcaatgctgttaaacagggagccatagtaagtgagccggcttttatcccggaaagcgggaggataggccagcttgttaggcacgggtagtacgagtccgcttgtgcccgatttatagatacctttggttttttttgccatgcaaggggtaaagcaaaaatctaaccagtgggatggtaatagccaggaatactttttgtatagaaaccgtaaatccgctccccctaaaaactatccgttatgacatcattcaccgacttcttcaccacttatggccgggcctccttaggcaacgatacaagtatcatcgccagttgttatgcagaaaacttcatggccgccgggccatcggggagcatgacttttaaaaatgatgaaaagttcacccaatggctggaagagatgtttaaatttaaccacaaggtcggcatgcaggaaatgaaagtcattaaagtagaaacgtcgccgatggggaaatactataccagggcgctggtcagatggggcgctgttttctcaaaaaatccggaggaagtcattgaatttgagattacttacattttacaccatcttaatgatgcactcaaaataatcatgtatatcagtcatgaaaacgaggaagatgttttaaaagagaaaggcatcatcagctaggcgccggtacaaatacaaaatcagtatattgtaagaaaaaaaatgcgccgtattatactcagcttcgtacttatcatcatgggtacctctctctacgcccaggcaccggaggaagcagtgaaagctgctattaaccagctgtttactgccatgaataattcagacagtgtagcggtggccgcctgtttcgcgccgggagcgatattgcagtcggtgatggaagacaaagcaggcaagcaaactatccacaccacgccggtcaatgaattttcctcttttataggcagactcccggcccaggcggctgacgagcgtattgtatttggctccgtcctgatagatggccggctggctgctgtatggacaccctaccgcttcttcttcaaaggacagttttcccactgtggggtagactccttccaactagtgaagctcccggatgggtggaaaatccaatatctcatcgacaccaggcgcaaagacaattgtgaagaatcagccatggccaaataatacctgcacccgccctgacccggtattacctcgcgcatgcttcacagatgcgtgaaaccagcgtatccgttgcgtaacccatgcactatgcatacagtccacatgcactcctcatgcactcatgatgcactccccatgcactatcaatgcactatcaatgtactatccctgtcaaaaaccagggtttcggtcagctttcagggtggatatgcccacatggataccgctcccgttttgaatcgatcaaataataacctacttttgccccgctatggttcaggtatgtccactccggatatacctgattaaaagggaactcgggtgaaaatcccggacagtcccgctgctgtaagtctcatacaatgctaaggcatcgccaatcagaccactgttgaacattcaatgggaaggtcgcctgaagcagagataagtcagaatacctgccatacaactacttttttaagctttcgtggaatgaagcttgggaataaattcaatctgcgggtatcccccgtatcttgtctctttcctgattatttttcttattgcgaaagctgttgatggaacattaacaggcttgggaatgatgcgttttaaaacaccggcgaaaaccgccgggatgttgctggtattgctctgtggggcagtgagtgcctttgcacaacaggccgacagtgtaaaatccaaggacctccgggaggtgtccgttacagccccgcgtacggccagggaagtaagccccgggcagaaaatgcaggcgaaagaactggagcggctgggcagccactccgtggcggatgctatccgtttttttgcagggttgcaggtaaaggactatggcggtattggcggtctcaaaaccgttgatatacgcagcatgggcaccaaccaggtgggcgtattttatgatggcattcaactgggcaatgcccagaacggacaggtggaccttggccggttttcgctggataatatggaggaaatcgccctgtacaacgggcagaaaagcaacatctttcagccggcgaaagactttggatcagccggggccatctatcttacttctctcaaacctaaatttgcaccgggagaaaaaacacatctcaggggtaccatcaaaaccggctcctttggcctgttcaatccctctttgctatggcagcagaaaatcagcagcaaagtatccgcctccttcagcaccgaatggatcaatgctaccggcaggtataaattctcctaccagaaacgtgatgaaaacgggcacctggtatatgataccagcgcttaccggaaaaacggcgacatcaatgccgttcgcgtggaaggcggtttcaatggcctgctcaatggcggcgagtggagcaccaaagtgtattattaccaatcgcagcgcggcctgcccgggttcattgtaaacggtgtgttcgggcatgtggaccgtcaatgggatcagaacatctttgtacaatccagcttccgcaaagatattaccaaacgttacagcatcctgctgaacgggaaatatgcctacgactatacgcggttcctggcgccggataccgcccggctttatatagataaccactaccgccaatatgaaatgtatttctcgatggcgcatcagtatgcccttaccaactggtggaccattgcggcttcgggcgactttcaatggaaccgcctggatgcggacctgaccaacttcagctaccctacccgttataccacactggctgccgccgccacaaacatcagcttcaaccgcttcagcgcacaggccagcctgctgggcaccttcgtgaatgaaaccgtaaagaaaaatgcttcggcgccctaccagcagaaatttacaccggcagtatttgtttcctggcagcccatgcgctcaccggatttccggcttcgtggcttttacaaacagatcttccgcatgcctacatttaatgacctctattataccgagatcggcaaccgcttcctggaacccgaattcgccacacaatatgatgcaggattcacctggaataaaacctttgccagcagctggctcactcaggcaggtattgaggcagacgcctattacaatgaagtaaaggataagatcgtagccgttcccggcgccagcatgctcagctggcaaatggagaacctgggatttgtaaaaataaaaggcgtggatgtaaaagcaaaagcgctgtggcttataaaaaaacaggtgcagttcagcacacggctcacgtatacgtaccaacgcgcacaggatttcaccgatccctccgacagtttttacggcgaccagatcgtttatatcccccgccacagcggctcgctgatactgggcgccgactataaacaatgggaagccaactacagcttcatttatacgggagaacggtacaacagcaaagaaaataagttaaagaactacgtggagccctggtataccagcgatatttcactgggcaaacaattcagttataaacataccctgttccatgtaacggcacaggtaaataatctcgccaaccagttctatgaagtggtgatcagctaccccatgccggggagaaattaccgcttcattttaaccgtgaatatttaatcgtcatgatgaaacagctaagaaatatagtattggtggccgccctggcaggactggccatcaccggttgccggaaaggagagaaaattgttccgccggaagtaacacccgtggataccgccacaccaggatccctgctcaatggattttacctgctgaatgaaggcaatatgggcagtaataaagcctccctggattattacgactataccacaggcatctacaaaagtaatatctatgctactgccaatcccactgctgtaaaggaactgggtgatgtaggcaacgacattgaagtatatggtacgaagttgtatgccgtgatcaacatttccaacaaggtggaagtgatgaatgcagccagcaccaaacgtatcaagcaaattgatatcctcaactgccgctatataacttttgccaacggcaaggcatacgtaagctcctatgcaggccccgtactgatagaacccaatgcacccattggctttgtagcagagatagacaccactaccctggaaattacacgcaaagtgattgtaggttatcaaccggaagaaatggctgttgtgggcaacaaactttatgtagccaattccggcggctaccgcgcaccaaattatgaccgcactgtgtcggtaatagatttgaatacttttaaagagataaaaaagattgatgtggcgattaacctcgaccgcctcaaggcagacaatgatggcgatgtctacgtgacttcccgcggcgattattataatataccctcccgcctttttgtgatagataccaaaacggatgctgtaaaaaaacaatttgatatcccggtgagcaacctgtgtatttccggcgacaccgcttatgtgtatggttctgtcttcagctataacaccggcaaatggacgatcacctataacatggtaaatgtaaaaacggagacggtgttaaacagcaattttatcactgatggcaccgataaatccatccgtatgccttacggcgttgcggtaaacccggccaccaaagaaatctttgtgacggatgcaaaggactacgtttcttccggaaccctttactgctttgataaaacgggtaaaaagaaatggtcggttactaccggtgaaatacccgcgcacattgcatttgtttccgcaactaaataatcataaccaactaaatgtatacaaatgaaaagtaaacttctacttgctgccacattcatcgctgttatggtaagcagctgttcaaaggataaagacgtaaccccgcccattgaggaccctgagcctaccggtcctttcctgaataaggtgaccaaagtttttgagtacttccccgcacccggacagttcaccaatgaacttcccatgtggaagcagggcgattcagcaaaacaaatggcggattacgcactggcggctttaggaaaagaagatatgatttccctcggcggattcggcggatatgtagtaatgggctttgatcataccatcaaaaatgtacccggcgaatactccttcgtagtattgggcaatgctttcaaccagtttgcagaacccggcgtgatctccgtatccgtggatgccaataaaaatggcctccccgatgatgaatggtatgaaattgccggctcagaatacaacagttccaaaaccgtaaagaactaccaggtcacatactacaagcccaacgaaacaaaagaaagggtgaccaatccggatgatccctataccagcgacacggagtatatccgctggaaagacaaccagggcaacaccggttaccttgctaaaaatgtatttcatgatcagtcgtattacccgcagtggaaaggcgacagcatcactttcaccggtactaagttaacagacatcaacattaaaaatacttccagcgatcctttctctcccttctatgtttcacctgctttctcgtggggttatgcagataaccatgcgaatgaagataccgatgcgaaaataaaactggattgggcagtagataaaaccggcaagccggtgaagctgacagggatcaactttattaaagtgcatacggctatccgtgcagaagctggatggttaggggaaatttctacagaagtgctgggcgtaaaagatctgaacctcgaataatatccatgaataatctaaaagaagggggcgtttgtaaacaaacgcccctctttctttttcgactatttcacgcttaccgggtgcttatcgtcgccaatggccaccaggctaaaagtgccggtgatggctttttcccgcgaataggaatacatttcttcaatgtatatttccaccaatactttaacactggtatttcctacttcggttattttcccgatcagttccacgatagtgcctgccggaatgggccggttaaaatctattttcccggaagataccgttaccatttttttacgcgcaaaacgcgtagcggtaataaacgctacttcatccatcagcgacatggccgtgccgccgaacaaggtatcatagtggttggtagtgctgggaaatacggctttaaagatccgggtttccgaatgaagaattttttcttctatagtcatgattgtactgtttttcttttttacaaagatgctttttcccgcatcacttccgctgcgcggaccatattcgacaatgccacttttgtttccggccatttacgggttttcaacccacaatccgggtttacccacaggttcctggcagggagtgtgatggcggctttctccagcagcgaaatcatttcttccgcagatggctggcggggagaatggatatcgtatacgccggggcctatctcgttgggatatttaaaatccgcaaatgcatccagtaactccatctgcgaacgcgaggtttcgatggtgattacatctgcatccatcgccgcaatatgctcaatgatatcattgaattcactgtagcacatgtgtgtatggatctgcgtttcatcctttacgccgctggcggaaatgcggaacgcctgtaccgcccattccaggtaagctgcgcggttttctttacgcaaaggtaagccttcccggatagcaggttcgtctatctggatcaccttaatgcctgcctgctccaatgccactacttcatcgcggatagcccacgcgatctggttggccgtggtggaacggggctggtcgtcccgtacaaaggaccattgcaaaatggtaaccggaccggtgagcatgcctttcatcagtttatcggtatgtgcctgcgcaaaactgctccaacgcacggtcatgtttgccggacggcttacatctccaaaaataaccggtggttttacacaacggctgccatagctctgtacccagccattttttgtaaacaggaatccctgcagttgctcaccaaaatattctaccatatcattccgttcaaactcaccatgtaccagtacatccaggccaatctcctcctgccagcggatcacctctatggtcgctttttcaatggcggcttcatattgtccggtggtcagctctccttttttcaggcgcgcccttaactgacggatatcatctgtttgcgggaaagagccgatcgtagttgtaggaaacagtggcagtccaaactgctgttgctggatgttttgacgcaccgggaacgtactgttcctgcgtgcatctgcggcggtaaatgccgctatcctctctttcacttctttcctatgaatcagcggcgaggtggccctgttatggatagctgctttattggcttccagcagcgccgtattgccgttcacaatatcacgcagctcattcagttcctgcaatttctgtttggcaaaggccatccagtttttaatttcgggagacagggctgtttcgttatccaggtcgcacggcacatgcagcaatgagcaggaaggagcaatggcgatacggtcttttcctaacacgtttactgccttttgtatctgctgtaaagatttttcataatcatttttccagatattcctgccatccactacacccagcgagaggtgcaaagaagtatgggcaatagctgtatcgaggatatcttccaattgcaacgggcaacgcacgagatcgaggtgcaatgtttgcaccggcaatgccaaagccaccggcagattctttccatagcattcaaaataagaagccaggagaatatgcagttgggggaaggctgcatgaattttcgtgtaggtattcgtaaacacctgcagggctgcttcatccaggtcgagcgacaggcagggctcatcgagctgcacaacttctgcaccggcttgtgtgagctgcgatagcacctccaggtataccggcagcagtttatctatcagcgataaacggttgaagccggccgttttctcttttccgagtaacaggaaagataccgggccaaggatcacgggcttagcagcatagttttctttctttgcttcgagaaactgcgctgttactttgcgggagaagaaatgaaatgtttggtctgccgtaaattccggaacgatataatgataattggtatcaaaccactttgtcatttccatggcggtgatatcgtcgccatcgcgctggtagccgcgcgccatggcgaagagcaggtctgtttcaggaagtttcttctcctgcaaggtgcggtagcgttgtggcacagcgcccaccatcagggaagtgtcgagcacctggtcgtaaaaggaaaaatcattgcagggaatccagtcgatccctttctgttgctgcagctcccagttgtgtaaacggatattacgggcggttgcctgtaattcatcaagagtaattttgcctgcccagtagctttcgcaggctttcttcaattcacgctggctacctatcctcggatagcctaagttgtggataatcattgctgattgtttaaaaggtgatacatgacgttcacgctcttttatatagtacagcaatgtttttgagaaaataatacggaaggagaaggtatggcagatacaagaacaagcatatagtatacatgattccatcatgcatacgcctgttctgataattaccgataccgaaacctgacacgcttcaatccccgaaagcattgtcaaagtgaaataaaggcaggtctcctggcttgttccgctggtaaacaccttcccattcctggccggaacagtggcatattatttaccagttgcagtgcatgtgcgctgccggaagcttacagttgcgggacagcctgtgatttgcacacagttcccttttaatcccgcttttcagcgggaaccattatttgcttcgattagtaatacataaagaaccggcgcgaagatagtaaatccccgcaactatcaaatccgtttcgttttcttacaatttcgggccgggcgaaaagcggagttttacatcataaaaacaaacagctatgaaacaggcaaatatactgatcaccggcgccaccggacacattggtactacattggctaaacagttatcggcacaaggcattcccttccgcgccatggtgcgcacaacagacaataacgtaaatgcccttgccgccttacccggcgctgaaatagtaaccggcgatttcaacgatgccaacagcttagtccttgcacttaaaggaatagagcgggctttcctgcttaccaactcttctgaagcagcggaaaaactgcaaagcaattttgtaacggccgccgttaaaagcggattaccgcatatcgtaaagctctcgcaactccatgcggacgcacaatcgcccgtacgttttttacggtatcatgccgctgtagaagaaaagatccgtgcatccggtatggcatatactttcctgcggcccaatttatttatgcaggggttactgggtttccgtgaaacaattgccagccagaacaaattctttgctaccgccggcgacgctcccatcagcgtagtggacacccgcgacattgccgccatagctgcggctgccctcaccggcaatgggcatgaaggcaacacctacgatatcaccggcccgcaatcactcacccatgccgcactcgcagaaacgctatccaatgcactggggcgcactatccgctacatcaacgttaccgcagcggagttactgcccgcccttctccacgccggattccccgcctggcaggcagagggcctcatcgaagactatgcccactacgcacgcggcgaagcggcggccgtttcctccgctgtaatggacataaccggcaggccggcgcgcgacttcgccgccttcgccggcgagtatgcaccggcgttcacctgagcggattttgtctttctcaggattacgctgattatactgattaattggattttgttctttgggatttttaaaggatttggggagatagaagcggattttgtctttctcaggattacgctgattatactgattaattggattttgtcctttgggatttttaaggattgggggagatagaagcggagacttttgtttttatctccttaattattattaatctaaaaatccaaaaaaatccaaaagcaaaatcagtataatcagcgtaatcagcgagaaagacaaaatccgcttctatctccccaaatcctttaaaaatcccaaagaacaaaatccaattaatcagtataatcagcgtaatcctgagaaagacaaaatccgctgcaaaattttacgcggatttcccgccaattgcttactttagttatcaaatcgagcaaccagtgagcaatgaagaagcggttttgctgcaacggctacagcaaggggatactgaagcgtatatcaccttatatgatcagtattacccctcactttacacttatattctccacttcatcaatatcccggaactggccgaagatgcactgcaggaagtgtttataaagatctgggagattagggagcggatcaaccctgaattgtcattcagtggttatctgtaccgtattacccggaatcatgtatttaagttaattaagaagatcagcgccgacgcagcgctccgtttacaggtaatgcaggaactgcagcatcagacggaagatgcggatacccggttattgtggaaacaatacgaatctttactacataaagccattgcgcaattgccccctcagcggcaaaaagtgttcaggttatgccgggaagaaagcaaaagctacgaagaagtagccgtagaactgggcatctcccgcaacaccgtaaaagaacatatggtgctggccatgaaaagcattaaatttttcttctatactaataccgacggtattcttcccctgttactggtttccggggttctcctcaactcctccaaataattttttttctcccggaccaccctacctgctttttttgggatagtatatatatgcccacggaaaggaacaatgaatattaccaattattgctgcaacgctggcaacaacggacttgtagtccgcaggaagcccttgaactgatggattacctgcgggacaaggattccgacaggacgctcctgaacgaaatgcaggccgcattccggcaggtgaagccggataacggctcccactccggcgaacccggcgaaagggtccggaaagggctgttacagcatatccagggcgccccggtaatatccatgtcccgctcccggaggaattatggtccgtttaaactcgccgccgcggcagccgtgataatcgggctcgctcttccggccatttattttttcaggcagccagtggttagcccgatggccactacagcgaaaaaggcgccggcagatgtggcgcccggtcagcataaagcggtactcaccctggccaacggggaaaagatagtgctggacagcgccggtatccaacaactggcacaacagggcaatagcgccatccgcaaccagggcggacaactggtatatgtaaaaacaaagggagccagcagcgctcctatctataatacacttaccacggcggcaggtgaaacctatccgctggtattggccgatggcagcaggatttggctgaatgcagcctcctcgatccgcttcccggctactttttcaggcgatgaacgccggattgagcttaccggcgaagcttactttgaaattgcacatgatgcgcaccggcccttccgtatccaggtaaaccagatgaccgtggatgtactgggcacaaatttcaatatcaattcctacgccgacgaagccacgatcaacactaccctcctggagggggcagtaaaaataaacagtaaaaagggcagcatacaactggcgccgggcgaacaatcgcaggtaagtcctaatgggaatgtaaaaagagtaaccggcgtaaataccgctgaaataatagcctggaaagagggatacttccagttcgagagcacagatctgaccactgtattacggcaattctcccactggtatgacgtggagattgtatacgaaggcaatatcaaacccaggaaattttttgggatgatcagccgtcgcagcagcctggtgaatgtgctgaaaatgttgaatgccaatgatgtgaattatcggttagaaggaaaaaaactgattgtacagggcgattaacgcccgcaggtgaacaattatatcaaccagcatgacggagatgtcatggtaacaaggatttattaaagcagatagcacaaccaaaccattctctcaatcaaaactcagcacaagtatgcaattacgtactattgccagttcccggtgtaaaaacaaccggcgtccaaccaaacatctaaaggtcagtcagttcctggccctgctatgtttcgccaccacggcacaggtgagcgcagccagaagccagaaccaggtagtaagtttatcactgaaaaacgctaccgccaaagaggttttccgggaaatcaataaacaaaccggcctcaatatcctggccgatgaagccttgctggaaaaaagcggcagggccaatatcacggtgaacaatatgcctgtaagtgatgcactgaatattttcatgcgtaatcagccgctcacctacagcatcgaaggaggtgctatcattgtaaaaacaaaaccggtgatacagccggccactacgcctccgccacctattgaagtacatggcgtggtaaccaccgataaaggacagcctttacccggtgccaccgttaccgtaaaaggtaccaaactgggaactgttaccaacaccgacggcagctttaagatcaatgccaacccaggagaaacactggaaatttctatggtgggttttaaaacctggtctgtgaagtttgatggcaaaaacaccagctttaaagtaacgctttctgaagaagtatctaacctcaccgacgtagtggtagtgggttatggtaccaccaaaaagaaagacctcaccggttctatcagctccatatccagcgaccagatgaacctcggcggtgtaaccagcaacgctgcgcaggccatccagggccgggccgcaggggtgcaggtgagccagtcgaacgcggcgccaggcggacaaaccattgtgcgtatccgcggcggcaattccatcaaatccaccaacgaaccattgtacgtggtagatggcttcccttctgaaaccgggaaagacatcaacccgaatgatatcgatgatatacagatcctcaaggatgcctcttccaccgctatttatggtgcccgcggcgccaacggcgtggtaatgatcaccaccaaaagaggtaaaagcggcagggcatctattcaatatgatggctactacggtacgcaaaggatcattaaggaatacgataaaatgaatggcctggaaaatatgcaggtcaccaatgcaaaagctattgaaaaagggcaacctgccttttataccgctgccgacctggccagtggccgggacaacgactggtttaaattaaccacacgccccggaatggtgcaaagccataacctgagcgtaagcggcggtaccgcggaagacagggttgccttatccggcagttacttcaaacaggatggtgcattaaaaaatacttcttttgaaaggtattcggtaagactcaactacgataagcagttcgcagcacgatttaaaacaggagccagcgtatacgcctcgcatgcttataccaattttaaaacctacgatggaaacattgtaccctccaacgtgatgtatggcgtactcaccgcttctccggctattcccgtatacaatgaagatggcacttatgcccgcttcaaaggaagggacaacccgctggcgtggttaatggcgcctaccaacgaccggtttgaaaacaaggtaaatattaacgtctatgctgattaccagatcctggacggacttaatttccgtgtgaacggcggtagcgagtatatgactaccaaggaaggcacctatcttccacgcgacctggtagacggtgaaaaagtacagggtaaagccagcttaaatgacatcgctgttacgcgaaacctggtggaggcctacttcacttacaggaaagtgtttaatgccatccactccttcaacgttgtagcaggggtatcttatcagtctgacaaaaccgaaaaacattattcgctggtgcagaaattcagtacagatgcatttctgtacaagaacctggaagcaggtacagagcggttatccagtaccagcaacctgattccatccaagatggcttctgcctatggaaggatcaactattccctgaaagataaatatctcgctaccttcacagtgcgccgggatggatcttcccggtttggtggcaacacccgttttggtatcttcccttccggttccctcgcctggagagcaggtgaagaagaattcattaaagacctgaacatcttttccaacctgaaagtaagaggtggttatggcgttaccggtaacgacaggatcggtgattatatttacatgcccacattcgggcctaccaacgtgtcgctcggacaaggcagcgacagttatggaggaattgttgccacccgtttagcgaatgcagacctgcaatgggaaagcacagctcagctggatcttggaatagacatgggctttttcaacaaccgcgtttctgctactattgattactatcgcaaaaaaaccaacaggctgatcttcgatatgcctataggcgactggaatggttttgcggtgcaaaccgtgaatgccggcagtattgaaaataagggcgttgaattatccgttactacagagaatattatcaatcatgcattcacctggaatactaccgtgaacattgcctacaacaaacaaaactgcctggacctgggcggccgtccttatatcattacacaaacagctaacctgtatggcggtcgtggtatggacttcaccaaactggaaccaggaagggaactgagtactttttatggttatgtttatgatggcgtgataaaaaccggtgaagcacatcccgcacaaccgaattcaaaagcaggtgatcctaaattcaaggatatcagtggtcccggcggaaaaccggacggtgttattgatgccaacgaccgcacgtatcttggtcatgcgaacccgcactatatctatggcatcaataacaactttgcctataaaggttttgaactgaacattttcctgcagggcgcactggattacagcctgtataacggaaccggtcttgtactggaatccgggccgggtaaagcggcactgaacaggtggactaccaacaacgaaaacaccgatattccgagagatggatacgcgattgcttacggcggtatgatgaactcccgctttgtggaaaacgcctcttacctgcgctgtaaaatgctgatgctcggttataatatcccggtggccaaaacttttctgaaaagcctgagaggcattaaagtatatggctccgtacaaaacttattcaccattactaaatatacaggatcggaccctgaggtaaacagcaatctcaatagcagcggcagcaacgccaacctttcatcaggattggattatacagctttccctgcgtaccgcacctttaccgcgggtcttaaattgaatttttaacctgtaaattccggaacaaatgaaatacgcatatatcgcattagccaccttgctgctcggcgccagttcgtgcaaaaaagaggtggaacctaaagtatacagttatctcactgatatgaatgccttcctctccctgagtgatgccaaagctgcagtgaacggcgtttattcaaggctcaaacaacccagcggcagatcggatgcatggatgtattatgcaggcttccaggttaccatttcagatctgaccactgatgtagggcacgccagctccggcggagacgtaggactgatgtctgattgccagtgggcccctgtcaatacctatcttgcctttgcctggcagcatcaatacaagctggtagcagatgccaacatctctttatactatattcctaaaatgaccagcatcacagatgcacagaaagaccagttcaccgcggaactccgtttcctgcgcgcattgggatatgtagatctgacagatgctttcgggccggtgccagtggtcacagaagaaaccgtagccaaaaatattgaagcaccggattatgaggcagcactgccaaccacaccggtagcagagatcaatcaattgatcatcagcgacctggaatttgcggccacccatcttcctgtcaactatttaagcaaccctatctacagctccaacgatataggccgtgctactaagggcgccgccatgtctttactctgcaaactgtacatgcgtgaacatgaatggcagaaggcactggacctcactaccgaaatcatgaagctgggttacggactgtatccaacctatgcaggactatttgcagagaaaaacaagtggtgccaggaaagtattttcagcgccctcgccgatccattggtagatgccgtggaaatcatgaaccacttcggccctatcaacaatccgcaggtaacagaccggtggcagtatttcgctttaacctggtacttctggaatacatttgcggctaacgacgaccgtaaaaagatgttctattccgattatatcggcaccgatggcttacattacatgcaggcgcctccgggacaaaccaatccaccggatggttactactacatgccagacgtagccactaccaaatttgccgatcctaacggctctaccacttattacgatggtcacgtattcccgatactccgctatgcagacatcctgctgtgcagggcagaggcgctgaacgaactgaatggtccaaacagtgaatccatcacgttgatcaaccaggtaaaagaccgctcccatgctaccaacctgggcgctgccggtaccttcaccaaagaaaccctgcgtaatgctatcctgcaggaacgcggatgggaattcttctttgaatgtaaacgcaggcaggatctgatccgtatgggtaaatacgaaagcgtggtaaacacctacctgaccgcggtaggaaaaacaccgaccattaacctggcaagagataaatatttctcttatccacaggcgcaaacagatcttaacaaaaatctcagcaacagtggccgccgtcaataacggcttgctatctttctgaattattcaatattgcaaatgattaaattgaataaaatacaacgcctgctgccattgttatcaatggcagcagcgttgttgttgtttgcacccggttgtatgaatagtggcggcaacgatattgtttccattacgctcaacccgcagggacaaaatgccatcaaggtaaaaacagatatcctgtgtaccgacacagtagacgcagcagtagaatactggccaaaaggacaggaacaacaacgcactaccacgccattgtccgcgcaccggatcagtcatactattgtgctcaccaacctgctgccggaaaaagcctacgagtaccgtatcttaaccggtcatggcaaagatctttatcccagcaaaacttatactttcaacacttccggtttcccggtatggatgaaagatatgttcagcgtggtatgcccggacagctccgtattaccagccaccttcaggaaaggctatgtaatgcttacccgccgggaagatcccggtgttcttttcctccttaatgcaaaaggaaatgttacctggtaccaccaggtaagcggcaccggttttaaagtagccaggtttacagacaacaacaccttcctcaccctgctgggcggtcctggatacgaaaccagctacggcgaccagatcctggaactttctgtttccggcgatacgctggccaatctcaaaaaaggacaacaggatttcaaacaaaccattcaccatgaaatactgttgaaccccaataatgagtttgtaacgctttgcgtggaagaaaggatctgtgacctgagcagtaaaggcggcggcaaacaggataccgtaaaaggcgacggcatcctggtgctggaccggcaaggcaaacaggtgtggaaatggaccgtgtttgatgcactgaatccactggacgataaaaacatcttaaaagaaaaacaagactggatgcacgccaactgcatcgcatttgataaagatggtaactacctcatctctttttataataacgggcagatatggaagatagatgcccgcactggtaagcgtctctggacatttggaaaaaacggcgactttgacctgccagccacggccctgtttgaccaggcgcatggactgcatatcaacgagcatggtgagctgatgttcttcgacaatggagtgagcaaaaaaacatcaagaacgctttcctttaaactggatgaaaacggaaaaaaggcgcagcttcgtatcaatacccaactgccacgggaaaattataacgagagaatgggaagcagctatttagtaggcgacactaccctgctgcaatgcgctacgaaaagaaataccgttatactaaccaacttcgacggaagatttctctggctgctgagaacaggcatgtcgtcttaccgggcctcttttatcccggcggaaagactggcgccttatattgttcagccaggctattaacaatcattgtgcactacaaaaaaaatatcatgagaagcttaattgtgattggcgtgatcggttgctgggggataatagccatcatatcttcctgtggatcacaggtaacaggagaaacaaaagcaaccgcagctaccctacctgaaaaagaaacatacatcaatatcgacaccaccctgataccaaatgaccaattcggcgagtccgtgaaatacggccgggagctgatgctcaatacggcccgctacattgggcctgatggcagtgccggcaagtatcttggtaataaaatgaattgtaccaattgtcaccaggatgcgggcaccaaagctttttccttcaacctgatgtcatcgcacgataactacccgcaataccggggccgggagggcaaagtacttacgctggcggaaagggtgaacaactgcgtcatgcgtccgcacaacggcaaaccactgccgctggacagcaaagagatggtggcatttctttcttattttaaatggatcagcacttttgtcccaaaaaacaaacctttcaaaggcgctaaaaatctgcatgtcacctttctggatatcgccgccaatcctgaaaacggacaggtactttatcaaaccaactgcgcgcgctgtcatggtcaaaacggggaaggacaatggactgcagacaaaagcacttacgtatatccgccgctgtggggcaacaccgcctatcaacccggctccagtatgcatcgtgtaatcaaacaggcagaatggctgaaaaacaatatgccttacgataaggtaacacccggcaagccattcctctccgacaaagaagcaatggacatcgccgcatttgtaaacaacgacaagatccatagcaggcccaatcccaaaagctttgactacccgcatattgcggaaaaagcaattgactacgatcacggtccctttgcggacaccttctccgtagcacaacacaaattcggcccctaccaaccgattatcgactactggaaggcgaaggggttgaagccgatttactaatgccgcggattttgtcttggctcaggattacgctgattatactgattttggggattgaccttttggatttttttatgattttgggagatataagcggatgtaatagtttgtatagattttttttatgattcggggagacataggcgaatatatccgcttatgtctccccaaatcattttataaaaacccgcttatatctcccaaaatcataaaaaaatccaaaaggtcaatccccaaaatcagtataatcagcgtaatcctgagccaagacaaaattcgcgtataatattaccttacttttgccttgaaaaaaggaaggaatggcagttataatgaacgaaaaggggtatagccgtaaacaggaaatcgtgaacgggctgatacatggagtgggcgttatttttggggtaagtgcattgcccatgctggcaggtattgccgccacgcataataatacgccgggcattgtaggcgcctgtatttacaccttctgttttatattgttgtttacgaactccactatttatcatttatcgcaggagctggccgtaaaaaagctgttcctgatatttgaccatatcagtatttactttttaatagctggtacctatacgcctttcctgctggtgtatatgaataatgcctttgggatcacgctattgtcgattttatggggacttacgctggtaggcgtcttatttaaaacctggtttacgggaaaatacgatattgtgtccactatcatttacctgttgatgggctggatcatggtatttggcggccgccggtttttcgataacctccccctgccggtgatcattatgctggccattggcggcggtttatacacgataggagttattttctatatctgggataaatatacttatacacatgccgtgtggcacttgctggtgctggcggcggctatttgtcattatgtggcggtattgatggccatgtaaagccacggaagtcatcagccgctcaatcccggttgataatttcgctctgcccacatttttttccggtagtcggtggggttaataccggtgtatttcttgaacgtcctgtttagatggctttcgtctgtaaagcccagttcatccacaatttcgctcatccgcatatcgctgtattgcaggcgggtttctaccagcttcagcttataattggttacgtaccgctggatgctttctcccgttaacttcttcacatattcactgatataatttggagagatattaaaccgtgccgccagtttttctgtacgcaggttttccgggtagtaaatattctggtggatataaccgataatatcgttggaagcttcgctgcttatcgctgctatttccggtgtaagcaacgatacattacgtgccacgatggtgataatggtatttaccagctgctgcaccacttcgttgcgcagggattgctcgcgtgggtattccagcatcagtgcgttaacaagcgcccgtacaattggtttatcttccgtattatgtaaaatacagccggggaaatggtaattattatggaagataaattccagtttctttgcccagtcgcccaggttactatgggtattgcccgtacgctgcgcttccaggtagataccgttaaaacggatgaacaggaagccggtccggctttttatgcgggtatactgtacatcctgcggcataagcaggaacaggttctcctcctcatagggaaaagcatgctggttgttgtggaaggtgccggtacccttcaggatatataccagttcaaagaaattattgcgatgctggcccatcgggcatacatcttcctcaatgtatatgatgtcaaacggcttaaaaagattaattacttccataacctatgattgtacaaaatgtaccctgattcgtacaagggtatacctgcaaatttattggaattttgattcatcaaatcacaaaaaaaacaaaataaggatatgaaagcaatcgtattaaagcaggtaggcggtacagaaaacctggaaatcagggatattcctgttcccgttattaacgataatgaagtactggtgcgcaaccatgcagcaggcgtcaacccggtagatgtttttgtaagagctaacgagggcgcgctgaaaggatacctgcaaccgcaggaaggcgaggatattatcattgggtgggatattgcgggagaagtgaccgcagtaggcaaaaatgtgaagcagtttaaaccaggtgatgctgtatttggcatggtgaattttaccggtcatggtaaagcctatgcggaatacgtggccgccccggaaagccacctggcgctgaaaccggccaacacctcctacgaagctgctgctgccgcttccctggccgccctcactgcatggcaggcgctggtaacttatggcaaaataaaaaagggcgataaagtactgatccatgcagccgcaggcggtgtgggacactacgcggtgcaaattgccaaacattttggggcttatgtgatcggtacgtcttccgccgcaaaaaaagaggccatgctccgttttggtgcagatgagcacatcgattataacagccggcaatttgaggaagtagtaaccgatgctgatatcgtactggattccctcggcaccccaggtcacctcgaccgctccctggcagctgtaaaagatggtggccgcctgatcagcatactcgcatttttcagtgatgagcaaaaacaaaaagcagcggctaaaaacgtgtatatacaccgcgtgtccgtagtttccagcggtgatgatatcaaatccattgcagccttgctggaacagggcgccgtgcactctgaaatagcacatgtgtatgcttttgaggaaatagccaaagcgcatgagcaggtggcaacggggaagacattgggaaaagtggtggtgaaggtatagtcttcgatttgactacaacaatagcagatccggctacagctgtttctttgatgctacggaacttcgtagcatcaaaaaaacagcaaaatgaaaatcattgttacaggttctctagggaatatcagtcaaccgctggcaacggagttagtacaaaaaggccataccgtggtggtaatcagcagcagcccggaaagacagaaagacattgaagcactcggtgctgccgccgccatcggcacattggaagacgtggatttcctgtccgccacatttaccggtgcagacgcggtgtattgtatgatacctcccggtctctctgaacccgaccggttaacatattacagccggattgccggcaactacgcaaaggcgattcaacgatcgggggtaaagcgggtcatcttactcagcagttatggcgctcacctggataagggcaccggcattattcttggcgcccataaggcagaggtgacgctgaacggattgcctggtatcgctgttacgcatatgcggcctacctatttctactacaatttatttagctttatagcaatgataaaaagcgcgggcgtgatgacggccagttatggcggtgacgatatgattcaattggtatcgccaatggatattgctgctgccattgccgatgaattggaaacacccgctgctgccggccataaagtgcgctatgtggcaagtgacgaacgaactgccagcgaaattgccggcgttctgggggctgccatcgggaagccggatttgaagtggacggttatcaccaatgaacaaatgcgaagcagcatggaatcacatggcgtacccgcagtgctggcaacagggctcctggaaatgtatgcgggcattcataacggtgcattagcagaggattactatctgcataaacctgcggtgatgggaaaagtaaaactggaagattttgcaaaagaatttgtggctgctttcaaaaaataacaatggcgaacatgcaacctcgtaagataaaaacgatcagcgaatttcaccagctccggaatttgcccaggcctcagcatccgctaatcagcgtgatcaattttgaaacgattaaacgcataccggacgatgagcccaaaagccaggtacaggatttctattctattgcgctgaaaagggccgtgaatacgaggatgaaatacggccagcaggaatacgacttcgacgggggaatacttttctttgttgctcccggacaagtgtattccattgaaacgcagaaagattttcaacattcgggatggattatactcatccatcccgattttctctggaatacgccgctggcgaaaaagataaagcaatatgaatacttcgactattcagtgaatgaggccctgcacatgtcagaaaaagaagaagtaacgattaccggcattgtgcagaatatggaacaggaatatcataacagcattgacaaattcagccaggatgtaatgatagcgcaactcgagctattgctaacctatgctgaaagattctatcatcgccagtttataaccaggaaaataaccaaccacacgatcctcgatcgtatggaaaacatcctcaccgagtggtttaacagcgattccctggcatcaaaaggcttgcccaccgttcaacacattgccggcgcacttaatatatcgcctggctatttaagtgcgttgcttaaaatactgacagggcaaagcactcaacaacacatccaggacaaattaatggagaaggccaaagagaaactatctaccaccggcttatcggtcagtgaaattgcatacgagctgggctttgaacacccgcagtcgttcagcaagctgtttaaaaataagatgaaagtgacgccattggagtacaggcagtcgtttaactgaaaataacaagcaaacagcaaatattaccagaacctcacataaataaccgacagcaacaataatatcgttacaattaaaatcacggaagaaggcttcagcttaaacatctcataatccagttcaaaagctttggcactcacctttggtcccgccaggctgatagccaccattaccagcaccgtggtaaggaaagaccatcccaggctgataaagaaaggtatttcgtattcgcccttggcattgtggaaagcggaatataataccgtttcaggaccaaagatttttacggctacctggttaaagaacagggaggccgcaaaaccggtgataatacccgctatggcagctgcgccgctggttcttttccagaacatgccgaggataaaagtagcaaatacacctgggctgataaagctggaatacttttgtacaaaagtataaccgccggcgccgccgatatccagcacatcgttccaggtgaataatacgcctatcacgatagcagctacaatagtgagccggccggtccataccagctgtttttcatctgctttcgtattgatatatttcttgtaaacatctaaagtaaaaatggtggaaatactgttggatttacccgccagcgaagctacgatagcagcggtaagcgcggcaatagcgagacctttcaacccggccggcagcagggttaaaatggcagcataggcgccatctttttgtcctccttccagctgaggcaggtgcccgtgctggtacaacacatacgctacaatacccggcagcatcacaattaccggcatcagtattttaagcagtccggcaaataaaataccggtgcgggctgtttgcagatctgcgcccagcgcccgttgggtgatgtactggttacaaccccagtagttaaggttactgatccactgtccggcaatgtacataccaaagcccggcaggatcaggtatttgtttacgtaatcctgtggcgcgccaacagcgggcttcttcagcatcatatggaaatgatcgggcgcctcctgtaccaggatattaaagccggccagcacatcttttcccatgccgaatttttcactcaccacggttaatgccatccaggtagtggccagtccgccgataatcagcacccctacctgtattacatccgtgtagccaattactttcataccaccaagggtaatcaccacggagaagatagccaaagccaccatcacttcatgaaaataggcgccccctagtagtccgttgatagcgagagcgcccagatacaaaatagaagtgaggttaacaaatacatataaaaacaaccagaatacagacataatcaacgctaccgtttcattgtagcgcgttttcagaaactgtggcatggtgtagatcttattcttgatatacaccggcatcaggaataccgccacaatgatcagcgcagccgcgcccacccattcatacacggatactgcaatgcccacaaaaaagccatccccgctcatcccgataaactgttccgctgaaatattggaggcgataatagaggccccgatggcccaccaggtgagagatccttctgcaaggaaaaaattcttggaagcgcttacagctcctttcttctttcttttataaatccaatatccgtaggtagcaacaatcacaaaatacaacgcaaataccaggtagtctttgaagacaagttgattactcataagtggagcggttgatcagcagttttttaacgtgggtggaaatacctggatataatttaacactttccggcatgcaaaaaaaaggattaccggcgacacatcagaaagttgcatctgcaccggtaatccataatatcactgttcaaaactttaaggtggatggtaagtacttggctaccagatcttcgtaatatggtcttaatactttccaatctggtggagttggactcttggagtacaggtcgtatggattaaacagatccacccatttaaacatttccacatcatgggcattcatcaggtgaccgtaagcatgttccctgtgctgcggataaaaggagtgataacgcagcatgtacagggccggttccggcaaatgatttttcatgatctggtaaatatattcgtcgtgtccccagctcaggtgtacattttccaaaccgcagttaggttcatatacaccatacttggtgttataatccgggttattgatatccggattatttttgaagaactccgggaaaacgattttatcagagaaggcgcagccaacagggaaagtgtcccctaccactgcccattgcggttcgccgaacaggcacaatactttgcccatgtcgtgaaacaagccggtgagcaccatccagtccgggtgaccatcagcacggatggcttccgatgtttgcagcaggtgctggaactgatccaggtctgtatccggatcggaatcatctaccagctggttaagaaaatcgaaggcatcccataccgacatttcccttttattgaaagaaagaaattccttttctttttctcttacaaatgcataagactggtaagtatgatttaaccggtaaaactcccgcaccgtatcgcgtggaggcgcttcataattccggaattcagcggtgcttttttctttgttgatattggcgggatctggatatcgctcaagtaaatcatcttcccattgatccagtgaagtaagtggtgcaggatttggctgcccgttaacgttatccataatatcagattttaaaagttcgtggaaatgcagaaaaatatcctgctctaaatatgcgatctttttaaaaatcttccgcataatagaataactttatttacttaaccgattaagtaacacggccattatatggaaaacgtcaccatcaggatgcttgcagaaaggttgcagttatctactgccaccatttcaaaagcgctgagtaacagtcatgaaataagcgaagaaacaaagcagcgggtgctggcgctcgccgcagagctgaattatgtacccaatccatatgccagcagtttacggaaaaagtcgagtcataccattgcggtagtaattcccgaggtggccgacagcttctttgcagaagccattaatggtatcgaatctgtggcacaggagaaaggctaccacgtactcatttatcttacgcatgaaagttttgggaaagaagaggctattttgaaagatttccagagcggacgggtagatggggtacttatttctgttactacggaaacatcctcgaaagcgcatggattggcgcagctggtgaaagaaatacccgtcgtatttttcgacagggtttgtgaagaagtaacagccgccaggatcaccaccgatgacgccaatgccgcttataacgccaccgcgcacctgatcgccggaggatgccgtaatatgggccttttatcagcttcacggcagctttctatcagcaacaggcgggcagatggtttccggcaggcactggccgatcatcagcttccgcttactgacaacagtattctctattgctccaatgatcctgccgctacccagcaactgctgcaaacagcattacagcaaaatcattacgatggcctgattgccaccacggaaaaactcgccacagcagtataccaggcctgtgaggagctatctctcactattcccggcgatgtacaggtgatcggcttctccaacctgagcactgcacgcttcctgcagccatcgctcaccactgtttcgcaacccgccttcgacatgggacacgccgccgccaccgtactgttcaaagcgctcaaaagcagcagcttcccattgcaggagcagcaacaggtgattccttcttcactgattataagaaactctaccaagtcagggctataaacaactatcccgcagcattttcatatacgcagtgcctttttcacgggcaaagctgatattgcgttcggggatattttccgggtggggatattgctgcaatgccttctctatttccgcttcccgcaacaaatgcagcatgggatagatggacctgttggtataattggccgcatcctgcagatccgtgccggcaaactggtacagcggatgaaaactcgccagctggtagataccggtgtacttctttttatagatcattttctccaccaccgataccaggtcgagatagtcacgaaacacgggaaagccggcagggaaaattaacaacgtagtagataccgccggttcactgtccagcaacaaacactcctgcaacagctcatcactggctgcctgcagcgatacggcgccgctcacctggtaccggatgctgttcctcttcacttccctgttggcaaaagggcagaagttacaaccgatcacaagttccctgacccagttctgagtttgtgtaatgaccgctgctgcctgttccggactgtataccatagcggtgaaggtacggataactatcttctggtgatcaccgtgctactgaagtgatcgcctactttatcatgactgatcacatactgttccataggtaaataagattcgatcataggtaaggcgggcgcataatggtaactaccaccggtttgcagcgatgccagtatttccatgtacttttttgcatagctcatataagcactattgctgcgctgatggtgatgcagaaaatgattggagaaagaaagattggagatgatggtgccccagctattgggctccaggcggtattccagccaatcggcagatccgagataactttccggttgttcaataaagcggtctattccatatgctttgatgccctgtttacgcaggtatcttaccaggtaagcatgttgcccgcaaccgatatccagtacgggacctttgatggcagcggggtttaaccgcagcacagacagttgcgtggcgggtgtatattctgcacacactacctgtttaacatgaggttcctgctcactgttcaattcttttacaaatggattggtgtgtagtaaccattttgttaagcgttgtccatgcaactgttccaggtcatcgaaattggtttgttttcttttaaggcgggtaataatatcttccattaaagtaacatatacggcctttaaggactccccggcaacgccggaaacattcatatactggttggcggcacaaaaagtaagctgggcctgggtggtgaggtaattaaccagccctgctgtcaacccatccgcgttcaattgtaaaatttcacgcggataggtggccagcaggaacctggtataaggcgtccacgccagtgcggcgcttttcccgccataaaaaagattcagttctttatgatgatcatattgtgatgaaatacttcttataatctccggtaaaacatacatgcctcaaaggtacgctgctttcaggtgatcacgggtaagtaatccgtacaaacctgttggcatcacggtaatcaaacttcgtaaaggtgcctactaccagcagcgacttctctcccacctgcggcaggatctgtgtaatacctccactgttggcgttctggtcgagtgttacgccaccaatagtgttataagaagggtgaaccgcgcctttgtcggtgagcacaatcatattattgcgcactaatccgctgaactctgtgaagataccgctcacaattacttctcctccgggcattacatgcgcattgaacaggtaaccattggaccccacacccacgttaaacgtgggatctatcaccccgttttcattgatacgggctacattagccagttttagtccgccgaaagtattgaagcggcctacaatgatcagctttccatctggttgacgggtcatgttcaggatattctgatccgggccggcgcctgctgaaaaggagggatcaatagaaccatcggggtttaacctggcaatgcggttcacggattgtccgttgtatttggtgaaagtacctgcaatcagcatttttccatcgggcaggaggatagagcggttgatataaccattgggcccctctttacccatgtgcttcgccaggtcgtagttgtaggtgctatccaggcttccgtcgggcattaagcgaaccaatccattgatctgcaccgaatcgagatgtacggaatcctgaccggcagcacccacgaggttgtagttaggttgtacataaaaccggaagaagccggtgagcaggatcttaccatccgcctgcacatgcatattggccacctgtccggaaataccgcctttcagggaagacacagtgatttccttcccggtaggactgaaaatcttatctgctgccagcgagccgttgttgttcagcagggcaatactgttgacgaagttcaccccttcatagttattaaaagcccctgccaccaggtatttacgatcggcgcctggaagtgcagcggctgtagccacaaaggtattggtaccatttttcttgtccgggccaaaagagccgtctactttaccatcatgattaatcctcgccacgcggttaagctttccttccttaccggagttatcgaagtctgtgaaatcaccgacgattagatatttcccgtcttccacaggtataatatccgagataccgccattagcggctactttactggggaaaagggtatccatctggaaaacacctattacccggaagaaaggtccgaagaaatactcctggtccacctgtgcagccacattaccggtagctgcctgtgcaggcacctttacgcgcacggtggtatctgtaagcgccaggatgggcgcacttataccattaaaaagaatggccagtttatctttgttcttcaggaatcctttcccgctgatcagcacctcctctcctatgtgtgcactggtgggagtgataccgtctttattgatatagatcgccggctgcacctgttctttataaggatcatcccccttggagctgatcttatcttttgtacaggcgcctaacactgccaggagcactattaaatacgtatattttttcatactgaatgcattaatgagttattgattctgcagttcctgttctgctatcctgacaaattctcccggccggaaaccgaagttgtgccggaaattcagcacatgcagtacgccgtttgtcggctgaatgtcggaggtcatcacctgcactttctggttattggcaaaagtcaccggatcataggtaatatctgtgagcaacagcacacgcgcgcctaccgcttccacgccattatagttctggtaaattaacccgatgttgagaatatagccgctgttcattacgtagttaatgcccgggtaagcgtatacattcaccggatcaatacgtgcaaacttattagccgtatacttccctttgagcatgtacatacccaggaatttcttccataccttagcgggaatatcagccagtttcacgctgtcttctaccatccggtaacggtactcgttcaggtcatcaatagcatccacaatactttgatctgttggtgtaaagaaggtaacagaatcgttctgcaacatttctttcaatccggctttttccaccacatatgccacggtgtcaaagaggtccgggttctgaaccaggtactcataaatagttcctttataatgcggatccgcagtaccgctgtcgatataataatcttttttacaggaagataacaacaggcttgtcatcaacaggatgccggctatgggcaatagctttcgcatagtgaatattttttacagttattgtatccagtattgatttctggtgaccagcggattgttgtttactgccgatgatgatatcggccaggtccatgcgcctttctccatgagatccggtgtgaggggattctccgtcagtattctgtcgccgatccttccggtgcggatgaggtcataccacaggtgtccttctcccatcagttccttttccctttcatagaaaatagccgttttcagcggttctccaccgccgccggcatacagcttggcgcctgccctgtcgcgtaccaggttcagcatctctatcgcttcggcatttctgtttcccaggttggccaatgcttccgccctcagcaggattacatctgcatagcggaacaggataaagttggcgtcataatccctggtaattggattggtgatcgcagaaaatttcaggaacatcggtttcttttctcccttggaagcatacggatcatcgaaccacaggtctatccgtttgtcggattcaccgcggggataaaccctgtcgaggtgccttaccatgggagtgatttcactgttcccgttcagtccatccctgataatgggatcgtgcagggtccactggcagataaggaaatggaaagcgccaccatagttagcatccagcgacagttcaaagatgccttcttctgagcggcctttgaaaatggtctgaaatgtttctttggtgtaaggcaacagtttgtattcgttcagcgccatcagttctttgatcagatcggcggtttgtgtccagtatttctgctgattggcggggtcaaaaccggcgctccacatattgatatgcgccatcagtgccagcgcagcgcctttggtgccgcgtaccgccctgttggtaggatcgtcgtaggaaattaccatatcgtctttacatccttcgaggtctttcagacagaagtccaataccgtcagcattttctcgcgcggcctcagcgtaatatcatacgggtctgtttgcaggggcacatctccgtatagccgtgacatatagaagtagatgaacgcgcgtacaaagcgggcttctgccaccagggcttttttctcccttgagctgaaagccggatcttcaatacctggtatcctgtcgatacaaagattggcggtagcaatcgcctggtaaaacaatccccagtccgggatatcttctatgccgtcgccaccggcctgcagcaggcggttggcagcgaggttgcggaaaccgttcttatcaaaccagttccagttgccggccctgaaatcgcctacattatatataacgccgttggtaaatttttgcagcagctttgaatatataccactaaccgccttctgtgcatcgcctcttgttttccagaaatcctttcctgaaagggtatccagtggctttacttccagaaatttcttacaggagcccacacccagcaaaaggcagaaaagcattcctattttaaaccaatgtttcatctgaaaataatttaagtgtcattaaaattgagcgccaataccaaatgtcaaactggtggcatttggatacccgttgatatcgtcccttccgagtgaggtaacggtttcaggattaggcccggtatactttgagaagatgcctacgttgtatgcagtgagataagcacgcaatacccgcagctttagccgcttcataaaatcaaagtcacggaactggtaagccagtgtgatctggttgattttgaagtaggaaccatcttccatatacaagctctgatccagcctgttgggcgctacctgtgcatcgtgatcaaaagaacctacgatggcaggatgcgatgctttgtcgcccggatttttccagtagtcaatctgattgatatcatacaggttgataggaccggcggcggtaccgtcgttcttactcaacaggttgggatactgcaggcggtagatcctcgcagcgatagcgttattcaggatgctgcggtctgccaggaaagtacagttgatattgagcgacaggttccggtagctcaacgtattgttcaaaccaccggtgaacattggttccgggttacccatgatcatgtagtcggcaccatccaatgcgtagtcgccgttcagatccctccagatgggatctcctgcctggaagtactgggtaccgggacctttaaacgctttgtaacgtacgcccctgatgggatctaccggtacatctgaagtattgctgtatacaccgtctgtctggtacatataattgctctgcggatttcttcctactttcaatgcaatgctctggtaagtgttctgatccactgctataaagagctgcgaacctccgggtaattccgtgagcacgcctttgttgtacgcaccgtttatggagaagatccactggaaacctttgggatcgcggttcataataggccgcgtggtgatggacagctcatggccgtagttcacaatagcgccgccgttgacctgcattttaccgtaccccgtggaattaggcaacgggatatcgcgcaccaggttgtaattgttcttgtaataagtatcgtagataacttctacacgacctttaaacaggcccaggtcaaccccgaagttaaattgggaagacttctccggttccatgtaagggttggcgagcacgccgtagttaggattgatggaaaccgcgttgttgtagtttttcacactttcatatgcacccagtgaattgaggatagtagcggtagggcggctgttaacgccataggttacacgcaccgatccataatccagccagttccagcgccgcatcaggttttctttattaaagttccagcgtacacccacagatggatttttcgtataggggttattgatacctgcagaagagtttccatccaaccggtaggccaggtccaatacatacttcgtacggtagttataggagaagaaccctgcccacgatgcagcatgatatacataagataccggcgtaccgtttacatttatttcgttggcattattccaggggttaccgggatagaaccgcggagaataaccacggggtccccagtagtaatcgttcggaccattgcgtatatctttcacatgctggtcatctgatttgatgttcacttcgctgaatacgctggcatatatgttatggcttttttccaggtcggcaggcctgctgctgtagctgtagttcacgccattcctggtattaagctcatcgtgccggcctacgaaaccatataaaccggtttggttgttattggaaaacgattgattaaaccggtccctggtatcggtgtagtagtcataagaagtagtggagttgatacgcagcccgttgataatttcatagtccacatccacgaaaccacggatattgagggtgttgttatcatctatattattttcatatccactcagctgggggttgccaacaaaggtagaagggccgggcatcagggaagaggtaaaggaatttcctgcaccattgttagtcaatccgccgccattaccacgttgcttttgacccagcgcactgaacaactgtgcaccgatacgcagcttcttgcttggttgcatattcagttgcatgttcaggctatacttattaaaaccggtatttttcaatacgccctggttcatctggtaagcaaagttggccttgtagttcattttcaggttacctccgctgatctgtacattattattggtatttaaagtggtttggtaaaataacccctgccagtcggttgaattattatagaaagcattcaggctgtctgtcaggaactgggaattgggatcgctcagtatgctgcgtgcgtcctgcaaatccctcgcatttttcatgatggagttgatacgataccggcgctcggcattaccaccaatagtagggcgcaaattcggcggcaggttcacaaacaaactgctgttgatgtcgatgatcggtgtaggtgaattaccacgtttggtggttaccacaattacgccgttggcgccacgcgaaccatacaaagcagtagcctgcgcatctttcattaccacgatggactctacgtcttccggcggaattaaggcgagcggacctgttgcggcgcctggttgcaacatcgactgggaaataccgccgtcgaaatctaccggaacgttatcaattaccagcaatgggttgttactggtaagataggcattatcaccgctgccacttacatccagctgggaaacccctctaacggacatggtaccacgaaaacccggcgcaccggaattgttctggatattgaggcccgcaatctttccctgcaggagttcctggatattggataccggcacatcctgcagcgcctttccgtcgatcacgcctgccgacccggatgatgtttccttggtacgcttctggtaacctatgatcaccgtttctttcagcgacttattctccgggctcagggtaatgttaagcgtcgttacacttcccgttttaaccgtttccagccgatagccgatgtaccggaactggatggttttatcgggttccactgaaatggtaaaacgaccggtggggtctgtaacaccaagacctttattattttttacatcaatgatggttacgcccgggattccctctttggaaccggcatccgtcaccctacccttaatggtaacagcctgttgggcatataccctgttgcctgctcctgtaagtaacaggagaagaacaaccaacgtatgtatgtaccgttttttcatggcactaatattttaatgattcagaatacagttaccggtttaatcgttggtaaacttgggatttactttaaacttaaagatcacgtcccagctgcctggttcaaatacggcaaagccgtagccgatacctgcctgccggcgcacaccataggaaatgcgctcatagatgaacatgacgctggctttttcattaatccccacgtccgccagtaccgggtaagggctggttacatcccaggtaacagtggcactgtctgatgaaaacttgcggttaaagccaaaattcacggtcgtaccaacggtgttgctgtaatatctcaggctgtcccatttggtaacattaaacttcgacattttaattggtaaggaatcctgatcataaaatttaaatgtcagtgtattcttagcagtacctgttttaacgaaatacacatttacctgctcgctgttaatctcattgttctgcatatcttgcacgcctattacggtaggatgattgtaaagaagattatcggtattaggcactttcttttgcaggccggtgatgtcatcaaactcgtaaggctcatatggtcgcgggcggcggaggtccagctttcttttctggaaagttttctgcccacctttgttcttcaccaggatatcaaaagtataaatgccctgttttattttggaggtatcggtggaccagaaaacaagatcgcctgaagtagagcgcatgtcaaggaccggccttttcacctggatacgtttggcttcaatttccgctacggttttttccgtaccgctataatactctttccactgccaggtattcacctgctccagcaattccggcgcaggcgtgccatcgggccgtgcgatgttctgcatttcaaaagtgagtggctgcgttgaattgtctgcattaaattttccgtagaacacattggtacgtccaaaattggcctggtacgtatcgccgtcaaagttggcgttattactgaaatgctctttctcatccggcaacaactgcttgtagcagcctgttaccgtaatcgccagtgtgccggctattaataaagtatatacttgccttttcattgctatgggtttattttggtgaagatgagacggtgcaggttcaggttggctttcttgatcatcactttcatcaggtgttttcctgcgggcagatctgccgttccgaatgcgccctgccaggtttgccagccgccggtaccctgtatcgggatgtcttcacatacccttacttcatctatcaaaagataaataagaccaccgccattcccggctatcctcagttctactttatattttcctgcttctttaatatcaacggtatatcgtacccagtcgccgtcgctggtccagccgatattatagttaccaccgggacttgtagcgccatcgccctgcgagcagttttctgtgcccggatcatcgggacgataagtatgcccgccattgggattacgataattgtaagccactcccttggggccttcgtcataatccgctgcattcacaatacccggtatttcaatcgggtagccgaggtatggcccctgcgccggctccagtgacctgggataggcttttccaacaaaggatgtaaatccgaatacatgccgggtttctaaaatgtgcatcaatccgttggtagatttgatgtccacgttttgcgtaagcgcaacggaccagtcttttgtaaacctggaatcatttttatcgctgtactgcaacaccgcggtgcctgcgcccactgcgccggaagcattggtgctggcggttttaccattcatttcatgaccgtacaaagattcgaggtcactgccatccgcatatctcagcgaatcggcggttaccagtccacgcacgatatagcgtcgcaaaagactatcccataccgtcagcggaatactatccagtgtccagttgcctttatcaccgaggcgttcccgggaaaaattcacgttcctgatggctgtggaaatactgttgtcctgcggaacaaaaaaagtgacctgttgatttttaagtgtatccgtaagctttacgcggtctatcagtaatagcagggtgtcatataatcctccctgttgcttgagaaaatcataagtacttaccttcacttccgatacgggctttgcattccggtagtcctgcattcctttttcgcatgcaaaacaagccgttacagccagtagtattaaatattttttcatggcagtgatttattatttccagaaagaattttgaaccagcgcgccattgttggccagcgcttcctgcgatagtggccacaaagcggcgcccctgtctacgtcagcctgtgtaagcctggtatactgcgggatctttttgaaatgtatgaggtcgtaccagtaccatccttctcctatcaactctcttctgcgttccagcaaaatagcatccagcagctcctggccggcagtagctacgtttacatttttgagtgcgcgggagttacggatctggttcaggtctttttgtgcttccgcggtttgtcctaaccgggctttagcttctgcgcgcagcaggtacaattcctcataacggaatacgattatacaagacgaatacattttcagtacgggatctttcaccgcgccgttgatttgtttcatcttgtaaaagatgggataagcttcttccatttttgtaaagaaataggtagggcgttgttccctcgattcgctatagatctttagcacactgtctttcggcacataaatctcagattctctttttggaatatagggttcacggagggtccagtcttccaactgaccggtagacgatatttccgcgtggtcaaagttcatatctatctggaaaatgttggccccgatacgtccgcggaatgcgccatccagcctggtaagatcgttcaggctcacaaaaccgtaaccggtgttcgactggttgttgatgacggtgttggcatactcgagcgacttatcgtattcgcctttccagttatagatatgtgcgagcaatgtataggccattcctttggtgatagtgatggaaatgtgatgtgattcaccctgaccacggtaatcgccttgttgttccggcgacttgccattgtacttccagggtaaaccatcaatacaggattttgcttccgcggctgcataatccagtactttatcccatttttcacgggagatcgtttttgcgaccccatctgacggagcaattaccagtggtacatctccccagatccttacaatataatagtagagaaatgcgcggatgtaaatcgcctgtgcgcggtccagcttcatatcgttttgcgagtaacgataatcggtagcggttacctgtggtaatttttctatcgtaagattgcattgtgctatagccgtataaaatcttcgccagtcgcgccattcctccatagtagaataactggcgttcaggttactttccactactgcgcgcagatcgccgcgcttggtcgactgaaagtcgccaccacgcaaatctccgtacacccagtgtgcattttcgtttgacatggcagcgcgcattaaagcatagcaggcagataatcctgcgcgtgcatcatttttagtctgccacatattttcttctgtcagggcgcgatgtgaaggcacatccagcattttcttgcaggactgcatcccgccagccagtaatagtatcaccccaacaacagcgatatttctcatgatcttgttttttaacatcagaattgaaaattaaagcccagtgtaaacgtgcgcggagccgcccagttataatatccttcgtcatatccgaaatagcttacggcttccggatcgccgcccttgtactttgtccaggtaagcaggttgttaccggtggcataaatacgcaggtgctcaacacccgaacgtttcatccagtctgtttgcatattgtaggccaccgttaatgcgcggagctttacaaaagaggcgtcttcgaggaacagggtctggttgggctggtaggcatatactgcgctccagggattgtattgcggtattttgctgtagtcgccttctactttcgaccaccagctgatttcctttatcgcctttggatcatcaatggcttccctgttggcaaagtcaaaacgatcggccaatgcctggttaatcactttacggccaaaagaatagttcagcaggatgttcacgtcccacgcgccataatggaaggtgttggtaaaacctccggtagcagcgggtgacaggcggcctttcattacacggtccgcatcattgatattaaaatcgccggttaaatctgtccatttaggatctccttttttcaaggttacaccctggtaagtcatcttcctgcctgtttttggattcacaggcacctcatcatcggagttgtaaataccttcgttgagcagcagccagtaacggtccaccggttttcctacgaggaaacggcggttattgatcaccaggtcggtaatcccgtcgggcaaagccatcagcttattctggtttgtatagatattgataccggtggtccactggaatttctttcctttcactaagtctgcatcgatagacaactcatagccgtagttccggatgtccatgccattttttacgataccggtatatccttcttcttccaatgtaggcaccttcagtaccaggttacgatctgttttggcgtatacatccagcgaggcgcgtaaccggtcgtgaaaaagaccgatatcaatgccgccattcagttgctctactaccggccacgaagtacccggcactacatagccggtggtgtagccggcgttaataacagggaaaccgttgtaggtagacatgttaggcaccccattccaacctgcgtctacgttatataccggtccgccggtatacatttcatccatcagcaaacggcctacacggccccagctggcgcggacattcaggttgctcagccaggaagattctttcaggaaatcttccttatgcactttccaggaagcagataaagtaggcgatatcagccagcggttatctgcatcgaggtaggagctgccatctcttctcacatacagggaaacaaaatatttttcattgaagttatatccgacattggtgtagaaagatgccagccgcgactgcgtaaaatctttagtgttaaacatcaggcggaagttgccgaagcggccttctttctgctgatctgtacccggctgatagatcttcacataatcgctggaacctttgtaggcgcggccgtaatcatagcgccatttgtcccattggccatactgaccaagtgttatttcaagatgatgttttcccgggaaagttttttcaaactgaagggaattgtccaggatcatccgcctgttcagtccatcataattggatacataactgttgccttcgccgagtgccgtaggtacaaagaagtcgcggaaattttgcccgtagtcaatagcaaaacgggtgttccaggtgaagtgcgataagaagctatacttcgcattggcaatgatacgggcagaattattcttgttccggttaatggtattttccagcgccgtataatactgttggagataggctttgttgggagataaaggtgcatcgtagttaaagagatagtcttcgtccccggcgcggtcgcggataaactcattccgtttccggttttggttagctacagaaatatctgttgtaaaaatcaggttccttacgggctggatgttgatcccgaagtttacatcgtagcgtttgatgcctgttttgtcatatacgccctgctgcgaggattgcccgatgctgaaacggaagttggcatatggcgttccgccgcttacggcagcctggataccttccgtgaatgcgtttctcaaaaaaagatcatcccagttggccgggccatagtagcgggcctgggaagaatctgccaggtagcggggaaagttacgccactgtgtttcatcagcatatttctggtagaagggcaggcgaaaatcactttcgtatctgccattcactgcatctaccgcaggttttaatgatacaccggcgtaagcatttaccgacacccgcatctgtcccacgcggggcgctttggtagtgatgttgataatcccgttggcagcattgggaccgtattttgcgctggcagcaaaatctttcagcacttcgatactctcaatatcattgatatcgaggaagccaagcaggttggtttccgttcccatcctgttaaaatcgaaccgctgaatgtcataggcgaaagcatgctccatgatcaagggcacaccgtcgaccacataagtgggttgcgcataaaacaaatcgcggttgcccaggagcagggaagaggtccctcttacaaatacgctgttgcgttttccgggttctgctgaaggaattcgtacatccactcccgttacccttcctatcagcatctggtcgatactggtgtagggaagttttttaacctcgccaatgtctactgaagaaatagccccactggcactacgtttcaggaagagttcattgttgggaaaatatcccagtgtgtcccgcctggtagatgtcactttggaaaaggcaagtgaatctgcattcacaccggaggtatctttgttatttttgaacaacacattctgtgcttccgatgatgtactcaccaggcacattgctgcaaaaaaataaatacctctgtgcaggaaaaagtaaaagtatttcatacatgcaatatttaggaatgagaatcccagggcgtaaaagaagctttacaccagattaactattttttgacatgaacgggcataggttgccctgttccctttaggggaatgtctgtgatttagagatcagcgttcgccatggctactacagcacaatatctgccatgcaaaatgcctcgtcagcataagcaggatgcgaaaataatgtcgactgtggaaacataacgcccgtgggtagttagggacagcgggtgaccctatcaggatgtaatgaacgttgagtcatggaaacaagattaattaacgtgaaattttcaatcggtctgtaattctggttttcagtaatggcagtactaatgcacagtggggaaactacagcaaacacagggtcttactggtcatcagtactatcaatgctctttaaattctggttgtttttttaacgctactgtaccaaatgtaattagctaaaaggatttttcatagttttttgtgaattattttttaaaatttaatccgggaggtaacaccgccttcatcttcgtgagccttttttcaaattcttcattcacaatgaccggggtagtcttcacaggtgttaataatgcaggactttatcgttatcatacatccccatgcgggtccagatcaatatgccctgtcggtggtatagcgcaccaattcctccaatgcggcccgcgtgggtgagggcggaaaagtaaagagtatccggaatgcttcatcgcggtattccatcattttttgggtggcgtaatcaagtccacccgactggttcaccgtttccactacaaagtttactttatccttgtcggtatgctggtgctttactatatgaaggatctttttccgcaacgcagggccggcatgctgaacggcataaataaggggaagggttactttcttttctttgatatcattaccggtaggtttgccgatgtcggtatttccataatcaaacaggtcgtctttcagttgaaaggccatgcctactttttgtccgaagttgtgcaacagctggatagtttccgggttatcgcaggcggatgtggcgccggcagcgcaggcagcggccaggaaggaggcagttttagcattgatgagatcataatagtccttttcctcaaagctgagtttattggctttcgtcatctggagcaattctccttctatcatttgctgaatagcggcggcgtagattttaagcaggccggggtcgttgttatcgagggccagcagtacacctttggtaaagagctggtcgcccaccattacggatacacgatttttccagagggcgtttacagaaaatgcgctgcggcgtttcatagcgtcatccaccatgtcgtcgtgcacaagggaagcggtgtgcagcatctccaccaggagcgcggcgcggtagctggcatcattgatggcgccacacaaccgggcgcacagcaacacaaacatcggacgcatctgcttccccttgtgggcagcaatatccgccatgattctgttcagcaacagtacatcacttcgcatggcatcatgaaaaatttcctcaaaccgctgtagttcgctaccaatcgtttcccgggctaattgcatatgatcatcactatgaacggggccgaaattacgacttctgtgggaaagtatgacctgggacctgacctttctttattgccggaagcccagcacaaaatgtaattgctgcatgtgttttaaaaaagccagcgtatcctgctccagtgtacccgtgtccgttatattcagctgcggcgcgtattccagtatatcctttaccgtgatgccgagtgttaactgctcagtaaggaaggccagccagggcgacaggtccgtgaactctacatgccctgtttccgggtgacggaacagcagcacaaaataaacgcctttatttttcagcagttctttcggcttcgctaccaggtgaacggggtagttaaaagataacagccggtgctcaggattgagtaccagcggggcatccagccagttgccggaaagggaatacgcaggtgcaggtatatcttccatgttatacacctccatttcggcccactcaaaagcgaggaggtcgttgaggaagggaataccataagcatcttcccagttatgctctaccgcgtaagtataaaactccagggggagtttccatacctggtacgactgacatgcatgccttgaaaaaaattccttcaccattttattccacctggtggtgggaatatgtttaaatgcaatggggaatgcatgctccatagtatcctggatcatgttaaataccagctggcgatagtgtttcagccggtgcggcgctacgccgggcagcttcactttttcaccggttctgcaataggtggaaaaagtttgctggatatgataagtgtcaggcaacaagctcatctttccgtttccattgtttgtgacaaatatttttcaacctggttaactccccctgcagttccgccatttccgggatattaaaatccctttccagtaaaaccggtacgggttgcaggtgctgaatggtccattcaaaaaggtcgtacaccgggtctataattggttccccgtgcgtgtcaatgatcagatcaggagctacctgttcatgacctgccatatgtatgtaagcaactttactaaggggcaattgtcgtataaatgctttggcatcatactggtggttgaaagcatttacataaatgttgttcacatccaggagcagctggcagccggattgttttaccacttcattaataaaatccacttcactcatttctgcggctaccggtgtgtaataagatacaatttccattaccagcgggcgttgcaaataatcctgcacctgctgtatacggctggcaatatgctttaccgcatccatccggaagggaatgggcaacaggtcgtacatatgcgcgttatcacacttggaatagctgagatgctctgagtagatctgtacgttgtattcccggagaaatgcttttatgtaccggagaaacgatttatccagcgcttcggggctgccgatagaaagggaaagcccatgacaaagcacagggtatttttctaccacgcggtgcaataccttcttccagtatccgccaatgttcatccagttttcaggggcaaactcaataaagtcggggcggatatgttcaccgctgatcatctcttccgcaaattccctgcgaaaacctatacctaccatggtcgtacattttaggaggttaaaatacgagtaaagaccggcctgcatatgataccggtctttaccttatccgggaaatcagctgccggattttgtactgtcttttttatgcttatctcctttcttaccttttttatcgccgcattttccttcaccacatttaccctgaccgcatttaccctcttttgttttacctgcagcagcgctgtctttttttgcgccgcatgacagttcaatcgcattggctgtattgccggatgcgccggttaatgtacttcttacggccgcgccggaacccaggttagtataactgccgggggttgcagttacctgcaatgcagccataccgaggatagcaccggcaacaagagagccggaaaacagtacttttttgctgataggattgttgtttttcatcttcttgaaaatttaagaaactggtgagaaaatatatgtttctgacagacagacgtgatgatcgttgtttatgtttcgtagtggaaagcttacggaaaattacctgttttagttttcccggcaaccaaaaaaaatgttaaaggcggataaccggtaaagagagtatggcaaatggtgtgataaccggcatcactattcagcattttatcctatttttggcctgtacccaatgaaatatgaattaaactcggcccatgaaaaatgaaatgtcgcctgtaacgtccgtttactttgtaacattattgaaggcatatttacgtggtactaaaacaagacaggaagtaatagatgaattgcgcagcgtatccccgctgcaacagaaggccggagaagaatcagacactgaagtgagcaggttactgttccagactgccagtgaaatcaatgaggattattaccaggatatagtcactgctatttcgcatgcttccgataccactcccacccgcgaaggggttattcaccagctggaagcgatgctgaccggctatatcaccaaggaacagctgatccagtgggccacctggcacaacgagcccggtaccgacgatggagcgggtttctttgatgatatcgcggtagattatttttgtacccagctattgcctgcttctgccggtgaattaacgttggtgcactacaaacaggcactgaggattttccggtcgggccagcataacagcctgaaagacaaggtggcgctggtgttgttatctgaaaaagaaagacagcggtttctcttttatctcagtgattacatacagggacatacttcgccggagcaactggatgtatacctgcttcataaatttggtatggaccatcattcttttccctatatgtcgtccctttccgccattatgcacgatcccgccaaattaccggcgcttctacacctcgccgccatggacgaataaacacatcatataaatttaacatactaactaaccatcaggctgcagcctcttaacgcagagttgtccagccggcccagtacttcaaaccggccatcagcatggatacggccaatgtcttccgtggcaatgaatgcacaggagtaaatattagccaggtcaattatgttcattacgcccgcgcctttgccggcagtaagctggaaaggatcgttttcatcacgcaggagtactttcatccaggggggcgtttcaaacaagccatcacatttggaataagcctgtgataacagctccgtcatgccatattccgcatggatacaggccgttcccagccgctctttgaggaaagcatgtacttcctcccgggtccactcctctcttcttcccttcatgccgccggtttccatgacgatggtatttttcagggaaagggtatactgctctgcaaaatccagtaatccgaaggtcacgcctatcagtaataccttttgtccgcgtgcttccagcgcctgcagctgttgaaacaacttatcatgttcatacaggtaaaagccgctttccgcgtgtccgctgcggagggtcatttcctgcaccatgcgcaccagtgaagaatgctggcgttccaggtaggaaggcaacaatcccactaccacgtagtcgctcaccgggccataaaactgttcaaacgctgtcatgaagctccgggtgtagatcgcagactccttcaccaggtgccggctgttcaccgtttgggtggtgccgctgctttcaaagatcagctcaggcacaaactgaccgcatacgacggtatgtgatttgaaaaattgtatggggagatagggaatttcaagaatgcttttcaccgaagcaggcgggatgcgcagggcatctgtataggccctgtacaggtcattttcccggtactggtactgaaacagctccagtgcagcggcttccagcccgttttgggttaatgaaaatatatattccggtgatacggcggtcatgtaaagctgaatttaaaatcgcacaaagttagggagaagaataaatctatccgcagtaagtaacaattgtcacaaaaaaacgttttggtatagatggatagcgataactgaatatttgtatatttcctaaattaatgtaggtttgttttatgaagaaaattctgtttttgttcctgctggccgggttattttacgcctgtaaaaaggataaaataggcaccaaacccattctcagcttcaaaggatattcgctcgacagcgtggtaaccagtacccaggtaatgtttgtaacgctcgatgtccaggatggcgacggggacatagaagacactttgcagatagcccccatctatgataccaaactacaggacaccttctatattgtgagacggatgcctgaaattggcgccaaccggggaaacagcgtaaaagcagaagtagctatccggctcgatcccgtggatttcagaacctaccaaagcccgagcgacagcattcatttcctcgtatttatccgtgataatgccgggaatatcagcgacaccatcgctaccccgaaaataccttacaacattccctgacaaacgttacattctaaaatatcatacatttaaggattccttttatcaaaggaatccttttatttttagctttacttttgatttttagcatatggataaaatagaagaactacaggcaaagatcgccgaagcaatgcttggcggaggagatgtacgtattgcttcccagcataaaaaaggtaagctgaccgccagagaaaggatacagttactgatggatgaaggttctttcgaagagctggatatgctggtcactaaccgcaaccgcggactcaccgccgaccaggaacagtttctcggcgacggcgtggtaaccggctacgggaccatccacggccgcttgacttatgttttttcacaagacttcaccgtatatggcggtagcttgtccgaaccgcatgcccgcaagatctgcaagatcatggacctcgccatgcagaacggcgctcctctcatcggtttaaacgacagcggcggcgcacgcatccaggaaggtgtggtgagccttggtggctatgccgatatcttttaccgcaataccagggcttccggcgtgatcccgcagatctctgccatcatgggaccctgcgccggcggcgccgtatactcccccgctatcaccgacttcatcatgatggtggaacaaacgtcttatatgtttgtgacaggccccaacgtggtaaaaaccgttacccacgaggaagtaacttcagaagaactgggtggcgcgcaaacgcacgccgctaaaagcggtgtaacccatttcgcctgcgctaatgaaatagaatgtattcagtatatcaaacagctcctgagctatgtgccgcagaactgtgaagaaaccgcaccggtatacccttacgaaccagggaacgaaatacgcgatgccctcaacacgctgatcccggagcatccgaaccagccgtatgacatgaaagaagccatcgagcagattacggatgccggcagcttctttgaggtgcataaaaactttgcagagaacatgatcgttggcttcgcccgcattgccggcaggagcatcggtatagtggccaatcagccggcccacctcgcaggagtactcgacattcatgcctccgtaaaaggcgcccggtttacccgcttctgcgatgcatttaacgtcccattgctggtgctggtagacgtgcccggcttcctgcccggcaccgaccaggaatggaacggcattatcaccaacggcgctaaactgctgtacgcactcagtgaagcaacggtacccaaacttaccgttaccacccgcaaagcctatggcggcgcctactgtgtaatgaattccaaacacatcggcgccgacctcaacttcgcttttccacaggccgaaattgctgtaatgggcgccaaaggagcggtggaaatcatcttcaaaagagaaatcgatgcggcgccggatccggaagcacgcatgaacgaactcgtggccgattacacggaaaggttcgcaaacccttacctggcagcagaaaaagggtacatcgacgaagtgatcaaacctgaaatgacccgtatcaaactgatcaaggctttcaaaatgctcgaaaataaagtggtaaacatgccgcgaaaaaaacatggcaatatacctttgtagcaaatggcgccccgctttttcatactaaaaagcggggtgctaaaagctaaacatatgctccgcagtcttttcaaccttattctcttcacctccgtttatatttcagggtgtgccatcctgatggtatggcaaaccaatcagttgctggcactcgattacccgcataataccttttacctttttgttttcttttccaccatctgcagttacaattttcactggtaccttacacccggcgcctactcggcctcagaaagaatcctttggggtaaccgtcaccgtacccttatgctcactttatgcggcataggcctggcaggctctctatggtttttctggcagctgcgcgagcactggctggtactcagtggcagcgcagtactcacttttttgtattctgcacccaaagtaccgcacaaggcattcaggtggctcagcaaaatagccatcgggaaaacactattcctcacctttgtatggacctatgtaaccactgtgcttcctgcgctgatagcggacaacgtgatcacccagccattggtatatctcaccatacaccgttttggtcttatctatgcgatctgtatcttatttgattaccgcgacctggaatcagataagaaagaaggcatccgcagcctgatcactaccctggatgagaaaaacctgatgcgactttattacgcttccctgctgatagccgccgtaagcgccggtttaatgtggccctataccacgctgcccgctgtggttaccctcctggtaccggtcatcgccacggccatcatcacccggaaagcgcagcacaccgattccgattacctgttctacttcgtactggatggattcatggccttgtcggccgtattatatctcatgatcgtttaacccggatgagcacaatccggcgttttccttacatttgtcgcgtcacaatctgcaaatattatgtctaaaaaacagaaatcaatattcaacaaggaatcactgacattcctggaaacgtacctgaataacccgtctcctaccggttttgagaaagaaggacaaaagctctggctgaaatacctgacgccttatatcgatgaatattttgtagactcctacggatctgcagtaggtattatcaatcctaaagcggaattcaaagtggtgattgaagcccatgcggacgaaatctcctggtttgtaaactacatctccccggaaggactgatctatgtcatccgcaatggcggctccgaccagcagattgctccttccaagcgtgtgaatatccatactgagaaaggtaccgtaaaagccgttttcggctggccggcgatccatacccgtatccgcagcggcgatggcaaagaaccgcaaccaaaagtggaaaacattttcctcgattgcggcgcacgctcccgcaaagaagtagaagaactgggtatacacgtaggttgtgtatgcacatttgaagatggtttcgaggaactgaactacgactactacatctgccgcgctatcgacaaccgtattggtggtttcatgattgcagaagttgcccgtttgctgaaagaaaagaagcagcagcttccttttggtctttatatcgtgaatgctgtacaggaagaagtaggtttgcgcggcgcagaaatgatcgccaaacgtattaagccaaatgtggccatcatcaccgatgtaacgcatgataccactactcccatgatcaacaaaaatattgagggagaaataaaatgcggcagtggtcccagcattacttatggtccggcagtacataacatcctccgtgacctcatcatcaaaaccgccaaaaagaacgacattcctcaccagctacatgcggtaagccgcagtaccggtactgatacagatgcatttgcctacagcaatgatggcacaccttctgcgctgatcagcttaccactacgctatatgcatactacggtagaaatggtgaagaaagatgacattgaaaatacgatccagctgatttaccaaacattactgaatattacgccgaaaacgaacttccaatatatctagcggattttgtctttcccaggattacgctgattatactgatttactggatttttacttttggattttataaaggatttggggagatagaagcggattttgtctttctcaggattacgctgattttactgattttacttttggattctttttagatttttggattccataataattaaggaagacaagggcgaaaatatccgcttctatctccccaaatcctttataaaatccaaaagtaaaaatccagtaaatcagtataatcagcgtaatcctgagccaagacaaaatccgccgcgatactaattcttaaagaagtccgctgcccggttcaccttctccacccatgcgccggaaccagcctgcattacatattcgctcattcctaccctgctggcgcccggggcccagtcgtaggtgtagccgagccttgtccacggatagtgcatatctgtggctgatgtcagcgggcggtagtaagcgaagatgatgtagttgttaaaccaggtggtgaagtccgacgatacgccgctgatggggactgcaccggtggttttggtagtaatggcaggattgccggcgggacggtacaacctggaggcacttacccacatggtagcgatatgggtatttgtttttgagttaacgggcggtagtcccagtaactggcagatacgctgaatggtatctgaagtaggcgtaagggatggtcctatcctggtcttcatctgttttgggatgaacagccaggattcgccccatacggtgttgatggaatcgccggccgggtaacttccggggaaacgcatgaaggtagccatcaacacatactgctgaccattaatggttttccattgcaggtcagggttgtctggtgtgatgggccacagtgcatcggtaatttcgctgctgtcggcaatcatggcatcatctacggcctggctgtagagctgatccagggtgtacaccggcggcggaggcaaaattgggtcatcatcatttttactgcaactggaaaatgccatagcggcaaatagagcgagtacggacagcttactgcccttagggaaatgtttcatagaagtggttttctggatgctggttatttaaattgagtcccgcaattaagtgtatttcaacagaataatcaaatttccttcattttcactcctactaattggtaatttgtatttcgtaataatttgctacgtttgctattcaaacaaaatcagatctatgatccgtcatgactggacgttagaagaaatcaaagctatttacaatactcctttactggaactggtataccgtgctgccactattcaccgtgaataccaggatacagcagaggtgcaggtttgcaccctcttgtccattaaaacaggcggatgccctgaagattgcgcttactgcccgcaggctgccagatacaacactgacatcaatgtgcatggccttctgaaaaaagaggacgtgatgagttacgcccagaaagcaaaagaggcggggtccacccgtttctgtatgggcgcagcatggcgtgaagtgcgcgacaaccgcgatttcgaccgtgtactggatatggtaaaaggcgtaaatgaacttggtatggaagtatgctgcacattgggcatgctgaacgaagaccaggcaaagaaattagccgatgccggcctgttcgcctacaaccacaacctggatacttcccgtgaccactacgaagaaattatcaccacccgcacttacgacgatcgtttacaaacgctggataatgtcagaaaagcaggtgtaagcgtatgctgtggcggtattataggcttgggagaatcgcatgaagaccgtatcgccatgctgtggacacttagcagcttaccgtcgcatccggattccgtgcccatcaatgcgctcacccgcgtaaaaggtacaccgctggagcatttacctaaggtagagttctgggatatggtacgcatgattgccaccacccgcatcctgatgccaaaggcaatggtgcgtttgagtgcaggccgtgcggaaatgagtatgtccgaccaggccttatgttttatggcaggcgccaactctatctttacaggcgaaaaattattaactacaggtaatccttcctttgaagaagaccatatgatgtttgagctgctgggactaaagcccagagaggctttcaaagcacaggaagcggtggcgccttcgacgccggaaattgtcttggagcgctgattacgctgattatactgattttttggatttgatcagttttgattttataagattaagggagatataagcggataagtccgcatatatctcccttaatcaattataaaaaatccaaaaaaatcagcataatcagcataatcagcgtaatcagcgtaatcagcgtaatcagcgctcaagacaacctccgcggcgccgaaggcgcctacaagtcgttcatcccgaaatactctactcccaattgatatcctttgagtccgagtccgcagatgcagccgatgcatttgggcgctatcagggaggtatgcctgaattcttcccttgcatacacgttgctgatatgaatttccatcaccggtgttttgatgcccgcaatagcgtcccggatggcaatggaggtatgtgtataagcgcctgcgttgagcagcacgccatcatatgaaaatcctacttcatgcagatagttcacgatttccccttctatgttactttggtggtagctgaaagttaccgccggaaattgtttttgcagatgtttgaaatactgttcaaaagattcgctgccatagatccccgtttcacgcttaccgagcaggttcaggttaggtccgtttataatagctatttgcatgataatggttatagaatgaagaatgagggactaagataattaatcctgtttattattactatcgcttccccagcggtaagtttgctgttccaggcctgcgaggtctatgatccggtccaccactgtggcggccatttcttcgagattggcgggaacgctgtaaaaggaaggagtggctgggcagataatgccgccggccagggtaactgcttccatatttttgatgtgaatgagattgtaaggggtttcccgtaccacgcagatgagctttcttctttctttcagtactacatctgccgcacgggtaataagatcgttggaaatgccggtggcaatgcgtcccagcgtacccatagaacaagggcagataatcatggtgttaaaccgtccggatcccgaagcgaaaggcgcgtggaaatcctgttgggaataaaaacggaaaggcagttgtttataatcttcgtctctgagctctgtttcccataccgttttggcgttttctgtcatcactacagctacctggtccagctgttcatgtgctgcctgcagcttctgtaacaactgacgggcatagatggaaccacttgccccggtaactgctactactatacgatgtttcattggctatgctgttgaatttacaaagctagcctatttgggtggttatacgccagcctgtgcaactatttcatccatggcaatgccgccatgactttcattgtaaacacattggccgttgcggatgaccagtacctggggagactcatgctgaacattatagacttccgcaattttattggataccggacgatgggcgatcagatccaggtaataaaacgttaacccttctggtacagccgaccgttccaacctggccttggccatcgagctgatagagcatcgcgtgctgtgtttgtaaataactaccggctgatgcgctgatactgcattgatttcagccaattgttcctcgctggttaacgttttccaattcatttaacatgctttgttatgttctatcgcaggcgacttggccatgcccttcatgggacagcctaatttctgatggcttgcgcaggacgttaagaaagcggcaaagatacaaaccatagcggtgtagcccaaaattcttacataagattgcatactggcagttttaaataatttatgactaaaacgaattttcacaggaaatatgatacgaccacttttttaatcgtcttttgtaacgttattttgcaaatatagaaaatacattaaaaaaaacaacaatgtaattttcggccagccgaaaatatccagcgttatgacaaaagtacattttattgccataggcggcagcgtaatgcatcagttggccattgcgctcaaaaataaaggttaccaggtaaccggcagtgacgatgagattttcgaaccggcattgtcaaacctccaacaggcgggcattttaccagccagtaccggttgggaccctgcccggataacgccggatctcgacgcagtcatcctcggcatgcatgcccgggacgacaaccccgagctgataaaagcccgggaactgcagctgaaaatttattctttcccggaatatatctaccaggaaagtaaaaataaaacgcgggtagccatcgggggaagtcatggtaaaactaccactaccgccatggtaatgcacgccttgcagcttaatcatcagtcgttcgactacctggtgggcgcccggctggaaggttttgcccagtctgtaaatatcacagacgcacccgtaattgtgtgcgaagccgacgagtacccggcctcggccattgaaaaacggcccaagttccactttctgcatccgcagatcgcggtattaaccggcatcgcctgggatcatatcaacgtatttcctacctacgaaatatataaagaacagtttgccatttttatcaggcagatggaagccggtcagatattgatctacaacaatacagatcctgaactcgttagcctggtaaccgctaccggcgaccaccttaaactggtgccatacggcctgcccgaacataccattaccaacggcgttacccgggttgtttttggcgaccagcaggccagcctggaaatttttggcgatcataacctgctgaacctccacgctgctaagctcgtttgtaacgaactgggcctctctgatgcggaattcctggcagcaattgctacctttaagggcgccgcaaaaagactggaactcgtagctaaaaacgatcattgcgttatttaccgtgattttgcacacgcgccttctaaagtgaaagccactatggaagccactaaacaccagtttcccgacaggaagctgatagccgtgctggaattacacacctatagcagtttaaatgcagatttcctggaacaataccacggcgccctcgatacagcagataccgccgttgtgttttacagcaaacatgcactggaaataaaaagaatgccggatctggcgccggaactcattgcacagcggtttggccgggatgacctccacgttttccataacagggaaaaactggaagctttcctcgccgcacaacaataccaggacaccaacctgctgctgatgagctccggaacatatgatggtctcgattttagcaaactgaaagcattattgccgtcagacaaataaatacattaaacaaattataaattattcataatgccttctttgctcctcaaaaggccgctggccgtaatcgatctggaaaccaccggtaccaacgtggcttccgatcgtatcattgaaattgctatcatcaaagtgtttccggacaaaaccacccagtccaaagtgaaacgcattaaccccggaatgccgatcccagcaggatctacagcaattcatggtattaaagacgaggatgtaaaagacgcacctacctttaaacaggccgctcatgaactcaaacagttcatggataactgcgacctggccgggtataactccaatcgcttcgatattcccctgctggtagaggaattcctgcgggccgacatcgaatttgacgtatcgaaacgcaaatttgtagatgtacagcggatcttccacctgatggaaaaacgtaccctgggcgccgcctacaaattctattgcgataaattgctggaaaacgctcacagcgctgaagcagacgcattggccacctatgagatcctggaagcccagctcggccgctacgaacaattgcaacaggatatcgactcactcgccgatttcacaaaagaggaagattatatcgactttgcccgccgcctcgtgatgcagggtggacaggaagtgtttaactttggtaaatacaaaggccgtcctgtcagggatgtgctaaaggcagaacctcagtactacgattggatgatgaaagcggattttccgcttaataccaaacagaaactgactgaaatcttccataatatgatgttaaaaaaaatgtaatgttattcgggaacgtcatatcttgcgccggaattgaattattttcgcagtccaaaaatatcatctgctgaattggaaaagcttgtcatcattcctacgtacaatgaaaaggataatatccgtaacatcattgacgctgtattttccttacagcagaattttcatgtcctcattgtggatgacggatcgcccgacggcaccggcgctattgtaaaatcattacaacagcaacatcccaacgaattattcctggaagaaaggtccggcaaacaaggtttgggtacagcttatatccacggtttcaaatgggcgctggcccggggctatcagtacatcatagaaatggacgcggatttttcacacaatcccaaagatctgccgcgcctgtatgacgcctgcgctaaagatggagcagatgtatccgtaggttcccgctacgtaaaaggcggcaaaaccgaaaactggccgtgggaccgcgccgtactatcttatggcgcttccatttatgtaggcatgatcacctggatgccggtaaaagatcccaccgcaggatttgtatgttaccgcaataccgtattggaatccattaacctggaccagatacagtttgtaggctacgctttccagattgaaatgaaattcaccgcatggaagctgggctttaaaataaaggaagtggctattacctttaaagaccggaaagaaggctattccaagatgagcaaaggcatcgtaaaagaaggcatcctcggcgtactcaaaatacagtggcaaagccttttccgcaattataaaagacgggttcagaattaataaattacatcaatcgcatagcatttagggatctgttcatttaaaaaaatgaccaggtccctaaatacattttaacggaccatgaagaaagcatttctccagctacacctctccgtatttctggctggatttaccgggatattgggcaaactcatttccctcaacgaaggactactggtatggtaccggttactgatcacgtccgttactttgtatgttctattccgcttccagggtacctttaaaaaactcccctggaaagacatcctgcccattggcagcaccggcgtagtggtagccctgcactggctcttcttttatggtagtatcaaatattccaacgtatctatcggggtaatctgcttttcactcaccagcctgttcaccgctatatttgatccactcatcaacaggcgccgcttcgacgtggccgaaatgctgctaagcatgctcaccctcctcggcatcctgcttatcttccattttgatacgcaataccgtaccggcattatcctcggaattatttctgccatgttcgccgcgctgtttaccgtatttaataaaagactgatcaaacggttcgatacctataccattactttttatgagctgtcgacaggcttcattgtgctcaccctcgccatgcctctatatctctacctgtttccggcccctaccctgctgccctcgtctatggatacactctacctccttgtactggcctggttctgcacggtgctgatgtacctgctgagcatgagcgcattaaaaaaaatctccccgtttaccgtcaacctttgtttcaacctggaaccggtttacagcatcgtgatggcgtttgtattgtttcatgaaaacaaattcctgaataacgccttttacgccggactgggttgcatcatcctttccgtaggactgcaaatgctgcgggtagtaaagggtaaaacggcgtcgtaatcccctccgttcatcctcatttatttgtaacttgagcgccgtaattattactttgcgcttatgagaaaagttttattaggggcatccctcctgggctcctccctttttacctatgcacagcaacctgcaaaaaagccgctggaccacagtgtttacgacagttggcaaagcattggcactaaactgatcagtaataacggacagtgggtagtgtatactgtagtaccgcaggaaggcgatgccagcctcgtgatttatgaccgcaaaacaggtcagtccaccaccattgaccgtggcggcagcccggtgatcacagaagattcccgctacgtgatctgcagcatcaaaccgttttttaaagatacccgcgaggcaaagatcaaaaagaaaaaagcgtcagaaatgcccaaagactccctggctatcattgcattgggacaaccgggtatcctgaaatttcccggtgtaaaatcttttaaaacaccggaaaaaggcagtggtctgctcgcctatcttttggaaaaaccagcagcagatagcaccaaagccaaaagaggcaaagcccctaaatcgctggatgataccgatcgtgcagacgacgacaaaatgcccgctgccggcactgaaagcggcacgctggtgatccgtcagctgcagagtggtacacaggataccattaagaatgtaacggaatttacattcagcaaacctggtaaccagctgctcatagaaacaaaggcagataaaaaagattcgctgtcgcgcaacggtgtactgctgtggcgtgccgccaacaggaaagcggtggcattgagcaacggtaacagcgattataaacaatttgctttcgatgaaaaaggagaacaggcggcgtatttcggcacgcgcgattctgccaaagcattacaacaattttataaattatattatttcaaacccgggcaggacagcgcctacgaagtagccgataaaaacagcagcggcctgccggccaactggagcatcagtcccaacagcctcatttatttcagtaaggatggtcagcgcctgttttttggcaccgctcccgtgctgcccgtgaaagataccaccatcgtggacttcgaagtagctaaagtggatatctggaattataaagatgattacctgcaacccatgcagttaaaaaatgtggataaagaactgaaaagaagttatgccgccgtatattatccaggcagcaaacgggtgatccagttaagcgataaagacctggaaaccgttgtcaccgctgcggaaggcaacagtgctaacgccctcggctatacggataaaggcgcgcgcatccctatgcaatgggtgggccgcacactgaaaacagcttacctcgtaaacataaatgacggtacgagaaaaaagatcaaagaaaagctggacggtaactttttcatctcccctaacggaaaatatattatctggtacgacctggcaaaccgggagtggttcagttatgataatgctaccggcgccgcggtaaatataagcaaaggcattcccaccaaagtatatgatgaggaagatgaccatcccgatgtaccggatgcatacggcatcgctggctggatgaccggtgacaactacgtatacatttacgaccgctacgatatatggcaggtggatccttccggtaaggcagcgccgctgaatatcaccaaaggcctgggccgtaccaacaaaatacgtttccggtacctgcgcctggatccggataagaaatttttccttcccggcgaccgcctgaccttatctgctttccaggacagcaccaaatacaatggtttctattcgctggaactgccgcgtaaaagcggtaaggctgctaaccttcaacccgtggtactcgggccttattcatacaccgatctgctgaaagcaaaagatgccaacgtgttttcgtatacccgtagccggtatgagctttccccggatgtttttaccggagatgatatcgcaaaagcgacacagatcagtcataccaatccccagcaacaaggatataactggggcaccgcatcgttgtataaatggacaactttcagcggcaaaccggcagaaggtattctttacaaacctgaaaattttgacagcaccaagcagtacccggtcatcttttatttctacgagaaattaacagatggattatacagttaccaggcgccggcgccaacgccgtcccggctgaacatttcgttttttgtgagccgcggttacctggtggtagcgccggatatcagctatgaaaatggttatcccggaaaaagcgcttacgattatattgtgagtgccgcagaagacctggctaaaaaagcctgggtcgacggaaaaaatatgggtatccaggggcagagctggggtggttaccaggtagcttatctcgttacacaaaccaatctctttaaagcagcgtgggcgggcgctcccgtagccaatatgaccagcgcttatggcggtatccgttgggaaagtggtatgaacaggcagttccagtatgaacattcgcaaagccgtatcggcgctaccttatgggaaaaacccgagctgtatattgaaaactcacccttgttcaacctgccgcgcgtaaacacgccggtggcaatcatggccaatgatgccgatggcgccgttccctggtaccagggcattgagctgtttaccggcctgcgtcgtttaggcaaacccgtatggttgctgaactataacaacgaagcgcataacctcatacaacgccagaaccggaaagacatccagcgcagggaacaacagttctttgatcacttcctgaaaggcgcaccggcgccgcaatggctggaaagcggtgtgcccgcaacagagaaagggatcaactggggctgggatctgcaacagtaaactaacggcaataataaaaacgctgcaggcgcctgttaaggaacctgcagcgttttttgttaatacgggaccggagataatgctattaacagctaatgctgacagatgaccgatttttgagaaatgccgaatctatatatcatagccggttgcaacggcgccggaaaaacgaccgccagtttcacactattacctgaaatactggactgcaaagagtttgtgaatgcagacatcattgctgcagacatgtgtcctttccacccggaaagcgttgctttacctgcaggcaggcaaatgttgcaccggatcagggaactggtgctggcaaaaacagactttgcttttgaaacaaccctggccaccaggagttgtgtatcgctgattgaaaaagcaaaagaaaccggttacaccgttaccctgcttttcttttggctgaattcccccgaaatggccgagagacgggtacagaaaagggtgaaagaaggcggccatcatattccccccgaaatcatcagaagaagatatcacagaggtcttagtaacctcatgaacttatatatccctgtctgcgacaactggctgatgatagacaacaccagtacaacaccattagaaatcagttcaggcactaacatcccttcggaatctttttgtatatgggatgtattccccctccactgtggcagggaggaaccggaagcagccggccaatatgaatttaaaatactctccggaagaataatgcagggccttgaaacagctatgtgtaaactggtagaaacgaatgctggtcttgaccgggagctcattatcggcgataaacaaggtaatatcctaagcattcctgccagagatatcccgctcactatcaggtgatttcatcttccaccaaatatatttttcttaatataaatcatttaacatatatttacaataacatcgccacttcagcgtatggtgtgatctgcagcgatagcgatatccttaacaccacattattgtacctatgaacttccatatccatcatcccgcggatgcattacgtccgtttgtaaagcaatattattattgggaagacgatacccgtggtattattcaactaccacaaaacctgtttgccctgggcgatcagtacatggtattcattctcgaagggaaggctgaagttaaaccagtgaatcacaaggcattcaccttgcctgcgggctctgtgctggggcatcttacctgcgcctgccagttacaggtgcaggggccggtaaaggcagcagtaatacagctgaacgcttatggatgctaccggcttttaggtatggatgccgctaatttcaccaactactaccgcaacctgttggccgccggacaaccggtgtggcaggaactgatcacggccctccaacaggaaaaggagccgcaacgcatagagtcattgctggatggcgcttgtctgcaggcgctttcacagcaaccgggcaatctccgtgaagtagacgacatggcagattacctggtgatcatgcagggaaatgtaagcatggaagaacttaccacccgctacggactttcccgtcccacgcttgaaagactcttcagcaaaatagtaggtattccaccgcaattatatgcgcggatgatccgctataaaaccgcgctgagtgcactccgccagttaaacttaccagaatggcaaacacaggtggcagcaacatcctggtacaaccaggccatgtttataaaagattacctgctgtttaatcatgaaacgccttcttactttactccgtcaacaggaactattgcacatatgcaggtagataacctgcagcaggtggcagtagccagctaagaaaaagctgctttttgcagcaatataaaaaaacaaacttccgggagcaggcaagcctgttcccggaaaaaccatgctcgatataaccctcaccaatacacgaaaaagtacaataccatactttttatttaacttactttttctaacaggcattactatgcaatattctgcagcccattggcgtgaacaactaaaactgcaatctcatgttgaaggcggcgcattccgcgaaacttaccggtcggagtgggtactcgacatgaaaaccctgcctgccggcatgagtggtaaccgcaatgcatctacctgcatttatttcttactggaagaaggagagttttctgcattccatcgtatcgcagccgatgaaatctggcatttttatgatggcagcacattgactatctacgagatcgttcccggtggagaactgctgatacataagcttggacgcgatattcaaaacaatgaaagcttgcaggtgatcatcaccgcgggcaactggtttgcttcccgcgtggaagtgcccggcggatacgcccttgccggctgcaccgtagcgcccggctttgattttgcagattttgaactggctgaaaaagcgccgttgcaggcggcttaccccgaacatgcagcgctgatcgacagtcttaccaggtaacggtaacggctatccgctgcaggctccttacttttcactaaatttaggtatgaaaaaagccctttatctcgttgtatttatattattcgcgctcctgatcttttggctgggcaagcgttttggcagtaccaatgtgagccagcaggtaatttccaacagcactattgtaaaagaaattgcagaactggccagcctggatgtacagggaagcgccagtatcaaaaggagtaatattgaaaacagcggcgactggactgataacctgaagaaagcatttcttgaaaatacagtatgggtaactattccgtaccaggccaaatacggcgtaaacatcgacgataagttgtttaaagtgcaaatgactgataagaagatcattatcagtttaccggcgccccgtttgctcagctatgaactgaaaatggaccggatggaaacctcgaaccgtaaaggctggctccagttccaggatgacgaaacctataccgatgttcagaaaagtctctatcgtacctcccgtgcccagctggaaaataaccccacttacatccagcaatccaaagagaaaatacagaaggtaatggagcagtactatgctccattcctgaaggaccacaccctggaaatccggtacgacggcgaaaccagtgcaccggctttaaactaaccgctacgccgcttcctgagcaatatattttaccaggcttcttttggcgatgggcagcaaagtttcatctaccggcaccaccaatggcgtttccacgcaatacaccgcagggttgggtaaattattccgttcccgtatcagcatgcctttaatatgattgatggtatgcaccaggtcttttttataggcctgaaggtattgagtatgaataccccggtatttctcgtcatgtctttcaaaaatagtaagccggtaagtgtataccagcgtttgccggccacgaccgtcgcacaacagcaggtacccttcggctgtttccagcggcacaagccccaccgggaaaatactgagatgttccgccacgtattcgtaaatctccgttccttccttaatagtgctgtttaactgtggcagggaataatggatgatggactccagttcttccatcagttcatcatcggcaatcaattgctcgtacaatagctccagcttctggatgttcactgcggtaagcctttttggaaactgctgctgtaaaaactgtttgttgtcccggaacgctatcaggttgttgtaatgaaagatgatgtctgacaactgcgggtacagcctgctctgggtaaagtgttgattaatgtcctgtaaataagccaatagcgtgtactttttgagctcaaagtctatgtaaccatcggcaaaccatgtttcacttaacgctcccatatgaatttaatttaatggatcatgtactgaatttacgaaaaaaaaaccgtaaaaaggagcgtttataggggtcagagcactattttaaataatatttccatgccagtcaaacaaagtactgcaaaggatctggctatgtcaagtggtagtaaaaaagaaggtaattacaaaaatattttaacgctaacttttttattagcgtaattttcataacttcagtatattatttttcatttttttaatttcagttatcatgaacatttacgtagccaacctgcactataggttgaacgatgaggatctccatcagattttcagcgattttggagaggttacctccgctaaggttatcaaagaccacgaaacaggccgctcacgtggttttggctttgtggaaatgcctaatcaagaagaaggagcaaaggctatggatagtttgaacggcagcgaaatcgaaggtaagcaattgatggtaaacgaagcaagacctaaacaaccgaataataatttcaaaggtggcggtggtaataaccgtggcggcggaggatatggttcccgcgaccgtcgttattaataatcccctttattcggcactaaggaactaaaaagagacgctttttcgggcgtctctttttttgtggctgttaaaagacaaaaaatgcagcagaaaaagattcctgctgcattcctgctaatacaatagctatcttaaattcctctcttcggatcaaaattctccagttccttcgctactgcgctcaggaaagtagaacccagggagccgtctacaatgcgatggtcgtaagacatcgacaggtacatcatgtgcctgatgccaatggtatcaccgtcttccgtttcaataaccaccgggcgtttcttgatggcgcccactgccaggatggccacctgcggctgattaataatgggcgtacccatcaggctgccaaaggtacctacattggtaagcgtgaaagtaccgctctgggtatcttccggcttcagcttattctggcgggcagaattggccatatagtttacctgtttggttaacccggtgaggttcagcatatctgcattcttgatcaccggaacaatcaggttaccacttggcaatgcggtagccatacctatgttgatgtctttcttgataataatcttatcgccgtcgagcgagcagttgatcagcgggaaacgcttgatacacttcacaatggcttctataaacagcggcgtgaaagtcagtttttcaccttcacgtttttcgaaatccccttttacacgatcgcgccacttcaccatgttggtcacatcggcctctgcaaagctggtcacatgcggactggtttgtttgctcattaccatgtggttggcaatcagtttacgcatacgatccatttcaataatttccacattaccgctataggttggggaagccacggtagtggtcaccaccggctgacgggtactggccgctgctgttgaggttgccggttccggcgttacatccggaatcacctttccttcgcggcggtcggctacgtattgaaggatatctcttttggttacgcggccatcgttgccggaaccggggattttttccaggtcggaaaagctgatgccttcctgttgtgcaatggtaagtaccagcggggagtagaatttggctccgccaccggaaacaggcgcttcggcagcaggtgtatatgccggcgctgtagtgaattttggttctgtggctgcaggtgcagcaggcgtaacaggtgtggaaaccgctgctgcatcggcattggtattaatgcgggcaatgactgtacctaccggcaccacatcattttcattgaagagcagttctgtgatttcgccttccgcggtggaaggaacttcgctgtccactttgtcggtggcaatttcaagtacggtttcatctactgttacgtgatcgcccgcctttttatgccaacgcaaaatggtggcttccatgatgctctcccccatttttggcattaccaattctacaatggccataagattgatttttgctttagtgcgcaacaaaaataagggaattgtaccaattcaaaatacgtgaatatccctattccagaatgagtttgcgcaactcattcatggcgtagacagctgtcatttgcgtattccgttcccggtcgtaacgcagctggtgttttatggtgacttttctcttttcatttcctaccgctatccaaacggtgcccaccggtttttccggcgtaccgccatcaggtcccatgatcccggatacggcaatggcataatcagtttgcagcagtgccaaagcgccggtcagcatttcaagcacagtgacctcactcacggcgccatgcgcctgcagggttgccggattcacgcctaacatctttactttcatttcattggcatacgttaccgcactgcctttgaaataagcagaactacccggaacagcagtaatccagctggcaatcagtccgccggtacagctttccgcggtacccatggttttccctttctcctttaacaggttaccgagtacttcgcctatagaaatatcctggtctgttaccgtgatatctgccagcaggtctttcagctggtgaaacaggatgctcacttctgccgccactgataatttatctttcccaaaaccggttaaccggagtttcagcaggctgtaactgggcaggtaagccagtttgatgtgggcaggcagctttgcttcaaaagcaaccagccgttcggcgataaaagattcgcccataccggaggtaaccagcgtttgatgtactactgccggggttttgaaatggctggtcagccggggcagcacgtaatcttccatgatccccttcatttcatgcggcactccgggcatggatacatagatcttgccttctttctcaaaccacattcccggcgcggtgcctctcttattttcaataaccgtggccgtttccggtaccaggctctggtccaggttcctttgcaggatgggcagccccctgctttcaaaaatatgcagtacgttatccagcgtttcctggtgctgtaccagcctggtattgaagtattcacacaaggtgggcttggtgatatcatcggctgtgggtcccagcccgccggtgatcagcacaatatccgacaccgccgattcttttgccagggcgtccaggatatcatccctgatatcgccaatggctacacgccggtgtacccatatgcccattgcattcagttgctgcgccatccaggcagaattggtatcaatcgtttggcctatcaacagttcatctccgatggtgatgatgctggtggtgattttatccataatgcgttgtttatactgctattcaaaaaacggtgccagtattttctgcagctcttccggcaggccggctttctgcttcgttttcacgtcaatgaataccagtgtggtcactccaacattcagcaattcattcttttcgttatacaactcactgtgaaactgtatcttagaacccttcggcatctccttcagtatagtcttcaccgttatcaggtcgtcgtaataggcgggccgcaggtatttcacattcagttcggctaccggcataatcacgccccgttcttccagctgcctatagctgaaacccagttcacgtatggcttctgccctgcctacttcgtaatacagcccgtaattgccataatacaggtatcccatctggtctgtttccccataacgcaccctgattgttgttgtactgataaacatggttccccgctatttttatcctaaacgtttacttgaaaattttatttgcctaatgcgccatccagtgaaaacctgcccggtcccgtgaaaagcagcgttacaaatgctgccaggaaaagaatcggcatttctttttctgataccgggtcgtggccgtgaatcataaaaatgatcactcccatacaaatgaccaatggcacagaagccagtctggttaacagtcccatgatcagcaacaccgcgcagaacacttctgcaaaaaccaccattcccaaagaaattttatgtcctactcccaatggatcaggaaaagaattcattttggcagtaaaattgatcagcttgggccagccatgcaggagtatcagaccaccggatatcacccggagcaccagcatggagaaacttacagcgccattcgagtagccggcagagaacagttttctcatagtaggtaaggtttttgttcttaaaattattttccgcaagataaatgaatagcttttgccttgctaccggagttatccacattgttagaaacacaatcggaaaggaaaagatataacttttatatttgctgataccacctggttcgtttctcatcatgaacgccggcggcactcaggcatcaaagaaacggactaccagggtcaggccacgacagagtacttccccggctggaaaatatttcctcccgggattcgttttaaacgcatattcaagaaataacagctatagcatgcaatttataagaagagtttttgttcccggacatctgtacatatcactcctggcctttacgggtacaggtttgatagggctgcctgccgcacaggcacagcaaacacgcatttatacagatccggaaaaagtgttcaaggacgcccagcaatatttccagcaggaaaaatatgccgtgtccatgcagcttttcaagcaaacccttgataacatcgactatttccacgaaaccaaccgagacctggttaaaacagatgcgtactactattataccatctgcgcactgaaactgcaacaggacaatgcggaaaaacaggcgcaggaattcctgaaactggccaataacaatgcccgggaagaactggtgagctatcaactggcaaaatattatttccgtcagaataaactcaaagaggccattcccctctacgagaaagccaatatcgaaaacctctccaacgcagaaattgcagaagcaaaatttgaactggcctattgctattttaatttaaaagattttaaaaaggcacagcccctgtttgcctccatcaaagaagtaccgggcaaatacagcattcctgctaattattactatggtttcatcagctactataaccaccagtatgcagaagcactcaatagtttccagaaagtagtgaacgaaccgaaatacagcaacgtagtgccttattacatcgctgaaatttattacttccagggaaaaacagatcagctgatcgcctacaccgagccactgctgaggcaaggcggacaatactacgaagcagagctgaaacagttactcggtaaagcctacttcgaaaaaaagaactatccgaaagcattgccctacctgcaggatttccaggataatgcagatgacgtgagaaacgaagatatctaccagttatcatacgcttattaccagacgaataacctctcaaaagcgatcgccggatttaaacaactgagcagctccaaagattcacttggacaaaattccatgtacctcctgggcgactgctacctccgcaccggtcagaaagccaatgcacgcaatgcttttgccttttgcgccaacaacagctccaacgcacagcaacaggaaatttccaggttcaactacggtaaattatcgtacgaactgggctaccccgatgcggcgctcagcgaactcacacagtttgtaaaaacatacccgcaatctgcttataacaaagaagcccgggaaatactcgttaatcttttcatgaacagcaataactacaaagacggtttagcgaccattgaatcgattcgcgataaaaaccccacggtgctgaaagcttaccagaaagtagcctacggccgcgccactcagctgatcaacgaccagcaactggcagaagccgaccgcctgctggatgtggccatcagcaacccctacgatccacagatcaaacaactcgcccatttctggaaagcagaaattgcccttcgtcagaataaaacagaccaggcggttactaacctgaacgcctatctgaataatacggccccggtgtccggtgaagctaacgcacaaaccgccagctacaacctgggatacagcctcctgaaacaggacaaattcacggaagcactgccttactttgaatccgcccagcgcaccagcggccctaacgcagaacgcattgccaccgacgccgccctacgcagcgccgattgttattatatgcttcgccagttcccgaaggcactggcgctgtacgaccgcatcatcagcaacaacgctcccggcgctgattacgccacctaccaaaaagccgtgatcctcggcctacagggcaagcaaggcgagaaacttgcactgctcaaacaactgggtaacaagtttccatcgtccggctttaataacgaaacagatattgagatagccaatacctatctctcggaagaaaaatatacagaagccattcctttcctggaaaatgttttacagaaacaacccaacggaccgaatgcaccacgcgcactcctgaaactgggtttgagctactacaataaagataacgacagtaaagcgctggcctattaccgccaggtagtggagaaattccctaactcgccggaatccaatgaagccctgcaaagtatgaagtcgatttatgttagccagggcaaaaccgacgactacctcgccttcctgaaagccagcggcagaaccgttaccgcttctgctgaagactccctggcctatgctgctgctgaagcccgcttcaccagcaacgattgtacaggcgccaccagcggcttcaacaactatatccagaaatatccgaacggacaatttatcctgccggcctacttctataaagcagaatgcgcttataacagcaaagactatacgagcgcattgcctgcctacgaatttgtattatcccgcaacaacagtttatatgcagaaagatctgcgctacaggcggctaacatcaatttctaccaggtaaaaaattacgataaggcaagaggctactacctgcaactgcaggacctcgctaccagcaaagaaaacagtcttactgccaccaggggactacttcgcagcaactaccagctgaaacgttgggacgaagtaaccaactattcagaaatgttactggctgccgccaatatcagcacggatgatcagatcatcgctcacttctatcatggtaaagcattgcagcaggcaaaagattatgccgccgccctgtcggagttcaaaacagttgccggcatgaccaaatctgaaacaggcgccgaagcccgctacaacattgcggattgctacctgcaacagaatgaactggatgctgctgaaaaagccggttttgatgtgattaaaaatacgccgtcctatgaatactgggtggctaaatcatatatcctgctgggagatgtatacgcccgccaacaggattatttcaatgcaaaagctacttaccagagcatcgttaccaacagctctattcctgagctgaaacaggaagcgaaagataaactggccaaagcggaagcagaagaaaaagcagccggtaaaaaaccgaagaaataatcacccggattctggaatctgacattaagcgcaacaaagcatgaacattcaagcaatatataacaaacgaacttttatcatatcagcactggggctgacgggaatgctgttttcacagaaagcagccgcgcaggaggtattgaaacaggaaacgattgatatcatttccaccaaccaacccaaactgcgcgacgcctacaaactcaatctcacagcttctttgccgggtatcgataccactcgtccttccatgaagtacgagataccggcgctgaacctgaactttatgtaccaggccatgccgctcaaaccgttggcactgggtaaagattcattgtcgtacctgcagaacaacttcgtgaaactcggatatggcaattataaaacaccctatgtgcaggctggcttcggcagcggccggcaggatatgtacaactacggtttgtacgtaaactacaccggctccaaaggcaaggaaattcctgaccaggattatagtaacctcaatgtactggctgcgggcacctacctgttgtcaaagttccggttcgacggaagcatcgggtacgaccgtaataccgttcactactatggctatggtcacgatacggccagctataaaaagaaggatatcgagcaaacgtttaaccagatcaccgcttcggtaggcatgcagaacaggccgcaaaacgactgggcatttaccttccagccaaaagtgaagtttattcttttcaacgactcctacaagcgtacagaaaataccttccagctgaatgtacccgtacgtaagcaggtgtttgaagatatctacataaaagtagaaggtgtatttgatctttctacctataaagaagataacaaccgcgccatcaacaacaacatcgcttctatccaccctgcggtggatatcatgaaaccggggtttgtgctgcatgccggcgtaaatccaacgtggagcaacggcgagttttacctgctgcccgacatcgtgaatgagtcgcacctgatccgtaaaaaactgatcctgagcagtggatggatttcctattttgaaaagaattcctatcgcaacctcgccaataaaaatccgttcctcgccggcttaccgggagaaatgatgaatacccgtgtagaagaaaaatataccggtatcaaaggtacgctgggcagccatttcaactataacactaaattcgcttctgttacctggtacaatatgccgctgtttgtaaacgacagcgccgataccaagaaattcaccacccgtaacgaagcccagctgcgcgctttccagctgcatggtgaagtaggctatattgaagaagaaaaattccaggcccgcgtaagcttcgactggtataattataacaaacaggaaacggaagtgcaaccatggcacctgcccgctttccagggcgatttgtttgcacaatacaccatcgccaaaaaattacacctgaatgccgacctctttgcattgagcggcagctattacctgctccccaacaaagactttggcaaaaccaaaggcgcatgggacctgaatgcaggcgcatcctatgatatcagcaaaaatttcggactgtgggtgaatgcaaataacctgttcaatacgcactaccagcggtattatctttaccctacttatgggttcaatattgtgggtggtgtgatgattaagttttaactttatacgcggattttgtcttgctcaggattacgttgattatattgattaccaggatttgaacttttttgattttataaaggattttcgaagatataagtggatatactcgcatatatccccaaaaatcaaaaaaaatcaaaaaagttcaaatcctggtaatcagtataatcagcgtaatcagcgagaaagacaaaatccgcagcattattcactaaaaattgctccacttgatacttcagcaatatatccaggaagtgctgtttaaacagcggatttgtgtagtaccacagctgggaacattttctgtacaacattttccggcgcattataacgaccacgcccaaacgcttacggcgccacgtgagcaggtgatgtttacccaacaatggcaggacgacggttcctgtgtggaatggatagcccttaaggaaaacctggtgccggcagtagcacagcggaagctggaaaaatacctggaagagctgaaagcagaacttcaatccgggaagccactggtattaccgggtattggtcagttgcagggcgactttaccggcaacattcacttccatgcagaggagctgccggtagaaaaagaaacactggatattaagccgatagaacgcacaacagatagccgctctgcgccggcatttgttccaccgccacctatagaggcgctggagcctgttatgacagaagaggtagaagacacgttagaagccgtaacagaagaaagtggttttaaatggtggtgggcagctattcccattgccgctattgtaattggattagccgcctggtggtatttatcgggtgtttcaaaaccagtagctgaatccgaaactcccgctgatacggaagtcaacgcgcaacagctcgccgccgctgctgcggattccatacaaaaggtcctggccgactccacagcaaaagctgcgattacgcccattacctattatgcagtggtggaaagatacaaagacagcagcatcgctgtaaaaaaacaaaagcaacaactcgcgtggggaaaaacgctggttctttataaaagggacagcatgtacagaactgcggtggaattgcgctcactggcagcagataccaccgtgcaaagggatagcatccgcaaaatatttggcaataaagtatttcttgaattttagctgttacgcttttatttcagcggctacaatttccagcccctccgcaaaagtacggggctgataacccagttctttggctgccttatctattatcagcccggttttggcaggacgggccgccggttgtgccagtgttttggcactgattttttctacgagggaagtatccagtttaaagtattcagccgtttgaatggccatatcatagggagtgagaatttcatttccggagatgttgaagaaaccgtttgctttcttatctgcaatcagcaaacaacccttcgccaggtcgtggcataaggtaggtgtacgccattggtcatccaccactttcacttttttaccctgctgcaaattattttttacccaggtaatcatattattgcgatgcgggtctgctaccacgccatacaccagtacagtgcggacaatggcccacttcagtttgctattgatcaccagtcgctctgcagctactttactggtaccataataattaataggatttacggtagcgtcttcactgtaaggtccctgtaagccatcgaatacaaaatcggtagacaggaaaatgaagaaggcgttgcaactttctgccgcgtgtaccaggtaacgggtggctcctacattggtatcccagcaggcatctttatttttttcgcagtcatctacctgcgacatggcgccgccatgaataatgatatccggctgatgtttttccaccagctgctttacgctgccggcatcgcggaggttcaccgcctcataagtgtatttatcccgcagggggaaacgattagggcctctgcctgtggctatcacatcatattttccatcttgcagaaaaagcgggatcagatgttgtcccaataatccgttactaccagttataagtaccttcataaagccatgttcaatacgctatttctaaagataagaaaaaaaagcttttagctgttcaccaaaatgaggcatttcgataacagctaaaagctaatcacccgcaactttacttgtgcatgcccaggttatacatggtgaacgcccagatatcagcggcttcatcaatcatcttggaagtgggtttgccggctccgtgacctgcctgtgtttcaatacggatcagggtcgggtttggcccggcgttgtctgcctgcagtgtagctgcaaacttaaacgaatgcgccggtaccacacggtcgtcgtgatccgcagtggtgatcagtgtagccgggtaagcggtacctggcttcaggttatgcaacggtgaatatttcagcaggtatttaaactgttctgcatgatcgctgctaccgtattccactgcccaggcccaacctatggtaaatttctgaaagcgcagcatgtccattacgcctacagcgggcagtgccaccttaaacagttccggacgctgcgtcatacaggcgcctaccagtaaaccaccgttggaaccgccgcggatcgctatcttgccgggattggtgtatttcgctttcaccaggtattcagctgcaccgataaaatcgttgaatacattttgtttcttttccatcatacctgctttgtgccaggcttcaccgtattcgctgccacctctcagtgatactacggcgtatatgcctccctgttccatgaagtataggttggaaacgctgaaagagggcgtcatggcaatattaaatccgccgtagccatagagcaacacggggttattaccattcagccggatccctttcttgtaggaaaggaatatgggaacactttctccatcggcacttttaaagaatacctgtttggtttcgtattccgcagggttgaattttacttctgccttattatataaggtagaaacgccggtagccacatcatatttatatacagcaggcggcgtaacaaaggaagtataagtataaaagaattccttgtcttctttcttgctgccaaatccaccagcggttccgaggccaggcagtttcacttcatgttccagcttacctttataatcatactggtaaaccctggtagaagcgtctttcagataggaaaggaataatttgccgccggcaaggcccactccctggagggcttctttcttttccggaacaattactttccagttggcttcccctggattggcggggtctatcagcacaattttatagttgggtgcgttatgattggtgcgcaccagcaatttatccccatcgttatctattacgtctggttcgttagcgaagccttttaccagcagggtgaattctttttgtgcggggttttgcaggtcgcggtaccagagttcccggccggaagtaccttccgaggtagagaggatcaggaaacgctcatcttctgttacgtctacgccggcgttgcgcagcgggtgttctttatccacatggatcaattcatccttctcctgcggatcgcccaggcggtggtagtatactttctggaattcattcttttgggatagtttgttttgttcatcgggtttgtcgtagcggctgtaatagaagccatcacctttccacgacaggccactgaactttacccattccagtttatccggcaggagctgccgtgtttccacgtttatcacataaccttcctgccagtcggatcctgctttggaaagcaggtaggcaaaatatttcccgtcttttgaaaacgacatgctgcccagtgcggtagtaccggctgctgacagtttgttgggatccaggaaaacttccggggtaccgcctaaagtggcagaacggtaaagaacggactggttctgcagaccatcatttttaaagaagtaataatagttaccgtgtttagcgggggcgccgtttttggggtaattccacaattcttccagtcttttgcggatttctgcgcggaaagggatgttggagagatagttttctgttaccttattctgggcgtccacccatgcttttgtttcggggctgtgatcgtcttccagccaccggtaaggatctgcgatcggggtaccgtgatagttatctatggtatccacttttttggattcgggataagtaatcgtttgctgctgctgcgctattgcctgcccggcgattaaacttacgctcataaagatccacctcctattattttttttcgacatgcgtaatattttttaaaaaatttatctactttgtttgatggaaattaaaaatttaggttatttcatcagataacagttagaaaacaattgcaaaatgttatttttgtgcgcctttaagatatttttttagcaatttatatgaaaaaactgaacaacattgcagtccttacatcggggggagatgctcccgggatgaacgccgccgttcgtgccgttgtaagaacgggcatttatcatcagctgaatgtgtatggcattatgtacggctataggggaatgttgaagaacgagatcttcccaatggagtcaaaatccgttgccaacattattcagcgcggaggcaccatattgaagaccgcccggtgcaaagagttctatgaatatgaagggcgaaaaatggcttatgaaaatctgaaaaaacacaacattgacgggctggtagtaattggtggagacggctcgtttaatggtgcgcaaaagttcagccaggaatttgatattccgtgtataggcttgcctggtactattgacaaggacattgcaggaactgattctacgattggatttgatacagctgtgaatacagcggtggaagctatcgacaaaatcagggacactgccgatgcgcatgaccgtttgtttgtaatcgaggtaatgggccgtgatgccggttatattgcgttacacagcggcatttccactggtgcggagcacatattgctgcctgagcgcaaaaccgaagtaaatgacattattgaagaactgcaggcgaacgaacgccgcagaaaactggttaacctgatcgttgtagccgaaggcgatgaaaccggcggcgctactgaagttggtcgtatcattaaagaaaggtgcccacaactggatacccgggttagtatcctcggacacatccagcgtggcggcgctcccacctgcacagatcgtattctggccagccgtctgggctatgcagccgtagatgcccttctcgaaggcatccacaatgtaatggtcggtgttgtcaacgacaagatccattacactcctcttgataaagctgtaaaagccaaacaggaaattgaccccgaatggtttaagattgttaaaattcttgcgagttaaaaaattagacttatgagtacaaaggatctttcgaaatactatcacaagcagatggataacgctgcgggtagagaacactcttcgcacaaaacaaaaatcgtggctactgtaggcccggcatgcgatacctatgaaggcctgctgacactggtaaaggccggcgttaacgttttccgcctcaacttttcacacggctcgcacgaagataaactgcggattattgaatacatccgccagatcaataaaacagaaccttacaccgtagccatactggccgatttacagggaccaaaacttcgtgtgggtgaaatcgaaaacaatgcactcccgctgaagaaaggtgatatcctcactttcgtaaacgaaaagctggtgggcaacatggaaaaaatttacgtttcctaccctgacctgtacaaagatcttagagttggccagaaaattctgctggacgacggcaaaatcgagacaattgtaaaagaaattactgccagcggtgaaatcaaagcggaagtatccctgccaggtgtactgtcttccaaaaaaggctttaacctcccggataccaaaatctccctccctgcgctgacagataaagatattattgacctggaattcatcatcgaccacgaatgcgactgggtagcgctctcctttgtaagaagcgtaaaagacctggccgtattacgcaaacgcctggaggcacgtaattctaaaatgaaggtgatctctaaaattgagaagcctgaagcgatacagaacctgaaagaaattatctgggaaagtgatggcgtgatgattgcccgtggtgatctcggtgtggaactgccggtagagcagatcccgatgatccagaaagatatcatccgcaagtgtattcaccgtgcaaaacccgtaattgtggctacacaaatgatggaaagcatgatggatcgcacccgtccgaaccgtagtgaaatcaccgacgtagccaacgcagtactggaaggtgctgatgcggtaatgctgagcggcgaaactgctaccggtatgttcccggaactggttatccaaaccatgaataaaattatccaggaagtggaaaaagaagcgatcatttacaaccgtaacctgatccctcatcgccactctcctaccttcctcagcgatgcactgtgctataacgcctgtaaaattgcggaagacctggacgctgatgccctcattggtatgacccagagcggttacaccggctttatgctgagtagctaccgcccacgcagcccgctctacatcttcaccaaagaaaggtcgctggtaaaccagctgagcctgagctggggtgtacgcgccttctactacgaagaagaagaaagcctggatgatatcgtattcgatcagatcaatatcctgaaagaaagaggattcatcaaatcaggagatgtagccgttaacaccggtagcacccctgtcaaagaacacctgcccacaaacatgctgaagatcacgaaagtggactaattgctataaggatttagtaagcggcggagaggaagttccttttcgccgcttttttgtcaataatatatacagacttgtctgtttaataaatttagcctaatattgccttatgaaagaacaaggcgcaaaagaaagaatcttaaatacagccagcgaattgttttacaagcaaggctaccaggcaaccggtattaaccagatcatagaagaagcggggattgccaaagcaagcctgtaccagcactttccatccaaggaagctttgctgacggaatatctactgcgaacccggacctacaaccacgccgagcggatggcttatattgaccagcttgcgcctggcagggaaaagctcatgggcctgttcgaataccgccgccgccacatggaaaaaaacaatttcaggggttgcgcctttgtccgcatcgcctatgaactgccaggattgaatgaggacgcacttttacaggtacggacgcatacccaaacgctgaaaacatttatcgccgaacaattacaaatcataaaacacccttaccccgcagcggaacttgaagaaatgaccggcatgctgttgaatctgtatgaaggcgcggggcttcagggctatatccaacggtccgcaaaaccggtagaagacacgaagaaagtggttgccaggttgctggatacactttgaagctgatagattgaggaattgcgaccaaagggaaacacatctttataaataccggcgaatgccggataaacaaaactaaataccagcaacactgccggaatatcaccagcaaggctggtaaaaagtgccgtaaaacattaaagttttcgcggcgtatttccatcaattatttagtgcatccaataacgttatctattataaaaaatttactctcatgaaaacagaccagtctgtatatattaaaccaaccactgtcaatccatggatatcgctggcaattatcctgctggcgccacttatcactgtgatcgatgtatttattgtaaacatcagcacaccggccattaaagcgtatttccatagttccgacgcagcactggaactggtgattgccagctatctcctgggttacgccgtgtttctcatcaccggcagccgcacaggtgattacctgggcaaaaagaaagtgtttatatccgggctcgccgcattcaccctcacctcggccatgtgcggctttgccacttccatggaaatgttgattgtgtccaggctgttacaaggcgtggcagcagccttcaccgtaccgcaaaccatcacgctgatacaactgaacttccagtcgcccgcagaccgtgataaagcctatggcctctatggcatggccctcggcaccggcgctaccctggggcagttcctcggcggctacttcattacctcgcacctgatcaccgacagctggcggctgatcttcctcgtcaatctcccgtttggtattgtagcgatgctgctggcctggttctttgtgcaggaatccggtcaaaacaaaagcacccggtttgatataccaggcatcatcctgctcaccttagccttatctctcctgatatatcctgttatacagggtgcagaacttggctggcctgcctggactatcaccatgctggcaggtgcattcatattattaggcgtattcgtgtggtatcaacactggctgggaaaacggcaacgcgatccgttagtaccgctggaactctttcgtatccggagttttaacaccggtgtcatcagcgtattattcttctttggtgtaaacaccgcttatatttttattgtagccatctactttcagaatggatttcatatgtcgccttttacagcggggaattatttcgtcatgcaaaccattcctttcctgctggcttctttgtggtcaattaaaaatgcagcacgatacggtatccgcctgctacagtttgcgtgtatactaatgatcctctcttttatcttacaattagttttatttcagggagatgtagtaacaccttacgatatcatgccgtgtttaattatttatggcagcggatctggtttgctgatgccatcattattaaaagtggcgatgtgggatatgccgccggctaaagcaggagccgccagcggcgtgtattctacggtacagcagttcgcctctgcactgggtgtaagcatgcttggaggtatttttctctacctcgcacggcactccggcaatttttatctcgcttataaaattgcgttgttctgcatgatgggttatttagtaatagtgatgatcgtgctaaaccgggttaagcggtaactgctctttttgttttcttataagtacccaggtaaataaccagggcagcggtaatcagcgcagtaccggccacgcatataccattccattgtgcaaaagaccatacccatagcccgatgccggagccaagtgaagtgccaataaaactggtagtcataaacaccgtattcaaacggttccttgcttccggcaataatgtgtagatgcgggtttggttggatacatggataccctgtaaaccaagatcaatagcgatgatcccaacgatgatacctataatattggctttaaaaacataaaagagaaaataaccgaggaacaaaaagatgataccataaccaatggcaatgcgcggattctttttatctgcaatgcgtcccaccagtggggcgcctaaagcgccggcagccgcagcaagtcccatcaacccgatttgttcactggtatatttaaaaggcgcatcagacaataaaaataccacggttgtccagaacatgccaaacatagcgaaacaacaggcattgatagccgaagcttctcttaataaaggctgttctttgatcagcgtaagcaatgatttcatcaggtcgccgtagcttcctttgaaatttggtttactggatggaaaagatgtaatcatgatcaccgccagcaaagcgctgatacacgcggctatccagaacatggcacgccatccgaaatgatgtcctactacaccgctgagggtgcgggataataagatgccgacgagtaagccactcataatagtaccaatcactttcccccggcttgcaggatcagaaaggcctgctgccagtggcaatatcagctgcggcactaccgaagtaaaaccaatcagcaaaccggtaattttcagcatagtgatatttaccgactctgcagccgccaccagggccactaccgcagccagtgtcatcaccactatctgccgcttgcgctctagtttgtcacccaacggcacacaaaataacaggcccagcgcgtagcccacctgcgtaaaaaatgtgacctgtccggcattactttccgatacgccaaattcgttgctcatcaacaccagcaaaggctggctgtaataaatattggcaacgatcaaccccgtgcaaagggccattatcatgatattccacctgctaagcgccataaaattgtactgttttttccgggagatgcaaagatagccttttcgtgtttagtagttgccctttagcttttaagacgggcttttaacggaaaaaggtaaatttgtcggactattcactaacagctaaatgctaaccgctaaaagctacccgtatgtttacaagcattaatccgtttacgcaggaaaccattgctgaatatgcagcacatacaccggaacaaatagagcagaaattacagctgggccataaagcataccgggaattattacaagtttccctggaacaacgccggcagtggatgatgcaggttgcacaatccatgaaagacaatgcagatgaacatgccgcgctgatcacgcgggaaatgggaaaaacgctgaaagaagcacgggccgaagtgctgaaatgcgctacctccgcagaatattatgcagaaaacatcgtggaaatgctggcacataaaccgatcggttccgatgcgtataaaagttacgtatcgtacgaaccaaaaggaattatactggcaatcatgccctggaacttcccctactggcaggtattccgctttgctattcccaatatactcgccggcaacaccggcatcctgaaacatgccagcaatgtaagcggttgtgcactggccatcgaaaaaatattcactgaaagtagttttcccgccggtactttccagtcgttactcatctcttccaaagatatagaacctgttatcgcagatcaccgcgtacagggcgttacactcaccggcagtacccccgcaggtaaaagtgtagcggcgcttgccgggaaatatatcaagaaaaccgtgctggaactgggtggcagtgatccttttattgtattgaaagatgccgacctggaagccgccgctaaaacagcagtacaaggtcgtatgcaaaacgccggtcagtcgtgcattgccgcaaaacgctggatcgtagaaaaagatattgttcccgcgtttaccgcagctgtaaaacggatcctgcacgatctcaaacagggagatcccacgcaggaaagcacacaaatgggcccaatggcccgccccgacctggcagaggagctggccaaacaattacaggactctattcgccagggggctaagctggagttgggtggcacgcatgaaggctgtaactttgcacctaccctgcttaccggggtaaccaataaaatgacggctttcaaagaagaaacttttggtccgctcgccgtgatcatagaagcagccgacgaaacggatgctatcgcactggccaatgaaacagaatttggcctgggcgcagccctgtggaccagcgatctcgacaaagccgccaaactggccacacagatagaaagtggcaatgtatttattaatgcgatggttcgctctgatgcacgcttacctttcggcggcgtaaagcaatccggctatggaagggaactatcactggaaggcacacacgaatttctgaatgtaaagactgtctatatacaacaataaagcactggaatgaccacctctctgaaacgcgaccgctatactccctatatcagtttctcccgtaaagaatgggcagaaagaagcaatgatgccatgctgcaattacaggattacgacctggaagcgctgcacggcatgaatgaaccactcacacaggaagaaataacacaggtatatcttccgctggcacatctgctcaacttatatgtaaccgcgtcgcaacaactgcatactgctaccagcaatttcctcagcagccaggtacataaagtgccttatattattggcatcgccggaagcgtagccgttgggaaaagtacgaccgccagggtgttacaaaaattattacaggcatggcccaatcatccgcgggtagacctggtaacaacggatggtttcctctatcccaataaagtgctggaggccaataatatcatgaacagaaaaggcttcccggaaagctatgatattaaaagactgatccacttcctggcggatgtaaaatccggtaaggaaaaggtggcggcgccactttattcccacctggaatacgatatcttacccggccagctgcagtggatagagcaaccggacattgtgattgtagaaggcgtgaatgtgttgcaggttcgtcaccggcagcaacaaaaagatccagccgtattcgtatccgatttcttcgacttcagtatttatgtagacgctgcggaaaaagatatccgcaaatggtacatcgctcgctttgaaaccctgcgcagaactgcctttcagagccccgagtcttttttccaccgttatgcacatctttctgatgcggccactatcgagttagccacacagatctgggatgatatcaacaaacctaacctggaacaaaatattgcacctacccgctaccgcgccagcctgatcctggaaaaaggtcatcatcatttcgttcaatccattcaactgagaaagacctgaatgcaaggcacacaaattatccgtcaacagctgcaggcactgctgaaagaacccatggttcactgggaactgtttgaagccatcctgcagccggtaactttccccgcaggcgaccacctgtcggaagcgggtaaaaccgccaatgctatttattatattgaagaaggaattgtgcgggtatataccatccacgatggtaaagacatcagcatggactttgcctttccgcataactttactacttcctacgcctctttcattacacaaaaacccgcggtagtaagtttgcaggcagtaacgcctgtacgtgggtacgcctgttattataccgatctgcaacaattatatcgcacctcgcaccagtcggagaagataggccggctggtagctgaacagcaatacctgcggaaatacaaccgggaactctccttcctgcaatactccgcacaggagcggtatacgcagttgctacaggaatatcccgaagtggtgcagcatatccctgtcaaacaaattgcttcttacctgggaattgaaccggaaagtttaagccggatcaggaagaaaagaagtacataacttgttcttcttacccattaactaacatttgtcaattttattcctccggaagatgtggatctttgagtcctaaaaaatatacaaatggctttcttttccggcttatgcagtattgccctcttactactggcgattggctatatcttccagatccctcttttacaacaactccctgcagatgcccgtatatccgctgccgttatgtttctcctaataggggttacacatttgatgaagccgcgcaaacttacctatatgattgaaggaatgatcccatatcctttattcatggtgttgtttaccggggcgctggaagtattactgggagcgggtttgctgttttctgccacacagtattatgcgggatggggattaatgatactcctggtggctatgtttcctgccaatatccgcgtagcggtgctgaacctgccggcgcctggcggattaccctccaaaccctggtacatctggagccgattattatttcaacctgtttatattttatggatatggtgggccatcaattaattgataactttatgccatgctataaaaaatttaaccatgcgcatacattatttacgcaatgccacattgctcatagaatggaataataagaacatactggttgatcccatgctcggcgttaaagacagcctggaccccgttcccaacgcagccaacagcatccggaatcccatgaccgatcttccgcttaacgacgacgatttaaagcagttgctgtcgtccctggatgccattctcgtcacccacctgcaccgcgaccactgggatgtaactgcacaggccatactgcctaaaagcattcctttattttgtcagccggaagatgaagccactatcagggaacaggcatttacacaggtgattcctgttgttacgtcggttacctgggaaaatatagtcattacacgtactggtggacaacatggcaccggcgaaataggcaaaatgatggcgcctgtttccggctttgtgctgaaagaagggaacactacattatacatcgccggcgatactatctggtgtgaagaagtaacagctgcgctggatactttccgcccggattatgtggtggtgaatgcaggcgctgcacaattcctgcagggagatcccatcaccatgaccgcagcagacgtgattaagaccatccggcacgcttcgcagcccaaggtagtagcagtgcacatgggcgctataaatcactgttttctcagcagggaagcgttgagagcggctgttgctgccgaacagctgtccgccattattcctgaacaaggcgaatggattaatctttcataaaaagatcttttgtacacacaaaaaaaggggctgttaccttccggtaacagccctttctgcataatgtaaggagttttttatacccactcattaacatgttttgcattacccatgctaacttcacgggccgaaatggtaaaggaaattaccattggatttttgttttcgtagtcaaaagactcttcaaactttactaaatacccttctttaaattccagggttttcagtttggaatcagtgtctcttttgtaaaaagtaatggtaccatcttttctttcaaagttgtttaccatccactcaaagagatctgtttttccggtagattcaacggtcagcttaatgcgtccgccacgggtgatggctgaagggcgaccggttgcatctacttcttgtgtgaggtcataagcgacatgctgtacattgtactcgttgccgcctgcttcaaatttggctttgaatgacatgttgggttaatttttaaggttacaataaagaaaaaataattagtatttatttatgaattataagtaccaaatataggatgaaaattttaatagtcaagagtcctaacaaataattattattccaatatttaccggattaatacccttctgaaagttagtgagcgcggctgtttagcaacatcatttgccggcagttatcaaggtccctgctcttgctttccagtttcgcattcaggtcggcgacctgttctttcagacctgcaatattttgttgtgcattttgcagttcgcggagctgctgtttggtttgttgcaacgacaaacagttctgcacaatattatcatacagcccgtaatgcgtcactgcatttttgggaattgagttgcgcatatccgccagggatgcggcaatcacctgatccatgtaattggcgttctggttaggaaggttaatagaatcgaggttatgttttaccttatccagcttttgcaggaactctgattggaacgcctgctcttccctgaatgaagtcaattctttccgcagggatgcgttttccctggcaggtacctggtaattaaagaatacagccaatacaaataaggcgaccgttataatgaaaaataacaggaaccaaataaaggatacatttctttcctgcctgtttaatacttgcatattgcggatcgttttttttagggaaattatcttgttgaatgatcagttaagcggaataaattcctgttgaaacatttagtgttattgcacctggtttgtacgcatcacaaacgtcagaagcgttgggtaatggctgttatattgctgccataacagcatgatactagtcggtaaagaaccagcgcttggttttatgctttcgcaggtattccgcgtcttcctgtgattcttcttttacgaaaatattgctgtcctgcttgcgtccgatataatccaatctgctcaggctttcaaacagtttattcacggcccttacaaaaggaatcatgggctgcaggcactctcttacatccaggtgtttatatttgatgttggcgcagttgatcatgagcgtttcaagttctccctgtcgcagttcgcaccactcagataagtagttcagcagctcctctttacctgcgccggcacgctgatcaatagcgtttttcatggtgcgggcaaggcctgcaataatttccagcatctgggccggtggttgctgtaatcctaaccaccggaattgcgtgatcctggtgccgagatactgcaccattctctccgtgatatacaatacgacaagtgccaggtcattttgctggttcctgccgtagatcttttgcacgatgtgtacgccgtataattccatttgccccaggaactggtccagttcatgaaagagatctatcaatgcaggatgtgcgctgacgatgctgcagggagggatatagtcatcatccatctccggacggccatcggacacactgatgcggcccagcaccatctggtagctgcctagctggccggaaggcagctgcgacgccggcgccacgtataaactatattccggtgtggcataaggcaatcttggtggatcttcatccagcaaaggctctccgctgggctgccggtcaaagggatttacctgtatgatgacgtaataagtagtttctgtatgttgcgggtcccaggtataagttgcttcggggaaggtagtagcatacttcagcgaatgcacggtatgttcagggatctcaatacggccaccaccgggagttaccgcgcggcattcggttaatttgatccgccacaactgctgattatcggtcacaaaccagcaacgcagcgattccttattttctgctttggggggcaacagtccatagttaagcgcatggataccgcatgccaatgcatccctgatctggtccagcaaagcattttccgtatctataaaatgctgcttttttatcttcataccatcaacccagttaacgggaaaatgctttagcggttctgccatagttctgctcttttacgataacataattctgttgcaaataatcacactgttttctttaatgccattcataaacacggccttgtcggggtccagtgttttagcgctgccaaaccaacgtggtttcaggtggaatacccacccatatggctgcccggtgtgatccacaaaatcaatcggggtattgggatagcgatcattataatcattgataaaatgatagaacaggtcgcccagatccatcttgataggtgtacgtgcccggaaataagtacggctgttgtcaagcggacctttttccatttccagtccaatgacaatcaggtctttcatttcatcctcattcacttccggtacctctttatagataggatactgccaccacttgtgcaccttcacaggaatggccatcatcttttcaaaagttttataaacaaaggtgggcagtacaaaggaaaacatgctggtgagcatcgggtaataaagaaacgtgtccttgtccaggaaccggtttaccagtacaaatccggcgccgccaaataaccagatggccagtatgaaagccagttcagataccagggtggtttcattggcccaaaagcgggtatacataaagtggcaatgcactacgcctaatcccaggaaccacacttcgtaaaaaagatattggttcatcaggttctgatgggtaaacaggaagggaatggaactgattacagcaaataccagcgtcatacacactaaatacagcagtgctttctttttataaagactgaaatttttgatgtacctgctgagcagagccactataaaggaccctattgccagggcgccggccagcatgatataaaacttagcggtgtatctcatagttctgttggtatgtcaaggtttttcgggtttgggtactaacatttcagtttttcagatggtcgttaatagcaaaaatgattccatgtaagcttctgccagctgtttttcagagaaaaaaattataccccatcagcccctgctcaggttgcttgtcagacaggattacttttttctctcctgaagacggcaccagcaaggtattaatttccacatctgcaggaaacaggtatccatagcaggtttccagcagcttgccataaggttgccagggcaggtaatcgtatatccgttggcgttttaccgggccaatgctcaccgttaccaccggcatgtccgtataacacgatgtgcctaccatggcgtctaccccaagcatgcattcgcccaggggaacactgcttccggtattaaccatttgcggctgacgttgccaggtgatcgttaccgtttcttccagtacctgttccaggcaaagcttcaccagggtcatattgcctgctatccgatgaacatatggtaacagttttactaacctgttcacggcagcatcaggaagcccgggaggcaactcccagaattcatgaaataactggtctgtgtcctttccgaatacgtcaaacaacaggtgcttttcccgttgttccaagtatacacgttgcaggaaaaactcattttccaggggttgaaaaaagcggcgtgcctgctgttgctgttgctgctgccttttataccgcaccaccatttcggcaacggcattctgcctggaagagggctcctgcttgaattcatgaaacatgccctgcggcagccggtcgtaaataccatcgcgcgaaagggaaaaactaataaacggctgatacggctgactgtcgtccagcttcaccccggtaatatctgttgcaaaagaacgggtaaatacattttgcaactgcaccactatttcttcttcccgcacatgattatcgagtaattcccccaccactacttcggctctgatgtcgtatggtaaagcattgacgtggtcaatcacttcttccagcacggcagccttctgcgcattatttaccatgaggttatatttaggtttctctgattctgctattagcggcaaactgttagcataactatctttcgtctatggttccgggctaacaactcagtaacaaaaatagcggtttgattttattattatgaatattacggcttaaattttgaaccgggaaaaaattttttctacggccattatctttggcaatttatctaaaaaaaacactaaaattgtaaaaacctgaaaaaccgatggccccccgtaaacccgaaaatgaacgcaaggtaaattcattcagaccctttggaaaaattgccagtcatgttgaccccatggtgctgtggaccttcctgggcctgttcctcataagcataatactgctggctttccaactcgatggccgggaagattgcagtaatacagatataaaactcagtcatattcagaatagtaacagtaaagcatacgccgttggagaagtgattacttttaatgccgaaaacgctgataaaaaaaacgcagactattcctgggagttcggcgactccagcgccagggccactggcaggcaggtatatcactctttcaacaaggccggcagctatatgatcacactcacttccggcaaatgcacctggcggaaagaagtactggtgatcatgaacacaccggcagcagccaacagtcagcccgatatcttccccgttattgatggccccgctgaagcatttgcaggcaggccggtgaccttcaccaactccacgccaaccgccaaaaactggacctggcggctgttgcaggataatgcggaaccacatggcggttcatctgttacatataccttctcttcccccggtgaaagaaccctgtcgctgatcatcaacggcgacagcagccatatggtgctaaaacatatcacggtattccctgcaagggcccccgaacaccaggagcagccggaaccggcctttaacccggcgccactgcctgcaccaacaccggaggtaccggtaaagaaagaagagccacgacccaccatctccgatgatgaatttaaatacatgctcacccaggtgaccctgaaacaaaaaacggcgtccgattttgcgcaatacctctgcaataatcttaatgcaagggtggtgctcaataccagcgatgtggataacttcacgcatttctgtcagcggatctatggcaagaagaaattcaagatcgaaagagtaaacctggcaaaagacgagaaaggatgcgtaaaggaaattctcatcatgtacgaccgcaaaaaagtgctgggcatattttaagctgatatcatgaaaggaaaatattatcaattacccatcgacttttcactgctgctgcagaaaaaagacatgccggccatttcgctggaagactctatcgcgcagcatattcacctgctcatcactaccgtattgggcgaaaacaaggatgatgcccaatatggctgccagtggtgggacagcgactttgacatcaaagcttccaataacgaagtaaaggagcagatagaaaatgcggttaaagcatccattacccggtatgaaaaaaggatttcccaaataagggtagtggccgctgtaaaccaggaagaattgttgctgccatctacccgtaaaatgaaaaagaaaatccgggtgacggtttcaggaaacgttaccaaaaacaatcatccgtttcagtacagcagcttcttttatatcagcccgttgtcgtacgattgattacttgtttattaaccgctctcatgaaagaaaaaaaagaaagaataaaagaccgcatgctgaaaacagctgcacggctctggggatacccggatgctgaagtggaaacttcgtttgacccggtagtgcagctgctgctggaagcatgcgccagtgagctggagaaaatttcaggagaagtggatgtttcacacgcccggctggtggaacgcctggcgcagatcatgatgccggaacccattaccagcagccagccggcctatggcattctccatgccattgccacagaaccggtagccgatattcatgccgatcaccagttttatcatcataccaaatcaggcatgcataaccgcgacctgttctttgcgccggtgaccagtcaccgcctgttccgcggacaggtgcaatacatggttattggcaacaagctgtatgaaacccgcgatcactggttcaaggagcagatattacaggggcaaacattccctgatatggccccgaatcatttatggataggcatttcactcgaagatgtaccgcactcctgggaaggtatgtccttcttctttgacctgcgtaatatccatcagcaggaaatgttttatcattatctcccgctggcaaaagtatttagcggcaaccgggagctgatgataaaaggaggctatcaccatagcaggactgtagctgaagaagaaagagataatatgatccaggtagcagtaaataacaactcccgttatagccagcatatcctgcaacgtttccgccgccacttccttaccatcacggatacgcagccacccctcgcttcccgcacaccggaagccctcaccaggattttcgggcaagataccgcccgcttaaataaagaagtacactggttgcgcatcgagtttcccgaagcgctgcatcacacactgctggaagacctgtattgcagcattaactgcttcccggttatcaacaaaaaaaataacgagcagtctatgaaactgaatcgttatctgaatatcattcccctgcaaacaccggatatcttttttgatatcaaacgtgtttacgacctcgaaggaaccgattactatgtacgtaacttctctacagccggacaaatgcaggaaggcgaactggtgatccgcagcagtggcatcgggcgttttgatacccgcgaagccaaagaagtgatcgcttatctcgtggaagtaatccgcgacgaaagctctttattcgaagaagtaaaaaatgattttgttaccaaccgcatgagggaactgcatcagttgattgcctcactggaagaacagctgcaacccggcaacaacaaaggaaatattccttatgtgatggtaaagcccaaagaaaatgcagaatatattttcctggaattttactcaacgaacggcaccgctgctaataatatccgcatgggtacgcgaatgctggaatatggtagtatcaacacccgccccaacagcatcacactgctgagtaatacccagggaggaaaagacaggctgaatatcgatgagaaaattaacctgtaccggtcccatttattgtcgcataaccgtgtggttacccccgaagatatcaaagcgctttgccgtactatttttggaaaggaaatgaaatcggccgctgttgttaaggggatggccctgcaacccggtatgaatgcgggttacagccgtacgctggatatccgtatttcattgctccatcaaaccgaacgttatcccgccgccaatttgcaatacatgaaagaggaattgcttttgcaactggaagaaaaatccagcaatacgttcccgttccgcgtgtttattaatgaagtgttgatgtaagtgcatcaaccggtgcgggtaatgcagaaatagcgctccggttatcggttcttccacgcaactgcacatctccgccggttttcagcaaatcggcaggcactccttttttaccatctgcggcgtataataccactgcattctcaaaaccaaggtccacataaatccggctacccaccacccagcctttgccggagaggcttgcatttttacggatatacacgccatttgcctgcaggtcgtccagcaactgaatgctcaccaactggccgtcttcaaaggcgttgctgattttcagccgcgcagcatatatcatcattgccggccggctaaccggctgtttacctacagagatacggatggaattaaaatctttgtcgcccgctttgcttaccggtgcaggagtagagaaaacggaaccattggcggagtttttactgaacacattgtatccaaaacctggcaggtataattcggggctttcaaaaagctgttttatagcgatgatcttgtagatatactgggcggtttcgttattcagcagtagctggtagtaatcactgctcccctggcgttttatgttccgggagatgttacccgaaccggcgttataggctgctgcggccaatgtccaggagttcagctgctggtgcaacagccgtatcagtttacaggccgcatgggtagccttgataagatgattcctttcatcgtagcccccgctcacagttagtccaagttcagcagcagtgccgggcattatctgccacacgccttgtgcgcccaccggtgaggtagcattgcttaaaccgctttccacaataggcaggtatttgaaatccagcggcacctggtattgttgcaggatgggttctattatcgggaaatattgctccgccttcaaccggagtgccggcagatagccctgatagcgtaggttgcgtttaataacatccatgaggcggtacgaaacaaaatccctttccattggcaccacctccccgcagaaatccacctgctgcgccgtggtataacccggcaacagcatcagcagtattcctatcagaacaacctgtttcttcatttggtttctctattgcttcgccagcatgtaccgggggaatacagttaccggcacatacaataccagttgttgttttccttcggttgtttgcagcacaatgatcacttcatcctctttccggaattgcttggagggaaccacaaatacttcgttggcctcttcttttggcgcgatggtttccggtccttttttataaaggatgggcatcgcatgcagcagggcggtatctttcttttccttgtgcaacaggcttgccttcactatttcgaaaggtacctttcctttattgcggatacggaaacaaaagtagttcatgttgttcagtgtcatggcctgcgcatatcctacgctcacgtcttccaccttcacttcatactggcggtttactttacggtctttcccgaagtcctccgctattttacctactgttaccgtatcaacactgatcaggtgtccggtttcttccggaacttctgccagggaaatttgcccgtccctttcgccatagccggcgcggggcgcctgcggtgttgcttccggagtagtaaatgcgcctgttgttttggctttaccggatagtgtgtatttcaggcgggccagatccactttatcgcggaaggcaataatcatgtaatgaatgttttctccttccctcactatcaggttggtaggccggggagtgggagttatcgggcgcagaaaaaccatgttaccatccacaatgcggtaatcgtagtcggtgttttttccgtcgccgatctgaaaggtactgataggcgcaccggatgtgatcagcgtcactgcccctttggtggtcagaatactatctgtgaccgtttgggcacttaccgttgacaaggcgcctgtgattaacaaacaaagcagcaaactgcacagcacatgtttcatcttttcaattggctttaatgcttatgatattttatatacggggttaaagcaatcagctccgggatggaaggttactcccacatacgcatttaagccccaaagctgaccgctgacggctatttaccatcctgttcgtaagtagtatcccaatctgccgcatcatcgcccctttgcccctccattttgatcaggaagtttttggcagggaaatatggcttcagatgaatatccaggtggatacggtctttctgtaccggatcctgctcgaaacggcggatattaaaatcttcgatcagcttgtccggcccggtgatcccatcaaggaagcggatgatctgtttcatcaggtccttgcgggtgttggcgttaaagttctcgaaggccctgcggttcaggaagtccatcagcactttggtaacaaagtcgaacacacgcactacggaataagtttgcaggcccaggttatccccgttgaacagtgttttcgcactgaatgccattacttttccgtattctttcaccatcggtaccagtcccattttttccaggctggcgatttcacttttcttcagttcaaatttcaccccgtctacttcgttcataccaccgaatttcttaccggcggtaacctgcgacatcagggttttatagatcttacctgccagtgcgccggaaggtggtacatacaagtgatcctgttctcctacttcatcaaattttccacggccaaccagccagttgcaggacatgattacattggaacgatgaatttccccaccggtcagattcgccagttcaaacatctccattacatcatccggtgcatcgagatgcgcgaaatcggttaccagcatggctttgttttcatgcgcgatctttgcccatttttctatcaccttattggagcccaggtaaccgggaatcaccagcaggctgtagttggtacgaagatccagtcgatcgtagttattcaccagttctgtgctgatggcgtcaatgaaccgggtgttatccaggtctttgagctgctccagttccacattgatgaacgacacattctttactttatcagactctgtgttcttgaagaagagtgccacattgcggtacgactgttccagttcacgggtagactctactgcttccccgagattagtggacagcaccttttccgcttgctctgcatgggaagtacagtagtccaccatttcaggcagttcgtttgtttcggacaatactttttcccagagcgacagtatcttctttaatttatctctttctgtttttttgccggcttctgtcaaaaagatattgcggcgcgccttacgatcggggttcaggttttgcgcaccttccaccgctgcttccagcaggtcgaagccaccatattttgccagatcttcaatacttccggcgaggtttacttcagattgctgtgaagacaggttctcattctgcagttcctggtttttctgtaattctgccataatcattgaggttatgttcccgtataggcaacggttaattatttggtattaaggtctttcatcattccacgaatggcgttcagcatggctttacgggcgtccggatccgccagggctgacttcaggatcttattcgttttcagctgcttcataattttcaggtactgctccttttcggtagccaggtcgttgagaaaggcgctttgtgccgtgataccttttacgccgaaatcgcccaggtggtggaattgtaatttttccggtacagggcggccttctgcatcatggaaacttacattcactgccggcttgaagtgttcaaacacactttctacggaagtaagcccttccactatttcgggtttaacaggcgcctgctgggttaacttttcagcaaacaaggtacggttatgcgagatttccgcgatggcttcgttggcgtccagcttcacttctgtgccgccaattccgtagttgtcattcatttgagataaatttagaattttgggaatctgacaatcatcaaattattgtccagtctaactgatcattttttatatccagtgttaccgtcatatctttccggaggctgccgtcgataatcattctcgacaagggcttccgtagttgtccccgtatcacctcccgcagcggccgtgcgccatactggggagaatatcccatcagcgccaggtgcctgcgggcagctgttgttacggtaaaactgatgtgctgctgctccagcagttgcagtaaatgttgcaaatgaatatcgaagatcttttctacgttggctgattgaataggcccgaagggaacgatctcggtaagtcttcccaggaactcaggccggaagtgacgggccattagctccatcaattgttgggaagcgggaatcacgccttcctggaaggaccgcgatatggcttcgctgcctatgttggaagtaaacaacaccagtgcattggaaaagtcgcctgttttccccagcctgtcgtgcagtttcccttcatccatgatctgcagaaaaatatcaaatacagagggatgtgctttttctatttcatcgaataatactacggcgtagggttgttgccgtattttattcaccagcagtccaccttcctcgtatcccacgtatccgggaggggcgccgtataaaagtgcggcagcatgttcctctttgaattccgacatatcgaagcggatcatggagcgttcgtcctggaagagaaaatccgccagtgattttgccagttctgttttacctgttcccgttggtcccaggaaaaagaaggaaccaattggttgtcccgggcggctcaggcctgaacgggattccagtatcgcatctgctacggctttgagggcatggtcctgccctaccacccgcttgcgcagttgcgcctccatgttgatcagccgttccctttcctgcgattgcacctttcccaggggaatacctgtaatggccgcaatcatggtagccagatccaccggtgttaccgcttcctgccgggaagaagcgattgtttccagttgctccagcaattgctgcaaggaggattgcagttccggcacagacgtaatcttatcaggatcggtttccgtatgtaaacgggatgatagtaatacgcccagcctttctttcatttgccggtaaaaccaatgaagatccgctatctgtaaggattccttactattaagatcagcaaattcctgttgtaaagtttgtaacagcggctggctggtgtcttccgttgcccttaccgcggccatggtgcggtccagcaggttcacggcgctatccgggaggcttctttccttcaggtaacgtttcgacaaacggatggcttcgtttatcccttcgggtgagacggtgagctggtaaaagttttcatacaccggcaccacagcacttaccatttttccggccagtgcttcgtcgggcgctgccaggttgatcgtttcaaaacggtgccgaaggatagcatccggctcaatgagtttacggaaaccttccggtgtggtagttccgataaggatgatctcccctttacccaatgcggctttcagcacattggccatgcctgtaccggtttgtttatcgagcaggctatgaagattatctataaaaaggatgtgcctccctgtttgtttaagttgctgaatgatctggagcagacggtcttccagttcacttttataggcggcgcctgctataaatgcaccgtagtccagcgcataaatatcggatgcctgcaattgcagtggtacctgcttctgcacaatggcgcgggccaatccttctgccagcgctgttttccctacacctccctcaccaataatcagtacgctggcgcggtctttacgtgtaagcacttccgttactgccctgatttccccgtcgcggccaatcaccgggtgaaaggttttcagcagttgcggatcggtaatacggtatacatatttcaatgcgccgggcttaataccgccgggcactgtggtattggtactggtttcttttccttttttgccggcgcccaggagctggtcgcgggtgaatggaaatgttttgagttgttcataggaaaaacctacacccggcgtgcataaagcaataagcaggctccatgcatccggttcactgtcgctatcctgtgctatactgatggcttcattcaatactgctgccgcagcttcatccggttccggttcatcgggaatacgcgatgccctgggcatctcatccagccggacttctgcccattcttccaggtagtatacatcgatatccatttgatgcaatgcaggggcgagacctgtttccttatgcaaacaggcgcgcagtaagtgcgcaggtgtaaactgcggatgatgatactcctttgcaatggccgttgcaattctgatagcagattgcaatgcagggccgaatatggtcaaggttgacagggtcatttggatgattccaggtttttcagaattcagttaacaattacaattttccgggttgcctcttttggaagcaaagtaaagatacagcgaaaacatatacgtagaattcattccggaaaaaaatgcagtctttttttaagcccaccaccaccggatatatatcttatcccccgcgattcataaaagccataaaacgcgctacagcaaagggttccaaagggtgtcaaaaatcaaacaatattatttatcttttttataatataagtaatcattaaaaaataacagcggatatagggaggatgtctaccaattaaataggaacgtgcggtctttaaatctccggaaaaaaaattacctggcatactcatccggtttttttatgacggagaaaatgcgcgggaagtccagataggcagattgcttttcaggtcttccgccaattgtaacattgacatgaaatccaggaaaaagttattcagcagctgccggttatgtaacgacttgttcaaagtggtttcaaaataatcggttccatgatcgatgccgatgtaaacccggttattataaaaagaaataaacaatctcgccccggtgcgttcgtgcaatgccaccatcctctccatcagcgccggagtaagcagctgctgcgctgccacctcatcaggagcgtacaccataaataatttattaaaagcggcatcagccggcaataccttctttccaagatgccaggtttgaatgtatccctcgccggccgcgctgttattgcgtgacagcacatacacaggcgtactgaagtaccggggaaactggccgataaaatagctgccacagaaaacggtgtcgggtccctgtccgcgtacggttaccaatggcatatgcatcaccgtgaggtcgcagaactgaaaattcatctccccaagtttaccatacacctggtcattacccgtcatctggtatgctttcttttcaaacagcccgctttctgtaaattcttcatagctggcatgattaaggggctggtattgataatccggatggatgaagctgattaatggttttacaatccgttgcttaaaatcgtgccggtaatctgttgcttcgtttacgcctccctgtttcatcataaaacggcgcattgcatagcctgtcagcgttacaagcagtaccaggccggcaataacgacggtcctgttcccttcatttcccgaagcgggctgcagggaaaaacgcacgataaagaaaacaaaggcagcaaacggtaccagggacaccacccacatccggcgtacccagttacggccggcaatacgttgtttttccagcgactccagttcatcattgagttgccgatccaggaaggcattaaattcttccagtgttttcatcacaaaattgttatcagttagaagaccaatgtgcagcagtgccaccgatgctgcttaccaccccgcctgaaaatggctggctgataagcgctttaaatggttgcacattttcagcagataaaggcagcttgaaaaaagaccggctttgtccgagttgtacatacgcatattccataggaaacaggcgtaccctgatgatccgcagcggcaaaatgagtttatagtccgtataggtgtccacgttatttactgattcacctctttccagacggctcacaaagtcattaattttttccggccgttttctgatctgtgcaaacataaaaagatatgggatcagcactcccacgggcatgaacagcagtataaaaagaacagcagcaggtgtttcagtacttctgcccgcaaagatgctgtagccgataagtccaaacaccagtacagccaatacttctgcggtgatcagggcggtgatggtctgctttttatctttttcatggatttccagcagcttggttttcagctcagaaaaattcttcatcggatatggttttgtaaatttattttgcccgcagtttgctgtaattgctgatagcgagatagaatcctgccaacgccacgagcccataggctgccatcagtgcccagatgctttcaccggttaccttatagatcagcatttcaattttggtaatactgatactgacatcgctgacggcgtgaaattgtttgtaacggtagaagatcagcgcgatacccgctatgccaagtaatacgccaacaataacaccaccccaggaaggcggatcatcgtcttcttcttcaggattacgcggacgcacgtctttaccaggttcatttgcattactcatccggatgatggttaagggttactaaatataaggctgctatcaatatttccgttcacagggcttctccgaggttaaccgaattgaaaccgaatcattcactgtacgaaaataaatgaaaaagacatcactcacaaacacattatggtgcggtgatcacttccggtggatacgcatagtcctgccaggctgcctctgcttcttctgcagtgatatcgccgctatacaccattacccggtatttcagctggtagcgggcatccggatacagctgccacggtttcatacgggtgggagtataattgaacatcagttcaccaccttccgcattttcgggccatacacgcaggggttcaggagaatcaaaattatcaggatagttcatgatcagcaatcctgcctttccctgtggcgtagcgccggatattttcacccagcgggcacgggtactgtcggcatcccggcgtgttttgctctcagacgtaagcacctggctggttttatctgtaaagtcggcggtggttcgtaaaccaaacccgccaccatagcggtattgcaacagggtaatgccagtgggggtagctggtgtaaaggtggaagtaaaatcccacaggcggcggtcgccgttgttggtggcgggatacgcctgtaccagccatgtttcatgaatggcggttttttctgtaccatctttcagaaatgctatatgatcctggctggcactgaatccgcaccatacgtttccggaaaatatttccattttacccgcaaagcgtaccttgccttctttcttctgcacattccagaaatcagtttcacgtccttcaaacagcgtatgggtccagggattccagatgcccatatgatgccggtgaccggcatttgggaagatattcgtgagcactacaccattaggcgcccagagcggatggataaatgcactgcggttatacacggtatctgtgccggcgggtgcgggcaccgttttaaaattatactgcaaaataggttgcgcggattgttccagcagcacatggccatcctggcggagcgccttcatgagggtgtcagttgcgcccttgcctttgcgcagttcatattttctttctgtacctgctgcagtagttcccgtaaggatccagcaaagctgacctgcctgccggctaacggatacgggtacacgcttattaccggttacttcttccagtatcaccggatcaccggcggatgacagaacgccggtatatacaatgctgttgtagcggttcagctttcctgccttcacagtaaagtgtgcaattacctgcgcatgggtgtccatataaaagaaaacaaatagtaacggtaacaggtggaattttttcatattcatctccggtagattccctgaaaaatacggtttactttttcagtatgcaaataccttgcgcagggaaatattaatattgtttgaagaccggcaccatattatcctttaattcaatatttttgaacgcttaaaggttaattatggcagcccctctcagtaacatgctgacaacaaaactcattataaccaataaatccgcccttcaacagaaatacggcgatgctcaccagcagattctggatgatataaacgcattgcaggcatttgataacaacaggcacctggatgcccacattattttcctggatgatgctgcccagatgctgggctgccagtcaaccgcagtaacagcagccacggacgatgcccagaacaaaaaagcgattgatgaactgtaccgcttcttttcgcccggatatatactcttgctggggtcgcaggatattattccgttccagcggctgaagaatttgttaccgggagataacgaccccgatacctttatacccagtgacctgccctatgcgtgcgacacgccgtatgatacagacccaggtaaatttatttcacccacgcgggtggtagggcgtttgccggatattccaggcgtgggggacccttcttacctgcacacgctgattacgaacatactggcagcagtgccttccaaacagggcgactacctcccctatttttccatgagtactttcgactggcagaactctacacaaaatacccttcagaacatttttggcagtaccagcaacctgctcatattccccggcagcgatgaaacgctgaacggtaccaactggaccgctgcacaactgcaggctaaaacgcatttcatcaactgccacggagccatctataatccagggttttacgggcagaagtccaccgagtttccgctggcgatgagatcagatatcctgaaagataagattacccacggcaccattgtggcagccgaatgctgctatggcggccagctgtttgacccgaagaaaaacagcggtaagcgcatcagcatggccaacagctacctgctgaatcatgcgctggcttttgtaggcagctccaatattgcctatggcccgcctaccgggcagggactggctgacctgctcacacagtattttgtgatcaatgtgctgaacggcgcttctaccgggagagccttgctggaagccaggcaacggttcctcaatgaaatgggccccatgctggatccctatgaactgaaaacggccgcacagttttatctcctgggcgacccatcatggcagccggtgatcaacgacaaagatcccagcagcaccggcgatacgcagctttttgtaaataccctgcaaaaccgccgcgataacctcgaagcaaggggtaaaatgctggacgacttcatcgcagtgccccatccgtctgatggctcgcacgccacagatcccgcactgcaccaggcgatgcacaagttgctggatgaaaagaactttgccgaaaaaagagatccgaaggtatttgtcaacaagaaaaatacccccgcagtcaaagaagatgtgagcggctccatgccatctgtaaaatttcacgtattttcggaatctgccaccactggggactccccttcaacaaaggtgatagtggtgaaagaaaagaataatcaaatactggggtatcgtgaatatgtcagcagataacagcaacagggacaaaaacagtccctttattacacttaccgggcgtttggtgctccgcacatttggtaaacacagcaaaagtgaacacctcggcgtattcctggtaacagaccagggagattacctgattcgcccttcaggagcaaatccttttatgcccaacccgctgatgccactggctggcaaaactatagtggccacgggttgcattgaagactatgttttccttgctcaaacctggaaagaagaagagtgagctgccttcaataactccgcaccagttccccacctgtcggcgtaaataatacggccgttttccattttaataccgtctgcgctatcttccgccagcaacagcggaccatccatatccacataatccagcatcggcagcagatgcgccactgcagaagtgcctaccgtgctttcgttcatactgccggtcattactttcatgcctaaacgctttgcctccgtaatcatccgcagcgctggtgtaacgccgccacatttggtgagcttgatgttgatgccatgaaaatagccgtggcattgggctacatcctgttccacaatacaactttcatcggctataaccggtaacaccactttttcatatacctgtttcattccttccttgtctgctgctgccatcggctgttcaataaattccacgcccagctcctttaacgcaatggcattacgcagggtttccactactccccaggcacaattggcatctacccggaaaatagccgtggtatgctttctcagctctttaataatcgcaatatcttcctttgtaccaagtttgattttataaatgggccacggaaattcctgtagtttccgcaccatattttcaatggtgtcaataccgatggtatagtctgtaagcggattatgcgaaatatcgagtccccatacctcgtagagtttcttttgctgctgttttgcgtacaggtcccacgcagcaatgtccagggcgcatagggcaaacatattatccttcagcagcgggtacatgtcttgccagaaaagctctggtgtatgcagggtatagttttcaataaaagaacggtgctgctcaagatctgccatcagccgtggcacggtcatctggtaataggcattgtcggcggtttcacccaacccgctttccccctcctgttccagctttaccaccagtaagggttgcagatctttggacttacgggaaatcgtaaacgtgtgcctgaatttcagttcaaaagggaaaagggtgagcttcattttactaacgggttctttctgtgaaaatacaatgcatttgtgatattgttaaccgcagctgatcatcgaacggacatcatctccggaaggttccgcggaatgcggtaacgccagtaatgcgatgccactgcggggatattgatcctttccgtatcaggattccgggtactttcgggggcttccgcggccaacaggtcctgcacctggaagatgcgccacatagcaggagacgccatatgccggctgataatttcgcggatcagttccggcgtagcagtggcaggtgctggtccggtatgttgcagctgttgctgataatatttccgggagatggatgtattttccttccaccaccctctcaaggtgctcatatcatgcgtggaaggcgttaaaacagacaggtagggcgcctttgatatgtctgcaaagagtgcgttcccggattttggcatgcgttcaatttccaggcttaaaatgccttgtgcctgcattacaccaggcacgcatgcgggcaccatacccagatcttccccgcagataagcatacgggtggccctttttatcagggggagtttatcaagcgcttcccggcgccagcagctttcctgccgcaggtagaagtagtcgtggtacaatgcctgcaaagcttccctgctcccggcatccaatgccgcaaacgatctggtggccgccatatcataacggggatggtacaacgttttactgtctccacttacttttataaataatacatcagctatcaggttatagaggatcgtttttatggtttccggcaacgctgatgccgccaccttttgttgcgtactgtatgccggcaacagctggtaacgtccgtccggcaagggatgcatcagttgctctttcatcatacccgcatagttgccaaacagttcttccaggatggcgtcggttatataaggcaggcagtacctgctttcttcaaactgaatgccacggcggcccatttcctccggtgtaacgggaacggcaggatgaaaatatcccagtatgccttgtatagcatcgcggggtatctgccagatgcggaagaagccaaggatatgatcaatccggaatgcgtcaaaataaacagacaggtgacgaaggcgctgctgccaccactccaatccgttttccctcatgtgtttccagttataggtaggaaatccccagttttgtccttcgctggtaaagctgtctggtggcgctcctgcctgcatatccaggtaataatgaccgggattcatccaggtgtctgcgctgtggcgggccacaccaatggcgatgtcgcctttcagggctacgttacaatcgtgtactgcggcgctggcagcggccagctgccgatgcaggtggtattgcacgaagaaatgatactgtactgccgcagcagcatcttcatctgctactgccagttgtttcactgccgtagcgtcatatacattatagccgggccattgagcgaaatcaccggtcccgtaacgatcgcgcagaaagcagtatacggcgtaaggcagcagccaatgctcattggccgccagccattgccggtattccggtgtttgtaaccggtgcccttccgctttaaacagcgctcgcagataagccagtttgaacgacattacttcttcatagtccaccgtttctttttcgttgagccattgccgtagccggtcaaactgccgttgcaacggatgggatgcaggcaaactgcctacgtcctgcaagcggatatattgtgggtgcagcgcgaaagaagaaatagcggcatatggataggaatctttccaggtaccggtttgtatggtatcattcaccgggagcagctgtatcagctgcagccctttctgctgcgcccattgggcaaatgccggcaggtctgcaaattcgccggtaccaaatccttcgggactgcgcaaactgaacacgggtacggccacgccggcgcctttccagggagcaggtgcaatacgcaaaaatccgtcgtgtaaaattacctgccgccctgttgttgcggtggtatgcaattcacggttgctgccggtttcatactgaacaaattgttgcctgtcctggtcgtaaatgccgtatttataatacatgggcgccgcttcaccggaaaggttcagcgctatggaaaaccagccttgttcatcgtattgcagcaacagtgggttactggtatcccagttgcctgttgacagactgccgcccagcaaacaaacggttttactgctatccagcagtggcgcctgcacacggaatatatgcgttgccgttaggggtgctgtaattgcagcaggggatcttttataaaaaacgcgggagaaaggagccgttagccaggcattttccgggcgatgcgcatcattccaggtatccaggaaaacgatatcaggatgttctcccggtataaaaacaaattcacgtactgcgccttcgtatatcacctcttccccttctcttaacaagtactggtatcgcagggtaaaaggtttcccgggagccagccggatatcggtgtaccaccattcttcgtttccccattgcataaggcgggcatgttggggcatatcattacccaacgcaggtaaattaccaagcaggtataaatcctgcccgtaatgagtatggtaacggatataaaaacgtacactgtaattcatcggatcccggctaagccggaacaaagtaggaaaaaacgcgcggattttcgcggatgttgtctttctcaggattacactgattttactgattagtttgatttttactttttggattttataaggatttggggagatgtaagcggtgattagtgcggatgttgtctttctcaggattccagggattttaaggattcaggggatttgatcactttggattttaaaggattgggggagatgaaagagaatttgatcatttttgattaaaaaaaagggagatataagcaggtttatccgcttatatctcccaaaatcctttaaaatccaaagtggtcaaatcccctgaatcagtctaatcaggttaatcctgagaaagacaacatccgcggcattattttacttcttcgaattctgcgtcggtaacgccatcgttagcaccaccctgaggctggccctgttgctgaccgccgtttggctggccgccttcgggttgaccctgagatgctttgtacagctcttctgaagcagcagtccaggcagcttccagttctgcagtagcagtatccagttgcgcgctatcctgtgatttgtgtgcttctctcagcttttcaagtgctgcttcgatagttgctttcttatcagcaggcagtttgtcgccgtattctttcacctgtttttcggtttggaatatcaggctgtctgctttattgagcttttcgatcttttcgcgttgttctttatctgaagattcgttggcttttgcttcggctttcatcttttcgatttcttccttgctcaaaccactacctgcttcaatcttaatgttctgtgtttttccggtgcctttatcctttgcagttacgtgcaggataccgttggcatcaatatcgaaagttacttcgatctgaggaacgccacgcggagcaggaggaatatcacccaagataaagcggcccagtgttctgttctggttagccattggcctttcaccctgcagtacattgatttccacgctaggctggctatctgctgcagttgagaaggtttcagatttcttggtagggatagtggtattggattcgatcagtttggtcattacaccacccattgtttcgatacccagtgacagcggtgtaacgtccagtaacagtacgtctttcacttcacctgtcagtacaccaccctggattgcagcacctacggctactacttcatccgggtttacacctttattaggttttttaccgaagaatttttctactacttcctgtatttttggaatacgggtagaaccacctaccagtatgatttcgtcaatttcggaagtgttcataccggcatctttcaatgctttgcggcaaggttccagtgttctttccaccaggctgtcgctcagctgttcgaatttagcgcgggttaattttttcaccaggtgtttgggaacgccatccactgcggtgatataaggaagattgatttcagtttcctgagaagaagataattcgatctttgctttttcagcagcttcttttaaacgctgccatgacattggatctttgtgtaaatctactgcttcatcttttttgaattcatctgccagccaatccatgatcactttatcgaagtcatcaccaccgaggtgtgtatcaccattggttgattttacttcaaatacgccatcacctaattccaggatagagatatcgaaggtaccaccaccgaggtcaaatacagctattttgctgtcctggtgttttttatccataccataagccagtgccgcagcagtaggctcgttgataatacggcgaacatttaaaccggcaatttcaccggcttctttggtagcctgacgttgtgcgtcattaaagtacgcaggtacagtgattaccgcttctgttacttcctgacccaggtagtcttcggctgttttcttcattttctgcaggatcattgctgaaatttcctgcggagtatataatctgccgtctatatcaactcttgtggtattgttgtctccttttaccactttatatgtaacgtggctcacttcactggcaacttcgtcaaaatgacggcccatgaaacgcttcactgacataatagtgtttacggggttggtaatagcctgacgctttgcggggtcgcctactttcctttctccgttctttaaaaaagccactacagatggggttgttctcctgccctcatcattggcaatcactaccggttcgttaccttccattacggcaacgcatgaattggtagttcctaagtcaatgcctattatttttcccatagtattaaagattatcctttagttgtaagtatttccgtgtttgtcgttggtttgtcaatgattatgccaagcaaaaaaatatgaaattatgtcagtcaggtaccctatatttgatcacagatcacagttattccgttggcaaacacctttttactaaataactgagtcgtttaatttgttcataacctcgcctttcttcagctattttattcctgacctcctgtttttataatgatacaaattgtgtaacctaaccgttatttcttatgaatacatccattttatggagggctgcgtgcttgttgttagcaaccaccccaatgatgagccaggctcaggatcaacctaccactacttctgccgtacccacagcaaaattattcagtggccccagtgactataaaacatggtcaattggcgtaaatggcggcgttttggcgccagtggctgccaccggtggcagtaacgactttaccaaatggaaaggatccttcggttatggcgcctatgttaagtaccaggtactgcatttctttgccctgcgggcagattatgtaggcggtaaactccaggcagataacagtaaagaactcggtaacggctcccttcctgtcagaccgtataagtcgtacgaaaccaaattaaactggtcaggaactttaaatgccgtattcaatatcaccaccgtcaattggttattccgggaaaactttgttcagctgtatgcctctgtaggcggaggattggccggatataaacctactgtaaccagaaacgacaacaccagtttcccctataaagcggaagacaaagccatcaaggaactgattatcccggtgggcgccggcctcaaattcaggctgtctgagttcattaacctggacctgggctataccatgtattacaccgacggggataacctggacggctacaactacggccccaacaaggataagtactcctatggctatgcgggactggaatttgcccttggcaagaaaggcaaaaaacaactgcagtggtctaacccggccaaagtgatgtatgatgagctggaagcccagaaaaccaccctggcagcttcgctggatgctgccaatcagaacaatgccaggttgaccgctgatgtggataaactgacaaaagacagtgacgcggatggcgtttccgacttcttcgataaatgcccgggcacccctgccaataccaaagtagatggctccggttgtccgctgccggtaccggaagtagtgaaaaaagaagaaaaagtagtgattacagaagaagataaccgtatcgtaagggaagccattcagaacctggaatttgaatttgcgaaggcaagcatcaagcccagctcctatcctgcgctcgaccgggtggcagaactgctgaaacgcaaaaacctcaacctgaagctgagcggccataccgacaatgtaggcagcaagtcgcggaatctcgccctgtcaaaggaaagagcggaatccgttaaagcatactttgttgataaaggtgtgaatgcttctaaaattgaagcagtgggttatggcatgtcgcaacctatcgcctccaataaaaccgcggcaggccggcagaaaaacagaagagtagagtttacaatattctaactgactgacaataagatcatagggattttttgatgtgaaatcaaaaaatccctattttcattttatggaaccatacatcatcagaacaatagctcctgcagacgatccggcaattgcccatatagtaaaaaccacgttgacagaattcggcatgaacaaagccggtaccgcgttttcagatcctaccaccgagcacctctcccggttgtttgatattccccgtgcagtgtattatgtagcgctggcagatgacagaataattggcggggccggcattcatccgctggatggcggcgaagcgcatgtgtgcgaactccagaaaatgtacctgctgcccgaagcccgggggaaaggactggcaggcaagctgatcaccctgtgcctggatttcgctaaacaaaacggctacacgcaatgctacctggaaacagcgccagaacttgccagggccaggaaagtatatgaacagttcggattcaggtacctgacaggcccgatgggtgataccggtcattttggctgtgacagctggatgctgaaggatttgtagtttccgcaacaggtggatttttattcctcattgtaaaccggcacacttcttgtcaactggggcttacaaaataacatatcatgaaaaaacttattctgtctggtgtattagccattggaactatgctggcagtacaagcacaaaatgtaaaattcggcgttaaaggtggtttgaacatctccaaactaacagataccgacggctccaaaacactcgcaggcttccacgccggcggtcttgttaacatcgggctgaatgaaagctgggcaatccaaccggaagtattgtattctgcccagggcaccaaagcagaaaagagtgtattatggttaaccacttccaacacggtgaaggttaattatattaatgtaccggtaatggtacagtattctattgtacctgaattttatttggaagcaggtccgcaggtaggctttctcacagccgccaaagttaaatccggcgatgtaacagtagatatcaaggatgatatgcaatccgttgacttcggactgggctttggttttggttataagttcgatatgggtcttggtatcagcggcaggtataattttggcctgaccaacgtatatgattccgacaaagtagacagcaaaaactctgtagcacagatcggcgtgttctacactttttaatgcaggcataaaatattgcagataagcgaaggttgtctttatcagacaaccttcgctgctttcggctaattaactatctttgcccctcgcattaatcattttcagcatgagtgttgtacaatccatcagaacggccgccgtggccgccattaattcactttacgatcagcagttaacagcagcagatattgctattaataccaccaagcctgaattcgaaggtgagtataccattgtcgttttctcttttacaaaattcagccggcagaaacccgaagaaacagcacaacgtatcggggaatacctgactgcccactacccggaactgattgcgcgattcaatgtagtaaaagggttcctgaacctgagcatcaacgatgcctactggacaaaattcctccagcaacattacagcgacgtaaacatcggattacagcctgccaatggtaaaaagatcatggtggagtattcatctcccaataccaacaaacctttacacctcggtcacctgcgtaataatttcctgggatatgctatcgccgaaattatgaaagccaatggctacgaggtgatcaaagccaacctggtaaatgaccgcggtatccatatctgcaaatccatgctggcatggcaaatgtttgcacatggcgacaccccgcaatcgaccggtataaaaggcgatcacctggtgggcgactactacgtgaagtttgaatcggtggtaaaagaacaggcagaaattatcatcgaccgcgtactggaaaatgacttccgtgacttcgacagcgccgaaaccgaaaagctggaaaagctggtaacagctctccataagcccgaagtgaaagacgataaagaaaaaactgccaagatcatggacgacatcaaagagatgtcgcgtaataaaacagagatcatgcagcaggcgaagatcatgctgcagcagtgggaagccggcaaccccgaagtaagggaactgtgggccaccatgaacagctgggtgtatgaaggctttgatcaaacctataaacgtcttggcattgacttcgaccagatgtactacgaaagtgaaacctacctgttaggtaaaaaccttgtagcagaaggattggagaaaggcgtgctgtttaaaaaagaagataactccgtatggatagatctgaccgccgacggactggatcaaaaactgctgctccgcggagacggcacctctgtatacatgacccaggacatgggtacggcgcggttgaaatatgagcagtaccagatggatcaaagcgtatatgtggtggcagatgaacaaaactatcacttcaaagtactccagctgattatggagaaactgggagaaccatctgccaaaggtattcaccacctcagctatggtatggtggagctgccgcatggccggatgaaaagccgggaaggtacggtagtggatgcagatgatatgatcactgaaatggtaaaaacagccgcagagaaaacacagcaatccggtaaaaacctggatgcgttttccggtgagcaactcaacgaactgtatgacacagtgggtatgggcgccatgaaatttttcctgctccgcgtagatcctaaaaagaaaatgatcttcaatccggaagaatcaatcgatttgcatgggttcaccgctccgttcatccagtatgcgtatgcgcgtatcaaatccatcctgcgggacgccggcacaacagcaggacttgaatcatatacctacgaaggagaattgctgccgctggaaaaggaactgattattctgaacgaacagtttccgggtatactggcagacgcataccgcgagctgagtccttctgtgatcgccaactacgcgttccagctggcccagttattcaattccttttatgccgagaaagtggaaggcgtacctacctattccattatccgcgctaccagtgaagaaaagaagaaactgcgtttacagattatcatgctcactgcgcataccattgctcagagtatgaaattacttggcatccgtgtaccggaaagaatgtaataacgaggaggttgtctttctcactgattacgctgattttactgattaccttgattttactttttggattttttgatgattttttaaaggattaggggagatataagcgaatatatccgcttatatctcccctaatcctttaaaaatcacatatgatcaaatccttgtaatcagtaaaatcagcgtaatcagcgagaaagacaaaattcgcttatattatcattaaaacgctgcagcccttacgggttgcagcgttagcaacttgcagccgccgtggccgaagttgccgaagaaaataccacagtaagcagcgcagcgaaaaaggagcttgcctatcctttatgcgctgtttaaaatccctctacactgtggcaaatatttttaccgggttgttctccgagtatgagagcttcatcgcataagcgttctcccttctcctgctcacccgcacccatatacgattttccgagcataaacatagcaaaagcattggtaggttgcaagtgtaaaacttttttccattgcactattgcccgtttaaaaagtttcctttcgtacaagtcgtgtgccagatgctgataccggttcacgcttttcagggtatccttaacaacgtatagcccagggcggtagtccgcttcttttttatcaaagtaacaggctgccggttcactatacactgcagtaagtaatacaatacaacagatactaacggatagctgacagggtttcataggtcgcggcacttatggggcgccggacaaatatatacataataaatcgtaaatgaaaacttatctatatgtaataatcacactcccagctcctcaccgctaaaggaaaggggcagtaaatcgttggcacgactgatcacatatattttaccgcttaaccccgccatgatcacccggatagggctttcctgtttccgttcgtactccgacaatgtttgccggcatatgccacagggagaaatgggatgggtactgtcgccgttgaggttattataactgatggcaatggtatcaatatcaatattgggatatacagaagcagcggaagccagggccactctctctgcacataacccgatcggataagaagcgttttcctggttagagcccgcaatgatttccccattggccagccggatcaccgctcccacctggaaacgggaataaggtgcataagcatatgccgttacttccctggcttctttcagcagccacgcgtcagcatcggaaagaccggtaagatcatcatatacctcgtattcaatatgcagcaattgtttctccataacaacagttgaaaagggttcttcgtatagtcgttgtcggggtaagacaacaacggaccggcagtatgccagtccgtaatttacttcaaattatatttcgggcggttgcttacttaatatttctgaagatacggctccagcggataccgccttctccatagctcatccagatcagccaggctttacccactacgtgatcttccggcacaaagccccagaaacgggagtcgagggagttgttacggttatcccccatcatccagtaatagttcattttaaacgtatagctatcagcgggttgaccgttgatgatgaacttaccatctttccgctccagcgtattgccttcataaacacggatcacgcggtcgtataaagcgatgttgctttcgtccagcttaacggtagcgccttttttaggaatatacagcggaccaaagttttcttctgtccatttgaaatgcgcggtatcgtgcgggaaaacgttattgtaattgaaatccgtaaaatcagactcctgatatattttaatgtctttcacgattggcttaaactgctcgagcgctgctacgttggccggtgtgaggttgtaaatgaacttgctggcatcaagctggtaaaagtccgggccggaagtagcaatgcccaggtcttccaggcggctgctgttcagctggtcgccggtagtttccactacatatttatgctggctgccgggaggaaccggtgctgcctgcccgttgacatataccgcacctttgatgatccggatggtatcgccggcctgggccatgcaacgtttgatataattctcccttttatctaccgggcgctggatgatcttataagagttctgcaccgactgccagccaaactgccgcaccatgccataatagctgggatcgggcgagtcaatggctacggtatctccttccgggaagttaaaaaccactacatcgtaccgtttgatatctgagaaaccgggtaaacgtctgtatttccacttcaccgcctctgaataggctttggcggatttggtaaagggcagggtatgatgtacaaagggtactgccagcggcgtcattgggatacgtggtccgtaactgatcttgctcacaaacaggaagtcgttcacaagtaaggttttttccattgaaggtgtcgggatcgtataggcctcaaaaataaaggtgcggataagcgtggctgctataatagcgaagatcgcagcgtctaaccattctctaaccgcagatttctttttcttaggctgactgtctttgttttttttccaaaatgccaggttcattcagttacgcttattagatgcttaaaaaggcaaatataatattctgttgctagcctgtcgctattactttacaaaagttttcttaaaaatagattaaaatattgtttattatagtttttaagtatatggtgtagccaccgctgaattacctaaatttggcatttaccatacctccgttgaatacatttacgatcagggatatcgaaaactttaccggtataaaggcgcataccatcaggatctgggagcaacggttccagctgttctccgccaggcggaaggataccaatcacaggatctatgacggggaggatctgaaagccttattgcgtattgcctatttatatcatcacgggatcaagatctcgcgcatagctgcgttgtcggaggaagaacagaataaactgtcgttgcagctggccgccgaaggatcggctgcaggtctccaggtaaatgagctgattgccgccacgctcgattatgattacttccgctttgagcgcattttttacagccaggtattacacctgggatttgagcactgtattacaaagatcatttaccctttccttgaaaagataggcgtgctatggcttaccggcaatgtgatcccggcacaggagcacttctgcgccaatattatccgcaccaaaataatgacggcgatcgacggccagcagatgaaccaacaggctactgcccattacctgttatttctcccggagggagaatttcatgaaataccattgttgtatgtgcaatacctgctgaaaaaaaacgggaaactggttaccagctttggcgccaacgttccatttgatgatctgaaaacatttaccccggtgcggccggtaacccatatgtatacccacctgcttaccaatgtaacaaaacaggcagtaacccagtttgtcgccgcactggcgcagcagttcccgggtattaagatcctgatgtcaggaccgcaggtatggcagctgaccggcccattgccggaaaatgtattcgtattgaaaagcctggatgagctattggcgtttaactgatctgtatcaaagcacttcctccaggatacgattgatggctgctgagcggttcagcaccataaaatgcccgccatcgggaatgaggtgtgtaggctgaagatatttaaccgggaaaggcaggtcccgcgcgccgtggatatgcaccagtccttccggcacctgctcattttcccagtgcaggatagcatttaccgcccaacgtgtaaaggtatagtcgcgctttgcaaggtattcattcaccagtttgcgttcttccggtgtttcgatattgaggaacttcctgacaaccacgcttctccgttgatacaacaggctgtcgggtaatttgtgcagtccgagtttctttacccagttataatagggaggcttttccgagctacgtttaatgctcgacaggaggatgttcttttctacgggaatatgccgggctatttccaggctcatgatgccgccgaaagacacgcctattagggttaccctcccatcagccgcaatgttttgggccatacgggccgcatagcggctgatgggttcctcctgcaatggagggatccattgcaggtgatgcacctggtagccggtgggaaaacgcaggttgttgaaaatgcgttcatccgcacccagtccactgatcagatacaggtgtttttgcatgttgttgctggttaagagcttacctttcttttatcgcggcttggcaccacgaaatcttccacgtcttccgcagtgatggttttacccgaaaggataacgagcctttccactacgttcctgagctcacggatattaccggtccagttgtgattttgtaaagctttcatggcatctttatccgctactttgcgggagataccatattcgctgcaaacgctgtcgaggaagctgtctaccagtaacggcacatcatcccggcggtcgttcagggaaggaacgtggatcaggatcacgcttaaacggtgataaagatccaggcggaagtttttgttttccacttcctgcagcaggtccttgttggtagcggctactaccctcacgtccacgctgatttccttatctccgcctacgcgggtaatttttccttcctgcagggcgcgcaatacctttgcctgtgcgctgaggctcatatcgccaatttcgtccaggaagagggtaccgccacttgcctgttcaaacttcccgatccgttgttttacagcggatgtaaaggagcctttttcgtggccaaacagttcactttcaatgagctctccggggatggctgcgcagtttacttccaccatagggccaccggcgcggttactgcgttcatgcagccacctggccaccagttccttacccaccccgttatcgccggtaatcaataccctggcatccgtgggcgctactttttctatcgtttctttaattttcagtatcggggtggattgaccaatcatatccggcaccttattcaccttgcggcgcagggttttggtttcggtaaccaggttggttctatccattgcattacgcagggtaatgagtaagcggttcagatccggcggctttgaaatataatcataggcgccttttttcaccgcatctactgccgtatcaatattaccgtggccagacaccatgataataggaatatccccgttcacctcacgtgctttctcgagaaactccagtccgtccattttaggcattttgatatcgcaaagaacggcatcatatgactttgcctggaacattttaaatccttccataccatccgcggcctcatctaccttataaccttcataggttaaaatttccgtgagtgttttacgaatacttttttcgtcgtctattattaaaatgttagccataatcagttttattttgtacgaccggcaatacctgccttttatacaacgggcaaaaataaagattaatcccttaaaattgcattatatcagggatcatttaacatgtcagaaacaattgagagattaccatatcctcccggcagccaggaacgcttgaatattagcagacagtctactacctttacaggattaatgcgtaatttcagtaacgattaaagtgccaatacctgtaattcgatccgcatatgaatgattttctggaagagttgaagcggcggcaccagctggcagcggcgaacgcctatcctgccacgggtgcagtagatgaatttgtgagccacctgttgaattggttatttcctgaacataccggccaggtaatccccgatccggtggcgctggaacgttttggccatgaactggaagcccagttgcagcaattgctgcaatcaatggaaaatcagctgcctgcggatgccgcggggctgagccgcgactttatgaacaaagtaccggtgatatatgatgaactgacaaaagatgccacggccatttaccagggcgacccggcagcatcctgtttatacgaagtaatccgtgcctatccggggttttatgccattgccttttaccgcattgcgcatgccctgtaccagctgaaaataccggtattaccccggatgatcactgaactggcgcattcccgtacaggagtggatattcatccgggtgcggtgatagcgccctggtgttgcatagatcatggtaccggcattgtgatcggggaaaccactgtaataggaccgcatgtaaagctgtaccagggcgtaacgctgggtgcactgagcattgaaaaaagtatggcgcgcagcaagcgtcatcctaccattgaggaacatgtagtgatttacgccggcgccaccattcttggcggtgatacggtgataggccatcatagcgtaataggcgggaatgtgtggctgattaaaagtgtggaacctttctcccggatctattataaagcagaacataaattttcagatacaaaccaggactagtacaatggcttccatcatagatctgatcggcaacacgccgatggtagaattaaagaagatatccgttaacccggccgttaaaattttcgccaagctggaaggaaacaatcctgccggcagcgtgaaagacagggccgcctatggcatgatcaaaggcgcgctcgacaggggcgatattaagccgggcatgaaactgatagaagctaccagcggcaatacgggtattgcactggccatgattgccagtcttttcggcattgaaatagagctggtaatgcctgcagatgctacccgcgagcgggtgctcactatggaagtatatggcgccaaagtaacgctcacgccaaaggaattgtcgatggaaggctctatcgactatgccaacgcccaggtggagaaaggcggttactatatgctgaaccagtttgccaatcccgataactacggcatgcactataaaactaccggacctgaaatctggaaagataccaacggggaagtgacgcactttgtaagtgcgatggggactactggtactattatgggtgtatcccgctatttaaaggagcagaacccggcagtacagattgtaggatgccagcctaccgaagggtcaaaaatcccgggcatccgcaaatggccggaagcttatctccctaaaatatttgaaaaaccgagggtagaccgtatcatggatatttcagaagaagaagcgaggatcatgaccaaaagactggcaaaggaagaagcggtattttgtggtatgagcagcggcggcgctgtggcagcagctgtacgggtatcaaaggaattacgtagtggcgtgatcgttagtatcatctgtgatcgcggcgaccgttacctttccagcgatctgttttcctgaaaatatttttaaagataaaaagaaacggagcgaagaaaatcttcgctccgtttcttttatattgatagcaggtgctatttcttcatgtacattacttctttcaccagtttcacggtacgttccacatccggcaggtattgcttaaccaggttgggagcatagtgcataggagcatcctgtgcggtgatacggcggatcggtgcatccaggtagtcgaaaccttctttctggatacggtaagtaatttcggaagaaatacttgcgaatggccattgttcttcaacaattaccaggcggtttgttttcttcactgattccaggatggtgaaccagtccagcggacgaatggtacggagatcgattacttctgcttcgataccttcttttgccagttcttcagctgcacccagcgctactttcatcattttgttgaaagatacgatggttacatctttaccggcacgtttgatatctgctttaccaatcgggatgatatattcttcttcaggaacttcccccatatcgccatacatcacttcactttccatgaaaacaaccggatcatcatcgcggatagccgctttgagcaaaccttttgcatcatatggattggaaacggagattactttcaggcccgggatattggcgtagtaactttcgaatgcagtggagtgctgcgcacccaattgaccggcagaaccgtttggtccgcggaaaacgatcgggcaacccacctggccgccactcattgccagcattttagaagcggtattgaggatctgatccagcgccagtacagcgaagttccaggtcatgaattcaactaccggacgcaggccgttctgtgcagcacctactccgattgcagcaaatccaagttcagcaatcggcgtgtcaataacacgttttggaccaaactcatccagcattccctggctcactttataagcaccattgtattcggctacttcctcccccataaggaatacccgttcatcacggcgaaattcctcctgcagggcttctcttaaggcttgtctgaaagctatctgacgcatgctattcttaattgaaagtttaaatgccttattgaaaggcagggcaaaaatattgtttgttagcgaaaaagcaaagcaaacgcccgattaataattattataccccccacatgcagtctgtatactattaattaaaataaatacatatatttatattttaaactatagtacacccggccaacaactttacccgctgtcatgattaccattattatcctaaccttatgctttttagctgccctgtcctgtaaaataaaaaaggtgaaagcaccggaaatacaggcgctcctgtggtaccttcacctggcttttggctgctttgcgctcctgtgcgtgttattgatgctgaacgactacggcttcaagggcacacaaaccgaacgggtgttctttaccctctacgcaggtaccggtatgctgatttacggccttaccaaaccggataacgacgccaggtacgcctacctgacagttttttttggcttcccgtttgtattgctgattgggctgctgctgccgccgctgcgtacccttaccctggtagccgctatcaccttattgtcggacagcgagtttcagcgctatactattgacgacgactacgccctgcaaacgaaaactaccggtatattatccaactacccggtttacagcctggtggaagataaatacctgttttttgagaaaatagtgcctgacgtggtaaaaccaaaggctgcattgcattcgctgaagatggtcaaaaaagggggagacagcgtgagaatacaggtaaataacatagataccgtgattgctatttattgatgaagtgtaaacctgtttcaggattatttctccaggtgtaaagttttttcaggacaaacccggggtggaagtgtatggggagtgtatgaggagtgtatcatgagtgtatggggagtgtatggggagtgtatggagagtgtatcatgaatgtaaggggactatatggggagtatagggggactatatggggagtatatagggagtacgacacatacacgactcctaagtaactgagaagtatcggagaagtatccgagaagtatccaaagagtattaacccgcttaccggcaatgccataacggccccgactgctgtaagatcaaaataaatcagccgtcagctgctggtttcgaaaaaaacagcagctgacggcctgtaattaaactctttctataatgatcgcgctggcgccgccaccaccattgcagattcctgcaacgccgtaacgcgcctgctgctgatgcagaatagcattcaatgttaccacaatccgcgcaccactgcaaccaataggatgtcccatggctacggccccaccccatacattcactttatcgagcgacagtcccaggtctttcgcattggcaataggcacgcaggaaaatgcttcattcacttccgccacatccatgtcgctgattttcaggccagctttattcagtgcgttgttgatagcttttaccggcgtagtggtaaaccattccggcgcctgcgaagcatcggcaaagctgatgatctttgccagtggctttaatcccagcgctttcagtttttcaccgctcaccagcactactgctgccgcaccatcgttgatgttggaggcattggcagcggtgatggtgccgtctttctgaaaacttggtttcagggaaggcactttttcaaaaatcactttcttatagtcttcatcttcagacaccgttaccacctgttttccgggtacctgtaccggcactacttcatctttaaaatatcctttctcccaggctgcggctgcgcgtttatagctttcaatagcgtaagcgtcctggtcttcccgggtaattttgtattcggtggcgcacagctctgctgcgttgcccatatgaaaatccttgtaagggtcccagaggccatcgcggatgatgccgtcggtaatggcgccatgtccgagtttataaccggtacgggctttatccaggtagtaaggggttgcgctcatgttttccatgccgccggccactactacgtcgttgtcgcccagcataatactttgggcgcccagcataatggctttcataccggaagcgcatactttgtttaccgtagtacagggaacattgttaggcacgcctgcagcgagactggcctgattagcgggcgcctggccgagattggcgctcagcacattgcccatatatacttcatttacttctgccggggcgatacccgccctttccagtgccgctttaataacgtgagcgccaagctgtgtggccggaatgcctgccagtgcgccattgaacgaaccgataggcgtacgggccacggctactataaatacttctttcatctgataaataagattgatttggctagtttataatctaccaaatataaggaaaagttgccgggaacagcaaccacgcctatatgctgatccccttctctccaaatcctaattttcccgtatgtttgcagttgcatttacgaaaccgtgatatctcagaactccatacaacagatcctcagccgcattgatattgtggaaattgtgggttccttcgttaaactgaaaaaaagaggcgccaactacttaggcttgtgtccatttcataacgaaaagtccccttctttcaccgtatctcccggaaaagaaatctataaatgctttggttgcggcgccagcggcaattccatcagctttatcatggagcatgaaaagtactcctatgtagaagcgctccggtggctggcacaacggtaccaggtagagctggaggaaacggaagtaagccccgaactgaagcagcaccagctgatggcggatagtttgtttatcatcaacaactacgcccgggagtacttcaccgataccctttttaataaagatgaaggccagaatgtgggtctgagttattttgaagaaagaggatttacggaagaaaccatcaaaaagttccagctgggctactgtctgaatacctttgactcttttgccaaatcggcactggacaaaggctacaacctggaatacctgcaaaaaacaggattggttaccatccggaacgatcaacctgccgataactatcgcggcagggtcatattcccgatccataaccagtccggaaaaatactgggcttcggggcgcgtatcctggtaaaatcagaccgggcgcccaaatacatcaattctcccgaaaacgaaatttatgtaaaaagccgggtactgtatggtacctactttgcacggcacgccatcgataaactcaatgagtgcctgctcgtagaaggttataccgacgtaatttccctgcaccaggcaggtgtggaaaacgtggtggcctccagcggtacctcccttacgcaggatcagctgcggctgattaagaaatataccaataacctcaccatcctttacgatggcgacagcgccggtgtgaaagcagcgctccgcgggctggacatggccattgaagaaggattgaacgtgaagctggtattgctgccggacaaagaagacccggacagctatgtgcaaaagatcggtgcggaagccttccgtgaattcattaaagataacaagcaggactttgtactgttcaagctgcagctgagcatgcaggaagccggcgccgacagtaataaaaaatcgcagctggtaaatgaaatcgctgaaaccatttcaaaaattgataaggcggaagattttacccggcagcaggattatatccgtcagtgcagccagctactccatatcgatgaacagggattgatccagctggtcaataaatttatccgcgaccgcctcgttaaacgggagcaggcctatgcgcgtaacaatcccgctcccagcgatgatggcctcagcgaagaagctattgccgccatggaggctgctgaaacaggcatttcagtagactcgctcatcaacgggcatgaaaagcaggaaaaagaactggtaaaaatcctgctgcgttttggcgataaacccttcagcgaagaagaaaacaacaccgtagccgactatgtgttccacctcccctacgatttcgaggcattggcagaaagtgagctggtgaaaaggattttaagggaatataaagcattgtacgatgcagggaacctgcaggacaaacggtggttcctgtatcatgaagatcagcagctgtcaaaacagattgccaatatactggaagataaagaagccgatttgagtattaactggaaagaccgtttcgagattgataccgtatacggtgataatgcctatctgagagataccatctccactaccaactatcttattctgcgtaagatcaagaagctgatccacgaaaaccaggaagaggctaaaaaggcgacagacatggaccagatcctgaactgccttgaaatgcagaagcacctcaactccctggaaaaggagctcacgaacggtatgggcactgttattttcaagtaaccgttaacgttagtatctcaaatccgctcccatacctggaaggagaacgggtactgatttttttcatccgcctcatggcgctcatcacttaccagttcaaactctgcgccatccagttgggggaaaaaggcatccccatgaacaaccgcatatacgcgggtgagatagatccggtctactaacgcccacgcctgttcgaaaatttgcgagccgccggtgataaacaattcatcaccgccgaatgacctggctttctcaacaccttcctctatagaacgcactacatatgcaccttccggctgaaaatccgtttgacgggtgatcacgatattgggtctgccgggcaatggtttgcccagggagtcaaatgttttacgtcccattacaatgggttttcccaatgtggtggatttaaaatatttaagatccagcggtaaacgccagggtaacatattgttgataccgattacgttattttccgaagcggctacgataatggatatacgcatatggaaagttatatggctaccggtgctttaatggccgggtgaaactggtaattcaccagttcaaaatcttcatacttaaaggagaaaatatcttttacgtccgggttgatcttcatcaccggaagcgggaatggttgcctgcctaattgcaggttggcctgttccatatgattgctgtacaaatgcacgtctccgaaagtatggataaagtcgccggcttccaggtcgcacacctgcgccatcatcatggttaacaaggcgtaggaggcgatattgaaaggtacacccaggaatacatctgcgctgcgctggtacagctggcagctcaatttaccacggggttgcccttttgcgggatctgcaggggttacataaaactggaacaggcaatgacagggactgagtgccatttccggcagttcgcccacattccacgcgttcacaataatacggcgggaatcaggattatttttgatggtatttaccgcttcggtgatctggtctattaccttgccgctgcgggtttcccagctgcgccattgctttccgtacacgggtccgaggtcgccattttcatcggcccactcatcccagatgcttacgccatgttctttcagccaggcggtgttggtatctcctcttaaaaaccagagcagttcatatataatcgatttgagatgcagctttttggtggtcaccacggggaaaccatcctgcaggttgaatctcatctggtagccaaaacagctggtagtgccggtgccggtgcggtctgtttttaccgcgccttcccggataatatgttgtaataaagataaatactgctccataaggtcgcaatttacgaagttttccagttgaaaaaatataacatatttaagtcaaagaaaaaaagcggaagtacccttaaaatttcgtaatctgctatatcattttacgttacaataagatcggcttaatgagaagtccttgccatcagagatgatgatgaaaaacctgtagtaccccttgtgcaaggatcgcaacaaattaacgctattaaacaaccaaaatcaaatcaggatctgtactatctataaaccagaaaaataatcagcaacatgatattgtaacctcgttttaatcatcattcattatctaaaccatttcaagctatgcttctaccaaaatccagcttgctggtactgctatgcctatgcagtaccctggcactatttgcgcagcaaaacattaccggaaaaatccgggatgccgtcagcggcaaacccattccgggcgtcaccgtacgcattcccaacaccaataaagggaccattactgatgccgatggcaactatacgctggccatcacggccggcactaccagtttaatggtgagctataccggttataaaaccaaaacaatcaatcttacaccgggtaacaacgtaataaacctgagcctggaagaagatttcgcccggctggatgaaattgtggtaaccgggttggccaccaatgtaaagcgaagtaatcttgccaatgcggtagctactatttccggcacggaattaaacggggtggcgcctgcgcaaacatttgacgcagccatcagcggtaaggtgcccggcgcactgataaccgccaattccggcgcccccggcggcggcatctctgtaaaaatgcgcggtatcacttctgtatttggcaactcgcagccactgtatgttgtagatggtattttcttcaataacagcagtattcccgccggattgaacgatgtaaccggcgccgctacctcgggcagtcccaacaaccaggacaacccttccagccgcattgcagacctcaacccggaagacattgaaaatattgaaatcctgaaaggcgcttccgccgccgctatgtatggcgccaaagctgctgccggcgtaatcatcatcaccaccaaaaaaggtaaatcaggcaaaacgaaagtgtccctcaaccaggaaaccggttttaccaaagtacggcacctgatgggcgtccgcacctttaccccggaaacagctgctgatcttgcaggtactgccgataaccctgatcctgccgtacaggcgaagcgtgctgcttacaaggcgcagttcaccgaggcaaagaatgccgggaagatctttgactatgaaaaagagctcttcgggcaaaccggactggtgctgaacaccggtgtgtctctcagtggcggcggtgaaaaaactaccttctatctttccggtaaccggcggcaggaaaacggtattgtgaaaggcaccggctatttcaacaactccatccggctgaatgtggatcataaggtgagcgatcgtatatccataggcgttactaccaactatatcaactcttccgccgacagggggctcaccaataacgataacaacggcgtttccctcggtgtggcgttgtcgtccacacccgattttgtgaacctgtttcccaacgcgctcggtgagtatccgcgcaatagcttcgccagttccaacccgctggaaacacgcgacaatatgatcaacaacgaacaaaccaaccgctttgttggtggtggtaatattgagatacggctgcagcaaagcgaccgctccaccaccaggctggtagggcgcggtggtatcgattacttcaatttcaaaaccaccgccttgtttccacgcaacctccagtttgaagagaacggacagcaaggacattccatccagggcaataccaacaacaccaataccaacatcggcggatttatagtgaatacgtttacgccaagcgagaagctcagtttaaccagtactgccggcgctaccctggaaaccggctatctcgacaatattgttaccgtagctaccaacctggtatccggccagagtaacctggatgccagcgccaacaccactacccggcaattccgccagaaataccgcgataacggtatttttatccaggaagacctttccctgatagacgccattactttcagtgccggcgtacgtttcgacaggtccaccaataacggcgaataccagaaatattacgttttccccaaaggatctgtttcctggaatattgccaaaatggatttctggaaggtagccggtgtggataatctcaagctgcgcgcagcttatggccaatccggcaacgtacctccttatggcagtaaatttacccagatgctcggcagcaatatcggcggcttccccggcgtgctggtagaaaaccagcagggcaaccccgatattaaaccggaacggcaaacagaatttgaaaccgggctggatgtaagcgtactgaatggccgcatcagcctggaagcaacttactataacaaaaagatttatgacgtattactgcgtcatgcgcttcccggttcttccggttatgctactgaatggaaaaacagtggtgacctgagaaataaaggaatagagctgggattaaacctgatacccgtgaaccagcccaatgtgcggtggaacagcagcattaactggtggcaaaaccgttccaaagtcaccaagctgatcattcctccctatgccattggcgcctttggtaactccctcggcactttttacctggaagaaggacaacccgccacacagctcaaaggcattgtaaacggcgacctgaagctgatcggaaatgctgaaccggatttccagatgagtttcttcaatgaattaaccgtgttcaaaaacttctccctgcgtttcctcatccactggaaaaaaggcggcgacaacattaatcttacacagctgctcaccgatgcaggagccacctcttttgattatgacgatgagatgaaaggcaccaaggcaggactttaccgccccggcgcaggcgatgcttccatttatgtgcaggatgcttcgtatgtgcgtatccgtgagatcggcctttattacaatattcccatgaaaaatacatccgtgctgaaagcaatccgtgtgggcgtatctgccaataatttctttacatggacaaagtacgtgggttatgatccggaagtatccaacttcggaagtaacaccattactaccgctcaaacccgcggcagtaacgggttatcaaccggagtggatgttatgccgttccctgcatctaaaagggccagctttcatgttggcgtcgatttctgatcattttccatctgcttaaaaacattacatatgaaaaagtatctttcaataacagcgatcgcttttttactgctggtgatgaacgcctgccagaaaggagagatcaacagtttgaatacacccgtggtaagcggcatcactaccgatccttccaggagcgacctgtttaacctggtaaccggcgccgaatccggcatgcgtaacagcctctctgcttacctcgatggcaccggtattattggccgggaaatttaccgtttctccggtgcagaaccccggtacaccaccgatttgctgggcggcggttccaaacagctggacaataacaccttttaccttaccaacccctggtcgggccgctaccaggtagccaggcagtgtttcattttactcgatgccatcagcaatacccgcacggaagtagcgtctgatgtgcaaaagaaagcctttacaggatttgccaaaacgctgatcggctaccagttgctgctgaatctcaacatgacaaataccaatggcgtacgtatccccgttcccactggcgctaccctgggacctgtgattaccaacccttcggtagtgatggattctatattgaaattcctggatgaaggaaaagccgatcttaccggatcggaggttatttttcctttgtcggatgggttcctgggatttaaagatgccgcggggctgattagatttaaccgcgccattgccgccagggtgtatacctatcaacagaaatggagtaacgcactaaccgcactcaatgaatccttcttcgacctgaacggcgctttaaacaggggcgtttatcatgccttttccaccaatggcggcgatcttgccaataccatgtatctcccgcccaatggcaacggggaaataagagtagcgcatccttcttttgctaccaatattctgccgggtgatgaccgcatctccaaaacatcgttgcggacttcttccgccagccagagtggtttaaccggcaaccgcgatgtgattgtatggacctccctgaacgcacccatcagcattatccggaacgaggagctgatattgatatacgcggaagccaagattcagacaaatgcattccccgacgccattgtggcgctcaaccgtatacgcacagcgcataaccttgcgccatatgccggtggcgctgctttaaatgcattaattactgaactgttgtataacaggcgctattccctgtttatggaaggacaccggtggatagatgtaaggagatataacctgttgggaacattgcctaaagacaggcctgatgatgatgtgtggccgaggtatccgttgccgcagagtgaaagcaatacttaaaactgatagtattatccataaagaagcgaagcgcatccaggatgcgcttcgcttctttatgacttatgccatggcccttctcttcatttccttcctgataagtgccagttcgcggcccatttgcccggcaatggaggtgttctcctgcgccctgcggatcaggtaaggcattacttcttttacgggaccatagggcaggtatttgctaacattataaccggcatgcgccaggttaaaagtgatgttatcgctcatgcccagcagttgtgaaaaacttacatgcggatggttatgcggcaatcctttttcgtggagcagcctggcggcaaacatgcagctgttttcgttgtgcgtgccaatgaaaaccgcgagtttatcgaggttatcgatgcagaattttacggcagcatcatagtccttatccgtagcctctttgcttggctggataggcgttggataattattctctgcagcgcgtttgttttctttttccatgtaggcgccgcgcaccagtttggcgcccagcaggtagccgttttttactgctttttccagggatacctgcaggaaagggtaacggtcgtggcaatacatctggaaggtattgtacacgattacctttcctttgttgaataacgacatcatttcatccgtgagcgcgtctaccgggtcctggatccaggattcttctgcatccacgaggatggctacgttatgacgggcgcctgcttcagcgatggcgtgcacacggttgcgtacacgggtatattcctcttgttcggcgggcgttaaagtttccttgcggtgtactttttccagcagatcgaaccgggcaaaacccgtgacttttatagcgatgaaaggaatatcgggtctggaggcagcatattgaatggcacggatgaattcaggaacagcggcatcatagctttcttctccttccatggcttccacgccatagtcgagtgccacccctacatgatagttacccagttgcagtgcagtggtagctgcttcttccagggtttcgccgccgcagaactgtgagaaaatagtgcttttaataattccttttatgggtaatcccagtttaaaggcgatgggagtcatcacggcgcctaattttaccagccagggcttcccgatattactaaaaagaaagttggcttttttcagtgccttgtcggtctttgcctcaaatgcgatagcggtattatcaaatgataaaggtagctgcttttccatgggccgcaaagttagggtgcgtccggcttctaaacaaaaatcattataatatcagtatatctttttaacagcgttaacagatattgtctattgcttctcagaaattgtttaagcatacccttatgccgctgtttattttattacttttaggtcttttaagatacatacaaaattcccggaatatgctatttaaacctgatactatttcccgtagttttttcagccgctgttcgctggcatggttactaacgggcggaatagtgatcaccggctgccagacaaaagcaccggaaaacgcacctgtgaacctgaaaacgccgggcattgaataccagacctataaaggcgccaccggccggcgtactgctattacgctgcccgacagctcccgggtaatactcaactccgcttctgtactggaggtgcccgccaattatttacagggcaaccgtgccgtgatcctcgacggcgacgcattctttgccgtagttccatctaccgatacttttacggttaccagcgataaattaagggctactgtactgggcaccgaattcaaaatgcgttcctttgccagtcagcatggcgctaccgtataccttctcaacgggaaaatccgcgtgggaaaatcctatcactctgccaccgataaccagccggaaatactggaacggggacaaatgatcctggccaataatgacatcgacctgatggaaaaagaaacctatcatcccgaagaactggaaacctggttatctgatacactgcggatcaataatgccaatcctatggcactttcccgcacactggaagaatggtttggcgtggaagtggaaatgaagggggatgcttccaaagcaccggcgattacagatgccgcgttttttcatgcttcattggaggaggtgctgaataaccttggtgaacaacagcatttcaaatataagatccgcgataataaagtggtgattactttttagtataggctttaacgttagatgcttttcgcggaggttgtcttgagcggaggttgtcttgagcggaggttgtcttgagcactgattacactgattatgctgattatcttgattatcttgattttacttttttgattttataaggatttggggagatggaagcggagcaggatttggttttataaggatttggggagatggaagcggagcaggatttggttttatagtgatttggggagatgggagcgggtttggggctggtttagaaatggattttcctgttgaaggaaaagatggtggcatcgggatttttctttccctgtatgaggtcagtgatgatattggcggccatctggctgaaagtgatcccgttgccgccgaagcccagtgcaaaaaaggtatgcggcataggtgcgaaagggccgataaacgggagtccgtcttctgtagcgccaaaggtgccggtccatttaaactcggtgtggaagcgcagctccgggaacttcctccgcaggtctttttcgagggcctttgctttttggtggattagcttatcccggcggccggggttataaaagggctcatcacgcccccctaccattatacggtgatcgctggtagtacgcatgtagaggtaaggggattttgtttcccatatcaggcaatcctgataccactgttcttctgcgtgattgggttcacttgcgatggcataagtggagtttaatttcagcagcggcgttttgatatattgcagcacctcatatcctgtggcaatcacgaggtaacgcgccgtaacctggtaccccagtgaagtttttaacactacgctgcgaggacggaaatcaatatccaccacggcggtacggtcaaatacctgcgcaccatgtttgatattgtgctgatgcaaggcatgggtaagcatatatgcatctgtttgcgcggcggtatgggaatagatggcagccggcgcatcaaagcccatctttgcttttactttcgccgcatcccaccactccattttcagccccagctcccggcgggcttccagttcttccgataatttttttatgtctttgaggtatgaagccaggtacagactatgctttctttcaaaatgcgggaaatgcagggctttgcaaatctgctccagctcgtggatagcagccacagacagttcatatgccctgttggcatggtaagtacccactttatcccgtagtaccgataaaggcgtatcaatttcatactgcaacagcgaggaactggctgctgtgctgccaaggccaatggtgcgggcatcggctaccacacagggaatacctgcgtttgtgagggcatgggccgttaaggcgccggagatgcctccgcctatcacggccacgtgcgtacgaatatcccgttccagccagggataattgtatgggaggccgttacggatcaatgaataagggtaacctgactgaagatccatatttattgattttacaaaagctgcaccagaaattcgtatcttctgtcagcaaaattaactgtcatgaaaacactaactttctcaaccggttgtttactgatggctgtgagtgctttttcccaaacggcgccctgctgccatacagatgccatcactgaatttgctgcactggccagccaggaagaattccgcatggcgcacaaagatccgctgccatttacctaccagggaactacgggcgctgccatcacctttcctgctacagatggaacacctgcgcacggctttctgttcaaagccaaagaaacctccggtaaatacctgttggtgtaccaggaatggtatggcgttaacgactacatcaaaaagcaatcggaacagctgtacaacgacctcggaggcaaagtaaatgtgctggcagtggatatgtatgatcagaaaatagctaccaaccgcgaagatgctgctaaattaatgcagggagcttccagggaaagattacaggccattatgcagggcgccattaactacgccgggaaaacggctaaaatagcttctattggctggtgcttcggcggcggactctctttgcaatcgggtttactggctgggcctcaaaacgcaggcgtagtgatgtattatggcatgcctgaaaaagatgtgaataaactaaaaaccctgcagggacccgtgctgggatttttcggtaataaagacaaaggcattaacccccaggtggtggatgaatttgagaaaaacatgcaggaagcaggtaaaacgctcacggttaaacgttatgatgcggcgcatggctttgccaatccgagcaatcccattttcgacagcgccgctactgcggatgcatatagtcatgtggtgccattcctgaagaaaatattttcattgtaagtgttaagcggagggaatgttccctccgctcaactatttttatttgccgccgagcctcagcagcaattcttttgttttcctgataccttcttcttcggataatttttcgccttcgtactcaatacccatgaaaccattaaagccggcgtccttcactgttttgaggatacgggtatagtcgatggttacttcattgccgttggcatcgaagtcgtatgtttttgcgctcacgccctttgcaaagggcatgagctctgccactcctttataccggtcgtattcttcgaggcaggtggttttagcccaggcttccggtgtattgctttccggtttgctgcgtttaatgcagaagttaccaagatccggcagggtaccgcaattaggcatgttcacggttttcattacgccgctcagccattcgccgttggatgacatgccgccgtggttttccacgatcacgttgatgtcgtgttcctttccaaaggtggccagtttagtgaggccatccgccgccgctttggccacttcttccggagtgccttctcccgctgcgtttacacggatagcatgacaacccaggaacttcgctgcttctacccacttgtaatgattttcaactgccttcattctcttcttcacatccaggtcgcccatttcaccttccccgtcgcacataatgagtacgctgcgaacgcccaggtcgtcggcgcgtttcttcatttctgtgaggtaggcctgatcctttgctttgtctttgaagaactggttcacgtattcaatgccttcaatgccaaattcattctttgcgcgggaagcaaaatcgaggtgattcattttaccggcaaacaacgctttatggaaggaccattccgccaatgagatcttaaagaaaagttcgcgggcagtggcttcaccgggtttggcagctgcggcgctgtcgccttcacttttagtggatttcccctcattacaggcggccagtatagcgggcaacattcccattcccatggtgtacacgcccatttgacgcaggaactgcctgcggttgttaacattactcatatacgtgggttttaaagttcattctcctaaaatattcatttacacgggggaaagcaagttaaaacgtataaattttaagagaagaaaaaaaagagcagttgaaaagggaagatgatcgcaggccgctgctataggcagactgccttagcgggagatataaatacagatagctcgccacgctgataaaaatcagcgtataaccgtgacagttactcctgcctatttttaattccggtttcttgttgaatacctttttattttatgtcatccgccaatacagccaggactccctgcaacaccgcttcgtgccgcatgatgcggaaatggccatcaccggtgatgcggagcgattgtatggccgggtattgctgcaggtagtcatctatttccgtggcttttgcaagggtatcggttgtatcataagccatccatattttatcggctttgatatgattgatatagcggtgcaggtccatttcagcaagatcttctttcagtctttgccggatcagttgctgcagcacgggcattaccaccgggtggatacggaacaggcggagtgcttcattaaaaaacacgggagcgctcaatgccgtgctgagcatcagcaggcggggcacgtgtacatttttgcgggagagtgtgagtgcggcattgagtccgccgaacgaatggccaacgatagcgtgcaggggtccttcctgttgcatcacctgttccagtacatgcatccattgtaccaggttggtgcgtttgcccccggagaggccgtgtgccggcccatcgtaggataccacctggtagccctgttgcaccagtgagctgatgagttgtttaaaatggagggggctgccaccccaaccgtggagcagtaatactttggggcctgtggttccccatcggtaggtggttactttcaggggagcgttatcaaacggatagctggttacctgcaaatgttgcaataccgcctgatcgcggaactgctgatgtaccggccggagcttcaatgcgggcggtgtgcagtacagccggtaaaacagtttggccgtggtaaccgggaacgggcggctcatggcggataatatcgcgccggtcatccgcagtgacaatggtaaaacctggtgttgcattatagaccgattggtttatttttagaacaaaaaaaagttaaagagaatgctgcctgatttcttctcttaacgcttccaataccacgagcatttgtttattatgtccgagcacgctgcttacgagtatagcgccttccagcatggtaaacatccggatagcaaatttccgttcgtcccagtctttttcaaactcgccatgctccttgccatactgcaccattttagcgatgcgcgactggtaatagagcaccagctcactcacctttcttttcagccccggattagtatcatccgcctcgacgccgaagttgagcatcgggcaaccgccggcgatcttttgttcctccgggtagcgggcataatactgaaacagcgcctcaaatttcccggccgaagtattagccgtggccgtcacctgccgcaggttcagcttctcctcttcagcgatataatcgaacacctccatcactatttcctctttggaggaaaagttcccgtacacgccgcccttcgccaacctggtggctttgaggatgtcactgatagaagtaccggccaccccctttttattgaaaataggagcggctttttctatgatgaactggcgcgttttttctgctttacccatgtgaggaccaaattagaccaattggtccattccaacaaatatttctcccgcgcggattttgtctttctcaggattacgctgattttactgattacctggatttttacttttggattttttttgatttttagatttttattaaacaatagttaagggagataaaagcgaatatccgcttctatctcccttaatcctttataaaatcccaaagtaaaaatccaggtaatcagtaaaatcagcgtaatcctgagaaagacaacatccgcgttagaaattgaagatgcgttcaatcgcaggcgcataggccgccccaatggggatgggaatgtttttgatgtaaagggagttgcggtcggcgcgttcaatttttttattggctacaatgtaggagcggtgcacacgggtgaaggagccgatgggcagcaggtctaccgcttcctgcatggaaaggcgggagatgagcttgcggtcggtgaggatgaagttcacatagttgccggcgctttcaaggtaaaggatatcatcgagtacaatacggaattgttcgtagccgcttttcacgaagatgtagtctgtttgttccttgcctggggcggggccattttgttgcttcagttgcagcaggttattggctttgttgcaggctttcatgaaacgtatcagggaaaagggtttgagcaggtaatcgatcgcgtcgagctcaaagcttttcaccgcatgttctgaataggcggtcgtaaaaaccgtcatgggcggatgagggagactggataaaaaatccaatccggatatatccggcattttgatatccaggaagagcaggtctactttttctttgctgagaaagtcgatggcttcaaaagcattggtaaaaaaacccttcatttccaggaagggaaccttggcagcgtgatttttgataacagccagcgccaccggttcatcatctatcgcaatagcagtcatctttggctattttacgggtaagcaatacagggatctaactaattttgccgagcaataatctccgggcttgctgccagagattctggtactggccgttttcgcggctttgccactcttttacgagggcgtcggcctgttcgcggcgcaggtcgcgggtagattcaaacaggtggtccaccgtttccttgtcggctgccagtgcggcggcctggtagtgttccattaattcctggctggtatctgtttgcagccttgcggaggctacgccctgggcggtggcggcagccagcttttcatcgtattctcctttgggcatcagtattttgctgagcaacggcattacttcaatgagggtaatgataaatacaatgaggcgataacgttgttttaccggcggatgcgtttcggtgagctcattcagggcttctatctgtgccaggaatccgttggtgagggtaccgacatatacggattctttcacgctgtcgacgctgtgcatacgggccatttgtgcctgcagctgttgctgctgcggctcccaggctctttgcatggcctgcagctcctcttctgatttgaggtaagccgatttttttacgcgggcaatgtccgactctcctattctgccggagccaccggtgccatcggtttctttgatataaccatctttatatactttcagctccgcggttttttgcgccagctgctgtttgccctgatcaagggattgctgcagggtggccatctggccggcattgagctttaccagctgcgcccggtaggcatcgagctttgcctgcttgccaagttccagctgggtatcaatatctttcttaaataacattaacaccaccggctgggaaataaacaaacctatggtaacggcgaggactaaacgaaatattaccggcatcacttttatgttgccgttggtacgggacatggcagcgatgagggtacggtcgaccgataaaatagcgaagccaaaaaacagcgccaatccggccaccaccatgtcatcgtttacgatggtggaaaagaaatagccccacgacagcgtagcaaacatccacgtaaccaatactgatacaccaatgatccggtaccgctctttctcggttttacactcctgcaaaacatcggcatcagcagcggccagccaccacaaaaagcgcgtcatgccatcaggcccgggtaccacttcttcttcttttttcatttacttatttattaacatcaatagtcagatggataaaaaactcagtagccgtgtgacggatactcagctcgtgccggtgcggatacaataaatttagtctttcttttacattattcaaaccaatgcccattccctccctttccggatcattttccgggcggggatgcacactgttatacacatcaaagaagatctgatcagtcgtacagctcagggaaatcacgatgcgagagcgatgccgcaggctgatcccgtgcttaaacgcattttccacgaaagggatcagcaacatcggcgcaatttcatgctggcattggctttcatctatatttacctctatcaggatatcgggcgatgacaatacgcgcaggcgttgcagggcgatataattttgcaggtaagccacttccttatccagtggaattttttccaggtggttatcatgtagcataaaccgcatcatatcacccagtttctggatgccttcgctggtgcgggcagcctcttcctggagggcggttccatacagcgtgttaagggcattgaataaaaagtgcggattgatctgggaacggaggaagtcgaggttggcagtggaatgcccgagcgcctttttcagcgttaccaccgtgttcacctgcttccggcggcttttaaacaacagccagcaaacaggcagtacaatgcctgccgataccgcgatgccgataaaagccagcgccacaaaccaaccgccgtcgcggtgcaccagtgcgcggcatatcagcgccagcaacacgttgcttcccaggatggtgaaaacaatatcccggatcaggaggcttttattccggtgagtgtcctcgaaagcgggaaatacctggtaacggagaataaagaacacggcaatctgcgaaggaccaaagaaaaagatcatcagcgccatatcccgggaatcggagaacgacaaacaaaacaataccacaaatacgccggcagcccagcaaatttctgtgagcatctgcctgaaagccatatccgttgcaatgcgcggatacagcatactcaccagcgctttccggaaataataatatgccacatacagcacgccggaaaagaccgtagtaatgaaagctgtctttgcaaaatacatatgcgccccccgcaccgtgtcatatacgcctaacaggtagccgttgtaataggagttggcgaccatcatcatcgcgaaataaaacaaccctaccgggatcagcagcaatatgccacccagccattttcccttctccaggaactccggtacaatgacaaagttcaccagcaggaaactcacatataccagtgtaacccgtcccattgagggcagcaggtaatgaatgtaataatcgaatacctggtggtaagtgtcgaattttctaccatagatgtcctgcaattcaaatacgttatacacaatgctgggatataggatcgaaaacatcagcaacacaaaaatggcggttacgatgccaaattcaattttcttaaattgattcataaggttgatgtatttagggcaataatagcatttgttgccatgcagcaggggcaaaatgggatgaaagtagtgtaatccggtatgaaatgggctttgacagtaagaattataataaatcggtaatctttattattttcatcgcctcaacaagcccgatatgagcacttccaacagacgtaaatttttaggaaccgcagcagcgcttgccgctggtactgccgctgccgcagcaatcccctcaacaaatatggaaaagaaatacccgattgtgcatcatgtgttcttctggctgaagaacccggattccaaagaagaccgcgacaaactggtggccggtgtaaaaaccctgtcgaaaattgaaaccgttcgtgacctgcgtgtaggcgtggtagcgagtaccgaaaaacgcgatgttgtggataacagctggggcgtatcagagctgatctttttcagtgatctcgccggacaggccacctatcaaacccaccccatacacctggagtttattaaaaactgtagtcatttatgggagaaagtaatcgtttatgatgccgtagaggtataaaaaaatatcatggcaacggaatactggatgagcgggccggtagaaaacataccggcattattgcaacccgtggcgcatgcgttattgcaggccaaccaggaaataaataccctgatgcaggatttcccggaaacacttttatgggaaaaaccggcgggactggcctcgccgggatatcatcttcagcatgtgagcggtgtgctcgaccggctgtttacctacgccagggcggaagcgctcagtcagcagcaatttgccgccctggccggtgaaggtaatccaggcgccaccctccacgatttgctggatcatttcaatgcacaggtacatcaatcgctgatgcaattgtcggccaccccggaaaacaccctcaccgatttccggggcgtgggcagaaaacaactcccctccaccgtattgggattactatttcatgctgcggaacacaccatgcggcataccgggcaactactggttacggtaaaagtactgctggaaatgcatgcccgttgaaagcagagaagcattacccttcatgtaaatccggattgtttttatccgtaaaactataaattagccctatgaaacgcttattcctcctttccctcgtgttgggttgttataccggcatgcaggcacagcaaacgcagaaaccacctttacacggcaaaaactggatggccgtaaccggcaagccactggctgcaacagccggcgccatgatcttccagcaacacggcaacgccgtggatgccgcctgcgctatgcttgccgctacctgtaccatgtgggatgtgctcagctggggcggagaaacacaggcactcatatacaatccgaaaacaggaaaagtaattgccatcaatgccctgggcgtggcgcctacaggcgctactcccgccttttataaaggaaaaggatacgacttcccacctgaatacggtcccctggcagcagtaacaccgggaactgcaggtgggttgtgctacatgctggcagaatatggcactctcagtttaaaacaggtattagcgcccgccatggaaatggccgccggctacccgatagaagcacaaaccgccaatagtattgaacgcgggaaaaaatatatcaacgaatggccttacagcaaagctgttttcctgacacatcccggcgaaaaaagagaagccccggaggcaggagaaatttttgtgcagaaagacctcctcgctaccctcaccaaaatggttgaagccgagcaggaagcactgcgtaagcataaaagccggaaagaagccattatggcggcatacgaccgcttctacaaaggcgacattgcgaaggaatttgtgcgtggctgccaggagcagggcggcctgatcaccctggaagacctggcccgctggaagccggtggaagaagaaccgctgcatattaattacaaaggcatagaggtgtacaaactgcaggaatggacgcagggacctatgctgctgcaaagcctgaacatcctggaaaattttaacctgaaatcgatggggtataactccactgaatatattcatacgttgtatcaaaccatgaacctcacttttgcggaccgtgatttttattacggcgatcctgcgttcaataccaatcctgctatcaaaggattgctgagcaaagaatacggcaaggcgagagcgaaacagatgaatcttgcgcaaaatgatgccaatgcaggaccgggcgatccctatcctttcatgggcaaaaccaatccttacctgcatttcctggaggagcgcaagcagctgacagataccagcaacggccgcaagcccggcggatttgttcccaaacatgacgccactatgctgcagcatggaaatgcggaccagcaatatgctgccaatgccttgtcaacagagggagatctaaatcagctgtatgccggcaatacacccgacagcgcctatatggaccggctgtggcgcggcaccaccagcgtagaagcagcagataaagacggctgggtagtatctatcacgcccagcggcggttggctgcctgcctgtattgccggtaaaacgggtataggaatgagccagcgggcgcagagttttgtattggattctgccatttgcccttttaatgtaattgcgcccggtaaacgtccgcgggtaacgcttacgccttcgatggcgttgaaagacggcaagcctttcctggcttttggtgtgcaaggtggcgatacgcaggaccagaacctgttgcagtttttcctgaacgtggtggaatttgggatgaccgtgcagcaggctacagaagccgcgaatatcaataccaaccagttgtggttgtcgttaggcggtactaccatcaaagacagggagccgcggccgggaagcattctgctcaataataatacctccgaaaaaacacgcaaagccctggagcaaatgggttatcacctcactttcggagagcgtaccagcggccccataaacgccatttacatggatcgtgtacacggcagtttatggggtggcagcagtaatcatggagaagattatggaatagggtggtaagtaaattgctcccgggtccatacttcatgaataggatctccttttgagcttttgccgctgtggtcccagttgttgccgtttacgctgcctttaaaagacagttcagcgccaatacgggagctatcgcgggaaaagaactcgattttttcggtgtaggtaccgttatcaaaagtataggtacctccaccggaaccaaagaactcgcctgtttcctggttgatggcgacccattgaaagcgggtgcccgtcagtattttcatggtgcgcctcgcactgttgggaatgggtgtcatcttaccttctctttcccgtgaagtaatttgccagctgccggccaacgggccggtgccatcgtcgatacgcgtccactcctgttttccaccaccgggactgctggtgatcagctgcccgttttccatgcctaccggcacggttgttttttgccctacctgcgaggcattggccgtgttaaaaagaatggctacatctacctgcgtgtcacccgcctgtttccaggttcctccatatgaagcaatgaaacgctggttattgtaatcggtgactgtaaaccagttgggcgtaatcagcaacacgctggttacatcgccggtcgctgatttccaggcgcctaagggtgagtcttgtgcgctgagtatacccaggcaggaacagcataacgtaaataacaggagtagttttttcataacatagcatttgtgtacttaagataagcaaacaaacgcagtaattaagcggtttctccctgtggtatgaacacgttttatttatacagatgctggtcctgtatataatcaacaccctgttttttgagataagcgattccccattcgctgacaaattcatacaggggagccagtgattttccttcggtggataagtagtattccacgcggtatggcttttgggtaatcacattcttttcaatcagcttatcgcgttccagttctttaagctgctggctaagcatcttttctgagatgcccggcaggttatctcttatttcagcgtaactttttttagtaaagtaatgcaggtggaagaggattaacagtttccatttccctccaataaatccgagtgttacatctaccgggcaggtgtatgttttattgttcagtgtgatcatcatcaaccgtgtaaagtggtttcgctatgcttcttccagtacgcgcttcaggatattcaggtacccgatatgttgttccgcataggaactgctttcggagagctgtgcccaggcaatttgccgttcaagggcgatattgatcaccggcttattggcttcttcaattacgccttcatctgccagctggccaaagccggcggcaattactgaagcatccaatgtgaaaataaagtgctggtcatcaaaagcaggatcttctttcatacgtatgatcagatcccggtccagcagcgtttcgttatactcttcaaaggccatttcccctaccgattcgatggtccattttaagcattcaatggtaggcgtggaaggatattcccggcgccattcccggaatgaggcaagcccggtgtctccttcatctgatccgaaaggggccagttcatcagcgggatcccagaaaaagtcttcaggtatcagggcaatagctcgtgcatgtgcatgatctttatctatgccatagatttcgtccttcataagatatgttgttttaaattacgctttaccccacccatcggcatttgagcaggtttcgatgccatgccttgtataccgctcaaattcttctccaaataattcctggtataccatatacccgataaatcctacaatttctgcttctgcatcgcaggtggcttttgaaggattttcgtcgatcatttcatagtacgttttccccattcctacaataaaacacctgcaataaaggaaaccgtcatctgatccatcggtatatgcatggatatcttcccggtcgatctgaaataatttttcctccatgatgtgattaaaccctgtcagctcttccttatccaattggagcaggatatcccggatattattggtaataacgccgtatacttccccggtcaggtcttcgatcaataccgcatcattggttttcaatgctgtattgcgcatatcccgtaatgccggggatgcagcccacgcttcttcaataatctgccagaatttaaattcattcataagagtagcaattaatgatcattaagaattaactgtaagatatacataggaaacgcagtgtaaatgcgtagtaaaaaaagcggtcagtgatccggtatcccttgaaaatacacaataattttctttcttttctacccatctgctaaaactttcctcctgtataaattattttattattaattccctgtcccctaaatttaccgggttattgtttttgtgagggtacaaaacttccagctttgccagacatttccctgaatgacgaacatgatttgctgcagaaagttgccatgggtgacggggatgcgtataccatcctgttcaggcattacagcggacaggtgtatgatgtggccatgctttacctgagagacagcagcctggccagggaaattgtacaggaagtttttatgaaggtatggctgaaaaaagccgatatgtcccacataaaacagtttaaagattacctgtttatccttacccgcaaccatatttacgacggcttcaaaaagcagctggtaaggctgaaagcctacgatttccatctgaaaaaccagccggaagcacagaatgataccgatcacctgttgctgcaacgggaatacgacgccatcctggacaaagccgtgtccggtctgcctccggagcgaaaaaaggtgtacctcgcccgtaaacagggctggagcaacgaggaaatttcccaacagctcaatatatcagtacataccgttaaaaagcaaatgagccttgctatgcacgctgtacgggcttttgtaaagtccaggctgcaaaatgatatcgttcccttcctcctgtttttaatcctcttccgcaaataacatcttccccgaaaaaaaaatttcatcccggatactccttttttaccggttgatcgtctttaccccatatcacccttccaaaatcgctgataatgtccataacggaagtacagttattgcttgaaaaatataagaatggccggatcagccaggaagaactgctgcgcctgaaagcgatggtagccggaaacgactacgagccggaaatcaaagcagatatcctgtcggcactgtacaacagcgggacgccgcaaagcggtctgtctgcggaagatggtgaagccattttacaaaacatcctgcaaacaacgcctccccgcgctgccggcaatacccgcagaataatctggtatgcagccgcagcaaccttgctgggagccacgctggtcacaggcgcactttatatgaaacggcagcaacagcccgttatagtggctgctccgaaagccaatcccctggcgcccggcaccaacaccgccgtactggtactggcagatggtaaaaccattccgctggacagcgccaacaccggcgcactggccaaacagggcaacagcagcatcgtaaattcagtgcagggccttgcctataaagcagaaggcgccaccacggaagtggtgtataacaccgtagtaactccccgtggcgggcaataccagcttaccctggctgatggcactaaagtatggctaaacgccgccagcagcatccgcttccctactgcattcagcgggaaagaacggctggtggagatttccggggaaggttatttccaggtagccgccaatgcgcagcaaccattccgggtgaaagtaaaaggcaatcctgatatggaagtaaatgtgctcggcaccagcttcaatatcatggcctataccgatgagaaaaacattaccactaccctggaaagcggcgctgttcaactggtgcatggcaacatccggagcgtgctgcaacccggctacggcggcagcctgaacaccggcgatgccgcattcaccatcgaaaaagcagacctggaacaggcactggcctggaaagaaggcaaattcaggttccgtaataccagcatacaaaccatcatgcgccaaattgccagatggtataatatagaggttacctatgagggtgatctgtcggatatccgcttaacagggatcatttcccggcgggaaaatgcagcttctttattaaagattctgtcaacaacaaaacgggttcactttgatattaatgacaaccgggtcgtggtagcaccatacgatcctgagcaatagacgctatttgtccacttatgaattgatcatttttaaatttatttaggttatgaagacgtaaataattccactgccggttgtaaaaaaaaaccggaagcagtgcaatgctcccggctatagaaggcaacccaactccctgaatcatttagaaaattgaattattaagccaacaacacaaaagtatggaactacttggtacctgcaaagtccccgggaaaggaggacgtatgcaaagaaaattactgttgattatgcgattaactgcaatactgacactggtattcacccttaatctgagcgccaaaaccttctctcagtctgttaccatcaaagggaaacgtcttcccctttacgatgttttcaacagcatcagccgccagacaggttatgaattcatttatgatgagaagctgctggagaaagcgccgccggtaaatctgaatatgaaccaggcctccctcacagaggtgctgaatgcctgtttgaataacaaactgtttaactacaacattgtagataaaacaattgtaatcagcccgaaggctaaagcaatggtgcccgccgccgcggtgatagctgccatcgacatacagggcaaagtgaccgacaccaaaggtctgccacttgtaggcgcatctatccaggtaaaaggcaccagcaaaggcactgttaccaacacccagggcacctttaccctggccgccaatcccggcgatgtgctgatcatcagcatcataggatatgaaagcaaacaggtaaccgtagggaatgatcccaacatccaggtaacgctggctgtacaggacagccagttaggcgctgtagtggtaacggccctcggtatcaaaagatccgagaaatccattacctattccgcccagcaactggatggactggaacttaccaaagcgaaagatgcgaaccttgtaaatacgctgaacggcaaagtggcagggttaactatttcttccagcgcttccggtgtaggcggttctgccaaagtaatcctgcgcggcagcaaatcaggattgggcagcaaccaggctttgtatgtaattgacggtgtgccgatgaacaacaccatcacaaaccagccgggaagtatttatggtggcagctcctcttatgatggcggcgaccctatctccaacctcaacccggaagacattgaaagtatctccgtactgaaaggcgcatccgcagccgctctttacggcagccagggcgccaacggcgtaatcattgttactaccaaaagtggtaaagtggggcgcactactatcaatatatcatccggattcaatgttagccaggctgcctataagccaaagttccagaacaactatggccagtcggccgacccaaccaccaaaagctggggcagcaaaatcagcggcgcaaccgataatgtatccgatttccttcaaacaggacgcaacttcaccaacgccatcagcctggccggtggttctgaaaaagcgcaaacttatttttcttatgccaatacctccgcgcgaggtttagaggcaggcaataaactcggtcgtcacaacctgagcttcaaagaaaccggtcactttctgaatgataaactcaccgcttctgcagatgtgaattacatgacccagaaaattgacaacacgcctttgtccgggttttacttcaaccccctcaccggtttatatcttttcccgcgcggagtggatatcagcccttaccgggaccagtatgaaattcctgatccttcccggaataacctcatggtgcagaactggcctttttcagaagatgtgcagcagaatccctggtggatcctcaaccgcaacaccaattcgctttcgcgcaacaggatactcgccaatgccagcctgaaatatgacatcaactcctggttgaatgtacagggaagaggaagtattgaccgtatgaatgatgtgtatgagcaaaagatatacgccggcactcaaaccacgctggcctccaagaacggcggttataactataccaacaataccactacgcaacaatacggagacctgatcgccaattttaatatcccggcaaatgattttcattttacgggtatcgttggcggtagtatccgcgatgttaaaacaaacggtatctatttcgcagcaggtcaggaaggtttatatctcccgaatatattcaccatccagaacatgaaaacgatcaacgcagcgaactccggtagctcacaggagaaacacagccagtggcaatctgttttcggaagtgtgaatatttcttacaaagactgggcatacatggatctgacggcaaggaatgactgggcctccaacctggcgtttaccaaccagttatcttacttttatccatcagtgggattgaatgtaatcctcacccaactgcttaaaatgccagaggctattacctacggtaagatccgtggttcctatgctattgtaggcaattctccgctggcctaccagagtaatacaccggataacctgatcaataccggcggtaacgtaaaagtgaataccacagctccattcagggatctgaaaccggaaaaaacaaagtcactggaactgggtacagaatggcgctttttcgacagccgtctgagcgtggatctcacttactataaaaccaataccactaaccagaccatggaaattgccgcacctaatgcaaccttgtataacacctactttattaatgcaggtgatatccagaaccagggtgtagaagccatgatacggtatgatgtgttgcgcgatacaaaactgaagtggaatactgctttaaactatgcagtaaatgacaacaggatcatttccctgtcgccgtttgtagaccgtttcagcctgaccggcgacggcaccggcgccaactacgcttcacaatttaaggtaggcggttcgtttggcgacatttacggtacggtgttaaaccgtgatgcacagggacgtgtgatcattaacaatggcgctccttctctcgcaggcggccagatgcaatatcttggtaatgccaataccaaatggcaattaggctggaacaataattttgcatacaacaactttaccttatccttcctgatagatggtaagtttggcggacaggtaatgtctgtaactcaggcaatgatggacggatacggcgtttctgctacttccggccaggcaagggatgccggtggcgtaaaagtaaacggggcagatgccaatggcaatccggttacctctgtggatgcagagaaatggtacaatgtggtaggcggcagaacgggtgcttccggggaatatatgtacagcgctactactgtaagactgagagaagcatcgctgggatataccatcccgttgaaaagcaatgcagtgaaggcactgaaggtatctgccaacggccgtaacctgttttacttctctaagaaagctccattcgatcctgagcaaaccatgtctacctccaatggtctgagtggtgtggatgtatttatgttacctgcttcccgcagctatggcgttactgtaaatgccactttctaatcatttaccgcaaaactgaaaacgatgaaactgtataataaaatgaagcgttacagatctggtttactggtggccactgccgccctggtaaccgggatgagtgcatgtaccaaaaactttgaacgttataataccgacaataccggcgtaacggatggtcagctgggacccgattttaattcactggggctgtaccttaaatccgcgcagatgtcgatcctgaacttttccggcggcggggatcccaactcttaccaggtacaacagaacctcaatgccgactgtttttccggttactttatgacacccaatccattcagcagctccaataatactaattacggcctggtgccgggctggaatggggaagcgtataaagtgggttatctcaatgtgatgtcgccggtagtgaagctgagggcaagcggcatagataaaaacttcccggcagtatgggcagtggcgcagataatacaggtaaccgccatgagccgtgtaaccgatatttacggccctattccgtatagccgtgtaggtgaaggcctgtcatctgttccatacgacagccagcaggatgtatacaagcgtttctttgcacagctggacaccgcaacagaaagtttgcgcgcccaggttaacagcggcacgcagctacctttcgacttttccaattttgatgttgtttacaacggcaattttgcgcagtggctgcgcttcgctaactcgctgcggttacgcctggccatgcacatcgtaaaagctgatccggccagcgcaaaaacggaagcagagaaagcgctgaaccctgccagcggcggcatcatcaccgataatgccgataacatgaccgtaaaagtaaccggcgactttaccaatccacttgttttcattgcgaaaaactgggcagacatccgcatcggcgcctctttgcagtgctacctcaccggttttaaagacccgcgggtttcaaggtacatggacaaagccactgatcctgccaccgggcttaaaggcgtatacaaaggcatccgtatcggtagcctggtagataaaccgaaataccagacctattcttccttaaatacagaagatggcgcttctcctgcttttaccctgaaaacgccaatgcaggtaatgactgccgcagaagtgtatttcctgcgcgcagaagcagctgtaagaggctggagcaatgcaggcggtagtgcgcaacaattgtatgagcaaggagttactacgtccatggcgcagtggcaggtaagcgctcccggctatcttgccaatgattcaagtcatgccgatgcttacaccgatcctaagaatgcagcgaataatataggcagtccatcttccattactattaaatggaatgaaggcgatgatgtggctaagaaaatggaacgcatcattacacaaaaatggttggccatgttccccgaaggacaggaagcgtggacagaattccgccgtaccggctatcctaaattgttcccggtagtgaacaacaatagcggtaataccattgacgcggccatacagatccgcagactgccattcccgcaaaatgaatataacaccaatcctgctgcagtggcggctgccgtgcagctgctgagtacaccggcagataacgggggtacccgtctctggtgggataaataaaaataaagagcatttaaggagatggccggtaaatggccggccatctcttctattactatctttaagttaacctgagcatacgtttgttataagagccaccagaccggaaaacccgtaaccaaaatttgaacccagatttcctgatcatttaaacattcattccattatgaaaaaacaatttcacccgttacggctattggccgtaggaatggcgtgcgccgccctgttttttaccgcctgtaaaaaagaaaacaacaccagcatttcaaccgatcccggcaaaatcgccaccggcgcgcatgtagaaaccgttaccaaagccggaggcatgtccgtttgctatgtggaagtaaacagcaacagtttactcaataccggcaagtacaccttaaccaccggcgggcaacagctgtttgatattgccattatttttgccgccaatatcaactacaacaccagtacccagaaagccgtgctgtacaacaatcccaacgtatccaacgtgctggccaacaaggctacgcaaattgtgcccctgcaaaataaagggatgaaagtattgctgtctattctcggcaatcaccagggcgcgggcttctgtaacttcaccagcagaaccgctgcacgtgcctttgcccaacagctcagcgacaccgttacgtactacggactggatggaattgactttgatgatgagtatgccgactacggcaacaacggcaccacgcagccaaacgacagctcctttgtgatgctggtagatgaactgcgtaagctgatgcccacaaaaattatctccttctactactatggcccggcagcatccaggttatcgtggggtgggaaaaaagtgggcgactttgttaactacagctggaatgctatttatggctcttattccgtacctaacgtagccggccttacaaaggcacagttaggccctgcggcggtggacattcagagtaccagccagagcactgccaattcactggccacgcaaacgaagaacaacggttatggtatttatctctggtacaaccttaccagcaccgataaacatgtgtacttctccggtgtatccagtatcctctacggcagtaatgttacctacacgccttaataaaaagaaaggagtcgtttataaaaacgactcctttctttttattcgatactcttctatttaatactgtcttcccttgccgataaacggaaccagtccttcgcgtaaggctttagcagggcggtagccgctgtgggcccccaggtgccggccttatacaaatgcagttctttcgccgggtattttttccaggtatccaggatgggcattactactttccaggcagcttccacctggtctgcacgcatgaacaaagtagggttaccatccagcacatccagcaacaatgcttcgtatgcttcgggaattgtttctgtataagattcctggtaagtgaaatccatctccaccggttttaatttcatcttcaaaccaggcactttactttcaaacaacaaacttatttccagctccggctggatactgatgatcagcctgttgggcgtgatatcgtctttaaaaattttatggggagaatctttaaactgcaccacaattacagacgattgcaccggcatggattttcccgtgcgtaaaaagaaaggcacgcctttccaccggtcgttgtcaataaataatcttgcagccacaaaggtttccgtattggaagcggacagcacatgttcttccttacggtagggcaaacgtggcacaccgtgtacattaccggccgtatactggccacggataacgtttttcagcacctgtgccggtgtatacggcctgatgtctttgagtacttttactttcgcatcgcggatcagttccgactggtaaaactccggtgaatccatcgcaacaatacacaacagctgcagcaggtgattctgcaccatatcacgcagggcgccgctgccttcgtagtagccgccgcgttttcctacgcctacttcttctgccacgctgatctgcacatgatcaatatattttttattccacagcggttcaaatacatagttggcaaagcggaacgccataatgttctgcacggcttccttaccgaggtagtgatcaattcggtagatctgtttttcagcaaaacgttttgtcaggaagcggttgagttttttagccgtatcaaggtcggtgccgaagggtttttccactacgatacggtccaggccatcgcggttgcaaatggtgtgcttgtataagccttccgcaatgatttcgataaagcgtggcgccactgcaaagtaaaagatgcgggaaccgttttgtttctgcttctttccaaacgcatccagcttttctttcaggccggtataggtttctgttttcaggaaatcgccctggaggtaagagatatttttagcaaatccttcccattctttcggatctgctttgccgttgcggctaaactcattgatccctgccagcaggtcgagtttaaaggcagtttcatcttcgggcaggaaatccacgcaataaatggtgaatacaggcggaaggtgtttatcggtgtacagattataaagcgcaggaatcagttttcttttagtcagatcccctttggcgccgaagatggtaatggcggcggggagtgtttttccagttttcatctaagcatcggtttattcccctgtaatttaagcatcattcctgtaatcttttcatccatttttggatgccggtggattcaaaagattaccggttgcgggccagtatggcggcgcaaacggccaggatacacgtcattggcgtgaagatcagctgctcccatttattgatggagatgaggttacccagggtgtttacaaaaaataaaagacacatcagccacagtaccaggcttaaaaccttgccattggcgggcagcttcaatagcttccttttccccagcaccaccagcaggaaaaatacattcaccagaacagagatagcctctaaccggtacatttccattggtgacctcagtcttcctccccatacaagggaataaggtaaaactttcgccacgatcagcaggtgaaaaagaataagcagggagaaaatagtgatcatcactatccccgctatttttggcatacggatactcataaagcgattaacttgcgtcaaaggtaagaatagcggcgttaaacgggcgggaaagaatttaaaccgcattggacccggattaaacattagcctaataatgcatattaatgtcagatggagttacgttttttgtctgcaaagtgatattattgtcttctattcttttaatttaaaaacgatcatgcttttcaaattaaccgggttatttctcgctatactggcaacatccgtcgtatccgcacaaacgtcttctgccaccatcattgtacaaggggaagttacccacccgctgaaactcaatgccgatgatatcagcaggatgaaaaaaacggaagtcacggctactgatcatgacgggaaaccgcatcgttattccggtatacctgtagcggaccttttgcagcgggcaggcgtaacacaaggcgctcagctgagaggaaaaaatatgtccaaatacctgctggtgaaagccagcgatggatacgaagcagtatttgcccttgcagaactggataccgccttcaccaaccgggtagtgatactggccgaccaggtggacgggcagccgctgccggccggcatagggccattcagaatagtagtgcccggcgaaaagaagccggcgcgttgggtacgggaagtaaccactatgaccatacgatttgcaaaagaataggtccggctggaaaggtcttcttccctgtagtaaaataatattttaatttatattatattacacatacacgcaatagagatctttcaaatgacacaaaacaagggcttaaagaaaacactgactccctttatgttgtggggacttggagtaggatacgttatttcaggaatgtattttggttggaatcttggccttgaaaaaggcggtacaggaggtatggccattgccacacttgtgatcatggtgatgtatgtaacgtttactttcagctatgctgaactggcctgcgccatccccaaagcaggaggagtttttgactacgcaaacagggcaatgggaaagaatatcggctttattgccggtatagcccaggtcattgaatttatcctggcgccgcctgccattgcattcgccatcggcgcttatttcaacgctttttttccgcaggtacccatcctcaccagtgccattgccatttattttgtgttcaccgggctgaatgtttatggtgtaaaagctgctgcttcttttgaggtgatcgttaccgtttttgctgtgggagaactgttgctcttcgccggtttgtcgttgccgaaattccaggcggtccaccttaccaacaacgcacttcccaacggatggggcggcgcctttgccgccatcccttttgccatctggtttttccttggtatcgaaggcattgccaatgtagccgaagaaaccaaaaacccgcagcgcgatatcagcaaaggttttggatgggccatcctcacgctggccattctctgtgtccttatatttatttccgccaccggcattgccggatgggaggcaattgtatataagaacgggatcagcggggaaacctccgactctcctctcccgctggcgctggcaaaaattaccgggagcagtcacctgatgtatcacctgctgatcaccgtaggattattcgggctggtggcttcctttcacggacttatcctcgccgccgggcgctctacttacgagatgggcagggtacacaaccttcctgctgccctcggtaaaatttcaccgcggttccatacgcccgccaacgcgcttcttggcaacatggtgatcgggatactggcactgctttcgggcaaaacttccgaaatcattatcgtatccgttttcggcgcgctcaccttgtatatcatttccatggtgtctattattattttgagaagacaggagcctgatctgccacggcctttccgggtagccttctaccctgccttcccggtaattgcactggtgatcgccagcatttccattgttgcgatgtttttcttcaacctgcaacttggactgatctatttctccctgctggccgtttcctttttgttgtacaaaatttttaaacctgctcacacatgacaacttccgaaatattaacgtacgtaaaaaaccatccgtcgggtaaggtaaaagtagcggtagcggacatcgacggtgtactgagagggaaatatattgcagcagaaaaatttgcgtctgtaacagagagcaggctgggattctgcgatgttacctttggctgggacatgagcgatgtggtgtacgacaacgtgaaatataccggctggcataccggttatcccgatgcacaggtaaaaattgacctcagcactttccggaaaattccctgggaaaacgatgtgccttttttcctcggggattttgtacaggccgacaatgcaccggtgtacacctgtccgcggcagctcctgaaaaaagtgctggcagatgccgaaaacagtggcttcctgccgtatttctcacaggaatttgaatggtttaactttacagaaacgcctgataccgttcaccagaaacagttccgcgaccttacgcctttatcgcccggcatgtttggatattctatcctgcgcagcgcgttaaagaatgagtacatgagcagcctgtttgaacaactggtaaaatttgatatcccggtagaaggattacatacagaaacagggcccggcgtttatgaagcagctattaagtatggcagggttttacaggcggccgaccaggccatactgtttaaaaccgcggtaaaagagatcgcgtacaaacatggcgtaatggccaccttcatggctaagatccatgaaagtctgccgggctgcagcgggcatgtgcaccagagcctctgggatgcgggcagtcaacagaatttattttacgacgaacacgacgaacataaaatgagtgccatcatgaaaagttacatcgccgggcagctgcactgtttacctttcatattacccatgatagcgcctaccattaacagctacaaacggctggtagaaggcgcctgggctcctactacgctcacctggggcatagacaacagaacggtggcattacgggccttgccgggcgataaaaaggccacccgcctggaaacgagggtagttggctcggataccaacccctacctcgcattggccgcctgcctggccgccgggttgtatggcgtgaaaaataaaatggtgcttgaaaaaaaattgaccaccggcaatgggtacaaagacacctcgaatggtgtattaccacagaaccttcatgtggccacccaacaaatgaaggaatcggcccttgcaaaagaactgtttggtgaaccttttgtggaacattttacgttaaccagggaatgggagtggcggcaatatgccaaagcagtgaccgattgggaacttaaaagatatttcgaaatcatctaagcatcagcatatggcatttcagtataattttcctactactatccgtttcggcgcaggcgtcatcagcgagctgccagcctatttacagaaaaacggattatcacggcccatgatcgttaccgatccaacgatagctggattatcattttttaaatcgatcgtgaatgacctgcaggcacatcacatctccgtggaagtattcagtgatatccacaaaaacccggtgaagagcgatgtgtataaaggcacagatctctgggatcatacacaacgcgacagtatcatcggtattggcgggggcgccgcgctggatgtggcacgcgccattgtgctgcgggttaatcaccgggaagacctgtttaaatacgacgacctgataggcggcgatatttatgtgaccaacgacgtacctcattttatcaccgtacctactaccgccggcacgggtagcgaagtgggcagaagcgccatcattgccgacgacgacacccatcagaaaaaaatactgttctcacccaaactgatggcgaagattgtatttgcggatccggcccttaccatggacctgccgccgtttatcaccgccgccacgggcatggatgcattgacccacaacatggaagcattcctggcaaagaatccacatcccctgtgtgatggcattgccctggaaggtatctatctcattaaaaactcactggaaaaagctactaacaaaccggacatagaaagcaggagcaacatgctcatggcttccatgatgggcgctatcgcttttcagaaaggactgggcgtggtgcattcccttgcacatcccctctcctccctgctggacacgcatcacggtctcgctaatgccgtaaatattccttatggtatgcaattcaatattgcgggctttgaagagaagttccggcgcatcgccagaacactggagttaaaagaagaaaccggcgaagcagtggtacaatatcttttcgatcttaatgcaaagataaatatcccgcatcacctccgagatatcggtgttaccaacgcacatgtggacacactggcagatctggcacttgccgatttcgcccatcccaataaccctaaaccggttacccgggaagatttcaaacagttgtacctaaacgcgctttagatcatgaagaaaaagatagggatcagctatacggaagccagttttgtcaattatgaaaactggtttacacccgaagacctcggcgatgacctcgaagtggtgatcctttccttcctgcgtaataacgtggaagatatttatacctgcgatggcctggtgcttaccggtggcgtggatgtgattccctcgctgtatggcggcgtcgaaaactatccgcatcagccgcaggaatttttgccggaaagggatgcttttgaaaaacgcatctacgagtattcccaacagcaacggctgcctgtattaggcatctgccgcgggttacaatacatcaacatcctggaaggcgggaaagtgtatgaagacatcggtgaagccgccaacaaaattcataaaaaagataccagcgataaaatacacggcgtaaatatccggaaagactcattgctgtacagcattaccggccaggaaaaaggacaggtgaacagcgcgcatcaccagggcatccacccggccaggctgggaaataatattatggtaagcgccacctccgacaccagcgatgaaatgattgagggtattgagttcaaagataaaaccggtaaaggctttatgctttgcgtgcaatggcatccggaaagaatgccggagaaagaaagcaacccgctttcccaacaaatcaaaacacaatttcttcaagcagttagaaaccatacgaaatgagaatctttaatcctgccaccgcacaaaccctcgccgttctcagagaagattcactggcaagggtagttgaaaaaaccgcgttgctgcggctggcattcgaccgctggtcggccaagccactggcagaacgcatcaaagtaattacccggttcaaccagcagctggaaaagagagtggaaaaactggcgggcgtgcttacagctgaaaccggaaaaccattgcagcaatcacgcaatgaaatcaacggcgccgtagccaggattaactggatgctggagaacgcagagaagtacctgtcggacgaatgggtaacgaatacagatagcttaaaagaaaaaatctcctacgaaccactgggcgttatctgcaatatctccgcctggaattatccctacctggtaggtgtaaatgtttttattccggccctgctggcgggcaatactgtgttgtataaaccttccgaatatgctaccctaacgggtatggaaatagagaaacttttttactatgccggtcttgagcaaaatgctttcaaggtagccattggcgggaaagccaccggcgaaagcctcatggatctgcgggtagacggctacttctttaccggctcttataaaaccggtaaatacatttatgaaaaagttgcttccaggatgctgccctgtcaactcgaactgggtggaaaagatccgctgtatgtaacagacgacatcgaagatatcgcagcagtggcatcagctacagccgacggcgccttttataacaacggccagagctgctgcgcagtagaacgcatttatgtacatgaaaaagtatacgatgaatatgtagctgaatttgtaaaagcagtgaaatcctggaaactgggactacctacagacgagggcgtgtactttggcgccatcacgagaaaggaacagttaaaagtactcgaaaaccaggtactggaagcccgtgcaaaaggcgccacgctgaaactcggcggtcatatcattgtacatgatggcaacttctttgagcccaccgttctcacggatgtggatcacaacatgaaaattatgcaggaagaaagctttggcccggtgataggcatcatgaaagtaaccagtgataaagaagctattcaattaatgaacgatacggagtatggtcttactgcatcggtatactcttccaatggtgaaagggcgcaggaaatcctttcgcaggtaaatgcgggtaccggctactggaactgttgcgaccgggttacagcaggattgccgtgggcgggcaggaagcactccggctttggcgcaacgttatcgcaccagggattgagagcgtttaccaaaacgaaggcgtggcagatgaagggataagttttatagaaatattgtttgtaaagcgtgatgcaatgttgaattgcatcacgctttttttatgagttaacaggttacaaaggcaacccatccactgaaattcctcctaccacatcattttggcaattatacctaattaccgtaggtttgcttccgcatttggttccgccccgtggcggattaaaagggaatccggtgtaaaaccggagctatccccgtagctgtaatcctgcatttatcgtcagataaattgtttttccggatgaactccataccactgtctgcctgtccggcagatgggaaggtcccggaaaagcaggtaagccagaagacctgcctcttgtaattaatcattcaacgctttcgggtgaaatgctacgaatgtgggcctgccagccattttatgcgctgttattttttttcgtttagccttaggcgtaatgcctgaggatagccggcattatgatcatttctccagggctttaccctgggagaaaaccacgttgtattttcttaataaaacaataaatatgaaaaaacagttattatcctttctgtctgcagcattgatgctgtttgttgcttcctgccaaaaagatgatgcgttacagccgctcgaacgccaacgcacaaacgaaaccggtaccggcggtgttacggcttcgttaatcgccggtaaatacggcaatggattttttatcgccaacgaagggtggtttggccacggcaccggtgacctgcatttctactcctacagtggcgatagtcttgtccctaacatttatcatgcagagaaccccgccggcgcgctgggcggcccttccaacacgctgcagtatgctactatcttcaacggtaaaatgtatattgttgtaaaagcaggcggcccgctggtagtgacagatgccggcagcctcgtggaaaccggtcgtattactaccctgccaggtaatgatggtcacgcttttatcggtgtggatgccacccgcggattgctgagtgcgaaagatggcgtatatcccatcacgttaccttccctcgctgtaggcgctaaaataaccggtgtagccggttataccggtgatatgttaaaagccggcagctatatttttgtgttgtcccaaacagatggcatcgttgctttaaacagcagcacctatgccgtagtaaaaaagttcggtgcggccaacctggcctttgctgccggtaaagatggcggcgtatatgccaccaacgcagattccctgatccgtatagatccggctaccctggcgcgtaccgcagtaaaattgcctttcacagtaccttccccatggggcgcatggcgtcatgcggccatcactgcctctacaacggaaaatgccgtttacattgtgcgtaacaacggctttgccgggggcactcaactgtatcgctatatcattggtaacacggcatctcttgcatctccttttattacactgccttccggccagtatttctatggcgccggcgcagcgtataacaaggataaaaatgaactggtgatgactacgctgaacggttccttcaccggggatgtgaacagggtgctgatgtatgatgccactacggccacattgaaaaaaacgctcacttacaacggatggtatttcccggccatgcctgtatttcatgagtagaggaggaaataaaaagagggtgcctcaaatttacttttgaggcaccctctttgattatttgccaattattcatccattaattccctttccatctcctcaatagtaggtagttgagtcttcaaattatccggtataatttcagagagctcaaaggaacttataccaataggtttattcaaatcacgtaaagcgtattccacttctattttatccttcattctgcacaatatcattccaattgagggactatcagtaggatgttttaattggctgtccactgctgataaatagaagtttaatttaccggcatactcgggttgaaattttccagccttcaattcaataaccacaaaacaacgaaggtgcaagtgataaaataataaatccaggaaataatccgattcactgatttctattttatactgacgaccaacaaaagcaaagccctttccaagttccagcatgaagtgagttattttctgtgtaagcgccagttcgatttcccgctcctgggcattctcttccaacccaagaaaatcaaaatgatagggatctttgatgctttcagctgcaaggtcagactgtggctttggaagagtaaatgcaaagttatggtctgctttcccttgccttaagtggtaattacccttaatattaatttcaagctgatctcttgaccagccatttctttgtgtggctttcgcgtactgtatggctattttaaggtcttttatttttgaaatcaggagccgttgataagaccagggtaattgtgccacaggttgtggcacaaattcaaattccttcgaaaagaagagataccattgccggattgtatataaatttcgtcgcgagaagccgtttatttccgggaaactcctcttcaaatcaatagcaagttgctcaagaaagttatccccccatttcgcttccatttgtcgttggacgatttccttccctagctcccaatacagttcaatcaaagtagtattgaaattggctgccgcttttaattgagcttgtcttactttattctttatttctagtagccattctttataaccatctctactcatttatttttatttaccgttaaatgatctgcatttatcattaggccaataaattaaaaaaacgatgatggtagaaataaatcaagtaagtgaataaagaagtattaactacctgataacattttggtaaataagaatgataaacgttatgctggattaagaatatgcgtgcttcaatgagttgctgatttaatgcaatcgccgattaggttgctaatactctgttagagatgataatgctttatttccggaattacacccttcattaaaaatccaacggcaatttcatattcattaccacaggctccagcttttcaagcgatttccataaacccgcttccaccttatctttttccgtgaaccggaaaagccattgccgtataaaatttttagggagataataatcaatagttaaccggcttctccggtctgttaccttttccaccgtatagtagaaagcgttatgccgcttctcatctgtttcactgaacaacgccttttgttccgggttgtacgagaaactgctggtgaacatgatcacatgttcgccattatccatcacatgccggtgacggctacctataccagggagaaaatgttctacctcatctattgcgatcacaccggtttgccacaggtgcctgaactcaaaatgcactacggtataaataagtgttttaatatccgtgtcaaattccttcgacacggaaatcatcttcgttttatttttaagctctacctgtgggtcgggatcgggtggtaacgtattgcgcagttcacttaaatgggtgtagtgaaaagaaatattaccggtttctgtttgtttgatgctggcatcccatgtcatccattgcgccagtccttccggcggctcatcacgcaacaggttatctgttaccagccagtattcatgctgctcaatatcatttttcaacagctggtgcgccacgatcacatctttccctatcagcttactgaaattctttacctggtaggtggtaaactcgccatagtgggtaattaccttcagggtaaggtcaatagcggatacacatgccttacactggcaaattttgcggtgattgtaattgaccaggtaccgatgaaattcgcagaacatcttttccacctgcttatacagtacttccagctccggcggggatccaaacttatagaacaggatggcgtcaccttccacttcagatacttccaggcccgactgattagcatttatcagcagttccaacagttgctggataatatggcggctgtgctcaatctctatttcattcacaaaacgggtaaagccacttatatccggaataaaaagcagccctctattttccattttttttattaaagttagagataaaaataataaaaacggcatatagctgctcttccgggtatgccggtccttatttcttctccaaccggaagatcatggcgtccgcagcatctaccgttacatggatcttccctttctctgtggatgttttagcggagaataattctttacagcgatattccccggtgctgagtcccagcttactaaaatcagcttcgaaaacggtgggtttcctgttgtagttcaccacagccaggtaggtaaaccggccgctgttgtgtacaaacaggctggaaggggtgtcgccggtatgatgatctaccggaacaaaaccattgggcaactgcgccgcttccatcacatcgcggttttgcagcagttgctgcgccacgccggaagcgctgctgtactcagcatagtcatcgccggtaataacggtgccggtaacgatggcagaggtaaggcgcgccctgttttcaccaggactggcgcccgcaaacaccacgtgatccgcatctgtaaaatcgtatactttattttgccaccaacccaaactggtggcattaagggtataggctgtttcgtcaatgttcttaaacgcatcgcaggcgatacggcgcatatgcacatacctgccggtggccataccgggcgaaatagcggcgtataccagcatcttgctatccagctgatctaccaggaattccatgcccttcctgaacgcctgcatgcccgtatgcacagaaggatcataccagccatctgcctctatggccgcatggccaatgaagtcgatcttaatcatttcaaagccggtttccctgaaccgtttgatgagataggcgatgcggtcgcgggtagcgggatgagtggggtccatggcacgggcgccatcaaaatcgtggtattgcccgtttacttttgtccaggtttcctcgtaattataacggcttccttctaccatgcgggaggatttggaccagtctacgaacggcgcccagtaaataccgggtttacatccccgttgtctgcaataagccacaaattctttcaactggctgaaatcgccggtcatgccgcctttggtcatgttatcccaataagagtcgaggtctatgtaaaggctgccatccttgccacggaacgttttacaggagtctgcaaaaaaatcgaccacctgtttggctttcaccaggttcaacttcgtttgcatacttccccagctgttccagcccagcggctttgcccccgtccattcaaaaatatagcggggctctgcgaggcggttagcactgccatattgctccatgcctttgcgccagttggccgccggcagtaccaggattttcggggagctgcacagggtatcgccctgcgtaactatgccatggggtattttgtcgcgggtaacaagactatcagtccaccccgccactacagaaacgtgtgaattttccacctttacccctgttttccaattgttatgctctaccgagccgagtatcagtccagcgttggtaagactgtcgtacaacgcagttacctctgaactggtaaatgccgggccgcgctgatccgctacatggtacctgatccatgcatcattatcaaaaggaacgactaccccgctggtataaatagccgcttcccctgttaaagggctcatggcccgggaacgggcgccctttccctgcagagttaacgaagtataaaaaccatctttccctttatatacataaaatatttgctgtttttttacgccgttaccggcagatgtaatcacataccgggttccttctcccataccatctttcacgggtacactggtaaaagtgcggttaacaggaagggtatccggccggccggcatcttcataaaacgcaaatgcatgccggatgatttcttttccgccggtccacacggagtaggtacctttccgtaaatcgtaggcgatgtaattgtttttcccgaaggaaatatgtttgacatgagcggcctgctgcgcatgcaacggcgttaacaggcaaagcattcccgtaacagataaaaggtatctgcaccagatcagagcgttattcattttgcaagtcctagtggtgaaaagatgataaatagcaacaccattaatatcaataaagcagcgctgtaccagtgccggttcttccagggttctaccgataccaccgggatcaccgccggctgataaggtacggccatcggttttattttaccgatgatcagcatcagcactgccgttatcacaaacgtcatcgccaacaaatgcaggtaatgaataccggtgtcgaatacccattgcagtaatacatttacagccaggaaaaataccaatcccgctttggccgccaccggcggaacatgccgggtagccatgcccaccaccatgatggtaaaaatcgggagactgaaaaaccccgccagcatctggatataattataaaaacctcccttgaacaacatgataaagggtgcaatcacaatacccgtgagcaataccagtacctggaacaggcgggttctgctgatcagttctttatccgtgatgctgcctttgcgggctatcataaaaggtttatacaaattcatagtgaacagtgtacccacgctgttcaaccctgcgttaaaagtgctgagcgctgcaccaaaaacaatggccgcaattaaaccggtgtataccggcggcagcacatccgccgccatcctgggaaacacttccgccgttgcctgtggatggatatacaggtgcacggcaataaggccgggaatgttgagcatgagcggcgacaacaatttacacaaacatgccagcgcaatccccttctggctttgctccaggttcacggaacccagcgcctgctgcacaataaactgttccatgccccagtaataaatattcaccagcagcataccggtaaaaatagtgctgaagggaactgcatcgtgtgcaccaccgatagcatttaaatggctggtatgggtgccgagtacggttagcaaaccggtttccgcatcgccatgccccaggtatttaaacccgaaatacggcagcagcaatccgccgatgatcataccgccgcccagcaaagtatcggagatactgatcacttttaatccgcccagtacattgtagaaaaagcccatgatgcctatcaggcaggccagcagccagatggtagaccaatagctgatatgcagcagctcattcaggtgaaagatcccgttaaaagccaccgcaccgccgtacaataccgcgggaatcaggtttaccaggtagctgagcaggaaaataacggaaacaattttcttggtgccccggtcataccgtacttccaggaaatccggtgtggtaacagcgcctatacgcaagtagatgggcatcaggaactcgcctaccagcaacatcgcaaatacagaagtaacaccccacgacataatagacatgttattgatgaaaacagattcgttttcaccaataaactggttggcgctgatgttggtcatgatgagcgcaccgcctattaccagccagtttaaactgcggctgccaaggaatacgtcggcggctgttttcaactggtgcctccttgtaatgtaccacgacaataccgtcatgagcaccacgaaaaaagcaaagcttataatagtagaaagtggcattaataattactgttacaaagattttcttcttatcagcacggtaggcaatacttcctggatcttctcccggttcagtacaaaaactgctgccttctccgccattaatttaaagtccgtggaataagtggtaattccattgcagataatttcctttaccacatcatcattgtgagataaaatgcctacatccgttccaagcgtcattttcttttccacacagtctttcaggatagcccacaactccgtattattgatggtgtaatatacttttccctttgccaccgtaccaggtacgtattccgttttaataacaccgttgatcttatgatcttttataaaacgcttaaaagccttgagtatttctatcggcgtatccgtagagggccggtaataaaagatcatttcatcaaactgctttatggtagctgttaacgcagtgaatgccctgtaggaagattccccgaactcctgcacaatgtaagaacaatccatgttcaacggttcgtagcggtcaatcatcaggaacttatccaccggcagcccccgcaggatctccgcggttttgggatgcggaataggcgccaccacgtacatgccatagcggccctttacagatgccacaatgctctcaaatacctcgatgttattgtgatgaaagaaaacatccagctgtatgttctccccgagatgtgcccggaaagttttataaaatgtttcctggaaagtatcaaacgcaaataataacaacgctactttcaactgctggccggtatcatcgctgcttacaaaaaagcccttccggttttgcgatgccacaatacctctttccaccagctccttataacctttggcaatagtttcccttgcaaatcccagctctccgatcaggttattcacagaaggcaatgagtcgcccctcgacaacaatcttgaattgatagcattgataattccctgaacaaattgttcatgtttagaaagaccgggaattccttccagttcatgtatctgttcgtatacgtcctgcatgtaaggaaaattaatctggaattaactgtactacactatcctactaagctattgcgttttttcaacacttgcaactttttgcagtgaataatgggtttcagacagggattgtaacttcctggcggcccattccggcgtaatatcgcgctgcggactggccagcagctcatatcctaccataaactttttcacggatgcagaacgcaacagcggtgggtaaaaatgcatgtgccagtgccattccggatgatcccccgaatttacgggcgcctggtgcataccagcggagtaagggaaagatgtttcaaaaaggttatcatattttgtggttaatctttttaaaatatccgccagcgcaagatgctcttcttccgtaaaatgtatcagatccggtacatgccgtttgctgatgatcatggtttcaaaaggccaaaccgcccagaagggcactaatgccacgaagtgatcattctcacaaacaatccgttcctgtttctttaactccagggcaacataactttgcagcaggcttttgccggtagcttcataatatttttcctggtgagatgtttccttgatcagttccgccggcaaatcgctggttgcccagatctgtccgtgtggatgagggttgctgcatcccatgatatcgcctttgttctcaaagatctggatatacctgatagccggatctgcggagagctgccggtattcctcctgccacaacgtgatcactttcctgatgtctgctacttccagcaatggcaatgtgagatcatgccgcggagaaaaacagatcacgcggcagatgcctttcacgccccgcgcatgcagtaagttatctgttattgttgcgcctgcgggcgtatctgccatcaatgcgccaaaatcattggtaaatgcgaaaggcgctgtgtaggccgggttcagatccccgcccatgcggctgttccccggacataagtaacaggaatcgtcgtacgccggcagcggatctttgtttaccttttctactttgccctgccatggccttttggtacggtgcggcgatactaatacccactcacccgttaaaatgtttaatcgctggtgtggatgttcttctaactggaaattgttcatagataatcaggatacttcgttgatctggataaccacgctggctcttttaacattcagctgcggattaaacccgatgttcattaaaaattcgccggtaaatataggactatccgggatagttgttgcttcgccgggataaagattaatttctttcaggcggtatttctttgcaggatccaggccctttaaccggatgggaaatttgctgccttcgccatagcggtaattgaccaggtagttaaacaacacgccggtggttttcttttcatcgagatacattatggcggctacgctgccctcgtgcggatctgccaaccggtactggtcgccgtgccagatcacctctttcaaagcaccataattgttaatcgcctccttgcagaaagcaagatctttctcttttaaatcttttaccacaatgtcaaaacccagcttgcccatcatggctacatccaccctgaacttaatcggttgttttccccagtcggttacatggttggcgctggcaatagccgggtagaaataggaattttcccactggatgtagatccgctccaaaggatctgtattatcgctgggccaatactccgtgaagtactgcaacgcggcatagtccacacggccgccgccaccggaacaaagcatcatcgacacctttggatatttagcgcgtaccctggccagtactttatacaggccccgcacatattccacgtataactgcgattgctgctgccgctggtaagccgaccatgtgttgtaaataacggcattacaatcccacttgatataagataatttaggcgcttttatgaacaacgaatccaccaccttaaacacaaaatcctgcacctttggattacttaaatccagcaccagctggttccggaaataatgttcttcgcggccgggttgtcttaacacccaatcggggtgtgtggcattcagctcactttttggattcaccatttccggctctatccagataccaaatttcaccccgttaagctgtgccatgctatccagtgcagcgatgccgttaggcagttttttgcggttctcctgccagtcgcccagcccggcatgatcactgttgcgcgggaacttattcccaaaccagccatcatccagcaggaacaagtccacgcccaggtctttggtatcttttaataaccctttcagtgcagattcatcgaagttgaaataagtggcttcccagttatttaataacgtgagccgttctccttttccatccggtattttataattcctcgcccagctttgcagcttacggctggcatctccttttccttttgtggaaaaggtatagaggaacggcggtgtttcaaaagcagtatttgcttttaatacatagggagatgcataattgttgatccctgctatgatccgtaagttatccaggttatcaagctccagatcgatcctgaaatttccgctccactccagcgatccgtataacacgctgccctggtcttctgtagccggttgatccagcgacaccataaacaccggcggctggaataaattggcgcgggtgcccagtttggagtccagcgttttaatgccatgtgtgagcagcccttcctcaggctgcatttcttttgcccagtcgccatgatattggcggagccagtaacggggagctttgagataaagattggcagatgcaaatttctgcagggtaacatttcctttttcctggtgcctgatcaccgaccattgctctattacatcttccgctttatatactttatagtacaacgttacttcaaacgggtataccgggtctttcagcaggatactgatttcttccacaccggcttcgcgggcagtcaccttatgacttacataacgcaggtccagtgcattgttgccatcggcatgcgttactgcgatggcgggttccatcaggttttttgtgccggcggcagcataagcggcattggatacggttgaatagtcttcggcttgtttgtatgccagcggcgcctgttggtattctgccgcattggatagcttagtgccaaagtagatggtagacagttgtccttttgcatctacctgtaataccacggcgttgttctttgattccacaggtatcgtcaatggcctggcatcctgtgcgaatgcttgtccgcagcagcacatcgccaataaccagatgccctgtttcaaatggaagaatcgtgtcatgaaaaaatctttttaaatttatagctacaggtcattatgcgcaatacggataacaggttgcccgctatggcaatcattttttaatttaagccgtaaatagcatacgaatatcgtggaacggtgtggtgatctcatcattcataacgcgctttcactaatcgatttatatcatctacatctgttctatactatactattctacaaatataatttccggtatcgaaacttccaaaaaaatccccctgccaccaccgggataaatatattagcccctcatacccccggcgatgaagccgccaccatcaatatagaaaagctgacaaaaatagcccggtggatgtatgccaccggctttaccatatccaatctgcagaacggccggcaatggaacccggctttcagctggaaaggtaaaatataagaaagcaactgcttagggcagttgctttcttatattataatctgctcctccttcatcaggaacacgccataagcattcaatgcatcaataacagacaatgcccgccgggctctttcagtaagcgcataatccactcgtggaggcttctcctggtatgccttcctggtgaccatatttttttcttcgaggtcgcgcaattgcgtgatcagcattttatcggtgatatgcgggatggattttttcagatcaccatatcttacaggtccttcctgcaacgcctccaggataggaattttccaggtgccaccgatataattcatcgcaaattcaacaggactgtaatacagcctgttctgatgccggaaatctttcatgccggaaatttactcacggattcccggttttttgcctttacataccaaaaagtatataacaaggctatttctattcgtaaggtggcgggccaaccggtatctccttaatgcctaaccgcttctgcaactgctgcacagaatcaagatgcgcatataacatcggcagattggccgccgcaaatgattttatatcactgtctgttgcattctttgctgcccgttgaaattcccggatgtcttttttatggtcgctgagcatcgcatttacataagccctgtcgaattcgtctcccttcttttttccaagccgatccttttctttctgttgggaatttgagatggaatccggcaacgttatttttttggaagcggctaatgcctttatttgcgctcccccgccgctgtgatcttttaccatcaatgcaccgaaatcctttacctgttggttccgggaatttgtttgtgccaactgtcccagttgcacttccatcattcccccactggctgcttccaccacgaaatcagcatctgcctgcgacaaaaccactgataccgagtccgaggacttgttgttcataatctggctgtcgatccgctcactattggcttctttggctttcttctcactatctgcagacctgttgttacaactccataaaaggaatgccaatggcaatgtataataaacgaaaagtgagtttttcataataccctcctttttcgaaaaaacgcccaaaacatatgccacgcgcttcaaagcaggcatttatttctttatgatcaccgaccagtcgtctggtttttgcagcaggttgaaacccacgtctgtatgtaggcgggtcaggttaagatgacagaggctgtcacccaggatgaggttggaaatatacacttgctcgaggtaagagggcagcaacggtttttcaaacgtaacagttttggtaaccgcgtttatgtgcacccggaaacatgcctgcaacaacataaataccgctgccactgaccacgcctgtggcgagcaggcaacaggataggctgtaggcccctctcccctgcggcggtccagtccgcaaaacagctccggcaaacgttgcaactcaataaataaacccgcatcaaacatgccctgcattatttttaacacctgttgctcaaagccgtacaacgataaaccataagcaatcatggcattatcatgcggccatatagagccgttgtggtatgacatggggttatatcgcttctcaacggcactcagcgtgcggatgccccagcctgtaaacatattattgctcagcagggtatcggccaaagttcgtgcatgctcttccgtagctatttgggtaaaaagacaatggcccgcattggagctcaccacccggcaaggacgtttattattatccagggccagcacaaagcaattcagctggtcgtcccagaattgttcattgaacttttgcttcagtagcgccgcttccttttccagctggccggcaagcgacaattcaccacggacgaccgcgagcttggccgcgtgtttttttgccgcgtatacataaccctgtacctcacaaagcgcaatggtgggttcggccagttctccatcttcatacataatagaatcaaaggaatctttccagccctggttggtcagtccgttcctggctttgtgcttatattccacccatccatcaccgtcgatatcaccataattatctatccaaaacaatgcagccgtgatatggggccatagctgtttaatggtatctgcatcagcggtgcgttcataatacatccccgccagcataataaaaagcggcgtggcatctatggtgccgtagtactctttaaacggaacttcgccagtgttggccatttccccgttacgtgtttcatgcatgatcttgcccggctccgcatctttttccggtatgaattcagtagcctgtttgctggcaaggaacaacaatacatccctgccgatagcgggagccagccataacaattccattgcagtgatgatgccatcgcggccaaaagccgtattataccagggaacaccggcgtaaggataatagccggattccgtacgcgtcaatagtgaaagcatatcagccatcgaccggttgatccagtgattgaactgggtattggaggtgtaaatgctggcaaacaggcggcgggtgctgctcaattcctcattggttgtttcctgtgccagctgaaaatcgatatccatatttttttcctggtccgttttcagataaatagtgtaactgataacggtctgctctgcgggttgaagcatcaccgtgaaatgtactgtatcccggataacataaaagtcggccgtactgctgatcacgatcgttgtttcgcgtgctacgttatccaatcccatgtattgaaagctgaggcggtcgccttctttctttaattttacagggggaatttttacctcccgctgcgtgcctcgcacttcaaagatgtccctgaaatctgcaccaaaagaaagggaaagatcaaactggcagggctgatcaccaaaatacctgcactgtagttcttctaaaaaaaccttattccggatcagttgtgtgcgggaaatatgaacggtattttcggctacttttccttctgaaagcaccgggttggtgaggtcaacggacaaaatttcgttatcttctttaatagcattgctcaatagcaaaggttttttaccatcgatagccagatttaatttatttaaaaaccgggtgccatcatgatagatcccctgcaccattttaccaccgggagaaatattacccaactggtcgaaaaggccaaacgtattacagtgattgagtaccttattccgctcatctatattaattacatcagctgatatatgaaatttagtttcttcttcagttggatgaataatattttccatagtactgtttttatagtttacaatacctgttgttgctccattaaaagatccaacggcatattgttacgtttacctgcgataatcaactcatataattgcacataatctgttgccatcctgtttgcagtaaatctttcttcaaaaacacggcgaacttccctgcgcgataaacgagtaattgctgaaacggcgtgcagtgcttcctcctgcgtttccaccataaaaccactgaccccgtttttgatgacttcaggtacagatccttttttaaatgcaatcacaggagtaccgcagctcatcgcttctatcatcaccagtccgaaaggttctatccaatcaatgggaaacagcaatgccatcgcatttcctaaaaaggaagttttctgcttctcattaatttcacctacatattcgatcagcggatgtgctaacaggcgctcaatattttctttataatactgctggtcttccctgtccaccttggccgctattttcaacgggcaatttgcctggatggcaatttcaatagccttgtccacacccttttcaggagaaatcctcccgataaaagccaggtatttacctgcctcttcctgtaacgaatgcagatgaacaggcaatccgtgatacactgtacctatccagttggctgccggcaaaggcagacgctggttatcggaaacagagaccaccggctgctgctgaaacatacggtaaactgattgcagatcaggaatatcaagccgcccgtgcaatgtggtaatacaaggcgtactgcaatgtgcactaaatggaaaatgcaggtagtcggtatgaaaatgtatgatatcaaattgatctgcccgccggatcacttcttccatttgcacaatatgatacgccagcggatcagtacagttaccatttaaccgcagcgactggccaaccgtagcaaccagttcagcatttgtaacagaatctcctgaagcaaacaaagtaacctcatgtccttctttcaccagctcctctgtcagataataaatcaccctctctgtaccgccgtacaaagagggtggcactgcttcgaataatggagctacttgtgctattctcataaattaattccatttgattcatcattataaaaacaagagatgtgccatttggaatataattttatgagaccggatgaaagacctacgccgttttttgattccgttctgcttcatctatccggaaagataccttacagatcaatccataagtggttatcttcccatcttttacatgcactttaatatcttttacgaaaacagaatctatattatggattgtttttgatacttctgttaccgcattactgatagcatcttcaatacttttttcagaagaggaaatgatttcaattacttttacaatagccataaaattatcttttaagatgtgaaagaaattgttttttgttcccttccgcggcacaaaaacccggccacccatgccaatttatctgctataaaaaaaataacgatcacgttttgaatcagcttcacgaacggctccagctgctatgggaaaaatctgctacagcagtgatgaacaattaatacatccacagatggtcgggggtatcataattgtgacggagcaggtaaaagacgtttaggcacacgttaaatgacagcgccggtttacaggccctgatggatgatatcgctgacaggtgcatcgttagtttatgggattccatacagcaatgatcaactatctgcaaaaggaagatcagcaagcggcgcagtttgcaaaaaaggcgatctcttgttttgagccatttaatcagaatgaacagcagtacgcaactcgttcaacagacatcattgcagggacgaaggtatactgcagtatgatggagtttgataacaacagctggaataccgaccagctggcagggagtgggccggcaattatgtgcctccattttatcaaaacgctatgatgcttttatctgcccggatgaaaccactgcgttgcatccgctgcacatacaaccacatgatgaaaagataccggaaacttatccttttggtatgtaaaactgtagttgctgcctccggcatagaagatctatgcctaattttcataacgcagcgtttcctttcctgatgttttttctgaaaaatacccacgtgaaagcaaccaggtaaacaaaaacagcaataaccagcaacaacggcatattcccgtaaatactaaactttaacaatatggcttccaacaagagtaaaccaatccaatactacacaaaaggcatccgcccgccttcattaaaacgctttagcaggtaagcgtatggccatacgaaaagcaacgcatcgagtaaggtaacaggcagtataaaaaataaaatggcagataataagttcgatttaaaggagatttacaatatgctcccacgccttctcattactcataaatccaaacacgattagcatgatcggaatatttctcagcataaaataaatcaggaacttttttataatcgctttattcattgtggtctcttttaaatcttcagctgtaattggctattatcctataggtgcgatattcttattaattattaaaatatgtaataaaatgctgaaaacttccacaaaattaatatgttctatggcagactcatttaacaccagcagcctcaaacaggtttatagattcataattcataacctattaattttcaatcatttaaacacacccctttttccttgagaatttttgctctagtttgtgcttccaaacatgaacataaaataagcattgtcaagtaagcaagcatacggggaaattgagctgatatcttcttttcagcagggcgaacacaaagcactgcatcaaatttatgcgctataccagcggccactctgcttttttacggaacagctgacttccgataccatggccgcagaagatattgtttctgaatgcttcatccaggcatttcaaaaaaaagaggactttcctacactcgggcaactcaaagctttcctgttcaccgcagcaaggaatgccgccctcaattatctcaaggcgcaaaaacgacatggtgatatccaccagtcgatagaaaggaacgccgaccgcttttccatagatgttgaaaaagcctatattaaaacggaggtcacccaggctatttttcttgaaattgaaaaactgccgccacaatgccggcaggtagtccgcctttccgttatcgacgggaaaaagccacaggaaatagccgacgaactcaatatggcctaccagaccgttctgaaccaaaaagcaaaaggcgtgggattattgcgtaccgcccttttaaaaaatgagttgatatccctgccagtcctcgtttccgcgctgttaatgctgcagcggtaaatttttttttgaaaagggcggtataaaaagaggagttagttgttttagtagtatcgacatgactgagaacaatcattacatagccggcctgattggcaaatacctggacaatagtctgaatgctgacgagaagatggcgttaacggaatggatcaacgcctccgacgataaccgtcatctttttgcggaattaagcgatcagcaacagctggtggcgaatcttcagcggttttatgcctatgatgctgacaggatttccaggaagatcagtgaacagattcccggatttgaccaacccattatgaggccggttcaccgggttcattttatccgcagatggggctgggcagctgctgcggcactgctgcttgcaggaagtacctacctgctggtaatgaataaaaaagatcagtctcccaccatcgcatcccgtgtagcggatatcactcccggcagccagggcgccatacttaccctggccgacggacgacaggtagtgctggatagcctgaccagcggggttgttgcgcaacagaacggcagctccatcgtactgtcggatggtaaactcaagtatgatccttccggggaagccgtctccgacattcaatataacaaaatgaccacgcccaaggggcggcaatttcagctgaccttacctgatggaacaaaggtgtggttaaatgcagccagctctatccgctaccctactgcatttgccggtaaggaacgaaaagtggagatatatggggaggcctgttttgaagtagcaaaagatgccaataaacctttccgggtaaatgtaaataataaagcttccatagaagtactgggcacgttgtttaacgtaaacgcctacgaaaatgaaaaaacgatcaatactacattgctcgatggaagcgtaaaagtaatcaatgaacctgccagcgtaatcctcaaacctggccagcaggcacagatcagcaacacaccgggaggaaaaatagctatagtaaacaaaccggacattgaaaaaataatggcctggaaaagcggcctgttcaactttgaaggcgctaatcttgaagaagtaatgcgacagctggaacgctggtacaatatagatgtagtttatgaaaatggtataccggatatacaattcatgggagaaatgagcagacaaatttcattaacagacctgctggaaatattaaggagaacagaagtggactttagagtagaaggacgcaaattgattgtgctgaataaataagtatcagttacactgcaccgggaatcacagaaggggcctgcatggcccggcctgactatgtaatttaacaagccaaccattaaaaaaccgtcacggattgcggccgtgacggtgtatttgacttagttggtttctaaacggtttattgcaattcacatttattaacaaccaaatctcatgcaatttatgcaaaaaaaatgctattggccgccggatcgccggggaaaaaacacgggcctaaccaaaatctttctggtaatgagacttactgtcattctattaacagccgccatctttcaggcaagtgcctcgggtcacgcacaaaccgttaccctgtcgggtaaagccatccctatcaaacaagtatttagtgctattaagcaacaaaccgggtacgtagttttcagtaataataacacgatcaatgatgcaaggaatgtatcgctttctgtacgggatatgcccctgaaagacttgctgaatgaagtattgaaagacttacccgttacctacgtgatcaaggacaaaacgattgtactgtcacgcaaaacaataccagccggcgatatcctggctcctcccaatacgattaccggcaccatccggtcttccactggtgaactattgccaggcgtatctgtccggataaaaaatacggtcaacggtaccatcaccggttccgacgggtccttcttctttaaccgtccacctgaagatgccgtattcgtgatcagcatgctggggtatgaaaccctggaaatcgctgttctgaagggcgacaacggatataccgccaacacgctggataaagcacaatcgaagtcgctgctggtgaaagaaggagccaacctcctgctgaacattacgctgaacaggaaagacctggaaatgaacgacgtggtgatcaccgggtatatgaacgtgaataaaaagaattacgtaggctccgtttattccgtaaaggcagatgatatcaagatcgccggcgaaaccagcatcgatcagatgttacagggcgttgtaccgggcatgtctgttatcacgcaatcaggacaggtaggttccacgccaaagatccgtatccgcggtacctccaccatcctgggcaaccaggaaccggtttgggtagtggatggcgtaatccagcgcgatcccctgccaatgcccaatggtagcggatcactggctggagatatgagcgaactgcggctgatcgcctccaatgccatttcttggctcaatccaaacgatattgaaaccatcaccgttttaaaagatgcttcggccaccgctatttatggttcacaggcagccaacggcgtaattgtgctcaccacgaaaaaagcgcgccccggccagttatcggtgtcttatagctccaacctcacagtgggtcagaaacctacctacggcgacttcgacctgatgaactcccaggaactgatgcagttttcgaaagaagtatacgaagcccgcgacagctataccgctgaagtattgccgatcggctatgccgcattgatccagcagttacagagaaaagaaatcgattatgccacttatatggaacgctaccgcaagctggaaaaccagaataccgactggttctcactcctgttccgcaacccgttcagtcagaatcatagcctgagcatctccggcggcaccgagaagatctccaacagaacctctttcagtcttcagcagcagaacggggaagccaaagggaatgaccttacttctttcgccgcttcctccaataccactctccggttcggaaaacggctgaccgtaaacctgatgctaaacggcagccggcgggaaacaaatggtttttcgtatggcgtagatccgttcaaccatgcttataatactgccagaaccattcctatgtataatgatgacggatcccttttttaccatgagaaaagaggagaacccagcaccgttttccccggcaacaacagctaccggtataacattcagaatgaaattaataatacaggaaataaaaatgttaccaataacctcgcatctactgtagatgtaaacctgcagttaacaaaggacctgcaataccagggactgttatcttacacccttaccaattccagcgtaaaatcctacgcaacggaattatcttactttatcactcaaacaagaggatatgagttcggcagcgtactgtccaactctccgcaggaactggccagccgcctgcctttcggaggactcgcacaactgcagaacgccgacaacagtggctatacctggagaaacagcctggtatataaccacttatttggtacccgccatgccgtgacccttcaggctggaatggaagccagatccgcattaatgcagggtaataccgatagccgttatggttatctacggtatcgcggggaaagctatgcacctgttccggtaatgcccgcgatgatttccgccaatggcgacaacctgcttgatctcatgcgcacaaattcaggaatcgtcaatcaaaaaagtaatttcctgagtgagtacttctctgcggtatatgcttttgatcagcgatttatcttcaacttcaatgcgagattggatgcctccaaccgttttggccaggataaaaacaagaaattccagccaacctggtcgtttggtggaaagtggcgcgttgccaatgaaaaaatcctgagctccgtgaaatggctgaacgcacttgacctgtctgccacctacggctaccagggaaatgcagtggaagcggtatctccttacctgattgccaccgatgggggacttagcaatgtcttcaaacaatatgtcctcaacatcaaatcgctgccttatcctgaactgggttgggagaaaacaaaaacatggaacttcggactggacctggcaatgtttaacggccgcctgagcgccaccgccaactggtacaaaaaaagcagcaatatcctggcttcacgggacgtacccattgaaaatgggatgaactccgctaccgtatttggttccctgatggaaaacaccgggtacgacctgatcatcagcgtagtgccggtgcgtacgaaagacttcatgtggcagttttctgtgaataccggtcttgcccggaacgtgctgaaacaaaacgaaaggatcaatacaaaagatgattacctgaacggaactgctattgtgaacggagaggcttactccaccttttattcctttgcctatgccggtttaaatccagccaatggcgtgcctctctttaaaaacatggatattaaacctactgccaatgacctggattacctcgttaaatccggtaagctggatcccgatttttccggcggattcaataccatggtgcgatataaaaacctttcgttaagcgcgcagtttgccatggctttcggaaatcaaaaaaggctgccggtgttctacaattcttccggggcgcctactcctgaacagaatgcacccaggatcctgaaggaccgctggaaacaaccaggcgatgagcagcacaccaacatccctgctgttccacccggtaatccccgcaggatagagttctacctgcccacgatagcgtcaaacagagtaacgccgtatgacctgtataatcaatccgattacatggtggcagatgctgactttatccgttgccggcagattgcgttgaactatgagtttacacaggaactgctgaaaaagatacacatcaaacgactgagtacgtccctcagcatgaccaacccattcctggtaacttttgacgacgcatggagaggttacgatccggaaacaaacggatggcctgcccgcagaacaacgtcattatcttttaatatgactttctaatattgaagcgcatgaaatataagttatttgctgttttctttgtcttcacggtgctgacatccagctgcaccaaattcctggaagaacaatcacagagcgagattattcccaaaacggctaccgacttccgggagctattgatgggatcaggttatatgggaaatcaggagccaactgattttctttcccgcatggacgacgatgtggacctgaacattgaatggggcgcgggcaccccctacactatcgtaggcaccgctacggttaaaacagattacctgttttatacctggcagccccagttggccgacaggaatgggttaggcgatcttatcagtgaagatcccgcgtctaccgcctattactatttttatgagaagataatgggatgtaacgccgtattggataatatcaataccgcgatcggtagccagcaggataaagacagggtaaaagccgaagccctggcgatgcggtcgttctattatttccggttggtaaatctctatggagcaccttacaacaacaatccacaggcgctttccattcctttaaagctgaactccaatgttacagccgaatacacggagcagtcgacggtagcaagggtgtacgagcaaatcgttaacgatctgaaagaagctgccacgctgatggatccgctgcctgttgcgcgcagggactttcacatcaatcaaccagccattcacattcttttgtccagggtatatctttatatggaaaaatgggaagagtgcgtagcagaagccagtaaagtttttgaacagtcgtcagtactgatgaacatgaccggcatcaccactggttactggctcacctataccaaccctgaagtagagtggatgtttggtgcaaaaccgcaagggggcgaccaaaccgcctttattccttctccggatctcctgtcagtttttgatcagaacaatgatgtgcgcctaaaatatggtataacgaattcaggtggcacaccgctcatcacgaagtatacaatcataaacggagaactgacccaatgcattcgtacagcagaagcagtgttaaacagggcggaggcaaacgtgcagctcggaaaactgcctgctgccatgaaagacctgaatgacctgcgccgtacacgcatcattggttacacagatgaaaatattggcgacaaggcagcactgctgcaggcagtccgggtagagcgccgtaaggaatttttcctggaaggattccgctggtttgatctccgacgctatggcatgcctgccattacgcaccggtatcagcatgagccgggggaagcagtattgcattataccctgaaggaaaaagatccgatgtacacgctgcctcttcccaatagcatactgcagagaaaccaggcactgaaacaaaatccatccggcactatgcccgacaggatcggccagtaatgtttaaacaagcaataacatcataacatgaagcatatatttctaatcggctgcatctccagcatattactattttcctgtgcgaaggatactgaaatcggcgcaccaacgccgatcggacctgattatgttttaccgcagggcaacgccccaaaagaggcaaatgataaaattcaacagctctataacaactacggatcttacttcctgtatgtgtttacacaaaaggattttgaatggatgcaggcagccggcggcagcgcatcaaagatcgatacagcggtattgggcaaccctgcttataccggtgatatgctgaatttcctgaacgatgtgtggttgaaattcctgccggatgatttcaagaaaaaccaggggattccttaccgcgttctcatggcagataccatcaaacaatacaggaccgggtatccccccggcagggaatacctctacttcgattacaaggtagtaggtaagtccatcactttcgccggcatgaacgcatcactgcgtaccatgaccccggctcaaaaggtggacaaaaagaatgtcctgacaggcgctatctggaactattatatcagtaataatattcttgatattccggcagcattctacacggtcagcaattatgcagcagaagcagcacccacagcgccgctgtccattcctgccaacctggaggccttccgcagcagcggctttttaccaaccagctatgatgccctcagtggcagaataggtgaatggtattatggcacctattcctggggaacggccaaatcaaatgatatcacgtcatttatcatgcatattacaacccggacggatgcacaaatgcagccttacctgcagtatccgctcattaaacagaagtttgatatcctggtggattattacaaaacaaaatatcatatagatgtgcgtgctatcgccaacgccacctactgatgtataacctttcctttcgcccggggcttcgtccccggcgaaaggtatctttcagcagcacatcttcataaaaaatattcaactgcaatcaccgtgtaagcaaaagcttacgcctgctatattatttaataaacaatccgtaatgaatggaaaacgccatcgtaaaagttgaaaatctgtctcaccgttacgcttcccagtgggcggttcgggacataaattttgagatccatagccagggagtggtgggactgctgggttccaacggagccggcaaatccactaccatgaacatcatttgtggagtattaaaacaatcgaagggagaggtattcatcaacgggatcaacctgaaagatgacccggtaaccgccaagcgcaacatcgggtttatgccgcaaaaactgccgctgtacctcgatttcaccgtggaagaatacctcacctactgcgctgatctgcggatggtggaaaaaagccagttaaaaaaagcagtcgaccaggccctggaaagatgcggtgtggcacatttcagggaacgtctgctccgcaacctctccggtggataccagcaacgcgtgggcatcgcccaggccattgtgcacaaccctaaatttgtagtgctcgatgaacccaccaacggcctggatcccaaccagatcgtggaagtacggaacctgatcaaagaaattgcgatagaccgctcggtgctgctatccacgcacatcctcacagaagtacaggctacctgcaaggaaatcaaaatgattgaagaaggccagatggtattttccggcacactggaaatgttcgataattatattgaacccaactcactggtagttatgctggacgcagctcctgcacctgaagaactgctgaagctggaaggtatcagatctatcgaacaactggccccctcccgtttcaggctcggatacgacggggaaaagaaaacagcacagcggctagcggaaataagtgtgggcaaaggctggggactaacagaactgattatcgaaaagagttcactggacgcagtatttgccaggttgtctaaaaaaaataccaaataaaaaatcattaaaagatattcaatgagacaaatttttaagatcgccaaagcagagttattcactttgttttattcaccgatcgcctggatgatcctcgtggtatttacttttcagacgggaatgggctttgcagacaccctgcaggagatgctgcgtggccagagcagcggtatgggcctctcctttattaccgctaatattttctccggacaaaggggaatgctggcttccgtacaaaattacctgtacctctatatgcccctgcttacaatgggattgatgagccgggagttaagcagcggttctatcaaattactgtattcatccccggttacttcctcacagatcattcgtggtaagttccttgccatgatgacctatagcttactactcatcgccgtattactggtgtatgtaatagtgggtatgtttgtggtagataactttgaactggcgcctgtactatcaggtctctttgccatttacctcctgatgtgcgcctatgcggctatcgggttgtttatgtcttccctcacctcttaccaggtagtagcggctctcggcacattggtgctgctgggaacactcagctatatgaacaaagtatggcagagcatcgattttgtacgtgacattacgtactggctgtctatttccggccgttgcaacgaaatgatcagtgggttgatctgcacagaagatgtgctttattttgtgatcgtagttgccatgttcctggcactgagcatcctgaaattgcagtccaaccgcacccatgcctctttttcctcggtatggagcaaatatgcagttgtagtgatcgccgctatggcgctgggttataccacttcccgcccaatattcatggcttattacgacgctaccgaaaccaagcggaataccctcacccccaatagccagcagatcatggctaaactggatggcggtctcaccatcaccacctatgtaaacctcctcgaccgggaaggctataatggtatgcccgaaatggtaaatgaagataaacaacagctgaaacaatacatccgcttcaaaccggaaacaaagctgaaatacgtttattactacgattctgccagcaataacccccgcctgaattttgtttataaaaacaaatcactcgcggaaatggcacaaaaggaagcagagatcaaagacctcgatattgatctcttcctgacaccggaagaaataaggaagaagatcaacctccgggatgaaggcaatatttttgtccgcctagtagaaagagaaaacgggcaaaaggcatttctcaggatctatgaagatatgatgaaatttcccgacgaagcggaagtatcagccgttttcaaacgcatggtaatgaagctgccaaaaattgctttcctgcagggacaaggagaacggaaaatagaaggggatcgtataaaagattataccctgttctcttctgttaaaacattccgttatgcgctcactaaccagggctgcgatgtggaaacgctggatctttccggtaataaccagattcccgcaggagtagacattatcgtgatttccgatatgcagcaggagatggattccgtttccaaacgaaaactggatacctatattgccaatggcggaaacctggtggtgacccttaaaccaggatcagcggtcatggaatctttcatttcccaatttggcgtaaaaacaatacccggccaactggtacaacctaaaatagatgtagttgcgaatgccgttatatgccggcccacaaatgctgctatcagcatcgcacctatgttcgatctcatgatcaaacaacatgcgtatgtgggcatggtgaaagcggctggtttggtaatggcggaaaacaaaggctttaaagccacccccgttcttcagaccgataccatgaaaacatggaatgaaacgcagaccatcgattttgtgaatgattctgcttccgtagatgtaatggccggagaaagggcagatagctttgttacggcaatggctttatcgagaaagataggtaataaagagcaacgcatcatgatcataggagatgccgactgtatcagtaacgggggtatgaaaccgcctatcagatattacggcgcttccaacttttctttgattccgggtatgttccattggttatcttacggcactgtaccagtagacgtaagccgtccgcattcaaaagacaacaccctctttcttaccaaaggaagcctgaaggtggtgaaatacggattaatgggcgtgatcccgggattattgctgataggaagcagcattttactcatcaggagaagaagaaagtaaaacaaacagctggtatgagcctaatgaccgataaacaaacgctgaatgacctgaacattttcgggaaaggtggaggcgattcaatgtacacgatatttaaccgcacctttacccgcggcggctctgagctgctggaagaaatgttccgcagcccgctctccgacgctgccgccatcaatgcgcgcagcaccatcatccgcgccttttctgaacagcagataagctttccgtatgagggtgaatggttcgatgcagcagaacaacacctgcaaaataccgatgagcgcacgaagctgaatgaccaggaacatacgctgggcagaaagtttaatcacctgattgccgccgacacagaatacaaagccattgaaaaaggcgtggtaagcctgatcggtatcttacaggccacccgggtgtttgcagacagcatccggcaacaggtagcaggtattccttacaacagggaactcgcttccatcgaccggttattacaaacaacagaattgcagtccctcctgcaggaacataccaaacagaaattttcttttgccaaggtagcggagtatgataaaatactccgcttccggcaacggaacatcatcctccaattgctgggacatatttacctggccgatgtatacctgtcggtggcccgtactgccagggaacggaagttctgcttcccggttgccctggatgcggaaaagcaaacagtaatactggaagatttttaccatccgtctttaaccaggccggtggcgaatacattaaccatcactccttccagtaacattattttcctgacaggagccaatatggcgggaaaatccacctttatgaaagcgctgggtattgctatgttcctgggccagatgggattcccggtgccggcagccaaaatggaattttctgtaagggatggtattttcaccaccatcaacctgccggataacctgagccagggggccagtcacttttatgcggaagtgctgcgggttaaaaccattgcacaggagctaagccgcgacaaatacctgtttgtcattttcgatgaactgttccgcggcaccaatgtaaaagatgcatatgaagccaccatcgccattacatcggccatcgcacgcaggaagaattgtatgttcgtggtatctacacatatcattgaagccggcgacgtgctcaaagagaaatgtgacaatatcaacttcgtatacctgccaacgttaatggaaggcaataagcccgtttatacgcataaactggcctccggtattacttccgaccggcatggtatggtaattataaaaaatgaaggtatcctggacctattggccaggaaaaaatcaataaagaagaccacatgagctttattgccgataaacaaacactggacgatctgtcgctgcttggaaagtataatgccaattccatcttctccctttttaaccaggtaaaaacccggggggcagaaaaactgctggatgccatgttcctccatccactaaccgatgcggatcagatcaatgccaggagcactgccttccgttattttggagaacagcccattccgtttcctttcaacgaacaactgctgggcaacacggaagccttcctggatgaaggaagtaacagcagcttccccctcgccctctggcaaatgggccggaaaaagttagcggcccttctggtaaaggatgatgcatttgaattgcagctgcagggaatagatacctgcgtacagctgctaaaaggcttttctaccctacttgatcatctcgaaaaagaaggtcgtgataaaaataccccttgggaaaaatgggtcacaagtgcccggaacatcctccgggataagcggctgcaaaatatcaattcccaaagatccctgctgcaaaccgccaggttacactatctgctcgcacacatattccaggataagctaaaaaccctgttggcactcacctacgaaatagaagtgtatctcaccgtttccggcattgccaaagcaaaaggattttcctatgcaaaggcattgccgaaagagaagaatacgctgatagccaaaggggttaaacatcccggcctggataaagcggttcccaacagcctttcgtttaatggcaacagtaatgtactgttcctcaccggggccaacatggcgggcaaatccaccctgatgaaagcgaccggtatcatgatgtacctggcacatatgggatttcctgtagcggcccgggaactggagttttctgtgctggatggtatttattcttcggtaaatgtacctgatgacctgaaccgtggatacagtcatttttatgcggaagtgctccgggtaaaaaaagtagcggaagaagtaaatgctgacaaacacctcttcgttattttcgacgaactgtttaaaggtaccaacgtgaaagatgcctatgacgccacactggcagtaacagaagctttcaccgccttcagggattgtttctttattatttccacacatatctttgaagtgggagacgcgctaaaaacagcaggcgatcatatacagtttgaattcctgccaactattatggaaggtaccgtacccaaatacacctataccttgcaaaaaggtattacaacagacagacaaggaatgattattatcgagaatgaaggtatcttagacatgttataatgtttaagccgcttctttataacgggaacatgttacacacaaaaaccaacaaaagataaacatctatgcattatcgttatctggccatagcaggactgctatgtctttccactgcaggcagctttgcacagggctccggtcagggccagctcattccgctggacacggctgttcgcacaggacaattacccaatggctttacctactacatccgcaaaaacaatgagccttccaaacgtgcattattctacctggccaacaaagtaggctctatcctggaagatgaggatcagcgcggtcttgctcatttcctggagcacatgaacttcaacggcaccacccatttccccaaaaatgaactgatcgactacctgcaaaaggcaggcgtacgctttggcgccgacctgaacgcctttacatcgttcgatgaaaccgtttaccagttgcctatccctactgccgaccctaagatggtgagccgcggactggatattatgcgcgactgggcacaggaagccctgctggaaacagatgatattgacaaagaaagaggtgtgatcattgaagaaaaacgcctgcgcgaaggagcagctgcacgcatacaggataagacacttcccgtggtgttaaataatgccaggtatgccaaccgctcccctattggtacagacagcatactcctgcacttcccggcagccacgctccgccgcttttaccacgactggtaccgtcccaacctgcaagccctcatcgtagtaggcgatgtggatgttgaccaggtggaacaacagatccgcaaacaatttgcagacctgaaaaaccccgccaacgaaaaacccagacccgattataaaattgccctcaccggtaaaaatcaattcctgactattaccgacccggaagtatctgccaccaacctggaaatcgccatcaaacataccgccggtaaattgactaccaccaccgattatctcaataccgtaaagcggtcgttgtttaaccaggtactcggcgcccggatcggcgagttatctcaaaaacccaatcctccattcctgggcgtaaatgcaggcatcggcaacttaatgggcggactcgatcagttctccttctccgtaacggcgaaacccggcaaactggcggaagcctttgccgccggctggtcggaagtagaacaagtgaaacgcttcggctttacacagtctgaactggaccgggccaaagcagcctatatggcaagcctggaaaaagcagcaaaagaaaaaaataaaaccgtttctgaaagctacgtgaaagaataccaggcactgttcctcgaaggagctgcttctccagggttcgactgggaatacaacttcctgaaaaaagaattaccgggtatcagcctggatgacctgaaagcagttgccaacgaatacatcacagataccaaccgtgatattttcatcgtagctcccgataaagagaagaataatcttcctgattccgccaccgttacaggatggtttaaaaccgttgctgcagcttcgctggcagagtataaggacaacgttaccgaccagccgctgttgaaaaaaataccggcgcctggaaaagtaacagcgcaaaaaaattatccggcattaggcatacagcaattaaccctgagcaatggtgtgaaagtatggctcaaaccaaccacttacaaaaatgatgttatccagttcctttcatttgcaccgggtggtatcaataaatattcaaatgaagactttcccagcgcgtccagtgcaaacggtattataagtggttccggtctggctaacttctcacccgttcaattatcgaagatattaaacggtaaatcagtctccgtaggcgccttcatcagcggacgtagccagggtatcggcggcgccagcatcgtaaaggactttgaaaccgcactgcaactgatatacctgcggttcaccgcaccccggaaagacaccgtgttatttgaaaatgcattagcccaatccagggagcagatccaaacccgctacaatgatccgggcaatgtatttaaagataccgtgactgcagtattgagcggctacaattaccgcacaagccctgccaccttggccaggctcgatagcatcagtttggaaaaagcttatgaggtttaccgcgaccgctttgcagatgcgtcccaggccaactttgtatttgtaggtaatttcaataccgacagcatcaaacctttgctcgaacagtatctcggcgcactgccttccctgaacagaaaagagaaagctgttaaactgccggtacttgtacccaaaggacaactggtaaaaacagtcaccaaaggaacagacaacaaagccagtgtattactggtttacaacggcgattgtgtttacagtacggagaacaaaatgcagttgcaggcgttgtctgaaatcctgcaataccggctgctgacaagcctgcgggaaaacgccggcgaagtatacaccccttcggtaaatgcaaatatgtcgaaagaacccgatcagcgcttcggcgtaaatgtatcattcggatgtgcacctgaacacgtggaacacctggtaggactggtacaacaggatattgcgaatttacagcagcagggcgccactaccgatgaagtacaaaagttcaaagccggctttcagaagcaatatgaattgcagtccgaaagcaatgagttctggttacaatttatctccgggaaaatagaaggcaaggaagaattgaaagagctgcccaatatagaaaaacaattgagccgggttaacggtgcatccattaaggctgcgtcgaagaactacctgagtggaaagaatgtgatccgttttgtggcattgcctgaaaagaaatagaaattgtttttgagtgatgatgtaaaagccgtttccttttttgggaagcggctttttttatggagaaaattttaattacggttacaccagaataatggctccgttattttgcctatttcttccctaattttaatgatcatgtaattcttcttatcgaatggggaaccaatctaatagtaaatcctccccttacatcccctccaaactctactactacgagtaacaaaaaaggcacggaataaagttaacttaatctacctaaattcttcaaccatgtctaaaactgctcccctggtatggcttgccggcgccatactattcgtttcctgtaacaaaagcactgaacaacctgccaacattgaagccagtgccggacctgccttccccgttacttttaatgtcaacgattttacgcagcagctggacagctttggccgcatcgccggcgacgctccaactgcaaaagattccctggatggtcatgtaaaatacctttactacaaagtgtatggtacgggtgcacaggcagccataaaacatgaaattatgcaggaagttggtaccccttcttttggtgtaatcagggatacattgccgccgggtaattacaagtttactttgctggctgcgggcgacaagtatctttcctacatcaccaatgccgggtttaaatatcccggcagtgatgccttcagcactcacttcgaaatggtggtaaacggaccggctaacgccaaagtttccctggatcgtattgtggcaaggctgcaatttattatccaggacccgctacctgctgatgctgcctggatggacatccagtttgggggcatcccacgggtgtttaacttcccgactggtgaagtgagcaaccctgccaacggtaccgcttattcgaattacatgggctatacgttccagatacccgcctataaccagggaaagccgggctttaaaacacaggcatattttcccctgcagggcagttacatcgtgccttcgataaccattgtctgccggagcagactgggcaatttgctggccaacaaagttattaacaatgttaagtttgaaactaacaaacgcaccgttttaaaaggtaatctctttgcgccaaccagcagtggtatagaagtggacctcaacgacaccaactggaaagcagacagcatcgctgtattctactgacagtcacttttattgctatcattccaccagcagcttctcttatgggaagctgttgttattggcagcatcatggtatgatttgtgggttccatccgcacaccaaactactgatgtatgcatattgttttaggcggcacaggacatatagggtctgcattggcagaaaccctgattaaaaagggggagccggttaccattatctcccgcgatcctaaaaagaaacagcaatgggaacaaaagggagcggaagtggccatcgctgatgcgctggatgtaaagcgtttgcagaaaatatttaataccggcgaaaaattatttctgctcaatcccccggcggatccgtcaacagataccgtagcacaggaaaaagaaaccctgaacgctattcttaccgcactcggtgaatcacagataaaaaaagtagtagcggagtctacttatggtgcacaacccggggacggcctgggcgacctgggtgtgctgtataacatggaacaacaattggctgaaatgaatgtgcctgccagtattatccgcggcgcttattacatgagcaactgggccacttcgctggcaacagcgcgtgaatcgggtattgtttataccttttatcccgttgattttaaactgccaatggtttgtccaggggatattggcagcgtagctgcccggctcatgctggaaccggttacccaaaccggactgcactatgtagaaggtccgcaacaatactcggcaaccgatgtggcagaagctttttctgctgcattgggtaaagacgttaaagcagtggaaattcccgaaaccaactggatgcaggcgcttaaagacgccggcttttcagagccggcagcaaaatcaatggcagcaatgacccatgttacgctcagggaaaaatacgaggatcccaatcctgtcaggggtacaaccacattaaaagcttatatcgcggatttagtggaatcagcagcgtagagcgactataaacccatcggcatccgggaacacattttttgtatatttatttgttgctccctttaaatattatttaacagatgtcgatacatgtagccattacaagaaaagtgcttcccggaaaagaagaggaatttaaagaagcgctcaggcaattcctcggtgaatcatttattcatggcggcgttcacggcgctgccatgatcacgtcgctgccaggttcagattccaatgaaattggcatcttacgaacttttgctgatgaagcagaaagagacgcattttataattcaaagctttttagagactgggaagactttgcctcaaaacttaccgaggaaccggtttacaggccgctaaccgggctggaagcctggttccgctaccctttgccgccaccacggtggaaaatggccattaccaccttatgcggtgttttccccaccagcctgttactaacatacacactcggtccttaccttcaaaaactgcctataccgctacgggtatttattgtcgcaggctgcatggtagccttgttaacatgggtagtgatgcccgtaattacccggctgttgaaaaaatggttgcgcccatcatgaaaataataaaaagacgatgtcatctttttctatttttgacctgttaaatgaggtatgccgggcctgaagacttcgcaccgcctcacattgattttaaatacatcatacgctggatgaaagaacaactaattacgttaattaaaaatttaaaagacaattcacttagtttcaaagaggtgattgaatttatagaaacttactatcaacaccagcctgcagcctttaaaaacggagaggtgcataatgaagccacccaaaaccagggaagtgcaaaggtgtttgctttcgcgcagctaaataacctggacaaagaagatacactgctgttatttgcagaacactaccaggctgtattaaatacaccggatggcacagatcaccagaatatcaggcaatttatgattcacggctggcccggagtaatctttgaaaggcaagccctgcttgcgaaataggtcacaatacttcttttgcagaggaaaaagattgtccggatatcccgcaggcatatccggacatctgctttattacacacgttacttacctaatgcgatttttattgcttcctctaccggactgcacgggcctaaaccactgatatcaaacccggttctcagtaacagcggtggctgggccataaacttaggtaccaggccacgatgccgctgggcagcatgcaccaggaacggatgacagagatataccgtgccggcctttcctgtagccaatacttcctctctctcaggtaatcccggcaacttcgttgccagttccatgaaagaaagtccgtcttcaccttccggccccagcaatcgggcaacatccatatgtgagccctttaaaatcctggttggcgcatcccactcgctcacatccgaaaatagaaacagcatcagcaaggcacggcctttagagtttacattgattctggctgcgaaaaagtcattaggatctacaccggcaaaacttgcatctacatgccaaccggtatccccggaatcaacttccgacgggaaacgaatgggaaaggaccccatgctcatacagggaatccatttttctttaccggccagctgatcgaatgcactatgaagaacggtggtattcgcagccttaataaatggctcctgtgcatacatgcccagccaaacgaccggttttgtccaggtgttgctgtcgttgggatcggccggaatatctttccaaagaatatctcttgcttcgctcgcaagatcagcagaaaaagcgttatcgatacggacaaagccgtcagtaataaatgactgtatttgttgaggattcagggtattatgcatcatgttatactataaaagttcagacaataaagaattgatgcccctcggggcacattggtcttagtggacttgaaaatttatattataacatcacagtcattctcatacagcaaatttattcatttgttttaaaaatacaagaggataggatcatatcaactttctgcttatcttatatgataatggcagagcaattttgtcaccggatcccattaaaacgcacataccgctatgaagcacaaacttttcccactgttccttccctttttgttggtccctgttttcctgtatgcacaggattttagtcatccggggcaatttgttcttaagggaaaagtgaagcattataaagataaagtgtacgaattcgggatgtccaccttttttggcagttttggagatacgatccggatcaaagccgacggaagttttgaacaaacggtgccggtgcagcaacggcagcatatatacttatacctggacgacgatcgtccctggtttaccgtggcagacaaggatacgatttacctgcaatgggatcagaaggaagaagtatcctcccttactatccgcgcccagaacgagggacgcacgaaagagataacgcaacaattacaactgcataaagtcctgtcggaatcatttagcaatctcaatcaacagttgagtactgaaatgaaaaatctcactgcagaagaaaaatttaaaaagataaacctgctctttaacagccaggcaaaaagcatatttgaagtaacggatactttttcccaattctctaccaggcaaatcagtgccttgtattttgagtattcgaacctcttatttatgttgcggctgctgccaaagtttgagctgagctttatagcggatagcgttggcaagtatacacaaaagcatagcaccatccaaactacccattacaaaacgttaaatgaaaactggttttggaacgtaccggagtaccgtactttcatttataattatctgcgcatggcccgtccgtttaatgcaactataagcgcaagtatccaaaccgctcccaatacaaaatctaattacacaatggactattatcacctggcagaggccaatattcctttcacggctatgaaggattggtttattaccagcagtatcatgagtgggtttgaatattacgaatttaacgatgtaaaaaaagtatatgatgcgtttatgaatacttgcaacacgcctttcctgaaggatacgctgcagcaatattataccacgattgcacatttaaaaccgggaagcccggcgcctgatttcactttaacggatgccacggggaaaaatatctctctaaaagattataaaggaaaagtagtgtacattgatttttggggagtaggctgcgggccctgcatttatgatatccaaaaccatgtgccgcagctgcataaagactttgagcataaggaagtggtatttctgaatatctgtgtggatgaaacagaagtgaaatggaaagatgcccttaagaaatatcatttggaagggataaacttggtggcggaaggatggacagaccacccggtatgtaaagcgtataatgtaaatggtatcccgcattatgttttgattgacaaaacgggtaagttatccaataacaatgcgccacgacccagtgatgcgtcattgaagggagctattgaaaatttgctgaaatagggagaaaattttcatcttcgataatttccgtcccgatctttacacctgttctaaaacccggatattctatccagctctatgacgtgcattccgggcgcgagtactttcggagctttggccattttctcagcaagcgtaaacgtaggtaatggacggaacttcctgatcaatcccaaaaaattcagcacttttaatgcccccgcggtcattcgttcacccaaccggttggtattcttccgcagcaataatcccggcctgaaaatgatgtattgctcaaatgccaggctggcgatcctgtcctccagattgccctttaccctggaataaaatacactgcttttggcagaagcgccgtaggcggatagcagcactgctttggtaacaccgtttcgtttggctatttcagcaaattttgcaggaatatcataatctatatgccattgcttttccttcgaaccagctgctttcatagtggttcccaaacatgaaaaccatacatctcctttgataacctcagattcattttctaatttgttgaaatcaatcacgatctctatcagtttgggatgaacaattccggtggaacggcgcacaaatattacaacggctgtgtagtcacggtcttgcaacaatacccgcacaagatctttgccggtagcccctgttgcccctatgattaatgctttcatacctggaatttagtttataaccggactacacctcctttgatcatttctttaccaaccaactttccactgcccttgaaaaatcagctacatcaataggatgcctgctggtaatcaggtttccgtctgttaccacaggttgctccaatacaatcccgcctgcattcttcaaatctacctgtatattccaataacctgttaattttctacctttcaaaatatcggcagatgctaatacaacaggtgcatgacagattgccgcgatcagttttcccgatctgttgaaatcctgtataaattttattacatccttatcgtagcgtaagttatcagggttccatgcaccacctggaatgaacacagcgtcgtaatcacttacctggatctgatccgcagtacggtcgaattttagccagcccacaggctgtaagtattgtatggccatgatatgtgtttttgccatttcaggaaacataaggccatatctttcgggcgcaggaacgtattttggtgccacgatatctactgtagcacccagttgcctgaaataccacacgggccccagtaattcaatttcctcgaaaccgtcggcagcgattacagctatttttttaccttttaatacggttacatcctttacaggagtaaaaaagaaagcccgcaaagcctcgtttccgggagcatttaataattgtgatacgggcatgtttaccactactgaaggagaagccaactgattcaatacagacagctcatggtcattgatccgtgtagtacttactttatcctgagcctccgcattgaatacagtaagaacccctgccatgcctgtcatgacgatttgatgaatagctttcatttttaaatttttattgttataaatgattgtgtttaagtcattgccgccttcaaggggcaaaggctatcagtctgtgaagacccgtttgaaaaggctgctttttgatgctggtattcaaataatcgatcacaggttgtataggagggaaatccagatgataccggaaggcatcttcactcctgaatttttcataagtaacaaaccgggtactatcttcttccatttgtgaaagctggtaattaataacacctggctcgctccggaactgcggcatggcagtgtgatacacttctttaaaattgcgttcggtaccttcccggctatccacaaacaacatgatagtgattggcttgtcttcttttaggggcctccgctgccattcgttctttgaaatcggctccaggtcttttatgtagattatttttgcaggttgtatcagcctcttttcagataataactttatcgggttgtatttcacacctcctctcacgttctccaacccgtttttgctatcccatctttctataagccacaacacggaagggttttcctgctcataatacgcttctgccataatgttgcttttatgagcgatagcatacttcacgtacttacgaagcgctttgctgaacttctttttgtaccttttcttcacctcgtacctggttaacgcggctacttcttccgtttggctatgacctgctgctaccaatggattcttctctatattatcccgtttttctgccattgcaaatgggctgctaaccaagaggcacataattataaatacaggaaccttattgaatagtgataaaaacatttttgttgccattactttttgtttttagttctcatcaatttgcttcaccctgtgctattgtgctatcttaagcaacaggtctgcaactacctgcggttgagacaggaatggcgagtggctggtatttacactgtaaatggttttgataccggctccggcgatcatacgatcctgcagacccggtgagatcacaatgtcccgaagcgttttgatatacaccttttctaccgtgccaaaggcggctgcggttaaggtaaccttgtcgccaaatggaatggccggttcagcgcgatagttatcaattacctgttgcttggcggccggcgcaccatcgttgatgaacaaataggtcaaactgtcgcgcgctacatcaagtgtcagcttatcagcagacagcgttagcaacgggccaagttttgagtcagggtctgaatttgccaggtcgccaagcgtttgtcctgatgttggaacaaaggctccgatataaaccagcttactgatttgggccggcactttctccgctaccgcggttaccactacgccgcccatgctgtgccctaccaggattactttttcacctgctttattgatcgcgtcgatcactttatcccggtaaacatttaaagtaagcgtgtgagccggtgtttggtcgctaccatgtcccggaagttctacgacaattactttgttgcctttttgttccagatcgctacgtacggcattccatacataaggcgcctgccaggcaccatgtaccaacacataggtctgttttttggcaatcttgtcatcatcattattattgcatgatgccaatgtcgaaagtgtgaaagctgcagttagcagcgataaaactatttttttcattttgtaaaaatttattaatgatgcgggctttgttcatttgactgatttatatttattcattattgccaggcgccggtatgtcaaatccgttcagaatcatagcgatgaaagtgtagccgctgatcaggaagaaaagttctgccacaccatcctttcccagcagatttaccgcatgattataggttgaatccggaacaatgtgaccagtcaccaaggcatgcacaatgtcgtgcacgatggcctcctgttcgtttaaaccggatggacggctgccagcggcaagtgtggcgataatacccggcgcaatgtcaaaagctgctgccattatctcatgtgcgtaaagctcaaagcgggcaccataagcaccacctaccgttaaaatggcaacttcccttactgttttagaaagtgttgcgtgcgtgtcgagcgtccgcagaaaactcagggctggtatgccaaactgtggatagtgcagcatcggcgcaaaagggcctaacaaggctccctgtgcatcgagcatgtttacctggctttgactccggccaacaagactggctatctcgttgtgtacattgcggacctcagggctaaggatatccggtggcaatggttttatacgcatgatgcttgtttgtggattaaacaatttcattggcaaactgcccatcgatcagcataaacatcatacggcagatcttaccggaccggttagcccaggcatgattggtgccgttctgaataacaatatcaccagcctggatgatggtctccccccgatcaaggatcaatgttatctctccttcaagtacaatcccgtaatccaccgtttttgtccgatgcatcaaggggtgaggtgcagctccatctgatgtggaggctttctcatcacccataatcctgaatttcgcggcagcatctgcagaggtaagtttctgtatttcttcgccctccggtggaaattcgatgacccggatgcgggtaccacttttagggggcggcaataccaaacccggttcatcccgctcatccggttgagcctgaataaaagcaggtgtttccaacgtatgccatacttcaaaaaaagtaggaccacccgggccgccaacaagttgtgtatgtactggaggagcatctgaaataatgattgccttcccgtttgcatcatgacctgttacaatacgcctgaatgcttttggttgctgattcataatcctggtctttaattgctttttgattttttgaaaacaaataccccgaggtaatgaaagagtatacctattgcccacgctggtgtggaccacagcggccagggataggtccggtcggtgaggtaccataccagccaggtggccggggtggcaagcaggaaaacaattaggtggatcctgaaaccctttttaggatcgataggggtagttgggtcccattgagttgaatatgtcatacaaatggttttgttgtttcatggctacttacatgccatttagcagaaacaaccctaccagaaaagtgtagatcattaatgaattgaaaaacaattttttagaaaaatatcaatcaggcgggggcgaaaaaaatacaggcaggttactccgaaacattggagtttaataacaaaactccggaaatatcggagtttgcaatgctattgatcaataaacaggaagaataaaattctaatcagtaaaaaatgctatatattgtataaaatgctttccatgtattccatcccatggccatgaaataagcattaaaaatccaatttgctccgaagatgctgtgatgatatttgctttctgagtcaaagtccctaaagatccaactcttcccagagttattaatttaaaaagaataacatgtccaggctgactcttatgtacatactgttcggtgtgctgatgttttttgacggacgatctcaaagttctgccaaaacagaagtgtcaggctattcttactatcatccgtcgaaggataaagagtcatggcagcggctgaatttgttgcttagctccacttatattgttgttgtaaaagaagggcagattagccatgatacttgtttatatatggccagccgttccctgggtctgagccgctttccggtgttggcggaaggaatcggcggcaacaaattgtttgagcaatctcattggattgaccggcgggaaccaggcgttggtattgatcgcctttcaaaagcaacaggccgggaacacctgcaattattgatactcctgggatcctactatgcttttcaacccgctaactattacggctataaggacagcgttgaatactttctgaacaaagcagtggaagaaagtaaatctttgaaagaagaaaagctgggtagaatagcactttgcctgcttggaaaaatgtatgtacaagtaaatgacagtaaaggtgattccatttataaccggctgatagatgaaagccggaaggccggggatagggaaacagaagcaagggcatttgcctaccgcggcatgtatacaagccccacgcgtgctaccctgcttacaaaagtcgccgacctgcagaaagcagcggagctttatcgcagtcttggcaatacagaagcggagatcaacgtattaactgatttaggctatctgctcgttgtaaccgggcaattgcaaactgccaatgaaatgttttcaaaagcactggcgctggctgaagcaataaactatccatatatccattataatacggaggcacttgctatggttaccatgtttcaaggaaaatttggggaaccattaaaatatatccttcaaacaatcaaagtggccgaaagctgccgggacagtattggctgggggtatttttatagccggctgtcgttcctttacgatgcagagggcaggcagaaagagagttttgatatggcgcaaaaggcaatgaaaaggttccgcatagaccgtaatccaacgatatacaacgtgttaaatcaggtagtaaactatctgaacgcagatgggcgtgcaaaagaagcgcttaaccttacgctggatatgacaaaaaagatgggtataccgtcgaatatttcggagcaaatattttattaccacacactttccaacagttatctatacacgggcaacctggatctggcggagacatacttaaaaaagatagactcgctggaaaccatagcggaaggcatcagggggccactccggagaacttcgatcaatgatcaatatgcgatcatcttgtttgggcggggccagtaccggagatcaagagaattatttgaaaaccattttacaactatttcatcagcagcccgggacttaccatctgacctggttgcataccgctggctgatcagtattgattctgcgctgggcgacaaagcgtccgcagcatctcattacgaaaaatacacacagttgctcgactccagtttcagagtaacaaaaatcaggcaggcagaggagctccgggtaatgtacgaaacacaggaaaaacaagaccagatcacattactacatgaacaggcaatactggaaagggctaacttaaaacaggccaaactggtgaaaaatctaacgcttggaggcattgctgccgtaataatcattgccgggttattatactggcaaaaccgcttaaaacaaaagaataataaaataatcacggacaaaaatgagcaactgcaaaagttgcttactgacagggaatggctgttgaaagaaatacatcatcgtgtaaagaataatctgcaaattgtaatgagcctgctcaattcacaggctatatatataaataacgatgccgcatttacggccatccaggacagtaaacgccgggtgtatgcaatgtcgctcatccatcaaaagctttaccagtctgaaaacattgcctccattgccatgcctgaatatatcaacgagctggtgaaccatgtccgggagagctttgatgccgggaaccggatagtttttgagcaggatattgaacccctggaccttgatgtatcgcaggcaatcccgttgggattgatcatcaacgagagcattgtaaatgccattaagtatgcttttcccggtgatcgtgaagggatggtgagtatcagcctgcgacataatgcgcctgatcagctattgctgagtatatcggataatggcgttggcctgcctgctgaccttgatatactggaaaataactcgctggggtttgatctggtacaggggcttgcaaaacaattaaaaggccgctttaatattacaagcgatgacggtctgcgcataaccatcagctttgccgttgccagcaaacaaattccggatgaagctccaggtaacttttaagcaacaaattttatgagtaaaagagtgcttattgttgaagatgaatttattgtagccaatgatctgcggttaatattagtacgcgccggctatgaggtaacaggtattgccgcttcagttgaagaggcgaatgaacatctgctgaagcaagaaccgggtcttgtaatgctggatatccggttagaaggaaatcaatcaggtattgactttgccaggaaattaagagctgaaaatatcgcttttatttacttgtctgcctacgcaaatcaacaaatactggaagaagcaaaaacaaccgaaccttatggatttcttgttaagccattcaaggagcaggacttactggttaccctggatattgcatggtatcgtcacatcaatagtcttgaatcaaaattgcggcaggaagaacatttgcaaaaacagttaactgcaataagcaatgaaacttcagatgcgccacaaaaattattgaaggtggccctggccatacagccttttataccatttgattttattacatcgggcatcaggccgcttgatgctgaacagtttggtgatacaggatatttgcgtatcggatttaatgaatatcagtttgttggcgaaaaagaattaatgacgattacaggtttaaataaaaaccagctttccgccattattgaaaatagttatacagatagcaacgcagttctttatagcagtaaaaacatcaataaaaacacgtccagcgcttcgctgcaaaggttaatgctggatcatttccagctgaagtcatatcttgtatttcccgtcacgttggggtatggcctatctgttcactattttttctacagccggcagcctaatatttacaccaaagatcatatagccttattgggccgcttgaagctatgcctggaagaactggctgaaaaaacaatctattataaaactccaccggccggaacaaagaaccggtcatcttctgccaataaagcaccgcatgaagtattaaaccatgccgggtttaaaaatatcatcggaagtcatcatcttttgttgtctgcattagatcttgcagcgcaggtagcgccgtatagcacttctgttttaatattgggagagagcggtaccggtaaagaaaaagtggcgcaatccattcacctgtcttcgcccaggaagaacgggccattcataaaggtaaattgtgctgctattcctccaacattagtggaatctgaactcttcggccatgaaaagggtgcatttaccggcgcctttgaaaaaagaaaaggacggtttgagcaggctgatggcggcactatttttttagatgagattggagaattgccacttgccatgcaggtgaaattattacgcgttttacaggaaagggaaatcgaatatgtaggtggcagatcacctgtaagagttgacatccgtgttgtggctgctacaagccgaaacctcgaaaaggaaattgcaaacggaaatttcagacttgatctgtattaccggttaaatgtttttcccatcacactgccccctttacgggaacgaaaaactgacatcgaagcactatccatattttttgcagaaaggttttgcagggcgttcaataaaccattcaatggcattgctgcatcaatgataggcgaactgtacacatataattggccgggcaatattcgtgaactcgaaaacatcctggaacaagccgttgttctcaatgatggtaaatcgaaattgcaattagtacgaaagctttcattaccggcctccaatctccctgtcagcactggtatcaacaccctcgaagagatgaagtacctgcatcaggaaactgaaagagactatatcatttccattctcaaaaaaacaaaaggccggatacggggagccaatggcgccgcggaattattgaatattaaacctactaccctcgaatcaaaaatggctaagttgaatataagaaggcgggattttatcaatgcagaaggaaatatataacacttattcacttaaccgtttacctgattgttccacttttaaaccgccagttcccatccggaacggcatatattgttgatacaaattgacttcagcgcataactttgatctcgtaatcttctgttaatccgtaatcataaacgtcatattcattccctggtggctgcgtttttacattgtaccatttacccggatcaaccaggcccggagccggcttgttgtaaaatggtcctaaaacattcttcaaactgccggttacggttacttcaatcttattagttcccttttttacaaattccccgatagacaacctgtcgggttcagcagtgatgacgccggcaagaatcccattgaccttcaccgctgccacagtgcccttccatttacctaactccactgcatatgacttgccgggatctgccactgtaaatatcttcgtataggtgataccgtgtccatataaaggcaatccctgtttgttccagtaaccaaattgtaatagttgcggtttaacaatgctccagccacgtgatgccgcttccaggttgaaatctcccaaaatataaaccggttcaatttcagcataaacgctcataggcgaaacggttacggccagttcattatctccggtttttaaatagctgccgatctggtatacgccaaaggagcggtccagccaccattgcccgggttcgtttttaatgtattcaccattaatttttacatcgtgccaaagttcaggttgttctattaccgctttgaaattccggaaatcaacgccagcctccacattgaaatgataaaccgccgtgtacccggtaccagtggaaaaagtatcccggcttacaatcgcctgtttaaattgtgtacggttattccagggattgcctacgccatccgtaaatccgtggtgtttgaaagctgtattggaggctacaccaacgtgtatattggtataatttgaatccggcttatgtaaatgaagatcgcagaaatcaatcgtcaggttgttgtcaaacggcctgcttattttagttgcggaagccttcacagtagcccattctgcagccggtgcttctattttatatcccggtaatttcttatccgcgataaacagtacctggcttccggctggcggaatattaaagtcgaaatgtacctcctgatcatgcagcgaatagttaatgcgggaaatgtttcccgaattcatatccatctttaacacatcctgtccctgcatgttgatgctgcccgaagaaataccggtcatgctggcattggtcagcagtaataactccccgttagccagtttacggcgctgatgataaatgttaccaccaatgctgtcgcctgttccacccgatatgctaaagccttcatgatggaacaggtccggtaatgcctcccggatctggctgatggtggaaagctcattgttcactgttccatctactaatcgtaattgttcaaaacagatcacccttcctcccgctgcaatataatctctcagtaaacggaaggtactgctgtttatattttccatacctggcggaatcactaccaccttgtatgcccgttgtcctactacaaagctgcttcccttaacactgccatgatctttgatcacgttttctgaccctaaatcatattccagatgcgatctttgcatctttgtcacgaaatcattaaaacttttggtgatgtcgaagaaacgtttgttctccccgtctctggcataatacatccaggccgaagtggtgggttcaattaccaggatattgttgtactgctgtcctttggataataaataagataaacgtgtgaagtaatgattcatgaaacggtaatagggccaccatggctcatgataagagaagctgggtggataatcgtatttgcgtgctcccgtcagcgtcataaacgataaatgctgattcaaaaagttaacgcctaatacaaactcccagtcggcaaggcgtttcatatccttaaaagtaagttcccaaccggcgccaccataggtttccgacagggtacgtgttttacccaattgattagctacactccccagctctttgacggcgcggatattgccaaactgcaccggtttatcttcattaaactggttgaacaacatatcaatacccggcatttgatgccaggcatacatggccatattatctggtccgtgataaggacttggccaaccatgttcccaataatgcccagtccaggtaagctggtgatcactcatataggtggacacgggtttagaccaccggtcaataaaaagttccagcaaaacctggtagtaattatggcgtacccgtttccaatcgcctgtttctttaaacagggatggcagatgtaacctcagatcgtactgccagtctttataaaacctgtcgaacagatcaggagtccagcgtacacagttatgcccttcgttgatgatggttggttcgtcagaaaaaacgcccttgatggttttgccaaattctttgcccaccactttttcataacttttgtatgcgatgtctatgaacttatccgtaacgcctttggccatcagatctacataagacacgcctataggacctgccaccgagccccggttcgatcgttgataatttacttttttgaataactgataatgtccggttttcccttcttcgtctttcaaatcattcgttacatctttataagatccattttcttctttaagaaataaaaagaaagcagaaaggtcagcaggcaaccgggttgcttcttccatatacaacatttgaccctggttgtaggcttcgggcatttgctctcccaccaatccgccggcaaagcctgtagggtatgagttttcgtcgtatatccagatattgagtcccagtttttttccctgctgaagggcatattcaaataaatcaaaccactcttttgataaatactccgtaattaaaccggggcgtggatgaatgatcacaccgccaaagtcattcttccggtaatcattcagcatggaatcgatatttcttttggtaattttcgtattccatacccagaatggcacggtaccatagtctctgccagggtttttaaaccccgctgcaacctcttcaaaacgttccaatggttgttgtgcatttgcattggaagaaataaatacggcagcgatgatcaaagcactgcataagaattggcggatacttcttggcatagattatgttttcggtttattgttattatccagtacggtacgcgtgataatgcttctgtggcctgcggaagtaacaaccaccgttttaagaatgattgtttttcccctgggaatcgtaataattattggttcccggtattcgtgatcataatcgcccggcggccggttgttcagcgtgtaaaatatcctggctccccgtacaggtggctgcacttcaaacctgaaggtaccggttacgattgttgtatctgtgcagttaaaaacggtgggtacgcggtagttgataccggctttgtcgaagcgctccaggtgcaatggtaatgctgtgccggcgaaacgtggatagtctttggccgtttcatctgaccatcctgtttccgccagcgccagcatacgtggcagcagcatatattggagtttggatacatcaggaatgctttccgtccatatgcaggcttccacgcccataatgtgtttatgttcttctccggtcaatgcggggtattccgggttgtactgataagctttccataccggctcattacctccatgactggatggttcctgatctgaagtgctttgcgcatagtcaaaataaagtccgttatgaccgggcgccagcactatgttcagccctttcttaacttgctcaatggcgcccttttcaccaaaccggttcatcaccgtgatgctgtcttttgcattgcctgctgctacttcatcccaggcaatcagttttttgtgtttggactgaatgattttgttcagccttgaaataaaatagctttgcagctcgtggatatcattgatatgatgttccttcataaagtcctgcacggctgtgtctttcttccaatatcctttgtagcattcatctccgccaacatgaatgtatgggtaagggaacaatgctgctacctcgccgaatactttgtcgaggaatttgtaaactctttcatcaataggattgagggaattgtctacatacatttcaaaatcacccgagggaaaccatttggcgaagctgctgcctggattcactttaatatcagaattctgcgtaacacacagctcaggatatgctgctatggccgccatagagtgacctggcacatcaatttccggaagtatttcaatatgtctttcagcagcgtaaaggatcacttctttcacttgttcctgggtgtaaaagccactatcggtggcaagctcgccaggttgtggaggcagggtattgccgccgaactcgatacgtggcacacgccaggcgcccactttcgttagttcaggacagcttttgatttccagccgccacccctggtcgtccgtaagatgccaatgaaaacggttcagtttatagtaagccatcaggtccagcaggtctttgatctgttccaccgtaaagaaatgccgggaaacatccagcatgagtccgcggtagccgaagcggggagcgtcttctatggttagacagggaatagctgctgttccgcttgttgacacggacaacaactgcagtaaagtttgcataccataaaacaagcccgcgtttcggccggtgagggtaatgcggtctggtgttaccaacagccggtatccttcttcgggtagttgttcagcaccggtagcagtgatgagcagttccggctgcagacccgctgcttgtgcagtgcctgtcattattttgtttctgaacttccaggtactgaacaaacgatccgtgaaatactcaacggcgcgcttcccccgaacgtccgtccggatcaacgtgttggcgttgaagagaaagttgcccgtatccatttttacagaacgcggcatgggaaccagcgccggtgttgcctgctgcgcaacactgctgccggcactaaagcccagtaacgccaggcaacaggtatatatctttttgctaaagtacatcactgataattgtcgtaaactatttttattttgtagaaacaggcgccgttcactattcttgatccctgccactgcccgcctgatgtatagaagtcaaccgtgctggcagaccagttattgagcaggcaactgatggcaggacgcggatttttattagcgtccggacgcaccagtacaatctgtccgctgggttggttccctatcccttttacaaaggtcaggttgtttgtgggggacatggaaaaggtttttgtagttttattaaagacatattcccctccgttggtagtgacccataacaggttggtattaccatagtacgcgcttacttcatggccccaggcagtaggtaacgtaacccggtactgtgttagttccgttaattccgggttggtagcattgccgccaacagccagggcagtgaggatatgcgcattattggataaatcctgaccggtaacccataatccattaattaccgggtcccataatacggcatgtgccgcgcccagggtaaactccgcataagtgttgttatccgccccctgtgaggaagcatacaccctgatccagttaccatcagatgctgcgagggcgatgttaccattgggcagcagctctgctgaatgcagattcccgctgatcacttttgaccatacccgctgcccggatggatagccaatcaatgccgccatgccgttgtcgctgataactgcatagctggcatcctgccagattttcattttccgtactttgaaatcggtgcctccaccaaaactcttaatttcatttgtgctgaagcccagtgcagtggtaggagaccatctccacttttttgcatccgcggtgttccagtccgtgatcattggatcatagatctctatctgcttgctggcgtcattggttaatgccagctgcagtcccggataaggctcgggagtttgcacagttggcggaccgggagcatctgctcccggttttttactgcaggccatctgaaaaacaaccaaagcgatagcagcgcccatccgtattattctactcatcatatcaataatagtttggatcaaatgctttcgctttataaatagcagctccgcttacagtacgggaaccggtggcagcaccggtggtggcattataaaaattaaccacggaggtacaccaattactggcgggatacaatgggcagccagtgctgggtcgtgtttctataagcgtattctgtccgggttgactgctgatagatttcgcaaagattccataggccgctccgggcatgtcgctgaaggtttccgtggatatatgaaaaatatgaacaccgccattggtcgtaatcagcagctggtccgggttattcacatcggctgcaaggtcgtgcccccagggacgtggcaaagagtcataagaagtatccaaacgcaacttggggtttgtgatagtgcctccggatccgggagcgttataagagtattttctcagcgcatttcccagcgcccagagcacctggtgtgtggcatcccaaagcaccgcatgagcggaggcaaaatagtattgtgtgtttacgccatgattgggtgatggctgtgacgatgaatagatacggatccatccctgcggccatttttcgccggcgctggcaaccacacagttgccatcaggcagtatttccatcgcatgcaggctggtggtatcattaaaacccattacccagagcttctgcccctttgtgcctgtaccggtataacgggctatggtggccaatctatatgacgtggcggtgatcacctgcgaggtgccggcaaacaccgtattgttcctcaccttgatatctgtaggcgccttccagagaggtatttcactcgtggcattgtacgacagtgcagtggtaggcttccagacccatttaggcgtagtccaggaagcatctgccggatcatatatctcaatgtcgtttgggacctcattcgtaatagccacccagcaacaggttgccagttctgttttgggttgcacctttgccggcgattgatcttcaacttgtatttgatctgcccgccgggagcaggaaactacgagtaaagccaatacaattgctttccaattcacacaggtagatcgcaggcaggaattacctgccttcatcataatttttttcatgactgtgagttttagttagtaacctggattctgagtaagtttatcattcagtaatacttctgcattaggtattggaaataacagccggttctgggtaacattataacttcctgcctgcagataactatacttcgccttttgttgaacaccaaaggcattcattacggcgatggcattgcctgtccgaaccagatcgagccaacgcttattttcaaaggccagctccactcttctttcctttaaaatgaccgtttgcaatgctgcctgattggtgctggtgatattatgtaacgcatccccaaaagcgcgttctcttactgcgttcaaataaggcaatgcttcacctgatttgccctgttgattcaggctttccgccagcagcaataaaacctctgaatagcggtaaaccggccagttgtcattggtttgattaccgatcgtatgcgtatgcaggtatttctttggaaacggccgcccgactttgcctgccggcgctgtataatctacggctgatttaaccgcagtagccgtaaaatcatcggtggcattgaatgtaccttcggctatagcgatcgatgcatcaagacgttgatcacctgattcatatgcattgatcaggtcctgtgtaggggtgttaaaaccacccacagtggtaacgctgttaaagtttacgccagtaaccaccgtagtgttgaccatgcgtggtaaaaaattataaacagatgcctctacattggcctgtggtacggccagcccggtgttgaactggatttcaaatacagactccttaccatttttattcaccagctgaaatgcatcgccataacctggaaacaacgcatagcccattgcagttacctgttttaacgcattttcagcgaggtcatatttcttcatggtgagatatacgtcacccagcagggtcaacgccgcgccctttgtagcgcgccctgtttgcggaaaagtggtggcgctcagtttggcagcggcatcagtagcatcagcaatgatcaggtcgtatacttcctgcgcggaagagcgcgggatgtaagtctcttcacggttaagcggtgcgtgtttataaatgggcaatccgccgtaataacgcaccaggtcgaaatacaccagggcacggataaactttgcctggcccagaatagcgttgcgattggcatcagacaacttaatatcatcaatatgatctatgatcacattcgccgctgatatggcgttaaaacccaaattccactttggaggtgtctggttattatatttatcatccagaaaatctgctactgcgtaacggttcaccgtggctactgcctggtcagatgatttgtaatcgtagtgcgtgttatctgaacgcatttcgcccattacccaggcgcttctgttattataaagcccgcgcaactggctataggcgccgtttaccgccagatcataatcgttctgcgttttgaagtagctgcccaatgttacattgttgggattgacttcggcgagaaatttcttacaggatatctccaccaaactcagtatcactaatattaaacaggaaatctttttcatttttactgatttttaaagaccgagattcaagccaaacgtaaatgttcgttgcagtggataagcacccagatcctgcccctgctgcgttacaaatgcgagtccaccagcacttacttcagggttccccgggtaactggtgaagatgtatacattttgtgctgatgcatacactcttaagctcttgataacaggtgtcctgaattttctcagcatatatccaagtgtgatattgttgatagtgagatgggaagcatcataaacgaacagtgtattatctgtacggtatgccccggtggtgttagctaaagtacgcgccacctttccattacccggattggcctcggagcgccagcgatcaagcaattccggcggaccgttaaatacaccgtccaggttgtacgtactttcctgcatgccatttttcagcttgttgccgtaagtacctgacatggcgatattcagatcgaagttttggtactgaaaggtattactgaaaccaaatataaatttgggattaggatctccgatcaccgtctgatcatccgggaaagtgatcttgccgtcgccatttaaatccttgaatctcactgttcccgcctgagagagtgtagtggtaccggttccataatatttaggaccggcatcggcttctgcctgatttttgaaaatgccgtcaaatatatatccataaaactggccgataggcttcccgacaagtgtccggtagtcggtgaattcagataatgtccttgtcggattgtcggcaaaagaaatattgtttaaaccaattcttttaacaagatttctgttaaatgagatattaaagtccgtattccatttgagttttccggtcagatttttagtgcttacagtaaactcatgtccccattggctgatatcacccaggttatcctgcacgcttgaaaaacccgaagattgcggaacaggtagtacgaataataatcccgtcgtcagcttattgtaataatcgtacgagaaattgatccggttgtcaaatagccccagatcaaagccggcatcaaattgccggttgcgttcccaggccagattcgggttacccaaactggtttgtacctttcccggagccaggccgcctgaaaaagaataattggcattaccaatacctgccacggtagtgtagttacctatctcattcataccggttaaaccgaaggtcgctcttagtttcagcaaactcaggttcggcacatttttaagaaaggattcatcactggcgatccagcctgcaccgatagaaggaaaagtcccccatttgttattatccccgaaacgtgacgacccgtctctcctgatggtagcctgcaaaaagtaacgctctttataactgtagtttaaacgacccagaagcgacgccattgtccaggcgttaaagctggaagtgttggtagtaaaacgggtagcggcacttaaataggaaacgctgttgtccggaaaatcgcggcccaccatatcgcttgcaaaacctgtagatcgttgtatcgtaaaaccgcccagtaaatccagtgaatgatctttcccaaattgacgccggtagttcaatgtattttcattgagccaggaataatcattattaacggctgattcacccaaagcagtgttgttgcctggcggcggattttctataggtattgcattaaagccgcctattgaagtagatggaataaaccggttgcgggtcatgccgccaacgtccgcactaccggatgtacggaaggtcagatgatccgtgatttttacttctgcgaataaattggccaagacccgtaaccggttagcatcgtcttttacttcgagcaattgcctcagcgggtttgcccatacaaactggttggtaaaaccagaaatacccagggccagtgagccatccgggttgtaaggagagcccatagtaggcatcatggaggcagatgcaaaaatggcacgctgtccatccacattaaaaccgtccccctgcctgttgttatgctccagttgtaaagacggtgcaacaccaaaacctaccttcacccgtttgccaggattgaaatcaccattcacgcgcaatgaaaaacgcttgtagccggtgtttacaaggataccctgctgattaaaataaccagccacgatactgtacgcagccttatcgttgcctgcattaatagacaggctataattctgcacaggcgcattcctggtcagcacgctgaaccagtccgtaccctctccatattgctccggattctgatatacagcaggtataccgccggtatagccttcgtatttgatcttatcttcataaaaacctttcatgtaagtagccagttgtgtggcgttcattacaggcgggatcaattcacgcatcaatgacgcagtcccgtaataggaattaaaatttatttgcgtggcgccggatttccctcttttggtcgtgattatcaccacaccgttggcggcgcgtgaaccgtataaagcggtggaagaggcatctttcagaatggtaaaggattcaatttcatcagggttaatattattgatattatcagggttgcccagcattggctgtccgtctactactaccaatggccgtacgttggatgtaaaggaggccgcgccgcgtatacgcaggtccatcccctgtcctggccgtccggtagtttgggctacctgggctcccggcagcttgccttgtaacctttcagcgaaagtgccggttggctgatctttaatatcagtggcagaaagctttgctaccgagcccacaatttcacgcgaattttgtcggccataagcgactaccacctcggtgagctgtgaggtggattgttccagctgtacgtcgataacagtttgccctttgatcggtatttctttgggggtataacccaggtatttgaatgataacacgccgcctccatcaggcacactgagcatataagtaccatcagcttgtgtggctgttccaatctgggagtctttaagccttacagcaactccgggtaatggatgattattggcatcagtaacccgccctttgatggtcatgttaaccaaggttggtgctgtttggcgcgtcaccacgatcgtgttttcatggattgagtaagtaaaaggctgactggcaaagcttttccgcaatacttcttctactgttgcattggttacctgtatggctacgggttgagcatcctttaaaatttcaacattccatacaacattataacccgtttgtttccggatctggcggaatacctcccggagagtaatttgtttagctgataatgttaccttttgagcataaccggaggcgctgacttccattaacgctgcgatcattaaaacaaaggtgagtttcataatcaacaggaattttttgtacgtggcgccggctttttttgggcacacgtcaggtatgtaaaatttcattacatttggatgtttgggtttaataatcagaaactgtgactacaatagctttcgaaacttgtttttcacagggtaagctcaaactatccgggggcgctccaacgctcccggttttttattgcgccctgtttgcagatatttttttatggcataactgtgatcctccttccgtttattttaaagtgtacggtacctgttaattccagcatatttaatacttcagaaacattttttgaccgcgataaactaccgccaatggcttttcctgacacgtcgccctggtaggtaatttctacattataccagcggctgatttgccgcatgatgctttccaccttttcattctcaaataagaagtagccatttttccatgcaatagctccttctgtatctacctcttttatattgatcttgccggaagtcctgtttaatattgcttccttaccaggagccagcaaggcatttgccccaccgcaatctacttttacagcaccttcaagcagcgtaacaatattgtgctggtcatcagggtaagcgttaatattaaaatgtgttcctaatacccttacggtcataggtgctcccgatcctgcatttaccgttacaaaaaatggcctggctttgtctttagccacttcgaaatatgcctcgccggtaagtgttacattcctttcatttccgggaaatgacgcggggaaacgcagtgatgaacctgcgttgagccacactttggtgccatcctgcaatgtcatctgatactggccgccatagggtgtactcagggtattgtaaacgatggaggcagcggagctaccagccgcctcctggttataaatcaggctgccgctaccggtcttatttactgaggcattgccctgttgggatatgagcccgtttttagcctcttccagcactatcttatcaccgttagctaatgttaatattgctttgtttcccccgggaccaatgtctttaatatcccgggcaatagcagcagggtgggatgaacggtggatctgcgggtaataaaaataggtggtcaatcccaggatgagcagtacagatgcagcagcagacaggtagtaccaaagccgcctggtagtacctggtttggttgcagggttattgatttgctgattcaggcgcaggagcatacgcaaacgtacctgttcttcttcatccgcattttctgccggccattcaacatcggtttgattatgatcctggtaccaggccattaactgctcttcttctgccggtgtaatcgtgccggcaaggtatttttcgatcaggtaatatatattgtccttcaatgtataaattttatccttatacagataggtaccataaggctgatctttacccttagtgagcggaggattttttttgaagaaattaagaaaggaacattttaacgattatgatcacccataaataagggcgattcaatttaactttcagtactttcaatgctttagtaagatgtgcttcggccgttttctcggcaatacccaatctttgcgctacttctggtatacttagtccttcttccctgcttagtttaaacaccaggcggcatttctccggtaaaacttccactattccattaatgtgttgctgcaagaatctggtgtagatcttttcttcatcccaggtggtgattatgggatcggctgcctgttcttttatctcatccctccgtttctgccgcacatattgtttaaacacagatagcctcactgcagtagcgagataggcatttacattatcgatataaagctctttccgcctgttccataggccgataaagacttcctgcacaatttcttctgcaattactttatccctgcaatgattatatgcaatggccagtaatttcttccagtagcggtcgtaaatttcagtaaaagcatctcccttatcctcgcgcaggaacattatcaaatctgcatcagtttgttgccggtactgcgtcatgtgattggtatggtacacaagaatataaaaataaatcgagtttttgtacctgtatatgaaaagataatatttaggagaaagggtaccggggcagatggtaaatcttaaaggcgaactaaatgcgcctgtatatttgatactggattagtaagtgcggggggaccatcttcttttctatatttccttttcatacagctgtttatgggtaacataaaaatatgcatgcccgttatgaagtacgtatcatagttttctttattttcacatggatttccacttttctttaatctgagcgtatgttggatattgtattacagtaattaccgtccaggtaattacatcttcagctgataatctattcatagctcctgcgccttcggcagcgggagtatcttctatttatttaattctatcagaaatgcacaaatacaattatactttcagaagggaagagccttctgatatcggagctatcgatcaggtaacgaaggctgcgtttgcctcagcagcatatagcagtggaacggaatcattcatcataaaagccctgcgcgcaaatggccggctgaccgtttctctggtagcagaagaggagggagtattgataggacatattgctatatcgccagtaaccatttcttcaggaagcgaaggctggtttggactggggcccgtatcggtaatcccttccaggcaaggatctggcgtggggtccggcctgatcagggccgccattgacgcattgcgggagttggacgcagccggctgtgtggtgcttggcgagccttcctattatggccggttcggattcaggagcgatgcccgtttgcagtacaagcatgctcctgctgaatatttccaaatacattcatttacaggagcgataccggaggggactgtggaatacgatgatagtttcaacgttaccagttgaaattaatcagatgtaaatagaagaggctgtctcaacaagattgagcagcctcttcttctttgggcctgatagcgaccggaaggcgttgaaaaatcctcaatgcgttcgaacgcactaactgtttctatcggtgaacataggtcctgctcaagtagcttgaaatttttttaatttatctccgccgggacgctggttcagatgaagcaaattggattacttattttataaggggcaataaaaaagcaggatacaaaacctgccattactgtaaaaaaacacgaccaaaaaactattagttattgcaatcaataagaatactattgaaaggcacataaaaaaagcctctggttacccagaggcctaaaattatttgtggagatggcgggaatcgaacccgcgtccaaacatattcgccgaaagctttctacatgcttatttacgcattgttttgtcgggatctggcaggggcgtaacaaaccaaccatctccttatccgttgtagcttcagtattcactcacagaaaccatgaatacctatccctatgggtttatgattcggcggcggaagtcgcataaggcgacaacttcaagcggctataatgggtgtctaatttataattaggcagccatggcgtagttagattcgccaattagagtttgaatattcagattatcgtgctaattatccaacgcacggcatgcttacactctcaaagatctatgctgtcaaaaccaggcatccccctgtaaaacagtttacaaagatactataaaaaactggcatttgatcattcatcacaatcaaatgccagtaatatttttaaaataatccactcagtagatttctccacacatccagcccgtttgcaaacaacagcaaactaaacaggatcagcatacctgcaatctgcgcgtactccaggaacttctcgctcggcttgcggcctgtaatgatctcgtacaacaggaaaagcacatggccgccatccagcgccggaataggcaggatattcatgaatgccaggatgatggataaaaacgcagtcatctcccagaacatctgccagtcccacgcatcagggaacagtttggcaatagacataaatcctcccagcgactcactcaccttcacttctttggaaacaaagatcaggcgaagctgctgcacatattttacgagtttgtcgacgctcttgtgaaaaccggccgggatagattccaggaaagtatacttctttactttatactcaaaaggatctcttggataaacaccaaatgtacctttctcactcagctttgcagccaggttcaacgtgtccttgccacgaaccagggtcactatcacattttcattcttgtgcttcctgatctccgttgcaaactcatgatagtacagatacggtgctccattgatcgcaataagctggtcgccgctcttcacacctacctttgcggccgcagatcccggaagagtactgtcggcgatataaggaagacggggcatggcaaaaggcgctttctgcttcagcagctgcctggtaaagccagccggaataggaagatcaagggttttaccatcgcgttctacctggatacttttggcttccgaaagaattacatctccggggattgcctcaaaggcttccacgtgatggtgatcaatggtaacgatcttatcaccgtccttcataccaatgctgcgggccagggaatctgttaccacgccatattttgcggcagaagtaggcaggtaggtttcaccccaatgccataagatcatcgcataaataaagaacgcaagaacaatattaacggtaacgccgccgatcataatgatcaaacgctgccacgccggcttggcacggaactcccacggctgcgggggctttgccagctgctctttgtccatactttcatctatcatcccggatatctttacatatcctcccaacggcagccagccgataccatattctgtttcacccttctttatcttgaagagggaaaaccatggatcaaagaacaaatagaatttttccaccctggttttgaacaacttggccgggataaaatggcctaactcatgcaacactaccaaaatagaaagtgacagtaacaactgtccggctttcaccaatattacctctgtagtcatttaattgtttctgctttaatctgcctaatatatcagttttaatacatattccggcaaaactctttgttaatttttactggcaatttatataacgatagaattgataagggatgcagcgtgttcacgtgcggcattatcgcattcataataatcgtgcaaggtgggggtttcaataaacggtattttacccagcgtttcctcaattacttccgtcatctgcaggaaacctatcctgtttttcaggaaagcattcaccacttcctcattggcggcattcattacacacgcagcgtttccgcctttgtgcatcgcctcaatagcaatggccaggttacggaaagttttggtatccggctgctcaaaagtaagcgtaggataattacggaaagagaaacgcgggaaatcattggccagcctgtcgggatatcccagcgcatactggataggcagtttcatatccggcaaccccatctgtgctttcagggaaccatccacaaactgcaccatcgaatgaatgatagattgcgcatgtatcaccacttcaatgttttccggcgccaggccaaacagccagcgtgcttcaatcatctccagccctttattcatcagggtggcggaatcaatggttattttagcgcccatactccagtttggatgctgcagggcatggtctttttttacattgatgaggaagttcggctttttaccgaggaaaggtccgccggaagcggtgaggattaccttttccaccttgctgaaaggctctcccagcaagcattggaaaatggcggaatgttcagaatccaccggtatgatgggtacatttttcctgcgggcggtagccattacaatatcaccggctactaccagggtttccttgttagccaatgccaccggggtgccctgttcaatagcagataatgtaggcgccagaccggcaaaacccatgatggcggccagtaccatgtcaatcgaactccaggcggctacttccaccatcgctttcggaccggcaaatactttgatgcctttatcaaataatacatcttttacctgtttgtactttgcttcactgcctatcactaccgcattaggcttgaatttcagcgcctgctcaatcagcaggtcagcattttgctgtgcagtcaatacttctacactaaacctgtcggggtgcgcagcgatcacctccagtgcctgtatgccaatggatccggttgatccgaaaatggcaatctttcgtttattcattacggtgatttacgtttttacagttaacaaaaatgaagaatcagctgccggtaaaatagcctgacagccgtcccgccctgaatcgccggttatttttgtaaatacgctgccagctcatctgcaagctttctgtcgttactcaaacgaggtactttgttctgacctcccagttttccaatggctttcatataatcgataaagccctgcttacgtacagtccttatcttcaggggttgcaaaatattaccggtcagcagatcatcataataaatattcttctgacgcatgttttcatctacttttctggaaaatgcctccatgttggccggcatattctcaaactctacaaaccattcgtggtaaggcagttcaccactggtttgcaccatcggggccaccgtaaactctgtgatctgcacattttcctccgctgccgccttcatcaggctgtgttccacctcttctcctatcacgtgctccccgaacgcagaaataaaatgcttgatacggccggttaccagcaaacgatacggattagtggaaacaaattttaccgtgtctccgaggttatacccccataatccggcgttgttgttgatcaccatcgcgtaatttacaccggtttgtacatctttgagcgacagtcgcgtaggatgctcattaaaaatttcctgagccgggataaactcataaaagatccctgaattggtgttcagcagcaaaccttcccgctcctgcgagtcctgaaaagcaaaaaagccttcagaggcaggaaacgtttccacagtgtgaatcggcgcacctatagatgccatcagcttggaacggtaaggctcaaaattcaccccgccgtataccatcacatcaaaattcttaaatatttccctgatctttttaccattgctgcgctccatcaggcggtcgaaatacatctgtacccatggtggtatgccgctgatcagcgtcatatcctggttaatggtttcttccacaatcttgtccagcttcgtttcccagtcatctatacaattggtttcatacgatggcagctggttggtacgcaggtaccggggaatatgatggtttacaataccgctcaaccggccggtaggaatgcctcccaccctttcgagctccggcgaaccggataaaaaaatcattttaccatcggcaaaggccgtactgcccgtttcccccatatagttcagtaacgcattacgcgcggtatctatatgattgttaacagattctttggagatggggatatatttaacgccactggttgttccggaggtcttagccaggtaaatcggctgccctttccacagtacattttgtttgccttccttgattttttcaatataaggcttaaactgctcataatcccgcaaaggcacagcctgtttaaattcttcgtgggtttgtaccccgctaaacttgtgatctgttccgaattccgtctttctgcctgtcttcaagagctcctgcaggatattatcctgatcttctaccgcccttaacatttccttctttatcttattatgtacgatagaagcaaatggtttggccagcagtgatttaaacttcatgcctgttgttttataattgagagactaaagctgagcatatttatttatctggagatttaattgcactgatttttagggagttccggaagaaatattccactctggcaattaaataagcaggtaaataaatgtcctcatcctatctgtttttattcgtgtaaacgacaaaagtatacaaaattgcgttggtttgcacagcaagatagctgtttttaaatgatcccgaaatagcataaaaatgtgcatatagcggtcaggcgccggaaatcattatttgttaaaataatttaaaattcaagaaagtatgtatctttgaaaagattaagctttaggcggtccttcatatgtgtttatacatggtgatttaaaaaagaccgaaaaactttgtctattagaaaacaaaaggttacttttgcggaaattatattttggataattatgtttgcagttgtaaaaatcgcaggtcagcaatttaaagtacaaaaagaccaggaaatttttgtacagcagttacaaggaaatattggagacaaggtggagttttccgatgtactgttaacagataatgctggtgcgctgtccgtaggcactgatgtaaaatcagtagtaaaagcagagattctggctcatgttcagggtgacaaagtcatcgctttcaagatgaagagaagaaaaggcttcagaaagaaagttggacaccgtacccactttacaagaatcaaaatcaatgaaatagcttaatcctgttaagctaaacttatttattagacaagtttaaagtagtaatacaatggcacataaaaaaggtgaaggtagtgtaaaaaacggccgtgactcccacagcaaaaggctgggagtaaaaatcttcggtggtcagccagctatctccggcaacattatcgttcgtcagagaggtacggtttatcatcctggtcaaaacgtaggcgttggtaaagattttaccattttcgcagtagcagacggtgtagtggaattcagaaaaggtcgcgaaaacaagacttacgtttctgttaaagcatttgataccactgctcaggcggaagcctaatcagtgttagccataaagttttttttaatacccaatttttttactaacccaaattcaaaaaacaatggcaacaattaaaaaagcggctgctaagaaagctgcacctaaaaagaaagctgctgctcctaagaaagctgctgctaaaaaagctgctcctaaaaaagccgccgctaagaaagctgctcctaaaaagaaagctgctgctaagaaagccgctcctaaaaaagctgctgctaagaaagctgctcctaaaaagaaagctgctgctaagaaagccgctcctaaaaaagctgctgctaagaaagctgctcctaaaaagaaagctgctgctaagaaagccgctcctgctaagaaagctgttgcaaagaagaaagctgctcctaaaaaagcacctgctgctgcaccaacagttcctccagctccggctaactaagatcggaattacaaaatgtagttataaggatcctggcatctatgccgggatctttttttatgcccattccccaacacattccccctccacaatttccgcgtaactccgtatttttacggcatggataattattcaatctcagataacttctccctcctgtccaaactgatggacatccacggagaaaacagtttcaaagccaaatccttcgccagcgcagcattcaccatagaaaagctgcccagtccactgaaagataccccccgcgatgaaatattccggataaaaggcatcggagaatccaccgggaaaaatatcctcgaaatgctggatacccaacaatgctccctcctgaaccactacatagaaattacccccgccggcatcctcgaaatcatgaagatcaaaggcctgggacctaaaaaaatcgccaccatctggaaagagctggaaatagaatccatgggcgaactcctctatgcctgcaacgaaaaccgcctcatgctcctcaaaggcttcggcgctaaaacacaggaaagcgttcgccaaaatatcgaattctatctctctaaccgccaccgcttcctcttcgcggaagtggctaccaccgggcacgaactggaaaaacaactgcagcagctcctggcccccgccgcggtttcgctcaccggcgcgtttcgccgcaacagcatcatcatcgatgaaatagaattactcgtcgccgccccggtggagatagtacaacagcaactcgccgccctccccggtttttcactcaccgccgccaatgccggtaacctggtatggcagctgaacgaaaaactcaaagtaataacacatagctgtactgctgataacttcgcggctaccttatttactaccaccggctcacccgcgtttatcgataaattcaacgccgcaggcggcgccgcattccttcacaacgccgcctcggaagaagctatcttcagcgctgcaggaatggactatataccccctttcctacgggaaggcatcaacgaattaacgctggcccgcaaccgtcaactgccggaacccatcgtcgccaccgatatcaaaggtattatccactcccacagcaactggagcgacggcgaatcctccctggaagaaatggccatcgccgctaaaacacaaggcttcgaatacctcgtgatcagcgatcactcccgctccgctttctatgccaatggcctgcatatagaaaggatcttagcacaacacgcagagattgatgaactgaataaaaaactggcgccgttccgcatttttaaaagcatagagtccgatatcctcaacgatggatcattggattacccggatgaaatcctggcaaaattcgacctcgtaattgcatctgtgcattccaatctcaaaatgacagaagacaaagcaatggcccgcttgctgaaagccatcgaaaacccatacactactatcctcgggcatatgaccggccgcctgctcctgagccgcaacggctaccccgtagatcataaagccatcatagatgcatgcgccgccaataacgtggtagtagaactcaacgcgcacccacgccggctggatatcgactggacctggctgcattatgcactggaaaaaaaggtgctcatctccatagatcccgatgcccacagcatccagggcttccaggatatcaggtacggcaccctcgccgcacaaaaaggaggcattacaaaaacaaacaatctaagcagttacactgttgacatgctgaataattacctgctgcaacgcaagcaacaaaaaaatatcctcccatgatgctattggcattggcggtggcgccgggttttgctatctgtcttttcatttacctggtggacaaatacgaccgggaacctaccagcctcctggtaaaaagtttcctgctcggcatgctctgcgtagcactgccgctggcagtgcagggtctcgctgtggaactgggcctccgcgaaaataatggtaccctcctgggaaccgccgcattcgcatacggcgtagtaggcctctcggaagaactggccaaattcctcgtactgctgctcttcgcctaccccaaaaaagcattcaacgaacccctggatggtattgtatacgcagtaatgatcgggatgggcttcgctacgctggagaatattgcgtatgtaagcaggttcggcgtaggcaccgggatcgcccgcatgttcctctccgtacccgcccacggcgcctttgcagtactaatggggtattatgccggcatggctaaatttgtaccgcagaaaagcagttcgctgctattccaggcactcctggttgccattttctttcacggaacattcgattttttcctttttctcggtaataacatcttcctcatgggagcctccgtgatcaccctcatctttgcggtacgcctatccatcaaggctatacgaaaggatagcgccctctccaagaaactgtctgaggaacacttttttgaagaagagaacacctgataccacctttttggcagtcagcttttagttacctttgtcaggggcctaaaagccgactgctatgagattcatttacatttacgatccgctctgcggctggtgctatggctttacccccgtggtacagcaactgcaggaacgcagcagcgggaacatggaattcaatatcctctccggcggaatgatcaccggcgataaccgccatcccttctcttccatgaaggcctacattcagcgggaacataccaacgtggaaaacgccaccggcgtgaaattcggcgctgccttcctggagaaattacttccgtcggaagaaattatggactccgaaaaacccagtgtcgccctcacggtatttaaacaataccagccggaaaatgccatcacctttgcacacgatatgcaggtagcgctcaactataatggccagagccttaacaacgacagcacctaccgctcgctgataaaaaaattcagcctgccggaagatgaattcatcagccgcctgcatgatgaaaattaccgctacgaaacccaacaggaattccagctgatccagaactggggcatcaccgggttccccgcggccatcctcgatacgggcaaacaactttatctctgcgcacggggatacacgcccctcgacaaactggaagaaaccatacaaaatatattgagagaaaataacagcttataactttatgtaccacgtcaaaacagctactgtaaacgatattcctgttatacaggaactaacagaaaagatatggagacctacctatcagtctattctgaccccggaacaaatagaatacatgatagacatgatgtacagcacctcctccctgaacaaacagatcacggagctgcaacaccagtttctcattctgcaggatgataacagccccattgggtttgctgcctacagcaccaccgatacccccggcatctttaaactgcataagatctatctcgatggaaattaccagggaaaaggaatcggcaaattcctactggaacacgtggccggacaggtaaaaaaccacggcgcaaataccctcgaactcgacgtaaatcgcttcaataaagcaaaacagttttacgaaaaacagggattcagcgtgtataaagaaaaacaaaccgatatcggcaacggctacatcatggacgattatgtgatgcgtaaaccactataaaaaaagcccggtaaggagataccaggctattcccaagttaaccattaaaagacacaactcttttttaaaaaaaataatgttaatctaaggttatgtacgataacgcccggtaagcggatttatccatagattaaaaaagcagtatcttttatattctaatataaaagatgctgcttttaagtttaatatctttctaaaaaaaattcccgcatagctgactatgcgggaatgcaggtgtgcctgaagcgcgtatatcggttattgatccaagccgttattatttggctgtgagcacggtgccttcatcgttatcatcatcatggataacagcaaccgccttattcagtttcagctcaggcgaaattttcaatacccctgcattggcagcagcagtagcatcacgcagtttcacagataccagtgcatctatttctttcacacggtcgtttaccagcgctacctgtatatcggtttcgctgaaagcgcaatcaccggtaatcttaaccatgtcgccgttcatgatcacataatccttaccgtaagccgccgtactggatgaatccacaccaaagaagatgttgatatcactaccggtgcaattcgtttgcacggtttgatccgcagctttcaccaggatacatttaaacatgctcacaggcgccgtagcagattcattggcatctgtcagtttcaccagggtaatgtaagccgcctggtcctgtatgtactgggaagctgaaatggaagttacatcgccgttataacctaccaccgcctcattctctgctttaatttcgcttaacaccaacacaacggtctccgccagctcaaagcggttgtcgtcttttatctttacattcaaactcgcagtagtagcgccgctgtcgatcacaaaaggcgctttgatgctgcttacaaagtcggcgcccggcagcgcagtgccattaccaaacttgtaagtcaacctcactggtttggaggtggcattgatcaacggggtattatcccgcttgaacaaaccggcagaaaacaccacatcggtagctggctcggcgccattgttaccaccaatgaatttcaccatagccggctgatccaggatcgttacctctccttttgacttggtaagatataactccgacgcatccagcacttctacatggaaagcttctttaccttccagcaggttatcactctttacagggatctggatagatttggagataatagctccggcagcaaactcagaaggcacaaaggaaatagttccttccgtaacatcaaagtcggttgaaccggcgccgcctttatgcggaatcgttttataatgaacgttaacgggtgtacgaacaccattgcttcttaaaaacccggataaggtaatggtgagcgtagcgttggataaaccattcaatggctcggaaacagctatatcgttgatagatacgccatgactgatcttaatgatacggttgccatcttcgtcaccaccgcctgctgccaggatttcgccggaagggctcatcagcagcgaagccagcgtggtttttgcatcatacttgcccagctgcttgtcgaacatcatttcaccatcaggactcagcttaatcatgcgatagccttcttttgccgccacgcagatttcatcgtcttcggtgagtaacaggtgctggaatacagaacccaggtttttatcaatggaaacagtaccgtccgggagcagcttcacaatcttacccgtgttgttgctcacattgccacctgccgccactactttgccgtttttgcctacttccagtgcgtataaagcagcatctgtttctttgttgaataactccgtgccatcaggacgcaacttaacaatgcggccatgatctttttcttccgcacaggcgaagatctggcccaggtcgttcactttgatggcattgaacttgccatccgcggtactgtactctttatcaaatactacctggccctccgcatttactttcgcaatgcggctggcattgccggtaccataagcgccaccgcccatcgccagcacagcgccatcttccagcagcaacatcttttcaaatgtagcacctggtttaccaaaggaaagctcaaattgtttttctccctttccatccacctttaccatgtatgcctttccctgtccatcacccacgtcgccacctacagcaacaatgttgtcatcttcatctatcagtacattggtaaaaacattgtgcgcaccaaaacctttgtcgaattctactttgccatcgggcgacatcttggtgatgcgggcctgcgcaggcttactaccatccacgccaacggtaatatagttgccatgacgatccgtaatgatccgggtaaaataaccaccctgaccgttaccgatgctcttgtcaaatactacttcaccggtagcagataatttggtaatacgggcattgccatatgcaatggtaccaccgcctactgccaccagttcattcttcggcagtaaaagcaggtcctggtaggctaccaacccgcctttattcagtttggcattgtaaataagagtgcccgttgcagataacttggtgatacaaccgttatctgttccgcccccgatggcaacaatagcattgttctccgcaatagccagtttcttatactggtttttgggagcactgaagctcttgttaaacacaacaggcatctcctgtgcgaaggcctgtgtgcctaccgccagtaatagcattagtgaggaaaatttgttcatttgtattagtttgatatacgctaaaaaataaccgataaatagtttattgaatcttaatctcacatcttctgttgataccctgcagttgtataaagtattccctgttagcctcgagccgctggctccccgccatccataccgggcgggtagatccgaaataattgatcctgattttatcaggcgctactcccctgctcagcaggcactcctggatgtatactgcccggttcttcgacagcgacaggttataccgctcggtgccaataatatctgtatgcccgttcaccaatatgatccggtgcgggttcgacttccatatccggaaaatagaatccagcttacgccattcctggtcctgcggcacaaaagaattcaggtcgtagtatatcacaccgggcactttccacaatgcttccagcactttcacaacactgtcttttaccagcgtataacccataccgttagcaatggcatgagggccgctaaccgactgctgccacgataccatttccgggctgctataggcagcctggccggcataggccgactgtgctatagtggtggccgcaactgccggttgaacattgctgttaccaggatgatcattttgccagggaataatttcgggagaactgtctgctgcggtgttggtgtaatccaccatgttgcgctccggactaacggcaacggctactgcaggaaccggttttaacacaacgctatctatcaccggcgttgccacaggtaggttgtcgtattgtttggttccaattaaagtcagctgttgacgggtatccgtctgattcatggtataaggcactcggtcgtcttcttttactggcttgccgggataaggcaggtccagctgtttcaaaggatttttcttcaggtttaacacatagatatgatcgttatcatgcgcgcctgaacggtctgacgtaaaatataataacagtttgctttcatccagtacgggattcagatcatcaaactgcgtattcacaggatacggcaaatgtacagttccttcttccggttttttaatatttatcataaagatgtccagtccaccaaacccacgaaggccattggaagaaaagaacaacttatcacctaccacaaaaggatacagttcatttccattggtatttacctgcggacccaggttcaccggcgctttccaccgtttggcttccttgtcccagtcggtgtagtaaagatcggtaccaccctgaccaccaggcatatcggatgcaaagtacaaacgtttaccattaggtgcaactgatggatgaaggaaagaatatgtttccaggtttttccccagcttcactgtcagcggcttactccacatatcatgatcgggctggtaaacagcagataataactgcgtgccgttattgtaattaatataggaattcttatcgttctttacatccgtaaaccggttggaagtatagatcaccttttgcccgttatcaaagaaagaagcaggtcctacctgtaatactccgcgcaggctattgttaaaaggctctaccccatcttcagaaatctggtataatttggaattggtatagaaagattgctgctcgtttttccggatatcattggaaagaaaaacaatgttattgcggtataaggcaagtccatactggtacccgggcaaattcaggcgaagactgtccacccttatattctccatggaatcacggttaaagaaaccgtaataattcaccagcgactctttcaggttggtaaaccgcgcattgttcttatagttattggcatacactgcgctgatctcctgggctttcaatacccttccggtgcgcttcagcaaatcaatgtaattggttacatccgttaccagcacgtctttttccggcttgtacaacagctcgtcgtataaactgatcgttttttcaaactgcctggtttcaaagtatacccgcgccagctgcaatttagcccggcgtaaaacttcttcactgccgccattatttattacttcattacacaaagagatcgctctctcgtattcttgtctcttgtaaagccgttccgcacgctttaccttagccatacttcccaagccacctatttgcactcggtcttttacaaaactgcaggaaacaaacagggaaacaatgctcagaaaaagtatgagggaagagaaactgtattttcgcataccattcttgatttttaaaattagaaataacgcggtgctaccactttccacttcgaccacgagaagcggtaattaatcatcacttcatgcgacaccgtttgcgcacctttcagattcgactgcataggcgtatcatacgaataaccgatctgcaggttcttcgttgcctgcacctgcaccaaacccgtcatcgttttttcagagcgccacgatgcacccagccagatcaggttcttcagaaggatattggcattcagatcatactgaaaacccgctcccttcacctggcgtaacaacacgtttggctttaacttcacatcatcattaatattgatcaggtaacccgtttgcaggtaatagtgcgattccaccaccactttattcacgctgttaccaaggtcaaaacttttaaaagtaggcgacgataacccgataaagaaccggtctgtaaacaacatgaaaccaaaacccacatccgttttccagtaactctggttttgcgcaaacaccggatcagtagtagtcagggagctgttgtcttccctgaagtgcgacatgccgcccttcagccccagggccaggtaaatcttttcattaagcttcacccgctgggaaatattcaggttcaccgccgtctgcgaattcaccgtgatcttttcattcatcagcgacacgccaaaactggtgttggtggctttaataggagtataaaaggaagccgtggccgttttaggagccccttccacacctacccactggttacggcctactgccgtaagactggaagattcatccatagaagggtaagccggattgataatcatgccattgaacatatactgcgagtacaacggttcctgctgcgcagcaacctgtaaacaacaacaccagcataagatagtaacccctaaagctttcataagatgctttttcataggtatcagcttaaatatttttttgtcagatgcatcctgcttaaaattcgtatgcccgttaacgttttatcacaataaacccggtgtaacgctctttcttaccatctatctctacttcaatattgtagaagtaagaaccatccggcacatcatttcctgaactgccgcctgcatttgccttaccgcggaagttcttcgatttgttatcgtagtgctgcaacttaaatacggtgccgccccaacgattaaatatcactacctcattatttggatacttgtcgatattttcaatatacatcacgtcatttcccatgccatcgttgttaggggaaagcgccgggtgtacgcgaatcttaccgctgttgttattgatctggcggccatccgtactatacttttcaacagcatcgtttacaccatctccatcagaatccaggtcgaggaagttagggataccgtctccgtctgtatcgtcgtcaaatggatcaccattgctgttgatgtcttcctgcttatctgttaatccgtcgccatctgtatcacaactgctgcacatcggatcatcattcaggatcataccggtagctttggaaggctcacctaaagttggcgtatgctggccggaaggaactgataccgtagtcatcttcaggatgaaggtttcattctgttcaaaggtcgtatcccctttaacattcactgttacctgcccgatcgtctgcaacgccgggatcaccgtttgagtaactgtgttgtcgaaatcattacccggcgtggctttgaagtccatgtaaggataagataccccatctaccgaagcctcaaaatcatagttaatcgtaatcggacgggaactttgcctgctcaactgtacattaaacctcagcggtgtattctccccggtattgccttctttcacgctgaatttgtcggcagcaaaagtgagggtcaacggatcgttatccgtgatcgcaacccttgcagtatccgtagccccggctttatataccagggtactgctgccgccaatgtagggcagtatcgctgctttcaggaagccgtcatcgtcattgatatcgttatcaccggtggtgataataaacgagtgttgctttgtaagcgccggcatgttgatggttaagatgttaccgcttacggtaccttcaccggctgtaaatgtacgggcggcatcctgcgtaatgcggaggcgtaccggcacatcgtaggccgcagatgcgggcgatttcaaggtgaacttcataccgcttccttcagccgcagtaacagcttctgctgatatttccaccaccagcgtatcattatcatgaatgattacatcagctgcggcgctcccagataacggccaggtaatacctgccatactgctactcactgcgtccagctgtactttcacatcttcatctccctcaacaatattgttgtcgatcggtgttactttaatgtctgcaccattctggccggcggggatcatcacagtgccactcagcttacggtaacgggtgtcagctacagcagtaccgctaacggtataggttacattcacatctttcacggcagataactgtgtatcggagaaccgtacacggaaagatcctggtacatccggctcggtggcatctgctgttttcgcaatcatcatctcccggcccggagcagagctttcatcatcatgcactatcagggtaacagtatccttatcatctacatccagcgcgatgttcttattaaaccgcttcatctgtgccagcattagtgccagcttcacctgttcatcgccctctatcactttattgtcaatcacattcacgggaacggatatactattctgaccggcaggaatcaccgcggatgtttgtaccggtgcaatgttggtagtgccggcaatgctgcttacgtaaaacactactttcacatcagctgctgcaatgctgctgcccggcagtttcaccgtgtatgccccgtttgtagccggttctgcggcgtctttgttcttttgcaatactacgcgcatatcacccgtttcagggatcagcaccatacctggctgggaaagtgtataacccgttgttgccagctgtgcggtaaattgcagttgctcgtctccttccaggatattatcgcctgttaatttcagctgatataatttactatgtgctccggcagccagcgttacctgtgcaggcataccactgtaatctgcatcatctgcagtagatacggcgtttctgctgatattgatcactacatcttcggaagaaatgatctggctgttcacaaacccgatggtcacatcactgttgctgccttcgtgtataacggaggagtcgatacgcatttctactttcaggttatccggattcaaccgcgtagcgtcatcaatcgttacagataatttatctcctttcatacctgcaaagccctgtggcgttgcggcgatccataacagctccggtttctccagtataaagtctgttttggcagtaaaggagaaggtagcatcaggtatacctgcaggaatgattacggtagccggcaggttatcaatatctgctgctgttgctacggatgttgcatccctgttcagggtaacaatgatatccttgctggcagtaacacctggcgccaggcttaccttcatctggtaagtatttccttccagtactttggtacccgctgttacggaagtaagatgtatgaacccggtaaccggatcatcatgtgttctgtctttgatcgtaatggtggtatctcttacaacagccgtattaaaagtagcatctgtaatgctgccattaaataccacggtttcatcatcttccagtaccaggtcttttaatgccttcagcacaaaggtgtgggtacccttgttttgtccttttttaataataatatcataaggagatggcaaggcattatgatctgcgtttaccgcggtactcagcgtgttatcttttgttacatgcaccgtgatgtccttgcccgccagcaggttgttgggcagctgcgcactcagcgttgcaccggaaccgttttcatcaatagcagccagtgtgctgttgagtacaacaggcgccggcagcggatactgcgttggatcatcctcaatggtgaataccggtttattgatggtgtaagtactgatgccatctgtagcgctggtattgatgataaaattctcgggcccctctgtgaagttatctttcttaatcttcaaaccggtaacgatactgttgccgctgttcaggtaaacgtcgggcgccagggtgtaatccagcccggcttccgcactgcctgccgattgtggcagtaatatatgaacaggtacatcagtggtaacgccggcaggtaaactaatagttaccgcgccgctatcgccttctgtcagtggtgttttccaggcgctaacattcaatgccaggttagcagcatcgctgcgggtaaggtcctgtatcgccagcggcaggttattaaccgtatatccattaatggtagcattcaccaccagtgtttcgttcttctccagcaccttgtcagccactgttttcagtagctcaaaggtagcagtggtttgtccgtgcggcaacacgtaggaagtggccgacagcgtatagtcatcaatgtttttagcggtagtaagcggattatttaccgccagctgtatgcttacatcttttgtagacgcataaggcaccgtcacagtcaccatcactttattaccttccggcaccagtgtggcatccggcgtaagcgtcatttttcttgcgttcggttgcttctctgtgtagtctttgatatacacgcctgcactggtagctggcatgttggtattccccttgttgccttcaatgaccaatattccttcatcatccagtatggcattggtacccgccgtaatggccggagcagatgcagcggaggtgttgttcaggatggtcacactggctggtaccgccgtatgacgggcatcagctacagtagaagcggcagcatccttcgccaggttgatcacccagtttttaccggctttccagccatgtgggaaagtggccgttatcaccgcactgcttccttcgtaaatgctgtcgggcgtactcgtgaggataatggaatcgcccacagggaaaggatactgcgcatctttaatactcatatccattgttgcaggcaggaacgtgtacacggtgctgagtgcatcacttactgcaggagtaatatgtatgtcttctgcatcttctaccaggatatctgatgcaacctttaactgtgcaatacccgaagcaccggtaaacgtagtatccgcaggcaggtaataatcagtattacgtatagccattccggtagcgccgcccattgtaatcttaaccggtatctcggtggttacaccggcaggtaaactgaagccaatattattgatactgttttcattcaccgcaccagatggcagcgtgaaggtgatctttgttttagccgcatccctgcgggtagcgtcattaagctggatagccgcatctgtaatcgtatagccggtagcggtaccctttatcttcagttgtttatcgttttctatcacttcatccgcaacggctttaataaccggtgcagcggtggtgaaggtgttgctgttcttcgggaacacaatgcttgtctgcaatgcggtatagtcggccgctgctgcatccgtaccggttggattggttgccaatgcaatcgttacgtctttggcggctgcatagcccgctggtaacgataccgtgaaagcagtgctactgccttctgcaagcggggaagtgaccgctgttaaagtcagtttcttctgcgcaggatcagtaccatccgtaatattaatgatagcgctggtagccggcatattggtgttaccggcattgccatctactttgataaagccaccgtcgtcgaatacgttgttggttttagtggtaatagctgcggtagtgccggatgcggcgttggtggcaatggtcacggaggcagggatcgtaccatgactggtatcagctgtcgtagagcgcagggcatctttcgccaggttgatggtccaggctttaccagctttccagccatgcgggaaggtagcggtaatgatagcagaaccgccttccgttaccgggtcaggcgtgctgatcagcaatacggaatctcccgcagggaaaggatactgcgcatctttaatgctcatatccattgttgccggcaggaacgtgtacacggtgctgagtgcgtcacttaccgcaggagtgatatgtatatcttctgcatcttctaccaggatatctgatgcaacctttaactgtgcaatacccgaagcaccggtaaacgtagtatccgcaggcaggtaataatcagtattacgtatagccattccggtagcgccgcccattgtaatcttaaccggtatctcggtggttacaccggcaggtaaactgaagccaatattattgatactgttttcattcaccgcaccagatggcagcgtgaaggtgatctttgttttagccgcatccctgcgggtagcgtcattaagctggatagccgcatctgtaatcgtatagccggtagcggtaccctttatcttcagttgtttatcgttttctatcacttcatccgcaacggctttaataaccggtgcagcggtggtgaaggtgttgctgttctttgggaacacaatgcttgtctgcaatgcggtatagtcggccgctgctgcatccgtaccggttggattggttgccaatgcaatcgttacgtctttggcggctgcatagcccgctggtaacgataccgtgaaagcagtactgctgccttctgcaagcggagaagtgactgctgttaaagtcagtttcttctgcgcaggatcagtaccatccgtaatattaatgatagcgctcgtagccggcatattggtgttaccggcattgccatctacttttataaatccaccgtcgtcgaatacgttgttggttttagtggtaatagctgtggtagtgccggatgcggcgttggcggcaatggtcacggaagttgggatggtaccatgactggtatcagctgtcgtagagcgcaccgcatccttcgccaggttgatggtccaggctttaccagccttccagccatgcgggaaggtggcagtaatgatagcagaaccgccttccgttaccgggtcaggcgtgctggtcagcaatacggaatctcccgcagggaaaggatactgcgcatctttaatgctcatgtccattgttgccggcaggaacgtgtacacggtgctgagtgcgtcacttaccgcaggagtgatatgtatatcttctgcatcttctaccaggatatctgatgcaacctttaactgtgcaatacccgaagcgccggtaaacgtagtatccgcaggcaggtaataatcagtattacgtatagccattccggtagctccgcccattgtaatcttaaccggtatctcggtggttacaccggcaggtaaactgaagccaatattattgatactgttttcattcaccgcaccagatggcagcgtgaaggtgatctttgttttagccgcatccctgcgggtagcgtcattaagctggatagccgcatctgtaatcgtatagccggtagcggtaccctttatcttcagttgtttatcgttttctatcacttcatccgcaacggctttaataaccggtgcagcggtggtgaaggtgttgctgttcttcgggaacacaatgcccgtctgcaatgcggtatagtcggccgctgctgcatccgtaccggttggattggttgccaatgcaatcgttacgtctttggcggctgcatagcccgctggtaacgataccgtgaaagcagtactgctgccttctgcaagcggagaagtgaccgctgttaaagtcagttttttctgcgcaggatcagtaccatccgtaatattaatgatagcgctggtagccggcatattggtgttaccggcattgccatctactttgatgaagccgccgtcgtcaaatacgttgttggttttagtggtaatagctgcggtagtaccggatgctgcattagcggcaatggtcacggaagttgggatggtaccatgactggtatcagccgtcgtagagcgcagggcatctttcgccaggttgatgatccaggctttaccagccttccagccatgcgggaaggtagcggtaatgatagcagaactgccttccgttaccgggtcaggcgtactggtcagcaacacggaatctcccgcagggaaaggatactgcgcatctttaatgctcatgtccattgttgccggcaggaacgtgtacacggtgctgagtgcatcacttaccgaaggagtgatatgtatatcttctgcatcttccaccaggatgtctgatgcaacctttaactgtgcaataccggaggcaccggtaaacgtagtatccgcaggcaggtaataatcagtattacgtatagccgttccggtagcgccgcccattgtaatcttaaccggtatctcggtggttactccggcaggtaaactgaagccaatattattgatactgttttcatttaccgcaccagatggcagcgtaaaggtgatctttgtgttggtagtattcctgcgggtggcatcattaatgatgactgctgtatctaacacggtgtatccggttaaaccaaacacactgcccgccaggcccagtcgttcgtcattttcaataatatgatcatcccccaccgcattgataacagtataagtagtagtataaggagaaggggtgttggccggtaaccggagggtatcttccgtcatccagccaaagtctgttacaccggcgtcggagccggccacttttcttgtcagcgcaattacaatgtcttttgcagaggtatatccggcaggcagcgcaatagtaaaacgggtactatcgccttctggcagatgatacgtcaggggggcaatggttaatttcttctgggcaggagaggtcgcgtcattgatgatcagggtaagactgtcctttaccaggatacctgcatccgcagtgcttcccactagtaccagcttgcgggtatcatccaacacctggttggtggtggttccaacaattaccgtatcagagagtatcctggctgctggtatggtaacggtacccgatgggaaagtataggtgcccgctgccgctgttgaagagccgccgggcgtaaagttaacctggatagggatttcggtggtaagacccgctggcagttctgcccatacgcccggagacgtgccttcattaatgctgttggcagcaatatgtaagataacaggagccgtcattggcaactgtgcatcggtaatatttactacaaacggtgtaacagttgtggtataagtagtggaaggtatagggtctgatgcagtaagttcgatctctatcttctctgttccttctatagcgttatcacttttaatcttgaacggaaccgtgatgcgaccagctccctggggaatagtaacgggtccggtaagttcatagtccgtaccatcagtagcagtggaagtgctttttttattgatgctcacatcaatcggcagatcggtagtaacaccggttggtaaagatatggttaccagcccgtcgtaaggctctttcagcaatgcaggagcatctgttgtaaaagaaagcaccgttaaagtaggatcaagccgggtagcatcctcaatgtggagcgatttggaagaagtttgtggttgtcccatcaccaccgcgtccgctttgaaatttaccagttcgtctttttccaggatactgtcttttacaggtcttaccgcgatgtttaccccgttggaatctttctctatataagcaatgttgttataggtaaaatctgatgcaaccgcctctgtgccggccaccactgataaatccacctgggttctttcagaagccagcactcctggaggaagtgttacacgaaccgaatcaataatgccttcccggatctttgccggaaccgataaggtaatatgtttgggttcatcatcctggatagtgtatacgctggtcgttcgcccggtgatgtttaccagtttattttcggtaacgggtaccagctgaaaggtcatatgccggctgtattccagggcgttgttaccaatgatttttatgttactcagtcgtattttatccccgggtacatatgctttcgcaggaatcataaaaccgccgtaaaaagtaaagtcggttccctgcaccgcattatgcaatccccccgatggaggcaccagcgccacttttacatacatctccgaggtaacggtagcggtattgttcaccaccaggtacaaatccggtgaggcgagatccccgttatttccttccaggccggtggcagagtctttttcaaacgacacggaaataggatcagtaccggtactaaggggcgatccctggagattaatatgcaccggtgtattgtcatatccataatcaactgccacacgggtaccaatagctttggtggtgggtttcacgccaagggtgatacctgctgccaaccctttaggggccgtgtttacgccgccttcatcaatggcgtttaccagcatgaagttgttaaagttctgcctgtctcctgccgacttggccacataggaagaaaaggtgctataggcgtgataggtatgtgagaattcgcctaccgtcgcgttgggataatcggaattaaaaccaggcggtcttataaaacctatgatgtccggattgggtcccccacccggaggattcatatacccggtagcacttctgttattatccagtataggccccaccggatcatcctgcatggtgggaaattcactcaggtacaggtaaaaagtggtagagggcctgtcgttataaaaagtataatccagtacaaagtaactgttgggcaccacgtaggtgatagtcatcagcacggtggcaacaaatggcccccttcctgcattttcataatacgagagggagtcaaccaaacaaaccttataagggtccgcaacggtgccggaacccattacctcggatatcttttcaaaattaatgtcaataggggtcggggtctgaaacccgctggtattttgcatcttgaaattcgaccggatccccatcacggagcttgagttttccttcctggattcagatcttccattcctggttacctcgtaggtgccatccgtattgatctttatcctcaatccatcggtaagcgtatttcctccaagggggttgatggttacctgcgcctgtacacccgtactgatcaggaaaaaagcggctatcaggaataacgcctggcacaggaatacggggatacgatggggcataccttgcttaattaatttcgtaggataggaaaggagtaacatataagcgtgtaaatttctatttatacatatagattttaagtcaaaaatgtgaaaaacagtcctttgtaaaaccctatatgcgaatctctgtaattggctctcccggcaggctctaatattgctccttcttctcttctgatgaaactgaaaaactagccgccggcaatttataatctctataatcgtatagtggtgggtgcctaagacgcgctaatgggcgttttttatgatttttataattatgccatacccttccatctgtcacacatctctaaacaattaaatataaaatcatatattttaattagcaaatttataataatatttatattaaatcaaattaatttatctaaccataagtgagggggccggaaacagtgattaacaaatttttaaggcagataacgccttatatatccgttgcggttatgttaaaagttaaaataaccctagatttgcaaaaaacaattcagaatgtcaacaattgcaaaatcaaacattgactttagcctcggatacaaggtaaaagacatgtctctcgcggcctggggtcgtaaagagatagaactggcagaagccgaaatgcccggactgatgtcactgagagaagaatatggtaacagcaaaccattgcaaggtgcacgtgttgctggttgtttgcatatgactatccaaactgccgtattaatagaaaccctggtagccctcggtgctgaggtgcgctggagctcctgcaatattttctctacgcaggaccacgctgccgctgctatcgccgctgcaggagtacccgtatttgcctggaaaggtctgaatgaagcagacttcgactggtgtattgaacaaaccctgttctttggcagccccgaccgtccgctgaatatgatcctggacgatggtggtgacctgactaacatggtgttcgacaaataccctgagctgatccagcacatcaaaggactgagcgaagaaaccactaccggtgttcaccgcttatacgaccgcatgaaagctggtactttaccaatgcctgcgatcaatatcaacgactccgttaccaaatcaaaattcgataacaaatacggttgccgcgaatcctgcgtagatgcgatccgtcgcgctacagatgtgatgattgccggtaaagtagctgttgttgccggttttggcgacgtaggtaaaggttccgctgaatcactgagaggtgcaggcgcccgcgttatcgttactgaaattgaccctatctgcgctttacaggctgcaatggaaggttatgaagtaaagaaaatgaacgacgccgttaaagaagccgatatcatcgtaaccaccactggttgccgcgatatcatcaccggcgaacacttcaaactgatgaaagataaatgcatcgtttccaatatcggtcacttcgatatcgaaatcgatgtagcctggttaaacaaaaactacggcaacactaaagttgaaatcaaaccacaggtagataaatacaccatcgatggtaaagatatcatcctgctggcagaaggccgcctggtaaacctcggttgcgctaccggccacccttctttcgtaatgagtaactcctttaccaaccaggtactggctcagctggaactgtggctccactcagaaaactacgaaaacaaagtatacgtactgcctaaacacctggatgaaaaagttgcccgtctccacctgaaaaaagtaggcgtggaactggatgtactgaccaccgcacaatctgaatacctcggtattcctgcagaaggtccattcaaaccagactactacagatactagttttttacgactgacaaatacaaatgcagcggagaagaagtcactactttttcttcgctgcattttttgtaaaagctaaaagccgtaattttgccacatgacaaagctgagtgtaaacatcaacaagtttgctaccctgcgcaacgcacgtggaggcaatctaccggatatattaaaagtggcccaggattgtgaacgcttcggcgccgacggcatcaccgttcacccccgccccgatgaacgccatatccgctaccaggatgtaagagacctgaaaccattggtcaccacagagttcaatatcgaaggatacccttcccaggactttatggacctcgtactggcggttaaacctcaccaatgcacactggtccccgatcctccggatgccatcacctccaacaccgggtgggataccatcgcataccagtcgcagctgaaagacgtgatctccaccctcaaaaaagcagggatcagggtctccatcttcctcaatgcagatgttacaaaagtagaaggcgctaaaaccgctggggccgaccgcatagaactctataccggcccttacgcagaagaatatacgaacgcacgcacgcagccgcaaaacctgcagctgttcaacgactataaaaacacggcaagagaagccaccgctattggcctggacctcaacgccggccacgaccttaacctcgataacctccgcttctttaaactgcatataccacagctgaaagaagtatccatcggccatgcactcgtggcagatgcactctacttcggtctggaaaataccatccagctgtataaaagacaactggccgactaacttatacaaaacaataaagccattccgtattattggaatggctttatcaacccttaaaacaatcaacatgaagttcataacggggtcacaacaaaaccggtatgaacagtatatagtttgccgtcatgactgacagcaatgttacacacttacttctttaataacgctatttccagcacttggttcatttgctttacataatgaaacttcatccccttaatataagatggattgatctccttaatatctttttcattttgccagcaaagaataatctcacggatacctgcccttttggcggccagtatcttttccttaataccacctaccggtaacacctgtccgcgaagcgtgatctcacccgtcatagccaggtatgattttaccctccggcccgtaaatacagaagccaacgctgtaagcatcgtgatgcccgcactcggaccatcctttggaacagcgccctccggcacatgcacatgcacactcttctgcgtaaacttcttcggatcaatacccgcttcctctgcatgggattgcagataagtcagtgctgtaacagccgactccttcatcacattacccaggttacccgtcagcttcagatcacccttaccctcgctcaaactgctttctataaacaggatatccccgcctacataggtccaggcaagccccaccgctactcccggcggattacctaccttatagatttcattggaataacggggtttacccaatatcttctgaagcccctcttcggttaacgcatccggtaatttctcatccatcgccacctgcttcgccaggttgcgcataatagcggcaaactgccggtcaagctcacgcaccccactctcacgggtgtaatcggcaatcaattgctctatcaccgtattgctgatctttaccttcgtatccttcaaaccatgtgcatccttttgcttgggcaacaggtgcctcttggcaatctctactttttcttcaatggaatacccgctcagatcaataatctccagcctgtcacgcagcgccgggtgaatagaactgatactattggcggtagcaatgaacaacaccttactcaggtcgtactccagctccaggtaattgtcgtagaaagtagcgttctgctcagggtccagtacctccagcaatgcggaactcggatcgccgcgcatatcgttaccaatcttatcaatttcatcgaggatcatcaccgggttcgacgatttgattttacggatcgactgtaccaccctgcccggcatagcgccgatataggttttacggtgcccgcggatctcactttcatcgtgcaaaccacccaggctcaggcgaacatatttacggccaacagcgttggcaatagatcggcccagggaagttttaccaatacccggagggcctacgaaacacagaatgggtgacttcatatcccccttcagtttcagcactgccaggtattccaggatgcgctcctttattttctccatgccataatggtcatggtccagtatcttcttcgccttcttcagatcataactatccgtggtgtactcgccccagggcaggtccagcaacagatccaggtgattatacaccacgctgtaatccggtgtgctcggatgcatacgctccagtttttcaatccccttcgcaaaagcttccgcagcggcagccggccatttcttttcttccgccttgcgcttcatttccttcagctcccggtcgttggcatctccacccagttcttccttgatcgacttcatctgctgctgcaggaaataatcccgctgctgcttgtccaggtcggccttggttttgttggtaattttattcttgagctctgccagctgtaattctgtttgcaacagtttcatcagcaattccgcacgggtacggaggttattgatctccagtaactgctgcttctctttcagatctgagttcaggttggaagaaacaaaatgcaccaggaaagaaggattctcaatgttctttaaaatgatgcttgcttctgaaggcaggttaggagaaagctggatgatctgtgctgccaggtctttgatggaagatatatacgcttcaaattctgaatcgtcttccgccgcttcatcgtgcaatacactgatcttggctttgaaatagggatcttccgtcactatctcgtctatcttaaagcgcttgcggccctgtatgatgatagtggtgccaccatcaggcattttaatgagctttacaatacgcgccacggtacccacttcactcagatctgtcacacccggatcttctatcgtactgtctttctgcgctaccaccccgatcgacttgtcggttttgtaggcgtcattgaccgcttttatggatttatcccggcccaccgtaatcggcagcacaacacccggaaataatactgtatttcgtaatggtaataatgccagttcatcgggaatcttttcatcctcctgtccttccccgtcttcattcaaagggataataggcatgaactccatttcatcttccgaatttcctaaataaaatctgttcatctgagatatttaaagcctcatgaggacattctgtcatacaacccggcaaaagtcctcgtttttttatgtatccctatatagtcaagtttgatgccaagtgacgctctggcaggaacggaagaacgcgcaacagcgttccttttatcacaaaaaagcagcaaagttaaagtatacactttaatctttgctgcttcatcaaaagttaacgctgaacgcgggaaactagaaggatacgcctacacccagctggatgctctggtttttccagttactggtgttagctacatctttgtaattgtttacgtcattaaagccaatcacataacgtgcactcacattaacaattggcagttgcagccacaaaccggctacacctgaaatgtcgccgcctttgaatgcttcattggcagcgcccaatacttttttatcgctcactaatgcgctgaactgaggtcctacctgtagtttcaaacgcggtgttcccaggtcaatgttggccagcaaaggaatactgagatagctcatagtaatcttcttaccattatcttccaggtttccagtattataaatttcactgaaatcgtctgtagtttttgttttggtagaagagaagattaactcaccctgaactccgaatcctttcaccagattcacctgggcaaacccaccgatgtgataacctaacttaaatccatcctgaaaaccggtaccatcaagctttccaagattagcaccccccttcacaccaaagcgaaggaatttcgtttgtgcattaacagttgacacggttgaaacagcagctatcatcagcactgctacggcgaaaaacagttttttcataaatctatgtattgttagtaatggttaaaatatagacgtccggagtaaaaaatacccctatgttgtaattacatttccagtaattacaaattccgtgctatttgttaataaaatcaaaaactgtataaaatacgtgccgtgaagtaactcataataccctgatctgtaccggttaagggcttaaaaaccgtataggaaggcgccaggtttatccgcccgataaaataggatacattcatggaaacatctattgcgcggggttcaaattcagtgtgatcttcaaaattaagctcgccaccgggagggttgcggagcttcaccatatggggcgaccggctgatatattgaaatgctttgagattactgtaatagttagccgttcccagcgtcatgttcacagaaggcgtcaccatcagtacatcaaaccggcccaccacgccggaaaaaataaaaggatgccttacagacgctatcacattgaaatcattgccatgcagcgtttctttggtatataagccctccgatacatgctttccccagccgtaatccaggctcaaaccgggttgcacccaccacttccggtaatagaagtaggcaaaaatttcattcttgatcggggtggaaggcacatctgaagaatcggcgaaaatatattttgtataagagataccagtaagaaagttcctgcttttcgtatagtcgtaaccggcggtgaagtcccattcaaaccagggcttatttaccgagttaaaaagataatacgcgctaacgccggcatacaggccgcttttgtgataataacttaaagaaggtgcgatgaatgtttttaaaacgaggggatattcaaagttagctactttactgccataagcaggattgttcccgtacccgataccggccactacttcgcttttctgctgtttctgcaacagcgaatccagctgtcgctccagctctgccaagctttgtcccgatgctacacggctacataacaacaggaaggtaaagaagtataggcgcatgttttaaaaagtacgtcgctgcaagataagcgtaaatcactttcatttaacccggcatccgcgaacaggacgaatatgtggttaaacaatgcttttctgtcggtcaatgcgcacaataccttcttataccaggtcgatcaccgtaatttccggcaaaatacccactcttcctggatagccaagaaacccgaagcccctgtttacatacaggaactgctcgcccttcttatataacccggcccactctttataaaaatattgggcaggactccatttcaaaccgggtatctccacaccaaactgcataccgtgggtatggcccgccagcatcagggcaatgtcgggatactctgtacgcacctgcgcatcccagtgggtggggtcgtgcgacagcaaaattttaaacggtatatgttccgctccttcgtaagcccttttcagatcgccgtaacggggaaaacgtttaatggcgctccagttttcaataccaatcagcgcaatctgctcaccgttgcggtccagcaccacgttctcgttcatcatcagcttccagcccagcttgccatgcaccgctttcaattcctccaggttctggtgctgcaacgcactgtagccattggcgtttttatccggccaggggtaataatcgccatagtcgtggttacccagggtggaatacacgcccatcggggctttcacctcccggaatacatccagccattccgccatttccaccgcccggtcattaaccaggtcaccggtaaacagcaccaggtcggccttctgatcattgatcattttaatccccttcataaccgcctcccggttagcaaagctgccggaatggatatcagagatctgcacaatgcgcagtcctttaaaagaggccggcaaatgcttaaaggccatttttattttatgtacccggtagttgtatttattggagaagccgtacaacagcgtaccaaaaaaagcgcctccggtgatgagtcccagccggttaataaactgtgaacgcgataatccgcccgctgccgggcttacagccgttgcaggcgcactgctgaatttgcggatcagccacaatacccctcttctgatgtcatctatcagcaggaacacggtcaccagcagctttgccagcaccaggcccatgaaaatcgccatcaggtaggatttgagcgtaggcgaccagttatgccagttgatatacggcaacaacgctatcatcaccacacagctgagagatataaaccagtaaatggaataagtgatgttccttacttttggagtagacatgtacaccatggccctgatggcctggaaaacgtaaatatccagcaacagcaggaaaacaatgagtatgacggaattcagtccgggtcgcattatagaaatttaatatagatacctaataatgaagcaatttaacacaactaaccgggtctgaaaagttaaaaccggtgcttgtaattatactagacgaataacaacgggaagaattgtatgttttatttttttttaccccgttaacaggttacggggcttgttctgcgaacactttgtgtataaataaatatactacagcgcccgaattttaggtaatcgttgtatttttgtccgattacgctacttttaatagagttacttttaaatataaggtgtagattaatcacggatgacggagagcagatttccccgaagttgtcgtgatgtattcaaatggattgattatgaagtatacttgctatggacattcctgttttgcggtggagattatggggaaaaagatcctttttgatcctttcatcacccataacgaactggcggctaaggtggatatccatgccataacggcggattatatttttgtttcccacggacatgaagatcatacggccgacctggtagacctggcaaaacggacaaatgcaacagtagtatccaattttgaaattgccacctgggcaggtaaacagggaatcgaaaaggtacatcccatgaataccggcgggaaatggaagtttgactttggtacggtaaaatgcgtggtggcacaacattccagcagtttacccgatggaacctacggcggtaatcccatgggtttcatatttatgacggaagaggggaatttttattatgccggcgataccgcactcaccgtggatatggagctgataccagctgttacttccctggattttgcagtactgccaattggcgataacttcaccatgggcatcgaagatgccattgcggccgctgaaatgatagaatgtgagaaaataataggggtacactacaacactttcggctacgttaagattgacacagacgaagcaaagatgcagtttattgatgccgggcttgaactgttactgcctgaaataggcagtactatagaggtttaaggaagaagtgatcatagctgatttatcctttatcctataaataaccttgaatttttaaattacacaatggctagaataatcgcaatcgctaaccaaaaaggtggcgtaggaaaaactacaagtgcaataaacctggcaagcagcctggctgtgctggaatttaagacactgctggttgacgccgacccgcaggcaaacagcaccacagggctgggtttcgacctgcgcaatgtgcagcagagcctgtacgattgtatggtgaatgacgtgctggccaaagacgttatcctggaatcagatactcccaacctgaaggtattgccttcccatatagacctcgtaggcgcagaactggaactcatcaaccatcccaacagggaaagagtgatgaaacaggtgatcgacaccgtggaagcggactacgacttcgttattgttgactgctccccttccctcggccttatcaccgtaaatgccctcgtggcgtccaactcggtgatcatacccgtgcagtgcgaattttttgcactggaaggactcggcaaactgctcaacaccatcaaaattgtacaaagccggctgaatatagaactggaaattgaaggcatcctgatgaccatgtacgatggccgtctgcgcctcagcaaccaggtagtggatgaagtaaaacaacattttgaagaaagtgtgtttaacaccatcatccaccgcaataccaaactgggagaagctcccagcttcggcaaatccgttattatgtatgatgcagccagcacaggtgcgattaactatctcaacctggccaaggaaatcctgcagaaacataatttcaccaaaattaaatctaaagacaaaatcctagctattaacgatgaccaatccaagtaagaaagaggcgttaggcaaaggcatccgctcactgcttcagaacatggatacagatctgaagcaaactgccggcgccctgggtgataaggtagtagctgctgctaccggtattgaacgcatatcgctggatctgattgccaccaatccgaaacagccgcgtcgtgactttgatgaggtttctttacaggagctaagccagtcgatcaagctgcacgatgttatccaacccatcaccgtatccaggatcagcgccaaaaaattccagctggtcgccggtgaacggcgcctgagagccagcaaacttgccggcctcaaagatattcccgcttatatccgccaggtaaacgaccaggaactcctggaactcgccctgctggaaaacctgcaacgggaaaacctcaacgccattgaagttggactcagctataaaaggcttatggatgaatgcagtctcacccaggaacaggtggccgaccgcatgggcaaagaaagaagtaccgttaccaactatatacgcctgctgaaactgcccccggatatccaggtagccgtgcgcaacggccagctcagcatgggccacgcccgcgtactcaccggcgtggaaaatgtggaaaaccaacttttcctgtataacgaaatcctgaaaaacggattgtcagtacgccaaacagaagaactggcccgcaccatcaatcaggccgataaaaatcatcagcaaaaagctgccaaagtaaaactacctcctgcttttcagaaaatacaggacaaactggccactcacttctctaccaaagtaaaactggacaggggaaaaagcggtaaaggcagcatcttaattgaattctattcggatgaagagctggatagtatcctcgaaaaaatagatatatacggtggctaataaggcgcattacatatttcattcactacgatactctttgttgtttttaatcgcggttgtaatggcagcgccattgcacgcgcagcaggataccctgcgcccggtagccaaaacaatggatacgctcatccggcccatccctgctccaggtacggacaccgtgaaagccaataaagccatcttcaccgacagcgcctatattcccgattccaaactcccccacagcccgcgtaaagcagccctttactccgccgtggtaccaggtctgggacaggcatataacagggaatactggaaaattccgctcgcatacgccgccatcggcacctgtgtgtatttcttcgtggataatatgaagacctacaaactgtaccgcgatgcctaccgcctccgggtagacggcaacccggatacaaacgacaccagcccggataccaaaccttatgatacggaatcactgaagctgggccgcgaccagttccggcagtatgtggactattccgtgttgttcttcatcctggcctatggcgtaaacattatagacgccacggtattcgcacacctccgcaactttgatatgtcagacgacctgagtatgcgcgtttctcccacactgatcaacaaccgtacactgggcatcggcatcaacatttccatcggcggcaaaaaggccaaaagccggtactttgccggccgctgatcatcattaatacatccacttaaatacaacttgcaagggtcatgaaaatagcgctcatcggatatggtaaaatgggacaggcaatagatgctattgccactgccaaaggacatgagataatactccgggtagacgtcaacagcaaacacctgctggaaaaagaacacctcggccaggcagatgtagccatcgagtttaccacccctgaaacagcttaccacaacatcgtaaagtgcttcgaggcaaatgtacccgtagtatccggtaccaccggctggctcgataaactgccggaaataaaagcgctttgcctggaaaaaaaccaggctttcctccacgccaccaatttcagcatcggcgttaatatcttctttgaactgaataagaaactggcagccctcatggccagccagccgcaatacaacgtacagatggaagaaatccatcatacccataaaaaggatgcgccaagcggtactgctattacactggcagaacaggtgctggcctccctgccccgtaaaaccggctgggtaaacgaagaaagcaaccaaccggaagcccttcccatcatctctaaaaggattgatccggcgccgggtacacacactgtaaattacacctccgccatcgacgatattaccatcacccacaccgcccactcccgtgaaggctttgcagccggcgcagtagtagcggcagaatggctgaaaggtaaaaccggcgtgttcaccatgcgggatgtattgaatttaggatagcagcagctaaacgcattagccgccggataccgctccggtggctaaaagccagccactcactgctggcagctaaaaactgcttatctttgcaggaatataaagtgtgcacggcactattagttcatccgtggagggatgcaaaaaagtcagtatgttatcgaaaaaaacgcaatacgcatttcacgcattagtacacctggcagagaacgtagataaaggccccatccttatatctgaaattgcacaggaaaaaaatatctctatcaaattcctggaaaatattttgctggaattgaagaatgccggcatcctcggcagtaaaaaaggaaaaggtggcggttattacctcatgcggcctccaaaagagatcgcactggccaaaatcatccgcctgctcgatggccccattgcgctgcttccctgcgtaagcctcaattactacgaacgctgcgaaaactgccgcgatgaagccgtttgcggcctcaacgaagtaatgggccgggtaagggactccgccctgaaaatcctcgagaacaaaactttgaaagacattctgacccggaacagctaatcagggtgtaaaatatccgagccggcccaaacgccggcttttccgctacagtagcaggttccaggatcaagtccacctcccctccaggtcacctccgggtttacagcacggatactcccagtgtaaagccactcctatcccagtctacagcggatatgtccccagcttacagcacatataagctactccttttccccgtccacagtaaatagcccccaggctctacccacgcccaatttccacccgccaccacagccattttacccgaaagaaataattttttaccttattagtctatcttttttataggttttatgtatttttgttgaaggagtgaccgtaatcgctccgctggcactagacatatcaattcaataaggaagatctacatgacagacattaccaccgcgctggtcaataaaccggttgaggaggccatacagtacctgctggaacaataccccggcgctgtagcattctccacctcttttggccaggaagaccaggtgatatcagatattatctggcgtaaccaattgccggttagagtttttaccctggacacgggccgcctctttcaggaaacatacgatgtaatggacctcaccatggcccgttataaacaacctgtagaagttttctaccccgacaccgccgcggtagaaaaactggtttccaccaaaggacccaacagcttttacgaatcagtggaaaaccgcaaagaatgctgcggcatccgtaaaattgtaccgctcaaccgggccctggaaggcgtaaaggtatggatcaccggcctccgggcagaacaatccgaaaaccggcaaggcatggaaatcctcgaatgggatgaacatcgccacctctataaatttaatccgctgatccactggggctacgacgaagtactggcctacctggatcaacataacgtgccctacaataaactgcacgataaaggcttcatcagcattggctgcgcaccctgtacacgcgccattgagccgggagaaaatccgcgcgccggccggtggtggtgggaacagtcgcagaaagaatgcggtctgcacggataaacaacatttgcttttagaataaattattatagtccatgactaatcaaataaattgggaatttcctcaggcactggaagatgaagccatttatatactccgcgaaacagtagcacagttcgaaaaaccagtgctcctgttctccggaggcaaggattcaattacactcgtacgactggcacagaaagcattttaccccggtaaaattcctttctccctgcttcatgtggataccggccacaacttcccggaaaccatcgaattccgtgattggctcgtgaattcactcggactggacatcatcgttagaaatgtacaggacagcatcgaccagggtaaagcccaggaagaaaccggcaaatacgccagcagaaacgccctccaaaccgttaccctcctggatgccatcgaagaaggaaaatttgacgcctgcatcggcggcgcccgcagggacgaagaaaaagcccgcgccaaagaaaggattttctccgtaagagacgaattcggtcaatggaacgccaaaatgcaacgccccgaactgttcgatatcctcaacggtaaaatcaatatcggtgaaaacgtacgcgtattccccatctccaactggacagaactggacgtgtggaattatatcgttcgtgaaaaactggaaataccttctatctatttctcccatgaaagagaaattatagaacgcgacggtctatactggccttactcctctttcctcaatactaccgccgatgaagtaccgttccgccagaaagtacgcttccgtaccgtaggcgacatgacctgtaccgccgccgtgttatctgaagccgataaactggaagatatcattgccgaaatcatggaagcaaagatctctgaacgtggcgcacgtatagatgacaaacgttctgaagccgctatggaaaagagaaaacaggcaggatacttctagcagcattccctgtaacacacactttaacttaattaaacacatcttttaacgccagccgctaaaagcaaaaaaataaaaataatggaggttttacgtatagccacttccggtagtgtagacgatggtaaaagtaccttaataggccgtttattatacgataccaattctattccgcaagataaaatggaagcgctccacgctgccagcaaacgcaaaggactggactttacagacctgtcgttgctaaccgacggactggtagcagaacgtgagcagggaattacgatagatgtggcacacatctacttctccacccctacccgtaaatacatcattgccgatacccccgggcatattgaatatacccgcaacatggtaaccggcgcctccaatgcacaggtatcgctgatcctcatcgatgcccgcagaggcatcgtggaacaaacacaccgccacttctttatcgctaacctcctccgtattccgtacctggtggtttgcgtaaataaaatggatctcgtggattacagcgaagcccgctttaaccagatagtggaagatttccagcaaatgctcgataacgccggttttaaaggacaggaagtgaagtttattcccatctcctccctgtatggcgaaaacgtggccagccgcacgggtgctatcaactggtacaacggcagcaccctgctggaatacctggaacaggtgtctttcgatcatgaagaccgtaaccaccctgcccgtttccccattcaaagcgtgatccgcccacgcaccaccgaataccacgatttccgtggctttgcaggcaaagtggccagcgggcatttctctgttggcgacgaagtgatctccctgccctccgggcaaaagagccgcatcaaaaccattgagcaatttgaaaaacaactaccggcagcgcatgcacgcgaaagcgtggtgatcaccctggaaggtgaaatagacagcagtcgcggtaacatgctcgtaaaaacaaacgaaataccaccgcaactaaaagaaataagcgccaatatctgctggatggaccagctgccgcttacttccggcaaaacctacctgttgcaacatggcgttaaccgcgtgaaagcaaaagtgcagcagatcaactacgtaacagacgtaaccaaccacgtacaggtaacggacaaaacatccatgacactaaacgacatcggcagaattacgctgaaaaccgcagcacccatattcgccgatccttatcagagcaatccggccaacggcgccttcattctcatcgatgaattcaacaacaccaccgtagcggtaggcttcatcgaagggtagcgcagcgcggattttgtcttggctcaggattacgctgattttactgattacctggatttttacttttggattttttttgattttttagattttcttataataattaagggagataagagcggatatccgcttctatctcccttaatcctttataaaatcaaaaaagtaaaaatccaggtaatcagtaaaatcagcgtaatcctgagccaagacaaaatccgcggcaatctcctatatatgctccagcatgtcccgcgtcattgccgccaggtcgaactctggcttccagccccaatcggcccgtgcctggctgtcgtcgatactgttgggccagccatctgcgatttgctgacggtaatccggttcgtaggccatggtgaaggcgggaatgtgtttctttatttctgcgcctatttctttcggggagaagctcatggcgcccaggttataagcggaacgtactgctattttagaggcgtctgcttccattagctcaatggtggcgcggatcgcatccggcatgtacatcattggcaggtacgtgttttcagagaggaagctggtatatttctgatgctctttcgcctcatggaaaatttcaatggcataatcagtggtaccgccgccgggcgccgatttatagctgatcaggccagggtaacgtaagcttcttacgtccacaccaaagcggtggttgtagtattcgcaccagcgctcacccgcaaatttgctgataccataaatggtggtaggctcaattaccgtgtgctgaggcgtttcctgcgatggtgagttaggaccaaataccgcgatggaacttggccagtatattttatcgaggttttcttctttcgcaatatccagtacgttcaacaggctttgcatgttaatatgccacgccagtaatggattcttttcaccggtggccgacaggatcgccgccagcagatagatctgggtgatattatgacggatcaccaacacatgcagcatctccttgttcatcacatccagcgacacatacggaccggttcctttcagcaaatcatgctcttcacgcagatctgaagccagcacattcgcatccccatacatctttcttaaggccagggtgagctccacgccaatttgtccgcaggcgcctataaccagtatcttatctttcttcatacaaaaatataattgtaagctattttaaatcggaccgtaatattaacgggttcgccgctatttccattcaccccgcctcagcgcatgacaatgctataacaataaaattaacgccaggttatacacatggttttcggattacaatgttatgacaattaccccaaatagcgtggcttcatcacctccctttgccagagaatgcctatctttgcaccttcaattaaatgacacaattttttcaagatatgaagcatttaaaatctttattcaaagagcaatacaaccccgaaaatttcttcctgattgctggtccctgtgtgattgaagaagaatccattttgatggaagtggcggaaaaagtatccaccatctgtaaaagattagcgatcccttatattttcaaggcttcttaccgtaaagcaaaccgtaccagcgtgcattccttcaccggaatcggtgatgtggaaggactggaactgctgcagaaaattggtaaaacttttaatgttccggttacttcagatattcactccgccgcagaagctgctatggcagccgcttacgtggatgtattgcaaatccctgccttcctctgccgccaaacggacatcctgctggccgccgcagaaacaggcaaggtagtaaatgtaaagaagggacagttcctcagcggcgaatccatgaaatttgccgtggaaaaaatcaagggagccggtaatgatcatatcatcctcaccgaacgtggtaccaccttcggctaccaggacctggtagtggactaccgcaatatccctatcatgaaacacctgggtgagcccgtggtaatggattgtacccactccttacaacagcccaaccaaaccagcggcgtaaccggtggtaacccgcaaatgatcagcaccatcgccagagcagccattgctaccggcgcagatggcctgttcattgaaacccaccccgatccttcctgcgcaaaatccgacggcgccaacatgctccgcctggatttactggaaccattactggaacaactggtggaactccgccaggtagtgagaaagttttaatccaaaccacataatgcaaaaaagctattatcatcttccggtggtaatagcttttttctttacatgaagctttgcacttttttcagtaaattcatgaaacacataaaactcagttcactatgattaatatccacgaattaaaatcaggtgataccattatcacaaattatggcgggacagaaaaggaagggaagattttgcaggtagatcatgaggataagaaagtgttggtggctacggatgaaaatgagttctggtacgatcttgataacctggaacctattcatctgaccgaggccaccctgctgaaactgcaatttcataaagatgaaacggcatcgtcgaaggcaggaggaacattgtatgtgagaggacccttctctatccgctggtttgaagaaggcaacaaaccgctgatgcagctgcattaccgggatgaaaccaggaatctcacagagccgatcacgttaaatgaattgcagaaccattatcaccagatgacattgtttcacctggaataaggaaaatatttaaaagaaaagaggtggttcacggataacgcgaaccacctcttttctttatatcaataacttataaataacgcagtggattcctccgggcatttagaatgtaattcttcatatttacccaaaaggcaagaatcatgtatacaatgagtggggagcccattgtcaggaaagtggcataaatgaaaaagatgcgaatacgggacgtggctacgccaagtttatctcctatagcggcacatacaccgaacgccttccattccacaaagtcttttatccggttcatacttcaaatttatcaaattccggctggaaaaacaaggaaaaaacggctggcagggctattccctgtaccgcgttgaatatcaggggaactttaaaagtacaggaagttttcaggtagttgacccgatgttaagtatttaatttaaaaacttgctgattttagttaattttgcgagcaatttttaaccgctcttaaataatttttttcccatggtgtttgatattgacatgattaaaaaagtgtatgcggcactcccgggtaaggtggaagcaacccgtaaaatgctgggtcgcccgctgacactggctgagaagattttgtacgctcacttgtatgcaccgactaccacgccctacgaaagaggcaaatcttatgttgaatttgcgccggatcgcgtagctatgcaggatgcaaccgcccagatggcattgctccagtttatgacctgcggtcgtgataaagttgcggttccctccactgttcattgtgatcacctcattcaggctaaagtaggcgctacagaagatctggcaacggctattgacaccaataaagaagtttacgatttcctttcctcaatttctgataaatacggcatcggtttctggaaaccaggcgctggtatcattcaccaggtagtgctggaaaactatgcgtttccgggtggtatgatgatcggtaccgactcccacacccctaatgccggcggtttaggcatggtggcgattggtgttggcggtgctgacgcggttgacgtaatggccggcttaccatgggagctgaaaatgccgaaactgatcggtgtgaaactgacgggcaaaatgagcggttggacttctgccaaagatattatcctgaaagtagcaggtatcctcaccgtaaaaggtggtaccggcgctatcgtggaatacttcggcgaaggtgcggatagcttcagcgctaccggtaaggcaaccatttgtaacatgggtgctgaaatcggcgctacctgttccctgtttgcatacgacagcaaaatggccgattacctgaaaatcaccggtcgctcagaagtggctgccctggctgatgaagtaagagaccatctccgccctgatgcagatgtatatgcagatccttccaaatactacgaccaggtgatcgaaatcaacctggacgaactggaaccttatgtaaacggtccgttcaccccggatctggcatggcctatctccaaatttgcacaggcagtaaaagaaaacaactggcctgaaaaactggaagtagccctcatcggttcctgcaccaactcttcctacgaagatatttcccgctctgcttccctggcacaacaggccatcgacaagcacctggagatgaaatctgaatacaccatcactcccggctctgaactggtacgtttcaccatcgaaagagacggtttactgaatacctttgaccaggtaggcggtgtggtactggcaaatgcctgcggtccgtgtatcggtcagtgggcccgtcatatcgacgaccctacccgtaaaaactctatcatcacttccttcaaccgtaacttcgcgaagagaaatgatggtaacgcttctacccacgcatttgtggcttctccggaaatcgtaacagcattggcgatcgcaggtgatcttaccttcaacccgctgaccgacaagctgaaaaacaaaaacggtgaagaagtaatgctggacgaaccggtaggttttgaactgcctccaaaaggctttgccgtggaagatgccggttaccaggcccctgctgccgatggtagcggtgttcaggtgaaagtatcccctacctccgaccgtttacaactcctggcgccatttgctgcatgggaaggcaccgatctgaaaggattgaaactgctcatcaaagcaaaaggtaaatgtactacggatcatatctctatggctggtccatggctgaaataccgcggtcacctggataacatctccaacaatatgctcattggtgcgatcaacgcattcaacgataaaagcgataccgttaaaaattccattaccggcgaatatggtgcagtacctgctaccatgcgcgactacaaagcacacggcttcggtgcagtggtagtaggtgatgaaaactacggtgaaggctccagccgcgaacacgctgctatggaaccccgtcacctcggcgttcgtgccatcctggtgaaatctttcgcccgtatccacgaaaccaacctgaaaaaacaaggcatgctgggtttgaccttcgctaacaaagaagattatgacctgatccaggaagatgataccatcgacatcctgggtcttactaccttcgctccaggtaaacaactcactgttgtgcttcatcataaagatggcaccaccagcgaattccctgtaaaccacacgtacaacgaacaacagatcgagtggtttaaagccggtggcgcactgaacgtaatccgtgcagaagctgcgaaaaaagcttaatcaggctactcagcataaaagaaacgggcaggaattttttctgcccgttttctttttaaattactccccgaaaagaaccctgcgtatgtcagcattaaatatcatctggtcctcccttcatcccaacacggatgtggcgctggttaacagctcctacgcggccctgctggatgcctaccaatcgcccggaaggtattatcacaactggtcgcatatacagcagctggtaagcctgcaacaggtctatgcgcatcagctcacagatccggaagccgtgctttttgccatcttctttcatgatatcatttataacccgcagcaacccgataatgaagagcgcagcgctgcagccgcagtagcccatctgcataaaattaattacccggcggaaaaaaccgcccaaatcagcgatttcattatcgccaccaaaacacatatcaatacccgtcaggatccggacctggattacttcctggacttcgacctgcaaatactcggcgccgcaccggaaacataccgggcctacgcacagcaaatcaggcaggagtaccaggtttaccccgatgaggtgtataactccggccgtaaaaaagtattgcagcatttcctggaaatgcccgccatttatgtaacaccggcgttccgggaacaatatgaaacagctgcccgcaccaacatccgggctgaattgaacactttataatcaaaaggatatgaatcgaattgttgtttactgtggctccagcgccggacatgatcccgtttatatgcaacaggccaccctgctgggcgccgcactggcccaacgcaaccttacactggtgtatggcggcgctaacgtaggactgatgggcgcagtggcagatggcgccttaaatgccggcggcaaagccattggcgtactgcctcacttcctgcaacagaaagaactggcgcataccggcctcacagaactgatcctggtggacaccatgcacgaacgcaaaacgaagatgaatgaattgtgcgatggcgttatcgcattgcccggaggcttcggcaccatggaggaattgtttgaaatgctcacctggggacaactgggcctgcataaaaaacccatcggcctgctgaatgtaaatggcttctacgacgccctgatggccctgtcgcaaaccatgtctgagaaaggcttcctcacggcagagaaccgtgatatgctgttatgcagcaatgatatcagcgacctgttattacaaatggaaaaataccagccaccggccaggtccaagtggatttcaccggcgcaaagctaaatcgtctttgatttccacaacggcttttccagggtgaaacggcgcaccaggctcaccctgaaattgcctgtgccaaaggtttgataagtatgtggtatcgacatgccgctacgggtgttcattcccacgtagtgtatccccgcaaaataacggctggaattataccccagcgaggcccgcaccgtattactgaattgcagtcccgctttacggctcacattcccgttttccaggaacagggtggtgatatttcctcctaaaccgccggtaagcgataaggataaaaagaagtgctccttcagcacaaaggtgtaagcatatcctacattggcagccagggaataaatgccggtcttatgataatgctcatcccgcagaaatgcggtatctgccatattggtggggatgagggaagaatcgcctttgatgccggcaaagaacatttctccgcctatgatcagcgaacccgcacttttcttctggtattcattctgtagattgggcgcacggtaagagaaacgtttgtcgttgaagatatatcccacattcaggccgaagtcggtgttcctgatatcaggccgctgcggataaggatgcagcgcagtataggctttaccatatacttcctccgggttggctacataatagcctttataatattgaccgtagaagtctaccacaattttacgcaggtatacatgcgactgcagatcgatgtatttcgttttgccgtacctgtcgttgctgttgataaatggcaggttaaacccgatgttaatgcctataaaccggtaattggcgccaaaccccacattaaaaggagtattgggacggtaaaggacatcagttttcgttttccggtctacgatgtcatacttggtgtacttgcgggagccgtacagccggaaggtaatatcttccgtatgatcttcgatatacgccgtatcattttctgttttcagccatttcaggaatcttccctgcgcctttgcctgcgcagatccaagtcccaatactaccagccatgctaaaattcgtaggttcataaacgttgtaggttataagcaatgatgttgatcagggcagttctatcacctcgagttgttgaatattaccagcctccagttgaaaacgcagcagcgtttttaccttgtgccatccttgttgaccgcatgcacccgggttcatatgtaacaaatgaagtgccgcgtccggcattactttcaggatgtgcgaatgcccgcagataaacagtttggcaggatgctgtttcagttgttccttcacgcccggggcatatttccccggatatccgccaatatgtgtcatcatcacctctactccttccaggttgaaacgcagggtttcggggtaacggatacggatatctgccccgtcgatattcccggaaacggccctgaaaggcttgaatttttccagtttatcggccagatccacattaccgatgtcgccggcatgccagatttcatctacttcttcaaaatatttgaatacctgtgggtgcaaatagctgtgggtatccgacattagtcctatctttttcaacggagaattgtattataattttatattttggtagtcatatgttaaaacaagaagtccctcatatcaccgcctgtttgcttatttgctgtcccgaccggccgggcatcgtagccggcgtatcacagttcctctacctgttgggtgcaaatatactggatgcaagtcaacacagtaccgatccacgggaaggattattttttatgcgtatggaattccagctggaacagcttgataagtccgcgctggaaacggctttccagcaacaggtagctaccccgctgcaaatggaatggaaaatagattacagcgatcgccgcaaacgtatggctatcatggtatcggcgtatgatcattgtttgctggaattattatggagatggaaaagcggtgagctggcggtagatatcccgctcgtgatctcgaatcatgcttccctggaaaaggaatgcactgcattggggatcccttttcactacctcccggtaagcagcggtaccaaggaattgcaggagcgcgttgccatgcggctgctggaagagcaccgggtggatttcaccgtactggccaggtacatgcagatcctgtcgccacagtttgtaagtcattatccgcaacggatcatcaatatccatcactctttcctgcctgccttcgccggcgcacgtccttacctcaacgcctatacgagaggcgtaaagctgattggcgccaccgcccactacgttaccaacgaactggatgaaggcccgattattgagcaggatgtggccagggtaagccacaagcacaccgtggaggacctggtgatgctgggccgtgacattgaacggcaggtgctcacccgtgcagtgaaagcgcatattgataaccgcgtgatcctgcatggcaacaaaaccattgtgttctgatggtttcagcggatttcgttaattttaaaagacatgttgcaaacggctttatatcattatctccgtaaggaatgcgatacggtcaccaccgcatatgccaccctgcgggaggctcccggtgacgctgatgccatacacgccatgcgggtaggcgtaaaaaagctgcgggcctttttttcgctggtaaaacagctgccggattattcgttcggggcgggtaaacatctacgcaccgccaggctgatacagtcgatcggcggcgcttccagggatacgcacctccaggaaaaaaacctgcgcagctatgaaaaaaaaatatcgtggcgcttttcatttgcgcatctcttactgcaaaacaaagccgctacagccagtgaaatgttagccgccacagtgaaatactgctccctgaaaaaactggagtcactgccggaaagatttaaagaggctattgccaataccgataccaatgctgctactgccgcgctgatcagctacctggaacaacagcatcaaaaaatcaccgtgccggccagcagcgcgcatcacacggtatggcacgaagtcaggaaagaagtaaaaacattgtactatcagctcaatatactggaacaggtactccctgctgttttcacagaaaacctcgccacgcctacccgtaaagcgggtgagcttcttggccaatggcatgataccagcgaattattgttgtttgtaaaggcaacggcagcacagctgaagaaagagaagattaccctgccggtaaatgcacaacagctgatacagctgctgcaaatggacatgaaagaacaactggcgcaatgcgcctggcaggttaaggaactgaaagccgctgccgtattttaacgtatacccgttaaagataacggctacacgctaaaatgcttcttccccgctatacgccatcactatctcaaaaaccagcgctgccgccagtttcgcagtgcggttatctatatccagtgaaggatttaattctgcaatatcggctcctgccactttcccgctttccagtatcttacggaaacattgcaggaacaaacctcccggcataataccattataagccgtagcgcttactcccggcgcaaagggtgctgcaaatacatccaggcaggtggtcaggtatactttatccacctggctgagaaaatgctgtatggcggcaaacaacgtgtctttatcctgcaaatgaaaagcatctgcgcttacataagtcgcttcttcttctcctgcagtattaaaaagctggcgggtattcccgttcttctggatacccagggccaggtaatgaaaaggcaggccggactgtttggcatcctgcgccagttgccagaagccggtacctgagctggcgccttcttcaccgggaacacggatatcaaaatgcgcatcaaagttgataaagcctacggattgctttcctgcaaaccggcggataccactggcatgcccatacgtaatttcatgaccgccgcccagtaacagcggcaggtaacctgccgtgaggatatcgttcaccgtttcgctgagcacctgctgtgcattttccagttcgccattgggacaaaggatatctcccgcatccagcaacaccgtttgtgcgttgaagtgaaccggaaagttggcaatcaccttccgtatggcggcgggtccttttgcagcacctgccctgcctttgttgcggcgcacgccttcatcgcaggcgaagcccagcaggacaatacctttctgacccggctgcaaaaccggcaagggcgtttgcaacaggtcggttacggtaattacctggtgccagcgcagcaggtcggggtctgtaccatcaatacgaccggtccaggaaccacttgcagtgggctgatagctttcttttgttatcatactaaaactcctttcttccataccagtgacggcttcatcttaccctggtaataaagtatgtcgcgataatccgcggtgggataagcctgcatatcagcggcgtaacctgccagcagctggcctgcatctttcagttgcaacgcaggcgctgctcttacggtcagcgcagccagtacttctgcggtggataacttttcggcggcgctcattacggcagcctgtatcagcaaatcgcccatgggggccgatccggggttccagtcgctcgcaatggctacacatgcacctgcattcagcagcctgcgcgccggcgcatataacatacctaatcccagtgaagcacctggcaaaactactgcaacggtatcagaattagcgagtaaagcaatttctttttcagtgctggcttccaggtgatcggcagataacgcccgcgcattcacggcaacttcagcaccgccggtgctgaactgatccgcatgcactgttgccacaaatccctgctgcatggcctgttgcaggaaaccggcagcagcctttgcagaaaaagcagtttcttctataaaaatatccacgcggttactcaactgctcctgctgcaccaccggcaacagttccgttaaaatccactccaggtaggcttcttcactgcctgtataatcacggggtttcatatgcgcagccaaacaggtggaaatcagcgtggcaggcgtgtgcagccccgcctgctgtatggcgcgcagcattttcaattcactctccaggttcaggccgtaaccactttttacttccatggtggtaacgccttctttcagatgccggttagcgcgggccaccgtgttctccgtaagggtaacaagatcggctatacgcgttttggtaaccgaatcccatataccaccgcctgcacgggctatttccaggtaacttttaccggctatgcgcatggcataatcacggttgcggctaccatcgtaacaaatgtgtgtatgacaatcaataaatcccggcaataacacgagcggtgtatcctggaaagcgatttcgcaatccgggtatttctgcaacagggttttgtaccctgctatcgcaatgatctccccgttttccaccactaccccgcccttctctatcacggtcaactgttcatcgtgcagggcgcctttcagcgacaagcccgtcattggcaggatctgggcaaaaggaccgattaatgttttcatgggcaatgattaagcggttaaccgctgtgattaaatgctgatatcaaatttttgtccccattcctgtgccttttcgtaacccgcatccgcatgacggaaaatgcccagcgccggatcattgaagagcacgcggcgtaagcactcagctgcacggtcggtaccatccgccagcactaccatgccggcatgttgtgaatatcccatccctacgccgccgccatgatgaaaagacacccaggtagcgccgccgccggtattggccatgaggttgagcaatgtccagtcgctcacagcatcggagccgtctttcatagattcggtttcgcgattgggagaggccacggagccacagtcgaggtgatcacggccaatcacaatcggcgctttcacttttcctgttctcaccagctcattaaaaataagccccgctttttcgcgttcgcccaatcccagccagcagatgcgtgcaggcaatccctggaacgccactttctcctgcgcttgtttcagccagttgatcaggtgggtattttccgggaacgcttccatcaacgcgcggtcggtggtataaatatcttccggatcgccggagagggctacccagcggaagggtcctttcccttcgcagaagagcggacggatatatgccggcgtaaatccggggaagttgaaagcattgggctctccgccttcccgcgcaaattcgcggatgttattaccataatcaaaagtaacggcgcctttctgctgcagctgcaacataaagcctacatggcgcgccatgcttttcagcgacagctcccggtattttgccgcatcgcttttacgcagttccagcgcggcctgcagtgtaatgccattaggcacgtacccgttcagcggatcatgtgcggacgtttgatcggtgaggatgtccggtatgatattatctttcagcattctttccagcatatcaccggcatcgcttaccaacccgatggataacgctgttccgttggcctgtgcttccttcgcccattgaatggcttcttcgtaggaataagtcatacggtcaatgtaacgggtatccagtcttttttgaatacgtgtaggatcaatgtcggcgccaatgaacacggctccggccatagtggctgccagaggctgtgcgccgcccataccgccaatacctgctgttaccagcagcttaccggccaggctgccattgaagtgctgccggccgcattccataaaggtttcataggttccctgtaatataccttgtgtaccgatatagatccagctgccggccgtcatttgtccgtacatcatcaggcccttggaacgcagttcgttgaaatgctcccaggtggcccatttcggcaccaggttgctgttggccagcattactcttggcgcctgcggatgcgtgcgtacaatacctaccggtttaccggattgcaccagcagggaatgctcgtcgtccagcgttaataatatttcgataattttctgaagagattcgcggttgcgcgctgcctggccgatgccgccgtacaccaccagctcatcgggattttcggctacttctgcatccaggttgttaagcagcatgcgcaggggcgcttcggtttgccaggatctggcgtgcagctgtgcaccacgtggcgctttataatgcgggtgagctgcatatgttttaataaagtccaaactggtcattataaagtccgtttaagttaagttgatgattagcggcagcttcattggctacacgtaccagcgattgatcgacaacaattttgtgcagggcggcaatatcattggcaaagatccggtccttatctgcaaaggttacatgtctgcgcgtatactgatgtacggcttccagtaccgggcctgatttcattggccggcgaaaatccactgcctgcgcggcatacaacagctcaatagcaagaatgtattcgagattgccgatcacctggttcaatttgcggccactgatagaccccattgatacatgatcttcctgacccagtgaagtaggtacgctgtcggcgctggcagggaaacacagggttttgttttccgttaccagtgcagcggtggtgtattgtggtatcatgaaaccggagttgagtccggcatcctggatcaataattttggcagcccgtatcttccttcaatcatcatataacaacgcctgtcggagatgttgcccagttccgcagcagccacggtagcgtagtccaggggcaatgccagtggctgcccgtggaagttgccaccgctgatggtgtcttctgcactgaaaataatggggttatcggtaacggcattcagctctatggtagtgagttcctgcaggtgttgccaggcggtgcgtgacgcgccgtgcacctgcggcatacagcgcagggaataagggtcctgcactcggccgcaatccacatgcgacgacatgatctccgagttatccagcaatgctttcaaacggtgcgctaccagctggttgccggggtacgggcggatagcatgtaagcggggatcaaatggtttggcggtgcccatcagtccttcgagcgacaacgccccgatgatatccgcggcttcgagtgcgttgtgcaggcgttgcaccgctttaacggcaaacgacaggatgaactgtgtgccgttgatgagcgccagtccttctttaggacccagcactatcggttgtatcccttcctgttgcatcatggaagcggtatctgttttcgcgccacggtacatcacatgccccagccctatcaatggcaggaacaggtgcgataacggtgcgaggtcgcccgaagcgcctacagagcccttttcaggcaccagcggcgttatcctgtgttcaatatgccagatgattctttcgagggtggacagcgccacacctgagtaaccctgtgccaatgcctgcactttggtgatgagcatgatgcgggcaatttcttccgggatattttctcctacacctacactgtgactttgcaggatgttgtattgcagagcgcgggtatctgcttccgaaatcttggtatcgcacaacgggccaaaaccagtgttaataccatataccgtggtgtgttgcgccacaatggtttgtacatagccgaagctggtttgtacacgcgtaatgacttccggtaccagtatgcctttcactttgccggcagcaatatcaatcgcgcgggcaacagtgagctggtcgataccgtacttaaaaatatcactcatgtcgttagatttttctggtgtatgaagtattataactgttgtctgatcctttctgataaagacttttgctgcactgactgttcaatctgggcgatggcagccagtatctgctggctttgtttgttttccgttgccaaagcttccatagcgccggtgatggcttcccatacgggttgtatctgttgcagcaggtcttcgccttttttggagaaagcgaccagttgccggcggccatcttccttacacggcgttgttttcaggagtcctttctttttcaggttggtcaccatctggcttacggcggagtgggatatttccagttgttctgcaatatcgatcatgggtaccggctgctgtctggataagaggtaaaacaccgggaaccagctggcatcaaagggtatgcccgcctgttcatataccttgtttacttccatgagaaagtattcgctcagcctgcgcaggcggctgccaaaaacgaggtagccaagtgatggataaaatgacatatgaaaaggttgatgttaatattatataagcgcttatacaatattacgaaagaaatacgaataatatagtcaccgggcaggaatattcactgctgtctgcccgcaacggtactattcgtactgcttcttactttttagcggtctgtttctttttagcggtctgtttctttttagtatcaaaccaaaggggggagctgtccgttacatcaccattgtagttgataaaaagctcttctcctttcttgatatcacgacgggtgatgatactcatggtttcttccttgaagtccatttcatactcacagttggggttgtaatcgtgattatagatagagcaaaagcccagtgccacgcaggaacgggtttcttttgcaccccagagaaaaatataattgtggagtcttgttttatccacaatctcagtatcgtcgtaagtgagaacgagcacgggtgacgtctcaattcttgttccggcagggattttttctttggtataaacaccccggccttttcctttcgacttatcaatgtacaaatacggctttatcatagcgtaatttcaaataaaagaagacgtaaagtaaagttaaagcaggaagttatcaaaatcatgtttaaaaaatttaggtttgccgcccggaaaatattttttttgcctttcattaacctgcatatatgatcaattataatccaaaggagtggtttacgttcattttccgtcttcataaagcggatacagtaaggaagctgttccccatgtttattgccctctccatctattctgccattgtagcctggctggaactggaggtctggaagatgtctgacaagagtgaactgaagaacatcacgctgatgtatggcctgctgggctttgtgatctccctgttactggtgttccgcaccaacaccgcgtatgaccgctggtgggaaggccgccggcaatggggcgccctggtgaacagcagccgcaacctggctattaaaatccaggccatactgccattggaaaacaaggccgacagggagttcttcaaagtaatgatcccgaacttcgcctatggcctgaaaaatcacctgcgcaaaacttatgtgcacgacgagatggaagctataccaggacaggagccgcttcatactgatatcagtaagcatgtgcctaaccagttgtcgcagctcatcatgactaaaaccatggacctgtaccgcagcgggcagctcagcggggatcagctcattgtgctgaacaacgagctgcagtcgtttgcagatgtatgcggcgcctgcgaacggatcaaaaatacccccatccctttttcctacagcgtatttatcaagaaatttatattcttctatgtaatgtccatgccctttggatacgtgttcagcctgggttacctcattatccccatgattgtattcgtattctttgtactggcaagcctcgagctcattgcagaagaaattgaagacccctttggcaaagacgccaacgatttgccgctggatagcatttgcagcaacatccgcctgcatgtatcagaattattataacgactgccccggcagcgtgctattttaacttaatttcgcagatagaggcaattgtatggaaaatgaagctttactggaaaaattccagacactgacaaaagaaagaaattaccgcgaactgtcagtatacctggacgaccagctgattacggatatagccgaattgattcacgaggtccccgaagatgccggaataatcatcaatcacctgtcgatcggcagagcggcagcggctttccgtatcctggactttcctttacaggaagatgtgatacgtactttatcgcccgcaaaaatagcagagctcatgaacgagctgccggcggatgaccgtaccgccttcctggaagagcttcccagcgaagcggtaaaagagctgatcaaactgttggaccccgaagaacggcgcatcaccctttccctcctgggctacaaggagaacagtgtgggccgtatcatgacgcccgattacattgccgttagagaagaatggaccgtgaaggaggtgctggattatatccgcgagcatggaaaggacagtgaaaccatcgacgtaatttatgtaatcgacgaaaaagggcagctgctggacgacttccggatacgtgagttcctgctcgtatcaccggaaacggtggtgcataccctcatggacgaccgctttgtatcgctccatgccaacgacgaccaggaagaggccatccaggttttccggatggaaaacagggtagccttgcccgtagcagacgaccagggcatcctgctcggtattgtgaccatcgatgatatgttgtggatcgccaacgaagaacatactgaagatatccagaagattggtggtaccgaagccctggacgagccttacctcgatatgcccctgctcaaactggtgaagaagcgggttggctggctggtagtattgtttatcggtgaaatgctgaccgccaccgccatgggattttttgaagatgaaattgcgaaggcggttgtactggcactgtttgtaccgctcatcatttccagtggcggtaacagcggctcacaggcttccacgcttattatacaggcaatggcgctgggcgaaatcagcgtgagcgactggtggcgcgtgatgcgccgggaaatcctttccggcctgctgctgggcggcgcactcggcgccatcggcttcctgcgtatcctgctctggaataccctgttcaatacttacggcgcacacaccgtgctgataggcgctacagtaggcatttccctggtaggcgtagtattgtggggaaccctctccggttctatgctgccgctggtactgaagaaatgcggcgcggatccggccacgtcctccgcgcctttcgtggcgaccctggtggatgtaaccgggttgttgatttactttacagtagcctataccctcatgaaaggcatcttgctgtaatgcgcaactatagcgggggaaaaggctttcctccgctaataacagatctctttaagcaccgttccttctcttgttttccgcactataaacaaccggtcgtattcattctctcctatagaatccgtatgtggcttagctttcaggctatgcaagatagggatcagggtattggaatgccctatcaccagcaggcgctttccccagtcctggtgccgggtaacctggtaaataaaagattccccgctggtatctgcggcataaaaacaagtatcgatgtgcaggtggatgcgcaaactatcggccgtggcaaccgctcttttataaggcgtgaagtaaattttattcaggcccgaatccttcagcagccggtataatgcgcctgccctttcctggcctgccagggttaaagtggaatccggacccgggtttctttctgcatgcctgatcacatagaaggtgcctgttaaaaaggtactgtcttcagataccggtaccggttggcggacgggcagcttcggcttacaagcggcaaggatcaggagggaaaggagtattgatatacgcatagcgtggatttaaggcagatgaccgcattacgtccatccaaaacttacggcaatttatgattaaaccgttacatttattccccaacaaaataatgaaccgctatgagaaaatgggttatacccgccattatttttttatcagccaaccgcatcagtgcccaacaggcaatgccgctcacggtagaaaagatcatgcgcgatcccaaatggataggaacttctcctgataacgttttctggggtaccgacaaccagaccgtttatttcagctggaatcccggcaagcaactgagcgactccctttactatgccggtgttaaaaacaatacgccccggattacaaccgcaggtgagcgctctcttattaacgccaaagctgccggtacctggaatgcagataaatcgctactggcttattcctatgaaggggatatttatttactggagataaaaagcgggaaaaccacccgcatcaccaataccaaagccgtggagtttaacccggcattcagtttcggcggtaaacaggtggtgtttcagcaaaaccgcgatctttatggctgggacaaagcttccgggttaatcagtcagcttaccagctttgaagcaggcagcaagccggccgaaaacgatgacagtaaaaccggcaacgcagaagaaaagttcctcaaagcacagcaagaggaactgttgcaggtgatccgtgataaaaaaacaaagaaagacgccgccgaagcttttgataaagcatacgaccccaaaccactacggtccctgtacctgcaaaacaaaagactaagggacctgcagatcagtcccgacgggcgtttcgttacctatagccttttcaccgcacccactgatgcccgcaataccatcgttcccgaatttgtaaccgccaccggtttcaccaccgatattgcggcccgcgataaagtaggcgcgccgcaaggcagcttcgaaagttttgtatacgaccggcagcgtgatacggtgctccccatcaaaaccactgatctccccggcatcaaagaccagcccgattacgtaaaggactacacgaaaaaggatacgcccaaagtaagggaagtaattgtgaacggtccttactggtcggaacaaggcacacatgccattgccgacatccgctcacaggataataaagaccgctggattgtactcctcaacgctgaaaacggtaccgtgaaaacactgaaccgccagcgcgacgaagcctggataggcggccccggcattggctggagcatgggtggcagcaatatcggctggataaatgaaaacacctgctggttccagtcggaagccaccggttattcacatctgtataccgccaatgtaaacgatggtacagttaaacccctcaccagcggcaactatgaagtacaggaggcacaattatctcctgataaaaaatacttttatattaccaccaatgaagtacaccccggtgaaaaacaattttaccgtataggcgttgccggtggaaaggccgaaaggatcactaccctgcccggcgccaatgaagtaactgtttctccggatggaaaatggattgcgttccgttactcctattccaacaaaccctgggaattgtatgtgcagccaaacacaccgggcgcaaaagcagtacaggtcaccaacctggcgcagaccgatgaatttaaatcatatcactggcgcgatccgcaggtaataacgattaccgcgcgggataaccagcccgtgtatgcccgcttatacaccccggaccctgcaaaaaataatggcgcggcagtgattttcgtacatggcgcaggctacctgcaaaatgcacataaatggtggagctcctatttcagggaatacatgttccataacctgctcaccgataaaggctataccgtactggacatggattaccgtggcagtgccggctacggccgcaactggcgtacaggcatttaccgctatatgggcggcaaggatctggacgatgaagtggacggcgcaaaatatctggcagaaaaattgcaggtggacgcccatcgtatcggtatctacggaggcagttacggcggctttatgacgctgatggccctgttcacccagccagatgtgtttgcatccggcgctgcgctgaggtctgtaacggactgggcgcattataatcatggctacaccagcaatatactgaatgaaccattcactgacagtattgcttaccgcaggtcttcccccatctactttgcagatggactgaaaggcaaactgctgatgtgtcatggcatggtggataccaatgtgcatttccaggatatcgtgcggctgtcgcagcgactgattgaattagggaagaataactgggagctggccgtgtatcccgtggaagaccacggatttactacgcccagcagctggacagatgaatataaaagaatacttttgctcttcgagagtacgctcttgaagagatgattgcattttaaatttttttatttagttccgtcgatataaaaaaattataaaagggggatacagtgaatgatgcaggctaatgttaaggaatcttaatattcgcaaggatcgttcccggtattccctttttcattttacattaggaccgttgtaaaatgcatgctgaccatatctttacttaaacaatattcacattttctgatgtgatcttaacattttaatgcgatattgcaatgataaaacctagcacaaatccaaaaaccttatgtgtggaatcgtagcttacatcgggcagagagaagcctacccggtagtattaaaaggcctcaaaagactggaataccgcggatacgacagcgcgggagtagccctgatcaataacgggttacaggtatacaagaaaaaagataaagttgccgccctcgaagcattcgtggaaggaaaagatctccggagtcatattgccatcgggcatacccgctgggcaacacacggagaaccctgcgaccgcaatgcgcacccgcatttatccggcgacggtaaactggccatgatccacaatggcatcattgaaaactatgtacagctgaaacaggagctcattaaccagggccatgtttttcatagtgataccgataccgaagtactccttcattttattgaggaaatcaaaaaacaaaaccagtgttcactggaagaagccctgcgcatcgctttaaaaagagtggtaggcgcttatgtgattgtactcattgatgaagaaaacccggataccctcatcgccgcccgcaagggaagcccgctggtaataggcgttggcaagggcgaacacttcctggcttctgacgcatctcccatcattgaatacacgaaagaagtagtgtatgtaaatgattatgaaattgccatcatcaaagcagatgaactgatcctgaaaaacatttccaatgaaaggcaaacgccttacattcagaaactggatatcgaactagctgccattgaaaaaggaggctatgatcatttcatgctgaaggaaatctttgaacagccgcaaacgatcttcgatagcttacgtggccgtttagacgcgaaaaaaggcaccctcaccatgggtggcatgcgcgaatatgcggatgtgctgagcaatgccaaacgtatcatcatcgtagcctgcggtacctcctggcacgcagggctggtagccgaatacatgattgaagaattatgccgcatcccggtggaagtggaatacgcttccgagttccgctaccgcaacccggtagtaggtcccggtgatgtcatcattgccgtatcgcaatctggcgaaacagccgataccctcgtagccattgaaagcgctaaagaaaaaggcgctatcattctcggcgtttgcaacgtggtaggttcttctattgcacgcttatctcacgccggcgcttatacgcatgccggtcctgaaattggcgtggccagcaccaaagcctttactgcccagctggcagtgctttgcctggtaggcttaaaactggcggccgataaaggcaccatcaccccgcaaaggttccagcacctgctggatgaactggagcaggttcctgaaaaagtagcaacggcccttaaactggataaccagatcaaacaggtagccgccaaatataaagacgcacgtgattttctctacctgggccgcggatacaacttcccggtagccctggaaggagcgctcaaactgaaagaaatttcctatatccacgcggaaggctatcctgctgcggaaatgaaacacggtcccattgcactggtagatgaaaacctgccggtagtaattgtagccacgaaagacagctactacgaaaaagtagtgtctaacattcaggaaattaaagcccgtaaaggtaaagtgatcgcagtagtaacagaaggcgacaacaccattcctcccatggcggatgatgtaatttttgtgcctgcggcagatgaaatggtagcccctatcatttctgtagtaccgttacaactgctcgcttatcatataggcgtgctcaaaggtctggacgttgacaaaccccggaaccttgcgaaatcagttacagtagaataaagacaatggagatactcatctggttattttattatctgcacgcataataaaataaccagatagtcatttctcctcaaatgatgtatcctcatgaataatatccaaaaaagacccctttccgatctggggtataatttcattgaaaccacgttaccgaaaggcaaagacgaatattatctccgtaatgaacaatggagcaggcaggaccagtacaggaaattaacagcatacgaaatagaatcgctggtacgtaatgataacacctccgacgactggaatattatttttgtttccaacgaatttgatccacaactggtacagcactgccactttttcgggatggtacgtatcgggaaactggaaccctactacctggagttccataaccttcggatgccggtgggattgtacaacagtaccatctgcgcctgcgacttcggcgacaatgtagtagtacacaacgtaaattacctatcgcattatatcctcggcaacgaggtaattgtagccaacgtaaacgaaatggctactaccgattatgctaagttcggaaacggtatcctgaaagaaggcgaaaacgaaaacggccgcatctggatggaactgtgcaatgaaaacggtggcagaagcgtaatgccctttgatggcatgctccccggagatgcctacctgtggacacgctaccgcgatgatgaacaactgcaacagcaattcaaatcgttcacagaaaaacaattcgataaaaaacgtggctactacggtatggttggcgatcgtacagtgatcaaaaactgtaagatgatcaaagatgttaccattggtaccgacgcatacctgaaaggcgccaacaaactgaaaaaccttaccatcaacagcagcagcgaagcttcttcacaaataggagaaggctgcgaaatggtaaacggtatcatcggctacggctgccgcgtattctacggcgtgaaagccgttcgttttgtaatggcctcgcactcgcagttgaaatacggcgccaggctgatcaactcctatctcggcaacaacgccactatctcctgctgcgaagtattgaactcactcatcttcccggcacatgaacaacaccataacaactcgttcctgtgtgcagcgctgatcatgggtcagagcaacatggcagcaggcgccaccatcggctccaatcacaactcacgcggcgccgacggtgaaatcattgccggcagagggttctggccgggcctgtgcgtaagcctgaaacataattcccgcttcgccagcttcacccttatttccaaaggcaactatatgtcggagctgaatatctccattccattcagcctggtggtaaatgatgaacatgaaaaccgcctgaaaataatgcccggctactggttcctgtacaacatgtacgccattgccaggaactcctggaaatatgtagaccgcgacaaacgcaccgataaacaacaactcattgaatacgattacctggcgccggattctgtagaggaaatattccaggcgctggcgatcatggaaactgccaccgggaaagcatggtacgccctgccggaaaatgcctccaaaaaagaactaacggaaaaggacctccgtaaaaaaggaaaggacctgttaaaaaatagtccggaagaagtagccaagctcaccattctctccaaaggatttgaaaacagctcgcgtgaagtagaactgctgaaagtacacaaggcttatccattgttcgtggaaatggtagtactgtatgctgttaaaaatattctcgccgcagaaaaaccatcattcctggctttacaggccgcagtaagcaccgctaaacgcggcgactggcaaaacatcggcggacaactgatgaaagcggaaacggtagccacgctcaaaacaaagatccggaaaaataagatcagcagctggccgcaactgcacacggcctatgaagaaataggcaatgaatatgcagccgacaaattacaacatgccgtagcctgcctgctggaaataaaagacagctccctgaaaaatatgaccaccgccgatctcgcgcaatggatgaacgattctgttgtaacgatggagtggatcaccgcacaaattaaacgctccagggagaaggactacaaaaatccgttccgccagctggcctatgaaagtgaaaaagaaatgaatgcagtagttggcagcctggaagacaatagtttcattaaacaaactgctgaagacctggaaaagtataaattgcaggtaaacaaaaccatcagcgaatgggagctatagaaaaagtaagatgccactggtcggagaaagataagctttaccaggactaccacgacaaagaatggggcacgcccagtcatgacgataaacatctctttgaaatgttatgcctggaaggtgcgcaggcgggtctcagctggtataccgtacttaccaaaagagaaaattaccgcaaagcctttgataactgggacgctaaaaaaatagcgaaatacgacgagaaaaaagtggaagaactgatgcaaaacgagggcatcatccgcaaccgtctgaaaataaaatctgtgatcggcaacgcaaaagcctacctcgcagtccaaaaggaattcggcagctttgacaaatacatatggtcatttgtcaaccacaaacccatcgttaatcactaccgcaaaggcatggccggcgttcccgccaaaacagccatttccgacgccatgagcaaggacctgctgaaacggggattcaaattcgtgggctccaccatctgctacgcctacatgcaggccaccggcatggtagacgaccacatggaggagtgctggaagaagcgcggataatgcggattttgtcttgctcaggattacgctgattatactgattagctggatttttactttcttgattttataaaggattaagggagatagcagcggagatattcgcttttatctcccttacttattattaaaaaaattaaaaaatcaaagaaatccaaaaaatccaaaagtaaaaatcccggtaatcagtataatcagcgtaatcctgagcaagacaaaactcgcggcgatcctactcgatccgtacctcactaagggaagcattgccgagaaaagagtagtccgtgagcgtgttcagaaagaaatacagctgccgcttttcctggtccgacaacgggatgccctgctttaccagcgggtcggtggtgggagtgactttcacaccgtggtcgtagaagtcgaaaacctggaaaatatcgaagaaacgcccatcgtgcatataaggggcgcttttgagaatattgcgcagggaaggtaccttaaaacgaagattatcatctgtgctcccggtgatcttcatccggccgatgtcattcaatgccggtaaataaggcagcccattactgcggtaggtgagatctgtgaacaatggttccttatgacaggccgcgcacttctcctggaaaacggtgtatcctgcgttttcttcagcagtgaaggcaacgccggggactttgagcattacgctgtcgtatttggaaccggccgataccatggtggcaataaactgggtgaaggctttgaacatgcgctcactggtgatttcttccgtaccaaaagcagcttcgaacatactcctgtattgggagtctgtccgcattttttgcatcagctccttcaggtccaccgccatttcgttgtggtctgttaagggagtgagcgcctgtatttcgagatgattcacgccgccatcccacataaacgctttttgccagatcatgttaaacagtaccggtacagagcggatgccctgctgaccggccacgccatgcgccaatgcgtgatcaaaatggccgaaagccgcaaactgctggtgacaaaaaccacaggacacggtgctgtcctgcgacaggcggtaatcataaaacataaaccggcccaatgccacacctggtttggtgagcgggttacgggtgaagtcgtataccggccgcggaaaatgcgcgggcagctgcagtaaaaaaggctccggcccttttaccgcgcgcttctttgtgcccgcctgcaccagcgccagcaaaaggcaaaacgccccaatgatgtatatgaccttatgattcacgcagcggctaattggaaatacctgttatgttaaacatatgctgataattgccggctacctgtcttgcttttacgcccggcgccatgatcacggttatctttttaaaacttacagtatccggtaaaaaccacttttccacatcggcagtaagattaatacggggttgtttacctgctgcaattgttaccggctgcggaagcggcagcgtcacatatttcagcacaccatcttttgttttataaccgccgcaatgaaataaaaattcctgcataggcgtgttaaccgcagcagaatgaccttctatctgcgccataatataaccgctgttccacgtccagaacatgccggattctacagccagcgcgccggattgcaccccgctcacattacggatactatctaccccgatcaggaaacggatactcttatattcgccggcaggaatactatccagcaggatattttttgaactgtcgatcgcatcatctaccaggaaataagccggtggcaaagtaaccacattgccattgacggcttccagtgaaaagttgctgaggaaataacggaaacggctgatggtaaaagcctctcctgaagcattggtgtaagtgatctctttccttaccagcggctgctgccccatcaggtgggtgaaagacaattgcagggaaggtacaggcccgggatcagcaggcgccccggcaaacaacatggttacaaccaggaaccagcaagcataggaagcaaaaatccgcaaaatcatggtatcctcttttgttaaagaaagttacaatgattttgcggattaaatattaaaaagaaatctgctgattaaactcttttatatcctttccagccgtacaaaaacacaacaacaaagcagaaagtaggaatgccgtaagaaatagccagcgactgccattccgttacaatccccatcaggtaagggacggatgcaccacctacgatagacattacctggaaagaagcgccgcgtttggtatgtacacccaggtcttttacgcccaatgcaaaaatggtagggaacataatagacatgaagaagaagatagcgataagcgcgtatacagaaggagccccgttaccagtcattacaaaagcgcagagtaggacatttataaacgcataaacagcaagcaattgattcggagcgattttgcgcataagtgctgtgcccacaaagcgacctcctgtgaacagtgccataccaatagagagcagaagtgatgcatttttagcagaggtgccatgccagtattcagttacatagttaataaacaaagcgcctacacctacctgagccgccacataaaagaattgtgctaccactcctaatacaaaatgccggtgagcaaaaagcgggcgggtatccgccatcacctcttcaccttcctgttttgcttcttcaatttctggcaagggagttcttacgaaaaaagctgctattagcaatactacaacagcaatagcaacataagtaatctttaccgtggtgagatctcctttaccagtgccgagaaatagccaggcaccaataataggtcccaggaaagaccccagcccgttaaaacactgtgataaattcaaccgttgctcggaagtagctttatctcccaacacggttacatatggattggcagccgtttccaggcaggccaatccgcaagcaagtataaacaatgccagcaagaagaaatcaaaattgagtgcgttggccgctggataaaaaagaaatgcaccggtagcatacaacagcaaacccagtatgatccccttcttgtagccaaatttgttcataaacattcccgcaggaaatgccatgaggaaataagcgccgaaataagcgccctgtaataaagtagaacgtttcgtagtaatgctcaatacttcctggaaatgtttatttaatacatccagcagcccgtatgccagtccccataggaagaacaggctggtaaccaggatcagcgggaacaggtagctgccaggctttgcgcctgtatctttactggtggtataggtggaattacttactgcgcctccggccataacgaagaatttaatgtttcaggtgattaaatgttgataacgtgtgttggctctttatccttagctgatggatctgtcgagatgcgtgtaaccaccatctacgtatacgatttgtccggttgtgtgagatgaacgtgacgacagcaggaatacggtgctgttggcgatttctgttgaagtggtcatccttttttcaaatggaatgttagccgtgatagacgccagtttttcttttggattgggcaacgaattaatccaggtttcatacagcggcgtccatacttcagctgggataaccgtgtttacacgaatggagtatggcagcaattccactgcccactcacgggtaagcgcgttgatagcgcctttggaggcagcataaccactggtgttcccctggccggtatcggctactttagatccgatgttcacaatatttcctttggtgaccttcaggtacggcaatgcaaaatgcgccaggttgtagtagtgtgataaattattttgcagcgactgcataaaccgctcggggctgccattttccagtcctacgccatcattggcgccggcattgtttaccaggccgtctattctgccatactttgctatcgtttcagagatcacttttttacaatcttccactttacccagttctgcggtaacggcgatcgccttaccacccaccgcgataatttcgtttacggttttttcattatcggcagtactgcggccggcaatcacggtaataccaccttctgctgctatcagctttgcgatagcttccccgattccttttgcaccaccggtaacgataatcactttctcctgtaatcctaaatccatagtatgtatgatattattttttatagatgataaaatgagcgggcattgcctcccattatctgttcctgttcacttgttgataaggtgctgatgaaatctgtcacgatgcctttcacttcgtggtacctggcggctaccaggcacacgggccagtcggagccatacaccagcctgtttgcaccaaaggcttccagcgctacttccaggaaaggccggaagtgtgccggctcccactgctgccagtcggcttcggtaaccatgccgcttagtttgcagtatacgtttggcgactgtgcaatgcggcgcatatgtgccgcccatgcgtccagttcaccggctttaatatcgggcttggccaggtgatcaatgatcagtggctggtcagggaactgctgtacaaattcttctaccgcaggtaactgtttcggatatacgagaatatcatacgtgaaccggtgcttcgccagcgctttgataccgcggcagaaatgttccccgagaataaaccggttatccgcctcaccctgtacaatatggcggaagcctttcagcttcggatgtgcagcgtactgttccagttgttcactgatattttcagcgcggaggtctgtccagcccaccacgcctttaataaaatcatgcttatccgccagcgccagtaaaaaggccgtttcatccggcgactgatccgcctgtaccgccacacagccgtgaacgccgttttcagccaatacgggggccaggtcttccgggtaaaagtcgcggcggatcacttccatagattcatcgatccatgcgtcgcggacaggatcgtattgccagaaatgctgatgtgcgtcaataaccatgtagatattttttgcataccggtcgccggaagttccggcggccggtatactttacaatgcaaaaatctgatccataatcacccacttctcaccttcctttgctaccggcaatgactgctggtatttccacatcagctgttcccacacctttacggcgggattggcagcgtccatcgcatctttacgttcaaaggagaaagtatcgtctacttccatgatcataaacaggcggttaccggcacggtaaatatccattacggtaatgccggcgtccgtgatactcttttttatttcagcggatacgttgcggtgatgcgcttcatattcgctgatcaattgcggatcatctaccagatccagcgccagacaatatcttttcataattattatttacaggctacagcagtttgtttggaagtacccaaaccatcaatacccagttcaatcacatcccctgctttgaggtatacctgcggattcatgcccagacccacaccagcaggcgtaccggtggaaatcacatctcccgggagcagggtcatgaactggctcaggtaagccactacataagctacgttgaatataaagttggaagtattgccatcctgcattttctgaccgttaacggtgagccataaacgaagattattcacatcggcaatttcatctttggtagccagccatgggcctaacggagcgaatgtatcgcagctctttccttttacccactgtccgtttctttcaatctggaaagctctttcgctgtagtcgttatgcaggcagtaacccgctacgtagtccattgcgtctttttcttccacataagtggcctttttgccaattactactgccaattccacttcccagtcggttttctgactgttgcgcggaatcaccaggtcgtcgtttggacccaccagtgcgctggtacttttaaagaacacgataggttctgtaggaatggctgcgttggtttcacgcgcatgatctgcgtagttaagaccgatacagataattttggaaggacggaggataggtgagcccaaacgtgtaccggcaggcacctgcgggcattctgcagcatgtgcgccataccattctgataaccgcgccagcccgttggtttcaaagaatttctctccaaaatcttcaccaaaagcactcacgtcaaacattcccgctgcggttgcaacacccggtttttcttctcccggtaaaccaaacctgatcagtttcatatcgatattatttatttattagtcttacttaatttctttcagtgttttaatctgtaatcttccgttttccacatgcaggtcaatcaccggttctgctttaccatcttttacaaaagagaaatacacatgatcattttgtcctgttggctggatcacacctttactgccactgggcacgggcatgaacatacttttacggagaccgccaaattccacatacagctccaggctgtcgggtgaggcatccggcttgatctctgcaataaaatctgccaggatgtttccggactggatactctttttatattgctgcaacatttcgccgccggcagataccttaccaagacccagcgtaccttccatgtatgcccagattggctcaggcggcgtggcagcccataatattttcatgtcttttttactgtctacaaaagcgtggtaataacgtggctgatgattcgctttcataacgccgatataacagctgttgggctcattccacaacaccttataaaggtcttgttccggtgcgtctttcaggattgtttgttcaaaagttttttcctttgttccttctttcagctgaaatttaatcgtgaccagcgaagtatctttttccttatcagaaaaagtaacagatacggtaccacccggtgtagccggtttaaccgctgtggcggaatccccggtagcagtttccttgttggtaccggaattacaggcagataatacggctattgctattgccagccctattcgaaaatgttgcatgatataactaaaaattaatgaatgaataacttgaaagatacgggtaatcgtccgcactttaaaacacacatcatattaattattaattattaagcctgataaaaccgccatcgatgggatagtcggttccggtaataaagcctgcttcgtcggaacacaggaataacgccaggttacccacttccactggtttagccatgcggccgatgggttgtgttttactcagcttatcaaacatttcagcttccctgcccgggtaattcttggcaataaatccatccacaaacggcgtgtgtactcttgcgggcgacacgcagttgcaacggatattagcgccgaggtaatctttcgccacggataatgtcatagtcagcaccgcgcccttactcatagagtaggccagcctgtccggtatacctacactggaagcaatggatgccacattgaggatcacaccgccgccctgtgctttcatttgtttaatgactgcatacatgcagttataggtgcccttcacatttacctggtacaccctgtcgaagtcctgttccgccgtattttcgaggttacccacatgcgcaatgcctgcacagttcaccaggatatccagtttaccggccgtttgtacaataccgtccataacgcctatcacggctgcctggtcggctacattgcacgcatgcacacttgcctggccacctgctgccttgatttcctctgctgtagctttaccaccatcttcattcagctccaggatatgcacctgcgcaccctgggccccgaatgtttttgctattgcctgtcctatgccgctaccaccacctgtgataaccgctactttattgtctagtctgaacagttccatcattaaaaaatttaagggttctaaaatacctattaatataaggtgattgcaattgtattttcactgtatttcatactttcttgcctaattttcgcaaaattcaataatcaggtccaaatacggggctttttctgcaattttaagcacatgaaaataatactgttagcggcgctcctgtggaccatttccggccagctatccgcccagaaaataccggtgaataaatacggactcgccgtattgagcacccggcagcaatatgatcagctggtgaaagccgacagcaaccagctgctcgtaaacctggaaaagtatatcccgggcatcaaaaaagatgtgcgctatgccaccaccaataacttcaccaaacaaaagctttatacccgcaccgatatttacctccggctgccggcagccaaagccctcaaagcagtacaggaagccctgcgcaaaaagggatacggcctgcttatttacgatgcataccgtccttatcatgtaacggaaacgatgtttaaaatagtaccaaacgatctctatgcggccgatccccgcaaaggatcggggcacaaccgcggcgtggccatagacctgagtatggtaagcctgaaaacaaataagcccgtggcaatgcctacggactttgatgattttaccctgaaagcgcatgaaaactacaccccgccggacccggcaatggcggccaaccgcaaattgttaaaagataccatgatgcaacatggctttaaaggaagttctacagaatggtggcacttctatctgccggattataaaaaatacccgctgatggatatcttcttttaagatcatggaatcttcacggtatccacccggttgggaatcccctcccactttaaataataggtgccgttatcggcaggtataaaagaatacgttttggtttgtgtagtaaatgcctgtgtacatacggtgcaggtattgtatatatattccgcctttagcagtacggtatccttgtccctcatctccacaattttgttgatggcgtagcaggaattggggaaggtacagcttacatcataaaaagcaccgttctgacctcttgcatcgctggtggatttacccatgtatttcgcgcccacaatattcacccatccgtactgggagcaattatctccttctttgctgcaaccggcaaagagtaaaaaggcaaggagtaagggaattgttttcatcaggcaaatatttcacccgtagaacggggtggcgcgggaaaagttacagcacgcggattttgtctttctcaggattacgctgattttactgattaaccggatttttacttttggattttttttagatttctttgattttttttaataataagtaagggagataaaagcgaatatatccgcttctatctcccttaatcctttataaaatcaaaaaagtaaaaatccagttaatcagtaaaatcagcgtaatcctgagaaagacaaaatccgcggctagtatatcttgttcagcgcgtccacgtaggcgtgcacggaagcgttcacgatatcggtggagataccgaaaccgtagtacgactggccgttatgttttacgcgcatgtttactttactcacatcatcgctgccgccgcgcatggattgaatattaaattcatccagttcaatatcgtctttaataatatcgtggatcgcattgatggtagcattaacgggaccattaccggcagcactggcttctttttcttcgccattgatacgcagtttaacggtagccatggggcggagcggatcgccgcaaaccacctgcagtaagattactttgatggcattgtcaccgtaggttttagcgtcgccgtcgcccatcagttccagcagatcggcatcattgatttcctttttggtatccgccatcagcaggaagcgttggtacacttcgtcgatgtttactctttccaggttgtatcccaggcgcgacaggtgatgcttcagcgcatgacggccgctgcgggcagtgaggataatggagttggagttgatccctacatcttcagggttcaggatctcgtagttctcgcggtgtttcagcacgccatcctggtggatgccggagctgtgtgcaaatgcgttacggcctacaatggctttgttgggctgtaccggcatgtgcatcatggtttccacgagattactgatttcatagatcccttttgagttgatctgggtatgataacccagggcatgatgcgttttcaggatcatggctacttcttccagcgaagtgttaccggcacgttcaccgataccattgatagtacattccacctggcgcgcgccgttgataatacctgcaatggtattggcggtagccaaaccgaggtcgttatgacagtgaacggaaatgatcgctttatcgatattggaaacgtgatctacgaggtacttgatttttgcgccatactgatcgggcaggcagtaaccgttggtatcggggatgttaacggtggtagcaccggctgcaatcacggcttcgatcatgcgggccaggtattcattgtctgcgcggccggcatcttctgcataaaattccacatcgtcggtaaacttgcgggcataggttacagcggctacggcacgttgtaaaatttcatcgcgggtgctgttgaatttatatttgatgtgcatatcggaagaaccgataccggtatggatacgtttgcgttttgcgaagcgtaaagcatctgcggcagcatcaatgtctttgttattggcacgggtaagtgcgcagatcacgggctctgtaaccgctttggaaatttccaccacgctctggaagtcgcccggacttgaaatcgggaaacctgcttcaatgatatctacgcctagtgcttcgagttttttagctacttcaattttttcaacggttgtcagttgacagccggggacctgttctccatcacgcaaggtggtatcaaagacgtatacacgatttttatccatgatagtgtaataattttattgaatgattaattcagattctctaatactttggcgcccatcgcatcggtgcccataatgaaatcgttcacggtgtgtttgttggcgatgtccattgttctgtaaccctgtctgagagtagcttccacggctttgatcacccgttgtgattctgttttcaggccgaaggaaatatccagcatgagggcagcggataagatagaagccagcggattggcaatgcctttaccggcaatatcatgtgcagatccgtggatcggttcaaagaaaccggtgctgtcaccgatggaggcagatgccagcatacccatggaaccagcgatctgggaggcttcatccgtaaggatatctccaaacaggttaccggtaaccactacatcaaagcgtttaggatctttgatcagctgcatggccgcgttgtcgatgaacatatgttctgtttccacatcagggtattcttttgctacttcctgcaccacttctctccagagacggcttgcttccagcacgtttgctttatccacagagcacagctttttgcggcgggtacgcgctgcttcataagctttgcgggcaatgcgttctacttcataacggtggtagatcatgaggtccgaagcggtgttgcggtcggcagtccgggtcttttcaccgaaatacacgtcgccggtcagctcacggaaaaagaggatatctgaaccgcgtaaaatttccggtttaatgctggatgcttccagcagttcatcaaacaactttatcgggcggaggttggcatacaatcccagttctttcctgatcttcagcaaaccttgttctggtcttactttcagggtaggatcgttgtcatatttagcatgaccgatagcgccgaacaggatagcatcggcgttccgtgctttctgcagcgtttcttcaggcagcggatcaccggtagcttcaatggctacgtggcccatgatcccttcttcgaaggtaaaagtgtggtgataatttttggctattgttgtcagcactttttgtccccatgcggtcacttcctgtccgatcccatccccgggtataactagtattttcttctcaacgcccatatatgtgtttagcttttagtatttagctttttgatgattagaaattatatgttcttgtggtttcgtattgttcaatttctttacggaggctcagcaggtaatcgatatcatcatagccgttgagcaggcatgtttttttatactggttgatatcgaagttttctttttcgccggtgctcacaatttttatgaactggttttccaggtctacttccagttcggctttaggatcggcttctatggctttaaagatccggtccaggaaatcttctgatacctggatgggtaaaatgaaggtgttgagggcgttatttttaaagatgtctgcaaagaagctactcaccactactttaaaaccggcatccgcaatcgcccaggcagcgtgttcacgggaggaaccacaaccgaagtttttaccgcctacgaggatctggccactgtagatgggattgttcatcacaaaatccgcctttggcgtattatcggcttcatagcgccagtcgcggaacaggttttcgccgaaaccttcccgggtggtagctttcaggaagcgtgcggggatgatctggtctgtatctatattctcgatgggtacaggtaccgcagatgaaacgaggtgttgaaatattttactcatgatgattttacagtttaaatttttgtggcggctactctcaggcgcacataatccgcatacaattcgccgttccgcatcagctgtggcgccagttcgtattgcacctgctgcaggatggcgcctttgtcctgttccggcacaccggcaaaaaagtgagcgccaaacatctccagccagtcgctgatgcctgtttccggatccaccagttttgaagggcggtcaaaaaaatgcaccctgtctattttaaagccttccttttccagcagggtagtatattctgccggagatggaaaataccagaacggttcgtaggtataaccccgttgctgcatggccttttccaggtaagtaaggatctgctgcacattgcctttgccgcccatttctatcaccagccggccgccttttttaagttgggcgtacatccggctgatggctttttccttctcccgcacccagtggagggtagcattggaaaagatgccatcaaactgttgtggcagggaaaaagtagtagcgtcgcccacttcaaaggaaatgccgggaaaatgttcacgggcgctgctgatcatagcggcggaagcatctattcctgttacggtggcgcctttttgcgccagctgcgcggtgagttcaccggtgccgcaccccaggtccaggatattttcccccgattgtggctgcagccagtcgatcaggctgttgccatattcaaacacgaaggcgtgtttttctttgtataagtcagcgttccattgatccatagctttcggctttacttgttctttttgttaactattacgccaacaattcccttacatctgttaccctgcccgtaatggctgctgccgccgcggtgagcggactggccaggaaggtgcgggcattgggaccctgacgaccttcaaagttacggttggaggtggaaatgcagtacatgccggcaggcactttatcttcgttcatggccaggcaggcggagcaacctggttcacgcagctggaaaccggcttcggcaaatattttgtcgatgccttcttccatggcctgggcctccacctgtttggagccgggaacgatccataccactacatcgtctgctttatgtttgcctttcacaaaatctgctacgaggcgtaaatcttcaatgcgggagttggtgcagctgccgatgaatacataatccacttttttgcccagcagttcggcgccgggttggaggtccatatactcaagcgattttttgaaagaaggcctttctttctcgtcgagctgctccagagaaggaatgtgacgggtaacgcccatgcccataccggggttggtaccataagtaatctgtggttctatatcggcggcgtcaaaggtaagcacctggtcaaatacggcgtcgctgtcggaatacagtgttttccagtattccagggatttatcccagtcggctcccttaggcgcgaactcgcggcctttgatataatcgaaagtgatatcgtccggcgcgataaggcctccgcgggcgcccatttcaatactcatgttacagatggtcatgcgggcctccatactgagactgcggatggcttcccctgcatattccacaaagtaaccggtagcgccggaagcggatattttagagatgatataaagaatgatgtctttagaaagtacgcccttgcccagttgtccgttcacttcgatcttcatccgcttgggcttgtattgcaggatacactgggtagccagtacctgttctacttcggaggtaccgataccaaaggcaacagcgccaaaagctccgtgggtgctggtgtggctgtcgccgcaaacgatggtcatgcccggcagggtgatgcccagctccggtcctatcacgtgcacaatgccctggaaccggtggcccagtccgtaaagctctacaccgaattcagtagtattttttgtcaacatttccacctggcggcggctcaatgcttctttgataggctggtcctggtgtaaggtaggtacgttgtgatcggcggtagccctggttttagccgggcggaataccgggatgccacgcttacgcagcccgtcaaatgcctgggggctcgtcacctcgtgaataaagtgcgtgttgatgtacaccgcatcgggatgccccggcttgctaaccactatatggccatcccagattttatcaaataacgtttttcccatccttttgcttccttttataattgtttataccttcaaatctaatggtccttaattaattgccatatcgctaaatttgctttaattacaacctttaaacaccactgatacacgttaatatactgtttatcaataaattacaagattttaataacgatgcccaacagtcaaagtgatgctttattcatattaataaaaaccttaacaaaagccgaaaaacgcaattttcagttggcgtttaacaaaaacaacaccaaggaagatgtactttttatccaattgttcaccacgctggacaaaatgaaagagtacgatgaagagcagatactgaagaaaataacggatattaaaaagcagcagctatcgaatgtaaaagcacatctttacaagcacctgttatccagtttgcggcagctatataaacaaaaggacccgttgatcgacctgcgcgagcagctggaccatgcgcgggtgctgtataataaagggttgtacaaccagagcctgaagatactggccaaagccaaaacgatggcgcaggaacaggaagaggtaatgctgacctatgaaattgtggagtttgaaaagctgattgaatcgcggcatattacgcgaagcctggaaaaccgggcggaagtgctgagtgccgagtccaggcagatagaacagcagcttaccaatatcagccgcctgtcgaccctttccctgcggatgtatggcctttacctcaagctgggccacgcgcgcaatgagcgggatgccgaaatggtaaagtctttttttgaaagccagctgccgcccttgcagcatgtgcatatgagcttttacgaaaaagtgtacatgtaccaggcatcgagctggtactactatattctgcaggacttcgtgatgtattaccgatatacgcagaaatgggtggacctgtttcgcaaatacccgtccctgcagcaaacggatatggacctgtatattaaagcgcagcataatttgctgaccgcgcatttttatacttcgaattttgaaaagttcaaaacagctctgcaggacctggaagaatttatccgggacaaccaggataatttccacgaaaacacccgcacctctgcttttgtatacctgtataccgccaaaataaaccgttatttcctggaaggcacgttcagccagggtttggaaatggtgccggaactcgaaacagagatcaccaggcataccctgaaaatagaccagcaccgggtgctggtattttactataagattgcctgtttatattttggtagcggtgacaacaacaaagccattgtttatcttaataaaattatcaatttaaaaattggtaacctgcgggcagatatccagtgttttgcccgtatcctgcacctcattgcacattacgaactggagaattacagcctggtggaatacctgatcaaatctgtttaccatttcatttcaaaacacaaggatcttggtttggtgatggaagaaatcatgaaattcctccgccgttatatttatgccaatcccaaagcattacgtaatgcgttcgtagacctgaaagaccggctggagcagatctcggaagatccgtatgaacgccgatccttcctttacctggacattatttcctggctggaaagtaagattgagagcataccggtgcaggaagttattcaccggaaatttgtgaataaagaaaaacgcatttaaataaaaccgacgagcatatgtctgctgacaaacagtatcatttcactgccatttccggcagtttacggaaaggctcttacaacacgatggcgctgaaagcgctgcaaaaactgtgtccttcaaacatcagggtggagcaggtatttttcgacaagatcccgatgtacaatgccgacctgcataccgagcaattgccggaagaagtagtgccgctggtgcataaaattaaggaatcggatggcgtgatcatcgtttcaccggaatacaactactctatacccggcgccctgaaaaacgcgatagacgtggtttccaggcaccccgataaacccttcagcgaaaaggcagtggctattatgggcgcctcgcagggccagatcggtactgccaggatgcagtatcatttacggcaggtgatggtattcctgaatgcgtttgtgatcaacaaaccggagatcatgattggcaatgcccagcataagtttgataccgatggtaacctgacagatgaactggtgattaagcaaatccctcagttgttgctttcactggcacggctgagcgacaaaatgggtcatgatcctgcttctatataaggttcatagctgcggtattttgtaaaaaagataatggccgatgctgtctgtaacaacagtacagccggccattcataatgtccgagcaccatgaacagcacaatgaaagaagtgagcatggtataacgtacatgcacctccggattcattttagggaaaaacaatagggtacggaacaggatcattaatgataatgccgtgcagaataccgttatcagtccccatggcgttgttttcgtatatgcattaacggtaatgatgatcatctccggtaaaaaagtaatcacatatacccccaccagccgcatatagtggctgaataaattaacaggaagattctccatgaaattgaggtacgtatcatcaaacgcgcgatgatgcaccatcagctgcatatgtgtaagcacgctgatcataacacccagctgtagtccgcggagatcgaaataatcacctctcgtcataatgagaaatgtgagccacagcactcctgcggaaaacagtttggtgctcacaatccggcgtggaaaattagtaaacagttcatacaggaaaaacaataccggcggctttgtgaagtgccggttgatccagcgttgcaggtggcctgtaaaaaagatgacatccggttgttccagttttctttcatataacgttaacggccatatgcaattggcaatattaacaaccgtgatgatcaccgcctgtacataatatccctgtcggatcgcaataacaagggcaatggccacatataccagtaccggcatataaatggccgtatggagccgcagccagataacgcggcgggttggtttatcgatactgcccatggtgggatacaggaaatcatatccctgcagctgaaatgttttcagcatgaagcccacgcatttgagcgcgtaggacgtccacagcaggagtaccaggaacaggaacgtataattgcccaggaagcccagcatcaatcctttgtgataggcgagcaggttggcgccgtttaccacgccgaacagcaaataaaacagtaccaggaaaaagcccgtattctgaatatagaaccgttgtgtgaatattttgctaagtattgccgtggtggtacgcatatcagctgagcgtaatgtttttatgagctactttcagtgtgcccgttaccgttaattcttcctcatccagcggctggtgggaagtgatacaaaaagaaacgcctttggcgctgtactcccggatcaggtcgtacaaaacggccaatgcgcgggtatcgatggtgataaggggttcatccagcaggatgagggccgggttaccggtaaaggccagcagcagggataatttctttagcatgccgctcgaatagctgcttaccgggttattcacaaagatatgcacacccagtttttcactgatggcccggatgtctccggggttccctcctttggtgttgaggtaaagctccagtaaatcgcggccggtgaggaaagaagggtaaagcggttccgcttccgcgtagttgatcaggcggcggaactgtaccgggtgttcccggctgctcacctttccctgcagcagtatttcccctttgaaggggattaagcctgccatgaccttcatgcaggtggttttgccggcgccgttctccccctgcagccagtaaatgccggcgggcagctccagccgggcaatatccaggacaggtacatcctggtagttcttcttaaccgcatgaagggctataaccggttcgggcatatgaaaagacttaaaagtgtaaatatgaaaaattatcgcatatatatctacggaaggtcctctttttaacaaaaattttccgggtacatttttatactgatcatcattcatttagccgtaacagttaaaaaaataatcatataagccagatttttgcatggcccttttcacatgctaatcatattacatatgcacaaagtgcaaaacgcgtgaaacacgcattgccactatactttcattaaagttgtatatcttttccacacctgttgaaaactatatcgggcatgccttacccggatgcttacatttgtaatcctgagcgtatggattttaggaagcagagatgttgaaatcggattgtgggaaagagaagtgaagatttcggtatgctgaccccaaaagaaaaaccaaaaaccttcgacagtacccataaaataattaaagatgagtaacgagaatgaaattcttttaaaagagaacaaggaccgttttgtgctattgccgatcaaatacccaaaaatctgggagcaatacaaaaagcatgaggccagtttctggacagcagaagaaatagatttaagcagtgatcttaaggattgggcaggcctgaatgatggcgaacgtcattttatctctcacgtactggcatttttcgccgccagtgacgggatcgtaaatgagaacctggcagtaaactttatgagtgaagtacagatcccggaagcccggtgtttttacggcttccagatcatgatggaaaacatccactctgaaacatatgcattgctgatagacacctacgtaaaagacggcacagaaaaagaccgtttgttccacgccatcgataccgtacctgcggtaaagaaaaaagcggaatgggcattgcgctggattgaaaatggcaacttcgccgaacgcctggtggcatttgctgctgtagaaggtatcttcttcagcggtagtttctgctccattttctggttgaagaaaagaggcctgatgccgggattaaccttctccaacgaactgatcagccgcgatgagggcctgcactgcgaattcgcgtgcctgctttacagcatgctggaaaacaaactgagtgaagaacaggtacacggcatcatccgcgatgcagtgagctatgaaaaagaatttatcacagaagccctgccggttggactgatcggcatgaatgccgaactgatgtcgcaatacattgaatttgtggcagacagatggatcggtgaactgggctacaacaagatatttaatgcgtctaatccttttgacttcatggaaatgatttccttacagggtaagaccaacttctttgaaaaacgtgtgggagattaccagaaatccggcgtaatgggtggtacaaaagaatcacagacattcagcctggaagaagatttttaaaacattttgaattactaacctcttaaattcgcaaacccatgttcgtaatcaaaagagatggaaggaaagaagcagtgaagttcgataaaatcactgcgcgtattgaaaaactatgctatggtttcaatacagaatatgtagatgccatagatgtagcgaaaaaagtgatacaaggtttgtatgatggtgtaaccaccagcgaactcgacaacctggctgccgaaacggccgcttcccttactacaaagcaccctgactatgcactgctggcttcccgcatagcagtaagcaacctgcataagaataccatcaagtcgttttccaaaacgatgaagaaactgtatgattatattgatcccaaaaccggcaaaaacgcagcgctgctgtctgacgacgtttgggaaatcatccggaagaatgcagaaatcctggattccagcatcatctacgaccgcgactttgcctttgactatttcgggttcaaaacactggaacgttcttacctgctgaaaacagacggtaaagtgcaggaacgcccccagcatatgctgatgcgcgtatctgttggcattcacaaagaagacattgagtctgccatcaaaacatacaatctgatgagtgagcgctggtttacacatgccacgcctaccctgttcaacgcaggcactccaaaaccacagatgtcttcctgcttcctgctcaccatgcaggacgacagcatcgaaggcatttacgataccctgaaacaaacggccaaaatttcacagagcgccggtggtatcggtttaagcattcataatatccgcgctacaggatcttacatcagcggtaccaacggtacttccaatggtattatcccgatgctgcgcgtattcaacgatacagcacgctacgtggatcagggtggtggcaaacgcaaaggcgctttcgctatctacctggaaccatggcacgccgacatctacgaattcctggatctgcgcaagaaccacggtaaagaagaaatgcgcgcccgcgacctgttctacgccctctggatgccagacctgtttatgaaacgcgtggaatccaacggcgactggtcgttgttctgcccgcacgaagcaccaggactgcacgaatgctggggtgatgaatttgaagccctgtacgccaaatacgaacaggaaggacgcgcccgtaaaacagtaaaggcacaggatctctggtttgccatcctcgatgcgcaaatagaaaccggtaacccctacctgctgtataaagatgctgccaaccgcaaatccaaccagcaaaacctgggtaccatcaagagttccaacctctgcacggaaatcatcgagtatactgatgcagatgaagtggccgtttgtaacctggcctccctggcgctgccccgctttgtaattgatggtaaatttgatcaccagaaattattcgaggtaacctaccaggctaccctgaacctcaacaagatcatcgataacaactactaccctatcgaagaggccagacgcagcaacatgcgccaccgccctgtaggactgggtgtacaaggtcttgctgatgcgtttatcctgatgcgttatccatttgaaagcgacgaagctaaaaaactgaacagcgaaatatttgaaactatttacttcgcagggttaaccgcttccaacgatctcgcaaaagtagacggcgcctacgaaacctttaaaggctcccctgcctccaaaggtatcctccagtttgatatgtgggatgtgaaaccttccgcacgctgggactgggaaagcctgaaaaaatctatcgtgaaagatggtatccgcaactccctgttgctggcgccaatgcctaccgcttccacttcacaaatcctcggtaacaacgagtgctttgaaccatacacttccaacatctacacccgtcgtgtactgagcggtgagtttgtggtggtaaacaaacacctgctaaaagacctggtagaactgggactgtgggataatgatatgaaaacaaagattatttcacacaatggttctatccagaacattgctgaaatacctgcaaatattaaagaactgtacaaaacagtttgggaaatcaaacaacgtaacctcattgatatggcggctgaccgcggagctttcatctgccagtcacaatcactgaacctgttcgttgacacacctactaccggtaaacttacctccatgcacttctacgcctggaagaaaggtctgaaaaccggtatgtattacctgcgtactcaggcagccactcaggccgttcagtttactgtagagaaacaaggcggtcagcaaatccagccagtagttgctaccggcggcgacagcgcggcagaagaaatggtggtgggtgcagtttgcaccatggaagaaggttgcgttacctgcagtgcataagggtttatgtaagtataaatgcgaatccctggtcaaatggccagggatttttttgtgcaataactttacctaataccttttccccggcttcgtggtacaaaactccttacgcgcaatttgtttaataaacgtttcaggcgtggttcccaggtagtactgaaaatctttgatcaggtgactctgatcatgatacccaaagtcgtggatcagatcaaaccagtcgatcgaatccgcagtattatgttctatgctgctgatcacctgcttgaagcgcagaaaccgcagcatttctttgggggaataaccaacatatttcttaaaccgcatctgcaccgtacgttcggagaggtctgcatctgcagcaatggctttcgccggctggataagcggatcattaaaataatcagcgccgtttaaaagcggcagcgccccttcctccgccgcatgcgtagcggtggagatataatcctttagaatgtctactctttctgctgaagaaggcgttcttttcaatacttcccataattcatgtgcagatgcctgctccataaaatcaccggggtgatggagctgttcactattcagtgcatctaccggcacctggaacagccggtaaaaaccatccaggttgaataccacggccaacaggtctgtttccggcagcaattcgtagttcaacatcttccttaaagggcctaaaacagccactttatctatctgcatatcatccagctcggcggcggcaaaagagaacctgacaggggcgccaaaattgaacagccacatcatttcatagttgggcgacaggtgcgcggtagtggtaacgaaatcccggccggattgcatcacgtaaaaatgcttcacgatatccgacaatggcggcgaaacttcgaaatgtgtacctgctaatgccataaggagcggttaattttcttcatccagatcgtgtgccttgaatccccattccgtcagtaaagtctgatactgttcttccggcaatccctgtttattgtaatgccctgcaatggttttctgacgcatggcctcataaatactcactgcgcaggctaccgaaatattcagggagcggataatacccatctggggaataataaaattcccgtctgccattgccctggtggcatcgctcacgccgttctgttcattcccaaaaaccaatgctacagagccactgaaatcaatatcataaagactcaccgcatctgcggcgagatgtgtcgttaatattttgtcatatttgctgcgcaatacggcaaaacaatctgccgcattatcaaaatcatgtatggtgagccactgtttggcactgctactgcttctgtggccccagttctttatccgcggcgcttttgatgtgatgatataaatatcctgtattcctacggcatcgcatgtacgcatcaccgccgacacattatgagggtcctgtacatcctccagcactacggttaaattagcctgccgtttgcccaatacagataataatttttctcttctttccggtgtcatacgctgattattgccgctaaaatacgaaatagtgcagagatggtcctgcacccacatttcctcgtttacacattatgcttatcttcacccccaaaatatagataacctatgctcaaaaagatcctgaaaattgtgggtatcacaatggtggtcttgatactggccgctattgccatcccctatttctttaaagacaaaataatagcgaaagtaaaaacagaactgaataaaaagctgaccgccaaagtagattttaaagatgtggatatcagcttattccgccacttcccccggctggccgttggtctggaagacctgcaggtgatcggcaccggcgaatttgctgccgatacccttctttctgtaaaacagatagacatagccctcaacctgatgagtgtgatcaagggagataaaatggacatctacaacattgcactcttacagccacgcatacacgctattgttaataaagatggcgtacccaactgggatatcatgaagcctgataccgccgccgtaagtcctgccgacaccggcaaaagcagcttctccctcagtttacagcaatataaaattgaagatgcctgggtgaattacgacgaccgccagggcaacatggaattactcgttacaggcctgaaccaccagggcaagggcgactttacacaagaccagttcctcctgcaaaccagtaccacagccggcggcattaccttccggtatggcctcgttccttatttgtcgcaggtaaaaaccaccctggatgccgctatccaggtggataataacaccaacacctatacgtttaaagatggcaaagcctctctcaacaacctggaactggcgctgcaagggttctttaagctggtaaatgattccacctatggtatggatatgagctttaaagcgccttccaccaattttaaagacctgttgtctttaatacctgcggtatataaaacagatttcgataagataaaaaccagtggtaccgccgcttttggcgggttcgtaaaaggcaattattctcctgtgcaaatgcctgcgtttggactggacctggccgtaaaagatggtttcttccaatatcctgatcttccaaaaccggtaaaaaatatccagattgccatgaagatcagcaatcccgatggtgtaccggatcataccgtgatagatatgcccaccggccacctggaaatggataacacgccgctggacctgcgcatgctcattaaaacaccggtatctgatatgtatgtagacgctgctgccaaaggcaaactggatctttctaaaatcacccagtttgtaaaactcgaagccggcaccaatttatccggcctgctggatgccgacatcagcgccaaaggcaacatgagcgctatcgaaaaacaacagtacgatcgcttctatgccgccggcacactgcaactgagcaatatgctctacaaaagcaaagattaccccgatggtgtaaaagtgaataatctcttcttgcagttcaaccctaaaaacgtaacggtgaaagaccttaacggtcaatacctgggtaccaactttgaagccaacggagaagtgaataacctgctcgcctatacgtttaaaaacgagccgctggacggacaaatgaatttcaaagcagatgaaatcaacctcgacaaatggatgggtaccaccagcaccacttccaccgatcccgccactgcaaaaaaggattccgctgccgctaccccatttgccgtaccagctaacctgaacttaggattgcaggccaatgtgaataagatccactacgataaagccgatcttaccaatgtatccggcaagctgctggtaaaagatgaaacagtaaccatgcagcagttgaaagccaatgccctgcagggtactatggaaataaacggcagctacagcaccaaagccagcaaaacaaatcccgatatcaacctggcctacgacgtgcaaaacctggatgtgcaacaaacattcaacaccttcaataccgtacagaaattaatgccaatcggcaaattcctttccggtaaaattacctcgcagttaacgatgcatggtaaactgggaaaggatatgtcgcccgatctgagtacgcttacgggagatggcaacctgctgcttgtacaaggattcctgaaacagtttgccccaattgaccagctggccaacacccttaatgtaacacagctgaaagatctttcgctgcgtgacattaaaaactatttctcttttgaaaacggacgtgttaaagtaaacccgttcaaagtaacggtgaatggtatacgaatggatatcgccggttcgcacggctttgaccagtcgctcgattacacactgcagctggcactgccacgcagcatgatgggcactgccggcaacacgctggtgaacaacctggcgtcgcaggcacaaagcaaaggcatccccattaacctgggcgacagcgttcacctgcaggtattaatggccggaaacattctcaagccgagcgtaaaaaccgacctgcgtgaaacggctaacaacctcaaatcacaggcaacagaactggtaaagaacaagatcgacaccgtaaaaaatacggtaaaggatagtcttaaccagatcaaaaataccgctgtcaattccctgaaaaatcaactcaaagatcaactcagcggaaagaaggattctaccaaacccgccacgggcaaaccactggacaacgtaggcaaacaagccggcgaatccgtgaaaaacacgctgaacggcctgttcggcaagaagaaaccggcggcggataccacgaagcactgacgcggaggttgtctttcccgctgattacgctgattttactgattactttgattttactttttggattttataaaggatttggggagatgtaagcggatattttcgcttatatctccccaaatcctttataaaatcaaaaaagtaaaatcctttataaaatcaaaaaagtaaaatcaaagtaatcaacaaaatcagcgtaatcagcgggaaagacaaaatccgccttttttacgtaacttatggtaaccaaaaccccggaccatgtggttacgtttcttacattccacttattgtaatccagctatttttgcgggcatcatcttttatctcatggggtatttcatacaccgtttcccgcctaaaagccccaaatcctggtatggttaccgcagcgtattgtctaccaaaacgcctgaaatgtggcgctctgccaatgaatatgccgcatatatttcgcggcgtgtgggcgtgatactggtggttagcggcgttgcatgcgcgcttctttttcagcgtcagtccgattggttctggtatatcacggtgggcgctgtagtagcagggactatgtacctggtaggagatactgaatgggaattaacccgtcacttcgacaaagacggcaaacgtatccttccggaataaaacaaagaaggcgctgctttcgcaacgcctcttcgtgtatgtacaattataaacccttctctttttattacaatctgccctgcacatcgtgctccggtacagactgataattctctttcatcttacggagcttctctttgccgtaagccaaacgggtgatcaccacgtacagcaccggcactataaagatagccaggaaggtggcggtaaacataccacccaatacggtccagcccattgttttacgcgcttccgcacctgcgccggatgaaaataccagcggcaggatacccagcaggaaggccagggaagtcatgataatagggcgtaaacgcagcttcgctgcttccaccgccgctgttaccaggtccatgcccttatccacacgctccttcgcaaattccacgatcaggatcgcattcttggccgacaaaccgatcagcgtgatcaaaccgatctgtgcgtatacgttgttgctcagcttcggcaggaaggtaagcaccgtaatggccccaaaggcgccaataggcaccgccaggagtaccgagaatggtaccgaccagctctcatacaatgcggccaggaacaggaacacaaagatgatagacagcgcaaagatgtacaccgttttggaacccgacaggagttcctcgcggctcaaaccggagaactcataaccatatccatccggcagggtttgcgccgccacttctttcagcgcattgatggcgtcaccactactgtatcccggagccgggttaccatttatttccgcagagcggaacaggttatagtgtgaaattaccggggcactttctatcaccttataagaagtaagagaactcagtggcaccatagaaccggctgcattgcgtacaaataactggctcaggtttttgatatctccacgataactggaatccgcctgcgttaccacgcggaagttacggccatagatggtgaagtcgttgatataagcactacccatgtatgtttgcaatgcagtagcaatatcagatatcttcacccccattttcttcgccttctcacggtcgatgtccagctggtagccgggcgtgcgtgcggtgaagaaggagaatgccttggctatttcagggcgtttgttggcggcagccaggaagttctgtaataccccttcaaacgctttcacttcgccgcttcctttttgctccagtataaatgagaaccctgcggtagatcccagacccggaatggccggaggcggaattaccactacgtttgcttctttgtatttcgatagctttttctgcagtgcagctaccagtccgaaaacctgcagggaatccggcttgcgttcatcccagggcttcagctgacaaaagatagtcgcactgtttgatttagtggcaaagtttaccacgttcaaaccgccgagcgctgcatagtgggcaataccttcggtgttgtccaggtctttcatcatttgctgcatgacagccagcgtacgttctgtagaagaagattcgggcaaatcgaaggtgatgtaaatacgtccgtcatcttctgtaggaatgaacccggtgggcttcgctttgaataacatcattgttcccacaaaaatgcagatcaggatgacaactacaaagcggaagtagcggatacttttcttaacccccatggaataacgggaagtagtatgcccgaaccagcggttgaatttaaagaagaacttgttcagaccttttgaatctttatccaggtgcattggtttcagcaacaggatacacaacgccggtgttaatgacaaggctacaaaagcagagatcattaccgagatggcgatggtgatcgcaaactgctgatacaggcggcctacgataccaggtataaaccctaccggcacaaacaccgccgcgaggatcagtgcaatcgcaattaccggcccggatatttccttcatggccattgcagtagcgtctctcggcgacattttctcatggtcaatattatgctgcactgcttccaccaccacaatggcatcatccaccacgataccaatggccagtacgaaaccgaacaaagtaagggtgttgatggtaaatccaagcgggatgaagaagataaatgtggcgataatggataccgggatagccaataccgggatcagggtagcgcgccagctctgtaagaacaggaacaccacgatcactaccagtatcagcgcttccacgagtgtgtgcaatacttcctctatggatacttttactacagatacggattcaaatggcactacatattccacatcgtttggaaactgcttcttcagttcttccattgctgccgtaacattcttcgctgtttcaatcgcattgcttcccggcgcctggtaaaccagcaggtaggctgcacgcttgccatccacaaagttgttacccgcgtagttgaatttgcctaactgcacacgggctacatctttcaggtataccagcgttccgtctgacggacgtgttttaatgatcacatttccaaattcctcaggggtggataaacgtcctttggtgaagatgttgtattcaaaggtttgcccggtttgttgcggcggcgcacccacggaacctgcggtgatctgcgcattctgttctgccagcgctgcgcgtatatcctcggcagttacgcccatttctgcgagcttatcgggcttcagccagatacgcatactgaaatcatctgcacgggtaaagatatcacccacacctttggccctgagcaacgcatcttttacatatacgttggtgtagttatccaggaaggtaatatcgtgtgtgcctttgggtgagtacaaagctaccagcatgagaatgctgggattacgctttctaacggttaagcccaaacgctgtacttcctgtggcagggtaggctgcgcaatacccacgcggttttgcacatccagtgcggcgatgttgatgtcggtacctacttcaaagtttaccgtcatactcatctgaccactgctggtgttgttggtgttgatataggtcatgcccggcgtaccatttacctgtacttccacgggcgtggccacggtttgttctaccgtttgcgcatccgcaccggtataggtacctgttacctgcacagtggggggtgaaatttccggatactggccaatggccaggttcatcatcgccaatatccccaccagcaccagtactatagatattactatagccgttacgggtcgttttataaaagtatctgcaatcatgatcttctgctgttgattctactgataaactatttcttcgcaggcgcgcctgttggtgcggctggtattcctatctgtatcttgccgccatcacgtaaacgctggaagccttctgtaatcactttatcgccggcctgtataccgtccatgatcacgatcctgtcgccgattcttggtccgagatgtactttttgctgggctgccacagaatcttttgcgatgaatacaaagtattcacccatctgctcggtgatcgctttgtaaggaatgatcagcctttcgccggattgttcgttcaacacacgcaacacgcagctcataccatctttcaggcggtcgtcggggttactgaattcgatacgcacgcgaatagtaccggtctggttatccacgccgcggtcgatagccaggatcttaccggcatgaacgaactctgtgccatcggacaattgcaaccggaaggtggagtcgctggctttactgccctgcatggcggcaaaacgggagatatcattttctgttaccacgaaatcaacacctatcgggttttcgctggagatggtattcaggagggttgtaccggggctcacctgtgcgcccagctttacctgtgagataccgatacgcccggtaaacggcgctttgatcagggaataatccaggtcggtacgcacagcagacaggttggcttctgcggcagccagctggctgcgggaagtttccagcgtcgctttcgcgttatcgagtatctgacgggccaccgcatcctgctctgccagtcgctggtaacggtcgtcatctttttttgctctctcaaaggtggctcttgcgctggccacatttgcctgcgcctgcagataagccgcttcatatttacggcggtctatttcatacagggtctttcctttctgcaccacttcaccttctttaaaaaagatcccggtaataaaccctgacacctgggaacgcagttccacctggttcaacgctactactgtggcgggatatttatcgtaataaacggccggtgctacggatgcctccgcaatatttaccggtgtagggggcacagcaggcgctcctttctgggcaggacctttacaggcagtaaagcccaggatactggcagcgctgattaagacaatgttgttcatttttttcatatccgttccggttaccatttaataattagcggttaaggttcctaatgctttttgcaggtctatccggctggacagcacctggtacatggaattataaaaattcagttgcgcagtgcgcagttctgtttcagacaccagtacatcgaggtaagttttaattccttctttatactgcagttgtaacatatcgtatacatcctgtgccatctgtacattttctttcaatgtgagatagtcgttataattacttttatatgcagccattgcctgtgcgtactgcgaattgatctggcttcttaaagccgcgaaatcccattgtgtacgctggatctggagttctgccatgcgaatgttatgcactctttttcctccctggaaaatgggtaaggataatttcaatccaagtaaagagttggggaaattctcactgtataacttgccaaattgctcattctggtaagcaaaagagtagttaataaaagcagatacggtgggcaggtaactccatttattgtatttcaggttagcctgcagtaagctttgctgtgtttcgagtaactggtattcaatgcggtttttataatcggccgtcaacagggtgtccgcgccggttacctctgctgctacggaagcggaatcctccgtcagcggcacatcgccgccgttcagcggatatcccatcagttccttcaggtaagcctgtttggagatgagcagttcacgcgcggccttttgttgtgcgcgggcattgttcagtgaaatggtagcgcgcttggcatccgttttatccacaataccgctggcgtattggttattcgcgtctctgaggctgcgttccaggcggataatgtcttcactcaataccttgatctgctgtgtagtgaggagtacgtcgtagtaagccttgctcacatctgccaccaggtctatctggttgcgtgctgtggtctgatggctttgtttccgtacatcccttgccgtattggtggccagtaagagatcgcgggtaaagaggttctgattcagtccgaactgcgcggtagaagtattggccacgcctactttggtaggattaccaccaaaaatggaagtgggcagttccaggtaatgctggatattataatccaggttgatctgtggataccagtcggccagcttacttttcactgttctgtcggtaatcgcttcatcgatgcgcgattgcctgatgaccggctgatgggaaagggcataccgcacacattcctgcagggtagcgctggttaacagagagtccgtagattgctgtgcaaatacctgcggggatataaataatccgcacgccacagctaacaaataaaatgctcttttcataaaaggcttttgacattcagttcatcattgtaccaatcgaaagaaaataatgtataccagcaagcggttgatttctttcatggcatggcattatcatcccgtatttgttgcagcgctgtacgcactccaacatttttaattgccgcaaaaacatgttaagctgtaatcattacagcaaacaggtaggtcgataagagagttgcgaattcaaaatcatctgaaactttatcagcacggtttccaggatggtttcaggtatctgaatacaacgtataacagcgaagtaggtgaacaacaaaatgattctgttgcttaggtaaaacgaattcgggcgctaagataacgctatgaaaacgaaaatccacccttttgggtggattttaacaattaagtgaaaatcagttccggtcatcctttattacgaccgctgacaatatgtttctctgcgtgataagatgatcttactaacggtcctgactctacgtagtcaagtcccatattgtaacctatctcacgtaattcggcaaattcatcaggatgcacgaagcgggcaacaggcaggtgttttggagtaggctggagatactggcccagcgttaccacatcacaaccgttgtcgtacaggtcctgcatggcctgtaccacttcttcttttgtttcgcccaaaccgagcatgataccgcttttcgtgcgcatgccaccttctttcaggcgacggatcacttccaggctacggtgatatttggcttgtatccttacctgtttggttaaacgttctacagtttccaggttatgtgatacaatttcgggcgccacatcgataatgcgctggagattttcccattggccgcggaagtccgggataagggtttccatggtggtttccgggttcaatgcccttacggcattgatggtgttggcccagataatggaaccgccatctttcagttcatccctgtccacagaggtgataacggcatgttttactttcatcaggtaaatggcttcggccacacgctgtggttcatcaaaatccactgcctccggccgaccggtggctacggcgcaaaaaccgcagctacgggtacagatatttcccaggatcatgaaagtagcggtaccggctccccagcactcgcccatattagggcagttaccactttcgcagatcgtatgtaatttatgggtatctaccaggtttctaacctgtttataattctcgcctatgggtaatttaacgcgcagccagtctggcttttttactcttgttgtagccggttcggcggctattacgggtagttcttgcatcgcttattcctttctttagaagagcaaagttaatacttatctcttattccagcgcttcccgaattggatgctgatatatgcattaaaaaagaactgtttatttgggtcaacgccatccactatcaccataatagggatcttttttgtgtaatattcagcatttacccctacttccagggcgctcaccacctcgttaaaatgggcccagtcgaaccgcatgcccaatttggcatgtaaacccggtaccacactgaggttattccagcccttaccaaagccgccggcgccattgatctgttccttatgcaggaaaaggtctgccgtttccgggctgtatttgatatccacattctcgccgttttcgtcctgtacgttcaggtaataaggtttcaacagccccagggatacgcctccgtaatagatggcgtctacttctaccccgtttttattggctttgccaccgatcagataccgctgacccacgcccagcttagcctggtagaaattattctgtttaccgtatataaatggacgctgggtaaaggcataaccgctgttgttctttacttccttgtgacttttcttctctccaaactcaaactggaaataattcacctttttcctggttttccggtatcccagttccgcaaagccggaccagccgtcggtattcagccgggcacccgcggaaaagtcgcgctggaaaacgttttccccttcttcctgttcacggaaaatggagatcttcttcagcttacgctgttccttgtcgctcttcttattagtgctttgctgctgccgtgaggtggattgcgcaaacaagccgccggatattgttgccaaaaacaggattaagtatatttttttcacagtgggctattgttataataattaaacgcttgaacaaaggtattgttatgtatatattacaaacgtagctaatttttttttagtttaccagggccttcactgccagggaatacacttataataaaaatacatttaattttacggattgatcatttaaaaagatatcatgcaaacagcatctattatctataccggcgaacttcgtacaaccgccacccacctgcaatcaggcactgttatcgaaacagatgcccctgttgataaccgtggtaaaggagaaagattttccccgaccgacctggtggctaccgccctcggttcctgcatgctcagcatcatgggcattaaggcgctggataataactgggctattgaaggcaccaaagtaagcgttcagaaaataatgggctcagatccccgccgcattaccggcgtaaccatcgtattcgacttccccgccggccatggcttcggtgaaaaggaaagaaccatcctggaaagagctgccctcacctgcccggtggccaagagcgtgcacccggatattgtgcaggacgtaacctttaactggtaaagcggagaatcgccttcggcgattgtaaattgtcttggagcaggattacgctgattatactgattggcttgatttttacttttagattttaaaaagattaaagggagatagaaacggatatacccgcttttatctcccttcatctttttaaaatccaaaaaaatccaaaaagtaaaaatcaagccaatcagtataatcagcgtaatcctgctccaagacaatttccgcatcgccgaaggcgaggcgccctcctcacacccccgcgatgatcttcgctcctatggcgcaatgcaggcacttcttctcgtcgcagtagtgttgcttcagctgcaacagggcttgcgattccatagcgctttcctgggttacgcccagccggctccagctgttggtgatgtggttcttttccggcggcagctgttgcaggaaatgcaacgctttttcctggtaatatttcccgttcttatcctgtccgtacaggaacagcaatggcaataccgtgttgatcaggatgccctgcaccgcctgttttcccggccgttgtgtgcgggccacggagtgtccgaagcggtagtgcgtatgccagtacgccgacggctgtacgaagaacagctgttccagcgctgttacgtcgggggcttccagtatgcgggaaaacaggtggggagattgctgcaaaagcgccgcaaaagtggccagccgcatggtaggaaaggcggcaggccgcatccgcagccagttccattggtgagcggccatagggcttagccggaacttgtgttgcaggtgcccgtaaacatcctgtaactgcaacgcatatccgtctgtttggggcgcttccagcatacctgcctggccaaacagcagggcctccagctgaagcaacaggtgccggtaccgcatcagcattttgtagggcagcgactgtgccacctgcaggaatggtaaggtatttacgggcgtgccataactttgcgctaccgcccagtaacacacctcttcccagttgtagcgattatgctgcagccaggcccgcaggctgccgatcttacgttcccagcgctctgccagcaagcgttccttccagctgagccagatgaggggcggcacccgcgcagcatgcggggcacagggaacaaaaggcgacaaccgccgaagctcctcataccgctgcaggagcaacttgggaatatgctgttgcaattccaggcagggcgcctcgcccattcctacggcgggcatatcgtgtacaaacaccacatgcaggataattcgcccgtattgcggattatgctggtgcccatgccggaaccagtcggatgtacgcaggtgcagctccacctggcctacccataaagtagccccgatcctgatttttgcggccgaaaaatccggcccgccattgtggttgtgactaccgggaaacaagacctgtactgattctccgccggtagtggttagatgatcctgcttaaatagccggaatgcccagatatgctggaacagctcttctgagagcaacgggttaacaaacataagagatatggttgggtacaaaataatatcatccaaaggtaataaaacatcgattaataaataaaattcaactccaatttggaaatctgctcaaagtcatattacctttgcgccagttcttacacatcacttatccagaaaggcggagggacttggccctgcgatgccttagcaacctttcctgattattatgatcaggaaaaaggtgctaattcctgccccggtgcgaatcggggaaagataagttggcagagataatacttcacagagatatataactttctaaaggagctcttccaacaaacgggagagctttttttatgccccttccccacccttttcatggatttgttgttgtttaagttgatctttaatgatatcgttgcagttggcaattgtgcacattgaacatcattaaaaataatttataacatgaaaacagctacacaactgattcatagcatcccggtagacgaactgacaggcgccatttctgtgcctatctatcaaacgtccacctttgtgcaggaatcacccggcatcaataaaggctttgagttttcgcgggcgaacaaccccacgagaaaagtgctggaagaccttatctgcaacctggaagaagggtttgccggatttgcgtttgccagcggtatgtcggccatagatgcggtgctgaagctgttaaagaccggcgatgagatcatggccgtggaagacacctacggtggcatcttccagatctttaatcacatgtttgaacgctttggcatcaaagtgaattttgtagataccagcaacctcgataaagtactggccgccatcacgcccaatacaaggatcatctggctggaatcccctaccaatcctactttgcgcgtatctgatattaaatctatcagcaaaattgctaaacaacataacatcctgctggcggtagacaataccttcagcacaccattactgcaacagccgctgacactgggcgccgacctcgttatccacagcgcttccaaatacctcgcaggacactgtgacgtaattgccggcctcgtagtcgtaaactcaaaaacactggcagaccagatccggtataaccagaatatttccggcagtatcctcagcccgtttgaagcatggctcaccatacgcggtattgaaacattatacctgcgcctggaaaaacaatgcagcaacgccaacgccatcgccaattggctggccacacatcccgctgtggataaagtattttatcccggactggctactcataaaaatcatcacattgcccgtaaacaacaaaaaaattacggcgcactggtaagcttttccctgaaaagcgacaatatcaaaaacgctatacgtatcgtaaacgccaccaaattatttaagctggcagaaagctttggcggcgtgaaaagcatgctggcccatccggccaccatgacgcatcgtaccataccggaagaattccggagaaaaacaggtctgcaggactcctgcatccgtttatcagtaggcatcgaagatgctgatgacctgatcaacgacctgaaacaggcgctggataaattaaaccatccggccggcaagcaaattactgttttacaatagccgtcagcggttagcacaccactttcaatgttcagaacctgatcatctctgtgcagcgaaagactgacccctacggcggaaagctcaaaaaaaagtatggaaaacaagatcatcaatttaggcattttcggatttggcgtcgtaggacaaggactctatgaagttttgaacagaacaaaaggtattaatgcacggatcaaaaaaatctgtattaaagaccccaataaatcaagacctatcgatagcagctactttacgacagataaaaacgacatcctcgaagatcctaccattgacgtagtagtggaactgatcaacgacaccgaagcagccttcgaaatagtaagcaaagcactccgcaacggcaaagccgtagtaagcgccagcaaacgtatgatcgctgaaaacctgcccgcactataccagctgcaggcagaaaacaaagtgccattcctgtatgaagcgtccagctgtgcgagtattcccattatccgcaacctggaagaatattatgataacgacctgctcaatgctgtagaaggtatctgtaacggatctacgaattatattcttaccaaaatatttgaagagaacctcagctttgccactgccctgcaacaggcacaggacctgggtttcgcggaaacagatcctacacttgatatcgaaggatatgatccgaaatttaaaatagtgatcctgctgctgcacgcattcggcacctttgtgaaaccggaagaagtgttcaatttcgggatccatcacctcaatgattttgatatacaatttgccaaacaaagaaattgtaccatcaaactgattgcgcaatgccgccgccagaacggtcacgtatttgcgtatgtgctgccacacctgatcagggaacacaacctgctttatgatgtgtataacgaatacaatggtatcctgctggaaagcgcattcaccgataaacaattttttgtaggcaaaggcgcaggcggtacggctaccggcagcgcggtattatccgatatctctgccctgttatacaactaccgctacgaatacaaaaagatcaaacaaaacaatcagcccaactttaccaacgacgtaaacctgaaagtatacctgcgctacaaaacaccggaccaggtggacctggcagagttcttcaatatctctgagaaatatgaatctactgaatggcgctatgtggtaggtactattaacttacaaaaactgagagaagccggctggctgaaaaataaagatgtgaatattctcgtattggaataaagatagtaataagcaaaaaccaatcatgaaaacggcgcagttccctgcgccgttcctcttgcttaaaaattttccagttcttccactaccctgctcaccggtagccccattacattatagaagcaaccgtttatactgtctatgcccacagcgccgatccattcctggatcgcataagccccggctttatcaaaaggtttatacttatccacataataagtgatctgcccggtggttaacggcttgaaatgcacggccgttgttttggaaaaagcgacttctttttctccctgttgaataataacgccggtgactacacgatgttcacgcccgctgaggcgcgacaaaatatcaatggcatcttcacggtcctttggcttgccgataatgttgttatccagtaccaccactgtgtctgcagcgataatgatatcgctggcctcacacaggtgctgcacagcggccgctttctgccgggcaatatgaaccgggatatcgggtatggccagcccgggaggaaaagtttctgcggtttctaccaccttcacctggaaagggattccggcctgctccagcagctgctttctgcgtggcgactgggaagccaggataacgggcgcgcggttatacatctctataaataaagtttaaaaaatatcattgataaaataccggtgagcataattaccttcaccagggaactcaccttgtgatagtgttccggcaggcttgctttttttaatctcaggtagatataggcgcagggcacctgcacaaacaggaacaaatagccgatggcaatataccagccaagtatccacacccggatttccaccaggaggataataatgatcaatgccagcaacagcgcattgcaaaagcgtttggccgccagcactccccaggcaatgggcagggtgcggcacccgtctttgctgtcgcccatcatatcttccaggtccttcacaatttccctgaccatagaaatgaggaatgcaaataacgcatacaccccgatgatctggatcagcttccgtccggtgggcgacaagatggcttcaaagctatgatagatctgtttttcgtaaaaacctaccaccactactgccagggcagttagtaatgaaatgaccacattcccgatgagtacctgtcttttaaaagaagtggagtaaaaccagagcagcagggaacagattacctgggtgaagccgaggtaaaactgctctgttttccaggctaccaggaaacccagcgacacgccggccaggttaagcatggtgtgccaggccatagcccagcggcggctgataattttgtccagcaccattttatcgggcttgttgacaatatctatgttaatatcaaaatagtcgttgatgatataacccgcagctgctaccaatatagtagacaggcttaataaaataaattgaggaaccggcagtgacggctcttcgccggagctgcgtaaaaccggctctactacgcaatattgcagtaaaaactgggttaggccaatatatatcaggtttgggtacctgatcagtttaaaaaatgcagcccagagcttcatagtttttcttttattatttcgatgctattccttcatccattaaccaatgtccattcagtttcaatactttttccatgacttccctcacgcaaccgtggcctccgggcaatggggacacatacctggaaatactttttatttcggctgccgcatctgcggggcaggtgggcaaagccaccagttgcataggcagataatccgggatatcatctcccatatataatatctcttcccagcgaagatcattttcaaaaacataatcctgcagcttctcctgcttatcatgtatgccggtgaaaatatcttttataccgagtccctgtaacctgctcaccacactttctgattttcccccggagatgatcaccacacgataacctttttttaccgccagttgtaaagcataaccatccttgatgttcatcctgcgggacatttcacctcccggcagcaattgcagggtgccatcggtgagtacaccatctacgtccagcacaaaggtggtgatagatttaaataaagccaatacgttcatggggccaaaaatagccaattacgcattaagaatcgcttattctctatttattatggaactggtaaatggcgtcagacatcacctggtaaaccagttgcagataggggtcaccggccagcaattcgcggtggaggctcatggtggtttcgtcctggcgcagcgccggaccggtttgtaccgactctggtgcaaacttctccagccggtcgaaagtttcctttataataggttgtaacaggttaaagtccagctgttctttttcacaataggcttttgcctgtgcgatcaggtgattggtaaaattattacataataccgccgtgaggtgatatttcagccgttgttccgaggaagtaatggtaacgctgccggaaatactctgggcgagagattgcagtcgccggagcacctcgtcgttgctggcctccagcatcaccgggatgggcggatagctcttcacttccttgcggatcgactgtaacgggtatacaacccccgtattagacgatatccgggagatcgccgccaggggtacagcccctgcggtatgcgccaccatacgcttccctaagcgaagctggtcgttcagttcggggatggctgcatcacttaccgcgagcaggtatacgtctgcgtccatatttatatcctgcagatcgtctgtataatttgcgtggagcatctctcccagttccctggcgtgttccttgttccggctcaccacctgttttacctggtgcccatgaatttttaagaggtgtccgaaacaatgcgcaacattgccagtgccaacgataactacatccattataattaattttaaaataacaaaccgccggtatccgtctgattcgtgctttctaatatacgggttttagcgggtccccgtttttttcattacattacaacgtattttaacgtttaagagtgccttattttttaatttgatggtacttttatattattgcggaattcattgcagtaattattttatagaatttgcgtatttagcagcacaataaagaagcatacatggcaaaaaatttagttatagttgagtccccggcgaaagccaagaccatagaaaaaatattgggcaaagacttcgaagtcaggtcctgcttcggtcacatacgtgacctggagaaggatgacatggggatagacattgaaaataacttcaagcctaagtatgtgatcccggaagataaggaaaaggtggtgaaagagctgaagaagatggcgaaggataccgatgaggtatggctggcaacggatgaggaccgtgagggggaggccatttcctggcatctgtgtgaggtgttgaacctggacccaaagacgaccaaacgtatcgttttccatgaaatcaccaagcctgctattgaggctgcggtacaacatccgcgtcacctggatatggaccgtgtaaatgcacagcaggcccgccgtatcctggatcgcatcgtaggttttgaaatttccccggtactgtggcgcaaaatgagcatgcgcaactccctgtcggccggacgcgtacaatccgtagcggtacggctgattgtagaaagggaaagagagatcaatacctttaattcggtgagtaccttcaaagtggaagcttatttcaccggcaaggatattaatggtaagaacatttccttcaaggcagatggtcccggtaagttcaaaaccgcggaagatgcggagaaattcctggaacaatgtgttggagcggcttataccgtaaaagacatacaggttaaaccaggtaagaaatcacctgcagcgccttttaccacttccaccctgcagcaggaagccagccgcaaattaggctacagcgtttccaaaaccatgttgctggctcagaagctgtatgaaagcggtaatatcacctatatgcgtaccgactccgtaaacctgtcggataccgctatcggtgaaattgaaaaagcgatcaaaaccagtttcggtgataaataccatcagcaccggaaatttaaaaataagaatgagtccgcacaggaagcgcatgaggccatccgtcctacctacatggaaaacaccacggtagatgacagcgatacccgcaaactgtacgaactgatctggaaacgtactatcgccagccagatggcagatgcggaactggaaaaaaccaccgccaagatcgatatctctaccaaccacgaagagctgagcgccagcggggaagtattgaaattcgacggcttcctgaaagtatatatggagagccatgacgatgaggatgaaacagaagaagaacaggaaggctctttaccgccactggcagtaaaacagtcgctggatctgaaagagatgaaagccactgaaagattctcccgcccggctccccgttatacggaagccagcctggtaaagaaactggaagaactgggcattggccgtccgtctacctatgcacctaccattaccactatccagaagcgtaactatgtagaaaaaagggataaagaaggaataaaaagagatttccgtatcctgagcctcaaggacgataagatcactaaacaaaccgatgcggaaaataccggtgcagaaaaatcaaaattattcccgaccgatctgggaatgattgtgaccgacttcctgaaccagtattttaataatgtaatggactacggttttaccgccaagattgaaggggagtttgatgaaattgccagcggtaagaaggtatggaacacgatgatcagcgaattttattctcctttccacaaagatgtggaaaacaccctggaaaatgcagagcgtgtaaaaggagaacgtccgcttggcaccgatgccgctaccggtaaacccattgtagcccgcatgggccgttatggcccgatgatccagataggcagtgtggaagatgaggaaaagccgcgctttgccaaattgaaatctacccagagcattgaaaccatcaccatggatgaagccatggaattgtttaaattgccgcgtaacctgggtcagttcgaggactccgaggttattgtaaacattggccgttttggtccgtatgcacagcacgataagaagttttattccctgaaaaaggaaatggacccttatacggtggaactggatgaagtagcgccgctgattgcggagaaacgcaccgccaaagacgaacggactatcaagatatttgaaaaggagaaaattcagatcctgaagggcccatatggtccttatattaagcaaggcctgaagaactataagataccgaaggagaaaatagataacgcagctgatctgacagtggaagatgccaaagcgatcattgaagacgttaaagcaaatccacctaagaaaaaggcgcctcccagaaagaaaaaagcttaacgctgtggtaagaatatgctgaaaaatggggcaatgataataactgcagtgtgaatggtatgcttattatttaatttgccgacaggatcacattatttaatgattaccacatgatcataataatggtatgaacgaaaacagagaaataaacgctttgttccacctgttggatgatccggatctggaggtatttgatacggttgccagtaaaatattactgtacggtaaagatatcattccgaacctggagaatttgtgggagaatacaattgacgaggctattcaggaaaggatagaactgctcattcaccgggtacattaccaggatttgcaggcggcgttgcgtgtatgggggctttcagaaagacaggacctgatgcagggcgccatactggcggcccggtaccagtttcccgatctcatggatgcgcagatcattgcggaaatagaccggatcaaacgtaatatatggctggaactcaataattatcttacaccgctggaacagatcaatgtgctgaacagcatgatctataactactttggccttaaaggagaagaagtttcttaccagcgtaaaaatcagttttttattaaccaggtggtagaatccaaaaaaggtaaccctgttaccaatggaatcatttaccagagcctgtgcacaatgctggatttaccggtgtatgcagtgaatattccccggcagtttatcctggcgtatttcgacagctacatcgatttttccaccccgatagaacctgatgaccaccggatcctgttctttatagatcccatacagggccagatatatacccagcaggatgtagacacttatctgaaaagggtttctgtgccaccggtgccttcttacttcaaaccacaatccaacaaacgcattatacaattcttactggaagaattatccaaatgcttccgcgacgacaaagacgcctacaaacaggatgaactgatcaacctggcgagtatactcgaggattagcgcgcgccttcggcgcttttaaattgtcttggctcaggattacgctgattatactgatttgtttgatttttacttttttgatttttcatagattttataaatgattaagagagataaaagcgaatatatccgcttatatctctcttaatcatttataaaaatccaaaaaaacaaaatcaaacaaatcagtataatcagcgtaatcctgagccaagacaatttccgcagcgccgaaggcgcgaaggcccacacacgaaaaagcccaccgcacaagcgatgggcttcttaatttcttgcaagaaaagatattattgttataataatctcttacttagctggagttgcagcagcagcagaatcaacaggagcagttacagcagcagaatcaacgtgagcagcagaatcaactggagcagttgctactggagcagcgttcatagtgtctactggtgcagttgcagcagaatcagcagcaggagtgctaccaccgttacaagcaacgaagaacatgccagcggcaacagcgaatacgaataattttttcattttttaggttgttttatttttaaaaccgccgcaaaggtatgcaaaatttataaaatacaaaatctgcggcctgctttttcggtaagtatttatttttttctgaagaagatcttcaacggaacgcctgtaaagttgaatttcgtgcggatctggttctccaggtagttacggtatggtgttttcacatcatccgggagattacagaaaaacgcaaatgcaggtgtatgcgtagggatctgcgttacgtacttgatacggataggaatacctcttaccaccggtggatgatacgcttcaatagctttcagcagtacatcgtttaacacggaagtctggatacggcgtttacggttttcgtatacgtccagggctgtttcaatcgccttgaaaatacgttgcttttcagttacggaagtgaagatgatgggcacatcggagaatggcgccagtcgctctttcagtgttttttcataatccctggcggtgttggtacctttttccacgaggtcccatttgttcaccagtactactacgcctttacctttgcgggcagcgagactgaaaatgctgagatcctgtgcagtgatacctttttcggcatccagcagcagcattaccacatcagattcatctacggccttgatggcgcggatcacggaataaaattccaggtcttcatgcacttttgttttacgacggataccagcggtatctatcagcatgaaatctttctggaacatattatagcgggtgtgaatggtatcgcgggtagtgccggcaatttcggaaacgatattacgctctacgcctaccaatgcattcagcagggatgatttccctacgttaggctgaccaatgatcgctattttaggaatatctgtgtccagtctggcgtcttccatttccggggtaataaagcttaccacatcatccagcaattcgccggtaccgctaccggtcatggacgaaaggaagtggatatgttcgaagcccatactgtagaattcagtggcttccagctgacgctgactgttatctactttatttactacgaggaaaaccggtttggaggtgcgacgcagaatgtttgccacgtctgcatccaggtcggtaataccggtggttacatcacacatgaagatgattacattggcctcttccatagccacttttgcctgcttgcgaatctcccgctcaaatacatcatcactgttggttacaaatccgccagtatcgattacgttgaaggttttgccgttccagtcggcaataccgtattgacgatcgcgggttacaccgctttggtcatccacgatggccttccgttgttccagtaaacgattgaacaacgttgacttgcctacgttggggcgacccactatagctgctgtaaatcctgccatttttttattatattttgtcgtactaacctggataatacatccaggaattttgcaatgattaatatccgtattccttcaggaaagtgtcgttgtcgcgccatttgccgcgtactttcacaaacagttccaggaatactttccgctcaataaatttctctatctcctgccgggctaatgttcccagctcgcggatggatttacccttttcaccgaggataattcctttctgggtgtcgcgggtgacgatgatttcagcggtgatctttgtcagtgtttccttttcctggaattgtgtaacaattaccgtggtgtgataaggaatctcttcttcaaacaactgaaatactttttcacggatcatttctgccactaaaaaacgtgtagacttatccgttagtgtatcatccggatagaacgggttgccatcaggtaacagctttataatttcagccagcaactctttaatacctttcttctgcattgcagacaccggtactaccgctgctgctttgccccaggctttggcgcgttctaccagaacttccatatcctctttgaggatattatccattttattaaggatgagaacgatcggcactttcagtttcagtgaatcaaataattccaggttttcttccatagaatctttcgaatccatgatcagcaaagccacatcggcatcctcgagggcggatttaaccgcacccatcattttctcatgcagcttgtatttgggatcaatgatacccggcgtgtcagaaaaaacgatctgatacgcggggtccgttaatacgcctgtaatacggtgccgcgtggtttgcactttgggggaaataatagccagcttctcgccgataatggcgttcagcaaggtgctttttcccgcattgggcttaccaaaaatatttacaaaacctgccttatgcatgatgacatttaaaacctggtgatgttgctttcacaactcaaacttaccgaaataaaaaaagccgaatttcttcggctcttaatcttttttatggacgctgacgtacctattttgtagcgaggagcggattcgaaccactgaccttcgggttatgagcccgacgagctacctctgctctacctcgcaatgagggtgcaaagatacaaatatttcaatccgctccaaatcttttttaaaagaaaaacaaaaagccaaccgtaactggttggctttcatattggaatgcttcatacattgttaaaatggaagatcgtcagccggctgctcctgaacgggctctgcctcgggtacggtcatctcggcgaccggcattttccgcttttcctcgtccttacggccgagtaactgcagtgaaaacacccggagccggatggccccgcataacgcaccggtagctgtacttacataggcctccagttttggagcgccttctacatacaccattacaccctgcgttaaataaggagctacattggccttgtcccagagcgagcaatccacccaggtggttctttcttccagtatgccctgcgcgtttttaaaacgctcatttaccgctaccggaaaattgaaaacagtggcgccgttgacttcttttttcactacatcgcggccaagatgcccgataaactgaagtttgatcatcagaaataaagatttaaatgattaaaaatttataaaagatgactgagagaagtatccccgaaaattacgcatttttccttctcccaaaaaataatttctgatttattatagatacaagtatacctttgcattaacacaatacatggggtgccttactttcaggctgagatcacacccaatgaacctggaccaggtaatgctggttaggaatgaactaacagaaaacaggatatttaaaatgaaacagctaatgttattagtgctgctatctgtagcaggcactttacatgcacaatccctggttaccggtaccgttaccagtaaagccagcggccagccactggagggtgttaccatctccatcaaccaaaccggcgctgttaccgacagcagaggccactacagtattcatcttcctaaaaaaggaagttatcccttaaccgccagctacattggcttcaaaacatttaccactaccattacagcgaataacactacacagctggcagacatttcgctggaaacaacagcactgtttgtaaaaccggtagagatcagcagtttacgcgccggtaaaaattcgcctttcgtaaacaccactttaaccgcggcagaccttaagaaagaaaaccttggccaggacctgcccatactgctggatcagcaaccaggcgtagttactaactcagacgcaggtaccggtatcggctacacgggcatgcgcgtgcgcggttccgatatcacccgcatcaacgttacggtaaatggtatcccggtaaacgatgcggaatcgcagggaacattttttgtgaatatgcccgactttgcgtcctctgtgagcagcattcagctgcaacgcggcgtaggcacctctaccaacggcgccgctgcttttggcgccacgctgaacctcagcaccaacgaattcaatgaaaaagcatacggcgaaatcagcaacagctacggttctttcaatagctggaaacatacggtgaaagcaggttccggcctcatcaacgatcacttcaccatcgacgcacgcctttccaaaatttcatcagacgggtatatcgatcgcgctacttcagacctgcgctctttctatacttccgccgcctacgtttctgccaaaacagccatccgactgaacgtcttctccgggaaagaaaaaacataccaggcatggaacggcgtaccacaggcacttctggaaacagaccgcacctacaattctgcaggcaccgataaaccaggcaccccgtacgataatgaaacggataactaccaacaggatcattaccagctattcctgaaccaggaagtaaattcacatctcaacttcaacgtggccttccacctcacccgcggacgcggctactacgaacagtacaaagctcaacaacctttctctgaatacggcctgcaaggaccagtgatcaacggcaaacaggttgataccactgatctcgttcgccagctgtggctggacaactacttctatggctcggtattttcggtaaaccgcaccggtgacaagttcaactggagcctcggcggcggctggaaccgctataccggcgaccactacggcaaaatcatctgggcacaaacaggcatcgataaagaccatgaatattataattatcctgctgctaaaaacgatttcaatatctactggaaaggagaatataaactcacttctgccctcagcattttcgcagatatgcaataccgcaacatcatgtacaatatggatggctttgaagccgcacccgcatacattgcacatgtgaactataatttctttaatccgaaagcaggtatctcctataacatcaaccctaccaaccgtatattcgcttctgtggctattgcacacaaagagcccaaccgcgtagactttgaaaataactttggtacagcaacacccaaaccggaagtgctccgtgacgtggaagccggttattcatggaacaacaacatcgctgccatccaggccaacgtgtattacatgaactacaaaaaccaactggtgcaaaccggtatgctcaatgatgtgggtgcatacatccgtaccaacattcctaaaagctaccgcatgggtattgaagtaaatggaaatgtaaaactgggcagtatcgtgagtgtggccgccaatgcagctttgagccaaaacaaagtactggactatcatgccgttacttacgatgccgactacgcatcacatacccaggtgttcaacaaaacagatatctccttctccccttcttttgtaggtgggttaaccttaaccgtgaaaccggttaaaaacctgaacatcgatgtgctgggtaaatatgcaagccgtcagtatatggataacacctccaatgtagccggcagcctggatgcttactttgtaaacaacctgcgtatcaactacgtagtgccgcaaccgttattccgtgaacttgggctgcaattcatgctgaacaatatcttcaacgtgaagtatgaacctaacggaagtacctacagcagctatgatcaggctagtaaccgtgtggtgtacgacaattattattacccgatggcggggattaacttctttgccggagtgacgataggattctaaagcataggcggttgatcaaagcggattttgtcttggctcaggattacgctgattttactgattagctggatttttacttttggatttttttttgattttttagattttcttaaataataattaagggagataagagcgaatatccgcttctatctcccttaatcctttataaaatccaaaagtaaaaatccagctaatcagtaaaatcagcgtaatcctgagccaagacaaaatccgctcagctattcagtaatttctccaacgctttatctaccgattcaaaagggaaactttttatcactgcatccatttgtgcggcaatttgctgtgtacctaaattaccgatgctgcctgcgtgggtatgttttacttctttatcaggggagaaggtgccgttttcaatgtccatgcctacttttttataagcttcgcggaacggagtaccttgcagcaccaggttgtttaccacttccacgctgaagagatactggtacttatcatcgtccagtatgttttcctttatgcgcacattttccagcatcaggcggctcatgcggatacagtctttcaacgtttggaaggcggggaataaattctctttcagcagctgcaaatcgcggtgatagccggaaggcaggttggtgatcatcatagcaatttcgttcggcaatgcctggagcttattaccatgagagcggatcagttcccatacatccgggttctttttatgcggcatgatgctggagccggtggtgagttcatccgggaagctaatgaagccgaagttctggttcatgaacaaacaggcatccatggccattttagcaatggtggcggcaatgccggccagtgcaaaagccactattttttccgttttaccgcgtcccatctgtgcgtataccacgttgtagttgagcgaatcaaaacccagcaaggcagtggtaagctcacggtcgagggggaaggaagatccgtaacccgcggcggagccgagcgggtttttattcactactttataagcgccctgcaacatagtgaggtcgtctaccaggctttccgcataagcgccaaaccataatccgaaagaagagggcatggcaatttgcagatgggtgtaacctggtatcaggtgtgctttgtattcctcacttttttgctgtaacaggtggaacaacgcaagtacttcttctgtcatggtttgcagctcatgacgcaggaacagcttcagatctaccaaaacctggtcgttgcgggaacggccgctgtggatctttttgcctacttcccccaaccggcgggtcagcaacagttctacctgtgagtggatatcttccactccttcttccagtttaaaatcaccggactgaatttcctggtagatgtttttgagttcctgttttaatatagtgagttcttctgcttccagcaatcctatactttgcagcatggtgatatgtgccatagaacccagcacatcaaacggcgccaggaaggcgtccatttcacggtcttttcctacggtgaatgtttccaccgccgctaaggaggctttatctttttgccacaatttcataatactatagtttttccacgctgtgttggagcatgaaattaaaaatcatatttaccaaagatacgctgcccttccatactactggatcatttcaagtaactggatataactctgtataccctctttgatttcatgcaggtgaatatattcatctgcggtgtgtgaacgggcggaatcgccgggacccattttcacagaggtagccgggatcagcgcctggtcagaggtagtaggcgatccatagcaggttttgcccacgcttatgcctgcctgtacaaacggatgatccattggaataaaggaaggccgcattctcatggaccgtggctttacttcgcaggatacattggcccggatgatttccagcagctcctcgagtgtatattgatcgttggcccgtacatccactacaaaggagcagtcggccggtactacgttatgtgctttattggaagtgttgatcactgtagcgctcatcttcaccgggcccagtgtttccgatactttcgggaaccggaaatctttgaaccagttaagatcagacaatgctttatacagtgcattctcaccttcttcccttgcagcgtgtcctgctttgccatagctggtacaatccagtaccatcaggcctttttccgcgatggccagttgtgttaaagtaggttctcccacaatagcaaactcgatagcgggcagttttggcaggatactttctatcccgttggggccgctgatttcttcttctgcggtagccgtgaggatgatgttatagcccaggtcactacgatgataaaaatgcaggaacgttgcgatcaggctcaccaggcaaccgccggcatcattactaccgagtccgtagagctttccgtcttccacatccggactaaaaggatcgcgggtatattgcggattgggttttacggtatcatgatgggaattcaggagtatattacgtttggagggatcgtaatgtttgttgagggcccagatattattgagatgccgctcatgcggaatatccattgccgtcaggaattcactgatcagttgcgcggtaccgtcttcttcgcggcttaatgaaggggtggcgatcatctgtttgagcagggccaccgccacatcatatagtttttcgttccacataggttagcatattagagtgcctgccactttcggggttgtattgctcagaacatcgtctgcatgccctatcagcacttcttttacaccattgtcaattgccccgaaagcgttttgcagtttaggcaatatcccttctgtcagtattttttcttccagcagttgctggtaaatttctttgttgataagatttataacggattcatcatctgcaggatcacgcaatacgcctttcttttcaaagcagtagatcagccgcacgctgtagtgctgcgataaagcaatggccagggaagaagcgatggtatctgcattggtattcaggatctggcctttaccatcgtgcgtaagcggggcaaacaccggtgtgatgcctgtatccagtaatgctttcagcggaccggtgtgcaagatatccgtgcgtacatctcctacaaatccgtagtcgatttcctttacgggtctttttacagcggggatgatgttggcgtctgcaccggttaaaccgatggcattgcagccattagcctgcagtttggctaccagctgtttgtttactaaaccgccgtataccattgtcaccacgtcgatggtgtctgcatctgtgatccgcctgccgtctacatacttcgattcgatacccagcttatcaccgatacgggtagcgattttgccgccgccgtgtatcaggattttcttaccgggaattgctgcaaacttctccacgaaggtttgcagcaatgccgggttatcgattacgtttccgcctactttgataatgaataagtcgatcataattatcctttgagtatttcactcaaaactgcctgggcagcccatacccggttaccggcttcccggataacgatggattggggaccgtccagtacttcatctgcaatcactacattccttcttaccgggagacagtgcattaccttggcagcattggtgagcttgagtttttcgttggtaaacatccaggaagggtctgtgcaggtgatcttaccatagtctttgtaagaagaccagtttttcacatatacaaaatccgcgtcctgcagggctttatcctgatcgtattcaatttgtgcgttaccggaaaatttttcgtccagttcgtagccttccggatgggtgattacaaaatcggcttctccccatgcgttcatccattgtgcaaaagagttgggaacagcctgtggcagcgcttttacgtgaggcgcccaggtcattaccactttaggcttacgggtttgctgccagttttccttaatggtaatgacgtctgttaaactctgcaaagggtgcagggtagcgctttctagacttactaccggcacgccggcatacttaatgaactggttaatatatttctcggtataatcttcttctttattcttcaaccccggaaaagtacggatggccagtatgtcgaagtactgccccattactgccgccgcttccttcacgtgttcggtggtgttgccgttcatcaccacaccgtcattcatttccagcgcccatccttccttgtcgatattaaacacaattgcttccatacccaggttctttgcagcgatctgtgtacttaaacgtgttcgcaaactgggattcaggaatatcattcccactgttttgttcttacctaattccttatccctgaaaggatctttcttgtagttcagcgcaatgtccactaaccgcgggacactgggaacatctgctgtagaaataaattgtttcatttcgcttataggctttaaacaggcagtggaaagatgttaaaggcacactgcctgccgtacatggttgtttacttatttgtttaatgcttttccgaatgcttccaggaactgatctgcatgggcttgtgtaagcgccagggaaggcagcaaacggatcacgtttggcttggcttcaccggtgaagatcttatgggtatgcagcagttcttttttcacatgtgataattcttccgggagatctataccgatcatcaaaccacggcctctgacttcttttaccttatcaaaggtgcgtagctgttccatgagatagttacctactgttgctgcgttctctatcagtttttcagcctggatggtttccagtactgccagcgctgctgcgcaggccaggtgattaccaccgaaagtagtgcccagcataccatacaccgcctgaaatttaggtgcaatgatgatggcgccgatcggaaaaccatttcccattcctttcgccatgctgtagatatctgcgtttacgcctgcaaaatcgtgcgaataaaacttaccgctgcggccatatccacactgaacggagtctgcaatgaacaccgcgttgtgcgcatcacacaggctcctgatcttccgcaggaacgattcgctggctacgttgataccacctacgccctggataccttcaatgataacagatgacacttcatactgctggaaagcctgatccagtgcggcttcatcttcccagggtaaaaacactacgttctctgtttcatttaccggcgcaacaatcttcggattgtcggtagctgctactgccagggatgttctgccatgaaaagctttcttaaaagcgatgattttctttttgccgttgtaaaaagaagccagcttcagggcattttcattggcttctgctccggagttgcacaggaacagctgatagtcttccttaccggacaccttgcccagcaaggcggccagctcttcctgtaaaggcatctttacagaattggaatagaagcctactttatgcagctgatctgtaaggcgttttacataatgtggatgcgtgtgaccaatagagatcacggcatgcccgccatacaggtcgagatattgtgtgcccttgtcatcccaaacatgggagcccagggctttttctataatgatatcgttaacgggatatacgtcgaaaagtttcatgtcggcaataaattgaaaatgataaaaacacttagaacacgatggacttcagtttcagtccggcggtttcatccaatccgcacatcaggttcatgttttgcactgcctgaccagaggcgcctttcagcaggttatcttcaatggaatggatcaccagtttgttgccggttttttccagttgaatcaaacacttgttggtatttaccacctgcttcagatcgatctgtttatcgcttacatgtgtaaacggatgaccggtgtagaagtccttgtacagcttcacagcgtcttccagcgataagtcggtttgcaggtacgaggttacccagatccctcttggataatcgccgcgtaccggcacaaagttcacctcaccattgaagcctggctgcaacagctgcaggcttcgtcgtatttctttcaggtgctgatgattcagcactttataggtagatatattattggctctccaggtaaagtgggaggtcgactgtaagctttgccccgctccggtagaaccggtgataccggtggtatgcacttctgtgagcaaacctgcttttgccagtggtaacaggcccagctggataccggtagcaaagcagccgggattggcaatgttctttgctgtttttatgagatcgcgctgcatttccggcaggccgtatacaaaagtgcggtccttcacggtttcgcctaaacgaaaatcctggctcaggtcaatcacttttacatgggcagccacatcggttgcttcgaggaattttttagattcgccatggcccaggcaaaggaacatcacatcgatatcattgctgagatcgccggtaaacagttgttctgtttcacccagcagatctgcatgtactgcatacaaaggattgcctgcattactacggctatgtacaaacgaaatggtaacatccgggtgattcaataaaagccggatcatttcaccgcctgtataacctgccccgcctacaattcctgctcttatctttttatcatttgccattgcctgctgatttagatagaatttttaacctgatgccagatcattgtctggttaccaaaaattttgctgaatcctcttacatcatctccgctccagccggtgttcatttcaccgtatttaccaaacttgctgctcatcagatcgtaaggcgagctgataccggtaacctggaaacggtaaggcatcagggtaacaaatacttcgccggaaacattttcctgggtgttttgcaggaaggcttcgatgtcacgcatcacggggtccatgatctgaccttcgtgcatgtagttaccgtagaactgcgccagttgatctttccagctcagctgccattttgttaacacgtgtttttccagtgcgtggtgcgctttgatgatcaccattggtgcagcagcctcaaaccctacacgtcctttgataccgatgatggtatcgcctacgtgaatatcgcggccaatggcaaaaggaccggcgatggtttgtaaatattgaatcgcttcagatggatgaccaaaagttttatcgttcacacctgtaagctcacctttttcaaaagttaatttcacgggttcttcaccctgctttgtgagctgggtaggccatgccgcttccggcagcataccgttggaggtcagtgtttccttaccgcccactgaagttccccacatacctttgttgatagagtacatggctttttcaaagttcacttctactcctttggatttgaggtaggagatctcttcttcacggctcagtttcaggtcacggatgggggtaatgatttccacgccggggatcatgatatggaacaccatatcaaaacgtacctggtcgttaccggcgccggtgctgccgtgcgctaccgcatcggcacctacttccttcacatattccgcgatggctaatgcctggctcatgcgctccgcacttacgctcagcgggtaagtattatttttcagtacattaccgaagatgaggtatttgatcacaccatcataataagaacgtattgcattaacagttttatgacttttaacgcccaggctgtaagcgcgcttttctatttcctgcagttcttcttcagagaaaccgccagtgtttacgatcactgaatgcacttcatatcctttttcttcggtcagatatttaacgcaataggaagtatcaagtcctccgctaaatcccagtactacttttttcattatgacatctttttttataaatccagataacaatattgacgaccctgtagtcagaacaggaaaaatttctttttagatccggtggcgccaccttcttttttacttttcagcaaaacaaatcttttaaaacgtaaccatcgctcgtagagctttatgtttcctttaaatctgcggcggcgtctggcgtggtgtatgtgaccgctggcgcttacggagaattgtggctctggttgtggtgcagcagcagtggctttttcggacattgctttctcttctgcttccttcagtttttccagcgggttgtacagcatggcggtacacaggcagtttttcctgtcttttgccgtaaggatatcgaagtttacgcagcttctgcagcctttccagaactcttcgtcgtcggtgagttcggaataggttaccggctcgtatccgagttcggagttgattttcattactgccagcccggtggttaagccgaagatcttggcatctgggtatttctctctcgacagctcgaatattctctttttaattgatttagccacaccgtggcctctgaaggcgggattaacgatcagacctgaatttgccacaaatttctcatgaccccaggcttctatatagcagaagcctacccattcgtctttgtcggtaacagcaattaccgctttgccttccttcattttcagttctacatagtcaggagaacgcttggcaatgcctgttcctcttgcttttgcagacgactccatctcgtttgtgatggtatttgaatagtgaacgtcgtcaggagtggctaccctaacgatgatatgttgattttccaactttttaaattgaaatcgtgaatcaataaactaacttgaaattccattgctggaaaggttcaccggaggattggggaatcgcggtgcgatagcggtcatattcagacaagcgctatcaaattctaggtcgtcgggaaagaaatctaaagacattgaacccaacagaatataccccctcgatgaaagcgggatgatatgcagaaatgttggtatgagttgcggttttttccaacttcagttcagcgttaaattgttataaatattgtctttagttttagattatccgcaaagttataacaatatccttttaaatagtcgaattttttttgggtagagaagaattttaacaaacgcggaggttgtctttctcaggattacgctgattatactgattataaggattgatcacttggatttttaaaggatttggggagatataagcggaggttgtctttttcgggattacgctgattatactgattataaggatgatcacttggatttttaaaggatttggggagatataagcggaggttgtctttcccgggattacgctgattacgctgattatgctgattatgctgattttaataagaaaatatattaattataataatgtatatagagagataaaaatggaatatccaattctatctccccaaatcctttaaaaatccaagtgatcaatccttataatcagtataatcagcgtaatcctgagaaagacaaaatccgcgtcggtgttaccgcgtgattacgcccaactcggcaattgcggcctgcgcctgcttttcgtctgcgggcgaagtggccacaaagcggatatagcgggcggtagtctttttgaaagccactgtttgctgtaccgggttgtttttgatattggcaaactgaccactggctaccgggctgccccagtttttgccatcggtgctggtgtaaaatccgtaaccataaataataccttcgccggtgggcggagtgtaggtaaatcctttcagggagagggtttcgcccagatccacctgcaactcatgcgggtatcctttattgcctgccacataaatagtagcggtattgccgtctattgctttagcagggtcattatctttggtggccgcttccggggaaattactttccatttggcagaagcgatatcaaaggtagcggtaacggtttcgctggcagttttgccgttgtcgaggaacgctttggcgtgtaccacaccgcccaggggcaggttgataaccgtactttctgcagatatatacttcggcgacttcacggtaggttcgctgccatccagggtatagtgaatatcggtatcgccggattcgctgtgtatccatacttttccgtcggcggtacgtcctatctgtggcagagtgagcaatcccggcgccttatagagctgcacttcgctgatcaccggcgccgccttggcatccatgatattgatacgcacctgggtggtggtgtaatctttcaaacgcaatatacgtttgtggccgatggtggtttcattggcaatttgcttccaggcgccctgttccagcacttccacgttgaaggctttcacacgctgccccagtgcaatatattcctgcagcaccagcctgttgaacgtaaccggctgtttatacgtaagcgtaatagtggtagcagtggcatcgtcggtggtggcccagtaggtgttgttggtaccatcattcaggtgcgacactttcaccgctttattattgctgcgtgtatgagtagccgttactacggcctgctttgccaggttggttttaaaagatacatccagtacacggcgcagttccatcaggcgggtggagtcgttggggtggataagaccatcgcggtcaaccggcacattgaggatcaggttaccgttgcggcccacggagccgtaataaatatcgagcagggaggacacggacttcaccttatcgtttgtttccgggctgtaaaaccatcccggccggatggatacatcgcattctgcgggaatccattgttcgccatcctcattaccttcattgagtgatttggtggccgggccgttggcgcccggtgcaaaaccttttacattcagcgtgctccagttggtggtgccggcaataccattctcattacctacccagcggcaacccgggcctacatcactgaagatgacagcattgggttgattcttatataccacgctgtggaacaggttccagtcgtacggctgtttgatattaccgccattggcgccatcgaaccactgctcaaacacagggccgtagctggaaagcacttcattgagcgtattggcgaacacctggttataaccgggcttgccatattcaggatggttgcggtcccacggagagaggtacacgccaaacttcagaccgtactctttacaggcggcagacaattctgccagcacatctcctttaccatctttccatgcgctttcgcggacagtgtgggtgctgtacttgctgggccagaggcagaagccatcatggtgtttggcggtgatcacaattcccttcataccggccgctttggcggtgcgtgcccactgacgggcatccaggtgggtaggattgaatactttaggatcttcatctccatgtccccattctttgttggtgaaagtgtttggaccaaaatgaatgaacatgtaatattccatgtcattccaggacacctgcgctttggaaggcagggcgccatagggcttgatttcctgggccattgccatattaaagcctagcagccccgcgaggagtaacgtgtttttcttcattgccggaaataaaagttacagattacgatgtgagcgaagatatagcagataatcagaatcattcaatctcaaattccctattattaattcaattttagcttaaaccggcctttgacacgaggctgatacgcctttgatacgcctttgaggtggacttgatccgctttcgcccgtctgtagcgcgaaataagccacaattcttcgccgtttatcacaaaaatgtaagattattccctattgggttggtttagataaatcaatttttataaatttagtccctcctaagacgtataatgtatacgctgataaactttgaacaatgaataaaaatccactgcatcgcagaagttttctgaaaaacacggtagcagctggcgtaggactttctatgctcggctcttctgccaaattatttgccaacgaaaagaaaccaaaagttagaattggtctgattggtgttggcgcccgcggactcggtcatctgaatttctgtctccatcgcgaagatgcggaagtagttgctttcgcagatcctgacaccgcctacaccctcccgaaggtacgtgccatgatcgaaaaggtatacggcggcaaaagaaaagtagctgaatacacgaatggtccggaagatttccgcaacatgctgaaacgcgacgacatcgacgcagtgattattgctactccctgggaatggcattctatcatggcggtggcctgtatgaaagcaggaaaaacaccggcggtggaagtttgcggcgcatcagatatccaggaatgctgggagctggtaaacaccagtgaagaaaccggcatccccgtatttggtatggagaacgtatgttaccgcagggatgtgatggcggtactgaatatggtacgccagggtttatttggtgagcttatccacttacagggtggctaccagcatgatctgcgtggcgttaagtttaacaacggcaagcagtattacggcggtggtgtggaattcggagaaaaggcgctgtcggaagccaagtggagaactaaccactctgtgcatcgcaacggtgacctgtacccttcccatggcctcggtcctatcaacaactatatcaatattaaccgtggtaaccgtttattgtcgctgacatccgtggctaccaaatcccgcggtctgcataaatacattgtagacaatggcggtgaaaaccatccaaatgcaaaagtagaattcaaactgggcgatatcgtgtctaccctgatcaaaaccaacaatggtgaaacgatcatgttgtcgcacgacaccaactccccgcgtccttactcactgaacttccgtgttcagggtaccaatggcctgtggatggatgaccaggaatctatttacgtggaaaagaaaagtaagtacgacgagtgggaaaagaccggcgactttaaagacgccaacagctactttggaaaatacgaccacccattgtggaaaaagtatgctaacgatgccgcaggcgcaggtcatggtggtatggactggtttgtactcaactctttcctggagtgtatcaaacgtggcgcaccttacccgctggatgtatacgacatggctacctggtacgctatcactccactgagtgagcaatccgtggcagaaagcggcagtgtacagttcattccggacttcacccgtggccgctggatgaacagaacgccgatcttcgcactggacgaccagtactaagcggagggagcgccttcggcgctgcggattttgtcttggctcaggattacgctgattttactgattagctggatttttacttttggatttttttagattttttagattttttaataataattaagggagataaaagcgaatatatccgcttctatctcccttaatcctttataaatcaaaaagtaaaaatccagctaatcagtaaaatcagcgtaatcctgagccaagacaaaatccgcagcgccggaggcgcctagtcaataatagaaaccccttcctctataatagttacatatacttccggctccttgccatattgatcctggtaccgggatttgatgaaggagacgtattcatctacctgatcggattttacgaggttgatggtgcagccaccaaaacctccgcccattacgcgggcgccggccacttcttttctttccctggcaagagatacgaggaagtccagttccgggcaacttacttcatagagtttgctcagtccttcgtgggtggcatacatcaattctccaaactgttgcaggtcgcctttcctgagcagtgcggtagcatcctgtacgcgttgtatttcagcgatcacgtaattacagcggtcgtatactttggaagaaagctgtgcgcgtacttcgttgagcatattcatatctgcatcgcgcagggatttcacgacggggtgatttgcctggatggcctttaccccttcctcacactgctgcctacgtacattatattccgaggaggcgagtgagtggtgtaccatggaattgcacagcactattttgtaatcggggaagctgaaagggaaatattcaaattccaggctgcggcagtcgaggcgcattacctggtcttttttaccatgcaagtttgcaaactggtccatgatgccgcattttacgccggggaaagtatgttccgctttctgaccgatgagggccatttgcatgcgatccaatccgtatgcgaagatgtggtccagtgcggctacgaggccaccttccactgccgcggaggacgacatgcctgcgcctacgggaatatcgccggccagtacacaatcgaaaccctgtactggtagtccgcgttcctgcagctgatacactactcccatgagatagttgatccatccgggggttggcttcacctcgtccaggctgaacgacacggtttcgttggtaaaaacggcgtgtacattacattgctgagtattgttgagcgcgatggcatatacaatttttttatcgatagctgcgggtaaaacaaaaccatcattataatctgtatgttcaccgatcaggttgattcgtccgggggaaacgaccatcagtggctctttttcaaataagtggataaactgctccctggtttcttgtatcattaaaagattattaaacgtaaaatttacacctaaaaatataaaaatgattgagaataaaaaaaggttgttccgattttcggaacaacctttcaaaaaatatcaggagtagttaattcttgcctactttatcgcctaccagggcataaaacaggatgtacaggtagcagggcaccatgcagtacaggaatgcgtgtctgaaatcgatgctgctgctgtaaaggaagctgaacatgctgtgctggtcgaacataccgctgtagatctgcgggattacgccaccaccggcgatacccattaccagtaaggcggagcctattttggtaaagcgtccgagtccgtcgatcgccattgggaaaatggccggccacatgagtgcgtttgccagtccgagtaaagcgatgaatgttaccgcagagaagccggtagcgaaataggcggctatggtaaacagtacgcccagtatagcagagatctgcaatccttttttacccgaaaggtatttcgggatggtggcgatacctattacataacctgccagcatggctacgagggtgaaggtggtgaagtacttggtatcgtctacgctcatgccgagggcttttccgtactgaccgattacgtcgccggccattacttccacgcctacataaacaaagatgcagagtacgcccagcaacagctgagggaactggaatacgcttgttttaccggtggtagctgcggcggtggcagcatcttccgaattggtatctatttccggtaaagaagaacgtttcaggagaaacgccagtatagttaatatgatagcgatagctacatagggtccgattacgcgggaagccaggctatcgagtaaagcatttttctgaactgcatctaccgcagcggcgatatctttttccagcttgtcggctcctttcagtacaatagagctgaggatcagtggtgccagggcgcctgcacttttgttacagataccgaggatactgatacgtttggctgcactttcctttggtccgatgatgctggcgtaagggttggaagcggtttgcagcaatgataatcccgcgccctggatgaacaggccggtgaggaacatggcaaagctgcgtgcgttggcggcaggaataaataccagggagccgatggctatgatgaggagtcctaaggccatcccattcttgaaacctgttttgttcaggataaaggaagaaggaatagagaggaagaagtaggccatataaaaggccatggttaccagcagcgcctgggaaacgttcagttcacatacgatctggaaaaactggatcagtgttccattgagccaggtaacaaacccgaatacgaaaaacaatatgccgatgatggccattgattgcgcatacccggcctgtttggaagggactttcattgttactgtttggttggacataagctgtcagaattatttttttttgataaacacgaacataattaaacttctcttatatttcttgtatatttcgcaattatttttgctaaaacgttttacccaatcactaaattgcaagaatattttgactttttaaaaaattttaaaaaaataattatacatttaaccggcaaaatttcaccgtaacttaacacgtttatgactgagcaatcaaaacaaaacgcacaaagcacccatccttcgttctttgtgcttattctggttttctttttctggggatttctggctgcctccaacagtatctttatcccattttgcaaatctcactttaaccttacccagctggagtcgcagctgatcgacttctctttttacagtgcctattttataggttcactgatcctgtacctggcttccactgctagaaaagtggatatcctcaacaagatcgggtacaagaagggtattatttacggattgctgatttcggtgcttggctcggtgattatgattccatgtgtgaataaggaaaagattgttcctattaaagaaaccattgctgacatcagcggtttccaggtagagcagcagttacagacttccgacaggcaggtgaagatccgccgtgagaaagaccctgacacttattcgctcctgatcagcagcaatgaatccgctgaaaagtacaccacgaatccacagttaatttctgcagtttccggtggttttacaaaagatgaggagcataaacaatatgctgccagcttcacaaaagccaacctggaaaagatagttacggtactggatacagattataaacaaacggttacattcggatattttgcccttatcctcatggctttatttatagtggccttaggattttcactgcagcaaactgctgccaatccatttgctattttactgggagatcctgccaaaggtacacaccgcctgaatctcgcgggaggtatcaactccttcggtactaccatcggacccatcatcgtgagcatgttgctgtttggtaatattaagggcggcgaagtaagtacggatatcagcaagatcaatactttatatttcctgctcattgcgttgttcctgattgcagctgctatttttgcttttgtgaagatgccggaaagccaggatacagaaggttttgaatcttctcccaaggctactaagtcattactggctatcacctttatgttcatcctgatcctcatggggctggtgctgaaatttgaattgcctatgttcattgccggtattgtgggtattatcggtatcctcttctataccaagatggcatctgccaacaatagtgaaggctggggtgccatgaaatatccgcagctgatcctgggcatgctggccatctttatatatgtgggtgtggaagtatccattgccagtaatctcggcgcattactgaagcatcctggtttcctgactgtaaaaggtttggcagaatcagaactggatccttatgtatcgctgttctggggaagtatgatgattggccgctggaccggtgctatcagcgtatttaatgtatctaaaaccacccgtaatattctctgtgtaattgttccttttgtggcttatggtgttattctcggcgccaacagcatcaagggcaatgatatcagtgttttatatccatatgtcatctgtatagtggtacagatcattggcttcttcgccggccaggacaaacctgccaaaaccctcaccatctttggtttgctgggtgttggttctgttctgatcgggctatttaccaccggtcagctggctacatttgcatttatcagcggcggattattctgctctgtgatgtggccaagcattttcgcattatctatcgcaggcctgggtaaatataccggtcagggttctgcgttcctggtaatgatgatcctcggtggctcgctcattcctcctgtacagggcggtctggcagacattgcaagcattggtatccacgcctcttatgttattccggcgctgtgctttgcttatctcgcgttcttcgcatttagagttaaaaccattttaaaatctcaaggaattgattatgagtcagcagttagcggtgggcattgatatcgggggtactaacaccaaatttggtattgtagaccgcaggggtaatattatatgtgatggtcggatgttaaccaatcagcacgaagatgtaaccggcttcctggatgaattgcacgaacacctgtccgcgcttattgaacaagcgggaggcatcgaaaacatgaaaggtatcggggtaggcgctcctaatggcaactactacaccggcaatatagaatatgcgcccaacctgcgctggaaaggcgtagtaccgctggccagtttgctggagcagaaattcggtttgcctaccgtactcaccaacgacgccaatgcggcagctttgggagaactgatttatggtgctgccaggggtatgaaagactttatcgtgatcaccctgggtacaggtgtaggaagcggtattgtagccaacgggcagctgatttatggccatgatggttttgccggagagctgggtcactgtatcgtgatccctggcggcaggctgcatgccggtaccggagcacatggttcgctggaagcgtatgcttctgccaccggcgttaccaataccgccatagaattcctggctaaccgcccggatacgcccagcattatgcgggagcataccaacgaagaaatcaattccaagctcatctacgaagcagccatggaaggcgatccgcttgccagggaagtatatgagttcaccggcaaaatactcggtgaagccctcgccaatttcgtgatgttctccagcccggaagcgattgtgctgttcggcggcttaaccaaagccggagacctcatcatgaaaccggtacgggaacatatggagaagaacctgcttcctattttccagaataaggttaaattgctgttctctgaactgaaagaaagcgatgcagccattctgggcgccagtgcactggcatgggaaatgaaagactagctttcagcggaagcagaaaagtataaaatgctttatatgagtaatagaagatcattcctgaaaacagcggccctcagcgccgctgttttctctttggacggagtaacgggaacgcctgcacgttcacagggaaaacgcggactggtaaaaggaaagccgattgtggtatctacgtgggactttggccgtgcagccaatgctgctgcgtgggaggtactgaagaaaggcggccgcgcactggatgctgtggaagcaggcgtaaagatcccggaagcagatcccaacaaccacaccgttggtttctccggttaccccgaccgcgatggccgtgttacgctcgatgcctgtatcatggatgaacatggcaactgcggctctgtaggcgcactggaacatgtaacccacgctatttctgtagcccgcctggtgatggaaaaaacgccacatgtgatgctggtaggcgatggcgccttacagtttgcactggccaatggcttccagaaggagaacctgctgacgcctgaatcagaaaaagcatggaaagagtggttgaaaacatcggaatataagcctgtcatcaacatagaaaacaaatcgtatacgcccaccaacggcgccaccgcgtttaatccgctgatgctgccggggaatgtatacaaccacgatacaataggcatggtggcaatggacgccgacggtaacctgtccggcgcctgcactaccagtggcatggcctttaagctgcatggccgcctgggcgattctcccatcatcggcgcaggattgtatgtagacaatgaaattggcgctgctaccagcactggtgttggcgaagaagtgatcaaaatagtaggcagccacctggtggtggaactgatgcgtcagggatatccgccggaaaaagcctgtaaagaagcggtagaccgtattgtgaaaagaagtccttccaaagcaaaagaaatccaggttggtttcctggccctcaataaaaaaggagagcatggcgcttattgcctccagaaaggctttagctatgcggtgtgcaccagtgataccagcaatgtgctaattgacgggaaacatcatttttagcagacagggatcagccgttgtggctgatccctgtactgatacctcattctcaaaagctattttttatgtctttcaccctcgaaatatgtgcaggatcagtagcatcctgcattgcagcggaagaaggcggcgcaaaccggatagaactgtgtgacaacctgctggaaggcggtactacgcccagctatggtgccattgcgctggccagagaaaaagtaaaaatagacctctaccctattatccgcccgcgtggtggtgatttcctttactccgacctggagtttgaagtaatgaaacgtgatattgagcttagcaagcaactgggctgcaatggtgtggtaattggtatcctcctgcctgatggccgggtagataaacaacgatgcaaaatacttgttgacctggcatggccgatgggtgttacttttcaccgcgcctttgacatgacagacaacccgtttgaagccctggaagatatcatttccatcggttgtgaacggatccttacttccggtgcgcgcaatactgcgctggaaggcgcgtccctattgaaagagctggtggaaagggcgaacgaccgcatcgctattatggccggttccggtgttcgtgccagcaatattgcccagctgattaccgctacgggtgttacggaatatcatacttccgcaaaagcctatgaagaaagcgggatgatctatcgcaatcccaatgtgagcatgggcggcattcccggcgttcctgagtatggcatctctgccacacagaaaaaagaagtaacattaatacgtgaaataggagagaaaacattactatcttagtcgctctgtttagctaaagatttattgaaaacccattattaattgcaggctgacgtgtgtcagcctaaaagtgaacaacgaaaatgaaaaaactgatcattgcaacaggtttgttgcttggcggattcttcgcgcaggcacagatcaaaggggtaaagcatgttatcctgataggcatggatggcttcggcgcttactgttttccgaaagtggacaaccccaacatgaaacaaatgatgcaggacggtgcgtggaccttacaggcccgcagtgtattgccttcctcaagtgcggttaactgggcctctatggtgatgggcgccggtcctgaagtacacggttatacagaatgggacagccggaaaccggaattgccttcccgcgagctggatcagtatggtatgtttccatctatatacacgattttacgtgaacaaaaaccaaaggcagagataggcgttatttacagctgggagggtatcggttatttgtttccaaaagcagcggtcaacaaagagcttggcacacacgacaacgacagcctcgctactgcggcggctgtagcatatatcaaagaaaagaaaccggacttcctgttcatccattttgatgaacccgatggaaccgggcataatattggtcataatatacagccttacttcgaccaggtagcaaagaatgatgtgttgctgggaaaaattctgcaggcagtgaaagatgcagggatgtgggataataccatcatcctgctgacggccgatcatggcggcatcaagaaaggacatggcggcaaaacgatggaagaaatgcagattccctggatcatccgtggccctggcgtggcaaaaaataaagagatcaaaagcagtgtggtgacctacgataccgctgctactcttgcctggatctttgggttgaaaacaccgcaggtgtggaccggaaggccagtgacggaagcgttcaaatgatattgatatgaaaaaaatgctgcttttaacggtggtatgttttgcaggttgcaccctttttgcgcaaacacaaaaagtaaaggtgcttacctacaacattcatcacggggaaaacatgaaacaggtactggatcttcagggaattgccaatgtaatactggccactaatcccgatctggtggcgttgcaggaagtagacagtgttaccggccgtaccagccagagcgatcagctgaaagaactggcttccatcaccggcatgtacacttattttgccaaatcaatggattttgatggcggcggttacggcaccggcattctatcccgtttccctatcagcagtaatactaccatggtgttaccttctgcaaaaggcaatgagcccagggccgccggtattgttaccgttcagctgccgggagatagttcactgcagtttgtgaccactcacctggatgcaggcagaaaggctaccgaccgtattgcccaggcaaatgcactggcagactatttcagggccacggctactccggtgattattgccggcgatttcaacgccctgccggcctcaaaggaactaaaagtactgaaacaggtatttacggatgccagcagcctgatgggaccaacctttcctgccgattcaccgaccataaaactggactatatcatgattgctcccaaacaacggtggacgatcaccggcgcacgtgtcattgaagaaacagtagcatctgatcatcgcccggtgttgtgcgaacttgaaatgaaataagagaaaaaacaatccattatatgacaatgaaaagagtaattcacctgtgcttactgatggcagcagcaggactgtggagttgtaccactcagcagccctccgcacccaaaggcagtgtgagcatcattcctatgcctgccagtgtcagcgaaacagctgattcttttttactggacaagcaaacggtgattgttgccaataatgaaagcgacaaaaaaacagccgctttatttaatgcctggctcaaagaactgaccgggtatgaactggcggtaaaagaccagggagataaaaatgcaatcctgttacagaccggcaatgacagtgctaacgcagaaggctatacgcttgctgcgactcacaacaacatcaccattaaaggtaacagcagcgccggcactttttatggcgtacagacgctgatccagttactgccggtagaaaaagcgcgcgccatgtttgtaccgggtgtgaatattaccgatgcgccgcgtttcgcttaccgcgggctgcacctggatgttggccgccattttttttctgttgattttattaagaagtacatcgacctgatggcgatgcacaaattgaatacgtttcactggcacctgacagaagaccagggctggcgtattgaaataaagaaatatccgcgcctgcaggaagtggcttccaaaagaaaagaaaccatggccggccgttatgccgacaataaatacgatggcaagccttatggcggctattatacacaggagcaggtgaaagaagtagtgcagtatgctaccgatcatttcatcacggtgattcctgaaattgaaatgccgggtcattcgctggcagcgcttactgcatatcccaacctgggctgcaccggcggcccgtatgaagtaggcacccgatggggcgtgtacgacgatgtatactgcgccggcaacgacagcgtttatcttttcctgcaggatgtactggatgaagtgatggcgttgttccccagcaagtatatccacatcggcggtgatgaatctcccaaagtacgctgggaaaaatgtcctaaatgccaggcgcgcatgaagcaggaaggtttgaaagatgagcatgcgttgcagagctatttcatccagcggatggagaaatacctgaacagcaaaggccggcagatcatcggctgggatgaaatcctggaaggcggtttggcacccaacgctacggtgatgagctggagaggcattgagggcggcattgcagcagccaaacaaaagcacgatgtgattatgacgccgggcgaattctgctactttgaccactaccagtccaaaggcacgaatgaaccactggcaataggcggattcctgccggtaagccaggtatattcctacgaacccatacctgcagagctgagcagcgaggaggctaaatacattaaaggtgcacaggctaacgtatggacagaatacatcaacaataccaactacctggaatacatggtatacccgcgcgcagctgcattatcagaagtattgtggtcgcccaaggataaacgcaactacgacaacttcgtggaccgtttaaaagtacatgtaaaaaggctcgacctgaaaaaggtaaattatgccaagcatgtttttgaagttaccggtaaagtaaccgataatagcaaaggcggtgtagcagtagtactgaatacaaaactggatggcggtaaaatatttttcaccatcgatagtactgcccctacccctcaggcgactccttatacagcgccggtacagattacccgcaacggcacgctccgtgcgcaggtattcctggatggcaaaccttttggcaacgaatacagccagacgttcctgtttcacaaaggattggctaaaaaggtaagcatggcttccgcagcagatgctgctcaccgtcctgccacgacctttacgctggtaaatggagtggaaggcaatgctgcttataacgacaacgagtggtttggctttaaaggaacggatatggaagcagtagtggagttggacagtgtgcaggatattcacctggtaggcattaatacaatcaatgtaaagggcgactggatctacccaccgaagcaggtagtgttttctgtatctgacgatggtaaaacatttaaagaagaatacaagcaaaacacctttgcgcagcagggcatcaacaagatcaggggccatttgcaggctgttcgcggccgctttgtgaaggtgcagatgcagaactttggtaagatccctgccggtgcagcaggagcaggcaacggcgcatggttgtttgcagatgaacttattatagactaaaatcgaaaaccgtcccggcaaatgcggaacggttttcattttatgactcctacaccaaaatatatgatacggccttcaaccgctgtatgctaaacatattaacgagatcaaatattaattggtttattacaagctaaaagaaatataatttaaatattgctaaataataatgcgcattagcagtaaattctttaattttccggctcgtttttaaaccgcatctaatcaaaaacgtttacaaatgacgattaatcatcaggaaatcgaactgatcgacagctttgaacaaattgctgtggaaattcacccttctgccaaagaaggttccaaagcagtagcacaggaaattgccgcgctgatccgcgaaaggcaggctgccggccaaaaatgtattttaggattggccaccggctctactcctaaatatctgtatgcagaattggtacgtctgcacaaagaagaaggactcagctttaaaaacgtcatcacctttaacctggatgaatattatcctatagagccggatgctttacagagctataaccgctttatgaaagagcacctgttcaatcatgttgatatccctgaaggccagtacaacattccggatggtactattccaaaggaccagatcaagaaatattgtgaggcttacgacaaacgtattgaagaattaggcggtatcgatatccaggtgctgggtattggcaacaacggccacattggttttaacgaaccaggcgccaatattaattcacacacccgtctcgttacactggacaacagcacccgtttggccaatgcgtacgagtttccgaatatgagccaggtgccccgtttggctatcaccatgggtctcagcagcatctttaaggcaaaacgtatcttactgatggcatggggttcccataaatccaaaatcgttcgccgttcggtagaaggacacagtaccgaccaggtgcctgcttccctgctgcaacagcattcaaactgcaagtttgtgatcgacgaacaggcagctgcagagctgacccgtttcaacgaaccgtggcttaccggcgattgcgaatggacgcccggtctgatccgcaaagcagtaaccagcctggcgctgaagctgaacaagcctatcctgatgctcaccgataaggactataacgaaaacggtttgaacgacctgatcgtacagtatggttctgcctatgagctgaatatcgaagaatttaacgccattcgtgataccattaccggctggcctggcggcaagcccggtccgcagttaccgaatcaccccgaacgttcagaacccgctaaaaagcgcgcgctgatcttctctccgcatcccgatgatgacatcatttctatgggcggtactttcatccgcctgcatgagcagggccacgatgtacatgtagcttaccagacttccggcaacatagccgtaacagatgagttcctgctgcgtttcatcgactttgccgtaggttttgaaggcatgttcgatattgataaaagcaaaagctccctgatcctggatgaagcgaaagccttcatccgcaccaagaagccgagccagaaagatactcctgagatccgcgctatcaaaggtttgatccgccgctgcgaagcaaaagctacctgccgttatgtaggtattgcggaagaaaacgcccacttcatgaacctgcctttctatgaaaccggtttggtggaaaagaaacccatgggaccagaagacgtggcgctgaccgtagagttgcttcgtaagctgaagccgcaacagattttctgtgccggtgaccttgccgatccgcatggaacgcataaggtgtgcctggatgtaatctttgccgcactggaaattgtgaaaacagaggactgggcgaaagattgctgggtatggctgtataaaggcgcatggcaggaatgggaagtacatgaaattgaaatggctgttccaatgagtcctgaccaggtaatgcagaagcgtttgggtatcttcattcaccagagtcagaaagatgtggtgcctttccagggaaccgatctccgcgaattctggcagcgtgcggaagaccgtaacgccaacacggccgacctgtacgaccgcctgggcttacagaagtatgccgccatggaagcatttgtacgttatcattttatgtaaataaatcataattttgggggactgtgataaccatcgcagtccctttatttttttatatgaatctgagcagagccatagaaatagccaccaccgcgcataaagaccaggtggataaatacggacagccttatatagggcatgtattccgggtaatgcaaatgggccgtaccgaagatgaaaagatagtgggtgtactgcatgatgtggtagaagacaccgactggacctttgaagccctcgaaaaagaaggactggcccctcacctgctggcggcactttactgtgtgaccaaactggatgaagacgaagactaccaccacttcgtggaccgtaccctccagaaccggttggcctgtatggttaaactcaacgacctgacggataacatggatatcaggcgtatgaccgatgtaaaggaaaaagatattgcccgcctgaacaaatacctgcacgcttaccgccggatagcggccgccgttatccagtagaatattttttcaacgccttccgattaaactattaaattacagtagaaaacagaatagccatcaatggaaaacgatatcctcattgactttaggttcgctgcaaaagagaagcccaggttcggtgaattattcttaattacaggagaagagaatcctaaatttccggccaggaacaaagcattcgcacaattggccccattgggttttgaacaactcgatgatttttttggtatccttaacagcgaagaatcaggcgacgatgtactgatatggcttttccccatgatcaacggggaagaagtatttcataacagcggtccgttcgacgctatccggctatcttacagcgcattacgcaatgctcccgcaactatcactttactgcaggattgcttcaatgccctccaggccttacctgaggtagaagttgaatttgaaggatcgcctattgccgactttagccccgtgcaaaagaaagcagacgagattgtggctcactggcgggaaaaccatatagaacccggttcagaacaaagtttactgattgacgatgatgatgcagacgatgactgggaagaggatgaagactgggaagaagacgacgaatgggaggaagaagctggtgataaaaaataaataacctgatttacgccaacggatcatgaaaaaacaagccaacaaaaaaggtaccaccgcattattgctggtggcctctttaatactggtattgcttatttccggtattccctctgcccgtaaggctgataaaaagaattgcacgccaaccaccggggtggtaaaagaaatcaaagcgggtcctcctggcattattattcacctgaagcagaatcccaggatctattacatctcccgtaaaactaataccagcctatctttaaaaacactggaaaaagaactgacaggtaaaaacatacaactttatactgcgcaggactggtcgccgctggacccgttttccaccatgaaacaggttcaccggctgcagataggcgacaccgttatattcacggaattctaggcctaatctttgtgcagatgccatgcgggtggaagccggagtccttccatccgcataaaacagtaactttcatatgcatctcaataaatatttatcctgcctctcactggcagtattactggtatcgtgcaacctgaataacaaaccaagtaaatacgataacgaagaaaacgccgaaaaaaacaataaaaaaactgctaccaccactgccgccaaaccagcacgcagcaaggctcccattgttggcgaaagaatcaacggcgctgctaccatactgaataatcccggcggagaaccactggttaccctcgtggattatatcccgttacgttgtgcgccggtgaaaaaagattggtaccctgtaagcgtagattttgatattacgaaagaagaatacagcaaacccatttttcacaaaggccgcaaaataaaagtaaacggcgtggatgcaggcgtactgcaacgcgatatcaaactgcccgtagccaccaacggggaaaagatgtgggctaccattgacggctatacgcaaaagaaaagtatccgcagcggcactatcattgaatctgctttaagcagttacctgaagcaacataccggtcgcagtaccgccgatatggagccttttatccacaatttcaaactggaagaagaaaccaccctcaagccttacctactgtatttcaattatgaaagcggtatcgatgatcccagccccttgtatcgcctcgcccttgttttccaggggaaacagctgataggcgtgctgcactcccggcccattcaactggatggcggcactccgcgcaggttgcaacgtggctttacggtgaactacctcagtggcatcgataaaagcctgaaagaagatttcgccgtgaagttcaataagttcattctttctgttgattaatcccataacttttggttatcacctatcacatatagacatttgacttccgcggcagcgatacggacctttgtatccaattacaaacgttcgtgtatgcaacaagagaagacaatagctacctggctgccggagaacacgcagaaaattatattccttaccgcagcagccattaccctgttgcccgtagtaaccccaccggtggcgctgttgctgggatttgcactggcgcaaaccagcgggaaccctttcactgcggtaacgccgcgcatcacgcactggttgttgcagctgtcgattataggaatgggctttggcatgaatgtacacagcgcgctgaaagccggcggtgaaggttttctctttacggttactgccattgcaggtaccctgttaacaggggcggtgctgggtaagctgttgggcatcgataaaaaaaccgctcatcttatttcctgtggcaccgccatctgcggcggcagcgctattgccgccattgccccggtaatgaaagccggtgagaaacagatatctgttgcgctgggaatcatcttcctgctgaatgcactcgctctttttatttttccggcggtaggccacgggttacatttatcccagcaacagtttggcctgtggagcgccatcgccattcatgataccagctccgtgataggcgccgccagcaaatacggcgaagaagcactgcaggtagccaccacggtgaagctgtcgcgcgccctctggattgttcccgtagcatttatgaccaccctgctgtttaaaacaggtgcaggcaacataaagatcccgtggtttattgcggtgttcattgctgccatgctgctgaatacctgggtaccgctattccagcacgcgggccccttcctggtaaaaagcgccaaaacagggttgtcgctcacccttttcctgataggcaccaatctcagccgcgaggcgttgcggggaatcgggcgtaaaccattgattcacggggtagtactatgggtattgatcagtaccggtaccttactggccatctgctgcctggcctgataccggggaaaaccccgtgataacccaattatcatttttacatatatttgatcatcgagcatttgtgatactggcagcatttatcataataaccaagatgactacacgtaatttatgagccggtccccagccacaaaatccggcacttatatggctgcattccgggcaatagaaagtacgaaacctgaaaaagagcgtttgttgtatgatccgtttgccagtgcattcctgtcaaaattctatcagatcttactggcaggttgcaccatcgccttcatccggagaatagtgacagcctgcatccagttccgctggcctggcagcttcaccgcggctgttgccagaacaaggctgattgacgacatgatcctgcatgccgtaagatcgcagggcattaaccaggtgatcatcctcaatgctacttttgataccagggcgcaccgcctcaacgtaggagtaccactgcattacgtggaaatggatcatccatcgctccagtatacaaaaaagaaaatactgtctgacctggtaggactaccaaccattcacgtggattatgtgcagctggatttaaacacgcagcagatctcggaagtattcccggaactcttctacggggcgcattacaaaacattgtttctctgggaaggaatcaccaccaagcaggaagccaaacaagcggaaacgattttccatcatgtgaaaaattttagcccgggtacacagatcatctttacctatgtagaaaaagcagtactggaaaacccctcggcattctatggatttgtgcgtatcaacaagctgctgagccgcgccggtgagaactgggacttcggtatccgcccggaagaattgtatgccttcctggaattacatcacctgaagctgcactatgatggcggcggcggggattaccgcgcgaaatatttcggagaaaagagtaagcagatgaaaggctatgaatatttaagggtagtaagagcagaagtgaaatagcagccgtatcttcggtgcatcattttagcgttctgcatatgcatattcactactttcaacatgtgccttttgaaggattaagctgcatcgccgactgggccaaccgtcatcaacaccaggtaacctatacccgctggtatgaaaacaccgataccagctccgttgcggcagccgactggctcatcatcatgggcggaccgatgggcgtatacgaacaggatcatcatccgtggatgactacagaaatagcccttatccgggatgctatccaacaaaataaaaaagtattgggcatctgcctgggatcacaactgattgctgcggcgcttggtgctaacgtatacccgcacacgcagccggaaatcggctggttcccgctggacctgagctttcagggccaggcggctccactggaaacagtactgccgcatcactttaacacctttcattttcacggcgatacctttgatgtgccggtaggcgcaacccgcttcgcggcgtccgcagcctgcagtcaccaggcattcatttacggcgaccgcgtaattggcctccagtttcatatggaattaacggcagaaagtttgcaggaaatgatcctgtacggcgccggcgccattgcagccggtggaccatttgtgcaaaacgaagaaaaaatccgccagcatatgaacctgctgacacaaaatactgaaaacatgtaccgcctgctggattatatggcagcgctgtaaataaaatatgattgtatgactgctgcgtttgacgtattgattatcggcggaggacctattggtcttgcctgcggactggaagctaaaaaagcggggcttagttacatcatcctcgaaaaaggctgtgtggtgaactccctctacaactacccgctgtacatgacttttttctctacctccgagcggctggaaattggcaacgttccctttgtgtccatcaatccgaagcctacccggccggaagccctggaatattacaggagggtagccacttcacatgaactgaacataaaactgtttgaagaagcggagcaggtaatacctaacgccaacgaatatacggttataaccaaaaagagtagatatcatgcacggcacgtagttattgctaccggcttttacgacattcccaacctgctgaacatacccggcgaagatcttcccaaagtaacacactattataaagatccccacttctacgccacacaggatgtagtagtgataggcgctcataactccgccgtagatgccgccctggaaacttaccgcaaaggcgcccgtgtaaccatggtgatccgccaggaagacattggctcccgcgtaaaatactgggtacggccggatattgaaaaccgcatcaaagagggatctattaaagcatggtttaattcttcacttaccgccatccgggataaggaagtggatatcgcaacgcctgacggccccgttaccattgccaatgattttgtgatcgctatgactggctaccagcctaatttcagcctgctgcaaaaggcaggcattgcgctgtctgatgacaatctcaaactcccaacatacaaccctatcaccatggaaaccaatatgccgcgcatctacctggccggcgtggtttgcggggggatgaatacccacgtgtggttcatcgaaaactcgcgggatcatgcggagaagattatggcgcatgtgcgtgcgaacgcgtagagcggagggcgccttcggcgctggtaaattgtcttggagcaggattacgctgattatactgattggcttgattttgattttgttttgattttacttttttgattttataaaggatgaagggagatataagcgaataggtccgcatgtatctcccttagctattttaaaatctcaaagaaaaaatcaaaataaaatcaaaataaaatcaaaaagtaaaatcaaaaagtaaaatcaaacataatcaaaatcaagccaatcagtataatcagcgtaatcctgctccaagacaatttatgagcgccgaaggcgctcctccgcatcaaacaatgttcacctcgcgctccagttccactccgaacttgtcctttacgctgtccagtacctgttgggacaggtggtaaatatcggcgcctttggcgtggccgtaatttacgagtaccaatgcctggcgggcgtgtacgcctgcatcgccgttacggtatcctttccagccgcattgctcgataagccagccggcggccagtttgaaatggttgtccgctacggggtaggctaccatggcaggaaattcggcgtgcagcttttcgtattccgctttggtgatggttgggtttttaaagaagctgcctgcattacctatttctgcggggttgggcagtttggaagaacggatgtttatcactgcctggctgatggcctggatagacagctcctgcacattcatccgctggagttcctcattgatagcgccatagctggtattgaaatgtggctgcttgcttaaccggtaggtaacagataaaatagcaaactggtttttatattcttttttaaagatgctttcgcgataaccaaaatggcaatcggcattgttgaaggtaacgatgctgtgatccttcaggtggagcgcttccagctcatgaaatacatcttttatttccacgccataagcgccgatattttgcatgggactggcgcctacgttacccggtatcagggaaaggttttccaggccggcgagattttgcgcgatgcagtgctgcacaaacccgtgccagttctctcccgcgcctgctttcacatatacgtagtcgttatcttccccggtaacggtgatacctttgatctcgtttttcagcagccagccattgaagtcctgtgtgaacaggatattgctgccaccacccaggatcatccggggcaggccgtcgctctgcggttgttctgtgaatgacttcagctcttctgctgaggaaaaggacgcgaaataacgtgcagtggcgttgataccaaaagtattatatgatttgagcagaacattttctgatacctgcataataacttaaatttatggtgagcaaagatagccgcaaatcatttagaaatcataaatcgagtttcatgaataaaacggcgattgtaataggtgcaacaggactcacaggcacccacctggtggcggccctgctgcatgacccggccttcagcaaagtaaaggtgctggtccggcagccctgggcccatgaccggccgaaactggaaagcattattgcagactttgaatcggatgagagcctggcggcagcgctgcagggagatgttcttttttgctgtatcggtaccaccatcaaaaaagccggcagccaggaaaatttcagggcggtggattacggtattcctgtaaaatgcgccaggatcgccaaacagcaaggcatcacacaattcctgctgatgtcgtccattggcgccaatccgcactcgcgcaacttttatctgcgtaccaaaggagcaaccgaagatgccattcaacaggtgggtttccacagtgttaatatcttccgtccttcggtactgatcgggcagcggaaagaattcaggttaggcgaatggatcagcagatatcttatccagcttttttattttttattacagggaagatggaaaaaataccggggcattaaagcggcaactgttgccaatgccatgatcatagcagcaaaagagaatgatgaaggtgtgagcatctttgaatcagatgctatccagagcatgggcgagtcatgaaaatccggaatttgagtcttatctttaacccgtatgaaaaaatgggtccttcttctggctgttgcagttattgcaatactgccgctatctatgcaggcgcaggtaaacagctactttcctgaaatatggaaagacaatccacagctgcataccactccagctaccgatgctccttacacgatcgtggattacagaatggtcagggattttaatgttagtccgcgtgataaagcacaagccacttcccactataaaacactctacaaaaatataaaagtcaacacccagcgtgcagccgacagcctcacccgcctggtaatgtcgatggagcccagcgaagctttgcgtggcctgcgcatccgcgtaatacatccgggcggcagcgtgaccagtctcaacgagcaggtacggatgattgaaatggatcgcgagcggaaagcaatagtagccaacaacctcgtactggaagccggctgtgaaattgaatatgagctgagcctgaaagtgcagtacgattatgcaggcaccgattacctgcaatccggtatcccgtgcgaccagcttagctttgtactgatagcgcccaaaactttggattttgtggtgaagcccagcgccggtttgccagcactgaaggacagtattacggataccaaccactactatcagctgaatatgcaaaatatgccggccctgcccagcagcgacctgtatttttacctgccacaactaaagcggattgatttcggattgaagcaggcaatagaaggaaaagatacagtacacatgacgtggcagaagtttggggaagataattatatcccttttgtggcggtatcaaaagcagaatataaacaactggaaaaagaattgcagaaatggcctttcctgaaacaacggattcctgttccgcagatgatctacctggtagaacaatttataaaatccaattaccggctggtagagacttctgaaaccggtgaaacggtggatatcatttccatcatccgtaataagcaggcagaaaaagcaggctttacccgtttgctgaatgcggtgtattatatgctgaatattcccacgcagatattatttactacttcacgcgacagtttgctgatggacagccagctggtataccggcagctgccaaccaatgtactactgtatttcccgggattgcaacaggcgctggccccaacggaaatgaatacacgctttccgtgttacccgtcgttatggaccggcattcctgcgctgcgctgccgtgatacgctggtggcgggggagagcaaggtgctgaccgattttattcaaacgccggcgccgccatacacactcagtaacattaccaccgaggccacgctccggtcagtaacagatcctacctgggaggtgaagcaatcttttggtggttatcccgcatctaatctgaaaacagcttttggcggtaccggcagtacgccggatggcaggctgcaggtatataatgccatccttccttttgaacctagtatcaggaaacccacggaagtgaaagcagaaaacgaagtgtttaataaccgctccctggataaacctgtattgctgaacagtacgttgcttaccacatcttccgtagaaaataaaaacaacagcattgttatccacgtgggtcctttactgggtggtaatatgccggttgacatcccgcttccgccgggcgatctgcctgtgcagatcacatttccctattaccaggaaaaacgcgtgattgtgccggtgccggcgggttataaagtagcgaataagggagatttttcggcagaaataagtgataaaggagccgatcctgcactgggttttaaaatgcggtgtgaacaggacggcaaccagctgcgcatttttgtactggagtggtacaaacaaactgatttctccggaagcagtaaagcggtattcggtcaattgctggaaaggatccatacactccagcagcaggacctgatactggtgaaagaataattttatacgccgtctacatccggtatgatcactaccgaacggaactttttttccgttttcagttgaataataaactcctgtaacacccttttgatatgagtgatcagcctggcttcacgtggcaatttgatcagcatttcctgtaaataattattacgtacccttgctaccagcggagctgctggtcctaccagttgtgcaccgatatgcggctgcagccagctggccaggatctgtgctgcctgttcagctgtttgctggtttttatgccggatagtaagcttcagtaaacggaaaaagggcgggtaaccaaatacctgccgttcagcgatttctgcttcaaacatgcctttatagtcgtgcgccatcacatagtgcaataccgggtgccgggtgttgctggcctggatcaatacttttcccagcccgtttttacggccggcacggccgcttacctgttccatcatctggaaggccctttcattcaccctgaaatcggggaagcccaggaggttgtcggcgctgaggatgcctaccaggttcacgttttcaaagtccagcccttttaccaccatctgcgtgcctacgagtatgtctatactgcgatcctccagcagctggatgagtttattgtggctgtctttgttcctcaccgtatccacgtccatacgggcgatgcgggcttccgggaaggccacctggaggtcgtcttctattttctcggtaccaaagcttttgggttcaatggtttgcgagccgcaggctgcgcaggtatgtacgtatggatacctggtgccgcaatagtggcaatgcagtttatcctggtttttatgataggtgagggaaacatcgcattgtttgcaatgcgggatccatccgcaggtagtacatagcaggaaaggtgcataaccacggcggttctggaacaggatcacctgtttgccatcggctatagtttgtgtgatggctgctttcagggcggaggtaaaatggccgtccattgttttttccgccatttcctttttgatatccactatttctatcgccggcatttccacgccgccgaagcgttctttcagttcaacaagcccatattttccctgttgggcgttaaaatacgattccagggaaggtgtggcggagccgaggagcactttggccttaaagaggccggcataataaatagcggcatcccttgcatggtaacggggagccgggtcctgttgtttataggaggcatcgtgctcttcatcgaggataataaggcccaggtcgcggaaaggcagcaacaggctggaacgggcgcccagtatgatttgcagctcccctgttttcaccttgttccatatttccacgcgttcgttgttattgaaccgggagtgatagataccaatgctggtgccgaaatgcttctgcaggcggcggatgatctgcgcggtgagtcctatttcgggcaacaggtacagcacctgtttgcccgcagccaggcattcttccatcatcttcacgtatacctgtgttttaccactggaggtaacgccgtgaagcagggttacctgtttatctttgaagtgtgtttgtacttctgcgaaggcagcttcctgtgcagggctcaggtcaaaatcgatctgtgtatctaccttaccggtaggaatccggtctaccgtgcgtttttctatccaaaggatatttttatctaccagtccttttaactgggcggtggtggcgccggattttttcagcagttctttctgcagtaccacgccctgtgttttgagcaggtggagataagcgagcagcagttccatttgcttgggtgcgcggcccatatcgttgaacaatgcggccagttgtttttcttcctggtagtccgcatgcagctgcacataattctcctgtttctcgcggtatacttctttcagctcttcatataccagcagtacttttttctctatcagggatttgataacagagtaaacttctgatttatcgagaatcagctgtacttcttcgatgcgcagttccttgcggatgaggagggcttccgcgatgaggtattcatcatcgttgagggaagtgaagtcgtcaccgaaggcatcgttgaagagcaggagtgtttcgctggacagcttgagatgggctggcagggcggcattcagcacttccccttccgtgcacatatagtaagcggccacccatgtccagaaggctaactgtgtgggatacacgataggttctgcatccagcatatccagcagcggcttggttttatacaggggggcctgttcgtgaatggctttcacgataccggcgtacttcttttgtttccctagctgaacggctacccggcttcctaccttgagggtggacatattttcgggaaccgcgtaagtataattttttggtaacgccaatggcaatattacgtctgcgtacttcatcctattggctgcagggttggatatttgtgatacttgcgtaattcggtgtccattgcatcaaacacctgttgtttgagggtgttgatatcatcgagtgtcattcctgttacgggtattggtggcaggaataccacgcggcatttgccgggggagatgtgcataggtcctttatgtggtaagcggtggcctgcatcgaggtagagcaccggtttgattggtttttgcaattcgatggccatacggaatgcaccgttatgaaaggggcgtaatggctgatcggtatcgttggtggtgccttccgggaacacgaggatggagatgcctgctttgagggcggtcatcatttcccgtacgctgcgggccctggcggctgcgctggaacggtccaccggtactactgaatttttatagataaaaccgaagaaaggaattttagacatttctacttttcccagcgggcggaaagggaggcgcattacttttacggcgatggctgcatcaagataagagcggtggtttaccacatagatgcagggttcattgtcgcgttcgcataaatatttgcgggtaacccacatgcctaccagcgggaaccaggtatgtgcccagaagcgcaggaaataaaatatgatgttacctcctttttgccggcccagtaaagaggccaggaaaatggggggcagtatcaggaacatgatgcccaggaaagtagcggcggcgtatatcacataaataacacgcaacggtttcagtaaaaaattcataaacgcctcgaaaggtttaatatggcggaaaactacgaagaaaattactaattacaccgaaccggtggccgatttaatcgcagtggcagacccagtccttatccaggtcgatgcaggtaattactttggcgtgctgtgaatcgcagggcgcaaaaacgatccgcaggtgctggccttcactggaataaccttccagggcatacgttgggcaggggcggtcttccgggttagacttttccgcgttgatcttgccttccgccaggatctcctccacttctgcggttgtcacctgacggcaatccatccgacaaatggcatgtttggtatattcaagatgggcatgcctgttaattacctcattggcgatagcgggactgctggagttattgcgaaccactacagggcggctgcccggggaaggagctgcgggcgcgcttttccaccacttctgctgccagccggcaagcagtaagatggacaacaggaagacgggcaggtatttttgcattgatttcataaaacaatagaacgccgcgcaaaatagtcaaaaattccttacctaactatgacataaaaagttcctacctttgcctccctttatggaacaggtaaaaacagtagcatttcatactctcggctgtaagctgaatttttcagaaacctcctcaataagcaggttgctggaacaggatgggtttgtaaaaacggattttgacggaacagcagatgtgtatgtaatcaacacctgctctgtaacagataatgctgataaagagtgccgtatgctggtgcgccgcatacagcgccgcgcacccggcagcatggtagtaatcaccggctgctatgcccagctgaaacctgaggaaattgcttctattgaaggggtggacctggtactcggcgccgctgaaaagttcaacatcgccgaacacctgaaaacgctcaccaaaggcgacagcgctaaaatctgctcctgcgatattgacgaggtgaatagttttcatgcttcctattctcttaacgaccgtacccgcaccttcctgaaagtacaggatggctgtgattatacctgtgccttttgcaccatcccaatggcgcggggcaaaagccgcagcgacagtgttgccaatgtagtaaaacatgcacacgacctggccgctaccggcgtaaaggaaattgtgctcacgggtgtaaacctgggcgattttggaaaaggctttgaaggcggcaagaaaagggaagaaaccttttttgaactggcacaggagctggataaagtggaaggtatttcccggtatcgcatttcttctatagaacctaacctgctcactaacgagatcattgaatttgtggccaacagccgcaggtttatgcctcattttcatattccactgcaaagcggcagtaatgagatccttggcctgatgcgccgccgttaccgccgtgagttgtatgcagagaaagtagcgctgatcaaacaatttatgccacattgcgccatcggtgtagatgtgatcgtaggcttcccgtctgaaagcgatgcgcatttccgtgaaacgtacgactttctgcatgaactggatgtatcttatctgcacgtatttacctactcagaacgcgccaacactggtgcactggatattaaaccggtagtacctgtgcatatccggaacgaacgcaataaaatgctgcgtaacctcagccacaaaaaacagcaatactttaatgagcaacacctgcatcaaaccaggaaggtgctgtttgaatcgctgggaaaagatggtatgatggaaggttacaccgataattacatcaaagtaacgactcctttccgccaggaatggcacaatcagctgatcgactgggatctgcgctaaccggattttctgcggagtaaaaatccgcggaaatggtcatgccacgaaatcaggttgccgatcaggtaataatctttcaggttatttttaatactgctgcgcataatgcgtacgactatacttttgcccacttctcccttttcctgcaccagcagcagcagttccagtgatatcaacgacaggatggcgctaatgaggaacaggaaattccattgatgcagggccagcaggtgcagcacctttgatttgtgtggccccgtgaatgttgcatcaatctgtatatgtcttgactcaaaaaagtcggccaggataccaccaaccagcggcgccagggcggaaaaaacggcggtaatgatgttcctggcggataagtataccaccgcatcctttaccggggccagtttaagcccgatattggttaacgagagattgatacctgcattggcaataccagtgaaaatatggatgagcaccagcaggattatattggcatacatctccgaataaattccaacaaaacaccacccgattacgcaaaaaatgtataacggaccgctgatggccagaatggttttattgctgtacctgtctgcaaacacgccccacatccggaatgtaaatactcctgtgagctggcttaccatcagcaatatagtgataacagacagggacaaatgcattccctgcatcatgaataccgtaaaaaaaggtgtggcaatattcagggcaaacacccaggctgaattgaaaacgagcagccggagaaaattattgtcgcgcaacgggcgcagcaataatttgaaaaaattttccttgtccatatacgactgtggttccggcgctccggccagtataaaagcccccgctatgccggcaacaccggcagcaataaacatacagtaataggtagtaagttcatatgcggggtaatgcctgcggatataatccacgccaaaagcggctgccaggctcagtactacgtttagtccctgcgtatagctgcttcgtttggcaaaataggtgcccatgatctgttccgggataaggtcttttatccaggcgttccagctggggccggcgatagagccaaagaagtagaaaaagaaaagaaagaagatgaggaaattgatattgcctgtttgcgggaacatcagaggaatagcgcctatcagcaacagcggtatcctggccagcagggaacacagcactgttaccattctccggttgttggtgcgccgcaccagccaaatggatattaattgaaacacgttggtgaaagtgggtaaggcagacaacaatcctatctgcagattattggcgcccatgagcagtgccattgcaatcaggaaggcgccgccggtgagtgtgatcatggcttccgccgccagcccgtcgcctatgatcagcctcatcccaattttcctttcgggttcagtaatgtcggtgcgcggtctcagattcatacttttgtatttcagtataaacagatacacgtgcaccggcaatgattataccatgccaacagcagggatggctatattacttcggaaaaccgggatcagcttttacttcttccagctgttgcgtgtgccggttagtatgcgccgcatccagcaatagtaactggtaagcatctactggtcccagtgccgggtgatccataatatgatcccgcaacgcatcttttgtgttggtgacatattcaatcagtttatcccgctggtctgtaaaagcttttatagtttctgcattagaggaataagtgtgttttggaacaccatattcgggcgcctttactttatggctgcggtcttccacattcttaataatctgttcgtcggtggctttaatatccttttttctttcaggattggcaggttgttgtatgaggtgttgttccccttccataattgctttttcaatcagggtaatatgctccacgcactcaatcactgaccagcgatcggcggcgggcttatattccagctgtgcatcagtaagtccctgcacatctttgaggagctgttcctttgtttgttgcagttgattgagcagaagggacctgtcttccctggcgctggttacaggctggaatgcggtaacagcagaaaagactgcaatagcaaacagcagcgatagctttttcatcgtggattacatttaggagttaaaaagaagataggtaagttacgaaaaaccaatgatctccagaaattcctcgcgggtaataaaacctgcgcccagcgaggccaggtggtcggtatgcacctggcagtcgatcatttccagttcgtgtgcataagtttgcacaaaggtgataaaagctgctttggaggcgttgctcacagtggcaaacatcgactcgccaaaaaagaagggacctgttttaacaccataaagaccgcccaccagttcgtcgttttgccagcactccaccgacatcgcgtagccggcgtggtgcagccggatgtaggcttcctgcatttcgggcgtgatccaggtaccggtttgcccctccctgggaatgctgctgcaccgggcaattacgcctgcaaaatcttcattgaaggtaatccggaactgttttttgcgcagtacctgtttcatgctggcggatatctttaattcatccggaaataatacgaagcggggatcagggctccaccattggataggcggttcatcgtaccacggaaagatcccggaacggtaagcgagcagcaatctttctaccgacagatcaccgcccacggcgagtagtccgtccggctccgaaagctgaacaggggggaaaatcagttgtttgttaagacggaaaacggacatatcaggaatcagctgcctgccatttcttcaatagtaacgcttagtccccgctcctgcagggcttcacacaggggacgcagtttcaggtattctccctgttttacggcatactttccattaaaatgaatgatcagcgcgcactgctctgcctgttcatgcgtgtgaccacatacctccatcagtgaagcaatgacccagtcgaatgtattcacctcgtcattccagactaccaggctgaacggaaactgttcatcttccgccaccagcacatctacctcttcctccggtaatccttttgtacttgtacgatcgctcatctttaataaaagctttatgcaaaattacatggattattcgttaatttatccatatttagcagagatctgttgatttcaggatacttccgaatttaaaaaatggttatgatgaacggactggttttattgatgaatacaaatttaccgctgaaagatccggtgcctatcttttcgctggtgttgtttataatattgctggcgcccatcctgttacgtaaactgcggataccgagtatcatagggctgattattgccggtatgctgatcggcgatcatggttttaaaattatacagaaagacagtattgacctctttgccaaagccgggctattgtatattatgtttctcgcggggttggagctggacatgacagaattccgtaagaaccgctaccgcagcatggttttcggcgcttttaccttctttattccccttacaatggggtttgtggtatgcacctatgtgctgcaatttaacttcatggctaccctgctggtatccagcatgtttgctactcatacgctggtggcatatccgctggcaagccggctgggtattacaaaaaacgaggccgttaccgtagccgtgggtggtaccattatcaccgacactgcggtgttgctgatactggccgtgatcaccggtgcgcaggccggtaacctgaatacttatttctgggtgcggcttggcatttcactggccatttttgccgccatcatcctctggctgatgcccatgcttggccggtggttttttaagaagattaaagacgataaaacttcacatttcatttttgtgctggcgctggtatttgcatccgcattcctggccgagctggccggcgtagaaggtattatcggcgccttcctggcggggcttgcgcttaaccagctgatcccgcatacttccccgctgatgaaccggattgagtttgtgggcaacgctattttcatcccgtttttcctcatcagcgtgggtatgctggtagatttgcgggtattactgaaaggccctgaagccctgatcattgccggcgcgcttaccctgatggcgcttagcagcaaatggctggccgccctgtttacacaactggttttcaagtacagcgccaaccagcgcaaagtgatctttgggctcagcagcgcacacgccgcggctactattgcggtaatactgattgggtacaatatgcatattgtagatgagcatgtgctgaatggcaccgtgatactcattctcattacctgcctggtgggctcttttgtaaccgaaaatgccggccgccggctggccatacaggaagctgaaggcaaaccggaagtggacgatcagccagagcgcatactggtgccggtttccaaccccgaccgtattgaggccctgcttgactttgcagtaatgatcaaagacagtaacgcccctactcccatttacccgctggcggtagttcaggataatgaagaggcgaaagagaagatccatctcaccaacaagatgctggaaaaagcggtaatacatgccgctgccacggaaagtgacgtgcaggtggtaacccgcatagacctcaacgtttccgatggcattacgcgtgccaccaaggagctgctgatcagcgatgtgatattgggctggacggataaaacaagtaccaccgaccgctggctgggcaacatttttggtaccactctcgataacgtgttacagcgggtatgggaaaccgtgtatgtgtgcaacttccattcaccgctgaataccaccaaaaaaatggtgctggtaatgccgcccaacgccgaatacgagctgggcttcctgcattacatgcagaaaatgtttatgctggccaagcaggcaggcgccaggttactggttttttgtaatgagaaaacacaaacgatcaccaccgcttttgcagagcaaacgaagatgagcgtggacctgggtttccgccagtttgataccatcgaggacttcctggttctttccagggaaattacccgggacgacctggtagtggtggttaccgcgcgtaaaagcacgctctcctatcatgcatatatggatggtattcctgctaaattagagcggcattttaaggacaataatgtaatcctgctgtacccggagcaaagagagtttgattcactggaagcgggccttcaatcggaagatctgacgctggcgcctatacaggaacaaattgccaacctgaataaactgggtaaagcggtaaaacggatatttaagaaataactattacagtccttagtggctaaacgcaaaaaggtcccgcattgctgcaggacctttttatttgtgtgtagtgtgggagctactggattcgaaccagtgaccctctgcttgtaaggcagatgctctgaaccagctgagctaagctcccgtaaagatcttttggaggtaggtgtagtgtgggagctactggattcgaaccagtgaccctctgcttgtaaggcagatgctctgaaccagctgagctaagctccctctttaagatctttggaaatatgtcaaattactattgtgtgggagctactggattcgaaccagtgaccctctgcttgtaaggcagatgctctgaaccagctgagctaagctccctcttttgtttctttcctatcgtccctttcgttcgattggatcgcaaaggtataaactatttttattctaccaaatattttttaaaaaaacgcggggatcgccttcggcgatgcggagtttgtcttgagcgctgattacgctgattatactgattagcttgatttttgttcattggattttttggatttttttaaatgattcttaaaaaattaagagagatacaagcgaatcttatctgcttatatctctcttaatctttagaaatcaaaaatgatcaaatccaaaaaatcagtataatcagcgtaatcctgctccaagacaatttacaatcgccgaaggcgatcctacttcttctttttcttctccgccttcttcgcgaagccgccttcaaagaagcatttgatgccgcgataagcgccgcagccgcctatttcgcggatactcacccggttgccggtgaactggaaggcgataccacaggaagattccttgtctttgtattcgccccggttgccaccaatataatgtccccggccgctcagttctcccttgcagttaccgttatcttttgagaaggtgatgaagaactggaaggattttggatcatcaccatccctgatggatacaatgctcatgtcgccggctgtataatcgccggaaaatttgtgtttgcggggtaatgtatcaatcgggttgaagatctggccggcgttcgtaggtccgttggagttagtcatgataagtgttaccgatccatcaggattcaccatgtaaaaatcttctttcaatgcgctccggctgcccgacaattttgtttcgctgctgatcttcactacatttttactgtctatcagcagggaggtaaccgtaccgtccgcactacctgtgttggctacacggatccggttgagatacttgccttttttatccaggaagcagagataacctaccgattgtgacctgccggcagcttttatagtcatatagttcacagtgttgccgggaatccgctgcagcgggaaatatttcaccggttcgtttttaccgaaatcacctttcgtcagcgtatctgttaaaaaccgcatggcggctgtatccagtcgcagtgaatccggttgtttcagttggagcgtatccggtgtaagccggtatggcagggtaccaggtgtaaacaatgcctggaagtcttcaaatgtcatgggctcagtgccgctgcctgatttcttcttcgatttgcaggctgctaaaactccgattgccagtaataataaaaggaaacgcttcattagaaaagttaattctgggcgaaaagttagatataatttttatatgtgcgcgttaaaaatcaaaaaacataccggatagagaaatgttcagaattattatttagatttgtctaaataatattttagatagcatgaatttatctatcgcagaggaaaaccatattaagtcgatatataagctgcaggaaggcgacgctgttgtaaccaccaacgcgctggcttatgaactggaaaccaagcctgcatcggtaacagacatggccaagaagctgaaagagaaaaagctgattgaatatgaaaagtacaaaggcatcacgctgtcggcagacggcaggaaagcagccctgcaaattgtgcggcgacaccgcctgtgggagtgtttcctggtagataagctctccttcagctgggaagaagtgcacgagctggcggaagaactggaacatgtgcgcagtgaaaagctcaccaaccggctcagcgaattcctgggcaatcccgtgatagacccgcacggcgacccgattcccgacgccaatggcaaactggcaaaacctcgcccccaaacttcgctggatcaggccaacgccaaacggctggtggtaacagccgtatcagatcaatcgaccgcgctgctggcctttctcaacgccaaagggattaagctgggtactcagctggaaatagtggcgcattacgagtacgacaattctattgaaataaaagtaaaaggacaaccggccatcaccatcagtgaacaggttgcaaaaaacattatggtcagacccgtttaattatcagcaatatactatgagcatcgagcatacacattcatcagcatcgttaagtgaggtacatcagagtgtagaaacgagtggaaaatccaggtggaaaaagatcttcgccttcttcggccccgcctatctcgtaagcgttggttatatggaccctggcaactgggccaccgatctggccggcggcagccaatacggctacaaattattgtgggtattactcatgagtaacctcatggccctgctgctgcaaagcctgagtgcccggctgggcattgtgcgcggccgcgacctggcacaggctaaccgggaaacctatccgccggtagtgaatttcatcttatatgtgctggcggaaatcgccatagcagctaccgacctggcagaagtactggggatggccattggtattcaactgctgacggggctgccgcttgtatggggcgtaagcttaaccgtactcgacacctttctgctcctcatattgcaacgttatggcatccgcaaaatggaaggatttattatcagtctcgttgccattgtgggcgcttctttcctcgtggagctgatcctcgtgaagccgcaaatgcatgaagtaatacggggctttatccccggcatccccgataacaccgcgttgtatattgccatcggtattatcggcgccaccgtaatgccgcacaacttgtacctccattcggcattggtacaaacacggaaaataaaaagggatgatgcgggtatcaggcaggccattaaaatgaactttatcgacagcaccattgcactgaacctggcgttcctggtaaatgctgctatcctgatccttgctgccgccgtatttttcaaaagtggcagaacagatgtggcggagatccaggatgcacaccgcctgctggatcagctgctgggaagcaaactggctcccatcctgtttgccgtggcattgattgctgccggtcagagttccactgtaaccggcaccctggccgggcaaattgtaatggaaggctatctccgcctgcgtatcaacccctggctgcggcgattgatcacccggctgctggccatcatccctgccctgctggtaatccttattgccggcgacgaagaggtaggtgcgctcctggtgttcagccaggtattgctcagcctgcaactgggctttgccatcatcccccttatccattttgtaagcgataaaaaaacgatgggcacgtttgccattaaacctgttaccaaaattttcagctggctggtcaccagtttattggtgtaccttaatatgcggatggtattatcagaagcctttgattatatgtccggtaccgggaatatttttgtagacggattaattatggccggctgcctcggcttcgtggtgttgctacttatcaccattgtatacccgctgcgccgccgttaccgcgaagatgctgcggcaggcatccataccacccaggttacactgggagaaatggaaaagcccacctatcagtgtattgccatggccctcgatttttcgcaacgcgataaagatattgtaaccaacgctatcgctcacggtaacgaacacacgcaatatatcctcattcatatcgtggaaagcgcttccgccaaatactttggaaaagagtcggacgacctggaaacacgccgcgaccaggaacagctggacacctacattgcgctgctgaaaagccgcaacatcagcgccagaggcgtgctcggcttccgcaggcgcgcacgtgaaattgcccgcatcgtacacgaagaaaaagcagacttcctggtattgggcggccacggccacaggggctttaaagactggctgtatggtgaaacagctaaccaggtaagacaccaggtaaggatcccggtactggtagtgcaataaaatttaaaaagtatgcttccgttattcaaacccggtgataccaaacatttcagccgcaccgtgcggcaggaagactgtgcctcttttgacagcggccaggttcatcccgtatacgccaccttcgcactggcgcgggatgcagaatggtgttgccgcctgtttgtgatggaaatgaaggaagcacaagaagaaggcattggcacccgccttaccgtggaacacctctcccccgctttagccggcagccaggtggacttcaccgcagtgatcaccggaatacaacaccacgaaatcacctgcagctacgaggccgtttgcaatggccgcgtgattgctacaggcatacaggtgcagaaaattcttcccaaagcaaagctggatcggttgtttgctggattgtagcgagttttgtcttggctcaggattacgctgattatactgattagctggatttttacttttttgatttataaaggattaagggagatataagcggatatattcgcttttatctcccttaaatattattaatccaaaaatctaaaaaaatccaaaagtaaaaatccagctaatcagtataatcaacgtaatcctgagccaagacaaaattcgctacaatcccagcgctgccttcaggcgcggataaccggttttgctcaccaataccctcgcgccactgcggagaatggccaggtggttttctttctcgtagggatctatacgggttacctggtttacgttgagtatgtaagagcggtgtacccgtgtgaattgttgcgggtccagcattttttcgaagaacgacatggttttatttttcaggaagctgccttcctgagttactatttttacgtagtcgtctgctgcttccaggtagtggatatcctgtaccgggataattttaattttaccattgagctttattaccacgcggttgctttgcaaaggggtggtggcggcggtttccagcagggcttctgtgttggtggcggcgggtgtttgaaaatgatccagccatttttgtacggccttatcaaagcgatcactggaaaaaggtttcagcagatagtcgaccgcatgtacttcaaaggccctgatggcatgttcttcaaaggccgtggtaaagatcactgcgggcatattttccacgagttccagcatttcaaaaccggtgatctttggcatctgtatatccaggaagatgatatccggctgatgctgttgtatggcctttagtccttcaaacccatcattgcattcctgcaccacttctatttgcgggaagcttaacaggtattccttcaccacttcacgggccaatggttcatcatcaattaatactgcttttatcatgcgattgtggtactttaataatggtagtaaaaatattgtcaatggcggtggtttccagcaggtcttgccgtgcaaacagcaggtacagcctgcgttgtatggaagttaagccgaaaccggttcctttgtttggctgttgcagttcgttgtcgaacggattttgtatggcgatatacaacatgttatcctgcaaccatgaccttatgctgatggtgatatcaccggtggtatcgtatagtccgaatttaattgcattttctactacgggctgcagcagcattggtggcatcatcattttatccgcttcttcgtaagggataacgttggtggttaaacgatgcccgaaacgcactttctctatatccaggtacagctgcaaatagtttagttcgtcggcgagtgtgatccattgatcatcctcgcgcttcaatgaccctcttaaaaaatcggagagcttcaataccatctcgcgggcctcttttggccgcagcatgatgagcgcgttgatggagttgaggctgttaaacaggaaatgcggctgcagttgctgccgcagtttaaagagctctgcttctctcactatcttttccgtagcctcctggcgctggcggtattcctgttgttcttccgcatcgtaccacatctggcttctgaagccgatacctgcaatcagcatgcaccctacgatggcgtgaacggggatggcgttgttcagccaattgagatacagcggatcagcgggaaatgcggataccagtatccagcggctcaggcatacccacaaaacagacagggcaaagcttactatggctacgtagccaaacttcatggtgccgtctgccgggcggtagtaagccacgttatggcttattacaataccggcggcccccaggagtataacgtgcactgcactgtctgtggccgatagccagatgggaaggtcgaaccagtaccacagcagcccgccataaaggaacatccagatggcgaaggatgcgaggaaagcccaccaggcgttacctttaatcatttgttttaccaaagaaggtgatttatcagttatacgttaagctcaaagtattgttgtccctgtaactgggcagatttcatctgcaaccaggcgatgtaggaattggggtctcccggttcttcaatgcgggagtacagttccatgccgtctgtcagctgatccagggtatatacttccggtacgttgatgaacttccattgtaccagttcctgttgttgatttttaaaagcatattgttcctgcataccaatttcgcgggctttatcgcaggcgtctttcttggtaacagcgctgattaatcttaattgttcatcaaattgcggggtatgattgccttcaccgcagatgatctggtatacaactttcgcaacaaaccaatgcataaaattaaaatttaaaagttggagaagatagaatacaggttgagagatatggatgttttatgatcagtaactttttatttctacaccaccgaatacacaggatcctttcaggaccagcagtttctcaatggatccgttagacatcatgccggtgtgacgtttgtcttccaccccgccgagcacaacatcaatatccacctgaactttccagtgggccggtacaatgatttcacaaccaccgaaaacggctgaaacatccatcacagcggtgccattgatatctgcattcatgaagttgataacggcgcctccaaagacagcgcttacatcgcctcctttaaagtttttagacatcaccattttattcacactgccaaagatagcgttggcactcagcgtatcctcgccactggcaaattcctggctggagccgaaggcgtgttttttgaatgtccagtccgtaccctgataactctttttaaagatcagcaccacacctaccaggatcagcactaccggccatataaactgggcggtggcgtatggcagctcgagtatttcgtttgccatgaaaattccgcctaccaggaccatcacaatccatcccccgaacctgaatttatgttttgcccctacaacgataccgatagcgatcaggatcatttgccaggagaacagccagtggggcagattaagatccaggcgttgcaataacaggcaggcaccaacgatgatgaaaactgcaccgcctataaagcggccttttctttttgatgcttcgatatcctcgtttttcatttgttttactatttatgatacaaatgtagaacggcgcactgttattggaaacagggtttaggctaataaagtacccttaccggtaaaaagcaggaaatcgccggtgaaaacggcgggctatatttctaccgttaccagtgcatcgtttccggccagttttaccaggatggctttcaactgctgtaccataggatcggggccacagatatagaaatgctggttgaaatcactgatcttctctttcaggtaactttcatcgatggtgtggtggtcgtagcccggcacttcctgtgctgtcagcgtattaataaagcggttgcccagcatggcttcaaattcatctttcagaataatatccgacagggttttattagagcagatcagctggttgctgcccagttggcctttgtgctgcaggtcacgcaggatggcgatgaaaggggtaacgcctgcgccgccggcgataaaggtgccttctcctttatactgaatggtcccccatacatcgtgcaggataagttgatcgccggctttcaggtgcccgagttcgcgggtaacgctgttatggtcgtcgtagctcttgatcgtgaattccaggtgatcccattcggtgagactggtaaaggtaaaggggcgtctttcttcttcccatccgggtttattaacggctacttctgtagcctgaccgggtacaaaggtatatccggcgggcttttccacggtgaattgacggacgttgtgtgttacgggggtaacggccaggatttttacaatatggctttccattggttcaggttttctttaagatgaatgtaggatattttttttctcagtgcaacgcttgtagcaacaaaggcagcagggctttggcccagcggctgtagtcctttccggaagggtgcaatccgtcgcctgccagcagttcgggatcctgagcggcttccctggtaaagtgcgtgatatccaggtaaggcaccagccactcttccgcaatggctttattgaccgcgttatacgcatcaatttcccggtgaatcagttcccggtcgccgccggtggcaaatggcgttacgccccagtcgggaatagacagcactaccacatgtgaaggattgttgccggcaaaaacgatggccttttgcaaaagggcggtaaatgctgtttcatactcttcctcggaacggccacggtattggttatttacacctatcaacagtgttactatatcgtaggttttacttatatgtgctgcggcaatgccggcttccagttcgtcggtggtccacccggtggtggcgatgatctgcggatctgatacgtcaaagccttgttcccgcaacaaagcggccgcctgcacaggaaaacgttcggagggggaaacttgttcacctatagtataactatcgccgagggcgaggtacgtaacaggaatcatgatggtatgtaagattttgttgctgcgaaaaatgaccagcaaaataacattaatcctaacataagcaaaaagttatatgtaggtgttaaatttggggaataaagggcaaatgttcccctgcgtaaacggaaaagccttacctttgcccgcgattacaacaattacgtaacgcataagaaaccgttttatgccggcagaaaaaatatcgatgaacaatggcctgttacaggtccctgcacaccccatcattccatttatagaaggcgacggaataggtccggacatctggagagccagtgtacgcgtattcgacgcagctgtagaaaaggcttatggcggtgacaggaaaattgaatggaaagaagtactggcaggtgagaaagccttccagcaaacaggtgaatggctgccaaaggctacactggatgcgctgaaagaatacctggtatctatcaaaggtcccctgtctactcccgttggtggtggtatccgctccctgaacgttgccatgcgccaggagctcgacctctacgcctgtgtaaggcctgtacgctggttcaacaaagtaccttccccggtgaaacacccggagaaagtggacatggtgattttccgcgaaaatacggaagacatctatgccggcattgaatatatgacgggtacgccggaagcaaagaaactgctcgatttcctgcaaaatgaaatgggcgttaaaaagatccggttcccggaaacctcttccctgggtattaaaccggtatctattgaaggtacggaaagactggtacgcgccgctatcagctatgcgctggagcacaaacgtccgtcgctcaccctggtgcacaaaggcaacatcatgaaattcaccgaaggtggtttcaaaaactggggctatgcactggcagaaagagaattcggtgataaagtatatacctgggaacattgggaaaaaaccaagaaagacctgggcgaagaagaagccaacaaagaactgaaagtagccctggcaaaaggaaagctgctgatcaaggatgtaattgcggataacttcctgcaacagatcctgctggcgccacaggattattctgtagtagccacactgaacctgaacggcgactacatttctgatgcactggcagctgcggtaggcggtattggtattgccccaggcgccaacatcaactacctgaccggctatgctgtatttgaagccacacacggtactgcaccccgcttcgccaacaccaacaccatgaacccatcctccgtgatcctgagcggcgtaatgatgctggaatacatgggctggaaagaagcggctgaaatcattgttcacggcctcagcaccgccatcatgcgcaaacgtgttaccatcgacttctacaacctgatggacgatgccaccctggtgaaaaccagcgaatttgcggatgaagtgatcaagcagatgctgcactaagcgcgaattttgtctttcgcgaattttgtctttttcaggattacgctgattttactgattacccggatttttactttttggattttaaaaaggatttggggagatatcagcgagtggatttaaaataattccgggatataagcgataaactttttggggagatgtaaacggatatatccgcttatatctccccaaatcattttaaatctaaaatgatcaaatccgggtaatcagtaaaatcagcgtaatcctgaaaaagacaaaattcgcgaaattttgtttttttcacagctattcgtatttttcgtgattatcccaattgggactcgcttgaataattgttgtgaaatgcttttaatttaattttaaaaaacccgaaatggcagaaaaaattaaagttgctaatccggtagttgaactggatggtgatgaaatgacacgaatcatctggaaattcatcaaggataaactgatacttccatacctggatgttgaaattaaatattacgaccttggcatggagcaccgcgatgctaccaacgaccaggttaccattgatgccgccaatgctatcagggaagtaggcgtaggtatcaaatgcgctaccattacacccgatgaagatcgcgtaaaggaattcaacctgaagcagatgtggaagtcccccaacggcaccatccgtaatatcctggatggcactgtattccgtgaaccaattgtaatgagcaatgttccccgcctggtgcctaactggactgccccgatctgtattggtcgtcatgctttcggtgatcagtaccgcgctaccgatttcgttacaaaaggaaagggtaaacttactattaagtttgaaggtgaaaatggcgaagtgatcgaacacgaagtatacaacttcaaaggcgatggcgttgcattagccatgtataacaccgacgaatctatcaaaggctttgcccgtgcatgtttcaaccaggcactgatgaaaaaatggcctttatacctgagcaccaagaacaccatcctgaaaaaatatgatggccgtttcaaagatatcttcgaagaaatctatcaacaggagtttaaagctgaattccaggcaaacggcttaacttatgaacatcgtttaatcgatgacatggtggccagcgcactgaaatggcatggtaactttgtatgggcctgtaaaaactacgatggcgacgtacaatctgataccgttgcacaaggctttggctctctcggcctgatgacttctaccctcattacccccgatggtaaaacaatggaagcagaagccgcacatggtactgtaacccgtcactaccgcgatcaccaggcaggtaaacctacctccaccaatcccatcgcttccatctttgcatggacccgcggtctggaattccgtggtaaactggacaacaacgagcaactgatcaaattctgccaggcactggaacaggtttgtattgaaaccgttgaaagtggtaaaatgaccaaagatctggctgtttgtatccacggtaacaaagtagaacatggtaaacactacctgtatacagaagaattcctggaagcactggatactgcgctgaaagcaaaactggcgtaaattcataaagacaataaaaaaagcagcggataaagtatccgctgcttttttatttaaccagatgggttgcttacaacttcatcctctttcttaatattttatcttctccataaatatcatcgtaaaaaacaagattaccattttgtccttctgcagtaaaataccgcaggtaaataggaatatgtttaggcagatctacctgtttcttttcctctctcgccagccatacgcgaacactgtctccaacatgccgtaagctatccgcccgcaccaggtactgcgccaggctatcccattgctgcacccgcacacaaccatgactcatggcgcgcatggaatttttaaacagtccgcggttattggtatcatgcaggtatacactgtacttattcctgaagttaaatttcatgatgcccagtgaattatctattccatccatctggcgtaacacataaggaaaatgccctttaccgagtttcgaccagtcgatggtataaggatcaactgcattgccatctctatctattacttccaggttcttagccgcaagatagccgacattctttttaatagccggcagcatttccttaaatacaatactgtaaggtacccgccagtaagggaacatcatgaagttggtcatataggaattgagcaacggcgtgcgggtacggggtgtacccacaattacgcgcgattccagcaccacttctccgctatccactaccttcagattgtagccgggcaagtttaccatgatataccgggacggcaatgtatcgggcagcttacgccatcggtcgaggtttacagcggcctgcataatccagtcgtgcatagagcggttcattgccatcactgttctctttcctgctacgccatcggcataaatattaaattctttctggaaagcttttacgccggttttcagtaaggctgaatccagctcccggcccgtggtatcgagatgaccgctttgtaccagccggttgatcaccagttgccggaatccaagcgtgtcggtataattgagcggtaaggtatcccagtgatagttttcgtatttggctttgaaagactggatcccttctttcagggcgatatacccttcatgcgtaggctccagtgaatgcaggatgtttgctacatttttttcgttcaatgcctgccgcaattgtgtgatcagttgttcgtcggtaaacgctgaatcctttttaagggtgatgctgtcacgcggagcaacgccgtagcggagatcggacgccattttcatgaaggcgtctgtcatcagcacatcgacttttgcccacagggcggcatctttttttgcggtagcatcgttggtaatctgttcccaggcagctgttagcgcgggctcatgatattgcgcaggcaacagccccacgtcttccgcgtgctggatcatatacagcatggaatcggctgcgggattggtaatcccgttctttgaccattggctggacggtttatcggctccgtaaaaatcctgtatggctgaagcacggaaagactgcaaactgtcttccagttcgccatcattatctttcagggccgacaatcgttcggtgatactctccgtgatcacttcatccaattgtttgatgtttgctacaatctgtttttgtttgggggcggtatgcttttttttatttacacaggctaacaacaagcacattccagatccgcataacaaactgataataaaaattttgttcttcatctgcagtaaatcgctatggtaaagataggaatttacaaatactgtgctgaaaatttttggagaacgggaaatggaagcggttagccttctactacggctgccactatagaaaatgaatgttttccggtttacaactatgaatcatgaagcatgttacataaaaaattgcagtgaggaatatgacgttgaagggtttgctggtgtatgagtattggattcttctgcataaagtgagaaaaccaacttttaccggaaatggtaatccggatcaaagttttacactataatcttatattttaatcatgagtaaagaaagaaaagaaatggttttacatgatgaggtattaatcaataaaatctattatatcaagggacataaagtaatgttggaccgcgatcttgcggagttatatgatgtaaaaccaatacggttaagggaacaggtaaaacgtaatataaacaggttcccggaaaatttcatgttccagttgacagaggaggaagtggaaagcatggtatcgcaaaatgcgataccatccaaaaaacaccttggtggctatcttccatatgtttttactgaacatggtgtgttaatgctggcaaatgtattacgcagcgaaagggctatacaggtgagcatccgtataaacggcatgatgaagcaggaggatagtctcccacaaaaccctttctgcaacaatccttcttcacaaaaagcgaccgggttggtattctactagtatatttagctgactttgctttatcctcccttttattttgcttgcattcgctaccagtaaatcataatgcccgctttaatttacctacgcagacaacacacataccatttattcgccatctgaaacgggacatagtgtattgggagtgcatggagagtgcatggggagtgcatggggagtgcatgaggagtgcatgaagagtccatggattccccataacatacgcatgtctgaagcatggctgaggcatctgcgaaataacaacgcgccaaaatacaaaagccgcagacactacatctgcggctttaaaaatcattccccctgctatctatctgcaacaatccttcttcacaaaaagcgactgaacaaatttcaatatgcttataacaactttcttcatgtccggattttttaaaaagagaagccacgatgtgcagcagcttctctttaaactaaaactaaaacaactaacttctatatcttatctaatggtatacgctcaggcgctttcaattgtttgaatttacttggcgtgagacccgttacttttttgaactgtgctgaaagatgggccacgctgctgtatcccagcttgtaactaatttcacttaagcttaattcattgtataccagcaactcttttacccgttctattttctgctgaataatatactgttcaatggtagtgccttccgtttcagagaaaagattactcagatagtgatagtccttctgcaactttcctgccagtaaggtggaaaagttttctttcatttcatccagctctgaatgatgcaccgcctgtacaataatactttttatgccggcaatcagctgctgttttttatcatctatcagtaaaaatccttcctgctgaagcgcttcggacaactgctgcagctgtttctctgaaacagtacctgcaacggttaccttgcccaattgtatatcctcaacgtccagttgctgcgcggcaatggtggtagtaaccactttgatgcagcgcggacaaaccatattctttataaacagatctgttgttgccatcggttactttttgatattaaaaatgttatgctccaccctgattaaaaaagagttggaggtattcctagccatatctccggttaactgggtgcggtaagacaagtccagcctggtggtgctgttaaaaataaactgcactgcgggcgctatgtccagataggaacctctgcccaccgcgtctgtattggttttgcccaacagttccacgtaaaggtttaaattggtttgctggaagcttttatacttcaccggcaaaaccaggcaccctgcagagagactataatttacggaactccgggagaagtcgtccgggatttcatccttcacattgttcatataacgggagtagcccaacgttgtggacaacgccagtttatgtaacagttgcgtagcaataatacccccgtttacacccgaagtagctccttccagatccagctccttattgtcgtacggtcgcatggcatgtgagccgtcgggcatttccgggtaatatggattgttgatcacggcgcctcttacataggcagccatgcggaaatgcgcgtgctgctggtccagcgacaggaaacggtatttggcgtatacaccaccaccttcgagttttacagagttctgcatcatattggacgcatatcccagcacatgcagcatgagctttttattagcgccccacatcacttccggctcaaagcgcattccattgtcgccggaatgcttcatgttgaaaaacttattggtgagcctgatccccagtgagttggcgggcatattgctcgccggttctgtatttacatacaattcctgggcagctgctatgccgttaccagccatgacgatcgtggctattattaaaattcttttcatataccggccagctattaaatggtgacgtgataaattcttttggaagcagcagcgccatcagtcttacagcagtcgcccatcatacctgttttataacagggcatagtggtttcagtactgaattttttaaattgtttggaagaaataaagtctttgtcaattacggtgatgtccttatccccggataatacctggttctttacatccataaaatggagggtgctgccggcaaatgctacgtgcgcatcgttttgcacgcttacagcatcgaaattggcagtcatcaccagcttacctacagaaaaaccggcatcttccactttacctttaatagcatcaatgctcaccggtgcaccggttttgaaggtaagaatgaaagtggtgttatcgaggtcggtatcaattttttcaacaaaaggaagtgattccagggcctcgtaagtagcttttgaacacatagcgcaggtaaggccggtggcgtgtacgctggcttttttaaattgcgcgtttgcgccgaaagacatgcccagtgcgagcaatataatggatactattttcatgatctgatgaaataaaattgaataataagatgaataacagtcaaagcaatagcggtgctgccttacagcaaccaacactacattaaaaactgcatcagatcaggaaagtacaattgcggaggaaaataggcgcagacggaatgtctggcggatcgtgggggcggctcacgaaaaatagttcctgcgccggcaaagcggaaacaggtaaaatcgttacgggcagctgcatatctgtggcagggctgaaaccggcttgcagcgctttggcggcctggtgcgattcagtaaccttacagaacttaaactcatctttacagcaatccatgccttttgaaggctttccgcattttccgcagtggtcagccggagcttcctgcagatctacagaggccagtttgcccatgcaataatgcacgtttactgcaaacccgctggtaagcgtgatatacagtactgcaaataatatggcgaaaaattgcttcatgatgaattacaaagataagaaaaaaaatgaccgggattgcgtcgccacaataccggtcatcatatagttatatgtaatagctagttaataaaccaccacctgagcgccaacctgaaggcgaagttattatacgggtataatggtccggcataattgttatcccccaggaaggtattcaggttttctgcgcgcacatatgcggagaaagatttgatccggaagttggcgaatgctgcaatatccggtaaagcgttactgatcttggtggcattctggtaaataaactgaccggtgagcggggaataatcatctgcataataaccggtgttatagcgcagttcaatccccgtcatgaggttcaggtttgtatacagtcttttttcgaaggcaaaccggttacgggtccagaaggtgggcacgttcaacgggccgttgccatgcagctgctggaaggcgatatctacataccaggcaaacggcttgatgttaaacttcttgctaaacgttatttgtaacaggttaaacagcgagttatactgctcgctgtgataataatctttaaaataggtgtaattggtaaacaggaaataattggctgccaggctataattcagctttttgttttcggtggcaaactgcagctgggtaatattttccttcgacaggctcgtattataccaggcatcatttgtactgttaaaatatttgaagacgtaagagggttccttatttacgttgctgaccgacaggcggacatccccaaggaagtcgttaatatgtctccttaacattccataaaaaccataatccccgatattctgtcctactacataaaactcacctcttgcagagaaatcccatttctggttgcgcgttttattgcggtattctccatgcacggccaggttggtaaaattaatatctgcgtccaggaaggtaccggtgagactttcgaaacgagcgccaatgttaataaagtgtccctggttaccgagtacagggaactggatcagcgacaggtcgttggaaatcattttccactggtgcttggatgctaccgtatcgccgggtaaaaagttatagtgacccgaataaaaagcggtatcagggctgctatccaggaattcgtagttattactctgataattgaacgtgtattgtacacggaatatcggatcatacttataataatcggtggtatcgtttacgtggatactgtcgccgcggccccagtcgtactgctgctggatcaggaaccctgtttcgcggtagttggatttcaccggtatgctgcctccaaagaaagcatatgttgttgacgcatcattacccaggtttaccgggatggttttgcgttgtttgtaagtgctgatgttcatgaaggaatcgttcctgatccccccgttctccccgccgttgatcttattaaagtaaaagctcaggtaggtatgggcacgtttattcttgctctggtaccgggccgtaaagcggtagatatcgtgattggtattttgtgagcgaaaatagccgggggcgtttattttgcggtagtcgaatgcaaagttgaagcgctccgtccggttttgggtatgggaaagcccgataatctgttcctgtttgctgcctaccaggtactgcagctctgtgtaagggcgtgtagtatagtaaaagcgggcatccttatgggaattggaatatacatcgtacgcgtgaaagccggcgtcaaaaccgggtttcatgcgtggtgtataaatcatgttataagctgcgctgccggtgttaccgagcgtggtgtacgaggaaggtactttcagataattggtctgaaaatcggccacggaggagtcgagcttataatcggtgggttcaccgaggatacggtaggttaatgtcagcgtatccggctcgtgttcatgtttccctgtatcccgctgcattttgctggtgccgccgccaccgcccatattgttgatgcgtcccgagttaaactgggccattaattgattcccgcacaataacagcagggctatgaaaatgaaaatttgcctcatccgaaagtaacaaaagcgtttatagttgccggattaattcactaaatatcagcgtaagcttaggttctgctgcttttgcagctgccagtacttcttcgtgggtgatcacattttcttcttcacggataccgatatcggtgatcacactcatggcaaatactttcaaaccggcatgtgccgctacaattacttcgggtacggtactcatcccaacggcatcgccgccgataatgtgcatatatttgtactctgcccgtgtttcaaaggtaggcccctgaacgcctacatatacgccgctatgtaaagatatattgttggccgcagcaattttattcgctgcatcgatcagtgttctggcatagggttcactcatatccgggaaacgtggacccagcgtgtcctcatttttgccccgcagcgggtgttccggctgcaggttgatatgatcccggatgatcatcagatcgcctacctggaaagatgggttcatccccccggcggcgttggaaataaataaagtatggattcccaaggctttcatgacccgtacaggaaaagttacctgctgcatggaaaatccttcataaaagtgaaaacgccctgccatagccactaccggcttaccctgcatgaatccgaggatcaatttgccggaatgcccttccaccgtagattcggggaaatggggtatgtcgctgtatggaatttcaatgctatcctcaatttcccctgtcaggttacccaggccgctgcccaggataatgcccgccactggcttgttttgccagaatttgctgatatactcccccgctgccgtgatctttgctgttaattcactcatctgtttatacattaataaaagccggatttaaaaaacaaacccgcgcaaagttattttttaattcacaaatgactgcagttttatatttaaatcataatgacctattttagcggcaaattttattccgatgaacttacacgagtaccaggctaaagaactgttgaaaaaatataatgtaccggtacaggaaggtatcccggtggatacccctgaagcggctgcggaagcatacaagcagctgaaagtgcaatttggtaatgaatttgccgttgtaaaagcccagattcatgcgggcggacgtggaaaaggtaagatccgtggtacggaacagagaggtgtggcagtaggaaaaaatgcagaagatattaaaaatatagcaggaaatatcctgggaggcaccctggttaccattcaaaccggcgatgctggtaaactggtaaataaagtactggtagcacaggatgtttattatccgggcgctaaccctgtaaaggaattctacctgtccatcctgctggaccgtgctaaaagccagaacgttatcatgtattccactgaaggtggtatggatatcgaagaggtagcacacagcactcctgaaaaaatatacaaagagtgggtaaaaccaaatatgaccctgcagccgttccaggcgcgtaacatcgctttcaacttcggtttgagcggcgaagcgttcaaaaacatggtgaaatttgtaaccaacctctataacgcatacgtaggactggattgcagcatgctggaaattaacccgctgttcaaaaccagtgatgagaagatcattgctgtggatgccaaagtaaacctggacgacaactccctgatgcgtcatccggacctggaagccctgcgtgatatttctgaagaagatcctaccgaagtagaagccagcaaatacaacctgaacttcgtgaaactggacggtaacgtaggctgtatggtaaatggcgccggtttggccatggctactatggatatgatcaaactgagcggcggtgaacccgctaacttcctggacgtaggcggtaccgccaacgcacaaaccgtggaagcaggtttccgtatcatcctgaaagatcctaaggtaaaagctatcctgatcaatatctttggtggtattgttcgttgcgacagggttgcccagggtgttattgatgcttacaaatctatcggcaacatcaccgtgcctatcattgtacgtttacagggtaccaatgctgctgaagcaaaagtactgatagaagaaagcggtctgaaagtacagtcagccatcctgctcagcgaagcagctgcgctggtaaataaagccgttagctgataataattgtcagaagatataaaaaaaggagcacaggtcatctgtgctccttttttatgttatctcccggagatcagcttcccagcttttccagttctttcctgtaattgtctgccggctgtcccatagcagtagctttggataccgcccaggtaaagtatttctttgcctgctccttatacccttccctgcacatatacgccatcatggagatggcttccaggctggagttttctgtaagagccggcgccgcccaacgcacatataaatctttcagttccggttgtttttccagctcccccgccatataaaagcgcatgtaacgcacccggttatcgttcagatccttatgggcgatggcaaactccagaaatgcctttgcgtttttgcaggtttttaaaagataattttctgcgtagtacatctctatttcgtgccagtcggccgcactgtatacctgctgctgttttgccaggaatgcctcaaatgccgtcgtatccagttgtttgggcagggcagccaggtcctgcctgagcaggccgtttaatatgttcttattcagctccacgccaaaacgatcctggtaagcagtcctgttttttatatagaactccctgtagttagctggcaggttgcggcataccagcattaccttgaatacggattccttaaacaggtctttttgttttaacaggtattcctttaccacggcgctatccggatacttcctgtcctttgcaaaaaagaaggttcgataaaattccgggtcatcggttttcaggctgttgccaaaaccgcccaggtactcacccgctttatatctggcaatattattttccaggaattgcaggaactgcggtggttcctggtaacccataccggtattgatcagctttccttccccggaaatgatcaggtaagtaggaaatccggtcatgaagtacttggcgcagagttccttcccaaactcctctttaaatacatcatagccggtgcaaatgaagtgctcgttcatgtacttctttacttccggtcgtggaaatacttttacttccatgtctttacaggcatggcatccttcaaaatacgtgtcgatgaaaatgggtttgtgttccttttttgctttggcggtgagttctttccagcttcccttgataaactgggtgctgtcctgcgcagccgatgccaatggcaacaggcctgccagcagcagtgctttgattgcatttttcattgtactgtttttttaatggtttggtggggcgaagctaataaataagtgcggattttgtctttctcaggattacactgattttattgattttaaggatttgatcattttggattttaaatgatttggggagatataagcggatattttcgcttgtatctccccaaatcatttataaaatccaaaaaagtaaatcaataaaatcagtgtaatcctgagaaagacaaccttcgcttactcgcctttcttgggcgcgggcggcatggtagctttcggcttgttttctttattgtctttgtgttcttcttttggctttgcgggcgcgggttcctggctgtcggcgccaggggtggcgtaatcgctggcatcgccggagccgtaatcgtcggctgaaccgttgcctacgttttcagattcagcgcccggttttacattggaatcgtaattcatgtaaatatcgtcttcgctcatattgggcggtaccgggaaatgatcgttggagcttactttcagggttggatcggcatacactttctgcatgaaatacgcccagatgggtaagccggtattggcgccctgaccaatggcggtggtgctgaagtggataaagttgttttcgcaacctacccatgcgccggccagtattttaggcgtatagcccatgaaccaaccatcggtgttatcgttggtggtaccggttttaccggctatttcaccctgaatgttaaagcgggaacggacacgggcgccggtaccacctggtgctaccacgccttccatcattttcaccatggtataagattccctttcgctgatcacctcgcgtttcaccggcgcgaaggtttccaggatgttaccattcctgtcttctatgcgggtgatgtaaataggtttggtattaatacccctggcggggaacatggtgtacccctgcaggagttcatacagcgacagctccacggcgcccagcgcaatggctggataggcagggatatcgctggtaaagcctactttatttttagcgaaatcagcaaacggcttggcccctatctgtttgattaggtaggcggccaccaggttcagtgattttgccagtgcgcccgccatcgtaatgctgccaccggtgctgccttccgaattatgcggcgtccagccgttgatggtaatcggttcgtttggcaaaatagtatttggcgacatgccattcataatggcgaagcagtacaggaagggtttaaatgtagaacccacctggcggcgtgtttttgccacgtgatcatttttgaagtagcggaaatccggtccgcctacccaggcctttacttcaccactttcagggtccattgccataaagcctgcctgtaaaatggcacgcatatatttaatggaatccagcggggtcatggtggtatctatttcattcaggtctggttcggtagaacttctccagccaaataccttcatgcgtaccggcgtattaaatgccctggcaatggtagaatcgtctgcttcgtcctctttcatggatttatacctgtcagattccttcatgtactgatccaggaatttgggccatttcttccaaacattgccagttttgatatcgttttgtgcagagagtgatttttgcagcaccgcaaggtgcttggccaccgcttcttctgcatacaactgcattctcgggttgatggtcgtatatattttgagcccgtcgcggtagaggttatactctgatccatcggctttcttatgcactttgcaccagctcttcagttcatcgcgcagcacttccctgaaataaggggccaatcctttgttgtgatcaattttattatagtgcagtacaatcggtttgcttttcgcggatgcggcctccgctggcgtaataaagccggcttcctgcatattgctgatcacggtgttacggcgctggagggcgttttgcggattccggcgcgggttatacagggtgttgcctttaagcattcccacaaggatagcagcttcttcgatagataaatggccggcatctttgctgaagaatgttctggccccgttttcaataccatatacgttatcgccgaaggcaacggtgttcaggtagagggtaaggatttcctgtttggtgaagttcctttccagttttacggcaatgatccactcctgcactttctgaaacgccctgccaatcgggttaccggagcgttgttttcccaggttatccgtttgcaggttcagagccagctgctgggtgatggtactggaaccacgttttttaccgatgagcaggtaaaaagggatagccagtgtgcccttggggtcgataccggagttatcataaaaacgggtttcttctgttgctatcagcgcgttgatcacgtttttggagatctcattataatcactgctggaacgatccacctggtagtacttaccgagaatggtaccgtcgtcggcaattacctctgcggccagtgctgcccgcggattttccagttcttccatcgacggcatgctgccaatgatccggaagttaatgagtaaaactaagagaacaattaatgctaagataccaaaagccacccgccacaatattttcaccgattttttcatgcgcttatttaatttgttttatggccagattttgcccgatttctttatatgaaagacaatttatcactatctgttggctatatatataattttttcaataaagtttatatgcaataaacaagcctgtttatggcggcccgaccgacaaagctatttaaaattccaaaaatacttactgggtcacataattatctgtaaaaaacttacggtaaccggccaggtctttggtgctgtttaataagatgaaattatccctggaaatcacaaagaaattgtactctgtgggtcttatccggggaatgatattcgcagcagcctcatctcggatctcatcgaagtaggccagggctttgtcttcgttggggaaaagccggaaaatcagcatcacgtcgttaggggtgagcacaaaactgccgacttcaattttatcagtggcatgtttggcggcgttataacgtgtaaactggttaaggccctcatccatgagctccttagacacgcgctggaaggaaagcactacaaaaaacgggttgtcgggcgatattttatagggcgttaccggttttggcggtgcgataggcactatgggcgcaggcagtgtgccagccataccggcggctattttagccgaatcggccggtgttttggcgccgttgatcctgtcggccagtaccggttgtggattttgccaggggtatcgcatagaaacatcttcatccagcaatacgccgttggcgtctttcttccttacttccagcttggcgagatagtcggaaagctctgcgcggtggttcagggcatccataagagcctgtgcctgagcgcgtaccggctcatccgcggcgtacttggtaagtactgcctgtactgctttacgcgacaactgcagagtatcggtggcgtacagggtatctgttttcacgatcagcattgcttccagcagatcgaatttggactggaggaagttaacgccgaaggtgctgtcggcctgttttttcatagccatcgattccgcatagttaccgtggcggaaggcttcataagcggcgtcgtaagcggcgctgatctctttctttttctggctgtcgatatcccttaatccgcctgagcggatgatgtccgcaaaattggtattaccgtactggttcagcaccattgatttatagtgattagcctgggcggtatgattgagtttgctatgccatacatacagggaatacaatacctccggtttctttggatgatccgggtagaggatcagcagggagtcgtaggtttctatgcccagtgaatagttctccagtttatcgtgatataatttgccgagatcgaaccaggcttcgtgtactgctttttgtgaggcggccagtttttccggtgtcagcggcaagcctgcggcaagggatgccgtgctgatcgtgtctgccggcacgtcgcccaggatgacggactttgtttcctctgtaatttctatcgggccggcgctgttggtagcatttaccacgccgttctggctgcggcgccagttgtctaccggctgccggctgccccatctgcgtttgaattcggaatagccggctgatttactgcctgcattataaaaataccagtcgcctttttcttcttttggtgaataggcggtgcctgctccggtcatgctgaaggaagacgcactttcctgcggattggcggcggccagtttatctttctttctcttttcggcggcttcactttccatgacggccaccattttcgataacacaatgttccggtcggacggggacatggcggctaatttctggagactgtcttcccggtgaatggtttccagccgcgccaccacttccgtgagcacttctttgcgggtttccacggtaggggcgtctgcaaaatcctttgtcattacgcccgcggtgctgtcgtaatatttttttgcatcggtataattgcgctggtcgtagtaaatatccgccatgcctttgtaggtgatggtgcgctgcatgaggttgtcactgggtattttcagtgattgtttcatatagttaagcgccgcttccgggtgatcgggatattcgagcacgcccatggtataatagatcccgtcgcggaaccgttcgaaccgttgctttttgagcatgcggcggaggcctgctatgctgccggctatgttaccggtggtttccgcgttggttctggcaatctgtaaccgggcctggaaatccatcataggatcgggtttcatgctgatcacgttgcggaactggtcgagggcggaatccgggtgctgctgctgcaggtagagctggccgaggatgtacgacatcctggctttggccactttatcatgacttttatcgatggccactttcagcggttctattgtttcggggtaccttttctggatatagtggctgtaggcacgtacttccgccaggtcgccgtcgaggcggtgggggaagttaggatcattgttcaggatattgagcagcgcctgtacttcatcgtattcctgttgttccagcagggtacgggccctccacaggaaagcgtcgttacgtgctttggtatgtttgaggcggccgaagacaccttttcttttttcttttgtggcgatggagatctggtcattttcatgcgctcccactactgttttgtattccgacttcgttttgggtgcgaaggcaatattgatgtactggaatgttttattggcattttcgaggtcgccttcataaaagtaggcgcgtcccatgagcaggaagcaatcgtcgatccatttaccgcgggggtcgtggagctggatggccatgtttgttttatcgatcacggagtccagttcacctttgctgaagccctggctctgaagactgaagggataaaacggcaggaggatattataattatcctggccgtcgcggttagcggttttcactacccggtcgagtttaaccctggcatgaaagtaatagttgaagcgggtagccatgttctggaagaattgtcttttccaggtccatttctttttctccagcattacttcagaagggggacggcggtcctgcacgcgttgttcgcgcggtttaaaaaggggcttgacggcaggcttttgctgctgttgctgtttaccgggggcctggccctgggaatttgtttgcggaggctgattttgagggttattttgtgcccgggcagcctgcaaaaccaggcaacatgacaaaattattattcccgaatattttggtagcagtttgatgatgcaattcatggatgccagggtgtataggctaaatatatataacttacagtttgaaaaaatattttaaagataggataaaatagttgattgaatatgcgtctggaagaagtgatgcagactttttccggtagcagatacattttaatcggctggttttcagataaaaagacttctttctgccggcaatcctcaaaacactgtttcctattttacaataatgattaactttagcccgccttaaaagaaatagcattctttaagaagtaccgcaaaacatggccaagaaggggaataaaaacagcagacgaaacctggaaaaactaagtcataaataccgtctggtaattatgaatgacgatacctatgaagaagtgacctcgttcaaactctcccggatgagcgtgtacattgccttcagcaccctttttgtattactggtagccattacagtagctacggtggtatttacgccgctgcgttattacatcccaggttatggagatctgaaacaacgaaaagagtttatccatctgaaaatgagggctgattcgctggaaacggctatcaatgcccgcgaccagtatctgaacaatatcaaaaaggtaattaacggcgattttaccgggaaagtggacaccacgatgttaaaagtgcctgccgtagataacagcacctattaatatataaatacaaaaattttatatatatttatttatattacacactaaacttgaaaaacctaactccctatgtttaatagcaatcaaaaatcgaaaggtgacagcaagtccatgttgccaacatcaacggttaatattataggcaatggcacttctatccagggcgacattgtatgtgaaggcgatatcagaattgacggacaggtgaatggcctggtatctaccaaagctaagatagtggtaggacctgagggtgaaatcaccggtgacctggtatgccagagcgctgacatcctgggcagggtaacaggaattatcaaggtagaagaattattatttctgaaagggaatgcattagtaaagggcgatgtatacaccgctcattttgaaatggagccttctgctaagttcaatggccgttgctacatggacgatcagcagccggctgataaccagaaacatggaaaaaccgtcctccaggaagccgaataaccgaaatctcctcttacgatatgccggattagccttccagatgatggctacactgggtttgggagtatttgcgggatataaactagaccaatggattggctggcggttcccggtattcctgatcattttttctttacttgctttagccatacttttgtggcaaattataaaagacacccgacggcatgagtgatagattttttatacggttattcgcagtttttggaattctaaacggacttgttatcatattcaaacccaggttgctggaccttggcacacatgtgaatgtgctgatggccggtaacctgatcatggctattatctccctggtgtcttatattatgagccgccggggactcgcttcttccaaccacaatgcatttatcagggccgtttatggctctacgctcagcaaactttttctttgcgtcattggtatagctgcttacgtgcttatttataagcccaatgtgagtaagctcaccattttcatgctgttgttcctgtacctggtgtatactgtatttgaaacaatcagccttttccggctgacaaggctaaaaaaataatctatttgaaaaaagaggcgcccttaaatgcactagcgtcctacttaccggaaggaactttcggacaggtaatggattttctgagtacctataaggtacacctgacggttacacgcgaacggtcgagtatactcggcgactaccgtcatcccgatgggcagggcaaaggacaccggatcagtgtaaatggctccctgaataaatacgctttcctgctcaccctgctgcatgaaattgcacatctcaccacctttaataaatacgccaaccgcgtggcgtcgcatggcaaggaatggaagcaggagttctcctttattttgcgcgactttgtaggtaaaagcctgttgccacccgatgtggaaactgcggtgcgccagagcatggccaatcccgctgccagctcctgcgcagatgaaaacctgatgcgggtattgaaaaactacgacctgcagaaagaaaaccatttcttcgtggaacaggttcccttaaacggactgtttaaaaccaaagacggacgcgtattccgcagaggggataaaataagaaaacgctaccgctgtgaagaggtagcgtctaataaatggtttctttttagcccggtatacgaagtagaacttatttcctaactcttctcccctacataatgcaataccgggaaagccatggcacggttgatcagctgaatttccagctgcacgatgccggcttctgctttggcctgtaacttaggcgcatcatcggtaggtttatgataatcgtcgtgaccaccggtatggaaaaacatcaccggtaccccgcttatatagaaattatgatgatcagaagcgcctttccccgctgcatctgtaaagtatttaatgcccggttgctgtacatctttgaacaccgcaggccactcttctgcgctgccatagccaccaatcccgatgcccctttccgggttgtagcggccaatcatatccatattgagcatgaaatgcactttatccagcggcatcagcggatgtgccgtgtaatattttgaaccctgcaaccccatctcttccccaccgaaagcgataaagaggaagttaaagggctcgcggccctggttctttacatagtgccgcgccagttccagcaggcctgccacgccggaagcattatcatctgcaccgttgtggatttcaccgatgggatactttccatcgaataaagcggccgttccgaggtgatcataatgggcgccaatgataatcgtacgtgcggcgccgttatcaagatacccgattacgttcctgctgggaatatccttatgttctttccgggtgaatataaaatcctggaagaagctgttgccatttaccggcttcagtcccagttttttaaactgttttgccacgtagtggctggctgttttcccgcccttttctgcggtgcccctgcctttcagtttgtctgacgccaggtaattcactattccctgaatgcgtgcggcatcaggaatagtgtcctgtgcctgtgcggcggtgattgtaccggcggcgcacatcaataaaaaccatctctttatcatatccgttcaaaaatagagaaggcttccttaacgggaagccttctgcgaaaaaatattattgaaatgttcagattgtattaatcctactttttcttctgtatgtcctgctggcgtttctggacttcttccagtttctcctgccatttggatttgctctttggtttctttttattttcctggatctgtgcgtgaattttatcatggttgatgataaacttctggatcacaaactgtaacagaatactgatcacgttagacaggaagtagtagaaggtaagtgccgcagcaaggcggttgaagatacccagcaacattaccggcattacgtaaggcatgtatttcattaccgggttgctctggtcggtcattccacgattgtagaacgccaggatcaagctggtgatggtcatgaggatggtgaacaagctcacgtggttgccatagaacggtatgttgaagccaaggttcaggatagaatcataagtagacaaatcctttgcccataggaagctttcctggcgcagctcaatggaagacgggaagaagctgtacatcgccaccaggataggcagctgcagcaatgcgggtaaacatccgcccagcgggtttacgcctgcactcttgaacagtttcatttgttccacaccgaatgcctgctggtcgtcgccatgttttgctttcagctcatcaatttcaggtttcagcactttcattttagcctgggaaacatagctctggtaggtaaaaggagctatcaacaggcgaatgaagagggtgagcaggataatgatgataccgtagttgctgataaatccgctgaggaagttaaacaccgggataatgataaagatgttcacatacttcacaaaagcaaagataccggtacccagcggaatgatcttctgcaggccgatatcaaaagatttcagtgttttatagtggttgggaccataatagatctcaaccgggaaggagaaatcattggtgcggctatacggaatctgtatagtgctgaatgtttgtcctacgatattagggcttaccggcactttcgtgtttacatccacgttagtgaacagttcctttttagcaatcagggtggtattgaagaactgctgttttacgctcacccatttcagtttgttttccagtttttcatgactggtgcggctgagggtgaagtaatcatgtttatcattttccagcatataatgcacctggttgttcaggcgctcattttcaagatcgtgttcctgtttatcttcctggctgttccactggaggctcagataattctggttgcctggcagtaagccttgcataccaaccgcgtgaatggtataatccactacatagctgcctggtttcagggaatagataaattccaggtaagaagcagggttattggtattaagacggtatgcgattgtttttacgccaccagcgccttcctggggttggccggcggtgaagaacagatccgcgctgttcagcatttttgttaagctggcaggcacttctactgaaaggcggttaaaagagccttccacgagcatcagcggaccaccatcataagttttgtattttttcagttgtacacttgccggttggccacctttattggaaaaagtgatctttaccacatcgttttccagtactgtgttctgcatgttgccggtggcagcagcggcaaatacgccaaattcgccgtttaacagcgcctggtgggctgaatccagctggcctcctgcggcggctgcagcaaggctgacagtatctgctaaaggtgttttaggcttgttaagctctgcgatggaatcttgcctggctttttcccttgcggctcctgcctgttgtttctggttgaagaatatatatcctaccaacaaaacgcccaacagtaaaaacccaatgaccgaatttctatccatgaaatgcaattaaaatttaggcagcaaaggtaagcaggattttatgaattgaccatgctttttaggtgaaacccctgttaaatgcggttaaaataataaataagtaaagaaaatgcgtattatgttgaggatcagagcggattttgtctttctcgctgattacgctgattatactgattaagggatttgaacacttttgattttaaaagatttggggagatataagcggatatgcttatgtctccccaaatcttttaaaatcaccggtaagtataagggagataagagcgatgtatccgcttctatctcccttaatcctttataaaatccaaaaagtaaaaatccggttaatcagtataatcagcgtaatcagcgggaaagacaacctccgcgcaggttacttcgcgatggtttcttccattttggctttgccgtttttggcttctgcgtactgtttggcggccttaataaaagacacgaaaacaggcgccgggctttccacggtacttttcagttccgggtggaattgtacgcccacgaagaacggatgggtaggcagttcgatgatttcaacaagaccgctttccgggtttttaccggaaagaacgaggccggcgtcttcaaactgctggaggaagtcgttattaaactcgtagcgatggcggtgtctttcactgatgttggtgccaccgtatatttcggctgctttgctgcctggtgtgagttcacaggcataagcgcccagacgcatggtaccgcctttagctgtcactttcttctgctcttccatgaggttgatcaccgggtgagcggtgtcaggattcatttccacggagtgtgcatctttccagccgagtacgttacgggcatattccactacgctcatctgcattcccaggcagataccaaagaaaggcagctgattttcacgggcatactggatggcgatgatctttccttcaatgccgcgatgaccgaagcccggagctaccaggagcccgtcgaggttcttcagcttttcacatacattttcaggtgtaatatgttctgagtggatattttgtaccactactttgcattcgttcagggagccggcatgtataaatgactccaggatagatttgtaagcatcctgtaattccacgtatttaccgatcaaaccgatggtaactttggatttaggatatttcagtttatccaggaattcacgccatttaaccagttccggttctttttccacaggtaatcccagtcttttcagtacagaaacatcgagtttctcgcgcatcatttccagcggtacttcatagatggtaggaacgtcgtttgcttcgatcacggcatctacctgtacattacagaacagggcgattttctttttcagatcgcggtacaatggttcttctgtacggcaaacgataatatccgggtgcacgccatattcgctcagcaggcgtacagagtgttgcgtaggtttggttttcagctctttagctgcacgcaggtacgggatcagtgtaagatgcactaccaggcaatcttcttcacccagctcccattgcaactggcgaaccgcctcaatgtaagggagtgattcaatatcacccacggtaccaccaagttctgtaataacgatatcgaatttgccatccttaccaagcaggaggatacggcgtttgatttcgtccgtaatgtgagggattacctgtacggttttaccgagataagctccttccctttccttattaattactgtctggtaaatacggccggtggtaacattattggcctgagacgtgggcgtattcaaaaaacgttcgtagtgtccgagatccagatcggtttctgcgccatcttccgttacataacattcaccatgttcataagggtttaatgtacccggatccacattgatatatggatcaaatttctgaatagtcactctaaagccgcgtgcctgcaataattttgcaagggaagctgctataattcctttacccaaagaagatgtaacacctcctgtaacgaagatatattttgccataaaactaaaattctgctaagaatacttgacctataaacggggaagtgccggactgcgtttggtgtaaaaccgatcaagtaaactacttccgaaggtcatgcaaagttacacaaatttgcgtcgctcccaagttttttacggcagcgctttatttgtttgttaattttttggagataatattcagctctcatcacttatctacagggcgttttaaagaattttcaagtaccggaaattatttgttaaaaacctttatctgccaacgctgttctgtaaatgcgtacgcgactataaatatataaacagtaaatttgcgtccgaaatacataaaagatgactttaacgccaaagagagcccaagactcgctgatacagatgaccgaactggttttaccgaatgataccaatacattcggtaacctcatgggaggccgtttgatgtactggatggacattgccgcggcactggcctgcatgaaacactgcagcgcacccgtagtaaccgcttctgtagataatatatctttcgaaaatcccattaaactgggaaacgtggtacatattgaatctaaagtaagccgggccttcaatacttccatggaagtacacatgagagtttggggagaagacccggtacaacagtaccgctataaatccaacgaagctttcatgacctttgtagccctggaccccaacggcaactcccggccggtacctggcatcctgaccgacacagaagaagaaaaaaagttatatgaaggcgctttacgccgccgtcagctgcgcctgatcctgggaggcaaaatgaaacccgaagatgcggatgagctgaaagcactgttcttcgagaagatatagcgcgtaggttgtcttactcaggattacactgattttattgatttaaaggatttgaacactttggattttaaatgatttggggagatataagcgtaggttgtcttactcaggattacactgattttattgattaagttgattttatttttttttagatttttaaaaaggattggggagatataggcgaaaatatccgcttatatctccccaaatcatttaaaatccaaagtattcaaatcctttaaatcaataaaatcagtgtaatcctgagtaagacaacctacgcttccccctcccactctttgtaaaaccgctccaggaatgcttccataaatgcgtgtctttcttcggccagttttttaccggtagcggtattcatccggtctttcagcagcagtaatttctcgtagaaatgtgtgatggtaggagcgctgctgtttttatattcctcttttgtcatttgcatattgggctttatggcaggatcgtagagcgacctgtttttgaaaccgccgtaattaaaagccctggcgatgccgatggcgccgatagcgtcgagccggtcggcgtcctgtaccacggctaactctgcagagaaaaatgttttttcctggttgcctcctttaaaagaaatgtgacggataatattctccacctgtgtgatgataccggccggcacttccaatgattgcaggaaagccactgcttttgccgggcctatattttcatcgccgttatgaaattttgagtctgcaatatcgtgtagcaaggcgcccagttctactaccagcatatcggctgtttcggtggcggcaatatgttttgcctgttgccataccctgtaaatatgccaccagtcgtggcccccttctgctcctgctaattccgtttttacaaaatccaccgttgcggtgatgatctgaccgtgagttatcataggtgcaatgatattaatttttgggaagacgatggaggaaaacaatacggttcctgtgaacgttatgtaaatatgttacaggttaaacggatatacgaagattatgcagataccgatggctaccgcatcctggtagaccgcctctggccgaggggtatttcaaaagagcgggcccatgttgatgaatgggcaaaagaaatcgctcccagcaacgaactgcgcgaatggtttaaccatgacccggcgcggtttgctgagttcaaaacaaaatataaacatgaattacaggagaaaaaagagttgctggccggtattaaaaagaaggcgcaacatcagcgggtaacattgctgtacggggctaaagacgaaacacacaaccaggcacaggtgctgctggagttgttgaaaaaataattacacaccttcactttcgggcttcaccagtacctctgtgatgctgttcagcttttttactttgctggcaaaatcaccggtcagtttttcgcggatcagcgataatttgttcaatacttcatcgagggtatccgggatggcttcctgcagcacctgtttcaggcgtttggcaatggtgggtgatttaccattggtagaaatagcgatcttcagatttcccttttttacgatagagcccaggtaaaaatcacaaagctcaggggtatcagctacattgatcagcactttgctgcctttggctttttcccacacataataattaaagtccttgttgttggtggctgctattaccaggtctttccccagcaggtcgccacatgaaaatgatttctgaacaagggtaatattgggatactggtgtgttaacgcctccagttcaggcaaaaaatccaatgacactactgtaatggttgcatctgcgcaattgtccagcatggcattggctttttccagtccgatattaccaccacccacaacgagtacatgcaggcggtgtaatttgaaaaacaccgggaataaatgattttcttccattatacggcaatttttagttcctctgacaccttgttcttcaaggcctggaaagcttcatggaagctcaccacttcgcctatcaccagaacggcaggattatgcagatcgtgcgtagcggctatttccagcagatcggccacgttgcccactcccattttctgggttggcaaagtaccattctggatgatagcggcgggggtttccccttttcctgctgcgctgtagatccctgcaatttctgcgagtttgctcatccccatcagtatgatgaccgtggtattggccctgatggcgtgatccagatcgcgggataaattcccgttctgtgtgttaccggtgatcacccaaaacccttcacttacgtttcgtgcagtgaccggaattttgttgacgcctggtacagagatcgcgctggaaataccgggaatcacttccgcggtaattccaaactgctgagcaaaggcaatttcctcctggccacggccgaaaacaaaggagtcgcctccttttaagcggacaacgctgccataagttaatgcatattttacaatcatcctgtttatttcgtcctgtgaatatacatgcattcctgcacgtttacccacaaaacgacggaggcagttagccggcgcatggtccagcagttcattgctggacaatgcgtcataaaggattaccctggcgttttgaatagcctttaaccctttaacagtgatcaattccggatcacctgggcctgcacctatcaatgtgagtttgggttgtatcttttgcatgagtggtcgtgtttttgataaataaataattaagcctgcaccagttcgctggctctctgacggtatacctgtgcagcattataaaatgactgcgcctgctggaaataagtttttgcaaaactttccgtaggctcgttaccgttaatctgcagcactactgttttaaaatcaggctcaaagctgaatttaccggtagccacaaaatgtttatcgaaatcgttcatgataccgatctgcgtattaccgctgatggcttcgccgagtaacagtgcttttgcgccctgcacaaaggaagaataagcgtgataaattccatctgaataggcgcctttaataatggcggcactgctcagttccagtttttcttctgcttccagcagcagcgtagccaccaggtcgatgattacaccggcgcactcgcccacaccgatcgctgtagcgtagtcctgtgcctgtccccagtcgataaagtcgcccgcggtgagggaactgagatctgccaatggtttcagcaattcgtagaaatacttttcacctttacggtcgtagtactcgttgaacagttcattttcctgggcattgatttcatagtcgtgcagcaggctgcgtaatacatccgggccgcggcgacttggtaccttaattactttatcggcaacgcggcctgcgccatcgcctacaataccgccaccgagtagtacctgcagggcgggaagtactttaccggcgctcttcatggagctgccgtggaaaccgatgctggcaataccgtgctgaccgcaggagttcatacatccgctgatctttattttgatgtctttgttataaacgagatccgggaattcatcggtgatcacatcttccagtactttggcgatgccggtgctgctggagatgccgaggttgcaggtatcggtaccggggcatgccgtgatatctgcgatgctgtcgaatccgggatctgcaaagcctgcttcttccagtacgctgaaaacatacgggagatttgccggcaggatgtatttcagtaacaggccctggttggcggttacacgtacatcgtcggctattacggggcgcagcgcttcgataagtttgcggctgatcgctgaaccgatgttacccagtgttattttaacgtaagccgcgaagtatcctttttgtttttgctcaaaggtgttggtagctttccaggcttcgtatttctttggatcttttatgctgtaagccggtgttggcgctgcgggaggcggtgttgttgcctgccatgcgtctgcatctaccggtacgctttttacttttatggctttgtattcttctttaatgaggcgctcaaattcttccattccaattttctggatgaggaatttcatgcgggctttgttcctgctggttctttcaccgtagcggtcgaacacgcgcagtacgttttcgatatatggaataagctgatctgtttcgaggaactcgtatactactttagcgagaaagggttgtgcgcccaaaccgccgcctaccaatactttgaagccacgtacttctttaccatcgatgatctttactttggggatcatgccaaagtcgtgcataaatgaccaggctgtatctttttcagaagaggagaaagagatctttattttgcggcccatttcctggctcaccgggttacgcaggaagtagcggaaggtggcatcggcgtatggcgtaacgtcaaatggttcatccggatcgataccggcgcggtctgatgcggtgacgttgcgaacggtgttaccgcaggcttcgcggatggtgatgccatcctgttccagtttagaccataattcgggggttctgtcgaggctcacgtagtggatctgtacgtcctggcgggtagtcaggtgcagattactggtggcatattcatctgaaatttcggtaatgcggtgccattgtttcagggtcattttaccgtatggcaatttgatgcggatcatttgcacaccgggctgacgctgaccgtaaatacctctggccaggcggaggctgcggaacttttcgtctgacacggcgccttcgcggaacaggcggatcttcttctccaggtctataatatcttgttcaacgattggattttctagttctgttctgaagctttgcataaaaagtattttcagtggtggtaaagcaattatttaattctggtttgggggtgttggtcgttttttaaataaaaaagcccccggattgttagcggaggcctcgtataatgttgatttacagcaagatgatcactgattttccatattacacgcgcctcatgggtgttgatgaacaacaactgtttctacgacaattccttctatcattacccatattccctataattttagtagagtaatacaaagatataaatgcagggcatctttccaaaacttttttcaacattcaataaggctccaaaaaggggggaaattagcagaggccgcaggtctgcagcgggcaggcggcctaaacgccggtctgggacggattggcggagaacagcctgcctggttaccgcagcagtgcgataaccaaagtttatggcgtataacttattgttatgggataaggagtaccggcaccctggtacgggttaaaccggaagtataccggaagcaaaggtggacttgaagcccaaatgcaggctggcaaacagttgccggtgtactgcgatctccccgcataacttcttatctttgccgcgcataaatggaaaacatatgatagatacggtaatatttgatatggatggcctgttgatcgattcagaacctttgtggggcatcgccatgcgggaggtgtttgcaacggtgggagtaaacctttcgccggagctgacgcatctgaccacggggcttcgcaccaaggaagtggtgagttactggcataattactataaatgggaagggaagagtgcagagcaggtagtaaatgaaattattgacagcgtaatacaaaaaattatagcggagggccatcctatggaggggttatcatatatccttcaatatttccgggagaaagggttcaaaatggggctggcatcttcttccccgctgcgcctgattaatgcggcactggagcatttgcagataaaagacgctttccaggcggtgtattctgctgagtttgaggattatgggaagccgcatccggctgtgtacctggcctgcgccaaagcattgggcagtgatccgttgaattgcatcgcttttgaggattctgtaacgggtatgactgctgccaaggcggcgcggatgactaccgtggtggtaccggaggcgcataaccggcatgatccgcggtatgcgttggctaatatgaaactggacagtttgctggaattcaatgatgcgaagctgtccttgctgatgaagtaaagaccggtaactattataaaaaaaatcccgctccgatgttactcgaagcgggatttattatttaatgaaaccggatcttattgcgcgcttttttcttcgccgccttcagattgtttcagtttttctctcagttcagctaaagcgccgagatcacctaaagtggctttctcaactttaccctggatgtttttcacagccttacgggttttatcagcttcttctctcttctctttcactacagcctgtttttcttccgcctgtgctttttcccaaaccctggtatgagaaaccaggatacgtttttcgctgcgatcgaattcgatgatcatgaattctttcacatcttccacgttgattggtttttcatcttcagttctgaggtgacgtgcaggagcgtaagcttccagaccgtactgcagttgaaccgtagcacctttatcatctttcttcacaacggtaccttcgtgtacggagttgatcgggaagatagtttcaaaagtgttccatggatcttcttcgatctgtttgtgaccgaggctcagtttacggttgtctttatcaatacccaggattactacatctatttcgttacctactttagtgtattcagatgggtggttgaaacgtttgatccagctcaggtcagagatgtggatcattccaccgataccagtttccagttcaacgaatacgccataaggagtgatgtttttcacgatacctttgtgacggctttcaaccgggaatttagtttcgatagtagaccatggatcttctgtcagttgcttgatagacaggctcattttgcgttcttccttgctcagggtaactacaacggcttcgtattcttctcctaatttgaagaattctttagcgttgattggcgtagaagcccatgagatttcagatacgtgaaccagaccttccacacctggcatgatttccaggaatgcaccgtagtcttcaatgtttacaactttaccttttactttagcaccttcggtgatagtagctggcaaagtatcccacggatgcggggtcaattgtttgtagccgaggcttatgcgacgtttttcgtcatcgaagtcaagcacaacaacgttgattttctgatccatctgcagtacttcgctcggatgggagatacggccccagctgatatctgtgatatacagcaagccgtccagaccacccaggtcgatgaacgcaccgaagtcggtgatatttttgatggtaccttccagcacctggcctttttccagtttgctgatgatatccactctctgttgttcgatatcgctttcgatgagcgctttgtgggaaacaacggcgttgcggatggtttcgtttactttcaccaccttgaattccattgttttgcctacaaactggtcgtaatctgtaactggtttcacatcgatctgagaacccggcaggaatgtttccataccatatacatctacgatcaggccgcctttggttttgctggtaacggtaccagtaaccacttcgcctgttttgtaaacttccacgattttttcccatgcacgtttctggcgagcctgtttacggctcaggtgcaggttaccatcgcggtcttctttttctactaccagcacttccacttcatcaccgatcttcagacctggtaaatcacggaattcgttcagagaaatcaaaccatcagatttgaatccgatgttgatcactacatctgtgttggttaaacctacaacagtacctgtcagcaggctgttttcttcaaacaccttgaaagtgctgtcgtaagtaacatcgtacttttctttttcctctttgctgtaagaagaaacgttacgtttgtcaacgctccagtcaaaatcgtcgtgtgccgtttcaacttttgctacaggtgcctttggtgtcgctgtttcaaccacagcagcttctgcttgtggagcctgttgttcagcgttttgttcgttagaaatgttgttttcgctcataaaaaattaaaattttacccggaatacccggataccctgttttatgggacggcaaaaatacgaaaaaatacccgtttatacgtatttttattgaagaaaatcaccttccgctgcggtattggctggtcttctcagatattttttaattgcattattaataatcttactacgacaaaaaattaaactgcgtaaacggcattttttttgccgcaggaagaaccagtatccggattaattgttgttaacaggtgcaggagagatgatattcattagcagtgaacaggcttacttttcgtgctttcaaaatgttaattactattatttaatcccggattttattttaatttgtgtatatgaacgggacctcatttcaatcggatattcgctactggctcaggcagggaaacacagttaactatttgcttttctggaatatcgtcatcttcctgggattaaatatactgcgtcttattgcgtttctgaccaagcagcccactccttttgaatggacctatgaccagctggccatgaatgttccgctcagcgcatttatcctaaagccctgggggctgatcacttacatgtttacacatgttggcatcttccacgccctcttcaatatgatcaatctttactggtttggtaacctgttccgggatttcctgggaaataagcgggtactccccctttatttgctgggaggtattgcgggcggtttattgtacctgctgagtgccagtctttttccgggcttcgtaggtaccactatggtgggcgcttcagctgccatcatgtgtatcctggtggcagcggcaaccctgatgcccaattttgaaattggcctgatgttcctgggcagcgtgaaactgaaatggctggcgatggccctggtgatactgggattgatctctatcccggatggtaacatcggcggcctgatttcccacatgggcggttccctgctgggcttcctctatatacgcaccctgcaggcagggactgacctctgccagcccctgatatggttatttgatttcaacaaccgccgccagcaacggccgacccgtaaattcaaacccaagaagtcgccgctgaaagtggtgaaaaaagccgaagacagggacccttccaggttagaccagctcttggataaaatcaatgaaaaaggttataatagcctcagcgccgaagaaaaagcatggctggacaaagtgagcaaagaaaactgattaactttgtccttcaattttctgccatttaacacatgaaaacatttaacgttccggttatatatcgcagtccgctgatcagcgccattaaaaaccagcgcaagcagcaggaccgcatgaaaaaggacttcacgcctaccgagctggattttggtccgctccggattttactggcccggcacttcgggttctgttatggtgtggaaaacgccattgaaattgccttcaaaaccgtggacgaaaacccgggcaaacggatcttcctgctcagtgaaatgattcacaacccgcatgtaaacaacgacctgcttgaccgcggcgtgcagtttattatggataccgccggccatcagctggttccctgggaaagcctgcaaacagatgatattgtgatcatccctgcatttggcactaccctggaaaccgagcggcagctggccaccctgggcattgaaccactgaaatacaataccacctgtccttttgtggaacgcgtatggaacaaggcggaacagattggtaagaaaaactatacggtaattgtacacggcaagccaaagcacgaagaaaccagggctaccttttcccatagcgcctccggcacgcctaccgtggtagtaaaagatattaaggaagcggagctgctggcagagtttattaccggccggcgtactccggaggaatttaacaccttgttcaaaggacaatattcacccggttttaacccggctaccgatcttcaacgggtaggcgtagtgaaccaaaccacgatgctggctaccgaaacgcaggccattgccgattacatccggcaggtgatgatcactcatttcgggcttacagaggctaccgccggcgaaaggtttgccgatacccgcgatacgctctgttacgccaccaatgataaccagacggccgttaccggcatgctgcaggaacctgctgacctggccattgtagtgggaggctataacagctctaatacttcgcacctcgtggaactgtgtgaagaaaagctgcctacctattttatctcatctcccgaaaaaatactatccgcaaaggcgattaaccactgggactttcaccataaagaagagattattgctgacagctttttaccggaaaaggaaaaagtaaccatcctgcttaccagcggcgcttcctgtccggatgcccttgtggaaggcgtgatacgccggctgctttcgttttaccagctggagcacaaggcagatgaaatggctataattgattaaaagtatctatctgtacaaaactgattaaaatgtcataaaagcaaaaaagacaccacgtggtgtcttttttctttggggctaatcacgctagtaatgcagagtataaaatctttatattgcgtttatattgaaatcgtaattcaaaagtagtttatctccaatatgcctgcaatagccatttattatatggtaggtaattaattataactggcataaaaacgaataaaatcggaatacgcacttctgcaaatacgctgtacatcctcatttagaactgcatcgcctttttcaggaactctgctttgcgtcttctggacacttctacctgtgtaccatcgctcatcagtgcaaagcctccttctccctggatatacgattgcatttgctgcatatttatcaggtgggaattatgtacccggaagaaatccacgtcagacaacagctcctcaaactctttcagggggcgggataccatgagatttttcttatccgtaaaaaagatgcgggtatagttaccggtagattcgcaacggacaatgttctgcacgggcataaacaccaggccgttgatagtgggtaatgcaattttcttgtgtgtttgctgtattgttttcatgttctgcaaaaacacttccatcggagaaatgccctggtcctttggccggttcaatttcttctccctgcatttttccagagcatcctgtaattcctttacactaaagggtttcagcaggtagtcgagcgcattgaacttaattgcttttaaagcatactgttcgtaggctgttgtgaagatgacgtcgaagtacaccttttcaaatagcttcaacagctcaaagccgttctggtacggcatttccacgtcgagaaataccagatccggctgcagttcatcaatcatttccttcgcttcccttacacttttagcccaaccaatcacctgtacaccgggacattttttttgcagcatcgtttgtagtgcatcaatgcagtgttgctcatcatcaacgatgatagcttttatttcgctcatacaagtagcttttgttagctgttagctatcagctgtttttatggtttatcagtgagtaagctaaaatataaattccgcaggtaaaattatagtcacctttgttccggtggcctttccggcttcatcttccaggtctgttaccgttacttttgcttccttgttattaatcttacggatcaggtctatcctgccttccgttactttcatgcctacagaattatgtagccgtcctttcttttcttttatttccattgctttttttctgcctatgccgttatcggtgatcgtacataccaggcttcttttttccagtacaatttcaatatcaaggattcctttttcatccgggtgtttatgcacgagtccatgccagatagcgttttccacatatggttgtaatatcatggggggtatcagtacttcatcatcattaatctccgcatcgatgaggaaccggtattcaaagatgccgttacagcgtaatgattccaggtcaagatacaaccttaatgattccagttctttattcagggtaacaaaagtgtgttgggtgttatcgaggatgaggcgcatgagccgggaaaacttggtcagatagtcggatgcctcttcctggttattgctccagatgtaccggtgaatggagctgagggagttaaagataaagtgcggattcatctgggagcggagcgaccgcagttccagctgtaaggttcgtttatttgccttcaggttacggtgacggatatagaacaaaccgcccacgatggccattaacaggaatgccgccaggaaaaaggtgaccaccacattgcgtttggtgcgtagggccgctatcactttatcatgttccaggttacggatctggttatctttccggtctacttcgtaaatggtttgcatctgggcgagggccattgccgacttctcatccaggatactgtctttatacaacagtgatttatcggtcgcttccagtgattttttaaagtccccgctttctttaaagtctgctgcgagtgctttatatgcgtccatcagcatggctttgaagccccagaaggtgctgatctcgatcgattgcagcatatttttcctcgcttcctcgtgtttcccttgtgcgcccagcagtttaccgatactgagatagctttccgccacatgtaccttatcgtctacccggtcgtttacttccagtgcttttttcaggtagtccatggcggccgtataatctttcttttccttataggcggcgccgagggcattataacatattgccataccgatggggcggtccattttctggttgatggccagggaacgtttatagtattggatggccaggtccagtttattctggccctggtatgcgtaaccgagattgccgaggttaatggctacgcccagttggttatcacttttctcttcgagttcgagggcgtggttaaagtgggtgatggcatccgcatatttttctgtagtgagctgtatattcccgatactgttggtggccacgcaaacattgcggatgtcgttgatcttttcggccagtatgagggcttttacgtggtagtcgaatcccttctgcagtttatcctgccgccggcaatctaccccggcattattcagggaaaatacgatgagggaagtgtctttcgcttcctccgcagctttgagtgctttttcgtgataatcttccgcaacgatatactgcgacttatttcttttggcggttcctaattcgttgtatgcctgcgatactcctttgggatatttgagctgtagcgataaagtgagcgcttcctgccagaagggattttctattttatgcgattcaaaaaagcggttgtttactccgccctttttcagcagtaaagacactttcccggtatcggaggggagccggcgaacagagtcgagcaggttgtatatccgcagggagtcctgggctatcgcctcaaaacaggcccccagcaggagcaagcataaaaaacatacaccttttatagacattggctggtctgtgtgactacacaatttaaaaaagaattacgaataacgcatagcgatctaaagatatccggttaaacgggatagcgttaccctttcactgacaatcaaagtgtttaaaaaagcgaaagggcgaaagaattcgccccttcttcctattaaccgaatacacctactgaaaacatggaacggccatggcgtaccacgccatcccacattacctttaaatgcctgctggcagcggttatgctcacgcagaccaaattttatattatagcaacattataatcggttaatagcaaagggtccttgtggatatagctaggataagacctttccgggagcacgatatatgataacgcgtcttacgcacttgttcttaatgtcttatacagtcgacagcactacatcaacagcacggacttttccatacaaaaattacctaagcagtatttttcagggaggatcaggttggctatgcagaaatggtcaataaaagttgacatcatttgggcatgaaaataaaattctactggaaattcgggaggatgtggaaaaattatcgggttggtgaccaacaggccacataacaaatgtataaaagagttttaataaaaggaaataatattttatgaggagtgcgccataatagcatcttccacccattgcatcaccagttgaagctggtcatcgaggttcaagtagctgttatccaggatgatagcatcttctgctttgcgcagcgggcttatttcccggttggcatcaatataatctctcagttcgaggttttgttttacttcttcgagggtgatgttcttatttttctcatacagttccttaaaccggcgctgcacgcggatcgcgatgtcggcggtcatgaagattttgagttccgcatggggaaatactacggtaccgatgtcgcggccatccatcacgatgcctttacgggcgcccatcttcttttgctgggctacggccagatcacggacttcctttacagcggctacctcgctcactttttcagctacgatcatttcgcggatcaggtgttccacgttttcattgttgagatacatttcgctgatgccggtgagtgagttaggaacaaaatccaggtgtacatcttccagtgcagtggccacggcttcatgcgacgtccagtcgatccggttttgaataaagtaaagggtaatcgcacgatacatggcaccactgtctatataggtatagttcagctttttagccagttgcttggccaaagtgcttttgccacatgaagagtagccatctatcgtgatgattatttttttcaaaactatctgtttaaatgaatcgcctatagggaagaaccctacaaaattggggcaaatctctgagaaaatcaaaacaaaaggctggaatttccggtagggggaaattccggccttttattgggctactactaccttgcaggtataagccactttcatggtgtctttatggtagatcacgaggaagtaaacgcctgacggcagatctgagatattcacttcggcgtcccttcttacctcgtactggcgcattacctggctccaggtatcgtgcagctgcatcagcatatcgccgcggataccgcggatagtgaccttgaagttaccgttattcggattcgggaataccttgatctgtacaaatggaggcaccgcccgtatttcagaataggtgattttgccgttcctgcctattgccttgatgcggtaataggtccagtcgtcgtaatcattcacatccgggaaggtatagctcaaaggtacgctgctattgccattgacggcttttgttggcagcacgccgattttcacgaatgcttcctgtctttcgtagcggcgttccacttcaaatgtggcattataaatttcacggctggtagtccagttcagctgcaccaataacggggcaatcctgtaggcttcaaagctgaggaacatggctggtttggcggagccgatcaatgctgtttttgtaaagtattcgctggcgcctaatgcgtcgaaatgccggaggtgcatggttgacggttgtaccatcgtcgtggtggttagtgtaccaggcagcggcctgttggtgattaccggtacggcgtcccatacgccgccaacgaagcgggtaatgaagctgctgtcgcgcgatgtagcataggccggcagttcgctgacgtccatgtgttgcaggatcacatatacttctcccccgctgttatctacccggcggatattccaggatttgttcacgaagctgtcggggtaagccctgccaccagccgccacggtaaatacgctgtcgtatacacgtgcgcctatcatatcttttgcgccggtaatgagcacagcggcgggtgaatagctatcatcatccgttcctacggggaacaccacttttccacttgcgttggtgatagcggcacggtacagtaatccgcctgctattcctttcccggtaaccacatagcggtagtcgctgtagccggtaatggtaccgggtgttttatcgcctacctggaggttccagccgttcagataaatgcgtccgcccgcaaaatgaaggttattcctgatcttcagatcgctgaagtcttccagcagtaagcccgccgggttattgagctgcaggttgggaaagctggcgcctgttccggcaataaagctgtaagcgccaaatatcctttgctgaccggcgccggaaaagaggaaggtgccgccggtaccggaagtaccgtctgcactttcatcgggcagcgtagcaccgtttccgttagtccataatttgctgaggaaataaaaggtggcattgggattagagccgaggacaccgttgtttgtcatatcagcgaagatacctacgttggtattgccggcgagccatacggtagcgccggcggggatgtaaacgccttgctgggcggatgtgaaacccaccaaaaacaaaagggataatatcagcaatagtttcttcaccaatgtttttattggattacagtaatatcgaaaagcctggtggttcctgacaaagagtaggcagcaacaccagtattgacaaaaactgctgttacggtgttatcagcggatacccttgaagaaattaagcgtaaagtaaagggaaaatcaaacctcggattgatgataacattgccgcccagcgcaagcctagcacccgttacggcgaatgttacggtggcagttgctgttgtgctgttaggaatgctggttgcaccggtaacaccgtttacaccagtacaattcacatttgacaccctgtatacaccgtttagcaccgtaccgtcagcgccaagtatggccgtaccatttacatccagcagagcgccgggagcgctggttcctatacccacgtttccgccgttctgcaggaacaaacggtaatcctgcacgttggtttccacaaagttcaatccgttgcttaacagattccagtgccattttggggtacccgcggcatcttcaaatgccagcacatcatttccatttgcacgtacaattaacgggtgcccgttaaatttcacggcgccgttgaacaaggttaaagtagaggcggaaaaatcaacgccgccgctttcggcagcggtttgtcccctgcttcccctgaaaagttctttattgttatacttcaccaccatatcaatggcattggtggttccgaggaattgcgtggcagtggctgcgttaccgccggtaagccaattggtggtagcagggttatctgttaaaataacgtcgccggtactgtttattgaaagcactttagaagtagctgctgccggcgtagcagtggccaggtttgttaagcgcaacccggaagtatttgctgagaaaggagctgaagtagacggtggccctgctatttccactttattcacgggagcgctggtgcctattcctaacaacaactttgtagcatcccagaatagctgtccgttattttcagtaataacatttccagtgcccacatagggaatggaaccgggtgttaaccctttcacggtaagcgttgtgccgatcacaccacttccggatatattaaaatttgaagatgcctgtgtagtagtggtattctgaataaaagtagctgcacccgctttagccatccactgcgttccattaaaagtaagtacatcgttattaacaggggtggtaccaaacaatacatcatagtcagctattttattagcgttccataatttgataccgtttttcaccgtcagctgtccggctgtgatggataagttattatcgatggtcatggaagcaacatctccgctggcatcctttcctaatatttttatgggtgtactaacgtcgttggttacacgcagtaagtaggtttgcagtccttctgtaaagttctttaatcctttaaacgactgggcgctgtaattaacaaatccaggcgctgtgagagaagcgtccggaatggtaaggttatgaataccgccggcagaggcaaagccaaaagtgccgcctggcgtgtacgtggctttaatttgctgtgcgggggaaaagtcgttgttaatggatttgatggcggcgccatctgctatcagttttgtccagtagttattggcccggacgcggaaagtattatcagattccaggtagatgatcatcccgtttaccggggtaacgatctgattggtatctgcaatgcgggtaaggaggagtgcctgctttttgctttccagttcaagtaaagcagattgttttatcagagaaggattagttcccagctttaattgttgtgccgtcagctgttgattgcccaggcaaaacagcattgcagcacatacttttataagcccttgcagcttcatacatcaacatttaaggaatgtacccaaaggaatagaacggctatgatttgcacatagccgttcctattattttctcagcttatttcttaattacgtaccagtttgttccattagactggagtgtgtagaaggtccagtcgttgtagatggtcagtttagctccaccttccagcgtgccgccggcggaggttatctgtacatcattatcaattttggtatcgtccggtgcggaggcagcgggtatctttttaactgtatagatacgtccggtacaggtggtagcatctggtaataccacgctgcaaacagcgtttgcgcttacgaggatggtattatctgttgcagctaccgtgtaagtgccgccggcagtaacggtggtaatagacatggatacagaaccggttacctgcaaggtagagttgccgatgttattggtatcgccgatgtgtacatttttctttatggaaacttcatcgccaaatttcttggcccctgcgaagctttgtgcagcgttgcttaccaggccaccggtggtagcgggtgaggctacgggaatgctcacggtcacttcatctgccacctgggctactgccagatcgagaccggcgtgacttgatttgaaggtcaggtctttaaatgcgctggcggaaagttttcttttcaccacattgcctgaagtaccgtcacggagtaatactacatcctgcgtggttccgtctgcgatattggtgagcaccacgttattgtcgagctgtgtatttccttttacctggagatcgttatccagggtagctttaccagtaacaccgagggtgccggccagtgcagtggcgccggttacattcagggtaccgctcagggtggaatttcctcctacagagagattgctggcagcgccaggtaatgttaagttaccggtgatagtagagttgccggtgatagtggcgccattagccaatacggttaatcctgttccgaactgacctttcttgaggatggtcagatcttcattgcctgtaacagattgcaggaaggtttttaaaccgtcgaacgactgcgcgcccgtagaaaccgcaccgggatgggtggcatccgcggcgtgcaggatcagtttaggcgctaccgccgggttggtgttgtcgatagttaaaccgtcgttcaccggtgtggcatcgaatgcgccgatgatcattgccagtgtggctttatcaaagcgcttgtagtcggccaggctcagtaaacctgcggttacttcaccggcgccggttacacctttttgtgtggcgatagtgagtacgtgtgtatctgttccggtagtagtgaaagcgtaatcattgggtgtggccgtaggcgcggcagtggtcagtttctgatcggctgcggttaaaccgttgatcttattgatcgctgtggtaaaggctgtttccgagatggtgcgtttgttgattttgccggtaacgggatcaatcagtagcacatccacgccggcggttaccaggtccagctttttcaggaaggcataaccgttgtcgatcacaaaaccttccacattgtttcctttgagggaaaacggtacgttggtggtggttccgataaaatcgccggtggtgccggggttacccctgaggccccaggtgttggctacatcgcctgtgttagccattctttgccagtagccgtgatttcttacatagaagccttcttcaccggcttttttgaggtagatgaccatcccatccggtggagttaagcctgtgatgcccactgtgtcggttaaacgtgggagtaataagccttgtttgtctgcgtccagatccaggatagcggatttttctatcgtagttggatttttaccgactttcagctgtgcatttgcctttgaggcgatcatgcccacaccgccaaccagcatcacccgtactacaatgcgtagagattttctcatagatatagggataaatattaaatgtcaagcccatctccggcatttggtctttgccggtatgacagtaataaggataaatagattcaattatcgtggtataagggattcatgtttctatataatctaaataatagtaaaaatattaaactgttatagtttgacataatttggattacatagatcatataaaaaactatgctgcaaatgtgacatattaaatctttttaaaaaatgacatgatcataccattttagttccgataattattcactgacggggtaaggactcactatatgtgggtcgtaaaatatggtatcggaagaaatatatgctgttatgggatgggggtgcttaaaataatctagtgcgggcagggaggttaacatgttcatgttataaaaaaagcagcccatcatttctgatgggctgctttggttatgttttgcgtgttattacgcttctgatttctctgatttactcttggaagagttgtttttcagggtaaagatcagcttttgattttccttatccaggtcagctacgaggatatctccatcatgaatgttcatgttgaggatttcttctgccagcggatcttccaggtatttctggatggctctgtggagcggtctggcgccgaactgctggtcgtaacctttatctgccaggaagcctttggcttcgtctgtcagttccaggctgaatccgaggttgttcaggcgtttcagtacacttttcattgtgatatcaatgatggtgtagatgtgctctttcgccagggagttaaagatgatcacgtcatcgatcctgttcaggaattcgggagagaaggtacgtttcagtgctttttcgatcactgacttggtattctcttcttcatttacggctctagcgctggtggtaaaacctacgccggcgccgaaatctttcagctgacgggctccgatgttggaggtcatgatgatgagggtatttttgaaatccactttacggccgagaccatcggtgaggataccatcatccagtacctgcagcaggaggttataaatatccggatgtgctttttcaatttcatccaggaggattacggagtaaggtttgcggcgaactttttcagtcagctgaccaccttcttcgtatccaacatatcccggaggggcgccaatgaggcggctaacagagaatttctccatgtattcgctcatgtcgatgcggataagcgcttcgtcggagtcgaacatatagcgggccagtgatttggcgagctctgttttacctaccccggtaggaccgaggaatatgaaggtacctattggttttttcggatctttcagacctacgcggttacgctgaatggctttggtaactttgctgatggcttcgtcctgtccaaccacggcgcctttaaggtcttcacccatgcggcggagtttttcagtttcggcctgtaccatccttttaacggggataccggtcatcatgcttaccacttctgcgatagcttcctcgtcgatcgggtagcgtttatgcttcacttcttcttcccacattgcttttgcgcgttccaggtcttcacccagtttcttttcagtatcgcgtaaagcagctgcttcttcgaagcgttggcttttcactaccttattcttttcctgtttgatatcttctatctgtttttccaggtcgaggatattctgaggaacattgatgtttttcaggtgaacgcgggcgcctacttcatcgagtacgtcaattgccttgtcgggcaggaggcggtcggtcatgtagcggtcgctcagtttcacgcaggcatcaatggctgcatctgtatagcttacgttatggtattcttcataacgcggcttgatgttattgaggatcatgatggtttcatccacgcttggtggttcaaccattactttctggaacctgcggtcgagtgcgccatctttttcgatgtacatgcggtactcatcgagggtggaagcgccaatgcattggagttcgccccttgcgagtgccggtttaaatatgttggaagcgtccagtgaaccggaagcgccaccagcgcccacgattgtatgaatttcatcgataaacaggattacgtccctgtttttctcgagttcattcatgatggccttcatcctttcctcaaactggccgcggtatttggtaccggccaccagtgcggcgaggtcgaggcttaccacgcgcttatcgaaaagcacgcgggaaactttacgctgcacgatacgcagcgccaaaccttccacgatggcggttttacccacaccgggttcaccaataaggatcggattgttctttttacggcgggaaagtatctgggataccctttcaatttcctgctcgcggccaacaatcgggtctaagctgccactctcggccagcttggtaatatctctaccaaagttatccagtacgggcgtcttggatttggtatttgtctgtttggctttgcttgcgtaactctttctttcgtcctcaaactcttcttcgcccggatcgtcgaattcagatttagggtccgcagattttacaaagcccagttcgtttttaaaagtatcgtagtccacgtcaaattgttgtaagatttgtgtacaaacgttttccttattcttgagtatagaaagcatgaggtgttccgtttccaccgtagcgcttttcagtgctttggcttccagtacggtaacccgtataactttctctgcctgtctggtaagcgggagactattgatgttagcgatattctttcctgtcttatctttaacagccagctctacttccttgcgtaactcatacagatctacgttcaaagcctgcagaatctttacggccgtgccctcgccttctcgaataatacctaacagcaggtgttcagtacctatgaagtcattgcccaggcgtaaagcttcctctctgctgaacgaaatgatctccttaacttgcggtgaaaaattctggtccattgtgagattattaaattatcaaaaacccttacgggggcttgcttatacaataataacgaataattctgacttaagattatcacgctttatgcggaaatgaagttattcctttttaaacttaaacaacttacactttaatagtataagattatttttgtggtgatgcgggtacgttcgtttaaaaatatctacgaagaaaaagaggtttttgttttcaatctcttgcggttatattttataggcgggtccctctgttcaaaatttatttttactaaaagtataaaacaacgtccaacgcatgaaattcaaaattgataccaaagaaaaaatagtcgttttttgtccggaagaagcagcattggatgctaatttgtcagacgactttgtggctactgcaacaggattgccggagctggaaggacgcaatctcatactggatatgacattggtacaaaaaattgatgcaaagggcgttgaagccattttaacagtttatcagcgtatgtatgacactaatttttcctgcgcaatcaccggtcttaacaacactttaacagctgagttgaaatctgcgggagatgatatgctcaatctggcgcccaccatggcagaggcaatagacctcgtaatgatggaagagctggaaagagaattactgaatggattggaataaggatggattgcagctcttttttactcccacgtaagggtgatttaaaaaaagaggcaattgaacgattaaagctatttacatgttcgcagtcacgatattaggtaacaattctgctatccccaccctggacaggcaccccactgcccaggtagttacctgcaatgagcagctcctgctggtagattgcggagaaggcacacaattacagatcgcgcggtaccggatcaggcgcagtaagctgagatatattttcatcagccatcttcacggcgatcattacttcgggctgatcggcctgttgaatacgctcagccttatgggccgtaccgacccgatcagcgtatatgcgccaccggagctggaacaaattatccagctacagctggattgctctggcactgtgctgaagtttgaactgacctttgtgccgcttcaaccgggatacagcggtattatcctggaggataaggaccttacggtaagctgttttcctacccagcaccggatcacctgttttggtttttcttttgagatgcagaaacgcaagcgcaagctgatccccgaacaggccagggcttatgagattccggctgcttatttcagcaaattgcaggatggcgccgattatcagcggaaagacggcaccgtggtaaaaaatgactgggtaactttacccccgcctcccggcaagcggtatgtgtattgtgccgacaccctgtatgatgtaaacttgttgccggtgctgaaggatgcggacctcatgtatcatgaaaccacctacctgcacgatttagagcagcgggcggcagagcgctttcacagcacttctgtgcaggcggcctccctcgcagctgcagcggcggtaaaacggctgctgatcggccatttttcttccaaatacaccgaattacaacctttcctggatgaatccaggccagttttcctgaatacggagattgcggaagagggcgtaacctatattatctaggtttataaaatgaaagcagcagccatccctggtggatggctgctgctttttttatttacattttactgttagtagttcttcagataggctgctatcttgctatacagtccgtcggtaacgggcagcacaggcaggcggaaagtattttccataatccctgcgtaatgcaggaatgccttgataccggcaggattattttcggagaacatcagttcaaatccttccagcattttgtaattgagcgtccgtgcagcgggataatcgtttaacagggccgcgtgtaccatgctggaaaaatcggtcgcaaaatagttggctgctaccgaaataacgccgtccatgccgcaggccagctgacccagtgccagtgcgtcgtcgccgctgataacgaggaaatcctttggtttatcgcgaataatctgcatgcactgcatgatatcgccggaagcttccttcatggccacgatgttttccacctcatgcgccaggcgcagggtggtttctgcagtcatattccggccggtacgggcgggaacattgtacaggatcaccggtttgggagaggcttcagcaatggttttatagtgctggaagatcccttcctgggtaggtttactgtagtaaggcgccacgctgagaatggcagccgcttcatcgagcgggcatttctccagccgttttaccacatcccttgtgttataatcgccaacgccaatcactacaggcacccgcttcgacaccttttcgaaagtgaattttatcaaatccagcttttcatctgcagaaagagtaggtgtttcgccagttgtgcctaaagacacaacatagttcacgccgccatcgatcacgtagttgatcaacttttccaaagcattccaatctatgctttcatctgctttaaagggtgttaccaatgccaccccggtgccttttagttgttccatattgcgtttacgggaaaataaaaatttcgaacttcgaaggccgaaattcgaaatttttattgttatctctaaatattttttatttctcttcgtagaaacccatgcgggagaacttatcgatcctttgttcgatgcgggtatccggatcaattttctttaattctgcgagtgtttccttgatgcggaccttcagcaggtgggccatttcatcgggatttacgtgagcgccgccgagtggttcacgtacgatgccgtctaccaggccaaactggctcatataatccgaggtcagcttcagctcttctgccgctttttccttgaaattccagctacgccagaggattgtggagcagttttcgggagaaattaccgtgtaccagctgttttcaagcataaatacgcggtcgccgataccgatgccgagtgcaccaccggaagcgccttccccgattacgatacagatgacggggacgcggagttttaccatttcaaagaggttgcgggcaatggcttctgcctggcctctttcttccgcttccaggccgggataagcgccgggggtatcgatgagggtaacaatgggcttattgaatctttcggccagtttcatcaggcgcagggccttgcggtacccttcggggttggccataccaaagttcctgagctggcgcattttggtgtttacgcctttctgctgaccaataaacatgacagtttcgccatccaggtcggcgaaaccgcctaccatggctttatcgtcttttacattccggtcgccatgcagttccgtaaaattggtggacattttttcgatgtacgccagtgtatagggcctatccggatgacggctcagctgtacgcgctggaatgcggtgaggtggtcgtagatattctggcgggtatcagcaattttttgctcatactcgctaacagtagcagaaacatccacacctgatttttcaccattttccttcagcttctccagctgatcgtataagtcagcgataggtttctcgaaatccaggaattgcataatttgattaaattggttaaagatcggatgtaaagataatgctgaaaatattttttaaaaaagatttgcttaattgggaactttgttgctatctttgcaatcccaaaacggaggaacacaacggattgggacacaagttcttaggacaaaaaaggaatggatcggtagttcagttggttagaatgccgccctgtcacggcggaggtcgcgggttcgagtcccgtccggtccgcaaaatctcgaaggaacccgcgctagtcgcgggtttttcttttatggtcgattagttagtcgatttccctttaatttccttaaataaaatacttcttatttatttcttagtgattcacccaatggcatatgttaatcgaatgccaggcaattttttgggggagggcatttgacgagtcaataatagtgagagaaagtgataaaaacggtgctgccatccggtacatagaaaagtaaaagcaaagctacaaactacttaacgtattctgtggctttgctcttttgttctcctaacagataaaggtaaccgacgttttaaaacatccaactattagtatctgggtttaaatccagggcgtgggccagatctggagaaacgattattttctcgtccttcaggttttggccgagcctcatacactactattgtctggccagcaactactgaattatttaattgcttaattgcctgtactgcattagaatcgtctggcatttcaacgaatgcaaagcctttagaacggccactgtacttatcataagctacattaatactatatacaactccaaacgggtcaaataaagaccaaatctcatcttcagttgttctatcacttatattacctacaaaaatattcacaaatataattttaattaaatatacatattactgaaaaatagggactaaaaaagaaaaagaagcccaagctaaatcagaagaagccaatgcaactttgctaaagttagagcaataaattgggtattacaggattactctatggggatattacaaatgcgtcaaaaattagctccctgcaactctaacgcccgttaaactaaaaatggttgttggtgattagctaacaaccatttttagtttacaggtaaagaataaaagagtggggtttaaatatttttaccaactctcaatattcacttcacgggtgccactatagaatttaacagacaaattttcaagaccgcttaaagctaatattaaataccttattcttctgcggatcgcttgataattgaaaccatgagctgctccatctttcataacaattagccttatttctcaatcaatacaacgtctgcaaatcctatccgcattgttaaaacacccattaagaaggaggcaaatcacgaacattctgtttggatagctaataataattttttatttctaacactctccttattttcatacagatattctcttacactgcactttcctgctctttttatcagatctttaggcagtatatttttataattcttaatcgataattccattgtacatgtctatataaagtcagaaaaggcaggtaacctattactcaataaactatagaagatctcctgatagaagtacgtgcaaaagacaaccgacaattatttaattacggcttgtatgttgaagtagttctaataaccgataatttaaatataacttttctttcccaacttgctcgctcttcagaaatccgttttcttctaatacctttaaataaccaccaactgtttttagattcccaagcccagctaattccaattgagaacgtttagtatatggtaatttgaaaaggacttcaatgagatctttagaatatatcctcggtaacttttcctgaatttcaacgctcatctgttccattagcctttcaatttcaataatctgatgacgtccttttgaggatgtctgctcaatcatatccagcatatataaaatccacgaagcccaatctttctcttccgttactctccttaaatttgcataatattcatttttatgccggatgatataatcacttaaatacaatgcaggtaggtctaataaccctgtcagctggagatacagtaatatgataattcttcccgtacggccattgccatcaaaaaatggatgtatagcttcgaactggtaatgaataacagccatttttatcaacggatctattccgtcttcagcatggataaaatcttcaagattctttaatttttcccgaattatagattctccttccgggggcgtatagatgatcttttctgttgccgggtttttcaattgtgttccaggtacattgcgaatacccgaattattctcttttataatctgcatgatggaaataaagagattagtagtcagaacgggctttttctgaatttgctttatcccataccaaagtgcatctttataatgtattacttctttagtagcagaggaacctcttcctttttcattaattgacgctctgaataactcatcctgtgttgtgataatattctcaatagcagaacttgcctgagcttcctgcaaatttatagtatcaataaataaagtaggattagggagattggtaattgcaccttttagctctgataaagaccgactagctgcgatggtctttttaaggatagtagtatcctctattactgcggtcggaggtaacaaaggcagatcattataaggaatagatgaattatatggcatatttttccatttaaaaacgcgagtaaattttgtcctcaaaagaagaacaagggcaaatatacgtaattttcgccctcgttaaataaacagaggtaattttcgccctcgttcatatttcaaggggaaatcatatattaatgacggggatctcctccaccccgcaaagccactctttaagagtggcttttttgttgaaaccatgtcagtaatcagacctgcctaccctactcttttaaaggtgagttgcggaaattattaagtctgcaacctctttgggatggcttatatagacactatggcttgcaccttctacttcaactattttcttactattagccctttttgcatacatccgttctaaatcagggttaataatcctatcggattttgctaccatataccaaaccggtttcgttttccaggccggattttgaatgatggcatggaataccacgtcagcagtaggcgtttgcgaatttgccataaactctgcttttgatttttgcaggtcacctgagaaatcagcggcaaacatctttgggttgatgtagtcccagccgccatttcccttgatcagtgatttataggcagccgggaaaattttgccgttgtcagcttcagattcaccatgatccggtgcatgcgcagcaatatataccagtccgctaacgagggaatcattacccgccgttgttattacggcgcctccgtagctatgccctaccaaaatacaaggcccgtcctgcaggtcaattacccgttttaccgcagctacatcgccgtcgaaggtagtcagtgtaggctgggcaatgctgaccttataaccttttttggtgaggatttcatagacctgttcccaccccgagccatctacaaatgcgccatgaacaagcacaatgttttggacctttggggaaacctgggcttgtaactttgcgacgaaaatcgtcataatacaaataaccagcattttaaatgtgcgaatgccacgattggaatgtaggttcatagtatacttttttaaaaatttgtttataaaatgacagagtgccgtcagttttcaattctgttgccggaaatccgacggtgatttaccggttttgtttttaaatatctttgtaaaatgagaggggtgttcaaagcccagttcaaatgcaatttcactgatgtttttctctgtgctccacagcagggatttcgctttgtccaccagttgcaggtgaatatgttccagggtggttttaccggtatacctgttcagcagatccgaaagataatcagcagagaggttcagccgggatgcgaagtattttacatcgggaagtccgtcatcgatcagcgaatcctttgaaaaatagtccagcagcaagctttcaaactgctgaaccaggtcctgactgggtttggaacgtgtgaggaactgccggtcgtaaaaacggctacagtagttgagcagcaattcaaggttatttacgatcaattcctgtgaatgtttgtctatgttttgcgaatactcctgcgtcacgttatccgcgcagttacgcaacgtcttcttttcatcacctgacacatgcagcgcttcattggcatcgtactgaaaaaatgagtatccatggatctttttgcccagtgcggtccggtacagcaaatcagggtggaagaataatccccagccatcatcataagaaatgtaacgctgtgtagaaacagcctgccctggtgcggtaaataccaatgtgccctgatcaaaatcataatgggaacgcccatagcccattgatccttttaactgtttaagatacaccgcataaaaccccaggcggaacacggtttccttttccggaaagttattcctgctgacctgctgcaacggaaggaaggaaactaatggatgcttcggtggagggcagctgtagagcttatgcagctcatgtatggtattgatatcgacgaatgatttttgcatgcagtaacagattagggagccaagtaaatttactaaaaagtgctgaccattttcaaggctgccacctgtaccgccaggcttctgtaacgatgattgtacgtttcataattgtatttcttataatgatttttttattgtcaggtgttaaacaatgaagcagaggtaattttctccttcaggcgatagcacctccactgaccagaagctgctggccgcttacaaatccagacagttcaccagcgaaaaattctgcaacatttgcaacatcctccggtgtgcccatccttcccatgggataaaatgttggtacgatggccctgataggcgcttctgcgtcaacaacagtatggattcctgcaccttcggttgccgtgggcagtatggcgtttacagttatgccccttttacctaactctttggccaatacctgcaccaggtacaaagcagcggttttgcttccaccatgcagcgcatagccggcgttgggcagtccggtagtgctggaaccgatataaataatccggccattgtcggcaacatgcctggctgccgcctgcatagtgaagaatgcgccctttgtattggtgtcaaacaggctatcaaattgctcttcgctaaacgcagtaaccggcacgcctaccaattccaatcctgcatttaccacaacaatgtcaattttcccaaattcctggatggcaacttcaaatagccggtttatttcagcgggctttgaaacatccgctttcactgcaatagcttttacctggtaactttcaatctgtttaactactgcatcggcggccacgctgttacttgcatagttaactacgatatgtgcgcccagttgggcatacctcaaagcaattgctttaccgatgcctcttgaagcgccagtaaccagtgccactttattttttaacggattcataaatatgtttttgagtttgaaaaattgaggaacaaacgcaaagcatgttcctcccgggagctaaataaacatcccacccgatatctcgatgcgttgggcatttacaaagcggctgtcttcggatagcattgatgcgacaaacatgcccacatcgtccgcatttccaagacgtccaagcgcggtcatgccggcaatttgctcgcgatggctgtcatcaccttttccaccaccaaattctgtatcaattgcccctggtgcaacactatttacacggatcttccttccggcatattctttggcaaaataccgtgtcaagccttctatcgcggacttaagagcaccatatacggcaacaccaggaaaggcgaagcgggcaagcccggaggaaatattaataacctggccaccatcaacgatcaatggaatcagtttttgcgtaaggaaaaacacgcctttaaaatttacgtccacaagttcgtcgaactgttcttcggttgtatccttgatgagggttcgctgggatatccctgcgttgtttacaagataatcgaagttctcccggttccattcctgctttagcacctgcgaaatctgattggcaaagccattaaaggagctggttttggatgtgtctaattgcaaggcaacggccttacctccgctgctgttgatggtatcagcaacagctttcccctgatcggagttgctgttgtaagtgaggataacgtcaataccacgttgagcggcatttaacgcaatactttttcctattccacggcttccgccagttacaaggacaatttttgatgctgttgttttcatctttttaaagttttaatttatatagcaaagttcaacagcgcggcgtaaggctacttatacatttccggacaggttttatacatttcggagatgctgggaataatgtagatatttcagtgaaaatctttactaacaattcaacacaaaacgcctcccatcagcgtggctatgcagactggtaattgtatgaataagtcactgcattccctgcaggaatggcagaacgaagtagtgattgtacgacttaaattccggctgtaagatttagaaatgaagagaattaacaaagctccggagtaccggaagggtaggcgcctctgacgattccaattagtttagttgaacacgctgaattaaacagctgtaaaataaatgacagcatccacgaatcgattatcgggtttttacctgatcctgtttgatgtaatttatatcttcacattaagttcttttaaagaaaaactcaaagattcagcgctatagcaagcccttttactggtgccggaaaatcgcccactgccgttgcggcgcctgtttccaggttaatcatatagagctttgttgtgccaccctctgtaaataacgcgtatgctttatttgaagcgccgctgatgtcaaaaccattggcttcactcgctcctataccaagtcgccctagtaaaataacagctcctccgtttggtggatcctgcctgtaaagtgagttgctcgcgtagcctatgtcgtacaatacagtgcttgccgatccggcggtattattgctataagccacagcagatataccactgccaggaggattaatatcagtgtctttagcgactaatgtgccgttttccggatgtatgcgcaggttctggcctgtgttgctgacgattcttaaccggtctacggatggattgaagtccactccaaaagcagtaccacttagtacttcggcgaaggggctcgcgttcaccggagtagccgctccggtggaagtattaatccggtaaagacggctggtgcttcctactgcatacagctggttgttggcagggcggatatccatgccaacgattgtttctccaggcagaagcccggtgattggcatggcagaagcggtaccaggtgaatgcaggttaaatgacagcaggttgtttccgcttgttgcgaaggcgttgataacaggcttatcttcctttttactttttttgcaggcaatgttggtagtgaggctaaataatcctaatgctactaaaatataaagtttcatgataggatgttttatggggttaatatctacataaaagtaataatttttgaataaactcttatttagtccatcaaattgcctcattgctatggcgccggggcaaatgcgccattctggatccaggcaagccaggctctcttaaattcttcgtggctaacaggtggcaatgttcttccttctccgggattccatccggccagtaccaggccatcactgaaaagttatcacctgaaaggtaagcaggtgattccctttaatacgaacgggggtgatggtatcgggagcagttttgacaaagtgaaagaactttgccctgatagtaaagtgcccgaaggccttacgatgaccagcggatctgaacgcgatggtaagttgctgttattgcaggcaataaagcagtggaagctgaaactgaagtggtaaaatggttaaggaaaattaatttcataaaatgataggaggctaaagtcctttcagtctcaacacatctggacacctcaactgttcattatttttatccagtctttgactactttctgaagatttgccttctgctttttcacctcctccattgaccggaatttggcatatgccttacctttaggtccgggttcgagaagaccggtattatcatttaacaactctcctttgtgaaaaatcactgctacaaaatcagttatccttggatttagtgttgccatgggctctttgtagtcgaaactcgggccgccccattttacatcttcttctatccccggactgacttcgcggattatttttactaccgatgctatttcagcttttaaaggatggttaagcttacttaaaaattcgtcaattttgtttgctttgttcatgattattagtttttcgatctggtaaaaatgaaataatgtgctaaaaacaatacctgttatcgatgagttgattaactggtaccacaaatatgaggcgcttgttttttttaaacatttacatttgttgaggaaatgaaaacgtttttgtgcatcctcaacaaatgttgaggatgcacaaaaatcagcgcgttaaactattttttagccgaaaagatcctgctcacctgggttggagtaattcccagatatgaagcaatgtggtgttttttgatgcgcttagtcaggtgggcatattttttaatgaagtcttcatacagatcttgcgacgcatgttgcctgaaaccaatttcttccggttctttttcgattatccaatgacgttccatatagtggatgtaaaatgccgcgatatccggatatttcagcgtaagtgctttaaataatccaaagtcatattcccaaactattgagttttccaatgcctggatagtggtcacacttggggttttgctcaaaagagaagttgttgatgccgcaaaataaccttcagaaaagaaacgtttgatataaatttttccattttcatctgaccagtactgagaaaataaaccccgggaaacaaaagaaacattccttgcaatatcccccgctttcaccaggaaactgccttttttatattcttttcgtttaagaatttgcatccatgcaaattctgcttcgggagttagtttctgataactgtttatttttagaaagaattcttccattgtattgaaagtagatgtcttgcttaaagataaattttctactcagcacttttacctttttggggtataaagtttaagttctgaaaatcaatgccttaaaataaaacccattgagaaagcagtaagtttgttacccccaggtgtggttccgtccggtccgtaaaaatatttcttcattccggctacgtagtttgtcgctcacaaacgtattagttatttatcaaccaatttactattctttcacccttcaattttaatacatgcgttgaagcagtatttagtaagaaaaggaaaaggggcaattttttttgacgaaaaatttgtcctcagggcgattccgccgggagctcaccgttgtctttaagatcagccatagtcgccattattaaaacctgatacaattattttatagccgcgtttttgaaacatgtatcgtgtccagcctccggacaacaggtatatccaaacaaacagaccaggataaatttaaaacaagcctaataaattccactatgaacatgagagcgatttacactttactactaacaattttttatctgactgcttcgcagggagtacatgcgcaagcgtacacctggaaccaggtccggataggcgggtccggttcgttgccctcttttgtggcgcaccctatggtacccgatctttatttcatcaccactgatgtaggcactccttaccgatggaataagaacctgcagaaatgggagcatttaatgctgttcaaaaaaataccagtcaactactggaactgggaagttaaccagcgttgcggcagcattggcgtagatcccagtgatgccaccggcaacattctttatgctaccgtggaaaacggcgccggttcggcgccgggcaaagggtcgagctcaatgggtactatcatgaagagtaccgacaggggcgactcctggactgacctgcaggttcctattgttgtacaccctaacagcacgcagacttacggggatcgtatacaggtggatccctccaatagcaatacggtatgggttgttaccgaccagaatggcgccctgaaaacggataatgccggcgccagctggtcgcaggtaagcgccatcaccacgcctggtaactgctcctttattcttttcgacaaaagcgccggcaccgtttccataaacggccagaatgttagcaagcgcatttacatcggccggcctacaggcgtttgggcatcagatgacggcggtgtttcttttacgctgatgacaaacagccccctgtaccctctccgggccgttattcacggcgatggcaccctgtacgtatctgccggaaccgagaatcaaaaaaaaggcgtctacaagtataagagtggcagctggcaggacgtgtctcctgtaactttagatccagatccggttaatagcgacagatacttctctaaagtggcggtaaaccccgccaattcaaatgatattgttgtaagcacccgcggcagctggcaaaaagatccttattatatttcaaggcagggcggcgccccgggctcctatacccagggaaagatcacccgcgataattcggaagcgccgcattcggcaaacgacgggttatattataattcacccgggcataatgctgctgcttttacctgggatcctttttacccgaaccggatatggctgaacgatatgctggacgtgctttccacagataatatctttgacccgatttccaactggaagatccgcgtagtgggcctggaagaaattgtggtaacaggccctatggcagctcctccgagcggcaagaacctgttgctcaccgctactgcagatgtgggaggcgcccatcaccgttcccttacagaaccattgaaccagggcgctgtttccggcaccgctctgcattacggcatcggctcagcgtttaacatgcagggagtaactttccagtataccgaccctaattttgttgtccgcgtaggctgcgacggccctgcggctaataagattgaagcatcacgcgcgggttactccaccgatggtggtgatacctacaccctttttgggaaatcgcccggtttgcgtgggcgtgtagccgtatccgctaatcggagaaatatcctctggctcacccaaatagatgttaatgatgctcccggtaacgtttactggtcggaagacctgggcactacctggaccaaatccaccggtacttcttcgggcatcttacccgctggtccgcagttcaacctgtatcccgggcaaaaccatctcgtagcggataaggtaaacggcgattatttctatatctgggaccgcggttctttttatgtaagcaccaatggcggaaaatcattccagaaaacaactgccactggtcttactgcaaacgccggcaacaacaccaatggctcttcttatgccactacctccaacattgaagcaacgccaggaaaaacaggggatgtatggatcgcattttatgatgacgcctatcctcaatacgccgccctttaccatacctcagacactggtaaaacattcagtaaggtaggtggcgaaaatttcaagcccaaatggatagctgctgccatgtcggacaccacggccaatgcgcacctggctttgtacgccaccgcccagatccttcccatcaatggcattacctacggcgccttccgctcagatgataccggccgtacctggaccaccatcttagaccgggttccaggcgtggtgcagaatattacggcagacaataaaggaagaatgtttcttgccatcagcgggaatggcatcttcttcggctccccggtagccggtcctgttcagtcggtagaaatagtcaatcccgcatcagacactattgtaagaggattctccgtgaaactgggtgcaaagctcacgcccacctatcccaccaatcctgccattacctggagctcctcggataccgccatcgctaaagtagatcaggtcgggaaggtgagcggcattaatgcaggtaccgccactattaccgttacatcggtcgatggagggaaaacggatacaagacagattgtcgtcgttcctcccactatatccaccggtattacgatagacagtgtgacgtatggtactatgaatacgcccaagcagcttatcgctactcttgtgccctcaaataccactaataaaacgctgaactggtccgtagcagatagcaccattgcaaaagtggatgccaacggcgtggttaccggcttaaagctgggcactactaccctcaccatttccacagcggacggaggtgctactaaaaccgtacagctggtcgtgaacaccattgtaacagccatcaatgcaggtacaacggccaccacgggaagcccggcaacgccacttcagaatacggcagtcggtcaatacatacctgaagggcccaccggaaccgataaactatggcatgcaggatatacctggagtggtcgcaataccgcaacgatggacctgagccaggtaacatcgcctgctccccgtcccgtatatgagtatatgcgcatcggcaaatattcgtcgagccagctgcgttactttttccgcgacctgattcccaatgccaactattcggtgcgcctgcattttgttgagccgagcgatggagacaaagctaaccgggtgtttaatgtgaagaccagcggcgacagtctcatcaacttcaacatttaccaggcggcaggcaataagctgaataccgtgatcacacgcacgcttcaggcaaaagctgacaacgctggtgtaataacggtgatgttcattccgaaaacgggtaccaacgatccttacagtgcttctatatccgcccttgaggtatctatcatcccgctccagggaatcagcatcaattcagacagcagtaatctctatgtaagctataaagacacgctgaagctgaccactacaccggcaaatgccaccaaccggaacctggtctacaaatcttccaacgacgctatcgctacagtagatctgaacggtgtggtaacaggaaaaggcgccggcacggttactatcaccgctacctctgcggaaagtaaatttacggctgcaaaaacctatactgttatctacatacctgttacatccttaacgctggatagcacttcggccaacgtatttgtaggatcaactttacaactgaacgccagcatcagcccggccaaagccagcaataaaggagtagtgtggacatcctcagataccaccgtggccaaagttagtaccaatggcaccatcagcggtatcaaacaaggcgatgcaatcatcaccgccacctcggcagataacccggctattaaagcacaggccaatattcatgtagccaatgtactggccaccggtcttacgttacaaccggccaccgctactatcggggaaagggatacactgcgcgtgaaagttaatttcgtgccggctaatacctccattaaaaaagtaagctggagcagttctaatacaagctttgctacagttgacagtacaggccttatcaccgccattaaacaaggtaccgttaccattaccgtcaatacacaagatggctcaggggcttcagcagttttgccggtaaccgtggtgccgtttgattcctgtggaggaatatccaattatggttttgaaagcggtgttattaactggatagcttataaagagtctgtcgctacagtgggcgccgtgtacgccgttagtggtaaaggccattcgggcgacaaagccgccaccctgggttccactacagcaagcaccgctttgaacataaaagattccatacctgtgagaggcggcagcgtcatcgtactcagtcaatgggttaaagtagaaaaagatgctacgggttatccctggtggtcaggatatggtgttgggtttgtaaataaccagggcgctgctaccggtaccgcttaccaaaaacaaatagataatgtgaccgcataccgcgagaactgggctcagataagagataccattaacgtgcctgatagtgccacagggcttacttattgggtttccaaggtaggattcggtacggtatgggtggatgactattgtatagaagttttaaaaacaaatcaatcggctgtttatggcataaacgcgggtactacgaacacgcctcccggcccgtatgcaaacaccacctttgcgcaatatgttcccgaaggacctaccggaaccgataaactatggcatgcaggttatacctggatacaaagagtgagttctcccgtagatgtgtcatatgtaaccgatcccgctcctccgcaggtatacgagtatatacgtgtgttcaaaagcaatgtttcccagatgcgttattacctgcgtggcctcacccctaacacggtgtatgctatccggatgcacttcgttgaggcacaggacgcagagaaaaataagcggatattcagcatcagagcctctaatggactggacagtcttacagactttaatatataccaggccgcaggcaacaggttgaataccgccgtaataaaaaccatcagggcaacagccaacagcgcaggtttgataacggtgatgttttaccctaaaacaggattgtatgatccttacagtggttcaattgccggtatcgaagtacggaacttaacagcggcagattcactgcaaagtgtaaatcaaaatcaaagcatggtcgcagtgactggcaataaattaagcagcggcgctaaactggattttacaacggatgtatatccgaatccttccggtggcgtgtttaatgtaaaaatgacttcttcctcgaaagcgccgacgctactcaggattgttaataactccggcaccatcatttattctacaaaaataaatgccggcgtgaattaccaggttggtgaaaacctgcaaccaggtatttattatataaatattagtcagggtacacaaagcaaaacgatgaaggtggtgaaacaataattttgtttttcttttaaaaaggagaacgcctgttaacaggcgttctcctttttttattcctttgctcaccggttcaagattaaccgatattccatctgccgctttcttataaaagataattgtttactgtttgctgtacatcgtgatttcactcatgttgatggaattggaattattcaccgtatgcaacactcttatgcggatgtaacgtgccggcggggcctgtgggatgaaattaaatttcatcgcttcatttccgtcgtctcctcttatggcagtggttaataatgtccatcctttactgctcatttcagcagcccatccgggatccgtgcttttcagcgacgtggctgcgttggaaatatccgcaataccccatacttcaaattcggaaggattattacaacagtttctgcccgtttcctctatctggcccaggttatataatttgcccatgtcgaaagtgagggtacgtggcagtgggtcgttggaaccattgtcgtcgctatggaaaatgttgggatatccctgcggacctacgctgccatcccataatttgctgacgcgggtgtccgactggtagatgcccatatcatttggcaggtcgtgttcctggaacaggcttttatcgcaggccaccagtttgtaaatatcggggaaggtatcgtagctgttggtataaaaagtatccagtgcgctttttgaagggatgtaggacgactggtaagtgaccgcctgacccgctttgtaaccgggtaaattaacagaatcctgatcgccggcaatggaggctacagcagccacaccggcggcattggtatacctgatactggtgctgatattaatagtatcaggtatggagaagaacaacgttacggagccgtcgtcacgaaccttataaggcgtagtcgcatcagggagacggttgtgtaatgagcttttataaatattgccgtatacatgcgcattatcaatttccgttacaatagaccggttaccggcggcatcataggaatacaggaaaaacgtataggcgtattcgtttaacccggtgataaggcaacgtaccgtatctgaaggattatgcgaggtagcattgatggttacggaatcctgccggttgttccagaacaacacatacttgctgatgctgggatcggggctgggcttccatcctatagccaggcggccgttgccgggaaacaacgtgatccctgatacggtaccagggtactgcacctctgtattgccgaggaagtcgcggaagtcagttgccttccgtgtacaggctatgaagaagaataaaccgcaaagtggtaagaggagttttgcagttataggatactttctcatctctttatatttttaataaaataactttaaacaataccggtaaaggggatcaggtaagatacgctacctgttatcgccccaaatactgagttccatgatgtgaaagaattcattgctatgcgctgcattggtaacacattcaaaccgcatataccttactttaggcaggttcagcgaaaagttatatccaaagccggcattccagaaagccagatcggcattgttatacgccggtgataccagtccggatggttgtgcaggcaaatgataaacgcccatattaatccatccgccgggcgttgcctgtcccaatgcaggaagattggtggtatccggtaatatttcatccaccggttcatctgcccggccccacatcacccaggtatccggattaccgtatccccagagataattaccatcatccaggcccctgccccagagtgtaaaccggctcagtttagctacctgtcccatgtcgaatgttacccatttaggtaatggcgccgtggtaggataagtagagtgatagccgggccggccgaggttattatcccacatgtaacgcagttcccatccaaagctcgatccatcatcggaattgagcttgtaaacattgaacttcgatttatccatgattgtttcgtagatgggcttgatagtggcatacaccgtgtcggagatattcccgaattcatctgccaggtatattccaaacttcctggggatggtatcatatcccctgatgctgtagttgatattttccaggttggtgtagttctggtttttgatctccatcttctttgtggtggcatcttccgtgatagtcaccaccccgatattatctttagcggtgttggtaacactgatgttgatgccgccaaaatctgcacgcataaccacggtgggcagcgcctgaagatatgtgggggtgccgggatgcaccgttacttttacaggatcagatttcacatccgcacgggtaacggtgtacagcgttaccgtataatcctggctttttgcaaaaccgcctactgcgatggtatcggaataaaaggaagacttggtttgcctgcttttggtatcgttgatcatgtattctgcctgcacatagagtacattttttgagtcgggtaaggtgtaggtgatataagcgccaccgtttttattgatcaccctgatattagaaaccggctgtggttttgttttatcatccgaaattacatcgttgtatccatcattcttcttgcaggaatactggatcatcagtaatgtaaccaccggtatcagcacgcggaatattttatatatagcatccatataaaaaattaaaaactggtttgaaatgatttcgtttacgcatgcctgttatcaccaataaggtgtttgtaccaggttgggattggtgagcatgtcgtagtcctggataggaaacaggtaatcccttagcccgaataccggctggtatacgttggtgagctggtagaatccctgcgtggtacgttgtttcgcgttccaaccctggaaaggaccgttgagtactgcctgcagttctttccatcttctcaggtcccatcctgcctgtccttcaaaggccagttctattcttctttcctggtggatgatcgctcttaatccttctttagaaccgtatttggtgggattacgggagaagttggaccatgcctgcaccactcccggcaagccggctctttcccttaccttgtcgatatagctgtatacttctgcacccggagcattggcttcgttcaggcattctgcgtacaacagccacagcgctggtaaacgcatgaatggccaggagtaattggtttgcacggatgtttgtccgaaggcagtttgccatggcaccagtttctttggccaatagccggtagcgttataacgggtaggtgtatacgcagcaaatccatttaccgcatttacataattggcgttgttatcgtctgtgttggcagagccaaaccagatgctgccgtcgaaggctacgtcggcatagtaccgggcttcgcggtaaaagttaccgcgggcagtggtgtagcctttgcggatataataccggtgcgcatcatcgccggtttgcactttgtaacggttggcataatcccaggtacggtcttcgttgataggtacgccgttttgtgtataaaacaattccgactgcgccattggaacggagaaattggaatacacggcaaaaccattggaagctgcatcagcagttactcttggggaagccatatactgccagccgaattgcgggttgagggtccatatctgttctgtattccacggatcggtgagtgcaccctgcaaggttaccagttgtttggtagtgtcggacatatgcacgatacctccgctggccctgaactggtagatggcggcacccgtagctacagcagcatcaatagctactttgcaggcggtggctgcgcgttgccatttagtggcatcatacgccaccgggaaaaggttttgcccttcttttcctttgatagatgcgtaatcaggattcccgttaaacaacgggcttgcctgtgtagccagcacttctgcctttactgctttggcaattacggccgtaatacggcctgcttctgcaccggcattctgtattacatccggcaggttgggaatggcctgatccagcaggcttactacataaccaaagcaggagtcaacggattgttgcttcaacctggtttcatctgtaggcgtattcacgggcaaggctacatccgaaataggaatggggccatacatcctgatgagccagtagtgatagtacgctttcaggaattttgcttctgccacccacctgttgcgctggtattccggaaggtccagcggctgatctacgttatcgagaaaggtgttacacatgcggatcgactgccacaggttcaaccccatattataaccatcccagtaatttaataatggattggggctgttctgcaaaccgcgcattacgttaaatccgttgtcgccgcctgcaccaccgagtgtgttcttatccagcaggtcaatcgggaagatcacttcgccggagctggtaaaacccgcgttacgcctcacatccgccaggccctgcatgttggaataacaaccaaacaggtaagcctgtgtttcatttgcgttggcaaatgaactgttcagcgtagcgacattgtccggtgttacatctaagtattttttacaggatactgataagatgaccggcaatactaccaacaatgttcttttaaaaaatctcattgttttatattttttatacttagaaattaagatttacacccaggttgaatactttctggatgggatatgcgaagccgttgccagcctgctccggatcccacagtttgaatttgctgaaggtgagcaggttcaggccactgaagtatacccggaagttggttaaccgtaatggtgcgatccatcttttcggtaatgaataacccatttcaacagactttaaccttacgaaacttccatcgcgcaaccaccaggtgctgctttgttcgttgttggcaatatgcgaggtggataaccgcggccagagggcgtacaggttctggttttcctcggaccagtgattgtcggcgtatacctgcagcaattgcgcgttatctgcaaatggtgcggtggctttcggatcaataaagaatgattcccttgccagtccctggaaaaatgcgctcacatcgaaactcttatacccgaaggaaaaaccaaagccataaataatctgtggcgtggtaggcaaaccgatgggcacctggtcgtcctggttaattacgccatccccgttaatgtctctatacttgatgtcgccgcctttagggaactcgctgccaaagttttgtacaggagaattagcggcttctttatcatctacaaaaagccgttctgccacatatccgaactgctggttaacggggttgccggtggaaaagcggtatgcatatttatactccggttcttcgtaatagcggactttattgtctgttaccgtgagattgcccataacagacaaccacatatcttttgaaaaattctgtttgtaatcgagatgaagatcgaacccttttgaatctactttacccaggtttgcctggagattgttggaggcggaaccttcaataccagcagtaacggggatatatccacgtttgatcaggatattgtaccggttctcgttatatacttctgcggttacattgagtttgttggcgatcgtcatttccacagcgaggttaccttttttggaggtttcccaggttacgtccggattggggtaagcctgtatggtagtacctttgagtgtgaagctattgttggtaccgaaggtagcgcccggaccattcgcgtcatcaggcgttacgctggagagatagaagaaacgctggctgccaatattatcatttcctaccaggccgtagcttccgcggattttcaggcgggaaacaattttggcgatgccgccttcccagaaagattcattggataccacccaggcgccgccgatggtgggaaagaagccccagcgatgttgcggtgcaaatctttctgatccattgtaaccaaagttaaattcaacaaaatactttttatcgaatgaataggtagctcttcctgaaaagccgaggttcctgtaaggtagtgatcctaacaaactaccggcgttaccgtaaagcgtttgctggcgggtacctatcacggtaccgctcaggttactttttccaaagtcgcggttataatccactgcgccctgtaaatagatgtagctatagatatttttagccccttctgaataaccgaggaattcctgtgcttgtccgggtgagctgttcagccagttgagcacataagtattggcatcggggtcatagcttcccactccataatagaagggtttataggagcggctcaggtcaaaataggaatagcggttggtgctgaaaatacctctgaaggtaagtccttctgtgatgaagttgaagtcctggttcagctcaaactgtgccgacatcctggattccgaaaagtttttatacccgtacatcaggctggcatagggattattcagcagggagccatcgttgccataggcgctgccgaataagatatgattggtgttcgcatttgccgcatccggttcgtaataggcagggaatgccaccgggctggtgtgcagcgccctggaatacaggtcggtggctaacccggaggcatcgccggtgataggtcccgtatagtcgttgaagttaccccagaggcgtaccactgcttcggttgttttggtaatctttacgtttacattggagcgcagctggtagttttcgaacttcatgccggagttgaagttgttcacgggatttacctgtaagataccattgtcgcgggcataggatccggcgatataatatttggttacatctgatccgccttgtacgctgaagttggcgcgcttggtggtcgtttgatctttgaacaatgttttcatccagtcgaccgccgggtatacatacggattgctccctggcgctttatcgatagtagctttggtagcgagtatggcgttgggggtgaagtatggcgtagccaatgggttcctggtagttactgcttcattgtattgattcatgaaagtaatcgggtctgccagtttcaggttttgcgtgggtgttgaaatggcatcttccaggcgtacgcttaccctggctttacctggtttgccttccttggtagtaacgaggattacgccgttggcgcccctggcgccgtacagggctgcagcgctggcatctttcaggatagaaaagctggcgatgtcatctacctgtaaacgggccaggtcgttggcgctcagttccacgttatcaacgaggatgagcgggctggcgctgtatcccagggtagtaaccccgcggataaagaactgggagttatctgctcccggctgaccgccgcgctggaaggcgattacgccggccatctgaccggccagggcgttggttaagttactggtggggattttcaggtcctccgggttgacgctggtgaccgagccaaccacggcttcctttctttgcttgcggccgaaggcagttaccactacttcatctaccgaggcgatcacactttttaaccggatgtgataatctttttgtgtggcgcttaccacaaaccggtgttcgataaagcctacgaaggttacctggatggtggcaccgacgggtacgtcgaggataaatttaccattccggtcggtggcggttccactggaacttttgccgtttaccgagatggtggcgccttccagggatctgccggcggtgtcggacaccgatccggtaatcgttacccgggccggtgtttgcgcgtgagcgctgcctgccagtatcaataacagcaggatcaaaaggtagcggggagcggataatgccgttggcaaaacggcagtaaatctcttcttgtagcaagtaaatttcctgaacatattaagagcaattattggaagtataaaaaacataacgtgtataaaatgcatagcgatgcttccggatatcctgcaggacaaacggccatcatagttatacgtggcactcagtaactaatgtaaagggagaaaaaaagtttatttcataacgtttacttcattcattccgtcataacctggaaacctgtaattctatcgtaattaatgattgatgttggtatctcgcgaaataggaatgtgattctgtactatcctatactatcctatagcaaatatatatttttttcataaccgccaaaagaaatgggcaattattttttgcagtgccgcaaaaaaggcacaggagggttaaaccgcaatcaggttaggataaaacaatatcataagaagcgtaaaggatacgtttaacacgtatcctctcgcttaaaaactttataaatagattataacgatttcctcctgataagtacagtggggattatttcccggatcttttcgcgggttaaaacaaaggcagcagccttttcagccatgagtttgaagtcggtggtataagtggtaatgccgtcgaaaatcagttcttttacaatatcatcgttgtgcgagaggatgccaatatctttaccgggcttgagtttcatttgtttgcaatccttgagcatggtccacagctcggcattgttgatagtgaaatagaccttccctttttcgagggtgcctggcaggtattccggttttatttcgcttttgatattaaaatcttttacaaacttcttaaatgcctgcaggatctctatgggggtatcggctacgggccggtgataatacaccatgcctctatattgcttgatcactcctgccagggcagaaaaggctttgtaggacgactgcttaaactcctgcgccacataggagtagtcaccgggaataggctcatagcggtctatcatcaggaacttatccatcggcaatgcgccgaggataccggcggttttattgtgcgggataggcgccaccacgtacatgccatacttgccttttatactgttaacgatactttgcagtacttctatattattatgatggaagaaaatatcgatatgcacatccttgcctaaaccagcgcgaaaggttttatagaacatttcctggaaggcatcgaaggcaaacaataccagggcaatgcgcaggtgctgtttgatattcacattggccacgaaaaaaccaacccggttcctcggctctacaattcccctgcttaccagctccttataggctttcgcaattgtttcccgggcgaaaccaaactcattgatcagttcattcacagaaggcagcatatccccctgtgccagtcctttattttggatagcatttaaaataccattcaccaattgttcatgcttggataatccgctcactgcctccatttcataaacctgttcaaatacgtggttcataccgggttaattaaattgtcactgttgaatatgtatttccggaaagcaatgctgctgtcctatcctataccaacaaaaatagcattccctttttatatctcctgaagaaaaaatccgttaaaagcctggctttatattcccatcgatttgttatattcggtcaatttcaacaagatggcaaaaaaacacagttttggccctgaaattatagaaggccatatcgacgaaaatatgcttaccgccaaagtgaagctggcggctattcccgaacctgtttccctgatgatagacccggaaacggttagtacggagccggacgactttacctccctggtggaagcaacaaagaaactggtggcctacctggatggtgggaagtttggagaaattgttgacgccgttgcaaagaaaatcaacgaaagcgcctatgggcagcaggatgtaccgccttcggctgatgagttaaccgccctaattaatgatctcaccttaatgggcattgaagtatttccggagggtttcatgcttaatttcatcgctgaaaagatctttccggggtcagagatcaaagtacagctggaggaggatttctctattgacgacgtatccatttatgactaaataaaaaatgcagatatgcagttaccaggtaactgcatatctgcataacatatccggcaattagtatcccgggttctgttccaggttagggttcagatctttttcccctaccgggatcggccacaggtagtcgcgcagtttatcaaacgtgcgggtttcaatcttcttaccattgtagttttcaataggtgcattcatcacggtttcagcggttttccagcggcggatatcgttgtaatacaatccttccccggcaaattccacgcgtctttcatgacggatttctgcgcgcagcgcgtctttggataaagaagtggaaatatgcggcattttcaccctgtcgcggatcttgtcgagcgcagcgaagatggtagcatccggtccgcttacttcgttttgtgcttctgcgtacatcatcaggatgtcggcatatctcaatacgataaagttgatatcagactggccgtctttcagatccgacttatcttttggcggtgcaatactatcataaaggctatacttcttcatgccataacccgtaatagcaaaacggctggcaggaataatggcgccgcggtacatatcggtcggataggtgaaggtaccgtataagcgcggatcacggcggagatacggactatctgctttatatcctgaagccggatcagtgatgggcaatccattattcatgtaataggttttcgccaggtccagcaacggtgcgttggtgttgtattgcgtacagatcaggtcgaatgagctgccctgctgcgggaaaatatactgcacatcaaaaataacttccttgttattttcattgggctgcaaaaacaatccgcggtaatcggcaaagagtccatagccggtgccggccagccccataacgctataggcggcatcggctgctgccttccatttcgtcaggtcgttggatggattcagcaacgggctggcttcatacaacagcaccctggctttcagcgccatggctgcgcctttggtagccctgcctacatccgctcctgtgtatttcactggcagaagcgtagcagccatatccaggtctttcaacacattggctaccacttctgcacgtggcgtacgcggtaacttagcctgggcggttctatccggcggatcgaggattaacggcactgcaccataataattttcaagtataaagtaataaagccctctcagaaaatatgcttcccctttcatcctcttccggatgtccgcctcaattgcagttacttcatctaccttcttcaaaaaagtattgcaacggccaatgccgctgtaacaatcggagtaacgggcagtaacgataccaccggtactcgacatctgggtaccacgggcaatggaattaaagctcatggcatccgtttggttgtaggcgttgggagaaagggtttcttcccaaagcgcggtggcattgttggaggttttaccaccaaatatgccctggttgcgcaatacagagtagcagcctacgaggccggcgttggctgcttccggcgtttgccagaatgttgattccgggtaacggtcgtgcggagaagtatcgagcaggcttttgttgcaacctgcagcaagaagacctgtgcaggaaagtaagagatatatctttttcatactagtcataatttggatgtttagaaggtaacgttgataccaccattaaaggttttcagcattggataagtatacaatgttgtttgatccaggatagattccggatcaaaatccttgtaacgggagaaggtgagcaggttttcggcgttgataaacacactcactttctggatccttgctttcgacaaccattgctgtggcagtgcgtaacccagctgaatgttcttcattctcaggtaagagttatcccttaaccagaaagtagagcgctggaaattatcaatgctgccggtgctggtggttacaataggcaggcgcgcatctcttttttccggtgtccaggcatcccttgtccattcccaggtagcattggcgccgttgttaaaggggtaagccaggttagcggtaggcagcacttttacaccgccaattccctgaaatgaagcactcaggctgatgcctttatagcctacattgaacccgaaaccataagtgtacttcggtacggatgaagagctgttcacaattacacgatcgtcgccattgatgatgccatctttattaacatccttaaatttgatatagccgggttttgtattggcagattgttttgcgctggcatctatttcagcctggctctggaaaatgccttctgcctgtaaaatataaaaagactcaatgggcgatcctgcctgagtaatggtacctgtaccataaataatttcaccatgcaggtccactacttcatttttattgtaggccacacttccatacacattcagatccacttcgccaatatgatcacggtattgtgctactacttcaagacccgtattatctaccgtacctacattctgtttggcgccggccaggttacctacctgggaaggcatacctacttcacgaaggataccattggtgcgtttcttataagcatcaacggtaaggccaatacgattattccagaaatttacatcaacgcccacattgtaagtattggtgatttcccatctgagtgtagaatccgcatccgcagtttttgcgccgccggaatttaatatgccgccgaaactatagtcttcaccgagatttacggttgcttctgtcgtgtacaatgcaatggcctggctacctaatttaccggcggaagcacgcagcttcagcacgttgatgaaatcagaatgaaagaaggcttctttatcaatacgccagccggcagatacagaagggaaaaacgcccagcggctgtgtcttcccaggcggctggaaccatcataacggaaggtagcctccagcaggtatttgccgtcatagtcgtagttcaaacggccaaaataagattccagcacatcgcgggtaagatttccggaggtagcgttccaggtagtgcccgcgcttaatgcatccagtcgtccatccaggtaaccatacatactggtggcccatgagtcggaatcgaaattgtcataactggcgcccagcatggcagagagattgtgtttccctttgaactggtgtttccagtcgagcgtgttatagaaatggatattcatatcattataatccgttttggctgaccggggcgcagtagcgggactgttccagttgatagccgcgcctgttttcggattaaaagtttgcatacgtggtgtaaagccgctgagcaaaccatcatatttatccacaccaaacttgatgttatagttgatatcgaaaggcagtttatattctgcgaaaacggtggtcaggaagcgctggatctgtttggtctgtaaaccattgtatgccagcatacgcggattctcccagttgttgcggccggctgttctgagccaggagttgccatagcggccatccggcagcgtatctgtgaggataggcaatgtacgggccaggtaagtccaggtatctgtataaaacggcgtggtgtaggttctgtagtaaccatccatggtgatcccggcgcgcaggcgtttggatacttccatggaagcattcaatccaacggaatatttcttttcatggttaccaggtccgaagaggataccgtccctgtcgaggtaaccgagtgataaacggtaattatatttttcgccgctgccggaaatagccaggtcatgtttctggatcacaccgtttttcagggcaatatcataccaattatttgcgggataggtgaaaggatctgtagccattcctttctggtactcctctatatccgcttctgcgtattcaatggcttttccttcattgatgagcgcctgatttttcagtttcatatacgcgataggatcgctgatcacatccggcaggtaggttgctttttgctgaccgtagtaatagctatagttaacgcgggaactgcctcttccttttttagtggtaacgaggataacgccgttggagccgcgggagccataaatggcggcagcagcatctttcagtactgtaacggtttcaatatcgtttggattgagttcatccatggagtactcgataccgtctaccaataccatcggctcattggctcttgcatcggtgctgccaaaagtattcagtcccctgatacggatggtgctgcgatccacacctggctgactgttgctcaggttggcgaatacgccgggcacgccatgcaatgcgttacttacgttggtaagtggctggccttccttatccaccatattcacggtggtgatggcgccggtgagcgtggcttttttctgtgtgccgtaaccgaccaccactacatcgtttagtttctggatatcttcctgtaacactaccagtacattggaagattttactttcacctctttaggcaggtaacctatgaaggtaaatttcaaggtagcgtctttaggcgcggtgagtttaaaagcaccgtttacatcggtggcggcgccgcggctggtacctgccacctgtacgttcaccccgatcagcggcgtgccattggcggcagttaccttaccggtaacgggaatgtcctgcgcctgcagggataagctgccggcgccgatgatcccgatacacagcaacaggaacgtggccggttttaacaggcggaatcgtgaaaagaatttcataagtgtgtttgtttttttttgttagtatactggtagataaataatggtcagagccctgcttcgcgtaatctgtttgggtaatcggtaataataccatcaacgcccagtgctttcagctttttcatttcgttaacgtcgtccactgtccacggaacaatcttaatatgtttagcatggcatttactcaccagttccggtgttaccagcttatagttaggattatagaaaaatggtgtgaagcccagttgctccaggtgctgatcgaacccgttctttttatcatctgtcagaaatcccagtgccatatcaggatacctgcggtgcagtacctgcagcgggcgcatatcgaaagactgcaccagcaagcgttttccaagtggctgtaattgttttaccgccattagtttatccatatactcttccggcgcgggttgttctttaccatctgatttttcggaagattttatttccagcagatagtaaggcgccggcatatgatgcgctttcgtataggcttccacggagtcgatcatttcagagagcagtggtgcgtaagaacgcatgcgctgttgttccggataggccgggtatggtttttccccgatgataaacggccggatatcggcatagttcatctggtaaaaaatatagtccgtgcgcttttctgccgggatatcttttccatccggtgtagtagtgtatgatggcgtaaacgacgcgtcgtggtacaccattacctggccgtctttcgtgatatgcacatcaaactcaatggtattggcgccttccgttaacccgcggtacatggcaggaatggtattctccggcattaaacctcttgtgccgcgatgtcctactttataaaaggaaggatacccattttttgcagcagtggttgttttagttgttttacatgcattaaaggtgcatacagcggctaccgccatggcgcagcctatgagactgatattaaactttgttttcattgcgcgtggttctaacgtgttattaattgcgtatataggtaaacgttatctacttcagtaacaggtacagtgaagcggcgattacagcgccggccagtggcccgaaaacaggtacccaggaataactccagtcgctgtgtccttttccttttatgggcagcagtgcgtacatgatgcgcggacccagatccctggcagggttgatggcgtagccggtagtgccaccaagcgacaacccgatagaccataccagcaacattaccggcatggcgccgagcgaacccaggcccaccggtgttttctccggtcctacttctgcgttggtgaaatagaaaatggtaaacagcaatacaaaagtgccggtagcttcacagatgaagttgcgccaggtatttcgtatagccggctccgtgcaaaacacggcacgctgcaaacctttgtcgggcgtattattaagatgatctttgtaattgagccataccagtgaagtacccagcatagcgcccagcatttgcatggcaataaacaaaggcacatctgcccagttgaatttgcccgcggcagccagtgcaatggtaacagcgggattaaggtgtgcgccgctgtaagggccggcgaacactacgcctatatacaccgccagcgcccaaccggtggtgatcacgatccagccgctgttgttacctttggtttgatgcagtaccacgttggctaccacgccgtttcccagcagcagcaataaggcagtacctatgaattcagctaaaaaaggatacatagtttataattttattggtgagcccatgcttttgcggcatttactgcgcggttccatccattgatccattgctggcgttgttcctgttccaggttgggagagaaacatttgtccattttccactggctggcaatttcttccaggttctgccagtagcctgtggccagtccggcgagatacgcggcgcccagcgcagttgtttctgtaatacctggccgcactactttcgtttgcaggatatctgcctggaactgcatcagcaggttgttaccggtagcaccgccatctactctcaattcctttatgctgatattggcatctgcttccatcgctttcagcacttccattgtttgataggcaatgctttccaatgcagcgcgtgcgatatgcgcggcgttggtaccacgtgtcatgcctacgagtgtaccgcgtgcgtgctggtcccagtgcggagcgccgagtcctgcaaaggccggtaccaggtatacgccatcgttttgttccacgctggcagcgagtacttccacttcagaggaggcccggatgataccgagaccgtcgcgcagccattgcacaatagcgccggcgataaagatgctgccttccagtgcgtattgtacctgtccgtttactttccaggccaccgtggtgaggagattatttttactgatgatgggtgtgtcgccgatgttcatcagcataaaacagccggtgccgtaggtatttttcaccatgccgggagcggtgcacatttgcccgaagagcgccgcgtgctgatcgcctgccacgcctgcaatcgggatctgtacggcaaagatgccgggagcggtttcgccacatacttcactcgattgttttacttccggcagcatagatgcaggaatatccagcatagccagcagttcattgtcccatgcctgggtgtggatattaaacagcatggtgcgggaagcattggtgatatcggtagcatgcactgcgccatgggtgaggttccagatcagccaggagtctactgttccgaaagccagcttgccttcgttggcgcgttcccgtgccccgggtacattgtccaggatccacctgatttttgtgccggagaagtaagcgtcaatgaccaatcctgttttttcgcgtaccagggtttctttacctgctgctttgagatcgtcgcagaaaccggccgtacgcctgtcctgccatacgatggcattgtacacgggcttaccggtttcgcgatcccataccaatgtggtttcgcgttggttggtgataccgatagcggcaatgttaccaccttccaggcccactttcgccattgcttcggtggctacgccgatctggctgctccatatttcagcgggatcgtgttccacccatcccggttgcgggaacagttgtgtaaattctttctgcgccgtggaaataattgcgcctgctttgtcgaagataatggcccttgagctggtcgtgccctgatccattgccataatgtatctgatcatgtttttcttttttcccgtggatttttacgtggatgttgatttcgtttagtctatgccgtaaccttcagttgtttataggtagtgccatttttcaggaggtagtgttgtgccacctgtataaaatccttcacttgtttttgttgccagttcatatccctgttcatttctgcggccataatggcggctgttacgggcgccatgtctatagcggcctgcgcatccaggaagagtgcgcgcaggcgcctcgccagcacgtcttccacggtttgggccatttcatgtttcactgcccatatcacctgtgctttgatgtatggcaggcgtggatgcagctgttctttcatatcgggatgcagtgaaataaatgcctgtatcctggcggcatcgctgccatatatatccagcggtgcgggcgcggatggttgttgctgatacccgtggatatgcagtgattttgttttgcatcccaccggtaccagtccgccggttttgatggcctggtccaccgtatcttctgccattttgcggaaggtggtccatttaccgccggtgatggtgatcagtccggagggcgctaccagtattttatggctgcgggaaatttccttcgtactgcccgtttctttttgcggtgctgccagtggccgtaatccggcaaacacgctgagcacatcttcccgtgcaggcggacggtcaagatatttacctgcggtatttaaaataaagctgatctcttcttccagtgctatgggttccatactgtgttcatcgagcggtgtgtcggttgttcccagcagtactttgttgttccagggtacggcaaacagtacgcggccatcatccgttttcgggatcatgatagcgcttttactgttgaggaaagaagggtccagcaccaggtgcacgccctggctcggctttaccatattgggcgccgccgggttatccagttgcagtacttcatctacaaatacgccggtggcgttgatcactgttttggcccggagcgtatagatttcattggtttccaggtcctgtgtgcgaacgccgcttattttgccggcgctgtttttaacgaggccgtttaccttgaaatagttgagcagtacggcgccgttttcagcagcggtttgcgcgatatcaaccgcgagacgggcatcatcaaactgaccgtcgtgataaacgattccacctttcagtccttccttccggatggtagggagcctgttgatcacttccgatctgctgatatgccgggagcgtccgaggctgagtttcccggacaacaaatcatagatcttgagaccgatggtataaaaggggccttgccaccagttatactgcgggatgatgaattgctggttgtgtgccagatgaggagcattgttaagcagcagtcctctttcgtacagggcttcccgtacgagggcaatatcgccctgcgccaggtatcttaccccgccgtgtaccagtttggtactgcggctggaagtgcctttggcaaagtccgcctgctccagtaataatgtccggtagttcctggtagcggcatccattgctataccaagacccgtagctccgccacctataatgataagatcccagggttgttcaccggcttcctttaattgcctgattgattcagttcttttcattttattcccctataacttttaatttgtttcatttgttttctttgcaatagtaataaaaacaaaaagaaataatttgaaaccaaagtataaaataaaatgaaaaaggtgaaaaagttattgatgaatggaaaagaaataaaaagaaaaatataatatcatattaatcaagtagatagatataaatataatatcactatatattcatttgatttcatatttcaaatttaaaagatcagaatgaaggatattaactacttaatacgtaatcatatttaaccaaatgaaacaaaattgccggatatttgtaaggagcatcttttttcagattatcccgtgtcaacacactttaatacgttatttttatctgatatgtctatgatcaatattgcggaacgtcataagtttattctcggcaaactgcacgagaagggatatgttaatgtactggagctatgtaaggagctggatgtatcgggcgtgactatacgaaaagatctcaagctgctggaggataagtcgctgctattccgctcacacggaggcgctacggtgcataatccatataccatggacaaaccggtgaatgaaaaggagaatatacgccgggaggaaaagcaactgatagggcaggctgccgctgcactcatcgtaccgaacgatgcgatcatcatcgcctcgggtacctctgtgcaggcattggcaaaaaatattcaacccaaagggcatcttaccgttatcaccggcgcgctgaacgtagcgctggaattattgcgccggccggagattgaagtgatccagcttggcgggcatctccgtaacagctctacttctgttaccgggtcttatgcagaaaaaatactggaagatttctcctgtagtaaactattcctcggggtagatggtatcgacctggagtttggtcttactaccaccaatattatggaagcgcacctgaaccagaaaatgatggccactgcgcagaaaaccattgtactcgcggattccaccaaattcggaaagcggggcttcggtcgcatttgtgccctcgaagaaatagatgaagtgattaccgacagcggtatttccgaacatatcgtcaggaaaatggaagatatgggtgtgaaagtaacggtagtgtaagaggaagaccgttgtcttcctcttttttttatttaatattctgcaaacgttccgtctttataacaccataaccactgctcgcccggctccgcggacgatatcacgggatggtccgtttgatgataatgctgcgtcatgtgctttgacggtgaatcatcgcagcaaagcgtaacaccacaggtttgacaggtacgcaggtgcagccatttaccatgttgtttgatgcattcttcgcaaacatgctcggcactaacctttacttcggttattgcttcaaggtgtgaacataaagccataaaaaatattttaaacttctgccaggtacttatgcaccaggctaatactcatggagccctcccctacggcggaggccacgcggctcatagcgccggaccgtacgtcgccggctgcaaagataccaggacagctggtttccagcagatacggttcgcggttgagcttccagagcttaccaaaataatcaaatgatttcatttccctgccggtttgcacatagcctttttcatctttgatgatgagatctcccagccaatcggtgtagggccttgcgccgataaaaatatataacgcatccgcaggcacttcttttacttcctgtgtttgcaggttttctatcttcagcttttccagccggtcggtgcccgaagcctctactatttcactgttgttcagaatactgatattgggaatatcccggatctggtctatcaggtaggacgacatagttgcattcagattttctttccggataagaatgaatacctcctttgcgaactttgacaggtacaccgctgcctggccggcggagttaccacctcccaggatgtacacgctccggtcgcggcacgaggcggcttccgtggtagcagcgccataatagatgcctgccccggtgaacttttctatgccaacggtatccagcttgcggtaatccacgccggtggtaatcacaacggcgcgtgcatttatttccgtaccattttccaggcaaacaattttataatctgctttgagcttgatttctttcaccgactgcggcgataaaaactccgtaccaaacctggtggcttgcgtaatcgcgcgccgtgtgagttctgccccgctcaatcccgaaggaaagcccaggtagttttcaatacgggaactggtacctgcctgtccgccgggcgcatgacgttctatcagcagggtttttaatccttcagaagcaccgtatacagaggcggccaatcctgccggaccggcgccgatgatcactacatcatagatctcattttttaaggtaggattcagtccgattttcgctgcaatatcaatgatcgcaggagccgtcatcacttctccatgctccagtattacaacaggtaaagcggatgtatccaggttattcagctgcaacagcaattttccttcgtcgctgttagcatcaatggaatgatagggaatcaggttgctggccaaaaattccttaatgcggtaggcatctgacgaaaaaggataacctactactttaatcccctggaattccgggcggtaattggtttgccagtcgtcgagcagatcattgataacagggtacagcttttcttccggcgggtcccagggcttctggagatagtaatccagccgcaattcattgatagcttttatagcagcgttagtatctgaataagcggtgagtaacacacgtttggcggcaggaaatatttccatcgcctgctgcagaaaatcaacaccttccatttccggcatccgctgatcggaaataaagatggccacagtatcattcctgtttttcagttccaccaggctttgcagcgcttcgttggcggaaagggtactcaaaatgcggtatgatttccggtaatacgatttcaggtcctgcgtgatggcgttcagcacctgtctatcatcatctataacaaatattatgggcagactcatatcttctacattaattattctctatgggaaatgaaatggtaaaaatggttttaccgggtacagaagtttgtttcactgatccgcgatgacgctgcacaatttgtgatactacatccagtcccagtcctgttccttttcccaaatctttggtggtaaaaaaaggttcaaatatgcgtgattgtatttcttcggggatgcccggaccgttatcggtaatggtgatatgcacacactggcggtcctttgtggtggctatttccagccgtccttttttagcaggctccatggcatccagcgcattatccacgaggttggtccatacctggttcagctctccgggcagcgcttttatttttggcagtgaggcatcataattttctaccagctccacgtttccttttctgaaccggtaatccagcatggccagcgtgttgtggataccgctatggatatcaataaattgtttatccggctcctggtccatgtaggtatatcttttcacggcgcttaccaggtcgaatattctttttgaagagatctgcaggtcgcctaccatccggttggcttccagtgcgccatgtatccagctgaagatcacatccaggtgcgcggggtcaaacagccggctgaaatcttccagcaccgtggtttctaccccatactccgccagtatttctgctatttctatccgggagatatttttgctgtccatccagtcttcgatagcagtcgttttatcagacaactccagcaccgtaggtgctttcaccggcttgttgctccaccattgctggaggttatcaacaatagcagtggcctgctcctgtgataaacacagcgctgccatctctttaaatatggcgggaatatggctgatattctcaaacagtttatccgagcttctgcaaatggcggctaccgggttattcagttcatgggccaggccagcggataattttcccagcgccatcattttctcgttctgctgctgcgaggaagtggtttcccgcacgcggctcgtcatgatatgcaccagtgcttccgtcagttcgtaatgttgttcaatatgtgctttaatcttttccgacgggcaaatcagcagccgggtatctttcagacacaggccatttcccatggcatttttcacgcgggaaaaaggcagccagccagtgatattatcgtcgttcagttccactatttcccggtaatgcccgttgatggtggcggagatgcgtatctttcctgaaatcacaatgatggtggccaccaccgggtcaccggctttaaacatcagttcgccttccggcaccagcttttcctccgactgggatatcagccactgcagttgttccagcggcacttctttgagagcaggaatactttttagttgtatcgcagtgataggttccatataattagcgctaatggtcagttctcaaatataagctttcagcatcccaaaagcaaaaggccgtccttccgggcgaccttgcttcttttaaccagtaataaagatatgcggctttacaataattcaaccgtatttttcagcctgatatcggcggaagaggcgccaatcatgagatcgaatgtacccggttcggctacccattgcaactggctgttgaaaaacgacagcttctccttgttaatggtgaagtgaatggttttgctttctcccggctgcagctttatcttctgaaaatctttcagttctttcacgggccgggtaacggaagcttcccggtctctcaggtacaactgtactatttcctcgccggcataagcgccggtgttggtgagtttaaacgctacatcgatggtctgactgccatttattttattggtgctcagtgtaagtccttcatatttaaaagtggtgtaactgagcccgtatccgaatggaaacagcgggtcattgggcacatcgaggtagttggaatgaaatttttgggtggggccttccggttgcggccggccggtatttttataattgtagtagatagggatctggcctacgttccgggggaagctcatggtgagttttccggaaggattataattcccgaagagtacatccgcgatggagttgccggcttcgtggccctggaaccatacttccagtaaggaagtagcctgttcattttcggtggtaagggttaatggccgtccgctcattaccactactaccagtggtttgccggtttgtgccagtgcggtcaggagtttacgctgactttccgggatgcctatatccgacctgctggcggcttcgccgctcatttcagatgcttctcccaccacggccactaccacatctgccttggcagctgtggtaattgcctctgtgagtaactgctccggtgtgcgggtatcgatgtctattctttcgccaaatacatttacttttttggcaaagctggtatcatcgctgatgttagcgcctttggcatagaggatattcacgctgctgccggctacctgtttcatgccgtcgagtacaggcactgataattgcgcgtcgccacttacggcccaggtgccgagcatattgcttttgttattggccaacggtcctatcagcgcgatggtgcctgattttttcagcggcaatgtttgccggtcatttttcagtaatacgcaggaacgggcgcccagctccctagcagcctgccttttatctgcgctcagcacttctttggcagcggaagcggtattgcagtagcggtagggatcttcaaacaggccgagtttatattttgcttccagcacccggcggcaggcatcattgatgtcgttcagtgttactttacgctctttcagtgattgctgtagggtggtcacaaaaccttcgcctaccatgtccatatccacacccgcttttaatgccagcgccgataccgtttgcaggttgcccaggccatgggccatcatttcattgatagcggtataatccgttaccacaaagccgttaaagccccattgtttgcggagcaggtctgtcagcagccatttattggccgtagccgggatgccatcaatttcgttgaaggaagtcatgacgctgccggcgccggcatctatggctgctttatacggtggcaggtagtattcatacattttgatgcggctcatatcagtggtattgtaatccctgcctgcttcagccgcgccatatagggcgaagtgttttacacatgccatcacactgtttttatcgtcgaggcggttaccctggtatccacgcaccatggcggcggcgatttttgaacccaggtacgtatcttcccccgagccttctgctacgcggccccatcgcgggtcgcgggcaatgtccaccatcggcgaatacacccagcaaagaccatcggcgctggcttctgttgccgccagccgcgcgctgtgttcaatcagcggtaaatcccagctgcaggataatcccagtggaataggaaaagtggttttgtagccgtggattacatcggatccaaaaatcaacggaattttaagcctgcttttagtaacggccagttcctgcgcctgccggatcttttccacaccaattacaccaaacaaaccgcctacatttcctttgctgatctttgtctccacatcactgcttaccactgagccggtagctacgccaccgccgggtgtaagtaaattcaactgcccgatcttttcttccagcgtcatttttcccatcagcgcactcacgaaagtattcattttcgcgttggttgtttgcgcctgtacctggccggcaaccaacagtatcagcgccaccagcgtacttttcaaaagggtatgtatatctttcatactgtttgttttattctgcttttatcacctttgttctggtagatacgccgttttcattaatggcttctatacaaaaataataggggcgatctttgtccatgcctttgaagtagtaatcattgttgttatgcaccatgatgcagctatacaatttatccggggaggtgccggtataaatattgtatgcgtatgcattatttacgggcgaccatttaatccatgcacttcgtttatccttctccgtgcgaagcaccagcaggtctttcaccgtatcgggcactgcgccgttgccgttgccaaatacccttagcccactgagtgcaaattttccgccgggcatatggatgttctccattttgatataacgcgcctgcaccggctttgctaactcaatataatcgtgcggcacatccttgcgttgtttgcttttatcggccaacatcttccagtgttttccatcttccgaaaaccaaagtatatactggtgataaatagctgtttgcttacccaggaaaggagcatcctgatcggcatagtttacctgcactgcatttacgcggcttactttcccaaggtctgtttgtatccattcgcctttgttgccggtggcggcgctccaataggtttttatgctttcatctacggcattattgggtacatagccaccatatgtggaagatacagcaactggtttgttatagttcagcagcatccaaccggtaaaccccgcgttatcgaaagcgctggtatcagcgccccttgaaatataatgcggatagtcgccgaaagaggtattacaaaacatcacgtcttctttatcgaatccggctggccagtagccgatacggcgctcgaagctgttttttaccgcaattaccatggtagatacatgccaccaaaatcctttattatcctggaacgtagcgccatgacccgcaccacgggcataacccccgggcttatacgaaacggggtctgactgcggcgtaaaaggccccagcggatgatcgcctaccactactccatcggcatagccgctgaactctgttcccggagcgccgtattgcaggtaatatttcccgtggtgctttgtcatccacgcgccttcaatgaaggggtccaggaaagtattatccaggttttcgccaaaccgttgccagccatagcggtcgggctccagcaggtacatttctttcctcgtgcctttcggttgcagggtgctgcgattcatttccacgccatacagtggataacggttgctgctgccgttgtacatatacaaacggccatcgtcatctgcaaagaaagcaggatcccaaccgcctatctgcagcgagtcgatcgcttctttccattcatttcctttgggattagtgctcatccagatggggaagtcgctggtataggtagatccgaatacgagcaacgtatcgcccattacccatgctgcgggcgcacacagttcatcgtacacatgatgatacggcttcaggaatttcctttccacaaaatgccagttgagcaggtccgggctccaccaatatccccattgattggtggaaaacaggtagtagtcgcctttgtaatttacaattaccggatcggcggtagcacggtgtttcccccaggtggtgaagttgggaataggacaatagccgtagtcgatattcaccgggttacaataggtagtttgcgcagttgtatccatacttatgaacaggatcaccagtgcatatatccatcttttcatcatcactatttttccgttgtttcaaaatcaagtttctttagtccctgcttaatctccgggcaactcatgaacaacttccacaacaacccggtgcggtagttttctatcattacgacaatgggtccctggtcaatggccaggtgcgaggatgcataccattgctttgtttcgttgaaagcgtcagtaaagccatactccgtccagattttatcgcccaggtcgtagtaaaaatgtttcaacgcctgcatagaatattcaggcgtgtatgggaacgccgataatgccgccgtgggtgtgatcgtacccaggtcgttttccggcgaatgtgcattatatccgtcgtaggtgtcgctggcggtgagtccccagcaattggcgccatagcctttaaatccttttggattacgaacacagtgttcgcggttgataagcgtatgatgcaggttttgttcccagtaatcggcgtaacggtcttttaagccgtgtgggtttaagcccaggaaagaatagtgcgagaaaaataacggtccgccgtaatcaaatcccagcgggagtttgatcccataaaaggtacggtcgttcctgaaataaatattattcacccagccctggtgatatacttccgggttgatggcatagctgggagatgaagcggccagtacatatgtgataagacattcgttccatcctttgatttcgtggttcatgctccagccgttgttggggctccagtgccagtacagtacattgcgtccgccctgcgtataccagttccattctgtttcattccaggtccagttgatcttatttcgtagctccgtttccgctggattgtcgttgctgaaatactggcgggcgcaaaggagtccctggaacaggaaggatgtttccaccaggtcgccgccatcatctttacggctgaagggaatcgttttgcctgtgttaccattcagccagtgtggaaaaacaccatggtagctgtctgccttccggaggaagttcactattttcagcagccgttgtgcggcagcttcgcgggtgatccatttacgttcagcagctacaatgatcgccattacgccgaagccggtgccaccggtggtaaccacttcatcgccatagtcaaaggatttgttgctgcgttcgcgcgccatacctgacaccgggtgaccaaaatcccagaagtagcggaacgtttgtttttgtaccagttccaataattgttcgtccgacattttttgccggttaactttgatcttcttttgtgccattgccggctgcagcaggaaaaacaaacagccaataaacagtatatacttcattctttttcttttttagagatgtgggctggtaaagccgaggttatgcatacccgtttttatttccgggcagctcatgaacaggttccacaataatccgctgcggtaattttctatcatcactattaccggcccctgatcgatggccaggaatgagttggcaaaccaaatgtgctgaagggagaaagcgtctgtaaagccgtattctttccagatcttatcgcccagtttgtaataaaagaatttcagcgcctgcatggattcctgcggcgtatacgggaaagacgacaacgcagcagtaggagcaattacacccacatcattggtgggtgaactggccgtatagccgttggggatatcactggcggtaagcccccagcaactggcgccgtagccataattcttttccgggttggcaacgcaataggcgtagttaatgcgggtatgattcaccacctgttcttcataatccgcataagtatctttcaatcctttgggattgatgcccaggaacgagtaatgcgagaaaaacagcgggccgcccatagcaggacccagcggcagtttgatattatagtaaagattgttgttgcgcatggcgccgttatttgcccagccgctgtcgtaagtagcttttggtaccggcgtttttgcggaggcagcgagaatataggtaataagacattcgttccatccttttaccggcaggttcatgtcccatttatactcgttgctccagtgccagtacagcgcgtttgcattatctttccggaaccagttccattctactgcattacaaacagcattgatatcatttcgtagctgcgtttccgttacatcggcatttttaaagtattggcgtgcggttaaaagtccctggatgagataggatgtttccaccaggtcggcgccattatcctttgtgctgaaaggaatagctgcgccggtgctgccgttgagccaatgcgggaaagcgccgtgaaagcgtgctgcctttgtgcccaggaaagtggttattttctgtatgcgtgccagtccttcgctgcgggtaataaagccgcgttctatcccggtgatgatggccatgataccgaagccggagccgccggaggtaacggtttcaccgctggtgtttctttcgcgtgcgaggccgctaaccgggtgaccgaagtcccagaagtatttgaatgtttgttgctgcaccagtgtgagcagggcatcatcagagatgcgtggaaacttatcagtggtatcgatagcggttaccagcgacaatgaaacggccgattggagcttcgcattttttaccgacaataaacttgtgcctacactaaccgtataggcggtgaggttagacaatggcgctaccggtttcagcacaagggtactgtcgccatgctcccacgctacattgtaaggcacgttgccaccgcttttactggtgaaagaacaggcggcggccacagcactgcgcaatacggcgtctgaaaaagaaatcctgatggcgggttgtgtaccggtaccataataggaaaaccccgcagacacgctatccacgctcagggcctgaaagctgaaggagggcggcgtaacgggcggaggcgacgtattgtcgcccccgcccttactgcaacctgctgttattatcaataataaacaagctatccatttcataaaaaaactatttaccccgcccttccagtttaacgagggcgctgacatccgcttcttccaatgctttattatagatccttacttcatcgagaccgccggtgaggtagctggcccagtcctgtgcggtggcttcagaagtgagactgggaacggtctggaactgtgaagtaccaaataccattttgccgggattgaggaactggatcgggcctgccccgctcatcacgtgtgtggcgatccttattccatttacatataccttaaaagaatccacaccgttatatgacagggcgaggttggtccacctgtcccatacattctgcacatcatagttgccaagccatgcttcgccctgcgcactggctacgtgcattttcagcaccgccttcgtatcggtactgccattttcaaaaaagatatcgatgttgccccaaaagcttttggtattgctgaggctcagcagtcctacaatacctttggtattctgcgggttgtttacccatagcgtgatcgtaaatgctttgaggccggtgatagcagttcccggtgtgaacagcgcgtatgctttttctgcgcctttaagggcgcggcctttgatgcctgttgtgaaagaggtaccgttgttgtcgcagtttgttttagagacgctgtcggtgaggttgtcattaaatccccagtaggccaccaggttgcccggcgcaatttcagaggcactggtataaccaccgatagacaatgccggtttatagctgtcggcatcaaactttttatagcaggacgacgtgaacagcgtgatggctgccagcagtgcgtatgattgatatctgaagttcataatagttttattagagattagtaacccggattttgtgtcagtgttcctgcgctgatatcaatttcattctgcggaacaggccatagctcatttttcccggccacgaagcctttggcgctaaacagggcagcgcctcttccctggcggatcacatcgaagtagcgatcgttttccattgccagttctactcttctctcatgccagattgcattgcgcaatgctactttatcggtagtggttacatccgggagaatgacggtattgccgccgcgggcacgggcccttactgcgttcagcgagctgagtgccagggcggtattgccctgctcattagctgcttctgcattcatcagcagcacttccgcgtagcggattgcacgaaagttctgatcggcgccttcattgtagccggttacaaacaaacggaaaggcacatacgctttctggttgaacattgggttatcgccggtaggtggaatgagatccccctgcggtgtggtttcccctctgaaaatgatggtggcatctctccgcggatcaccgggttcatactcgcttacgaggctttgcgtaggtacgttgaagccccatccgccgcctacaacaccttttacgccctgtatttgtgagtactgggagttagaggcgtctttactgttcaggatcagctgacactggatttcaaaaacggattctttcgaattttcattggcgatgcggaacagttgctcatagttgggatacagggtataacccagtcccattacctggttggtatagttgagcacatccggccattttttgagatataaagccacctttgcatgcagggcgagtgcagcgcctttagtggcacgtcctgcatcggaggcgggatatgccggcggcagcacagctgcagcttccgtgaggtctttttcaatagccgcccatacttctgcctttggcgttcttggtaaattatactcgctggcgtcaacgggtattttcagacgcaggggcacatcgccaaaggcgcgtaccagccggaaatacgcatatgcacgtacgaattttgcttccgcgaggtagcgatttttcagggcatcgtccatactgatggcaggaatattatccagtacctggttacagaaattaatttcctggtattgccctttccagaaatcaaggatctggccttctgtggcggttactgaaaaatcgtcgtacttagtgaggaagctggcatcggatgcgttacttcccttttccgcgtcatcggaacccaggctttctatcgctatcgcggcaaatcctaactgtttccattcccggaggttagcataaatggcatttaccgctttggtggcatctgcttcatttttccagaactgctcactgggttgttgtccctgtggcggcacatccagaaatgattttccgcaacctgcgatagccagtactaccggtaatataacaccaccggctaaacgttgtatattaagttgaatatttcgtttcataacaagtctgctttattatcagaaagtaacatttacaccaaaattgtaggttgcgtagagtgggtatacgttgttgtcgataccggcttccctgggcttaccgccaatttccggtgtgaatccccggtattggaagaagttgaacgcattctgtgcgtttgcaaatacgcgcaggtttttcattccccatttttccgtcatagtagcggggaagttatatcccagctggatgttcctgatcctgaagtagctgccgttttccacgaagaaagaattgggcaggtagttatcgcggccgccgatgaaagcagaaggataggtattggaagtaccttgtccatgccagcgtttatcataaaaatcttttgtgaaattttcattaccaaagcgcgcaccgaggtttacattgtaaacatctacacctgcaacgccctggaaatcgagggcaagatcaaattgtttccaggtgaaggaggtgttaataccatagctgaagcgaggattagggttacccagcggcacgcggtcgttcgcatcaataacgccatcgggtacgcctttaggtccgcttacatccctgtatttaaagtcccctgctcttgctttcggttgtgcggagttcaatgcttccgcatctgtctggaaaattccatctaccatataacctataaactcacctatgggcctgtcgagcatagtacgggtgctcagtgcgccactggtgagcccgccgccgccgccataaataggatttttaccggataccacgcttaatactttgttttcattatagccgaggttacctccaacggagtaggtaaagtctttctttatctggcttttccagcttactgcaaattcaaaaccgcggttctgaagatcggcctggttagcgatgatagtacctgaattggtacccacagaacctggaatgtttacatcaaaaatggcgcgtactgttttccggttatagtaacctgcttccaggtacaagcggttattaagcatactggcttccaatccaacatccgtacctacgcctttttcccaataggtagtaggcggcactacggagttgatgctcgcgccggtgtatacattaccaccaaaaactgcagtgagataaggatcctgggctactctcaatacggagatattggaagtaacagaggcattgcctatctggccccagctgccacgcagtttcaggttatcgaagaagtgctgttgcttcataaagctttcctcgctgataatccagcccacccctaaagaagggaaataaccccaacgttgatcgccgtagaaccgggaggcgccgtcggcacgcagtgaagcattgaggaggtacctgtttttaaaggaatagttaatccttccgaagtaagaagataccgtgtagatgtctccttcatctgttatttgcctgccatcagtgctgcccagtttcaggtacatatctccctcactgttattcggcacatttggtgcgctggcagtgagcttataagtttgatagcgttgcgcaccctggcccagcagtactctcaggtcgtggtctttaaatttattctgataggtcagtgtattttccacgatccagttgcgggtatcagtattttcacgggtgagtttactgttgttggcgcgttgcgcaatggtagccacaaacacgggcacataattgcgcatcaggttttcgccatattcgccgccgatgcttgtatgaaaagtaaagtgtttggcaaaccgcaggtcggcatataaactacctgtaacggtttgttttttagtgaactggttgaaaaagtcgagggttgcctgtgggttgaagttcgcgccttcaccgaggttataatcgttcggatctccgtaagcaccatcggcgtaatgtaccggcaccaccggacctgcactgtacaactggcgccagataaagtcgggaacgtcatttgatttattggcagacgcagtaatagtataaccaatcttcaggggttcaaatacctggaagtcgttttgtaaccgggcagtgtagcgggtaaagtcgtttgtatttaccaaaccttgctggtgcagataacctatggagaaattataggtagatttttctgacccgccgcttacggacaactggtgattggttaccattgcattccgcagggtttgatggtaccagtcggtgcctcttccaaactgggaaggatcatcgaacaacggggctttatcattacgttcctgcagttcatttaccagggtggcatactggctggcatccgccattttcacctcgttggttactttctgatagcccacatagccgttataattcacgactggttttccggattttccttttttagtggtgacgagcaccacgccgtttgctgcgcgtatcccgtaaatagcttcgctggaagcatctttcaggatactcatattttcgatatcggcagggttgaggaagttgatatcatcataccacacaccgtctaccacatataatgggttggcgctgccatagatggtacctgtaccacggatcttgatttccggtgctgcgccgggtttacccatattggtaatggttacgccgggcacttttccctggagggcgcttactgcgttattgataggctgtttattgatttcttctcctttgatctggctgatagcgccggtaacatctaccttgcgttgcacaccataacccactactaccacctgttccaccatactcaccgattctgccagggttacgttgatcacagagcggctgttgaccggtatttcctggctggtgaagccgataaaagacaccaggagcgtagcgttttccggcaccgtaagcgtatatgtgccatccggccctgtaacggttccgcgggaggttcccttgatgctgatagtagcgccgggcaccggtgtattgccatctttactggttactttaccggtaattttgatatcctgcaactcccctgtgttagccatgatgaccaccaggttgttctctatcactttatatttcaggccggtatcgttgagtatttcgctcatgagatcagccagacgtgtgttggtcacatccacatccactttcttcctgatatccttcaatgcgttgttatagaggaaccggtattcgccttgtttctcaatactactgagtaccttggcgatctccgtttctttgagccggagggttatcgttccctgccccttcgcattggcagatacctggagcacacctgccagcagcagtacggcggtccaattcataattaataagacttttttgaaggcatgggaaggtcgcttcgcagttgttagcgattttttcatacttttagatctagaggtaataaaatggaagccagctgtttttcacgattggcgaagcttcctgttatgcttcagggggaaatgttggcgcatttccctttttagttaccagcagctcaagacgaattaaatctgtttccttttttcataacggaaatattactggttaataataatttcagtaccgtggatggtataattaaatgcggcagtcatttgtaatgcctgcaacgcctgttgaatattttcctgtgcaaatacgccggtgaaccgcagctcttctttctttttatctgcaaactgaatagttaccccataccagcgttccatgcgggcggccagcgatgcaaatgactcatcacggaatacgagtttattttccatccaggaagtttctacaatggcatcttctttttcagcatagtaagtaagatgttttaccgccatcaccggatcattggtttttaccgtgtgtaaagagtcatctgataccaggattttctctgtgggtttcaggatgatccgttcaccggggcggctggcgagggaagcttcaatgctgccctgcagcagtgtggcttctgtcattttatctcccggataagccttcaggttaaaccgggtacccaatactctcacatccatgcgggcagtatggataataaaaggataatctgcgtttttagcgatatcaaaaaaagcttcgccgctaaggtttacttcgcggttgctgttgccaaaatctttgctgtaggtaagtttactgccggcgttgagccatacatgtgagccatcgggcaattgtatagaagtgcgggaaccgttgcgggtggatacttcgctgatggccggtgcatgtaccgcttttcccgcaggccaccaccaggtggctgctgcaatgaggatgccggcaactgcagcggcagccaggtaacgcagccatggacttcttgtccgggtttccagctggaaaatggcagactgttgttcttctgcagataaaccaatagctatccccttctcctgcatacggccaataagacgggtatgcgcgtcctctccttctgccctgtcggccggatcaggcgtggttttccagatatctgtaatggcttccacgggaaagtgaagatcagggtaggcacgcaataaaccttccagctcctgcagttcttctgcagatgcttctccggccagttttctgccaatcaattcccatacgcgcttattattcataacgtttcgatagctactctgtatataggtaccatttgaaatcaatatctactaaaggaaacaaaaatattttccgggcggggtatcagcgggaggatttcttcaactgcacattcaataccctggctattttagcgagggcaacggccagctggttatcaatggttttaacggatacattcaggatttctgctatctctttatatttcaggccatcttcacggatcagcttaaaaatgatcttgcaacggggcggcagtccttcgatggcggcctcaatgcgcgagagcatctctgccgtcagcagcatttgctccgggttctggtgcgggcttgccagctctacagataattcatcaatggtaatcgcagactgcttcctttgtttgagcaggtatttcagcgaggtgttttttacgcttacataaaggtatacctgcaggttattcacattttccagctgctggcggcgctcccacaggctgatgaacacatcggatactacttcttcggctgtttcggcagacttcacaaaagaggtggcaaacttcagcagcggcttatagaagcgcaggaacagttccctatacgccacttcgtcgtcgtatgagctgatacgacgctgccattcctttatttcgtttgcgtggaacataaagtgaaagtgattagctgcttctatggacaaagtaaagaaaaaaaacaatgcggcgcggggcaaatgggggcataaaaaggtttttgcgtttatgcaagtagacaataaggaactgatttttaaatttacgagggctgataccgggaactgttgaaaaagttttaccagaaagaaatagggttttactatatttaagtacttgttttcctattttttgctagctgattttttttagatatgcgtccctataaattgtcttctttcctgatacatttcaaagaaaggaaaccagctatagaaagttgaataagaaaataattccttttactgttaaatcatcatgaaagcaataggatttactattctcattgttattttctcatcctccagctgtgcttcacagaactttatagccaatcaaaaaaaacaaaacaaaattgtgaagaaaacaaagcgggccgactcttctccatcaccgatattgacctaggtcaatatcggtaattggctgagctctgctttatttcaataccaccaaatcaaaaggcgccttccggtcagaagacgccctcataaaacttttattctttattcagactttatgtatatcgccttcaatcttctatcgtgcaataatcgcagcaatcacactgctttgtgcgagtgtattttcaacgaagaacattgaatgtaaaggtgttgtggacctaaaatctgtaacaacaatatcgcagaaatttcgcccttcgttaattggcacttttatgtctgagcgaataagatcattaattctaaagtgctcgatactctctttgagcttaatccatttccctctattgtagtcataaactataattttagtttcattctcatgataatagattagatagttcattaggcttatcctttctccactcttcttcacttcaataaccgcccagtccttatccttccaatcaaaatcagggctgatctgttctaaaaaaagccaccttaaagattcgttattaatactgccaggcttaattttccaaatatcagacattgcatcaagcttactttgatataaattcctctcttggtcattattagctgatcttgttgtcatatccaaagctgcaagactggtcttattccaatgataaaataagttataaatatttggctcttgcatattgttaaagacccctaatataaataagtaaaaattgaataaaataatcataatagtgatttttttctaatcggacttaatttcagatcaaacttatactccaatggcttgagcttcggaggaattggataaaatggctgcatccttggtttagcgccctgctctccccgaatccttgagtccttttgcctggtttttacttcttctctagacataggtaaatttattggcaaattagcattatcaggatcaattatcttaggcatttccgacggatcatgttgtccatttttattattctcggcatgtatcaactcatgagcgagtcccacctgaggaggtctacccgttgttccatcttcattaagtattctccctccattgtcttccgggttaaaacgcactatagatccagaccctactttaggatctacagcacctttagaatccgtcgggtctgtttcatttgattcatcacctttcccttcagaaatagtcgtaatatgtttggatgcaattagcccactaactaaggcagttccttctggttttgtgccatcaccagcatttgtttcttctacttttccatcttccctcattaccaaagttgcacttgtcagcttttgtaggctagctagcgccttgtccttaaaatccttatctcctttcaaaatgatatcttcgggtcccattccatccggatcaataaaccttatcggattatcaaaagcataattatatggtgagtgtcgacgcatcttatctgctaaaggatctaacacgtgccatcttcctatctgtatatcatacatccttgctccataatcatataactccaacccgaagccatctccaaactccctactctgcaactccatcccgttatatttcattcgattttccggataattcactcctttcaacgcattggaactaatccccgccatcgtcaacccaaacggataataatagcgtctcctccaataccggtctcaaagaactcctaccgcctaaaaataacggattttattttttcatatgaaagaaaaaaatctgatcggtcataaaacgcggtcaccgtccggggatggataatgtgttactgctgctggttttatattctcatgttgatcatagatttatcgttcagcctatattctgctgtcccccacatcatccatccccggacggaagcgcgattgtacaaaagctgatcagggtactactgctgatgttcacgcagcttattcttccgccgccgggccagcggtataacgctgatggctatattctgtcgccctaacaaaacggtcttccgccccacaccgccattcccccctggccgctgcggcggcagccagagcgcaggccctgaagcgcagcggaagggcctagcgagggcgagccgcagcaggccgcgccttcgtcctttatctcgccgggagcgccagcggacggcaaaatcaaaaatggaaggccaggggggatagcggggggcggacaaaaatggacagcgaagggatggcgggcattaaggcaaccacgattaaaaacagcccttagccagaccgggagctggacgaacggagggcgagggagcgcaaaaagcgtgacaggccacagcgcagcccctggagcgcagcgcaaggggcaagcgtaggactggcgcgcctttttgccgactaagcccgcagtgagaccgcttttccttcaacataaaggctttataataacgggtagggatatatcattttagatagaacccgcactatttcaacggatggtaccgttgcaaggcattttgaagatcatccatgttgctgagtttataacgctgcgtactactcacataccggtgaccagccatatactgcacctgtcgcaggttgtattgttttaaccaatttgttattacactgctcctgatctgctttgcatcgatcactttagcattaagctgccgtaactgccgcatcataccacccacctgatttacgatgttattagcactcgctttgcgtttcttattttcctgtagcaacggaccggttttaaacttattagcttttatataggcttgtagttccagcacctgcgtagcttccagccttagccacctttcattactatgactgctgccactaataaaaaccttaccttcctttaggtaaatatccgttacatatagccgtttcagttcctccaccgttactccctgatggattatcagacctaacataattttctttgaggcatctaccagtaattgcaacctgtaacattcatatagatggatcatttcatcatggcttaacaggctattaggcaaccgccggataatgcctttcataaacaagcctgtagcggggttatcggtacgtttactttccgccaccaggtaattaaagtaatgtcgcaccgggcataagatagcatttatcagggctttacttttattcatggattgcagatgacggataaaatccagcagttccgtataactgataacatcagctgataactgctcctgttgtaaccactctgtaaggtaggccaggtacttgttgtaagtgctgatggtagagccactgtgccccttctgctttagataatcagtgaacatcatagcatatcatttacaaggtgagtataaatctgtgtgctgtctaatacctcatgtcctaaaaaatcctgtatctgttcaaggctcatacctgattgtaacaagtgggtggctatgctgtgccgcagcgtatgtgtgcctatatttttgattaatccggcctttttagccagtcccttaatacgtacatataaactctgcttcgtgagccctctgcccttatttgcgcctataaacagcatttgtgaagatgtttgcaacaactgagggcggccatgttctatgtataaccgcaactgttcgtaactgccaccagccataggtacatacctttccttgtaccccttacctttacgtacatacaataaccgacgatctgtaacaacatcgcctacctcaagaccggctccctcattcagtcgcagcccacaaccatagaacaccgccagtatagcttggtcacgcagacctaacacactatcatctgtagcctcatatagttgctggatttcctgcacggttaaccatacaggtttatttctgctatcctccaaccattccagattaaagcctatcccgcttttactggtttcacgcaggtaacggctaaacagttgtaaagcctgcacgtacttattaatatgtcctgcactatatccacggccagtacggataccggtttgcattttcaggtgatctatatagctggtggcatcggctgccattagctgctgcagccccatcttaccgcgctgctcctgataatacaggaacccacctacataacgcggcaggttatatacgctacactccgcataattaaccgtttcaagccactgcttaaagcctgcacatagtaatacatgctcattactgtgcagtacgtacactgtttccataaacaataaattttaataataagggagggactaacggggtaaaagagaagataaaaattactactatagtctttttcactgtcgtagttgtcgcagtggactaaaacctttactgtggcacctcttactacgacagtaactcactgtcgtagtactgtcgcagtagacgtagtagattttaacccggagagtattacttgtaattgatcatctataaggcgggtaagctccttatattcattgccatctaagataacatattcaaaaccctgacggtgtttataaccgcttacttgacggatataaccgtattgatgtaactccctgatgtaacgctgtacggtacggggttgtaaccggaactgctttcttacctgctggggagtaaaactatcctcccctttattatgaagataatcttttagctgctctaaaaagattcttgtagcctttgccagttcatcacccttactaaacatcacctcctttaacaactcgaacgctgacgcaatatcatccggcgtagtttcaatatagggctgcccgttactatcccgctttacttcccgctgatactgatgataaaaggtaatcgtttctataaacgataataacagcgtcatagttctgcgtggcttaaaaatttgctccggtagctggatacaacctgcataaggattcaccacccgtaccggttgcagcacctgctgtacattcttaaaaagctgtttaatagcctgttcctggctgtagttaacggctcccgcactctggcgggtctggtattccattatacggcggtcctgttccttactagcatccacatataacagcaggcaacggttggcattatcttcgtatagcttttcccgcgtcgtacaaccactcacacttaccgggccgtctaccgtaacagtaaccgttttcaggttgcctttattgtcttttagtgtaaccgttttagtgatacgctttttactttgcagctcccgcaagggatacagggaggtttccgccccgtccagatcctcgatcagcagcagcttatgttttaactcgtcctgcttaaagtagtaaaacgcattttccgtgatttgggtaatctctattttctctcctgcagggatcaggtctgatacccgttcctgcagataggttttaccgctgccactgctgcccaaaaacataatatgcagcggggtatgttgtttgcggctgctgtacaccaggtaagcaatcatacggtttacttcttcccctacaaggcccgacctgcctatatcttcaccagtgcgttttaacagatcaggcgctttcaggtaattaatagctgcttcacgctgtgcgggtgacaactccggtttagctgctggcttaggttgcatactttccatacgctgtacccggtaaccttcaagcccatttgtaagctgcgcaataacggccgtaactacctgctggctcatgtcataggacactgatacctggctgattaacccttgtgtatggctatggttataaaggtccagatgatggcgtaacggcaataactgtttttgcttatgctctattttcagcgtcacccgcaaccggtctaaaccggttattttaataccacctaaaacagtaataagcaatacaccaccatcataaattaacaactccggattaactgtatttagtctggtatcaccctctaccaatacaggtgtagtaagactttcagcaggtacggtttctggtacagtataaaaagacacgggctgcctgccttcgatcagttctaccaggacacggctatcatcatgggattgcagcacgctgtttatatcctcaccatccggaaggtttactgtagtgatctttacacggggaagcaactgcaataacgtgttactgtgttttatagtagctacttttcctgcatcatcaccatccagcataaagataatctcctgtaaaccggtgctggcaatgatggcctgctgatgttccgtagtaagaccattagtgccatacaaggctaatacttcatacgctgtactgatttccgcttgctgtaacagactggcagcatctattacactttctgtaagtattaaccttgtggcagcgggtgtagggtaacagggatataggccagaccgtccggttaaataaaaatgccgctgatcttcattattattgatgctacgaccatataggcatactatcttattttcatgattacgtaaagggaagattatgcactcctttgcccatacgctgtaaccatgtactgcattagctttcagcagcccatactttaccatgctattaaccaggtggtggtttttactttcaatatgtaatccgccactgttataacccatatcatgcagcccgtaatctatactacgacattgcaggtactgggtggcttttttactggcgggtaatgcttttttaaaagaactgaacacctttgccattaacgcttcccgctctaacagatccgcttcattacttaatgatgacgggatttcagatactcgcattagaggtgctacattacctgcacccaacaaggacttagctttcataatagcttcatgtgtgctacacttttctatcagctgtataaacctgattacatcaccggtacctgcattacagttactactaaagcaatgataggtgtctgttttagggtaaagctgtaatgaaggtgttttatcaggatggaacggacacaatacccgatgatgcttatcaggctgtaaaccatagtggataagcacctgaccgatagacaactgctgcttaatgtccttgatttccatgaccaggctttctttttattatcagtgtttcttctcccactgtaatctccacctgatcccccacattaaaacctgctttctctaaccatagcccactgacattgagccacgcaacatagcgcccgcccggattgtagcaatcttttaattcctgatatttgccatgcagctttactagtcggatttgttttgttgccatgtggaaaaatattttatagtactaattggtaacaaaagtaatggattggtttcaattaaccaatacttatttattttgactagcctaaataagtaactaaatttgttaaccccctgcatttacagggtatttaaagtacctttttatgacttttggcgaacacattgctacgcaacgtaagcagcttaaaatatcccaggacgaactggctaaaagagtgggaacatcagcacccattattggacgctatgagcgtggtgagatcaagccttctattgagatggctaaaaaaattgcagatgaactgggtgtgaccgtggactacctgattggcggttctaccagcatggtactggacaaaaaattacttaaacgaatagaagatattgaggccctaccggaagaggagaaagaaaaaatttattacttcattgatatggctatcacctataacaaaactaaaaaagcatactcccgctaaacagcgaagccgcaggcattgcctgcggcttcgctgtttagcggatccagttacgacaataacataagtctttatgtttctgctgtttttatcacatttaccataataagaccaggctttatccttaaacaaaagaaccaaacattctcaactccttcaactttagctggacgttcattattaagctcaatttgtaattccgatttccctttctcacctaaaaacttcacctgagacaaatccaaacttttaccccacaaaatcatagcagcatttatattagatccattaacctgactaatatatgtcccgcctctaaattccataataaatgtatatatatccataccctaatttattaattacttcccttagcttttctactatgattttctcctgtattgtccattttcttcttttcatgatctacagttctctttaatttatccaatgaggccttgtcatcctttgtcttgttgggcttgctttttaatgcctcgtattctttttttgccgcctcatatctatcttttgctgattctctagctttttgattagcatgttgcccattcttacctccaccatgtttttcaggtattgttatggattccattttctccagtttatcagcaacttccggagatacctgaggctttgatttttcatcaatgactttttctggggctggcaatggaactgctgtctcatctttagccgcaggggtcacttctttccccttaggcttagctccatcttttcccactccctctgataacaaattaatagctgtatttaccgtagcataggttcgataactaaaaagtgcaacttcaattgcctcaattactattggaacaagtacaatagggtttcttccatctgggtcaccatatctaaccggattattaaatgcaaaatgatatggtgttaaatcttcctgattattctcaatttcaggatctatttgtaagaatcttcctatttgagcattgtaggtacgagcattaaaatcatacaaatccaaccctgatccatcactgaactcccctgattgcaactcatttccgttatatttcttcctattttccgcataattactccccttcaacgcattcgaactaatccccgccattgtcaacccaaacggataataatagcgtctcctccaataccggtctcaaagaactcctaccgcctaaaaataacggattttattttttcatatgaaagaaaaaaatctgatcggtcataaaacgcggtcaccgtccggggatggataatgtgttactgctgctggttttatattctcatgttgatcatagatttatcgttcagcctatattctgctgtcccccacatcatccatccccggacggaagcgcgattgtacaaaagctgatcagggtactactgctgatgttcacgcagcttattcttccgccgccgggccagcggtataacgctgatggctatattctgtcgccctaacaaaacggtcttccgccccacaccgccattcccccctggccgctgcggcggcagccagagcgcaggccctgaagcgcagcggaagggcctagcgagggcgagccgcagcaggccgcgccttcgtcctttatctcgccgggagcgccagcggacggcaaaatcaaaaatggaaggccaggggggatagcggggggcggacaaaaatggacagcgaagggatggcgggcattaaggcaaccacgattaaaaacagcccttagccagaccgggagctggacgaacggagggcgagggagcgcaaaaagcgtgacaggccacagcgcagcccctggagcgcagcgcaaggggcaagcgtaggactggcgcgcctttttgccgactaagcccgcagtgagaccgcttttccttcaacataaaggctttataataacgggtagggatatatcattttagatagaacccgcactatttcaacggatggtaccgttgcaaggcattttgaagatcatccatgttgctgagtttataacgctgcgtactactcacataccggtgaccagccatatactgcacctgtcgcaggttgtattgttttaaccaatttgttattacactgctcctgatctgctttgcatcgatcactttagcattaagctgccgtaactgccgcatcataccacccacctgatttacgatgttattagcactcgctttgcgtttcttattttcctgtagcaacggaccggttttaaacttattagcttttatataggcttgtagttccagcacctgcgtagcttccagccttagccacctttcattactatgactgctgccactaataaaaaccttaccttcctttaggtaaatatccgttacatatagccgtttcagttcctccaccgttactccctgatggattatcagacctaacataattttctttgaggcatctaccagtaattgcaacctgtaacattcatatagatggatcatttcatcatggcttaacaggctattaggcaaccgccggataatgcctttcataaacaagcctgtagcggggttatcggtacgtttactttccgccaccaggtaattaaagtaatgtcgcaccgggcataagatagcatttatcagggctttacttttattcatggattgcagatgacggataaaatccagcagttccgtataactgataacatcagctgataactgctcctgttgtaaccactctgtaaggtaggccaggtacttgttgtaagtgctgatggtagagccactgtgccccttctgctttagataatcagtgaacatcatagcatatcatttacaaggtgagtataaatctgtgtgctgtctaatacctcatgtcctaaaaaatcctgtatctgttcaaggctcatacctgattgtaacaagtgggtggctatgctgtgccgcagcgtatgtgtgcctatatttttgattaatccggcctttttagccagtcccttaatacgtacatataaactctgcttcgtgagccctctgcccttatttgcgcctataaacagcatttgtgaagatgtttgcaacaactgagggcggccatgttctatgtataaccgcaactgttcgtaactgccaccagccataggtacatacctttccttgtaccccttacctttacgtacatacaataaccgacgatctgtaacaacatcgcctacctcaagaccggctccctcattcagtcgcagcccacaaccatagaacaccgccagtatagcttggtcacgcagacctaacacactatcatctgtagcctcatatagttgctggatttcctgcacggttaaccatacaggtttatttctgctatcctccaaccattccagattaaagcctatcccgcttttactggtttcacgcaggtaacggctaaacagttgtaaagcctgcacgtacttattaatatgtcctgcactatatccacggccagtacggataccggtttgcattttcaggtgatctatatagctggtggcatcggctgccattagctgctgcagccccatcttaccgcgctgctcctgataatacaggaacccacctacataacgcggcaggttatatacgctacactccgcataattaaccgtttcaagccactgcttaaagcctgcacatagtaatacatgctcattactgtgcagtacgtacactgtttccataaacaataaattttaataataagggagggactaacggggtaaaagagaagataaaaattactactatagtctttttcactgtcgtagttgtcgcagtggactaaaacctttactgtggcacctcttactacgacagtaactcactgtcgtagtactgtcgcagtagacgtagtagattttaacccggagagtattacttgtaattgatcatctataaggcgggtaagctccttatattcattgccatctaagataacatattcaaaaccctgacggtgtttataaccgcttacttgacggatataaccgtattgatgtaactccctgatgtaacgctgtacggtacggggttgtaaccggaactgctttcttacctgctggggagtaaaactatcctcccctttattatgaagataatcttttagctgctctaaaaagattcttgtagcctttgccagttcatcacccttactaaacatcacctcctttaacaactcgaacgctgacgcaatatcatccggcgtagtttcaatatagggctgcccgttactatcccgctttacttcccgctgatactgatgataaaaggtaatcgtttctataaacgataataacagcgtcatagttctgcgtggcttaaaaatttgctccggtagctggatacaacctgcataaggattcaccacccgtaccggttgcagcacctgctgtacattcttaaaaagctgtttaatagcctgttcctggctgtagttaacggctcccgcactctggcgggtctggtattccattatacggcggtcctgttccttactagcatccacatataacagcaggcaacggttggcattatcttcgtatagcttttcccgcgtcgtacaaccactcacacttaccgggccgtctaccgtaacagtaaccgttttcaggttgcctttattgtcttttagtgtaaccgttttagtgatacgctttttactttgcagctcccgcaagggatacagggaggtttccgccccgtccagatcctcgatcagcagcagcttatgttttaactcgtcctgcttaaagtagtaaaacgcattttccgtgatttgggtaatctctattttctctcctgcagggatcaggtctgatacccgttcctgcagataggttttaccgctgccactgctgcccaaaaacataatatgcagcggggtatgttgtttgcggctgctgtacaccaggtaagcaatcatacggtttacttcttcccctacaaggcccgacctgcctatatcttcaccagtgcgttttaacagatcaggcgctttcaggtaattaatagctgcttcacgctgtgcgggtgacaactccggtttagctgctggcttaggttgcatactttccatacgctgtacccggtaaccttcaagcccatttgtaagctgcgcaataacggccgtaactacctgctggctcatgtcataggacactgatacctggctgattaacccttgtgtatggctatggttataaaggtccagatgatggcgtaacggcaataactgtttttgcttatgctctattttcagcgtcacccgcaaccggtctaaaccggttattttaataccacctaaaacagtaataagcaatacaccaccatcataaattaacaactccggattaactgtatttagtctggtatcaccctctaccaatacaggtgtagtaagactttcagcaggtacggtttctggtacagtataaaaagacacgggctgcctgccttcgatcagttctaccaggacacggctatcatcatgggattgcagcacgctgtttatatcctcaccatccggaaggtttactgtagtgatctttacacggggaagcaactgcaataacgtgttactgtgttttatagtagctacttttcctgcatcatcaccatccagcataaagataatctcctgtaaaccggtgctggcaatgatggcctgctgatgttccgtagtaagaccattagtgccatacaaggctaatacttcatacgctgtactgatttccgcttgctgtaacagactggcagcatctattacactttctgtaagtattaaccttgtggcagcgggtgtagggtaacagggatataggccagaccgtccggttaaataaaaatgccgctgatcttcattattattgatgctacgaccatataggcatactatcttattttcatgattacgtaaagggaagattatgcactcctttgcccatacgctgtaaccatgtactgcattagctttcagcagcccatactttaccatgctattaaccaggtggtggtttttactttcaatatgtaatccgccactgttataacccatatcatgcagcccgtaatctatactacgacattgcaggtactgggtggcttttttactggcgggtaatgcttttttaaaagaactgaacacctttgccattaacgcttcccgctctaacagatccgcttcattacttaatgatgacgggatttcagatactcgcattagaggtgctacattacctgcacccaacaaggacttagctttcataatagcttcatgtgtgctacacttttctatcagctgtataaacctgattacatcaccggtacctgcattacagttactactaaagcaatgataggtgtctgttttagggtaaagctgtaatgaaggtgttttatcaggatggaacggacacaatacccgatgatgcttatcaggctgtaaaccatagtggataagcacctgaccgatagacaactgctgcttaatgtccttgatttccatgaccaggctttctttttattatcagtgtttcttctcccactgtaatctccacctgatcccccacattaaaacctgctttctctaaccatagcccactgacattgagccacgcaacatagcgcccgcccggattgtagcaatcttttaattcctgatatttgccatgcagctttactagtcggatttgttttgttgccatgtggaaaaatattttatagtactaattggtaacaaaagtaatggattggtttcaattaaccaatacttatttattttgactagcctaaataagtaactaaatttgttaaccccctgcatttacagggtatttaaagtacctttttatgacttttggcgaacacattgctacgcaacgtaagcagcttaaaatatcccaggacgaactggctaaaagagtgggaacatcagcacccattattggacgctatgagcgtggtgagatcaagccttctattgagatggctaaaaaaattgcagatgaactgggtgtgaccgtggactacctgattggcggttctaccagcatggtactggacaaaaaattacttaaacgaatagaagatattgaggccctaccggaagaggagaaagaaaaaatttattacttcattgatatggctatcacctataacaaaactaaaaaagcatactcccgctaaacagcgaagccgcaggcattgcctgcggcttcgctgtttagcggatccagttacgacaataacataagtctttatgtttctgctgtttttatcacatttaccataataagaccaggctttatccttaaacaaaagaaccaaacattctcaactccttcaactttagctggacgttcattattaagctcaatttgtaattccgatttccctttctcacctaaaaacttcacctgagacaaatccaaacttttaccccacaaaatcatagcagcatttatattagatccattaacctgactaatatatgtcccgcctctaaattccataataaatgtatatatatccataccctaatttattaattacttcccttagcttttctactatgattttctcctgtattgtccattttcttcttttcatgatctacagttctctttaatttatccaatgaggccttgtcatcctttgtcttgttgggcttgctttttaatgcctcgtattctttttttgccgcctcatatctatcttttgctgattctctagctttttgattagcatgttgcccattcttacctccaccatgtttttcaggtattgttatggattccattttctccagtttatcagcaacttccggagatacctgaggctttgatttttcatcaatgactttttctggggctggcaatggaactgctgtctcatctttagccgcaggggtcacttctttccccttaggcttagctccatcttttcccactccctctgataacaaattaatagctgtatttaccgtagcataggttcgataactaaaaagtgcaacttcaattgcctcaattactattggaacaagtacaatagggtttcttccatctgggtcaccatatctaaccggattattaaatgcaaaatgatatggtgttaaatcttcctgattattctcaatttcaggatctatttgtaagaatcttcctatttgagcattgtaggtacgagcattaaaatcatacaaatccaaccctgatccatcactgaactcccctgattgcaactcatttccgttatatttcttcctattttccgcataattactccccttcaacgcattcgaactaatccccgccattgtcaacccaaacggataataatgtgtctcctccagcagtggtcctgaattaaccgctaaaatcacattatcaaagaacacttcctggctaccctcattgctggtatatacgtacagaaagccggatttatcgatcaccatcttatcctggctgagcgtctgcaactcatccggctctgccttcatctgctttaccccactattcgcgtccactaatttaaactgatcatcgaatagcacaaaattaagataggcttttggcctgtcagtatttggttggtcggcgtctttttctttcagccgctggtaatcattattataaaaattgctgttaattggtgtctgccgggctgtggcacttataccatgtgcacctgcctctcccgatcctccattaaaggcctgaaccaggtctgccaatatgttttccgcattggttgttccatcctccttctccttagggccaccggatttataaaacgctttggcgctgagctgaatagtatcccctgccatgacacgtaacacaatggaggggcctattttcttgccaacaccggtagcggtgagttttgcgacagacgcattctttccggcgctttcatctaccggatagccggcaggcttatcggcgcgtgtattgtcaacattgctgaacaacgctgtttcagtggcagcagccggcgcttccattgtggcagcatacatagaaaagtccgtttgctccgttaacaccatgcgggtatttcccaggtgatcctttacaaaataatcatacttgaacgccagtggttgtccagccgcaaaaacagcacgtacccgtccttcctcatgacccaaaaactgcaaggtgtcattctgatacacaaaaccatctatatagtctgtggtagtaactttggccggagtaactgtattatcggtaacgatttttttgagcttgctccccatagcatcatactggtatttaatcaatccctttccggtaatagtaatactctcaggcaggttcaggtgattataactgatgacagtaatatttttattattgtcttttgtcaggttaccgttcgcatcgtaagtataatctgcagtttcattattggtaatttctttaaaatcacccaactgggtctgggtgttattcttgcggtcggtaacaaatgataatttattactgccggtattgtaaccatacttcaggctatccagggtgagtatcgtcaccccattcatgcccatctgattcatgaactggatattaccattagcatcatacgcaagtccgcctacagaaaaattcttctggtcgcttgtccaaccggtgctgccagtgttttgctgggtaaaatcggcttttgttaagcggttcactttgtcatagccatatccataagccctggctgttccatccccacggcttttccatttagcaccagcaatattaccattgaactgggaattggtgaacccataatcataactcaggtcctgcccaaaccaattagcagtgcttcctgcggttgaaatgaaatctttattgatgctcttaagccagccacgaatattgtattcataattcagcgtttccaattgggtgctgattcctgtaacacccaaacgctttttctttagctgtcctaactcatcatattcattggcaacaatggtcctttccgatgcgacatcatcatttagccgtttctttatattgagcaggcgcccgcccgcatcatatgctatcatggtcagtacagaagtctgtgacgctgttccactgcgcttattgcggtgacgtagataactgctcagcagcataccattaaagtcatacaaattagtgatgacatctagtccaccacttatgttatccgatattgactggattaaacgccctttatcgttatagtgattggtcgtggtaagccattgattagtgcccagtacctttactttggttcctgtaaccagtccttttatcatcgagctggccaccggcggcaaagcttctgcatatggattattacccgcttgtggtttggtgatatccccgctgacatagctttgcttacccgtgaagctataatcttcataaaaagcataggtcaatggggttagcgcgcttaccgggatatttggtagcgggttggaaactgtaacactggtattaccattggtagcagccgcattgatctcagctgttatttctgttccggttccggaatcgaaaccatcttccaaggtaatgctattggtagcctggtacagtaaactaccatcatgagcagccaacaccaaatcagcagtaccaggaaaagtataagggatagattgtgtattactgatggcggtattcatagtggcctgaagcccttccctggtgctggcgttgttatacagtgccgtcatggtaggccggttcagcacatcgtagaacgtgacaagccaatttatccctttcatgttgccatcccgggaaaaggccagcctgtccctcacatcatacaccatctcagtggaatcagcgccgggtactttcttgactatcatacggctgcgaccatcataacgataaataaaacaaagctctgccgcaatgccagtactaatagtccagttactgatgatagcttccaccgctttcggaggaatcacaaaacgcagattacccaattcatcataaacataataagtacataaccagcccacatgcccggtaccaggtgtggcagctaactgtattttttttaatacaacccgcccctccttgtccttgtattccacaacctggctgccggcctcatcggtagtgatggtcttgaatagttgccctgcagcgtatatacggccagcaccactggtaggaataatgccacccacagcaaaatcccagatacgtacagaatctgacagcgcatttatcaggtactgattagcaagcgggtggttaccacctctctccacggtagccgcatcattcttggcccaactgttacccggagcgtatgttttcattacacgattcagcggcgaagcttcatagtcaacacgattataatacacactttctcctatcacaccgggcgccagggtagcgttctggtaaaaagctttctgcgcattaaaagggtctgttttgaatttaccatcgctggtattcccgctctgctgcacgtagggcaaatatttaaactgctcccggccaaaagcgtcatatacaacagggctcaccaggtctttgccagaaacgctcatactctttgacacagtttgtaacggacgcccaagtccatcaaaatattgtgtggtctgccgtacctctgttacaggtcgactgggcgacactacatatgatgtatcagtaagcggcgcagctggctcccagatacgtacataattaatagtggtattggtataggctcccggtaccgtagccggggcaccagctggccgggctgtgacatccggcttattctgctgtgcatgcagtgttacagcaaaacccaacaacactataatgagataaaatttatgcataatattactcagttcaatagggataacaactaatttttcttcttcatttccttctttaacgtctccaattcggcgcgctgcataatactctctttcttcatttcaatcatatacaaggtcagctcttcgatcttctgcaacagtttcttattcatctctcccaaatctaacccctcgctttctatctctctggccgaaggtatctccggtaaatgcctgttggtctggataaaacgctctacttcctgtaatgcaggtagctcatagtccggatgaaacacaaaatctgcccagcttccctgggttaccttcatcctttttgcgccaatagtaccttccactgcaagcttataactaccgggagtcgtagtaccaattccaacattaccggcgctattgatagtcatcctgatggtagcggcagcactcaatcgtcctgtttcaaaatagaggttactgctggcatttgctgctgaaatatgcaaatcgctgtaactttcaatcacgttcttcttacgatattcaatcacaggaaatacagtactcgcgcttccgatatacaataatgaattcgtcacacccttattttccaacctgacaaaattatctgtagtactatcgggagtttccacgcttaatcgcgcgcctggggctattgtcccaatcccaacatagccattgggcttaaagaccatccagggagattcattggcggcagctgcagatgtatttccccctatgtaagtataggtaacggtgccattaagccccagaacaccaaaagaggcgagttttccggtaccgttgtacgatattccaaattctcttgcccaggtgccggtgaagttaacatccacgttgattccatttggataaccagtaggattagtaagcttaatatttcctgcatttacatgcaacaacgctgatggtgaagaagtaccaatccccacattgcctgttgatggaaataaattttgggaggttgcggttaacacacacaggaacaacataacaatgttcagaaaaaataatttcatagatatatatatttattgcaattacaaacaaaattcaaacttgtctctcttgattcgatacagcgatattacaggcacctttagtgtttagagttacttcgtctaagttgatctacaatacactattactaaaccacgattgccctggttccattatcgaaatgtcagtctcatattcctgaacgggataaaaaaccatttagttcgattagggccagtggattacgaagggttgcgttaacaatacattgaacatcttcatgggtacagaaagtttactaaagggctaaaaaattgtttaattcggcgataaaaattcaaaataaaagtacatacaattcatcatattctcaaacagcagttgaaaaataaaatatttcacgattcaaagcagccagtatacaaatttgcaagcgtattagcaagttaccaacgctacactgaatattaaatttatatgaacttggattctttgaaaggaaataactattttcacacgaattataatcctaaccgttaacctatactaattatgaaatataaatacgcgttaaccaacatttcccccctgttctttgggctaaataattaaaagccttctaaagcattcatgttcttttcacaaacctgaatgttagcacagcaaatttatcatgaaataataatatcatacttatatatctatgaagaagattctcacgaatttatttagttgtttacttttcccatttttactgaaagcacaatctgaagctgtaactttacctaagttgattactccatcacccgaagctgcttccatcacaaagtacggcatatatccagtcagcctattcaccggtcttccctcaatcggtattcccgtctacaatatcgcagtccggaatttcacactgcccatctcatttgattaccacgccgctggtataaaagtagatgactacgcaagctgggtaggaataggctggagtttaaacgctggcggcgccatcaccagaactgtaatgggagttccggatgatgactccaatggttcattttactatccgattaaaagggaaaatgccattacaggcgatgactacaacaatctgattgatatcactgatgggaagagggatagtgaacccgatatcttttattataacgttgccggtctgtctggaaaatttgtatttggccccaataaggaaataaggtccataccgcacaataatctgaagattaactacagtggcggcattttctctatagttgatcataatggcactacctactggtttgagaaaaaagccattagcagttcatatcctgaattcggtggaattaaatattggcctgttacaagctggctgttaaccaaaattattcttgataacaaagtagacaccatttcatttgattatgtaggatatagtcagggacgaaggcagacaattgattacagtctttcattgggaagaatgcctaaactggtacccaggtcttgtccagatgggacctctggctgccaatatgtaagctttagctcttcgtttattcctgtaagaaatattaattatcaagagtttgaagattactatctcgataagattaccttcccgggcggaaaggtcaggttcgttgctggaaaaaatgaacgcctggatttcgggggactagtactagattccattattgtggaaaacaatacgaaaccagtaaagaaaatggcgttgacgcacgattatttttattcagatgaaggctacaatttctttgcctccatccgggataaataccgattaaaactaactggaataaacgaagtgggtaacaatcaggattcgatattgcgtcataaaatggagtacgaagaacaatacaaactaccccctagaatgaattgtggcattgactggtggggatatagtaatggtcatcctgaaaatcaacaactaatctctctcgatgagatgggaagacagtatagttattcagatattataggttataccacaacctctgtaataaatccggccgccaatcgcgagccggatgaaaataatatgcgggcgggtatattaaaaaagatttattacccgacaggcggatatacagatttcgagtttgaagccaaccgcattctggcacctaaaacagagagcgatcccggtggaagctattttatagcagcaaagaaggacgatcctcctaatgtcacttacagaacagttgaatttatatcctccgctacaattggcataaacgatccattgcccgcagaattaagattgattattcccttatggacaaatgccacgcaaccttatgtcctatttgagaatttaacaaccggcgcgtctataagatataccactgtggctggggagcaggtttcccggacaattagagtcgccttaacagccggtcagaaatacaaaataacagcgaatatttatcctgatccatcagaccccaacgatgatactgatgacgaagttttagtgacacttacctgggctggcagagggactcaccaagtaacagtagtgcaaaaagggcccggtctgagagtaaaaagtattaaatcatatactgccgaaaataaattagcaaaacaagaagattataaatatggagaaaatgaatcgggcaatggcaacgttagttttattacctctttatttcaaagccgtacttatgaacaaaattataatttttgctggacagcttcaggatctgatccgaagataaattcccaaccatattccaggttggaaatacttagcaaaccaatcttttcatactccgacattggaggtagcagtatattttaccctgttgttactaaatacgaaataggcgaaggaagcgacaatgggaaaacgatttataggtatgattatgaattagacgaaaaaatcgatgctcattacccggaccctcagttacttgtcagcgctggctggaagagcggtaatctaatatctgaaagtacctataagaaaaaagatgatggatatcaattaatatcagaaacaaaaaacacttaccaaacatatttttttgatactacatatggtcttaaagtaagacagaaaataatatacacagccggaaggaattgcattaatgaaggattgcccggtggatacagattcaacgatgattttggctattttgaatatcccgtcgtttccggtgtcaagaaattactgacctctgtcagtaaaacttttacggataacaatgatagtttatcctcgaccatcctctatggctatcagaacttaatacacctgctgcccaccactatcgaaacgttaaacagcaagggagtcgcattaaaaagcattttcaaatatccccaggataaagcgggcataataggtatgtctgctcaggaatccgtcgcagtagattcattggtaagcaaaaacatgatagagaaattagtcgaaaaagaggaatacgaaaataatatattggtccaaaaagcacattacgaatatagtatttggggtagcgccaaatacttagttgcattgaagaaattcaagctaaagctaggtagcgcctcttctgaagatcgttttgaaataattgattatgataaatttggaaatattctggaacaatctaacagtaataacatacatgaagtatatctttggggttataatgacctttatcctgtagctaaagttttgaacagtagctacccagtcgtaaaatctctaatcaatccctctataacgcaaaatccggttagtgatattgtattacaggcagaacttgacaagctacgcaacagtaccactttaagtaacagtctcattagtacctattcttatactcctttgttgggattatcaggtacaaaagatgaagccggaagaaacatctattatgagtatgacggattcggaagattgaagttaataaaagatcaaaatgggaagattctaaagttgattgattatcaatatcaacaagcattaaataaataatatttaattgcgtgacactatctccaaactatattttaattaaaatatagtttggagatagtgtcaacttttacgcatgttatttacgacatttaatatattaagtcaattcagggcaggacttagtattaaatccattcttcttgtcatctatctactcacttctcaaactctttacaggattcacaacagctgcttttacagactcataactcaccgttatccatgctatcgttaatgccgctaatgaagccatcaggaaaatagcccaaccaacatttacacgataagcgaaaccgccgagccacttattggtggcaaaccaggcaatgggtattgcaattacaatggcaatcaggataagctttgtaaatcctgttgataacagatataccacgttgaatacggatgctcctaacacttttcttacacctatttccttggtgcgttgctccgccataaatgccgataagccatacaaacccatacaggaaataaaaatggcaatcatggcaaatacattaaacaggctacccatttgttgctcccctttgtataaattattaatgtcctggtcaacaaaaccgtaagagaaggggaaagcaggattaagctgtttgcttattttctccaatgcctgaatggtggctgctgttttgccgggttgggtacgcactaacacaattcctccattccatttattgaacgcaaggatcattggctcaatggctgtttgtgcgggtttataattaaaatcttttactacgcctacaatagttcctttatcgcccgaaaacgtaagcgatttaccaatggcggctgccggggtcatccccataatttttgctgctttttcattaatcacataattgcctgagtcagcaaattcggtagcagacaaagcccttccgcttaccattttcatttgaagcacatcgaagaaattgtccgttacccatgtttttgaaaaccagatgttcttatcctgcaaggccattccctcccattctacccctgtggtgctgctcgtcaggttagatatcgggtcggtgatagcagtaaaatttgccgtaagtggatttgctttgagctccgtatttaataccagttgcttgtctcccatttcgccggttatcgacatataaagcaggttcgatttattaaacccaatatccctgtttttgataaaatttaactgtttatatactacagctgtaccggcgagtaatgcgatcgaaacaacaaattgcataaccactaacccattacggaaatatagattccctcctgtcattctcatgcttccctttagcacctccactggcttaaatccggatagaaacaaagcaggatagctgccggaaacaagcccggtaaacaatgcgatgccgagcagcaatgcaattaattttccatccaataattgtatagaaagttcctttcctgccaggttattaaaagcaggcagcaacaggcatacaatgccaacagccattaacatggccataaaagaaatgaataatgactcgccgatgaactgaccaatcaattgtctgcgacccgcacctaccgcctttcgcaagcccacttcttttgcccggcgcgcagatcttgcggtggccaggttcataaagttgatacaagctaccgccaaaataaacaacgcgacgataaaaaatatgtttacatattggatattgccctggccgggcaaattagactggtaatcagaacgcagatgaatatccgttaaagcctgcagtttcatatcaggttgactttcctttacgtgctctccaaaaattttatttacctgcctgttaaggccggccagggcgaccggcgtagccttgaaattttcatcgagttgtacatagtcatagaaatcataactagcccagatgtttcggcgcaaacgccaatccgtctgtgcaatggcagacagcggcatgataaaatcaaattgcagatgtgagtttgccggaatatttttgagcacacctgtaacttctacattatctttattatccctttttaaaattttcccaattggatcttcattgccaaaatatttcttcgccatattttccgtaattaaaacagcatcaggccgtattaatgcagtttcggcattcccgcttattaagggaaatgaaaatacctgcaacagggaagaatcggcatagaagacggctttttcttcaaacttttttgtacccgtttcaaaaacagtagtagtgggctgactaaaacgtacaaagttttttatagcaggaatccttgctttaagttcgggaaccatgggcccggaatttgttgcaccacccgcagtaaggcggtagatagtacccgcgttttgatggaatttgtcgtaactcaactcatgctgtacccaaagcaaaatgaaaatactgcaagccatgccaatggccaaccctgcaatattaattgtagcgaaggccttatgccggacgatgtttctgaaagcaatcttgaaatagttctttaacatggctgttttattaggtttccagactcattgacagggatgcccaaagaaatgccaaatagtaatttattgttacttgtttttttatagatatggtatttatttaaactgtccgtttatgaactgggtatgttcactttcaggagatgataatgcagctatacttctcccatacttctcggatacttctcggatacttcttggatacttctcggatacttaggagtcgtgtatgtgtcgtattccccatatattccccatatattccccatatagtccccatacacttcccatatactcataatacactcacgatacactcatgatacacttccaatacactcccaatacactatgtctcgtcctgaaatagctatacaggtgaagaaataatcctgtttaaagtttacaatataagttttaaatcctggaaaaagtttacagtgcggcggcataatccggcaaaaagcggcaaaagcggcggatttgtttttctctggtttcacacgtccatagctttgtatcgtattccggaatataacattgcaggctcggatgggaaacgaatactggcacgggtttatacccctgtacggaatacaagcaggaaaacaacgctgaaatatccccacgccagtgaaaacaggatatgcaccgtggtttcaaaccgtttacctctccataacaacggcgagtaaacaaagaactggaaaagcagccggcataaccagaatacaaataacccaaacgccagcagatgccccaggcgcgtatgcaggatgtcgtgggttgcataaatacaccctagtcccatcagcaacaccatcagcgcaataaaaaaagtatgcacatacatcatctgcctgctcaaaagactgatcgccgtgaactctttcttccagttaaaataccgcggaaagaaaatgtgtgtcagcgataatagcaccagtatataaccggtaattttaagatgcaattccattcttttgcaatataaaggccgacaaaaaaggggtgatcttcttttcttttacaacgatcaggcctgcgttgttgaatgcccgcttccaggcagcacgcgaaaagaaatgcaggaacccgatcgtatatgcgatgaagttaggcgcatcccgtaaatgctccagtaccactattcttccatcagcagccaggcagcgatgcaactctttgaaaaaaataatcctttcccccggatccctgatttcatgcgcggccagcaaaagaaacaccacatccactgatgcagcttccagcggaacagcggccgtgctgatggttttcgtaccagcataaggcgcatatcttttccgggcacgttcaatagatacctcggtatgcatctccggattataaaaatcaaatacctgtaaatcagctcccgggtatttatgcgcaagcagctggctggtttcatcaaaccctgcgtggatgtttactatacgcccgtgtggccgaaactttatatcgtccagccaccgtaaggtatataaatctgaacggtcgtaaatataccaggaaacaactaacgacgataaggtagcgatggcagctccccacaacatcagcctggttaacgggtattgcgtgaatagcaaccctgctaccagtagtagcaaaaacaacacataaaagtgccagttgaaccggataatatttacgatgccctgaaacggcgttctgtttatcttttccataggtccacttttccttttttccagtaataaggaatttgccggatgataaatgcgttcgccagccgggcgccctgtaaggcaggcgtgctcaaaaaaccggcttcgctatgcaacaccgataccggtacaggcgtccagttttcccgcacaccttcaataatcagcacttcgccggaatgttcgttacaggtaaatgtaaaaggcaacggacctgcaaaccgccgcgcctctttccagtcagcaaaaggagatcctgctggtaatgccgcttcatcacccgtattcacagtgatattcaaccccgatgccgccgatctaacggtaacaataccatcttctcccgtaatactgatatcggtagtggtataactgtaatgggtaaacaggttaccgaaaaattccatcttcttactgtctgtttctgattttaaaatatataacccgcgtaaccgctttccttcactattggtataacgcacaaacacccggtagccggttaacacaaaatcatttcccataaatgcaggaaagcctttaggccgcaggttcctcgttttcacaatggcaatggctatgaagacccactgatcctggaatatatccagctcgagttgcggaggtattaagggttccaacaccgataccggcaacgcataggtaagcaccagggagctttcaaagaacgcttccacggcaaagggatgatttttaagaaaggctaacatgggtgctatattcattccggtaaatgataaatataaaagcggcagcgatgataatattcattctcccaaacaataacaggtcgggtgctgctataaactctatgatgttcatagcggctaccagcagcatttgtaaaataacacaccagcgggattttatccgggaaagtatccatatcgccattccggcttccaggacaccgatgatacgggtcagtacaggcgcatgggtttcgccaagtattcttgctacaattaactggtgccggggaacgtagttcagcactttacagtacacgccatttatcatccacacaagggctattccggtgttaaccacatttttttgcttactaaaggccatgggaccaactttatcaatacaagttaacacaaaaagcgccggtctcaaaaaagagccggcgcctgtctataaataattcccccttacttacccaggtcccacgctttcaatccattcaactgcacatcgccgttttctgcaaacacagccagccccgtagccgctttatccgggaatattaaagtggtaagcactttctccccgtcgtttacaaatacctctacagacgatttatccagcagcacctgcaacctgattttattgttggcagatggaatgctcatttgttgcacgtcttttccatcgcggatgtagagctcattccgttgtacattatagcctaccactacatcctgtgctatcttaaaaccaaaatcagccgcggtaccaatggtaaattcggcatccacccaattagtattggtattaaaacctttgccgcttaattgcagttccttgctgttaagggtttgtgcttttagctgcagttttttagccgcaggtaatttccggagataggtactgatctcagcagatggctgctgaaataaacgtatacccgctgccgtagttttcaattgcagatcgcgtggaatcgacatttgcccgcgccacggtgaagtgggcgtttcaaatggcataagccagccgatcatcatctgccggttgtccggcagatgattgtaaggaatggcggcataaaaagttttgccgtaatctacaaacaactggctttccggcttgttgtcattggtgaatgttttgccgtcgaaatcgccggtaaaatactgcatgccggtagcggcatcagggttgccggacgacaccatcagcaaccatttctttttcgcccggtcaccgtctacatacagcggcgttaaagacgggcactcccatattttacgggtatcgccctggttgccgaactcactcagcagctcccagttcttcaggttttcagatgcgtagaactgtactttatgctcggcaggtaccgccaccgtcatgagccatttatgctgatcttccagccagatcacgctgggatcgcggaaatcttttttctgtatgtctataacgggattgccgctgtagttggtgtaggttaaaccaccatcattactataggcaataaactgtgattccttttgctgcttcggctgatctgccgtgtaaatagctacaataggagccttcccgcttttaccaaagccgctgctgttatgttcgtccagcactgcggagccggagaaagcccaggtggtggtatctttcttttctatttccggaatggcaacaggcaggtgtttccagttaagcaaatccctgctggtagcatgcccccaactcatatgcccccacttgttttcaaagggattatgctggtagtacaaatgatacacgccgtctatgtagatcagtccattgggatcgttcagccagtttttaggcgctgtaaagtgatataccggtctccattgcggagtaggtgtggcattatcctgtgcgtgcagccatccgggtaataatcctgccagtaatatggaaaagagttttttcttcataacaatgatatttaatttttaccagccggtgttttgtttgtataaccctttgctgtagttaatctggtttaacggtatgggcaggtattcatccctgcctcttttgaaggaagcatcattcaggtgtgaccggcgtgttttttccacggcaaaataagcattgagataatctgctgcaataccccagcgtaccaggtcgaagaaacgggaaccttccatggcaaattccagccgccgttcccagcgtaatgcctgccgcgcaaagtcggtggaccaggtgcagttaacgcccggctgataagtattcatcttgtaactggaagtaaaggtaccatttgcctgttttaataagccggtactggcagccgctctttgccgcacctggttgatgagtggcagcgcttcggcagcgcgtccaagttctatcaatgcttctgctttaaataacagcacatcagcataacggataatctcccagtttttggagctcgacataaaaggcggtaccttctgaaaagtagcatcgccgggcaataccgcttctttgaggctcaggtagctgccatatacctccggcgcacgggcccaggcacgctggtacagaaaagcaggatcatatttgtaaggatgccccgggatagccacggtatgatctaagcgcggatcaaaggtgtgcgtatgaaaatccgcttccgtaacgatgttcacattattgaaagtttcaaacatcggcagcccgctggcgcttgtttgaaaagcattcaccaggttactgctgggcgaatgaaaaccgcaacaaccataggcctggttcatcgggtaatccagtgcatgtccgtaatcgaggcggcctttaggcgtgccgtcatcctttgaatactggatagcgaaaagggattccgggccgttttcacctttcgacaaaaagttgttcgcataatcaacggccagctggtatttgccggaggcaattacttcattgcacagggtatttacctgttgcagcaaagccgcatcaataccggttacatggttattctcatcctgcttataggcttcatacaataatgttttggccaggtaagcttttgcggcgaatttattggcccttcctatttgcggttgtatatcggggagatgggaagcggcaaaagtaaaatcatctgcgatcttcgtccatagctccacgttggaataagtacggttggaaatggtatcataggtttcctttggcgcattttcatcgatgtagggcacatacttgaataatgttttcagcaggaaataataatgtcctctcagaaacttcatctctgcctgccgcactgttttttccggaaattcgctttcattcactttatttaaccgtgccagtgcatcgtttgcgcggccaatgcatacatacaggcgaaaccataccaggtcggaagaaccgttatccaccctgttcagggaaaaggtttcatagaagtgataatcgctgatatcgccggcgccatcaccgcctttatatgcatcgccactgcggatattaccatagggccacatgctggaataaggagcggtatagtgatcgttgcccagtgaagcataggcggcggtcaccattttttccaggttggccggcgagttcaggtcgtcgcctgaaataacgccctgcggcgtttgatccaggaatttgctgcatgcgccgagcaacaggcagctgaataaaagaatatattttgtgtacttcatggtggctgtgttgtgtgtttaaaaagacaggtttaaaccgatcgtgccaatcaccggaatgggataggcgttattaggattctcaggatcggtggcagtaaaacctttgttttttaacgtgagcaaattgctgccctgcagatatacccgtgctgtttgtaaacgcttgcttaacatatgctggaaactataccccagttgcaggttcctgagtttgagataagaacctgattccaggaaataggtggatgtccggttttcgttgttacggtctaccagcgtgagcgcgggtatggaagcatctggatgttgcggcgtccatgcgtccagcgtacgtgcgccccagttagttcccggccagatggaagagaagtcggtgtatgttttgtaagtgttatatacctggatgccctgtattccctgcaggaagaaggtcagatcaaagtgtttatactccagtgttacattcagtccgtaggtaaaatcaggatctcctttgccgatatagtcgcggtccttgtcatcgatcaccccgtcgctgttcaggtctttataacggatgcggcccacgcccttcccgatttgcgtggcatagtcatctacttccttttgtgagcggaacaatccatcggctacgtacccgaaggtggaattaatagagtggccaagaatagttttatcctgtccgttgccgggataggaagtcagtacttccggcggcagcctggtgatcttattgcgataggtggctacgttaccggtaacggtgagcgccagtccgggtgcaatgttaccgttatacgacagcaatacttccagccctttattttgcatggaggcgccattaacgaacttggtaccgccttcgccgatcaccgcgaggtaagccgggctgataaggatatcggatgtcttcttaataaaataatccaccgaaccgctaaggtgattatcaaacaaaccaaaatctatcccggcattagattccatggtgctttcccatttcaatgcgggattgccctgctggatcagtgtatatcccgatggcaactggccggagcccgcaccaccaagatcgtacgcactgccgctgtcgaaatcccaggtgggatctatcccataaatagcggagtataatgtgtaggtggcgttgttggcaatttcctggttgcccgatctgccccagccatagcggagtttcaggtccgacaggaaaggcaggttttgtttgatgaaattttcttcacttacgcgccatccgagagataccgcaggaaacatcccgaaacggttttctttaccaaagcgggaagagccatcgcggcgcaatgtcaccgaagcgaggtatttattatcgtaagaatagtttgctttaccaaaataagacaacaacgtatagccgctgccggtaccgccgttatctttattggaagatcctgcattcaggtaagcatagtcaatattttcgagcgcgtatccctgcctgctggcgtagaaattctgcgcgatatatttaatctgttcccctcccagcaggaaatcgaaccggtgcttctgcagggccacattgtaagtgagcgtgttttgccatacccagttaccattataatcctgtgaggtttgggagaagttggacggatcagaaaggaacccggaagtatacgacttacgcagggtacgctgataggtaccgttataatctataccatagctgcttttgaaatggaggtttggaataatttccaggtcggcatatacattaccaaataagcggaggaaattacttttgttctgccggttatcctcaatgaggcgcacaggattctgccggtcggtcatgccgggtgcggggccaccccagccaccgtcgacggtgtgtaccggcactaccggttgttgcaccagcgcggcgaagagaatatccgtggctggcaccagcgcgtccctgatataggtagccgacaggttttcaccgatcttcagcctgcctttaaaaaaggaataatccgtattaaagcgggcggttattttccgttgctgtgtttcttttacaatgcctttattgttatacatgcctactgaaaaataagagttacctctttcgttaccattggcaatagacacgttataggtttgcaacagggacgtttgtgcgatctggtcgtaccagtaagtatccgccggcttcatggttttggcggcatcaataaattctggcagattaattttgttgagcaccgggttgttgaaatcgccattccagtcgtattggtaaatctggttgttgttgggatcggtgcggtcatttaccgcagcctgccaataggcgcggccgcggccttccgtgttcagcgtttttaacttggtactgtaatcctgcaaagaagcagatacatctgccgtgatgcggctgtagcctttcttcgctcttttggtggtaacaatgatgacgccgtttgcagcgcgggagccataaatggtggcagcagaagcatcttttaatacctggatggattcaatatcattctggttcagttcctgcaatcctcttttggttggaataccatccactacatacagcggatcgttgttgcccagcgtgccgataccgcggatacgtaccgtggcattgctgttagggtcgccgttggaagtaatgaatacgccgggaacgcggccctgcagggctttcaccgggttgccgagcggaatgtcttttatttcgctcacatttactactgatacggcgccggtaagatcggcttttttctgtgtctggtaaccggttacgatcacctggtttagatcggtggcattatcttccatttctacggacatactgccttccgaagctttcagcgacattggcttcatgccgatataggagaagttgagcacttcccccacggcagccggtaatgtaaattgcccgctgccgttggtaatggtgttcctgttgcccgactgtacggttacgccgggcaaaggcgttctgttttgtttactgataacggtaccggtgatgtttcgttgctgtgcaatggcgaagaggccgaacagcaacatcggtaataagtaaaacaactttttcataatggaatttgtgaaatggtggtgtggaaatgtaataactggctaagtgtgctgtggtattttcatcaggctgtatatctcggatggatcgtatggcggacagccaccggggcgggatgccaccagtgcgcccaatgcattggcataggccaggctccaggcaggggaacgttgttgcagccggcatgcgagaaagccggcaaggaaagcgtcgccgctgccaatagtatctgctactttcacggtttgtccttcctggtagtaaaaagcttcatctatatatcccatgcaacctttgctgcccaaggtgacaactattaccgggatgttaaaccgggaagacaatgcctttacctgttcttcgtgcgtagaccatgcgccataccaggcgctgatcagctccagttcagcaatattcagctttagcagctgacagctgtccatgagccattccagcgtttcgcgggagtaccagggagtgcgcaggttaatgtccaatacttttgtggcggttgattccaatgctttacggagcgtattcctggatacctcatgccgggccatcaaactgccaaaaacaatatactgcaggtcatcacccgttaataaagcctccagggaagcattccagccaatatgatcccaggccaccgggtacaggatatcatattgcatatcgttatgcgcatccatccaggcatttactttacccgtggcgtaagtagtattcgtttgtacgtaagcggtagagagctgcatgttgttcatcagttgcagcagtcttttgccatgatcatctgcacctgtagccgataccatggcaacggactgcgacagtttctgtaaatgatacgctacgttcatgggagcgccgccgggcagttcctggtttggtaatatgtcccacaatatttccccgaggcaggcgatgttatactttgttgtcataaaatgtttgtttaatgcacgaccattgtcatttcaatttcttccagggtttgtccttttgtttccggcatccagcgccatacaaagagtagttgcaataccatcatcacacagaagaaggcgaaaatgtgaccaccgccaatatggctggcgagccagggaaaggtaaaagcaatgacggccgccatgatccagtgggtaaagctgcccagcgtttgacctttggcgcgtaccgcgtttggaaatatttcagagataaatacccagatcacggcgccctgcgagaaggcaaagaatgccatatacaccagcaggtaggaaatcacggcaataccgccggtatgcatataaaaggaaatagcggtgaggcccagggtggcaataagcccaacggtacctatcagcatcagttgccggcggccgatgcggtcgataaaccgtatagccgttaacgtaaaaatgaagttcacgatgcccagtccgaccgtagaaagcaaagaagacgccgtgcctaaaccggacatttcaaaaatgcggggagcataataaatgatagcattaatacccgacacctggttgaagatggcaaacaatactgccagcactaccggcgtgcggtacttgccggagaacagccgttcctttggcgcgccaatgctctggtgcctcgactgccggatggtggtgatatcgtcctcgtaaccggcggggttgatgatttgcagggttttgatggcggcagcttcttttttaccgtgcaacagcagccagcggggactttccggtacccagcggagcagtagcaggaacatagccgcggggaatgcctggatgcccagcatcaggcgccaggagttttcacctccatatccgccaatgaaatagtttgataaataagacacgaggataccgaaaaccacgttaaactggaataaagcgaccattcgtccgcggtaggaagcaggtgatacctctgaaatatataccggggccgttacagaagaagcgcctacaccgagaccgccgataaaacggcataccaggaaaaagtaccagttagtagccattgctgtacccactgccgacaccaggtataccaacgctaccagcagcagggtggcacggcgtcctagtttatccgaaggcgtgctgcctcccaaggcgccaaacaccgttcctattaatgcaatggataccgtaaatccatgttgtacttccgttaaatgccagtattgctgaatatgttgctccgcaccggagatgacagcggtatcaaaaccaaaaagaaaaccgccaagtgctaccacaaaagcccagaagaaaacaatcttgttgttcataacgtagaaataagttttgatcgataagtcaaacctacttctttgctaaaggctgccgttattgtattgcaccgctttctttcgaaattataacagcgggcataaaatcagttaatatattgacatatatatttttatacattaagatagatatatttcaggctaacgtctttcaattttgtatcattgtttttcgaaataaaaccaaaattattccacttgccagcagtattaaaacgatatctctgtttaataagtcttttcctgttgatgtatgtcgcaggatgccgcccggaaaccggaccgaaataccggatcggtttttcccagtgtaccggcaacgacgactggcgccggaacatgctcacggaaatgaagcgggagctgttttatcatccggagatgcagttattgtaccgggatgcggaaagtgacagcaagcggcaggtacagcagatcgaggaactgctggcggggaaaatagacatcctggtggtatcccctaatgaggccgcgcccctggcgccggtaatagccgccgcctatggaaagggcatcccggtgatcatcctggatcgtaaggccgccacggactccttcaccgcttacatcgggggcgacaactacaatatcggcaagctggcagcagaatatattgccgcccggctgaatggccacgggcgtattatagaggtgaccgggcttcgtggatcttcccccaccgtggaaaggcaccaggggttccgtgatgccctcgcacactaccccggcctgaaagtgatagccaccctggaaggcagctgggtggcagataaaacgcgggaagccgccgcacgcaacgattccgccgtgcagcaggcggatgtaatcttcgcacaaaacgacgtgatggcgtatagcatgtaccgttattgccgggaaaagggcctcaaacaaacccggtttattggtgtagatgcttcaccttaccccgatgcggggatagacctggtatcacgcgacatcctgagcgcgtcgctgctgtaccccagtggcggcaaagaagccatcagcatggctgcggatatactcgccgggaaaaaggtgccccgcaatacgctgcttcaaaccgtactgatcgacagcagcaacgtaaagttgatgcgcctgcagatagataagatacaggcccagcaccaggaaatagaaaagcagcaatcattgctgcaggagcagctttcgctgtaccaggaccagcagcacctgctgcggatagtggtcaccacgctgggcatcgccttcctgctcggtattgtgctgatcttcattttacgcaccaaccgccggatcaatcagcaactgaaacaacagcgcgatgaaattctccagcaacgggaccagctggtggaaatgaccgcccgcgcgcaggaggccacagaggccaagttcaccttcttcacaaacctctcgcatgaattccgtacccctttaaccctcatacaggcgccactggaaaacctgatgggcagcaggcagctctcttcctcgcagaaacagcagctggaactgatgcgcagaaatgtgacccacctgatgcggctggtaaaccaactactggaattccgccggattgaaagcggcaaactgcaactgaaagtatcagaaaatgagctgcccgcctttatgctggatattatggaagcatataaaggcattgcggttaaaaagcatatcgatttccggcttattagccggcagcccggcatcaaagcctggttcgaccaacacctgtttgaccgggtattatataacctgctgtccaacgctttcaaatttaccagcgactacggcaaagtgcatatttacctggaacagcctgcagccgggcaggaagcggtaatacgtattgaagatgatggcagcggcatggatgaaaacaccctggcacatgcctttgaactgttttaccagagccgcaacaatgaacataaaggaaccggtatagggctggcgctcacccgcgaaatcatttccctgcatcatggcagcatcaccgtaaaaagcagtaaaggcgccggcaccaccttcagtattaccctgccgggtacttccgccccttttgcaccagaggaaattcagcaggaagatgaacatatgaatgtgatcaatcactcgctgcacagctatacggacgacctggacgacacgccggcagaagaaataccgctcaccctgcaggcacatcctcattcggtgctgctgattgaagaccacccggacctgaatcatttcctggccgattttctcagcggtcaatatgaagtgttccacgccggcaacggcgcagatgggttaaagctggcctttgagcatgtaccggacctgatcctttgcgatattatgatgccgggcatggatgggatccaggtgctggagactttaaaaaaagatatccgtacctcgcacatcccggtaatcctgctcagcgctaacagcagcgaggaacaacgtataaaaggcatgcagcacaatgcagacgcctatatcagtaaacccttccacctgaaatacctggcggaaagcatcagcagcatgctcaataaccgggctttgctgaaagatcactatatcgccgagcctgacacccgggtacacagtacccagtccagcaaaccggaccgcaaatttgtgaatgactttacggccatcgtggaggcaaacctgggaaacgaccagtttggggtggaagatatctgtcagcagctggctatttcaaaaatgcagctgtaccgtaaagtaaagttgttattaaattgtaatgtgaacgactatatcctggatgcgcgggttaaaaaaggcaggtacctgctggcgaattcaaagttatcggtagcggaaatagcctatgagtgcggattttcctctccagcctacttttccacagtgtttaaggcgcgtacacagcaaacgcccaaagcattccgtgacaagaaaagcgagggatagttaagggcataaaaaaagggctgatcttgctgatcagccccccagaaaataagatatgtaaacttagataacttttacgttaactgcattcagaccttttttaccattttcaacttcatacgttacggtgtcattctcacgaagttcgccagtagtaccggaaatatgaacgaaaatatcctgtccaccattagatggagtgatgaaaccaaatcctttggattcattgaaaaatttaactgtaccttgttgcattatattgtatttgctcacaaggtagtctaatatatccgtatcacctaagagtttttttcctgatagtggtccggcttgctctaaaacaagagctgaccgggttttacgcggtcagctttttttaataaatataagtgaacagcaaattattgcttaattgcccaccataatggtgttaatacttcgtctccgccagctccaagaaagctgacagcctggttgtatccggcagcattggtattcttcagggaagaaggatacttcagccgctgcgggaagaacttcacattgctggtcatataattggaagcattgagtgtgggcaatgtacccagtggctcttccacatttggattctcgaagaaaggcaaaccaagtctgcgtttatcattccatccttccagcggcagccagggcacctgtgctatatatttctgggtaatgatctttgttaagagatcgtttttaacggtaccattcttatacaggttattcacggggtacttgattgccacggtgcctgccgtattggtataaccatttttgaaatccatggtatgggtagcagggggctctatggtatgatcccagctaacagaagtaccagtcatgttatagctggtagaggccaggtaagtacccaggaaaccatccacctgccagtattcgaaactctgggcgatgcctttttcgtaggcggctttaccacccagtggcaccgtccatcctcttaccgcagcttctgccagcaggaaatgtgtttcccagggagcaaagaagatgcgtttgttagcgctgttcctgaactgctgaccaagacggggagcagcgccagggaaagccctccactggttcctggttccttttacgccccatgcgcctgcattggaaccgttccaggcaaatttaccgtccagtgttttcaccacggcgccggtaccgtccagcaggttacgggcagttgtttcccaggtgggccggtcgtaagaaggatatttactaaagttgggatttgtaaaatctcctgctgggataaatgctttataagcacgggggtcaaccgtttgcggtaacccatcgaaccagaaacctgcaaacggatcattcgtcatggtagagaaatggtctgtcagctgcaaaccggcccagttggctggtctgatgtatgattgcagggaagcatctacctggtcagcagtttttacacttcctaaaccggtatagatgttttccagggtggtagacaggatctgggaattccattcgcggctcattacgccgctaagtgcatcccatcctggtttttcctgtacctggaaaatatcggtcatgttagtcatcaagtcgcccgctgctgctgcctcaaattctgttttagctttaccgggatctacttcagacaaacgcatggccaggcgtaaacgcatggagttggcataacgtttccacttcatgaaatcatatccaaaagcgggatcggttttcttcagttcatcagatgcgacaatagtggtgttcagcttggagctggcatccttcagttcatccagggcaaagtagtatacatctttcacgcttacgaattcggggttggtaccctggaatgcgttgatgggaataggaccgaagttatcggacaattcactcagcaaataagcgcgccagatacgggccacctgtttcaggttatctgtataaggtttggtatcgccggcttgtgttttttcatcagcaatctggatggctgtattaatgctgtttaaccagccggagctatagcgatagtattcggaagaccatccgtcatctactgcgccggaagacaagcctccgctgaggtgctgccggctggcagttttccagtataatacaaaagaacgttcagcaatattgggatccatctgtgcgccgataatggaattattgataaagtattccacctgtacctggttaaggctggcgtctttcggattttgattgatctcttcaaatttattacaggcagacatcaccatcgcgaaagcagccaatgcccagcctgattttatgagtatcttcttcatttcagttacaattaaaagttaaaaactaaggctcaggttcaccaggaaagtacgggtggttggaggagcaccgttttcaaaaccagtggcatttgtacctaccgcaaatacggattccggatccaggccgcgcatacggctggaaatcatccatacgttgttacaggatacacctactttagcagactggataggtgttctgcccagtaatttttttgataggttatagctcagctgaacatttctgagacggatattggaagcgtcgtagatgttcagttcagacacgccgagattacctacgttggtattcactgattcccaatattgctgtgtagtgattgatttggtattggcagtataaccgccggcgccatttgatactaccccggcaagtgtcatgtcatctctttttccaccgggtgcagtgatatccgctgttccggctctctgcatcattgcctgggttacagagaacatgtctccgccaaaacgggcatcaatcaggaaagccaaggtgaagtttttgtaaccgaagctgttggtaataccgagtaatgctttggattgctggttacctaaacgaacattctgttcgccacgttgtggtctgccttctgcagtgagcagcagctggccatagtgttcactcttttcgtctgttacacgcaggaatttactgccgtaaatttcaccgtacaattgacctgcaactgctacgatggatacatcatcgaagccacccagctggtacctgtttacattatttgcggcagagatttcaatgatctcatttttatttttagacaggttagcggagatattccagataagtcctttggcattatccagaatctttgcatccgccatgatttcaaatcctttgttctggatattaccagcattgatctttcttctctcataaccgctggcagggtccattggcaggtcgattagctgattagtagcattggatttatagtaactgaagtctataccaaatctgttatctacaaagcgaagttcagcacctacttcataagatttgatcagctcactacgaacatttggatcaaagagggtagttttcctggaggcaatcgggttgccatttggatcgcgatcaatggtatacgtattcaatatctgatatggggataagccgttgcccaccgctgcataggaaccacggagtttgccatagctaagccattttggaagactcttgaattgttctgtaaacacataggagaatcccaacgaggggtaaaagaaagaacgattgtcaggactaagtgtagaagaccaatcattacgcatggttgcatccaggaacaagtaaccatcccagtttaaaccggcagtaccatatacagaattaatacgctgttctgttacatcatctgtaatacctggatttccctgtgaatttttgatgctaaacaaatctggcaccagcagggaggctgcattattgctcagcctggaggagtgttgctgcatgaggttaccacctacgctaacggagccgcctaaacggccaaacaggttatctttctttgcagtgatcaatgtactatagttcaattcagagaatgtaaacttaccaacactgtaactaccattggtagagagtggactacctgaatatgttttagcttccgtatttgttgtataaatatcggcacctgcttttacttctgcatttaaccaatcggtgaattggtacttaatgcttccgttcatgataaagcggttacgtttatcctgattctggctataacggctggcccaataagggtttacctggttaccggtaccataccagcgcatggtgcctagctcatttaaaggatttttaaactgagtgatgtccatactaactggcattgtatacagcagggaagaatagttcctgctgtttactccactggtgggcctgttagtagcatctgtatttgaatattgtactttgaaatcggtagataaccgttctgcctctccgtatttggtagttgccctggccatgagatttactcttgaaagcttcgtaccaggaatcaggctgttatcattcatgtagttaagagaggtgtacacagacgttttatccaattgttgctggaaagaaatgttttcgttgtgattaactcccgttttgtagaaattgtcgatgttattaaagtaactaagcttttccgttttgccgttccagttagttacatcctgtcctttgatttttggtccccaactatttccaccaataggatcaaacgcatctacagaaccctggccgaaactcttttgcatctcggggtttgtaaacacgctttcaaagcccactgtagatgacacagcaatacccataccgttggatttcttaccagttttagtggtaacaaggatggcaccattacctgcacggctaccgtacaatgcagctgcagccggacctttcagcacagagatactggcaatgtcgttagcattcagatctgcaagaccattacccatatccagtgatggattccagaaatcgttattgccatcagttacaccgacaaagttatcgataggaacaccatctaccacaatcagtggctgattgctacctcccagtgagttgtttccacgcaaattgatcttcgaagaacctgcgggacctgtgctggagcgaatcacttgtaaacccgccaccacgccggtgagcgcgttggtaaggttgggttcatgcgcatcgatcagtgtggcgcttttcacctcctgcatcgcatagcctagggacttcttttgacgagtgatgcctaaggcagttactaccacttcgtttaaccctttggaagtttcttccattaccaggtcaaaattaatggaagtacctaccggcacttctttggtagtaaatcctacgctggaaacaaccagtgttgccccggggcctacctggagcttaaatgcccctttttcattggttgttgcgccattggtagtacctttttcaatgactgttgcatagattacgggagcgccggaagcgtctttcagggtaccggatacccattttttttcctgtgcggaaacgctttgatagcacgtagccactaaacacgttagcagcaggaagcctagccaccttttcattagtgtgaatttagatgaagatgaataatcaaggcatagtttctctgatggcatgggaagcccgcatgctgcaggtagttactgcctcatttttgattgatacaagtgaacgttattgctttgttttactacagttggcctttatcgaggtgttccataacaagtgctgcagcgccaagtctttccgccgcataccccagaggcgagattattatttcaatattttcagcgatttttggtatacaatgttcatttaacgcatgctgtacaggcgccagccataactttccggctaatgttcctctcccgcttaaaatgatcaggttaggattcaacaagtgaataaggatggcgatgccgcgtccgatatgataacccgcctgtgataataattccactgcgtaattatcgccctttaccgctgcatccataatttttctaaacgtgtcgtcgcggttgtccatcgacaaatctttcataaccgtagttcttccttccctgataccagctactgctttttctgcaatcaccgacaatgaggtttctgtttccaggcatcccattttcccacagctgcagatcttattattggtaaaaagcgggatgtgtgagaactctcctgcaaatccgttttctcccctgaaaagatccccgttcaacaccattcccaaacctataccccagcctatattaatgaccagtgcattttgcctgttccgggctgctccaagcttccattctgccagcgcaattaagctggagtcgttgtcaatgatcaccggtaaaccggtaagtgcttcgaggtatccattgatactgccgtattgcttgtcgaagaaagaataattaatgccctttgttacatctacaaaacccggcatcccgataccaatgcctgcgaacttttccaacgggattcctgaatgatcgataaatgctttcagttcctgccccagttgtgcgatggcgtccggatgtgctgacaggtccagcgacaccaggcgttcttctcccactatcctgttctgcatatccagtatactgatactggttacaaactggtccatcgctaccgataaaatgtacatgtagtccggcttcacagagtacatctgcgggcgccttccgccagtggaaatggcataccccgattccaataccaaaccgcttttcacgagttcattcaaagatttggtggtatgcgggagactcttgccagtgagcagcgtgagatcggcacaggataattccttgctaaagtacaggtgttttaataacgtttttttaaatatttcctggcgatcagacaccatttagatgattgtttgcttacagtttaaatctacatcaatttggtacaagtgaacaacattatcagtaaaatgctgattcaagataggcaaacttctgtaaattttgcaagaacttttatgaaaattttaattagttggcgataattatccaaattatacgataagttatctagtaaatgttaattctgcattataaaaaagcaaaatagttccagatcatggccaagttggccccgtgcaccggtatgataattgatccggcaccggtatgccttcatctgtggtagcccgtatgatatatgacgcagaaacgcgtacgctccggattatattcgtgtcggggatgatatatgattacaaggacgtgcctgaagcggtatacctggcaatgaagtcgtccggttcaaagggcatctatctcaacaaacacatcaaagggcattatgattttgaaaaggtaaaataaccattatgcggcgccatgcatggcctgccgccggatatcgctcatccccttccggtaaaaccgtttcatcattttattcaggtggctgctgtccgtgaaaccaaggtcccaggcaatttccttaaagggcaggtcggtgtacagcgccttcgcctccgccagttttaatttggaacggagcacaaactcctggtaggtttcaccggcgttacgtttgaaatattcgctgaaataagtagccgagatattgaaccgctggcataaataagacaacgtaattttttcttcgtcgagcaaatgatattgaatgtgcaacagtacatctgcaaaacgtttgccttccaccccttgtgcaccgggaagctccatcgccacattgcgggctatcagctccagcacggctaccatcagtccctgcataatgcgccgggaatgattatcggaacgctgctgctcatacatcagtaactccagtaaacgaaccaggtgctgtttgtcgctatccacggtgatcagctcccctgccctgcggttataattaccaatgatgaaattgaggcggcagaaccatttcccgaaatctatcacacagtcctgttctcctgaaaaaaaactggcgttgaactggataaacaggaaagtagtgggctgatctatccggtaggtatggcagtcggacgacggcaacaggaaaatacttcctttgctgtaaccggaacgggtatgctctacctgctgttccccgctgccttcgaggatatacaccagttcaaaaaagttgttcctgcggttgcgtttttcccagcgctccagggtggtgatgctgatgctaaacgggtcgtgtaccttttccatactgcaaatgtaagtaataaactgccgctgcataaggggcatcccatcctgttactgctgtttccttttacggtacgggcgtaccggcgggcggctggttagctttgctgtcataaaaaatgaagatcatatgaaagcaattattttagaaagactggataaaaacgcccccctcaccctgtcacacaccgccataccggctattgctgaggacgaagtactcattgaaaacaaagcgacaggcattaacccggtcgactataaaacactggaggactataccacacccgacggactacgggccagctgggcccctgccctggatggtatttcgccgctgatcctgggatcggatattgccggcgtggtaacggcagtgggcagcgccgttaccaagttcaaaacaggcgacgaagtattcgggatgatcaggatgccggggcatggccgcgtattcgcggagtacgttgcggcgccggctatccatcttgctaaaaaaccggggaatatatcctttacagaagcggctgcagcaacactggcagcggttacggcatggcaaaacctgcatacgcattacacggtaaaaaaaggcgaccgggtgctcatcaccgcaccggcaggcggcgttggtcattatgccgtgcaaatggctaaagcagcaggcgcctatgtaatagccgtaactaccgccgccaatgctggttgggtacttcagttgggcgccgatgagatcatcgactatcatcactttgattttgaacaggctgatagcctgcaactgaacctggtactggattctggcggaagatacccggcctccctgtatgaaaaacacttcgctccgggcgccgccctgttctacctgccgcatggcctgccggcagctaccacccaatactaccagtcgaaaggatttgatgtacgcttcaccggcgttacctccgacgaaaaagcgattgacgccatcgccgtattgctgcagtcaggaaaaataaaatcttacatcgataaagtgtttccgttcgaccagatgcgggcggccatagatgaaatgaaaaagggcactacgaaaggaaagatcgtagtaaccctttaacaaacatggataacagccggggtatttccggctgttattaatgcggtagtagctccgccagttttttatccaggtcttccccacgcaggtttttggctactattttcccggcaggatccagcaggaaattttgcggtactgcacgaacgccgtacaatttcgctacttcattttcccagtatttcagatcagatacatgcgtccaggtaagttgatcggtatgaatggctttcagccatgcatcgtgcccgttggcctgatccaaggatacgcccaggatggtgaaggactggtctttgtatttattataggctgctactacgtgcggattttctgcacggcaggggccacaccagctggcccagaaatccaccagcacatatttgccgcggaaatcggtaaggtttaccggcttgcccaatgtatcattttgtgtaaacacgggcgcagtagcgccaatagcggtttgcttccagccattgatcagcgcagccacttcttttccctttttgctttccttcaccccggcagataaagtgttgaaaaccgtttccagctccgcagggttttcgggaatggagccggcactgctttgcagggcatccaggcttaccagggatgcaggattttcttttataaacgcctggtagatctttttttcttcttcgcggatagccttactttttccatcgtaagttttccggaattccggtgatttacgggcttcttctgtagcggcaatataatcttccgtgagctgatctctttgtgcagccgttgctttcagctttgcctgcaggcgctgctgatcgttgttaagacgggaaccttttatggtagcattatacacagaatctttaccactgagaacaatggtacctttttcaaggtataccgccaacatatcagacttataagacatcatattggtaggcggggtatgacgcagtaccagcgtagctttcacagggtcgcccactttgcctttaaattcaaatacgccctgctgcaaggcggctgaatcccttacgacagtgccgttggcccggtaagtgagaaacagtttggcgggagcatccaatgttcctattttccctttcagcacatatgttccgtcctgcgccaggagcgctgccggcaataacgccagcattgatactaagatgtgtttcatttggtttttaattttatgatttaaaatggtcttccatccagcggtatattccattgcgggttaaacttcaatatcacgttggagatggttaaaataaagtcttttgaatccacggttccttcatgcgtttccgtgcctatcttatgttgtattttaggtttgcaccagggcttgccggtttcgaggcaaagtcttttcaggtccaggaaacgcttgaatgaacctagcggcagttctcttcttctttcatccagcacctgctgaatcacttcatcctgggaccctaccggaagcgtaggcgttccggttttgtaacgatagcggcgcagggtattgaggtcgccgatggcggcggccagctggttggtgcgggcatatccttctgcacgcatcagcaacagttcgggatatgagaacccggcggtcatgttggttttggaaccgcgataatactggatgcggttaccatcatcatacaccacattattgtaagtggttttataccccggcgctgttaaaaagaaatatttaaaccggaggtcattggcctggtcgtacaacgcaatcacttcatcggaaggatagctggaggaagacctgccggcgccggcatcgagattgcggtacagcaggttttcacggctgttggcagcgctcaggaaattatccggtcctttaatggtactgttgataaggttggtgggatccgtccacgaaaagctgttgtagtcataaatcagtttatcggtgccccctttgctggccgccgtccacgcgagattggcataatacaccacgctgtcgtacttctgggtaaacaggtgatagtatgccagcaatgcctgcgctgccactttattcgggcgggaaggccagttggttacttccggcacatccggtaaagcggtgagcacatcattcttcacctgtgcaaaggcctgttcctgtgtggataaatccggtaatgctgcgcctatatcagcactggttacataaggaatggttttggtatcgttgggtgaaccaggcttatacaccggaccatataccagcgtagtaataaagtacgaccaggctctatctaccagcgcctgtgccactactgtttttgcatactgctgattttctgcactgaggttgggaatagcgcgtatgccatctatcacgttgttgaaataagccatagagcggtaagtgccccagtcccagaaataatccgatgtagacggatttttataaggctgtctgaaaacatacgcccagtaacggtcgatgttaggatggttgttggctttgtaactaatattaccgataccatcggaaagcgacaggttatctgtcaggtagccgaggttacacccggtgttgttatcaataaacacccactgggcaatattgctgttatccagcaggtgatcaaagtctgccacctctgaagggatcagttttccttttggttttacatccaggaattttttgcaggagctgatacttcccgccatgataataaccagtatgagtatacgctgtttcatgatcgccgtagttaattgttaaagactgaatgataaccctacataaaattccggccgcagcgacagggaagaaaatccttgttctgtaaatgcgccggtaccaccggacaggttcagttctgatgtttcaggatcacggtgatcgctgttagcggtgatcatgaacaggttccttgtctggaaataaatccgggtactggtgaagccgatacgtttcagcaggcgcgggttaatatcataggttaatgttacatcccggagtttcatgtagctggcgctttctatgagaatgtctgaataagggaaatagaacatatccatattccagctgctgagtttaggataaatagtgttggcttcatcgcccggttgtttccatctttccgatacatgtttattcaggatattagatccgctgaaggcatctctcctcaatacattcccgagctttgcaataaacataaaagataaatcgaaattttgcacacggaaagagttggttaagctgatcgcatatttcgggcgcagggtaccgctgtaaatcaggtcgcctacagccacgttaccaccgccgcttttttctcctttggcagtatagaattgtgacacgccattattatcaaggccggcataccggtagctataaagggcatccagcggatcgcccgcttttttgatcgcaccattggtgacgctggaagcatactggtaatttacattataggtgacaaccgtattattgttgtagctgaagttgaggaaggtgttccaaacgaaattacgtttccgtaatacatcggcatttattgaaatttcatatcctttgtttcttacttccccgatatttttcaccagggaactgaagccacgggtaggatcaatagcatcggatgccagcaggtcactgctgttacgcaggtaataatcggcggtcaaattaatccgcctgttcagcagggagatatccacaccaaagttggtgctttttgttttttcccaacggagcgagttattaggcggtgaagagatactgtaagatacatctccggtataattggaataactgccaggggtaatgatcaggaaaggacctgagttcagggaaatatttccgttgataccataggatgcgcgcagatccaggcgatcaatcaatggtacatgaaagaatttttcctccgccagtttgtaggtgcccccggcagaccacaacggtttgtagcggtagcgcggatcggtaccaaagaaattggtttgatccagccggatacttccactgagaataaagcggttattatattcataggaaccgttggcataccaggaaacaaaacggttatcctggtaggcgtaactgcctatgctggctgtaggtctgctggtgcccagcatatctgcattataggaccctgcattataatcggcatagttaaaagtagaaaacgtacctgcctgatcgttgtatccaaagcgggttggcagggcattgttatctgccgtgttccggcttatttcattaccggcgatagcgcttacgcggtgtttggttgcaattacccggttaaagttcagctgtgtgcggaacatatagctctggttaaaattgcgcgcttcatttaccactgcgccatccgggatataatgtttggaaccgttggagatggaagtattatcatcgtaccattgccgcacccggtaagacgttttatcgtacagcgacctggtttgtgcatcgccgcggctccaggcacctcctgcctctatgttcagcccgtcgaagatctttacattcacgctgccgcccaaccggatctgcaatgcttttgtgttgtaggtttccagaccaagatcatccagcggattatagtacagtggtttcaaccctgttaacgcagcataccggtcttctttcttctggtttttagatggcacattcagtgtttctcctgtagccgggtctaccagcaggttgtacggttgtatcagcgaggtgttggtgaatgccagcatatcctgccagccgcgtaccggtgaagcggaagtggcatagttcacattggagaacaggcggatgttcacacctttgcggggctgccagtcgtttttcacatcaaagatgaggcggttgtctgaattccggacggtgttattctgattggatacatatcttactgcggcgttgagcatacttttttcactgccgccggataaggagatattgtgttgctgtgtaaactggtttctgaaataatatttctccatctgtgccagtccgtcgtttttcttcagggcatccagctccgcggtcacatctttttcgttcatccatccctgtgactttgcgatcagcaggtagttaacacgggaagtgctgccgtagttattataggtagtgagatagtcgttgggatcctggttatagagctctatttccgcatccacgtaatcggcggacgatgccctgttaagattcgacagatcgggtttcagcgtgatgccggtagatcctttatattctacctgcaacgcaccttttctgccggtgcgggtagcgattacgattacgccgttggaggagcgggcgccgtaaatagaggcggctactgcatccttgagcacggtgatcgattctatgttatcgatattgagagattccagtcctgcgctggaagggtacccgtcgattaccagcaggggcgcgctggcagcagtgcccagcaaggtagacacgccacggatttccaggttaccttctttggtgagcaccaccccggtggcttgtccttcaagggctgatttcacatccggtttcagtttagcgcggaggcgatagggatcaatgaccgaaaaagaaccggtggccctttcccgggaaatggtctggtagccggtgttcaccacatcgatgccggtgagcctattattggatggtttcagcgtgatgctgataacgccgtttttgcccactacaagttcctgtttttcgtagcccacataagagaacgacagcacggcattttcgtctctcactgcaacggtatactccccgttgttattggtttgtgtgcctttgccggtgcctttcaccactaccgaaacgccgggcagcggaataccattttcatcggtaatacgcccggtaattacgatctgtgccgggacagcgggcaatgccggcgtgcggggcacgatgcgtgtaaccgtaatggttttgtcttcgatggcatactccaggttctgccccatgagtgaaacgtgcagtagttcctggatagtggcgttcttcatatccagcgtaacggggcgggtactttgcagtgcatcgtaattataaaaaacgatgtagcccgtttgccggttgatggtggtaaagaccgttgataacggtgtgtttctgacagacagtgttatgcgttgtgcagcgcttttggcgctgacctgcagcatgcctgccattagtaataaagcagataacctcatgatcctccaaattttggttggcagattattttttttcattgtaccggcaaataccgggttgtaagatctgcattggtggtgatgctttccggaagtgttgatgtggtgatgatcaggcctgcggacaagggaatacgatccctcttctctgttttggaacaaagcagttaaaatcatacatttgatttcggtgataaaaatgagtttacacgaataatttattgcctgtaaccagtgatgtttgcccatcactggttttttaatggcgctggttttagttgattttgattacttctggtacaatagctggtcagatttaagtgttaaaaaatatggcatgcttacgatcgtaatacggttatttttcttccttctattttaaacagtactccatttttttctaatattttgaggatgcccgatagggacaggctgcgctgcataccgccgccaaagcgcatttcgggcggtgtaccttcgtatacaacttctatatcgtaccagcgttccagctgccgcatcacggtggtaatgtctgcccggtcgaagataaaaaagccattcttccaggctacggcttcctgcacatcggtacctgttactgtgatgttgttactgttgctgatgcgtgcctgctggccgggcagcagtttttttatgacgccattgcggcctacgttcacagcgccttccagcagggttactgccagcgcattttcattcgtatatgccatcacattaaaatgggtgcccagtacggtgatatcggcgccgttggcctttaccagaaatggttttccgggcgccttagctacttcaaaatatccttcgccggtgagttccacggttctgttgttacctgtgaaagctgtaggaaaacgcagggagctggctgcattgagccatacctgggtgccgtctggcagggtaagttggtattgtccgccacggggagtagttaatgtattataagtaaccgcggcggtagcgccggtggcatggtacaatacctgcccgttttgtaatttgatgatgctggtgctgccttgtttgccgagcgtatcatttttggcttcatccagcacaatttgggagccgtctgccagggtgagcatggctttattgccgccgggggcgatatcatttttataacgctgtgcgagtgcaggaacgggtttcatggtggctaccggccggagcaggaaatataaaccggtggctaacagcaggccggtaactatggcggcagcccaccagaggcggtgtataaacttcaccggttgcacggtttccacaaaaggagtggtaaggtctgcgccggtaatactttgcagcaaagcggtgcgggcggcggtatcgacgggggcggtatccgcaggcgcctgccacatcaggtccgtcagcgcggccatgagtatttccatgttgccgtcgtcttccagcaatgtgtacaactcttcctgctcttcgaccgtttcgttaccggaaagtcgctgttgcaataaatatatgaccctttgctcctgcatgcgtaaaaagaaaaccgggatttaaacggctccccggtattaagaataggctaacgacctaaaggacctatctgtttaaaaatatttttacctgcaaataaaaatcaggtaaacaagcgggatggcatgcccgttgcgacgcaggtgctcccgtatggctttcagggaaaacaccagggcatttttaacagagttgggcgacaaatccagctccgtggctatttccgggatcttcataccacgattgcggctcatctggtaaatgcgccggcgttgcggcgacagcaacatcacggcttcttctataacagtatgcaattctttcagtgtgagccgccgggtagcggtatcggcgtcatcggcggtaaccactgccgttccgcgcaggcggtattcgttggcttcttttttcaggtaagtataacactcgttggcggccactttaaacagccaggctttcggatggtcgatgtccgcgagcttgtcgcggctcagccatacccgcaggaaagtagcctggatcacctctttggcgttctcgggtgacttcatcattttccggataaatggttccagcgttgtcagggaagtattgaagaggataccaaacgccgcttcatcgccctcagaaatgcgctgaaacagtgatttgtcaatatagatattgtcgtgcattatcgttgcagaatacgctgatggttgataaggttggtggtatcgccactaaagtaatgaaaattgagcggatcctcactgcctcctcatttgaataaatcagatctcattcaggaagtctgtcatcgactgctccgtcagcaggttcagtttcttccggaggcggtaccgctttatttccacgccccgcaccgaaatggccatcagctgcgcaatttctttggtagataatttcagctgcaggtaagcacaaaccttcagatcggtattcgtcaaggcagggaatttgcttttcagcttcttcaggaagttattgttgatctcatcaaaatgagcggcgaactgatcccagttatcattattcttttctacatcatttaacaataacagcgcgttcttgatttccgggttgttaccattctttttatataccgatgccaggatatcttttactttcaccagcgcatcgcctctctccaccaggtgcatggatgcatctgccagcgcattgtttttaaaatgtatttcattggccagcttttcattctgcagtttgatgatttccttttcgtttttttccagctccagctggtgaatatatttaagacgctgctgctcctcgtcaaagcggcgctgctggatgcgcagggtcctttcctgccagcggttcaggagatatagcacagcgaggaacaacaacacatagccaatatacgcccaggtggttttataccatgcgggcagcacttcaaaactgtaggtcaccacttctgattcatgtccgaggttatcgtgtgcttttattttaaaaagatatttaccgtccggaaggttggtgtaatccttctctgttttgggcgaccaggcggaccagcgctgatcgtatccttccagctggtagctgtattctatattactttgcagtccgtatgccggcgagctgtattcaaaatggaaggagttatatccttttggtaaagccaccatttcggtgtcatcctgtaaataacccgcagctccgcggtgatggaaatagccgccgaaaataacactgtcggatttaccaaaagcctttacctgccccagtaaaaccttcaccgcctgtttgttggtggtatacttttcatagttcaggtgaatagtgcctttttcggagccaatgaaaatattctctttattatagggataaatgttttcaaatcccagtaatatcttgccgttcagctctggtatccaggtaatggtaaatggtttatcgccggaagactggttgaaattcaccaccccaatatctttgccgctgcagaaccagatattgccgtcggcatcttcattcatataccgtatttccatgttgcccagtatgggcgtcaggaaggcggaaggaacaaaccggttggtggccggatcaaattcatacacccctttacccgtgcagaacaccacgcggttctttatcttaaaaacataattactcagcgctgaaggcagccccgcactatccgtgagtagttgggaagaaacggttttgttatcggcggacagctgcagcttataaacgccccggtacgggtgcgacgcccagatggtgttgttattatctatttccaggaagcgcagcgactctcccactccttccagttttcctttatcggtaaactggcccgcattgtattccagcagctgcacgccggtataactgcctaccagaacgttttttgcaggatacactgccgataccggtttatacagccaggcgccgggttcagcaaatagcggcacggcactgtgatctttcagtacagcgctgccggtgtgttgtgccagcaggatatgattgttcacctcatcgaggcgccacacttctgccttgctgttccttacgcgggtaaaatcacctttggagaaactgagatcgcccgaggcagccgccagcggcacgtaccatgcgccgtccgatgtggcaatgtacagttcattattaaagatacgggtggagtatcccgacagctcattgcttttactgggtgtaatatattttatggcggcattgtaggcgataaagctgataccattattgagcccggcccagaggttattatgtttatcaaggaagacgctgatcacgtcattattctggagtccttccgtgcgggaaatcttttgcaccacttcgccgttgaagttgagcaccacgcaaccttccgtggaggtgcctgccacaaattccatggcgttgatctgtgcggagatattcacattgccggtggaaaaggctgcgtgttgctggatgatggagtcgttgcgcagaaggaattgtccttttgcctgggttatcaccaggagcgtatcagccccgatgcctataatgccggatatgaggccgtctgtaaatttacggccggtattaacgggctgccattcattatttttaaacagcatcaatccattatacttatcctgtgcatacagtttatggccggcctgtttcaggtacagccactcgctgggatatactttaatactgttattccggtattcgaagatgcggtcggaggcctggaagaaaacagcttctttataaatttctatccgccagatgtccgcaaacttattatgtgaggcaggaacaaggtccctcagggaggtataaacgagattaccgtttggcccgggtgcgaagtagccgagttctccctggccaccggcatagatccggtcgaccgtatcaatggccaatgcgcgcacaatagtacggtttggaagcgggtatgctttccagtgactgccatcataggtaagcattccttcgttgttggcgaagtacatgatgcctttgctgtcctgttcaatatcccaggtttggatgcctgcctggaagtcgcttttactataattgatgatccggggtaacccgatcgtattctgacctgcggccatccggaaacacccgatgcataaaaaaaacagccaccatcttttcataaaatataggattacttccggtgatgtagtaatgatgtagtttaaatttattaataatcaatcatttatccaattgtgatgcagtatagatgtagtcggaaaattggcttcgttctgtggaaggtgtaattttagcccaatcaaaacagtataaaaatagtacttagtcaactgaaatcatccatccatttaaaaaaatgcagaacaccacgatgctgtaaaaaagatcacctgcagccataaaatgaaataaacatcaacgggatttcacgtttaccgccagcacaccgatgctggtgaaagtaccccgcatgtaaaatcgtcaacaaaaaattcacgtatgaaaaaactcttacaaagcattcttatcccgctattgctattatttgcctccacattgtgggcgcaaaacaaaaccgttaccggtaaggtaacagatgaaaccggggcgcctatacccggcgcttctgtaatcgctaaactttccaaaactgccgtagcagcagatgccaatggcgccttttctatatccgtaacaccggaagagaaagtactggatatctccgccatcggatataccacctttcatatagcggtaggagcttccccgttagcagtacagctggcgctctccaataaagaactgggagaagtagtggtagtgggttacggcacccagaaggtaaccaaaatatccggcgccatctccacagtgaagggagcggatatcgccaatctccggcccgtaagggcagaagaagccctgcagggaagggcttccggcgtaagcgttatccagagcggttcccccggcgccaagcctactgtgctgatacgcggtatcccctcttacagcggttccgacccactggtggtaatagatggcgtgcctcaaacgctggacgatctgaatgccgtgaacgcagcagacattgaatccatcaacgtgctgaaagatgctgctaccaccgctatttatggcgtaaaaggcggcaacggcgtgattatggtcaccacccgcagcggcagaaggaatcaacggcccgaaattaccgtgaacgccaattatggcatacaggaagtattcaaaaccataggagtgctgaatgccactgaatacgccggcatcatcaatgaaggcagcgtagcttccggcggcaacatcatctttccagacctttccaaaatgggcgtaggtaccaactggcagaaagagattttccaccaggcgcccatgcaaaattataatgccagcgcaagaggcggcggggacaagatcacctatttcatttccggcagctacctcggacaggatggtattgttggcggcggcagtaaatccaatttcaaccggatcaatggtactgccaatatcaccgccgatgtcaccaatcgcctcaaattgatcgtgaacaccagcttcgccaatattaaaaataaaggaatacaggaaaattcgttcaattccattatcggcagcgcactgaactttgatcctaccctgccggtatataatgaaataccgaatacacccggtaaatatagcttcagtaacctccttacctccgaaattttcaacccgcttaccaaactggaaaatacctacaatacttccagcggcaacaaactgttcggaaaagtagaactacagtacgacatcctgaagaacctaaaagcgaccacccgctttggctataccaattacgaccaaaccggcaagaactttacgccgctggtgttttatggtccgctgaacgtggaaaacaccatgggtgcagatggcaatgccattccgctcaaaaatgaactgggcatgctggcgggttccacccacaacagcgtgagcgagtttaagaacagcgcagccagttttacgtcagagacctatctgaactataacttcaatatcaaaaatgatcatcactttgatgcggtagccggtatctccttttttaaatctactaacaacggcatgaccgttacccggcaggacgtacctttcaactcgtggcagtttgcagattacaacgccgccaccggtatcaataccgccgctattccttatattatagatacggtgatcaataatgtaccagtaaagatctataactccaaaggagatattcccgccaacctgaacggacaaacagccagcaaatacaacggattccgtaaaaatttatcttacttcggcaggatcaactatgattacaaagataaatacctcgcctccgttaccatgcgcagggatggttcctttgcctttggtacagataataaattcgcagacttcctttccggttcactgggctgggtagcgtcttcagaaaatttctttcactttgattttgtcaactatctgaaaataagaggcagctatggtactgtgggaaatgaaaacaccaacccggctttccccaggattgtaacaggcggtcctaattacgacgacggcaataacaacggatatacttttggcaatactttcctgtcgggatctaccgtaggttcttatgccaatactacgctgagctgggaaaaacaaacccagtttaatgctggctttgatgttaccttcttccataacaagtttaacctcagcgccgattacttccagaaaagcgtaaagggtttgctgttcaaacctattgtatcccttttcctgggaacggctaaagtgcctgatgccaacatcggttctaccaaaagtagtggtatagatctcaacctcggttacaccgataaaataggccgcgacctttccattaataccaacatgactttcaccacttccaaaaacgaagtaaccggcaccaactctgataactccttcatactgtatggtggcagttatttcaatggtcagtcgcaaacggttactgcttttgaaaccggcaaagcgcccggctatttctacggattcaaaacagccggcttattccagtcggccgacgaagtaaacaaagcgcccaaacaaagtggcgcgcagcccggcgatatccgctttgtggatgtaaacggcgatggagaaattacggacaaggataaaacaaacatcggcaatcccttcccgaaattcacgatgggctggaacctttctctgggttataaaaacttcgacctgaacattttcacgtatgcttctgttggcaacgacatctaccgggcatacgaaagaaatgctacatacaccaacaaattccgcgatatactcgcccgctggaccgggcccggaagtaccaatgatgcccgtcacccacgctactcttttacggacgccaacaataatgcgcgggtatccgaccgctacgtggaagatggttctttcgtaaaactaaaaaacatacagctgggatataccttcccccgttctgtgctggaccgtgcaggatttaaacaggtacgtgtgtttgcccaggttaaaaacgcgtatacgtttacccgttactccggctttgatcctgaaatcgccggtggtataatggaatcgggcatcgacagaggcgcctatccacaggccaggacctggtctttaggtattgatttaaaactgtaatgttcaaagtaaaaagacaacaaatgaaaaacatactgaaaatagcaggcatactttatttcacgattgccatgagctcctgcaaaaagtgggtcgattacaaaccgagcgacagctttaacgtaacagaccaggattacctgaaaagtgaaagcgattaccggaccatggcggtgagtacctactctcctatccagtggctgaaccagacggtacccattggtgatattgcttccgacaactccgtaagcggcggtgaaagcgcctccgatgtattgggattacaacagatggatgattatgccatcaccaccaataatgattacttaacggagatatggtctgcttcctatgagggcattaaccgtgtaaactacctgacccagtttaaggataagaaccccggcggcggcacggttgattttcccggcaaagaagcgctgtatggagaaacctatttcctgcgggcgtattattatttcacgctggtgaaattttttggagatgtccccctgtttgctgataaaagattaacactggccgattccaggacattgcccaggtctcccaaagcagatgtatataaacagatagagctggatctgaacaatgccattgctgtattacctgctacgcagccacaggccggacgtattaccaaatacgccgcacaggcattgctggggaaagtactgctctatcagaacaagttcaacgaagccgcggccatgctggagaatgtggtgaatggtccgtttacgctggtagctgaatttggagatatttttctgcagtcaggagaaaatggtattgagtctgtttttgaaattcaatattccaatctttctccctactacaactggggcgccgctacccgcggacagggcaactatgctgtacagcagtgtggaatacggggattaaacggtggcagtccctatgcctccggatggagtaccaacttacctacccagaaccttgccaacgcctacgctgcaggcgatcagcggaaagacgttacggtactggatatagaagcctacaaaaatgcacacccggattttaaaattacttaccaggtagcaccttataaaaataccggtttatacaaccagaaatatttaccaagaaaaggagaaacttccggtcagctggaactaaactatctcaataactacagaactatccgttatgccgatgtattactgatggccgcagaagccaacaaccgtgctaccacacccaatgatgccaaagcacaaacttacctgaacaaagttcgccgccgtgctttcagtgataatgcgcacgatattaccttaaccggcagcgccttaacagacgccatctggaaagaacgccggctggagctggccatggaaggcgaccgcttctttgacctcgtaagaacaggtaaagctgctgccaccatcaccggtttcaaaacaggtaaaaatgagttgttcccactgccacaaagggaagtggaaatatccaacttaccacagaatccagggtattaatcgcttatcagtaaaacaaaaagcatgaaaagactttcatatatactactggcatttgcgctaagcagttgcaccaagttaacagacgacgatctgtcgtttttaaattccatacaagcgccttccgatgaatcgctgttgtttaaaattgcggatgataattccgggcaggtaaccattacgcccaacagcgcaggaggtaccagctatgatatttattttggagatgggactaccgcacccgtaacggtgttacccggaaagaacaccacgcatgtatataaagaagggatatatcccgtgaaggtggtgaccaccggtttgagcgggttaaaatcggataccaccgcacagctgaccgtcactttccgggcgccggaaaatgtaaccgttactactacgggcaacgcgcatgaactcaccctatctgccactgggctgtatgccaccggtggtttcaaagtatctttcggcgaagttccaaacgaagaaccggtgctgattgccgccggcgccaatataaaacacacttatgccaaaggtggtgtgtataccgttaaagtggaagcattgagcgggggaaaagccaccaccgttgttacaaaagacgtgacgatttatgatccgctcacactgcccatgacctttgagctgccgaccgttaactatgcctggggcgactttggcggcagcgctacttctgtgatcgccaatcccgtgcggagcggtattaataccagtgctaccgttggtaaaattgtaaagacaaaagcggaagtatgggccggcaactttattgtaatgaccgatcccattgattttacgcagcacaaaaagttcagggtaaaagtatattcctggcgcgccggcatgcgggtattactgcaactggaaagaaacggcgataacactttccaggaaaacgtggagatgaccaccactgtagcaaatgcctgggaagagctcacctttgatttctccggaaaaataaaagataacagcaaacgcctgcagaacatcctctttttcctggacaacggtgtaacgggagatggcagtaacaacttcacccttttgtttgacgatattactttaactaactaatccacggttatgagaatacatataaagctattaacaccggtgctgctgtttgtattgatggtgatgaacagttgtaataaagatgatttccggttcggcgatatcatcacaccatccaaaccggtcttaaatattgagatcacgggtaaagacgccacacatccaaatggcggcggcgcaggaacgatagtggtaaatgttgctgccgacaataccatcaactataaagtagattttggtgatggcaaacccgctaaaacatctaccagctctgtttttcaataccaatatgatcatacgggcatcaaaacgcttaccgtaagcgtaaccgtttatggaaaggccggcaacttcagcaccaatgcacaggagatcacggtattcagggcatttgagccggatcctgcttttgtgaccatgcttaccaacaacggcacaaaaaaatggcgggtggataaagacaatcccggccacctcggtgtatctgatgcggcggtatttaccccagcatggtgggcggctggtccggatgaaaaagcgggcctgggtatttatgacgacgtgtataccttcactgcgaacggcaatgcatttacccatgaaaccaacaatgatatttttggatctaaagagtacctgaaagattttgatccgtcgcttaccggcgagggtgactttaccttaacaggtcctaaagctgccggctacacggaaacatttggttacgacggcagtgccaccgcggagtatattactttttccagcaaaggacacctgggcatgtataaaggcgtacataaataccaggtacttgaaagaacggctacgcagatgaccttgcgttgcttacagagtcccggtgcatggtatgttaaaataatagcaattcaatagcgtatgaaatatatcacaggaatgatgctggcattactgatcagtactgccagctgcggaaaaaatgaaaaagcgccaccggcgaaaaccgcgcccaccaatctgacacttcatgtggtggtaaatacagacaacagcggggcagtagcttttactgctgctgccaataacgcggttagttatgattatgattttggaaatgggatcaataaaaccgttgccaatggtattaccaactatacctatcccggcagcggcacctataccgtaaaagtaacagctaaaagtgcagatggacttacgctgagtaagtccgccgacgtaacggttactattgcttccgggctggtatggtcagatgattttaacaccgatggcgcgcccgatcctgccaaatggggctacgacattggcaccggcgataatggctggggcaatgcggagtcgcagtactacaccgaccggtcgaagaatgtgagtattgccaatggtatcctgaaaattaccgccatgaaggaaaactattccggcagtgcttatacctccgcaagaatactcacccgggataagtttgcctttacctatggtaaagtagaggtcagcgccaaactgcctgcgggcggcggcacctggcctgccatctggatgctgggcagtaacattactaccgccggctggcctgcctgtggggaaatagatattatggaacacaaaggtaacgagcccaataaaatatatggtaccgtgcatcatcccaatcatgccggtgctaacgccgacgggggtacggtaatggtgcagaatgaaaccaccgtgtttcataagtataccgtggattggtcacctgcattactgaggttttatgtagatgaccaactgttttatactttccctaattcaggcaatgtgccgtttaatcatgatttctttgtgatcctgaatttcgcaatgggagggcatttcggcggggccattgatccggcgttcaacagtgcttcgctggaaatagattatgtaagggtgtataaaaattaagagctactaaagaaaaaaggcgtccggcctttgcccttaccagtataaaccaggtaccgatgcgggttcccggttgtctggtaagggcaaaggccggcgccttttttattaacttatctggcgggagtatcgctccagtttttctttttctgttttggttagactgttaatccccttatgatggattttatcgagaatcgcatccagttctttctggcggttggctttttccacattgtacaggtcatcgatatctgccagcacatgatgctgattataaaagtagttatcgaccaggataatatgcggcttgtgaataattacatacatgaagaatacacagggtactgtgagcgaaataataacagcgatattttgtgtaatcgctgccggttcaatcattaacccgatgagcatgcccgccatagcgccgcccaggtgggcatcgtggcctatgttatcgcggcgtgacctgataccgtaaatagaatacaatatgtatacgatgccatacacccatccgggtactggaaacagtccgaagaagctcaccatcatacccggatacaggacgatagaagcgaaaatgattccgcagatggcgccggaagcgcctactgcactatagtcgttctcacgccggtgaatgtacagggatagcaggtttccgccaataaggcttccgaggtaaatgcaaacgtaagcgacgggacccatattagcttccagcatgacgctgaaaagcaggagggaaatcatgttaaagatcaggtgtttccagctgacatgcaggaatccgcaggtgatcaaacgccggtattccttgtacagcaggattctttctacttcaaactcatacttattgaacacggtgcggcttttaaatcctctccaggaaataaccacattagtgagaatgattaacagggtgatgataccggtataactcattttatttacgggtcgtttacaaacacccctgcaatatgtgaaatactttaaatatatcaaaatccttgtaatggttcttttcaggaaatataaccgttcccgttagggtcatatgctccaaaccgtttacagtaaaggattatgtcgatgtatatttcatccacaggttaataaatttctgattttattcaaaaaaatttggttgtttgaaaataatgttgctacatttgcactccccaaagggggatatagatcggctgaaaggcccgtctgtattaaggatcggtagttcagttggttagaatgccgccctgtcacggcggaggtcgcgggttcgagtcccgtccggtccgcaaagccactcttaaagagtggctttttttattaaaacccactagaattagggttcaagcaagaaaagcatattaagtaataacaaacattaccaaagagaaagggtacctgttttatttccgaaattggtaccctcggttaaccctatgtttttgtgagaagggtttaggaacgagcgaatttttattcgatcacctaaaatgtgtgttatgaaggttaatgaaaaactttccattctattaattctggaaaaatcaaaggcatctaaagacggaaagatgccaattactatccgcctgactgtagactccaaaagagcggagctatccctgcgtcaaaaaatactacccgatttattcattgctttttacactgtcgtgtgttaacaaaaaggcaaccttaaaaaaatcgctggttaaggccggcatgagtcagctttttcataactttaatcgagtcgggcaaagagaacccgctccggatctgctaattggtcgcctaacgttagcggcaaccctaaaatagcactaaaaataagatgaaacaggaaaatgtgcagccaaacaaatgggaaatattcagcccctatttcaaacaaatagaggttccagctaaattcatcctcttgcaagaagggaaagtatcaaaaacgatgtactttattgaaaaaggatgtttgcggacttgggttaacaatgacggcaaagaaataaccactcaattcttctttgaaggtgacagtgtatcttccattgaaagttttagaactaaccggccaagtttatacagtattgaaagtttggagccctgtgtcttacagaccatttcacaaaaagattttcaagatattattcaaaactcacctgagctaaaagacaatctggttgaacatctatttatgcggcttataaaaagtcaacagattttcttttcctatttaaaaaatacgcctcaacaacgctatgcagaattgttggaacagcatccagaaattataaaacgcatcccacagcactatatagcttcttacttaggcattacttctgtatccctaagcaggatacgtaacagaagataaaaaaactttattaacaattgttatcgtccggcggttaaatccttctcaattttacattgtaaatgaacaataaaaatgagaacagtaatcgtatataaccatcctttcgaaggaagctactgcaatgccatacttagcgtggttaccaatgggcttcgaaaagccaaccacgaaattgacctgatgcaccttgaccgggaagaatttaaccccagaatgtctgcggaggatttaaaaggctttgtagcacatcaagccgtagacccacaggtaatcgattacggtaaaagattggaaaaggcagaccatctgatttttatttttccgatctggtgggatattatgccggctacaaccaaagggtttatagacagagtattagcaccagccgttgtgtatgatcatcacccgcgaggtttcgggctcgttccccttttaaaaaacctgaaaagtattacgcttattaccacaatgaacaaacccaaaataatgtattcgctgctcatcggaaatttgattcagaaagtaatgcttagaagcgttttcaaaacgatgggatataagaacctaaattggattagttataacagggtaaaatcggttacccaggaaaagagagtcaaatggttaaataatttagaaaaaaggtttactgattttaaatagactttaacaaaaaaaacgaattctaaaaaatgaaaccagacagaaaatatgtaacaccattcatctccttgctatttatggtcttggccattacggggatttttatgttatttcatctctttgacggatatactgaagttgcacatgaattaattggaatcgggttcgtacttgccgcaattttacatattgtactaaattggaaaggcttaaaagtccattttatgaaacaagtatttatgccagcggccattgctgtaacagtattaactttaacttttgtttatctggaacgaaagcaacttccattagacattgttattgtcgacaaaacatttaaagctcctttaaaggaatcatgcaaaattctgaacatagactatccaatagccatcagaaagttagaagaaaagggctataaaataagcgacataaaaacgcttgaggatatttggaaaaaaaatgatacagatccgcaggaagttattgaattacttatggactaaactttttgaaatcaacagggcggcagcctgtcaggatgataccaatgaggtaagtccagtttaaacttacttccagggttacgttttaactgtattgggcgcgatttaatccgacaaattaaaaatttattatcctaacttattcttacaattaatgtataacgctttgttgaaaaaaggcaattaactcttttgctattttttccgggctgttgtcattgtcggcggccgtatgtcctaaaccatggaattctacacgctttgcctttggcaaagtggtgcttaatgtatcaagtgcaagtttaaggtaacgttggctccttgtccctcccatcagtagcacttcagctttaatttctttacaaccgtctatcagtccggaagattcacggaccaatatgagatcgtaatgcatcgttggaattaaggatttaaagcacacgtcatcgcccgattgtttcttagcatttgcgtttatagccatatttagcaatggtgcaattaagaagccgggcagggctgtaaacaatgaggagtcgtcggtgccttttatggcagtgaacattgcttttccaaggtttccacgggagagggctgattcatagcgaccgctccaggccgcagggtcggttcctttaaccgggatcggaggttcatagaggaccacttttttaagcgctggttccatgatggccgcttgaagtacacctattgcaccagagctaagcccgaatatcttatcagttgccgtcttatggattaatgccagcaaatcctcgctttctgatccaatgccatagttctggccaaacgggccacttaaaccgcgaccccgcctgtctggaatatatacagtgaattcagctgataagaagctagcaagtttgatgaaatttttagaagtcatcataccgccatggacaaggataactccaggcccggccccaatttgtctataaccgactcttgttccatcctttgacaccacatagtccgtagtataattctctgggaggttcattgcctgatctacgtttataggtaagaaaaagttgtgttaccctggttcatttctgtccgattaaatatcagcaattacatataaatataacgacaataaccagcatttataactttccctataatggctgaaacttcttttgctttacaatggttggatatcatttccaagaatggtcagcatcgctctaaagaacaaaataataagtcggaataagctaggttaaataagggaattaggctttcttccgttcctctgataccgatttctccatttctcttagaattttatagacagaagaatcggcaggtgcctttcgatattctagtttgatccttgtttctccaagtttatcaatacgaaaaaagccttcagatgaatagtctgaaggcttttttcgtattgtgccaatgaagctattccgttttcaaactccgcaccgggttgatcatagcggctcttactgcgtggaaactcaccgtaagcacggtgataccgacagtgattatggccgccaggatgaaaaccagtggtcctatgctgatgcgatatacatatttctccagccagctattaagaaaatagaaggccagcggagaggcgatcaaacaactgatcatcacaagaataacaaattcacgggataataatgcccataactgcatgatagacgctcccaatactttccgtatgccaatctctttggttcgctgttctgccatataggaggccagtccaaacaaaccaagacaggaaataaaaattgccagcagggagaacagaccggttaatttaccgatcaacatttccagttcaaatttctttgcataagcttcatcggcaaatttatagatatagggataagcggtattatactgtccaaagatcccggcaatcctgtcaaccgcttttgttgtactcacctttggagacaaccggtaggtaataaatcttgctccattagggttgtacataaagactgtcggagtcggcgacgaaaaaggagattccataatagcatccttggccacacctatgatctttaaattatgacggccattataagcaataacctgtcctatcgggtctttcagcttcatccgtttaatagcggcttcattcacgattacattcaacgaatcggcgcttgtgtttccggtaaagtccctgcccgcagccagatctatatccatcgttttgaaataattattatccgcaacaaacacaactgcggcgcccacttcctccacgggtgtttttcctggccagttttcgatactactgaagttcctgagtgcaatgactgtctccgaagacatggttacatccgttaccacaccactctgcagcaaatcattttttaaagccggataatttttcttcagatcgctgctggcgtcagtcatcatcaaccgttgctgatcatagcctacaggacgttcctgtgcatattttatctgctgataaataatgatggtgctgatgatgagagttatggaacaggagaattgtattaataccagcatttttctcgaacgcaccgctccacgatctgcttttaatatcttgacaggtctgaaagaagaaagataaaaagcagggcggctacccgccagtaagccagtgagcagcagatagctgaacataatgatccagaagaatacattcgtataaggaatgcggatagttgcctgtgttagtgtattaaatgaaggtaatgcaatctgtaccaacagcagcgatacgataaatgcggcaaaagtgatcacaaaagattctgccagaaattgtaaaatcagttcatatcgctgggagcccatgactttcctcacgcctacttcctttgctcttttttcagaccgcgctgtagaaagattcataaaattaatacaggcaatcagcagcacaagtatcccggtgatactaaatactcttacatagctgatcatcccacccgtagcaaccccatttttaaactccgtatagagatgccagtctttcatttcctgcatgattacttccgtatgcgaatgcttgtattcttcaggattatatctggctatgatcttcttcagtgcgggctccacctgcgcataggatactcctggctgtaatgacacatacacattggatgtaatctggccccacatgttgaggtattcttttatatcgctgttctgaataagatattcataagggataacgtagttaaatttcaaagtagaattgtccggaatatcttttaacacaccagtcactttcagattgttctgattatcgatgcggacaatcttattcagcggatcttcatttccaaataatgattttgcggtcgactccgtaagtacgatcgaataaggatcatttaacacctgctctgcgcggccttttaacaatggatattgaaatattttcaggaaatcattctccgctattattcccggcaggtatatcttcttctcgcccgccaccagtccgtgaggttttatccagtctgtcatgaccgcatgtttgatacccggaacgtcccttctcaacgcttctgccaatggcataggtgaaacaaggtaagcatatacctctccattattcccggtaccttttaaccccgccttgtagatctgctgactatcaggaaggaacctgtcataagaatactgataccagatccacaaaccaatgatcaatgccactgccatccccgtggcaagacccaatatattcagcagactatataatctattgtggataaggttgcgccaggcgagcttaaaataatttttaaacatggagataggtttgatatcccgccactaataaaataccagtttataatattataaaaatcaatgaattaaaattgctggtatttttcaacctgtccggttttgtacagttgatgtccggtttaaagatctataaatcggtcgctttataataattggttttctttaccgggaaagcaccttgtgtcagcatttgtttgtaaacattgccggtggctactaccgctcccctgtttcccgggttactggggtaggtcatcgtggagctatgtgaatagccgatcatatggcccatttcatgtactacaataaaacaaacatcagcagtcaggtagtcattcagtatatgattggctaccccaaaagtagcgccaccacctaatccgaaaacattaaccaccaccccgcaattaaatttaggaatgtctatcattttttgaaacgcggtacttttctgttctgttgtcatcaatacctgctcgttgctggtaattggttcgtttataaatacactcctggtagtatctgcctggaaaaggtaagccaggttaataataaagccggtaaatcttctcacatcctttgcatcgatattttccttccagttattattggggtcatcggttgggtcaaaatcatggtatttaatagtccatttcaatttggccagtgacttcagttttttaatcaggtctgtttcacccgtaaaatcaaatattaccttgctggtagcaataccggatgttttataggcagaaaggtctacttctttattgtcagtatcaaggaactttgtggtggttccggtaaacgggtagttgattgcctttatgccatgcgcccttattttactgatcttaaaaagtttgacgggcctggcctggcctgctatagttaacaggatagtggcgtcctgtatatctaccggcgcgaagttggccacttctatcgttacggaatcaatggcttttactcttaatactttccctatttcataccgccgggattcagacgtcattacctccatagactcgccatctttgaacatcagcccggaattatcatcgctgtcaaacgaatattcagcggtagcgacaggggcaggtccaccgtctttggatttgtcttttttacagctaaaaagtgcggtaataagcacgaataccagaagtttcttcatagattgattgatatggtcagtgataatgttgataacataaactcaatgctaattaggcaaaaaggaaccaaccaacaacttctatcctgataaatatcaatgtttttttgacgatagtgctaaaaagccggatacaaacatctttacaaaacaaaagggtatcaatggtcattcttataaccactggtacccttcctctttgcattatcttacttgctctttgccgcctttttatagtctgccagggcatcctggtattccgtaacggtgtaatcaagtatagttcctagccactgacctttctctaaagcctctttcgcaccagctatcgccttttcttctgccgcaacagcgcctttaggatcaccggctttaccataggctttggccagctcgtgataaatgagcggtttaacgccaccttctgcttccagcgcagttttgaaaagatttgcagcataggtataagcctgtttggaaagatcttctttttctaaaatagtgctggccacaaaggtgcttatgtgctgattttcttttatccactgtttagcataattaagtgctgtatcttcgctgaaatggctgagtaatgcagagaacttcatatttttcagagagatggccaggatgggattttcaggaatggccttatcgatcataccaaacgctttctcaaattccttcgctttgatagctgagtcaataggttgtagtacgttattgaactgtttggagacggcggcattttttgcagttttccgttcaaaatcttttgcaaaagcggctatatcaaattttccggagataaccaatcccatgatagagtcgagaacaaccggatgaccgatccagataatctttccttcctttagcaggaaagtggtaggaatgccgttctggcccgatgccttcatccatttattacccatgtactgatcgttgttgtcggcaatcacattgtacgccattttatcgccgatactgtttacgaactttgtaacagccggaagagatgactcatagggtttgtcgcccgttttttcccagacattcacaccaacaaacgtcgctttgtcttcatatttttttgccagctccgataaatgtggcatagcagctttacacggaccacaccaggtagcccagaattcaaatacatagagccggtccttttggtattcagtcaccggggttccctttatccatttggcgtattttaatggaggtgcggcatcgccgacatgcagggttacatcctgggcccgggcaatagttgccaggcagatacatccggccaatacgatggcctgtttgaaaaatcgcttactgtgatggaaaatattcatattaatgatgggtttacttttttattattgtttaccgtatccggggttttgatcgccaatcaaaggattggtattaaattcatccaatggaatgggaaagtagaactgctgtgtagatgttatggttggtttaagcaattttacttcgtcgaaaggaagccgcattaatgcccgccattcaatgccatcttccccggtcaggttcctggctacttcataataattctgcagcaggagatccgccgcagtattggcattgtcgacggccgtaaagtcggtcacaccgcccttagccatcactgttttaatcagcgttttagctgtttgcagatttcctccggcagaccggataatagcttccgcctgcaacaggtatacttctgataagcggatggcatatgaagtttcagaaagctgagaagtattgctcccgtatgcgatatatttcaggaaataataggtattgggagaataagcctggtaaggcgttttcggcccaatcatccagctccccctgggatcgttttccaacaggtccttcagttgctgtgtagcggtaaaaagagaagactgcaccggataatatgcgcggctttgaatatagtaaaatgcctcctggttaggttgtggtttaacgccgagtattacttccttgctggttaatccttttacataaaagagatccttcaggttgttttccagggtgtacgtgctgttttgaatgatatcatttcccagggtcgcggcggctatatagtcggcctgctgtccgtgacatagcagcactctcattttcagcgccatggctgcccatttggtaacatagtagctgggatgatctgccggcgcgttagcaatggcaaagtcgagatcttccaggataaatgaataagattctgccacagagctgcgtgctttagggatattacttagtgtagaaaacttatccctgatcagcacaccaaagcggctgtctgttttaaaccattccgcaaaataaatgagcagggtaaagtgtccatacgcccgcatgaagcggctctcagcaaggatctcatttttccgggtgtctgtaaaagctttgtcaggaactgcattcacgccgtcaatgacagcgtttgcagcgttgatcaacaggtaactttccgtccagacggcgggtatataaccagcgcctacattgtcatttttttcttccgctaacttcccgaatccataggcgagtaacccggagagcattccgccaggaatatgatgttcccgccataaggtaatattgtcggaggtcacattcgcgaaccggtagtatacgccgttcagcgcggtttgcgcggttttctgatcggtgatagcagtgccttccacgcgggcattggccggcggttcactcaattgcttgttgcaggaaaggaatgttccacagccggcgagtagtattatatataatgataaacgtttcatttgtctgaatttttacttgcttaaaatccgattcgcatcccgaatgtgtattgacgcatagaaggataggctgctgcatccgtataaccactgatcaaactatagggatcattgcttacttcggggtctggcccgggatagccggtgatgcagaacagattgctgcctgaaacatataccagcgcggtacgcagatgcagcttgttgaggagtttgtccggcagctgataattaatggagatagatttcagtttgatataagaggcatcatgtactgttgcactggaactgccggttccgtaagtattgctttctttaagaagaagcgagggcctgtcggcatcagtatttccggcactgtaatgaggaagcaatatccgtgtgttccggtttccgcggtcaccaagaccaagtgcatttacatccggcaggtacaggatatctcctccgcaggaataagtcagcagggcgattacgctgaattgcttatagctgaaagtattggaaacaccaccgtagaacttaggctgggcgctgccaattacgtcgcgtttaaaatatcccttgtataccccggtatctataaggccgtacttcggataacccagcgccaggttttgcagcaagcctaattttgcgtaaatactttctgccttgtattcttccagctctttttctgttttaataacgcctttatactcgtatccataaatcaatcctattggctcgccttcgcgtaataccgtattaccaatggagaatacggagttataataaggatcgctgtacccggtgctttgtggattttgcagatcctggttgatacgcgtaacggtagatctattccccgaaacatttgccgagacactccacccccaatcttttttacggataatatctgcacgaagatctatctccagtcctttattggtgatgtcggcgacatttaccaatgcggaggtaaacccggagctggtagctacattatatgccagcagcaggtcggtagtttttttatggtaatagccaatggcgccccggagcctggaattgaacaaggcaaaatcaacgccggcgtctttttgaagggttgtttcccatttgatgtggtcgttccccaattgcgtaggaatcagcgcattggtggatgcgtaggatcctggcgtaaacagggtgtagaacaaattattgccaagattctgagtaccggtgtaacctgcgctggcacggaacttcagctcattgagccaggtagctcctttgaggaaaggttcttcatttgctctccacgctactccgaatgaaggaaaataacttacgcggttgcttttaggaaattttgaagattcatcagacctggcagttactgtaaacaggtacctttcattcagcgcatagtttgcccttaaataatagctcaggagcgaactttgtgtttcactggctttgggaggaagtgcgagggcagcagatgacaatccgttcaggaactgatcatccgggaatccctggccggaggcagaaaatgtttgtgtattggttttctgccaggacgttcctaccaacaggttcaggcggttgttgtcgttgaattgtttgtcccaggtaagggtgttttcatagaacacatccgactgttgtgtttgcgcctgtgaagcgatgcctccgtcggagctcaccactccggatggatcagcaatgttgagcgaggaaggaatataatttaactggtggtagttggtataattaacagatgcggtgcttctgaacttaagcgttttaaagatgtcgtattccaaagcaatggagcccagcagcaatgcatttttcgaggtgttgatcccctggaggagcgccatcgggttttgaatacccgagccggcggatatagcgaaagtagcgggatcaaaaaccgctggggttccatctgcgttaaaaggcgcaaaggtaggcggggcaaaaattgcggaggaatagagcccgttggttacattattttttgtaaaggcataatccaggttggtgatcacccgcagtttcggggtgatttcattgtccaggttaattttaccggcaatgcggctgaaatcagtgccgagcagtgtgccggtttgtttggtatacgaaagagaagtataatacctggaaccgcttccgccaccccgcacgctgatatcagcattgtgggtaatgccggtacgggttaccaggtcgagccagttggtgttggcggtaccgaggaaatcggggttattgataatggatgtcgcaatggcgtctgcaggtttactttgcgaagcacggagcgcattcaggttttgggcgccttccagcattacacttttgtactgcgaggcgttcagcagtttttctgtgattgccttactcaggccggtataataattagcctcgagtataggcttctcattttttttcccttttttggtagtgatgataactaccccgtttgccgccctggaaccataaatagcggtagcagaggcatctttcaggatatcgatcgattcaatgtcattgatattcaaaccagccagggtatttaaaccgcgggcaaaggaagaacccaccgcattttttgcatagccgacgtcgtctcctaaagtttcaaccgggttcaccaggtctgcaccactctgtacataacggttttgtatggttacctgaacgccatcaataatatacaacggatcgtttccgccaatcagggaagtacctccgcggatgcggatttttgccataccaccgggggagccgtcagcctgtatcacctggacaccagtggccttccctgccagggcctgatcaatgctcacaaagggcgtatttttcacttcgttcacatccaccgaagccaccgatcccgtgaggtctttacggcgcgtggcgccatatcccaccattaccatttcattcagggtctttgcctcgggacttaagctaatgaagatattcctggtggtgccgtttactttgtaggtttgtttaccataaccaagaaaagagaattcgaggacggcgttttcctttacattcaatttgaaataaccgctttcatcggtttgagtaccggcatccgttccccttactattactgaaacgcctttcattggttttttctccgcatctgtaacccggccttccaccgccatttgcggggaaatgttttcacccggatccgctgtacgggaagcgttttctccggcaaccggtttggccgacagtacaatggtattgcctctgaagataaagttgagcggctgatctttcaataccagctgcataaaatcacccaggggcatattattggctgataccgacaccgccttcccttttgcaaggtcttcacggtttacaaacaggacatagcccgtttgtttcttcacaacagcaaacacctgttttagtgaaaggttgttgcccgaaatggttacggattgcgaatagctggtagcttttgcctgaagaaagatggcgatcgataaatacagtgtgagcttcatcaccagtaattttttacggatggatggattcatctcccggtaccctctgaaatttaaaaatggtggattgattttgaagaggtacggaaagccgtgaacccaataagattttttttgcatagattgcacttaatttggttgatttaaattgcatgacagcgtttattccgatcaagtctcaaccggaagtgggctcaatcacttccggttttatctttttacagaaattttttataagggcagaacgatcagtttcctgccttccaggcgaaaacggacgccggtggtttgcaggttggcaagcacatctatgagcggcatatttcttcccatctccccataaaaatagatatcagggattcctttttcatagacaacttcaatgttataccaacgcgaaagttggcgcattacctgttcgaggttcgcgtcctcgaaattaaagagaccatttttccatgccattaccttatttacatcggcgttagtgacttgaatactgttcactgcggtggaatcagtaacagtgttcattacccgggcctgctgaccaggctttaatatcacggtgtttgtatatacttcgtgttgttggtgatttgatgcagaacgtacattcacggctacagatccttccaggagcgtggtggcaatatgttgctcatcttcataggcatttacattgaaatgcgtacccagcacctgcagcaccgctttgttattaatacttaccaggaaaggcttgtcctggttatgggctacctcaaaataagcctcccctgtcagttccactttcctgtcgtgccctgtaaatgccgtaggatagcggatagagctggccgaatttaaccaaacctgcgtaccatcgggaagtgtgatcccaaattggcggccttttggagtggacatcgtgttataagttgcttcctttccggcattgttatattgtaacgtgccattgatcacttttgcggtggcgctgccgtgaagcggtattacaccattttggatggtatccagcaacacgtgggaaccgtctgccagcgttaaaatagcacccgcttttcctggttggataccggcggcattgatggcaaccgtaaccggatccgtgcttttcctggctaccaggaaataacttcctatgcccagtaccagtataatggaagcagcaatccatctccactgatgtaagaaacggctgcgcaatgatacaaccggcgtatttttctcctgtccatccggcgaacccaatatcctattcaatattggttgtcctgtttcagacgtataccggccatctgtttgctccaattgctcccaataggcagcaatccaatcgttcagctcctggtcgtctgtaccggcagcaatttgcgctaatacctgctgtgtttcgtcctcagtggtgttgccagcgaggtagcgggaaaatagctcttggaaaccaggttttgccatgtgcgtaacggtgatttatataaggacgattcagtatgacaaaaagtaggtagccggataaaaaaatcaggaaaaaattttcaaaataatgataacagctactcccagcccggctttttcttttacataatgggtgatggaatgaacggacaactgcatatatgattttacggtagctacagagatgcccatcattttggctatttcggcctgcttcaggcggtttcgcctgctcagcaggtaaacgcgttgctgttgcggagggagcctggcaaccgcttcgtcgatcagcgtatgatagtcaggctcgtcgtctgcgctgttttccctgagaaactcggactggtactggctttcccgggcatgccttgcggccgttttgcgtagcgcgtcaatggccaggtgttttgccatgacccagagaaatggtttaaaccggtccacatacaccagcgcctcccttcccatccagacttttaaaaaaacatcctgtactatttcttccgttaatatttcagagcgggttaaacggagaatgagggtggaaagaagtggataccattcattaaaaagcctggcaaaggccgtttcatccccttccgaaacagattgaagcagttctttctcgttatatggttgattggttgacaatatctgaaactctttctgcgtaagttgcaaactataataaaaatctgaaaagacaggatttaatatctgcttagtaaaggtgatcttcttatgccagcgttgacgaccaggtgattacactatcatctcccctccctccaaaaaacttttaaacatctgaatgaaaacagattatctttatagcaccaaccatcgtatctattttttatgtcccagtatgatatatatacagatgagcaattgatgtcactgcttaaatgcagtgatgaagcggcttttactgaaatttatgatcgctactggaaccagctttacagatctgcctgtcgtaagaaagcagataaagagcaggcaaaagaaattgtacatgatgtattcctggacatctggaaacgccgggaatccttaaccatcagccatctgcctgcttaccttgaacaggcggtccgtttcaggcttattaattatattaatcgcaataagattcccgcttttttcgatttattcgaaaccctgctgttttcgccttacgaagccgaccagctattgaaacagaaggattttataaagctgctggaaggatggacggacgtattgccggaaacccagcgccggatctttatacaatatttcctgaaagagctgtcggtaaaggaaatagccgttgaaatgaacctttcgaccaaaaccatacagaataatttaagtctttccctccgtcatctgcgtacccgttttggtactttattaactatcctgcacttttttatctgataaagaaaaaaaaataatttttttccgggaagatgtgtccttttttgtgactatactaaaaaggcgttttatgcaactttctgactggcaccagaaatatttactatccatacttgaaaagtatcatgcagggcaggcgagtccggctgaagtgcgttttgttgaaagttatatggatagcctggatgacttggataacgggtcagacaatatggaggacgacagggagttgcaggaggaaataaaagcaacgctgttgaaaagtattcatcagcccggaacgaaaaaagagatgtcctttataaaaccgaaggtggtatcgcaccggcgacggctatgggtatggagcgccgcagccgctatcgctgtgctgctggcgggcgccggcatgcattggtggatgccatatctgaaggaagcttccccggtgctggccgcaaaaaaggatatagcccccggaagtaacggagccgtgttacatctttctgacggcagtacaatagtactggacagtgcaggtaatggcaccgtggccgtacagggacaggtgaaagtggtaaaggagaacgggatgataaaataccagggagcagcaaaggaagaattgtataacgagattgttaccgataagggtaaacaatggagaatggtgttgccggatggaagtggcgtgtggctcaatgcagggagctctatccgctacccgctaagctttaacggcaaagagcgactggtcgatattaccggtgaagtatattttgaagtagtgcacaatgagaaacagccctttaaagtgcgcacgggcaaatacgtgattgaagatattggtacggcgtttaacgtcaatgcctatgccgacgagccggtcatgaaaacgaccctgatagagggcttaatacgcatcaacggaacactgatgaagcccggagaacaggcacaggccagcgcggggcaagagcaggtaaccgtgagtgaagtggagaatccggccgatgctatggcctggataaacggacagctttccctggaaagtaacaacctgcaagcgctgttaaggaaaattgcacgatggtataatgtagatataaaagtcgagggaacattgccggaaaccggctttatcggtatgattgaccggaatgtatatttatctgatgtattaaaggcattaactgtttacggcgttaacgcgcgcctggagaaccggacactaatcgtttccgctaagtagaatttatttatcaaccaaaaaccaatttatatgacaacaggatagttgtaagccaccggtatgcctgaaaataaaagccggaagtgattacgactcacctccggcgtgatattcagggtaccttatcaaccaaatctgcttaaaggacctcgtttttaaagtaccgccaaacaaaccaaatttatgaaacttattgttaatgggaacgcccctgtgggcaggggagcattattgtctcttttaatctggaagatcatgcggctgactatattattactcgccatcgcactgcatctgagcgctactacctactctcagtacattactatcaaacaggagcatctgaccataaaaaatattctcagtgaaataaaaaatcagaccggttattcttttatcgctgataatactttgctggagaataatatggtgcgtcatcttcaactgaagaacgttaccatgaaagaggcgctggatgcctgctttaagggactgccctatacctaccggatagaagatcaccttattattatcaggcatatgccgaataatatgtttccatcgattccgctgcaggtgttagtggccactactatccgcggccgtattacggacgaaaacgggaaagccctgcccggtgtgagcgtgcgtgtggaagggaaagcgatgggcactgtcaccgatgagaacggggaatttgcgctgacaggcgtagatgaagacgcgatattaatggtgggcagcgtaggttttgaaaccaggaaaataaaaccggacggcaaaaaatttctcaccatcgtattaaaaacaaaaaccaaccagctggatgcagtggcggtggtatcaacaggctatcaaaccatctcaaaggaacgcgccacgggttcatttgacgtgatcagtaaatcacagctcgacaaacccgctgttaatattgcccagcgccttattggtaccactgccggcatgcaggcaaaactggatgttgacgggaaccctacctttgagatcaggggaaaaaccagcttatatgctaatgccaccccgctggtagtagtagatggcttccctgttcagggagatttcaattccattaaccctaatgatatagaaagcatcactatcctgaaagatgcggcagcggcttccatctggggtgcgcgttccgccaacggggtaattgtcgttaccagtaaaaaatctgcccgcggcattccgctccgggtggagttatcggcgtttacccgtgtgggcagtaaagtagacctggattatgtaaatccgctggcatcgtctgctgaaactgtggattacgagaaactcacttttaaccggtggggcgcccaggttaactccggcgatcttgcttccaactattggatgcaatggtcacaggcaacggttgccctaagcgaaaattatctcggctacctgtcggatgccgatcgcgacgctgcactgacgaaactgaaaacacaggacaaccgttcccagatctccaagcacctgctggcaaatccatcggatcagcagtacaaccttacgctttatggcggctcccagcgaatgagcaatgtattgtcgctgatgttcgggaaaaagcagtcgaactttaaaggtaccagcggaaacaactacatgtttaattaccgcaccaatgccaatgtatttaaatggctggacttcaatgcctccgccatggttcagtacaacgatgcgcataacaacggtgtatcactggccgacatacagggattatcgccatacgatatgctgcttaacacagatggctcctataccaatatcagccaatactactggcctatactcacccggtctgtaccgatgaataaatttccttatgccgactggacctataatccgatccaggaggtagccaaccgcgatatcacttccaaacagttaaatgcccgcatacaggcaggactaacgttccggttaatgaaaggactgtctttcgatagcaagatccagtatgagttgtttaacacgtttgaccgcggcttatacaacgacaaaactttttatgtaagaaacacagtcaacacggctgccagctgggaccagtcgaccggcgccattaccctgaacctgccaaagggcagcatactaacgcagagccggagcaagggagagtcctataatttccgtaaccaggttaacttcaaccgcgggttcggaaaacagcatgaagtaaatgtgatcgccggttccgaagtaaccagtttcgttacacaaacttttggcaatccgaccacctatggttataatgaccaaacccttaccctgggcacgtttcctaacggaccgggaggcacttttgcaccaattaaagactggatgggcgacaaccagtcattcgcctactccaatactttttcctatgcaacagaaagatacttttctttttatgccaatggcgcctatactttcaaaaacaaatacaccctgtccggcagctaccgtacagacgcttccaacctgattaccgatgatccgcagtaccgctatgctcctttctggtctgccggtgcggcgtggcaattacaaaaggaacgctttatggccggcatttcctggatcgactggctgaatgtgcgggtgacctacggctttaacggcaacgtggataaatccaccgccttccgtccattgatctccaccacggcaataccggatctttatacccaggactttaaagcatccgtttccagctatggcaatcctacgcttcgctgggaaaaaacaggtatgtggaacttcggggttgactatacgcttttcaacaacctgctgcatggtaaggtagatgtttacaataaaagtggaagggatctgattgccatattgtccattcctgcagtaaacggtaccacttcccagaaactgaacaatgcagagatgactaaccgcggaatagaactcactattggtaccaccgttcctataaaaggcaatgatattgtatggagaggagatgtgaactttgcctataataaaaataaaatcacaaagttgtttgttgccaactatgctgcctattctctcttttccggtggcagcggcgcttatgtagaagggaaagatgccaatacgctctggagttttcagtatgccggggtgtatgataaacaaccctacgtaaagggtgcaggaaaagatatgtacaattttaccggctggactcctggcgatggccggaattacatgcaggatatgggaacattggtggcgccttatacactgggttggatcaactcgttcaaagtgtatgactttgatgtatcgtttatcgttaccggtaaattcggtcatgtgtttaaccggatgtcgtttaactatcccgtgctctggggatcgagggtattgcctaacaagaagctgggtgaagtaatgaatggcgatcctatgaagatagtaccgctgccccagaatgataatgaacccagattttatttctgggaccggttttatccttacatgaattacctggcggaaaacgcttcgcatatccgcatgcaggaactgaatattacgtatcacctgaaaaacaggttagcatccgcgatgcacattggcgggctgcagttatatgcacagggtaacgatctttttaccatcctggccaacagctccggggaagatccggaatacccgctgggtgggatgaagccgcagcccaaatttacgttcggacttaaattaacgctttaaatctgccatcatgtttatcaataaaatataccgcttgttgccggctatggctatgctgactttcattacctcctgtgataaatacctggatgagccgccatccaaaacatcgtcgctggtagttaccactactgcccatctaaatgcgctcctgaataattatgtcaccttttacagggaagggaacaggactgctatttacagcaccgatgatgcggatcttccactggatgtgtataacgcccgcccgtccaccttttccatggcacaggtagagtttacgctgtgggatatcaataacctgccggatgatggccgggaatcattctggagtggtgaattcagtaaaatctttaacgcaaacctggcgctttcttacgtggataaagtaaccggcacagatgaagagaaagcagtgataaaagcggatgcacatttcatcagagcttacagctactggctgctggccaatacttattgcctgccttacacagatgccaataaacaggaagccggtttacctataaaactgagtaccagttttgaagaacccgtggccagacaaccattggagaaagtatatgagttgattgaatcagacctggcggaagcgctgaaaacgcctgtatccttgtcggcgagcggaacgccccgccattggcgggccagcaaagcaggggtaaatggctttgcagcacgctattacttaaaccggaacaattatgcagaagcgttaaagcacgccgatgcagcattggcagaatacagccggctggtggattataatacagaaatgagatatggtatcgacggaaatataacgatcaatgcgggtacccccagcgcacaaaccgtgactattaaatacccgtacacgcataacaaccagtccgacatgaccgatatgataggctggaaggaattcctgtatttcaggatgctgaaccatgaatcgtggtggtatatgcccagcaaggcattactggatctgtacgatcatgatcatgaccttcgctatgaatatcatatcgtagaaaattattcttacgaccggggtttgatcaaaccggcatatagctatcccgggtatattttcttttttaaagacagaataccttcgggacctaccgttgccgagatgctgctgatcaaagccgaatgcctggcacggaccggcagcatcggcgaagcgctgaccgccgtgaacaccctgcgcgctaaacgcatgaaacccggtccctgggtaaatctaacagctgtcgctaaagatgccgctataaaaataatcctggaagaacgcaggcgtgaaatgccttttactcaacgctggtttgacatccggcggttgaataacaatgacgacccaaccgatgatgtaatactgagcagaactttttatccttacaccaatgcacaggtgcaaacaggacaacctctccagacttatacactgcctaaaaacggaagacgttttgcagcacctctcccacaaactgagattatttcaagtaatggtttaattgaacaaaacaaatactaaaaacacttctatatgaattgcagaaaaatgatgactaccagcatagccttactgctttcaggactggcggccacgcctgttgcggcgcaacaggcaaccatgagtgcagataaattaaaagcggtgataacaaagtatcctgatagcctgggggcgcatcgccagtttattgaagtattccgcaaaagcattcccaacgcatctttccgcaacggcgattccgttgtatcgttactgaaagaccaatatgcacaatgggcaaaacgatttccgaagtcggcaacggtgcctttcgctatcggagaggcttatgccgatgtggaaagcccgaaggccaaaccctacctgttaaaggcagtagagctgaatcccaaactggccgcggcgtggaaggacctgtctattgatgcagatcgctggggcgatcaggatggatcgcgggaatacatggggaaggcatcggcagctgacccttcggatcccggctatgctttttattatgccatggattttgagcatgttgacgggcaaaagtggcgcaccatgttgtatgatctggccaaacgttttccacaaaatgaacgcggcgcccagggtttatactggctcggcgcccggagccgggatacagcggaaaaaataaaagtatatgagcagctccgcgccgcatacccgcctgcaaaattcagctggtcggccggaggaatggaagacctgtttagcatctacctgaaaacagatgcccggaaagccgctgcattagctgccgcgttgaagggccaggagggctggggcacaaaagatacactggctggaaaaattattgcaaccaatacgtatttgcagcagcagcaattcagagaagcagccgacctgctggcaggattgaaatcgccgcgttatggaaggcagcagactttcattaccctgctgaaagccagggcggaacatggtatgggaaatacaaaggatgcttacaatgcactggctgccatttatgcaaaggacccaacagatgatgtacggagtgaactggaagtgtacggaaaggcgcagggaaaggatccgcaacagatcgataaagacatatggcagataaaagagcagacgattaaacccgctcctccttttaatctcgggttgtatacttcatccggaactgcttccctggaagattacaaagggaaagtagtactgctcaccttctggtttcctggctgtggaccctgccgcggcgagttccctcatttccagaatgtgatggataagtttaaaggacaggaagtagcttacatcggtatcaatgtttcaccggaccaggatgattatgtgttgccgttcatgaaaggaacagggtattcctttatcccgctgcgggctaccgacgattgggccgccaaggtatacaaagtacgcggagagcctactaattttctcatcgatcaaaagggacagctggtgtttacagatttccggatagacggaagtaatgagcggacactggaactgatgatccgttcggtgttggacagaaaataattttaggaaggccgggagatataaatttttcccggccctttttttgtccggaaacctgattgtgttaacagacttatttgagatacttctcagccggcattactactccgcctctttgatgctccacggctttgtagctggaaggatctcccggatctcctccggtatattcaggaaattgaggataaggataaaccggtcgttgaaacctgaatgatgaatcggcgccgcaacaacccaaagcagcggcaataattttagccggagccaccccttcttccacccacttcaccagcgccagcaaaatatcgtgttcactgtcctgttttacagcggtccggagattttgtccgaaatcattgatgcctggtccgccaccacaatgtcccatacccggtatcaaaaaatacctgaaaaaatgctgcgtttttttcaaacttccctgcagatgtataacccgctcatagtagttaattgcatccggatagggaacaagggcatctgctgttccggtatacataataagtttaccaccggcttttttaaagttgcccagatccggattgttggcgttaagcaccggagcgagcatggagtctaccaccgcctggtgtttatcaaaatcaaagctgcggtaatcaaaatcagcgcccagcgcccagcggtaaggatacaacaggctcgcagctccttttgcggtttgctgaagttccagtccgcctccggagctttcagttccgggagggggcgcagcatagatctgctcccttgtacgtggattcaccgggccctgatatattttttttaaggcggtcaactgcgcttcggtcaggcgtgggacttcctcctttcttccgcgtttaaaaagctcaccaggatcgaatctggcaagtctcggatcagtaaggaagctgtcggatggcgccccgccatccttaccggcatatgcggaaacaatcgtttttgtaatatacgccaggtccgccggtgaatacctgtttcccggagtttcattgatggcattatagtttaacaggaacccggtatgtaaatgcgtgcggttatttgccggcgctcctgcaatgatgccgttataatcgccgggataccgctgcgcctccatcaatgcctgctgcccaccagttgaacagcccacaaagtaggtatgatgcggcgccttaccataatatgcttctactatctgtttggaaacaaccgtcatcaaatgagtagaacgataaccgaaatccgcccatcgttccgggtgattaacagcggaatccacgccaggtgaggtacccatgtctgtattagccgttgcaaagcccttttttattccgttggccagcctgtcataaataatggtgccgccacctccgccattgcccgtccctaaaaacctgccgttccagctattgcggggcatccacagttgaattcttatattggatacaggtgttggtttaagtgttattgcaacgaggcaaaatgccggcaaccgggtaaatgttgttgttgaaccaaccggctggtaagggtcctcattgatgtattgaatatccgtgatagttaaccctggtatttttagtgcaagtattttctgccgcaggctgtctgttgcggtgacaggatgcatggcttctgcagttagcaaacccaataaggccataaggaatataccggtgtgtataatggctcgtagcatagctttcataaaattgtataacgtggtgggttgcactataaacactgaaggatgccggaacaattcacggcaccagcgttatttactgcacccaaaatacaaattcacggatattgccggataatttttttgttgatgttattgcgggagtctcttcgacgattcccttacaatcaacgttgttttcaacgatttcagcactggtgagtagtcttctcccttttttatagtgtccagcaatatagctgctgccgacctgccgatatctgctaccggctgctgaacggtggtgagcgccggttcaatcacttctgatataggatcgttactgaaaccaacaatgccaagctcggaggggatatctattttccgttttttggcaaccagcatcagttgaatggctaccggatcgttcacacaaaaaacagcatccggccgctgtttcaggttcagtaacttttcagcgcaatggatggcatctttttttgagagattgcaatggacaaccaattcttctttaaagggcaggtgatatttttccagtgcatcccggtatcctcttagccggttatgcgttatcagtaatgcaggcggaccgcctatatgtgcaatattgcgatagccgtttttaataagatgctccacggctttaagcgctccctcgtaatcattaacaagcaccttggaggtattcatctcatcgcagatccggttaaagaaaaccacgggaatgccatgccgctcaaatgccttaaaatggtcgaattttttggtttcccttgtcatggaaatcaacacgccatcaacccggtttgccagtagtacattggcattggctacctctgttttatatgattcctgcgactggcaaatgataacgttatagcccgcctccgcagcaacctgttgtgcgcccatgataatggtaggaaaaaaatacgtcaggaactcaggtacgataataccaatggtgttgcttttactttttacaagactttgagccagcaggttgggctgataatcaagctgcctggccatttctaataccgctgcttttgtttgcggattgatatccccatgttcatgcagtgccctggataccgtagacttggatatgttcagcgctttggcaatgtcaacgatcgtggtcatgtgctttttaagctgccgcatatccacagaattttccccgggaagtgtgaaatagatattacaatccttacaataatagcgctgtttccctcttacaataccagattttgtgatcgtgtgtacttgactgcaccggatacattttatcattaaaacagaagaattttaaattggtcgtactaaataaagtgcttttgcccgtttgtctgccacgctcccgttactccgtgactaccggtatcgtttgcggtatcgttcccggtagattctgttttcccggaagctggaaattctttcattgtttaatattcttctctaacattgctttaccacttatgactaatgttttataaaagttaaagacgcttacgttatgaaaaaaacaagctccttgtttaaatcacgggatcttttcaggatcctgctgcttgtacctttttccctttttgcgctgccaacaaatgcccaatccgttttgccaaccgtttcaggcaaggtagcggatgagaatgggcaggcattgccgggcgccactgttgcggtaaaaggtacatcaaaaggaacggccaccagcagcaccggcacgtttacattaaaagaggtaacctccaacgccaccattaccgtttcgttccaggggtatgtaaataccgctattgcagtccgcggccagtcatacctgacagtgatcttaaaacctgatattagtaaactaagcgatgtagtggtggttggctatggcactcaacgcaaagcggcatctacagggtccatcgcatccgttaaagcggcggatattacgcaaacacctgttacgaatgtggcccagggcctggctgcccgggtacctggcgtacaaattacacaaaataatgcggccccgggaggtaatatcagcgtacgtatacgcggtaccaattccatcaacggctcctctgagccactctatattgttgacggtatccagatctccaacagcggcggcgtaaatgatgtaagccctttatccaccatcaatccaaatgatattgaatcggtggaaatattaaaagatgcatcctccactgcgatttacggcgccaggggcgccaacggcgtagtgctcatcagcaccaaacgcgggaagagcggcgttacgcgggtgcagctggatgtttaccagggcgtacaaaacattaccaaagaactctcaatgctcaacgcaacacagtttgctcaacttgaaaatgacgtttataattccccgatatacaccgacccgtcttccctgggaaaaggaaccgactggcaggatgtcgtttaccgcaaggccggcatacaaaactaccaggcatccgtaagcggtggttcggagaaaacacagttctctttatccggcaacttcttcaatcaggaaggtattattatttcttcggatttcaagcgctattctttaagggcaacgctggatcataatatcagcaaacgctttaaagtgggtacaagcctggttagcagctacaccatcaacaataacattccaacgggtataaataatattgacggggcacttgtaacccaaagtattataggcgccacccttggcgcacctcctaccctggtgccataccgggaagacggcagcctttatccttttgcagaccagttcaatagccgttaccgggaaattgccaacccggttgggctgacgaatatccttaaccgcaataccattaaacgcacgctctccaatgtatatgcggaggctcagatcatcgacgggttaagctaccgggcctccttcaatgcagatattggcagcacgctgaacgattattattcaccccttagtattcttggtaaagcggaagttaatgccaattcaggtgttgcttccaaaggaaacatcaatactaccaactggttgcatgaaagcattcttacctataatcgcctctttggagatcattcgctcaagttcacgggtgtgtatgcgattcaaagtaatttatataacgacaatatcatcaatgcaaacggctttccgaatgatgccaccagcaatgaagccgttcagctggcggtaaacagaacagtactcagcagccgtaccaaagaagcactcaattcgtacatgggacgtatcaactatggctatgccaataaatacttcctcgacatcactgcccgttatgacggcgcctccaagttcggagaaaaccacaaatggggtttcttcccggccatagccggcgcctggcggatcattgaagaacctttcctgaaaaacagccatttgttcagcgatctgaaattaagggccagctacggccgtacaggaaacgccggagccattgcaccctaccagtcattgtcacttgaaaattccggaagtaattaccagttcaatcatatctatacagtaggtatcagcccaacaggtattcccaatgctgacctgcggtgggagaaatcaacccaggccaatgcgggtcttgacatcgggctattccaggacaggctgaccattgtggtggattattataataaggaaacaaaggacctgctgtttgtgaagaacttaccactttcttcggggtataacgccatcaccggcaactttgccagcatccggaacaaaggtgtggaaattgccgccgatgccaggctgtttaccgggaaattcaaatggaacgtcaatgcaaatgtttctgtaaaccgcaaccagcttttaagcctggagggtggtacaaatgaatacgtgctgagtccctacagtgtgctcaaggtagggcagccccttggcatcttcaaaacctatgtatttaacggcatttatcaaaccggcgaaaccgtgataccaggcagcgggagcagaacaggcggtgtaaaagtagcggatctggacaaagacgggcaaattaccggggcggatcaaaggatcaccggcgatgcaaacccttcctatattttcggattttcttccaacttcagctatggccacttcgacctgtcgttctttctttcaggcgtgcagggcaacaagatctttaacctcagccgctatacgtttgaaaacggtttggggggaagaaatgtgttgtcgggcatggtggaccggtggtcgcccacaaaccccggcaatgaatatgcgagcggcttccagggaggcagaataccggtatcggaccgttttgtagaagatggctcctatatacgcatgaaaaatatcacccttggttataaacttcctgctgtaaaatatatcaccaacgcaaggctgtatgttagctgcaacaatcttttcaccatcaccaactatagtggctatgatcccgaagtaaattcctttggcggttcaaacacacagatcggggttgacaatctcgtttatcccatggcaaagtctttcatcgttggcttacaggttggtctctaaaaaaatgatacttatgcaaacaaagaagaatatacaattcctgcttgccggtttattactgatgcttgtgcaaacatcctgcaataagctcacagaaagcccttactcttccatttttactgataacttctataagacggcatcagatgcagaagcagcgttgacagcagtttatgggccacttggcggtatatatggcaccgccggcaccggggcatcagacttcagcgcagaccagatctatccccggcccgtagtaggcagggatacctacacgcttttcagttatgatccaaactatactactcaaaaaagttttaacaggcagtttgaatctcctcagcaaatctggcaatcctgctatcagggtattgaaaaagcaaactgggttttgctgcgcgtacccgacaccaatatggatacggcaagaagatcagttattctgggagaagcatattatatgcgcgccttttatttatggatgcttaccaagaactttcgtgatatagtggttaaaacaacacccagcactaatattgatactgctatcattggcaaaaccatgcaggccgatgtctttaaacagatataccaggaccttgagcaggccgttgccaaactgccttcctattctgccagtatccagaaaggcaggccttcaaaagaagtagcgctggcactgtacgcaaaaacagcgttgtatgcacaggactggccaaccgcactggataaagcaaagcaggtgctgaattccggcaaatacaacctgatgccagacgtgttggatgtttataacgttaccaaggaggacgccgccaggcaggaaaacatgtgggcgcttgaatgtgaaagcacttcgccgggtatttctacacagattatcagcttgtttggccctaagaacagcgacgggccgcaatatgctgcctccacttttggctctgcatttgcctaccagtctttctttaactcatttaacccggcagaccgcaggcggttgttgctggacaccaattatatcaacaggcagggaaaggtagtggcacagaaagatattacacctatcacgccacaaggcgtactggttaaaaaatatatggaccctaactctattggtggaaatggggccgttaacatccctattctgcgcctcgcagatgtttacctgattgctgcagaagcatcggcacagcaaaacggtccgtccagtgaggcatatggctatattaataccgtcaggagcagggccggccttcctggtttaacaaccggactgggcaaggcgccgtttgttgattctgtattgcaggaacgcagctgggaactctttggagaaggcgaccgctggtatgacctgaccaggaccaatacttttttacaggtaattccaaaagctgtaaataatgtattccctgtccggacaccacaggcaaaaaaccgttactttcccatcccgctggatgagatcaatgcgaacccgaaactcgaacaaaatcctgattggaaatgagatggataataaccgctgtttgttttcttactttacagcctgcatgggcacagcataaaacgctattcctggctgccggccaaagtaatgccgttggccagggagacagcaccgcttcggtacactgcaccgccggaactgcttttgaatatcggttctcgggagataccctgcttgctttaaaagatcctgccgggcatcgtgaactacagtttgaaaaagctaacagcggcagcgcctggccggctttcgcaaaagcctaccacgacctcacaggaagccaggtggtgattgtgccggcggcaaggggcggaagctcctgccactataaagcggaattaaataattacggcacctgggataacaggggcagactgcctttgttcgacagcgccattgtaaaggccagggctgctgcccgcaaaacaggcttaccggttaccggaatattatggagccagggagaacgggatgccaatgccattaatgcacaacagctttctccggatgaatatgagcaacagctgacatggctgatcaatcaattcaaagcggcgcttggtaaccaggtcaacttctatatgatacaaaccggccattacctcaaccatccggctaagggttttgatatcgtacgtaaggcacaggaaaatgttgcccgaaaaatgaagcatgtattcattgtgtaccctcaaacagacagctttaaagaaaaaggatggatgaaagatgagatacactataatcaaaccgcattaaataacatcggagcagcagttgcaaaacaggttgcacttaaaggaaaaaagtaaacatgaaaggaatattattttgtttgttactggtcattccattcttactctttggacaacgccgtactgataacagcttaaacagtgaatggaagtttgccgcggaccccataaaagtgggggaaaaagaacgctggcaggatacatcatttgcaaccggcagctttgataaagtaaaagtgccgcattgtttttctacagatacccggtacttcttttacaccggcacggcatggtattttaagcaatttgaagccgctgcaccgggcgacaatcacgtgttcctgaaatttgacgccgttttctataaaacaaaaatatggctgaacggcacactggtgggtacccacgaaggcggctatacgccgtttgagtttgacatcacagccttgcttaagagcaggaatacgctggcagtacaagtggataattcctgggataccaccaccattcccggcgctaaaacccctgttccctattcagccgccaatcaccgccagttttatccatggatcaattacggcggcattaccaggccggtacatcttgttacacggcctgctacatatatcagcaacagtaaaatcattgccatccctgatctgaataagggagatgcaactatcaggataaaagcatttatcaggaacaacagtgcaaccgccattacctccgcagtgaatgccggtgtttatcgtaatggtgcaaaaagcagtatccgttttaagccgcagcaggtaaaggtggaaccggacagcgttgtttcggtggagatgaccgccaccctgcccgcatcggaagtggctttatggagccccgacgcccctgcattgtatagtgcagccattgtttccggtaaggataccgttgaaacaacatttggcatccggaaaatagaagtgagtggcacaaaactgctgttaaatggtgaacccataaaaatgggcgggtgtaacaggccgctggattatcccggctatggctccatggatcccaacgaagtactggaaaaggacctgacgatgatcaaaagcggtggtatggagctttcccgtattagtcactacccggtaccggaaaccatgctggaatgggcggacaaacacggccttctcattattgtagaagcgggcaactggcaaatgacacccaaacaaatgaacgatcccctgatgcgcaataagttccggtcacagatgagggaaatgatggagcgcgactggaatcatcccagcgtcatcgcttatagtgttggcaacgaattccagtcacaaacggaagaaggcaaagcctgggtacgtgatatgagcagttatgtaaaatcactggatgactcacgccttatcaccttcgccactatgctcctgggacgtgaggatatcaggaaacccgaagatgaagcatcgcaatacgttgactttgtgagcgcaaatatttatggtaatcatttaaaagtgctgcagcatatacatgcgctgtatccttcaaaacctgtttatgtgagtgaatttggcgtaagaacagatgccgttggatctgaagaagagcggattgcctatctcaaaaaagcgatgcaggatttccggcaatgtgattatttaataggtgcctccgtgtggaccttcaatgattatttcagccgcttccccggcaccaatgcaaacggataccggccatgggggctggtagcgccagacaggacgctgcggggcatgtacacggcgtggcaggaagaattttctccggcaaccattgagcttgttaataaaaccgcggggcgggcaggcatccgtattactgcaagaaaagatttcccctcatacacaatgaaaggttaccagttaaaatgtaacggaacctatatacctgtaaaaaccctgcatcccggcgagagcgtggtgcttaatgttgacttggccggggaaacagccgatgttgcgctgataaaaccaggcggttttaccatcatccaaaaaacccttaaataatgataagatcagaaagcgcggataaacgtacattcccacttgtaaaactaaaggccgatctgatcgtaacgggcggcggactgtccggtgtttgttgtgctgttaccgctgcaaggcatgggctgcaagtagtgcttgtacaggacaggagcgtgctgggtggtaatgcaagtagtgaaatccgtttatggatcctgggggccacctctcacatgggcaacaacaatcgctgggcaagggaaggcggcattgtagacgaaatactggtggaaaacctgtaccggaacccggaaggtaacccggtgatcctggatgcgatattactcgacaaagtaaccagtgaacccaatataacattgttgctgaatactgctgtttatcatgtagagaaacaggacagtacaactatctcctcattaaaagcttattgtagtcagaatcaaacggaatacaatttaatggcgccgctgttctgcgatgcctccggcgatggtgtagttggtttcctctccggtgcggcattcaggatgggcgcagagcctaaagaagaatttaatgaactgtttgcaccaacaaaaacctatggcgaactacttggccattcgctttatttttattcaaaagacaccggcaaacccgtaaactttattcctccctcctttgccctcaacgatattacacagatacccaggttccggagctttaactcgcaggagtacggctgtaaactatggtggatcgaatacggcggacgtatggataccgtacacgacacagagaaaataaaatgggagctctggaaaatagtatatggcgtatggaactacatcaagaactcaggcaattttccggaagcagacactttaaccctcgaatgggtaggcatgatccccggcaagagagagagccgcagatttgaaggcgattatattttaaaacagcaggatgttgtagaacaacgcctgcatgatgatgccgtagcttttggtggctggagcctcgacctccatccctcggacggtatttacacttccggacctggttgcaaccagtggcacagcaaaggcatttaccagatacctttccgcagtctttattccaggaatatccacaaccttttgctggcaggccgtattatcagcgcatcgcacgtggcatttggctcaagccgcgtaatggccaccagcgcatatgtttcgcaggcatcggccatggcggcagtgctttgtacctcgctgggatgcacgcctgcttccctctataataatggcagcattccgaaactgcagcaattactgctgcgcagcggacaatatattccgggtgtgctgtcaaaagatgaagaggatattgtacaacaggcagctattacagccagcagtgaactgttgctttcgggactggaagaagatagggcgccgctaccgcttgatgtttccgtagcgcaaatgattccggtaaacgcaggaaaactgccggcctttcagctgcatgcgtacagcgatgaaacaactaccctgcatgctgaaataagaacctgctcccgcacaggcagttatacgccggatacttccattgctgcttttgagttcgccattcagcccggcaggaattgtatacagctgatatccggtgctactgttgaacaaacgcagtatgtatttattatgcttcacaaaaacccgctggtaaagatcagcaggtcagataaaagaatcaccggtatcctgtctgtttttaatacggttaatcccgctgtctccaattatggcaaacaggaggcgcctgacggcatcggcatagacagctttgagttttggtgcgcccagcgcagaccggcaggacaaaatattgcgctccggtttgacacccctttgcagtcatttggccctgccaatataggcaatggctttgcaaggcctaccacacaacccaatgcgtgggtggccgatcctaatgacacagatcctacgctgaccctgacctggaaagcgcccaagcatattaaaaaattgatcctttcctttgatacagactttgatcacccgatggaatctgtgctgatgtcgcacccggaaaatgtgatgccgttttgcgtccgcaactatgccatctttgatgaaaatggtcgcaaggtgtatgaaaaaaaggataactaccagacaaggaacgagattgattttcccgacgccattgtcacttcaagccttaccatcaaaaccacgcatccttcggccagcacgccggcagcaatttttgaaatacgttgctttgaataaggtgttctgatgtgcggatgattacctgtgagaaaagttcttttctcacaggtattttttatatcattttcaattaaaaatcttctccaactctttatataactgctccccacgtaaactcttagcaataatttttccactggggtcaatcaggaaattttccggaattgactggatcatatatttgctcccggcttcattcttccagcccttcaaatcggaaacctgtaaccagggtaacttgtctgccttcaccgccttcaaccacgctgcgcggttctcatccaatgatacggataatatttcaaggccttttttattaaaagtgttataagctttgagcacattaggattttcagcacggcaggggccacaccaggacgcccagaaatccaatagtacatatttgccggcataatcggacagtttaacgatcttgccatcaacaccgggttgattgaactcaatggcctgcttaccgggccctatttgtaaccgctttctttgatcagctattgcactgataatattttttgccatgaaagatgattgaagttgtttatcgaactgcttcaattcattctccagtcccgtcagcccactttcttcgcggggtatgtagtcacttaaaaggtacagattaacaaaactggcaggatgtgtacttgtgtatgctctcatataatcagtatacttttccatcgctgttgctccttccttttcgagggcggcaagtttcgctgtatcattttttttcatggctatttcatattgctttcttatttcagttcttcctgaaatgttgttcgcattttcaaataacccggtatattcatcctgtactgcagatccttttatttgcggatcctttactgaattttcatcccaactgtatttgccggtaacggagatatttgaattttcaagaaacatcgccaggatgacaggggaattacgctctccgggcatacagaaaatataggccatggaaggttcatcaacatttcccgtgaaaacaaaacggccatcagttagtttggcggaatccgttgtgtaggcgccgttacgcactattcctgaaaggtaaatatatcctgctgtaaagttcttccctttagcatacccggccttactcaccaggccttcaatattaccggttaaggtatactgtgcattcttcacctgctgtccggatacggtcagagaaaataatattaaaccaaggaaaaaaaatagtctattgctgttcatacttctggtaaataatagtaaataaaaaattattgcttatctcagttagctgatctataactgagatttataatctcaccaaacccggtgaacttcttaacataggtgtgattgataatatctcccaggttatccaggtcgaaataatatacttcccccgcggttcctgtgttagttgccaccacaattctcttactggtaagggacaacattttcaggtcttttatttttacgccatcgggaaacgtgtataccattttcgaagaattcgccagtatatcatagagataaattttattatctgcggcataataaagatgctttacaacaccggaagcagcaaaagcagtagctttctctatatccggactattgccgatctgctggtttaatgccggggttgccccgttaagcgagtacaggtaacggataccggcatcatcctgcataataaagtagatttcatcagatgaaatgacagactgcgttccatagctccagccaatcatcttctttccaacatcagccatattgaaaccagcacccggagtcgcagatacaggacttaacattctgccgcccaacggaacagacataaatcgcctgtacttattatcatagaataaagtgacagaagtggcggagtttatcacaaccgggaaaagggtataatcacctgttaatctttcagaataaggcttcaacacatcctgtggataaaacacaggtccgatgccggcatacagtcctccgtcagcaacaatatactgatcgtaaggtattttattcatggcatacgcgcatgaagcagtaaattgcttcggctccggaaaaatatctgctgtagtaccattctgaataaaatcgtcggcattaaacctgtaaacaccctggtcggtaaaaaacatcaccagcgcaagatttgcataaatactggtaataccggcactgacccccacggcctttccagggtaagtggtcttgttcacatcttccgccggagaaaaaaacacggaatcgtttgcccggataaaagacaaccgcgccttcccgtcctggtttgcagccaccagccacccctcataaaatgctccgtttacagtaagcggatacaacataaaagaagatatacctgtcttcacacttgttacagtatatatcaggtcatatgaccctggtgacagtttaactgccactttcaggtccttcttatcagataatatcacggcatcttcccctaccatataggctttccactcataagtataactatctcctgaaggcatggactctgtcagttgtgtttgaatactgagtgtatccagttgtgttatcacaaatgaagaatcagctgttttgatcgaaaccgtatttagtttatcatagacaaaccgctgattatccttctgacaggaagcccaggccagcgccaatattgcgaggaatgctctgaatatataattacgcatgaatttaattttgagttgaactaaaaggtgacctcgttaccggattcatctatcattggcccattgacggcttcatattcagcaagggcattttgtaatttaaccggcaaattgtagtaaccatccacgccgattgcatcgtaagaaaaatcagaaaggccggtaacctgcaccataaacctgaacttacgctcactgaatgctccgaatgcactctccacgtcgtcccaataagaaggtttaatgatcttgttactcacgtcaatgataattttttcgaggctggttgttcctccgatctcacgccctgtagcgcctacctggaaatctttacccggtgcaacctgggcaacaagccggaaagtggtggtagtcatctccggtgaattcaacagtaccacaggatacagcaccgttaaagcgccggccggcaacgtaatttccggtagctcatagtctttaccctgcctggccgttgaccccgcgcccgctgttacggaaataacccggggatagtcagctgccgcacctaccacacgcattttaagaaaaacggtatccctgtttttgggaaccggggaatacgcaaaagaataattgaggctgtctacttcatactcatctacataaaatgtaatcccgtcgggacctttataggttgatacattctcctttttacaggctgccatcagaaacaatatgctgagaaataacaggtacttcataaaaacaggatttatcagttgtagttaggattaaattccagttcagacgcgggtataggaagcgcatacttactaagcggaatctcagcagtcataaacagcattttggttacctttttccgtttatagtaaaagaatagctgcccttccgcgtaaaactctttctgatattctttagtgatttctttctccagtgtttgcggggtaatggtacccgcctgaagctcaggcagcgccctgtttctccgcacttcattcagatatccggcgccttcttccggtgttacagccgcttctgccatgatatagtacatttcagataaacgaatggcgggtacatgctgatccaatctgtttgaatccagtgtattaaactgatatgtctgccagaatttagaaggaaaggggacgcctccgtcctgttcaatacggtaaagaaatctgaaatcagtggccccgcctgctgcagtttcataaagtgtattaaagttggcggcacttcttgtcagctttatgttggcgcttccgttaaagcggaaatattgttgttctgcccagttctttatattgcgcacacggatacaaaatatctcttcatcaatataaagacgatcccggtaacctgcagtggatgaagcggcataaggggttacaaacgggaatttaccggaggtcaccaccacggaagccgcctggaaagctccctgtttgtctcctgcgtaaatacggatccttgcctccagggcctttacagcaaaataattcatcctgatacgcctgttctgtgaacctgttaaaatgggatcagcatctttcatcagatctgctgcctcgctaagatctgcgagcgccagtgtcactacttctgatgtaatggaaggtatttttgcgtattggtcagcagtggttttataggggatggccttaatcgctgcgcctgcggtatactcaggaccaaacatccgcaatacttcaaagtgaaggaatgccctgagtgcaagcgcctctccccgtataagcgcatagctgctggcagagagaacatcctttcttttttcagtgttgacaatgatcttgtttacaccggcgatggcagcatatgccgtatcccagatattgttggtatatccaattacctctgcagatgcaaagttcaatgcccgtgtttgaacaaatggggcgccggctccggacactgcgtagttttgtgccagtgccgatacaaatcccattgacaggttatcgccatataacgcccggctggccagctgggaatatacgccggtaagcgcctgttggaaaccaatttcagaagcgaacagctgatcttccgaaataacggatttaggctttacgtccaggaattttttacagctgctgaacccccaagatgcgaccaggcatattattatagtcaagctctttttcatattcataattttaaaaaccggctctgagtgaaagggaataagtacgggcaaatggattgctggtaccacgttctatctgaatactacttgcacggaaaaagtcattggtaatggctgtcacctgtaaactccgcataccaattctttttataaacggactcctgtaaaagttatatccgaaggaagccgaactaagcgtcaggttgttatcgttttgaacaaaacgggaggtcaggcgggtaggttgggtggaaacaccgatacgggtatacggacttacatctcccggcccggaccagccgagatcatatgccctccggtccacgttaaacgagggatccacagattcaacacggtctatcagcgtttgattatagagctggccaccacattggtaattgaagatcaggttgacctcaaagcccttcagcataaagttggtgccgaaattaccattccatttaggctgactaatgcccaccggtactttatctgctgcatcccaggtgaaagttctttttccgtcttttgtaagatagacttccgaaccggttgccgggtctacacccagcgaacgaaccgcataaatggtattaatagattctccttcttcaaactgtacattcggagtgacctgatcactattagccacattgagtttgttattggaagccttcaatttattggataactctttcaggatatttttattggtgaatccatttacattcactgaccataaaagtcctttagcgctcttctccaggattttataccgtacagagaattcgagtcctgtattctgtatctggcctaagttctctgcataactgctaaatcctgtggagggagcaagggtaatctgcgtcagcgagtttttggtattctcacgatacaggtccagccggagatccagtttctctcttaataataccgcatccataccaacattcgccttatacacattctgccagctcaggaactcattgcccaacccgatgaggaccgctcccagttctccgaaatagctggtgttcacaccaaagttataccgggattgggcgctgtaagccggaatattgagtgaaccggtagaaccataactggccctcagtttaagcctgttcaccaggctgcttttattgaaaaatgcttcattatggatattccagcctataccggccgaccagaatgttccaaatttcttttccgttccatattgtgatgatccgtcccggcgggcggaaacatcagccaggaagcggttgtcataactatagcttccactgtacaccacacccactctcctgatggtactctcatcaccggttggtcgcccgtttgtttcgtattgtgccgcaaacaacaggttatccagcttatcaaaaggaaagccctctgtcaccacggagtaatagttgctgttactgttggaaacattaaacccaagcattgaaaacaactggtgaggtccccgtgagatattgaggttagcggtggtcagactctcatagctagaactattttcatttcttacggtataacttccctttctgctgaggtccgttatctctgcaaaacgggaatcctgggcggaataaaactggtctccggaggcattctgcttattaagactcaggcttgtttccaggtacaggaatggtaccggcgtataacgcatctggaagttattggaaataccaaagtactggttgctgtttacagaatgaagactcgcatcatacgcgggattcgtttgcgtgtaattagtgtaattgatcagcagatcctccagcatttgttttggtttccctttctcatcataaggcgcccaatagggattcattgctacatattcactgaagtcgccgtaaggagattcgtttgacttattctggaagatgcggacagagtttttgaactgcagtttattgactacataattaagatcaaactgcccggaataatttttccggtcttgtcctttcattacacctgattgcagatcggcggaaaattgtaatccatagcggattgattggtctcccccctgcagatatagtgagctgcggttactgacgccatcctgaaccgggatcctgagccaatcggtattcacgccgcttttcatggctttgtacctttcattgcgaagcacattcagcttgtgctgagcctgcgcacttgaggaagtataaacgccggcgcgctgttcaaaatcaagtttttccgcagcgtctaaaagatgatacacggacaggtcgggggtcgtaaaccggaaatcattgttgaatgttacctgtatcctgcctggttttggtgtaacagtagtaaccaccattacgccgtttgccccgcgggacccgtaaatggcagtagcagacgcatctttcagcaaggtgatactattgatcaggttcatgtccaggtccacgatacgctgaagcgttacttcaaatccatcaaggataaataaaggggcattaggattggcagaaagctgaccggtgagattgggaaatgagttctgcccgcgcatctggatttcaggaagctggttaatgttgccaccggccacattattgggcacaatcctgagagaaggatcaagtgcagatatagctgcgaatacattattggcgctcacctttttcagttctgcaccggaaattgttttcgatgcgccggtaaaattattgcccgaacgctggaaaagtcccgttaccactacgccctcaatgcctttgatcagcctggccaaacgcacatttaccataccggaagacagcatgcgaaaattgctttgggcattgccttcggtttgatctggttgcccgttgccggtagtaatacggacaggatccgacataatagtattattggccgacagtcggagccccattggcatataaccaatagatgatatgacaatgctggcattgtccgatatattattcagcaggaaacgtccttgtccatcggtggaagtagcaatcgttgttttccataccattactgttgctcccggcagcgggtttccgtcaatatcagttacctggccggaaagagaagcggcgggggctgttacctccttctttgcctctagcggtgccggacctttcatctgcaatgcgatggtattatcatccagctcataggtgaacggcgtttctttaagcagctcgtccaggaattgcttaagcggcatattcttcgcagcaatggtgatattgctggtttccgtcagccgctgaatttcacggctcttgaaaaaagcgtagaagcccgtctgttgttccagcgcattgagtgcttttatcagtggtacttttttagcagaaaaagtaaccgattgcgccagcccggatgcagacacctgtagaagagctcctgttaaaaggagaatggttagtttcattaccagcaatgtttggttgataatcttttttttccggaccgccgccatatggcacgcgccgaaaatgcttagctgataagcagttttttgcataatttgcaggtgtttggttgataaattgagcggcacgctctttaataactaagctttataccggaagtggctccaatcacttccggttttcttttggttggcctttctttcttacatatatacttttatctgaaatttattttctttctgttattatcagcttacggccttctgcgaggcgaaaactaagccctgtaccatccattaacctgactaacgttttcaggctgaccttccggcttattttgccgccaaacgggacctgcgaaatatgatgatcataggtcacctctatatcgtaccagcgctccagctgtgtagctaattcttctatagttacattattgaaatcaaaagcaccgtttttccaggcaatagctttattgatatctgcatgatcggcaacggtaatatcgccggctatactggcttcctgccctggtaccaggatagcttcagccttcccgctacggatatttaccttacctgttaccagcgttgctttcacccgtggctgatcgccgtaagcgttgatattaaaagaagtacctaacaccaacacctgggttttatcattcaccaataccctgaagggttgggatgaattttccgcgacttcaaaataagcctctcctgtcagctgcacctggcgttcttttcccgaaaagcgaacgggaaaacggagtgaagactctgcattaatccaaacctttgaaccatccggtaaaacaatggagaactgtcttccccgtggagtaagaacagtattcagctcctctgcaaccatctctccggacgtggcaggtgcataggccaggcccccgttgttcagcactatgtcaacacccgcctgcgaagccactgttccgttgcctgcggtatccagcactactttattaccgtttgccagtatcagcaccgcgccggggcgaccagggctaatgtcctgaaccgcgatctggttttcatggaccggctttgtttttaaccggttaacggtgtaccagccgatagccagcatagtaagtacggctgccgcaacagacaaccatttccgccgttccggcaggagccttttcacaggcgtttctgcctcgatttgccggagtatttctttcaacaccacctgttgccgcgtttcatcccactgctgggccgttgattcgagtgagccctggatggacgctttcacggtttcatcgtaaacgcccgtacctatggcttctgtaaattcagacaactcgccggcggaaatttcgttcttacggtatttctcaagtaaggattggaaataaatctcatccataaacggtttttaaagcgatacaatataaagacgaccaccaggctaaaagtgggtagttgaattgaaaaaaaatgggtgttgactattattgcatcaacaacaccaacaaaatcattaaaatttcagggtcttctatatgggccattacatagtggcgaactgcccgggtagccaatttcagatgggttcgcacagtctggatgctgatctccattctttctgcgatttcggcatgggaaatgcctgattcttttgccagttgaaatataatacgttgctgcggggtaagggattccaccgcttgcttcaaaattcctgcgtattctttggcagccaggatcttgataggtgaatcgggaccatcgtgaagcaattcgcccagctgtagctggtgatgtagctggcgtgcacgcgctttaaatgtgtcgaaaataatattccgggcaagtatgtacaggtaatgttccggcttttttaatgttcccggctttgtgcgggtttcccacatacgcataaaaacaagctgcacgatatcttcacatagtgactgatctcctttggtaaaaaccatagcggtgttgtatactgcagcactatatttatcataaaaaatagaaaactgccttacatcttcatccggtatctttttatcactggctgtattgatattagaatgctgattgcccaacctttcgcgtttggtcaaatttagaaaaaaaccgcgaatagtgctaatggctggcggattgcttttgcatcaccatcattgcatcaaacttctctgcaatcacttttggatcaataccctccgcaaactcactgaccaggtaatgccgttcatcgtttggcgctaaacgccacaaatttgttccgtcttcaaaaatgtggttatatccgcgttcttccagcctgaaataaggctggtgccctttcaccgccacataaaccgcaatcaggtcggcgctgtggtgccaattccttttccagctttccaggaacagtttgtaggcatgcgccatcggcgtgtgtttatattgttccctgaaaaaaatcctcccggttggcacactgtcagcgaaagccccgccgccggtgaaatatatgcgggtaggccatgctgcaaccacatgttgggtggcgtgcggatcggatttgaaatttccccagggccttgggtcctgatctgccggatacctgcctcccatgcataccaggcgcttcactttcttctttaccaggtcaatacccttcaattcactaaactgatctgcttccgtttgcagcagtttggaaagattggtcaggtcgcccaccgtcaccaccaccacgcttgtatccggttgtgacgacagtatcttccggtacagcaacgtagcttccggcatatcttctcctaatttaacattggggttaaattcttcgcaaagcctgcgtgcatatttggacttatgatacacgccaaatcgctgcacagcgccaatagggatatctggcctgccgtagtaggtattaatcacatcggctgctcccggcgaccatggattaaggctggataccataaccgccagtatctcggcatccccgagattggcgaaaccatggagcatagccagggcgcccacgtcatcgacgtcggagtccatatcagtatcaaaaataattcttacgggctgcgcgaaggcgagatgacagagcagcagactaaggatcaacaatccgagaggctttatttgtttcatctattcaacgtggtcaattgggtgatcgttttcagtttacgtggtacttccgtaaaacagacgttcaaccggatagttaggacccattgacagcgaaaaaactagcttaaattttcaacctggtcatgaagctgctgatcccagataaattctatattgaacttaccatcaggctccaatctgaaaatggccctgttccatttgttcgcccctccctcagtagtaatactgtgtaattcttttatccaattcctgatctcccggggaatttttctgacagacaggtcaacggcggtactaccagcctggtagtcgcccgtgtaacctaccactccattggcaacaacttctatatccaatttagcatttgtccagttactttcgtcgatagcattagcgatgccttttgctatgcttaaataaatttcatctgctgtcataatttaattttaagctgttcttaaatagtcctggtaatttaactatttaattaattacttgctttaatggaaaaattatgcttgataacttataacaaatctctgctataatactacctgaacttctaaattttagtccgctatatcggtaagcattttattaacaatcatccaccggttattgattttatgaaacgagagaaattcgtcataattaaactcatacattttaacgtgaatttttgccatcgctatagtattaacaacatcaatcgagatgatggttcctttaaaaggtttgccggaatctttcacactttgtcggttctttacaccatccaggtactgatcaagggttttggcgtatggctggccctttacatctccgaacaatagggtaccgggatggtagatatttttcaggatgctgatgtcgccttcgtaaattcctttgaaataatattcttccagcgcctgggcaattgccagggaatcctgttgactggtttccattttcattgaattttgtgcttttaataccagtatgacgccggacaaaaaagcggttaaaaaaagtgttttcatgttatttcagatgatgtcctgccgccattccgccgtctacgtcgatgatggcgcctgtaataaagttactcttagcaacggtataaaccatttcagcaatatcttccacttctccaatgcggttcagtaaatgcagtcctgcgctctgaccggcattatcaccgcgcataggtgtgcgtattacacccggggcaatggtgttgaccctgatgttatccttgccgaattcggcagccagctgcagggtgagtgcgtgtatcgccccttttgatgccaatggcgcagtagatggagcgcctcccaacgcgtggtttaccaatggcgtaccgatgttgatgatcacgccgtggtgctgccggagcatttgtggaataaccgcctgggtagtgaaaaaagtacccttcagattggtatcaagaaatttgtcgagataagcttcatccacttcaagaaatggctttgtttcataaatacctgcattgtttaccaatacgtctgccgaaccaaattcctccatagctgttgccagtatcttctcaccggtacttttatgtttcacattaccggctaccatagccaggttttcgcccgcgcctaactcctggtaaacctcttccagtttcccggcagttaaagaattaattactacattatctccgttttttaaaaagtgccgggctacctctttgccaatgcccgatgaggcgccggtaactattactgtttgctttttcatggccttattttttttcagcggttatccctttctctcttaatacagatacctgttccccggcaacaccccagtcgtccaggtcatattcccggatgaccacaaaggtcagttgcggatctttattcagggtgtcactgatcaggtcagtgacacctttaatcaggatttgcttttgctctcttgtaacgccttcacgggttacttctattttaacgtatggcatgacttaggtttttatgctaaagccgttttcaggcggctttagcggttacagttacgtttagttcaaaatcgttatagattaaggtatctcccaggtttttaaagaaattacctgagcggaactttatgccgtacctggtacggtcaatcaccagcttgccggtagcagttacctggtcgccgttaatattaaccgccacatcaaaaccgaccggatgcgtaatacctttaatggtcagatcaccttcaacatgattgcccaccacggaggtgatttccaatgttgcctccggatatttatcggtagagaaaaaatcatccgaagccaggtgaccaaagaactgcgcatttgttgcagggtctgttacatccagtattttaatggaggtggtgtcgatgacgaacttaccaccggcaagttttccgtcattcaaaagaagttcgccttctttaacggcgatggtgccgttgtgggcgccggttacttttctgccaacccaatcgatgttgctttgggtgcttacgatatcaaatttttttgtttccatgtttttatgtttttatgttaccccaaagtacggtagcattttcaacacggctgcgtgatctacatcacatttgaagggaggcattacttatgtgatccaggtcacttttcatttaatcgaaccttaattgggaaataaaaaaagcaggtatttaaatacctgctccagaaaaagatatagaccagcttatagattacagcctgctgagggtttcccttgatacgcccagatatgcggcaatgaggttcttaggaaccatgttataaagttccggatatagttttaacagctcctcgtaacggtatttcacattattgttcataaaggacaacaaccgcttttgagcagcaacatatcccctgttggtcctccatctgaaaaaatgctctacagtatgcagttcgttacatagcttttccctgtcgctgctagtaagcgcaagaacatccgcatcggttatacaatctacattgatggtggctttggtttgattatataacgcattgtagtcagaagcccaccatgtgggcatggcaaactgcaggatgaacattttcagatcatcattgataaaaaaagattttaagcatcctgaaatcacgaagtattcacaatctaccgtatcgccctcgacaataatagcctgcccttttttaaagctcagtggcttaaaatgtgaaaagaaataatcaaactgctcatcggttaaactgacaaacttcccaatatgagctttcaacgtttctttagcttccataagtgatttttactaatgctttgaccttttcaaaggtaagcattcttccaaaaaatataaatatggaagaacatgaccacagcgctatttctctaaaatcaattgattactttggttatcaatagaccagcgccggaatttgttaagaaaagttttgccgagcaaaaaggtatctgcttctttagaggcaccaataacgaggttattaacggtgaatttacccacctgaacattgttgatcctgtacacatcacacaaaatctccttcccgctggcaagggtatatgtttgctgccccaggaaatcattgccggaaaccagttttaattgaagcaatttattgatcatggtatctgacaccagcatgtcagtggcgccgcaatccagcatccacacatttacgagcggtcctatttttactttcagcttcgtcatggcgcttacggtaattacatcaatagaatcgattttcctgttactggttacatccaagctatcggtcgccctccaggaagtggtaggggatacttttttatagggatacccaccgcaacgataggcaatttcattaaataacatggaattgggatcgttcatatctttaatggtttgcgtatttattttccgctttgtcataatagataccgcacaatcacaatatggatttatcttgctttcatccagtttctccttttgattcccgcgaatataggcggccatagaatcacgataagctaaaatctgagcgggtgagaaaaagagattggtctgggaaatatctttgtaacattgatcaatgcgagcctgaagcagggtatctttttctataagtttagccagtgaaaaattaggatacaagcgctcatactcctttatctttttcataggaaaatacccgtcgatcgcgtctacctggcaattacagatctgaacggcctctttatttgaggcatccgctttcatcccatttatgcaacgccagaacagcgtacttttcgaccaaacaattttccactcccgggagcggacatattgctcgccatccgtaaactgggcagatacactaccggcgataaaaagtaatattaaagtaagaaaacgcataaacagatgctatcagtgtggaagcaagttaattaaaagtgtttaaagcaaagagattcgcacagcccgatgccgggaacaagataaaaagcccctgcaaattttcattgcaggggctacaccgctttggcaggcacttctattgctgctcctttcttacattaaagaagagatagtctgttcccggggcatccgttatcccgatacttctgccgatagtaactatctgtcccctgtgataggtgccatgattaacaaaatgttgtatatactcatagcgggattggttggcttcaaaccagggacttaccacttttattttttctactaaatcattccgggagaatgattttatctcatttgccagcacttgcgacctgttaataagtccctgaaaaacttcgtccgcgttgaggtcttctatgccataacgatttataaagtctgtttgctggcaaataatggaataccaatattcttccattccccaaatgtgattcaaggttttgaggatgctggaaaaacttgacggcgactcctggttcaactgttccgttgttttattggacaaccaatccacaaactggtggtttaccgacaaattatagccggcataatttgtaactaaattttgcaaatccatttttattcatttaatgtttaagcaaaattatgtgggggtattgacagccctatgtcaagggtaggaaggggttagtaatatttgtcaaaatattcctgcaaggtcattttatgaggggtaaacttttcagacagggtttccagtcgtttaatcctgtccaggcgaaaataccggaactctttgcgtaagcggcaccacgctactaataaccagttctcctttgtgtttaataatgcaaaaggctcaatcaacctgttggtcactttgttggcttcattggcatattcaattcttgttacataaaaattggtaagggcaaactgcagatcagataagttattactgttcctttccctgttaaggttctggtcaaactgtgtccgttctgccaggagattggctttatcttttacatgatgtcttagtaccgcttttattttttcgatggctgctgaataatctttaatgaaagaagcatccttgtttttcagcactaactgttctgcaagaatcaaggcgttggcctggttctccgtaaacataacgggcggaatccggtacccttccatcagggaataacctcttccttcttctgtcaggattggaacgcctgcctgttccagtgctttaatatcccggtaaatggttctgttgctcaccgaaaatttaccggctaattctgctgccgtcaaaagccgctttgtttgcaactgggttaagatggcagtgagtcgcgacagccgctttatatcattatcaatcattatcgaaatttcccggcattgaattttgtttatgatttcctgttcagatctgttatcagcagagggttatcttttttcagttcactgatcagcgtagccacttcagtagtagtaggattccgcatcagtctttccagttcagcatttgttatgcccaccagttgcaggaaagacacttcgccgtgtggcgtttctattcttcccagttcggggtcgagcgccagcacaaaagcggttatctccgtttgggtatcgagccgtatagggcctttggctggtataaaatgattttcttcaaaccatttcccactgttaaatacataccgcgcaaggttgttcattacatgaacggcccacagcgggtcatccttatcttccgcaaatggtttcaaccggaaggtaaattcaaagccccatttgctgaactcaccaccagccttgtcctggtcgtagtacagctccgacatgccataactgataatatgcctgtggtattcatgtttgctcgaatcgtaaatgcttgcgccatcgatggggtcagtgcctccggccataaagtgtatgccacagagcggtccgtaatgacggggttcggttttaccgtacaccgtttccagggcactgtctattgaaagccatccaacgggatcatcttccctgaacctttgtttgtactcttctgctctcataagaatagtaggttaatggctctaatataagccaagttgtgaaaaaagccatgcccgtatgttgattttattgtcgcaattgccctgcaaattggcatttttgcacccatcaggatcgcgtgttttgatgtaggtttaccctatcaaaatacatatcatatgcaacgcacatccattatttttatactcttattaatcgtaacacatttgcagatgactgcacagcaaaaacaaacgggccactatgcagcggtgaatggcttaaagatgtattatgagatccatggcagcggggcgccgctggtactgcttcatggcggaggttctaccattaagtccaactatggtgccatccttccggagctggcaaaaacacaccaggtaattgccatagaactgcaggcgcatggtcatacggccgacatcgaccggccgctgagctttgagcaggatgcggatgatgtggccgctcttctggggcaactgcacattgccaaggccagctttatgggtttcagtaatggaggcaccactgcgctgcaaattgccatacggcatccggagctggtaaataaactggtactggcctctgcccttttcaggcgcgatggtacacctcccggtttctttgatggctttaaaaacactactctggacaatatgcctccgcagctaaaagaagcgtacctggaagctaaccctgatcccaaaggacttgaagcgatgtttcaccgggatgtggcaaggatggaaaattttaaagatatcagcactgaagatataaaaagtatccaggcgccagcgctggtgataaatggttacgcagagcctatactgccggaacatgcgctattattagcacgcgtgttaccgcatgcgcaactggcgattctgccgggcggtcatggcgactatatcggagaaatttgtgcaccagataagcaaagtaaaataccgctgctggttaccaccatgattacagcatttcttaaagaataacagggccgagaaagagttactccgccatacgtgcctgcgctgacggtgtgaggtaaggataaaacatggcggagaaaattttactgtaatgttttatcgcctggcttcccctcagcttcccggttaattcattattcgacaaccaaaaatctcccataataaatatctgcgttaccaacgactcccagatactttccggaaaatcggtccggaaaatccccgctgctttcaactggccgaaaataataaagaattctttttcccggcgtcgtgtgagcgcataatagtctttcctgatggcaggcacgcgcaggcttatctccacaaaatgtaaaaatataaaacggtatttatatgccagctccagcgaacggacagaaaaatcctggagcgtatccagtgtaacgggattaattaattccagttccgaaaccagggcatcaaaaccggcggccaactgctcataaagcgtctttatgatttcatctgtttgcctgaaatgataatgcagattccccgggctgatgcccatttttgccgcaatatgcctgctggtaattgtgtttacaccctggctgttgtaaagttccagcgccgttttgagaatatttgtccgcgtatccataatcaaatttagaacaattgatctaaaaataataatatttagtacatttgttctaaataccgataatatgaataatgaaccggatgatctgcaggaggaagaccagcctttactgcaaagattaaggaacagcattcttcctgttaaatcaacagatgccacacccgtaaaattgttgaaagacagtgcgttttacctgtttgccgtaatggcgttacttgttacactgctgctcggaggcgctattatgtttgtattgtaaaatgaaacgcttatttgatccattattcctaagttactgcggactatggagtatcatccacatcttccggcatatggggcacccggttccgctgctcaacggacacctcaccgatttcatggcggtacctgctatagcgcatcttgcgcttgcttttacgcgtagctacattgtccgcgacgaaagttacagctatccaatttcttacctgctgtttatcgcactatatatgtcggtagtttttgaatgggtaatgccacagttttctgctgcctacaccggagatatgtgggatgtagtaatgtactttggaggaggattattttattattatgtacatgaaaaacggattacattaaaggggaagatgccttcctgatactcatctcaagccaatacaccccgccaccatcaatgccaccgtacctacagccgccaccgtccgcaccatattcaaccggttccatcgttcctcgaacgctgcccgctgctccgccagctgccccgcagaagtagcggtaagatccgctttgtccaatgcattattgagcggaacattgccggccatcgtcacaccaaaaacgccaataaaataaacgaatgtagcacctaatacacaccagcttccaggcgacactgaataactgaaatatgcccaggtgcaaacaggcaataaagcaagggagcctaaaaaagaagcaaaaaataccggattgaggatagcccggttgatagattgcatggccgacaaataaccgatatcagataaccggccaagccccgggttaacagaacaggaataggcgtagaaaaggcctcccatcaatgcagtggaaacagccgtaattcccaataaaatctgcaggaaagttagtcccatgaacgaaaaatttaaatgacgtggacaatatatcttacatgaaaatataacatccccctcatataaactataactgatttaccagctgagctccgtcaaactcactgtaccactcatgtttaggttctttattaaattggggctacaatacaatgatctgagagaccgtaatccacggattttcagggtcgacaaaaacatattgtcatcgaggtccaccttctccagttttttcaaagatgtaagatcaatggaagaaatattattattgttcagattcagttttttcacccccgatccttccgccacgaattctaccaggctattatactgcagttctacattttccaggttcggcaggtgactgaaattcactttaaataaagcgttccggtacatcttcaggtcgttcagcttattaagcccggtgagatccagcgcacggatcttgttatcattgaggtacatggtttccaggttggtgaggcccttcacgcgtgcatactccatgttgttattagcgccgtaaatgcttctcaggctggccatcccttccaggtccagtgttttgatctggttatcataaaaaccaaattccttgaggttggtaaaatttttaataccggtaagattggcaataccagcgccatttacatacagccgggtcaccttctgggcttcggctgcctgtatctccccgtcgttgttggtatcaaagccctggttgatcagcgccgctttgaaattggcatccggaattttgacggtttgtgcctgtacttgcaatgccatcaaaagaacagcaaataagaatatctttttcatggctctgtttagttactgataacggtattcactacttctccctctttatttacttctacaaatccggctacttcatcttctgcttgataataataagaataggcattataaataggttcagacctgacttcattgccgctgtatacgttgtaaaaggtacgggtaccggtgcggaggataagattcttcttccgctcatactcaatccaggtaacgagataatacttccccggtttgagttctgtaaattcaaagttaccctggtcatccaggtagcggccttctatgcggtaagtgaaggcgtcgttagtcatggaggcttgtttctttcctttgttgtacttcttcttcagctcaagaaactcagtaaaataaggggttaccggaaacaggatgatattatggccttttgtggcaaaattaactttgcctttctttttcagagaagcattaccccggatggtagcagtgccgggctccagtaacttgttggtagccgcctcatcgaaggaagcagcagggagaatatattccactcctttttgcgcagatgccgtgatggaagccgatgcaaagtataacatacaaccgatcagcagtgatttccggttcataacaagttctgtttttaatattccagccacatgataaccatgggggaaattataccccaaaagacggaataccacggcaattcagcaatacctgcaaacagtcatttaaatctacctggatacaggtataaaaaaaccgcatggatccatgcggttatatagctttcccgagatgactaagccagtgtttctgtatattttttgaaattatccaggatagcctgccagccgccctgttgcatttcaacgctatgggtgtcttctgcgtcaaaggtttctgtaacagcggtggtgtcgccggcagtggagaaggtcacccgtactgttctgccatcacccatggtgtaggtaatgagttcgtgttccgtcacttcgtcgtacacgccaccgaaatcaaaaccaaaactgccgtctttagcttccatgcgggtttcgaacttaccacccgggcgcaggtcatttacagactttggagagtgccagtcctctgaagcagtattccacttaacaatatgttcgggtgcattccacaactcccatacttttgcaacaggtgcattaatggttgcgcttaccgtgatcttcgttgtgttattagctgtttgcatgtttttaagatttaaatgttaaccgttattgttaatgcaaacatagcatgagtattttattcccggcatggctgaatacgacaaaatagtgtcgtatttgcgacagccgccgcaataccggtttacttccagtttaccaccgtaaatacaatggaagaatagtggtccttttcatacagcacacctattttcttccggcccagctgcacaatgtcagagtatgccgcgtagccatatccggctttttttgagccatcccctttatagatgacatagcttttcttccaggtgcgcccgtcgtcgaaactgatgcggagtgtgaggttatccctttccagtgaatcggcggcattgcaaaaggcgagtatctttttgcctttagaagtacctatgtccaggatgctgccctggcatacggcgtctaccagctgctggtcaaaataagtggtatcccaggtagcgccgccatcactgctgacagacacgatccgctccttcacatcctttgcctggttacggctgttcatcatcagcttatcgccggagagttgagcagccattgattcattgctaccgggcaaattaatactgttgcctaaatgaaatgttttaccatgatcatcggtgtagtacccatgtgccacataatgccgcgcgccgggcaatgctttaccagcagtgtgattggcagcaataaaaattcttcctttaaatttcccctcagaaaactgcataacatggccaggcgtattggcgtaatagcgccagtcttccgcaaaattaaacgccgggtcaatatcaggttgcttaggacgatgcacctgcaacgtaatatccaccggcgccgcccacgtgcgaccgccatccgcagaggtgatataatagcaatgctttattcctttgcctttaataatatctccctccttatgtgtacccgtgttgtaaaaaagaaagaccctgccctgcggataggccggatcggtaagatcaaccaccggcgcgggattggagagttgcaggttatcggcgcctgccaccacctgcatgggcgaccaggttttgcctttatccttactgcgtttcatcaccatatcaatatccccgaaatcgtccatcccgtttacacggccttctgcaaaagccagcaaatcgccaccgggcaatgcaataattgcagggatgcggaatgttttataaccatctgttccggaaataaaaacgggtatttctttttgttgcgcatacgcagtgccgaggcatatcagcagcagcacagtcattatctttttaatcattattatttatttatcaggtcaatatcattggttttcggacgcaaaaaacatagttgaataataatcgctaccagtacaattcccgccagcatggcaaagctttgcccgagattgcccgcatccgtggagcgtcccagcagatcggtgataaaagcgccggcaaatacgccggacatattcagtatcccataggcagtagcccggtaccccgatggtacaaactggcagaggataggcatgttattgccatcaaacataccaaagcctacaccaaacagcacagccgctcccattatgtgcgccaggctgtgtcccagccctatcagcagcaatgcagggatggtcagcgataagccgatggcgctggtgtaaattcttcccttgttattttgctgtacccacttgtcagataatatgcctccgaaaattaccccgaggaaagaagaagccgcgatagtaatggtagataaagggcctgcggccgacatatctatctgtaaactttcagaaaataaagtcggcagccagtttttgatcccccagccaggtagactcggaatagcaaaataaaacaagagtatccagaaagaaatatttgtcatcagtaatccaaaccctttcagaaaaggcggccgctcctttaccgtatccggcgggcctttcacggcttccctcaaacatacgatcaacaccagcgagtacacaataccaatgataccaaacgtatgaaaggtagcatgccacgagaacctggcggcaatagtagcgccaaaaccgccaagcgcctgtcccatgtaaagcccggtcatatgaatccccacagccagcgaccgggtggcagaggaatggaaatctgctatgagcgacagtccggccggtatatacaacgcctcgctaacgcccatcaccgcgcgtaaccaatacagctgctgaaaagtagtagcatagcccatggcaaatgttacccccgaccacacaaacaggctgcccacaatcagccatttccggttaagcctgtccgcaataatacccgacaacggactcataaatccatagatccataggaagatggccatcaggtagccaaaattcgtggccgattgcaaagctgcaatatccacctgcatggcgggtttcatggtcgacaacatctgcctgtccatgtaattcagcaatgctactacccatagcaatcctactactacccagcgataacttcctttattggacatgatactcagatcagttgaaaaataatttacccgaaattatcaccggcgtgcgcactcccgcttttatttccccggaaggaatcatgatcaccccgttccacagcaacgcggtggtggtaacaggtccttccatcgttaaagcgtttgttgctttccattggccggtggtggtgttatatagtaatacttcttttgtgaatcccggatgtgtattcagcaacgccttcttttcatttgtcagcgcttctttcctgatggcatcagtagccgcactgatggcggcattcagcgcttccatcttactgaatacggctcctttgtcgccgctgcaatacaggatttcatgatcccccacggcgagccccgtgcctgcggatacagggtaaggcagcggatttttccgggtccatgcttttgtatgcagatcatagcggtaagtggtattaaaaatatcgctgatgctgttactgtttttccgtctgcctccgaccaggtacacgccgccatcctgtaccgccattacagcatgggaaacggccaccggtatatctgccagcgtttgccaggcagcgcccggcgtggatacatccagcgaaaagaatttagcggagggaccgttcaccgattcgccaccggctatatacagcgtatgctgataacaggcgcccgataaattggtgagcgccaccggtaatgatggcagcgatgtgaaagtaatttcaccggcagtgttacatgttagcaacgttactttatccgtgggaccgtgatcattttcaccacctgcgtaaataaggccttccggcatgctcacattggcgctatacgccagcggttgcggcaatgattgccggcttaccacacccggcagcacatttccttttccatcttgccggaaaatataaatgtcctgtttataattctttataccgccgttccacggcatggccgccgggaaattggcgccaccggccacgatcattatatcattactaatgcctgctaccggcccggctacgccgggttgcaccggttgcccggcagcaggcggaagcactgccgccacagaccattgcacatttcttacctgggcgttgatattgttcaccgttgtcatcataaatatcgaataaagcaggtatttcatgaatgctgtactttctgaaaaaatgaaatggcttccagctctttatacaatttatcgtattgcgcgggagtaaacgtggttaaaggcagccggcatggccccaggtcccagcccagcattttcataatcgccttctgcgccggtataggcgggtattttgcaaagatcctgatcgcctctaccatgaataaatgctgttgctgcgcggcttttatatcgcccttttcaaaatacgcttttgtttgcagatacagcggtgcggcaaaagtatatgtgctgccgatagcacctttggcgcctacagccaatgcaggcagcaacaactcatcgaatccgaacagcacatcgaagcgaccgttctgataattaaaacaggattgatattcctggatggtggaagaggtgtatttgataccagcaagattggggatcctgttgccggctatttccaggaactccatcatatccatgcctacaccggtgagcgtaggaatatgataataataaaaaggcagtgcaggcgcggcagcggcaatatccgccatggcatcggcgagcacttgtaccgaagtaggtttaaaataaaatgcggccaccgaggaaaaggcgtctgctcctatggaggccgcatgggcggccagcttccgcgattcggcgatgctgctgtgaccaacgtgcacaatgatcagcaaccgcttagcggctgcttttacaaatgcttctgctacctgcattctttcttcggtggtcatgttaggaccttcgccattactgccgcaaacaaatattccttttaagccgtcttttaccagcttatcggttaaagcgggtaccagctccaggttcagggagctatccccgtgaaagggagtaaatgcggctgcgatcagtccttcaatatgttcatgcttcatgaaatgatacttttatattgggttattcgggtttcgaagtagcgtaaccaggcgtttggttaacgagcaaatcggtggtccatacgttggcatcgatcggccataatattttatatgcctgtgtggctttattcagcacgccaaaaggatggcctgcattgataaataccagcggttcattgccgtatttcatcctgcgcaaatcgtaccagcgtttgccttcatgtacaaactctttactgcgttctgcgaagatggcaagttcattggcatctttagacgaatttacgaaaggagccggatcaataccagggccgccgaaggcacggtcgcgcacggctttgatataaggcgacggatcgcccccttctgcattcactatttctgccagcatcagcagccggtcggcctcgcggtaaacgggccaatcgtcggagaaatatctcttttgtgttacggcatcaaaagtgccgaggaatttacgtaatacggtgttccgcactttcaccacgggggttccgctggttttatctactttataaaaatcgtaaaaggtagccgctttgcgttgatccaggttatcataagcctggaataatttaaagctgtaacggtaacgttgaatgatctgttttgaatttacctgtccgatgttcagcggatccgtgagctttggacccgaggcgagtgaatcggcgtaccagtcctgcgccataccgggcaggtcgtaagtaaacaatgatacgctggacatttcagcttcgtttaccatgaaagaaatcgcaaaaatgatttcgttattttttttgttggcataagcaaatacgtcgctgaactttggcaacaaactggtacctgttacagcattgagcgcagattttgcggtggccagatccgccgtgttaccatacaccctggctgaccataaatatatttcgcctttcagcattaatgccgccgccggcgaccattgtcctttggattttgccgctgccataccaaaattagtgaccgccttatccacatccgacttcaccgacgccagcactgctgcttccgtagcccgtggcatgcgcagtaatacgggatctgttacaccgttagccacatcaggggttagccgcagcggcacaccaccataagtacgtaacaggtgaaaatagtaataggccctcatggcatatgcctggccaagcaggtatttctttttatcatctcccaaaaaactggctgcttccactttttgtataaagagatttatttgtaagatgggtccgtagaatccggcccagttgttcacaccggaaacgttttcttccaaccgttgctcaataaggggactttcctgcaacgataatgaaaaagcttcttccgtggtaaagccaccaccgcgcatttcccccaaccggaagaattggaactggtcgttgcgaaactcattatgcaagcctgtcataaagctgttgatctgtgcttcgttcttccagaagttaacatctccgaaagaatcttccggcgacaactgcaatgtttttttacaggagctggcagccgttactatcagtgccagcaggaaaatatatgttgttttcatgagtgctgatttgattgcgttagaaggtgaggttagcggagaataccagtgaggtgggaatcgtatatacaccatcctgctgcccggtgcgttccggcagcgccagcattttattgctgatgtatccaaggttttgcccggtgaccatcaccgttaagcccgcaatatttgcgttattaagcatcttcttcggcactatgtagctcagcgttacttcgcggaaagcgagatagctggagtttttccagaacatatcactgtggcggtcatagttctttttcagctgctgatcctggtttacgtagatcgggtatttggcgttgggattttccggtgtccaggtatcttttaccaggtcggtgccgttgaattctccctgcatgctgccgagcgcccacatttgttttacatccatctgcataaaaccgatggcgtaatcaagacgggcaaacagctgtaatcctttccagccggcagctacattgaacccgccggtccaacgcggaatggtgtgacctaatgatacacggtccctgaaatcgatcgtatcgttcctgtcgaggtctttccatttcatatcacctaaactggtagcccagaatccggtaagcccgtttttatctatcagctgctgactggccaccgggcggccggcggcattgttcagctgcacctggccggcagcgagatctattttattataggccgctaaatcagcggttgttctgatgatgccatctgttacatagccgaatacttcgcccggctcctgcccttcctgcaaaccgccggcccatataagcctgccggtagatggatcatagatctgcaccccgttctggcggttattttcatttccgttgtacggcaatttcaacactacatttttattccacgccacattagcgcccacgctaacattccagttgcccgactgcaatactttataattcaggtctgcttcaaatcccctgttccgcatggatccgttgttggtgagaatgctgcctacaccggcggatccgggcaggtttacgctggcaattttatcggtggtgatccggttgtaataagcgatgcttccgttcaggcggttattgaataatccgtattccacggcgccttcaacggtatttgttttctcccaccgcaagccgggattgggaatattacccaatgaaaatccgatcacactttcataacgggtggtagccgggtaaccaccctggagggaatatacatcgatagtgccgtcggagcgttttcccacttcaccgatgttaccattctttccccagctgccgcgcaatttcaggaaggataaccacttgctggtgttcaccataaagttctccttgtgcagcaaccagcccacggaagcaccgggaaacaggccatactggttatcgcctatcagcctggaatagccgtcccttctggcggtaaacgtagcgaggtattttcctttccagtcgtagttaatacgcccaaagccagagaagatacgttcccggagatgatacgaattttgcccgcgggtgttggcgtcgctggaggttaatcccaacgtcgggaaatcatctgtaggcgccagtttcccgctggccgacaagccataattataagcgtcaaaaaattcaccgccgatcatggcgtcgatgttgtgatcgtcgtgaataattttgttgtagtgaagggtggcgttataggtttgacgcaccgtgcgatcaaaggctgcactgctgttgcgggtgcggtcccatcctgcgttgggatcggttttactcattacgccggtacggaaatctttgttgaatgattcgttaaagctttcgtcgtacatgagaatagcgcccactctgaagtaaagatctttgtacaggtcaactttaaaagattgggcgagggtaaatttatctgcctggtttttccgggaatatttgtccatgttcacggcggggttaccatcgcctgcattccttcccaggagcggttccccgttggtgttgctgccacgcatggtaggcgcggccatcagcaaacgcccccagtaattcacatcgctggtttgtgcctgatcccgggagttggcgcgggaaaaggacacattgctttccgacttcagccaggttcttattttgtaatcgccgttgagcgtaaaattcaatcgcttgtaaaacgatttgcgtgcaataccatcttcgttataataaccgaggttggcatagtaggcgcctttttcgttaccaccagtcatactgatattataatcctgtgtgagtgattttttattaaaggcattgtctccataactgaagcctttatagataaggtctgcataggtaccgttgggatcatactgcccggcggcattggtggggatagcgtctttcattactttccagccatcgttggcagagagcagttccctgttctgatcggtgaggcgcatggggctgaataaggcattgaggttgtagttgccgtctacaatatttccatcggcatctttataaacgttgccggtaccacgtggaccggaagcattgatcaggctttggttaccgtttaccttgtaggtttccaccagtgcttttcttccccagtataaatattcttccggggtgagtaaggtgtagggagaatttaaatagttgaatcctgtttttactttcaggttaatttccgatgtccctgactttcctcttttggtggtgatcatgatgacgccgttgctggcgcgggcgccgtagatggctgtagccgatgcgtctttcagtacttccatactggcaatatcttccgggttgatatcacttaaagaggggcggaattgtccgtcgatgatgatgagtggactgccggagccatcgaagttggtaccaccgcggaggatgatgttggggatagcgccgggtttaccggagttggtggatactctcaccccggcaatggtgccggccagcgcctgtgcggggttggcgcggataccagattcgaggatccgtttgtccagtcgcgctactgatgcggtcaggctgctcttcttttgtgtaccatatcccactactattacttcatccattttagaggtagcggataccagggagatgtttaccgtagtgcggtttcctgctgcgatttcctgcggcgtaaacccgatataggaaatgcgtagcacatcttcgggtgcagctgctatgctgaagtagccttccgcgttggtgatggtggccgttttctttcctttgatgacaacgcttacaccgggcagtggctgctgatcttctgaagagatgatcctgccggtgattttctttggttgagctacagctattgtactgatggcaatggcaaggagtacccccatcagtttgttgagagcaattttcatacgggaatttgtttagacaattaacttgtactaatattcttaaatacttatgtactacatattaaaattgcctaaaaaaatccataccgcaaaacatttttcaaaaaaagaaaatgccggtgtatggaaagatgtatgaaagcgaaggccatagccacttttggagcaatggactggcgtaacttatcgtgcttactttttcagctttttgaaatgatgttcaagatgtttccgcatgccttcgcggaattcttcccgggagccattcttcaacaggtttaccaaatcgatatgtgataccttgcctacgatcggcactttttcttcgttcaccaggtgtccgaaaataggaagcagcatcgtctgaaaacgttgcatggtgcggttaccggtcatctggtaaattttaccatgaaattctacttcatgtttaatccggaaattttgtttggtgggtgttgtcttctgactgagggcaattttctccagttcttcaatgtccttttttgttttgcggatatataaaatatcagccaggcccatttccagggtaagccgcaattcaaaaatatcctgcagcgtggtatcgtcgatgatcagcggatccatcacacgttccatggagcccaggatatcggggctggacagtaccatgcctctccgtttctttgtttcaatcatgcccagcattctcaagcggctgagggcctcgcgcaatacattacggctcactcccagggcttctgtcaactccatttcttttggcagggcatccccgggtttgaacgattttcgtttgagatattccagcagcttcatttccacctcgtctgccatcgttttataactcacttttccaatatcgatatgtaaattctcaattcccataaaacaagctgatattttgtttaaatgtactacaaattaacagatcaccaggatcacatcaataatatgcgtttactcatgcagcatcaccggctgctcttgtaattgacggcgggtatattcaagcccggctgcataaatagcctccaggtgcttgaagtcaaacataccgaatttacccaggtctgttggttcaataaaatagctgcacagcaacttgtttttcagtaccggctcacgaatggccaggtgaagggttctttccacattggccaggaagccttctgccgggttgtaaggcgtaagcggatttacatgcaccccaatgatatcgtggtattcggccaggagtggttctatgggcaggttgccggaaaggccgccatctacatactgtacaccatttatctccaccggcgggaacagcagcggcacagaggacgcggccaggatagccgggatcaagggaccttcactgaaaatacgttgattgcccgttaaaaaatcagtggcggtgatatacaaaggcgtattcagttcttcaaatgtctgatgccggagtgtttgctttagtacttctgctacttttttgagagacagaaaaccggcacgccagttccgccagtgcatcgacagcccaagcttatgcgcccggaatatttccctcacctcatcggtgttgtatccatcacaaataaaagcggctgctatagaacccgcgctggtagccgaaattgcttccgggtaaatatcctgttcggaaaatgcttttaaaacgcccaggtgggcatatcccctggcgccaccaccggataaaacaaacgggcgtttcacagatgggcgggtttgctgatcattcatccggctaatataaaaaaaccttccgcattttacggggtagtctgaaacattatataaaccgggctctcccccacttctaaacgcacagcagtatccccggttttctcccacttcacctgctttgcaggttcatctgcggtggtcatagcggtagcgctcaccggcaacgacggcagattatccagtaccgcatttaccacatgtggctgatagcctttctgctgatgggttttggcgccggtaggcgaccaggccacccataccagcatcttcggatcatctccctttataaattcaaacacatacagggaatctgtttctttttttacaacacgccggaaacggtagtctcccaatgtctggtacagttgcttcaccgcccagaacgacatcttcggaacaaaattccgcgtaagcccggaagcggcgtgaaaagaagcttcatcttcatcattatagtaatacaggtaagcacgccgtatgtcaagcgtagcgaacatcagaaaagatcgcaccaggtactgcgcctgctgcagatcgctggctccctgccagttcagtttcagcgcccagtctttccggtgcttcatggcctccggcgtacatgcatcatacccgaattccgttacccatacttctttgtcttttgcatgctgattgcgccatgtaatggcatcctctattactttgagatattgcagggaattatcttcaggataacttctgttccagctgttttcattgccggctgattgtgctatggtaggataagtatgcacattgatcacatcataaaggggaagtatttttttatctatatacaaatcattcaatccctgtgaatatggatctgcctttacggctactgccggtgtaacaattttcatagccggatcgccggcacgcaccccgtcggccatttttgtaaacagcgttttgaaaagcgccggatcaaacctggtacctggctcgttatcaatttccagggaagtacataatttttccgctcctgatggcccgtaataagccgccattgctttgccgtaatcatatgcccactgttccttaccggcccataactgtttgtagttaggacttcccaatcctacccccaggaattgcatacagatatctgtttcaaatcccgcttctttccagggtccataagcatcgcgtttccagttaatattattgatggtgttagggatggtgatgggatcgccgggggcttttacatcccagctgatattatgataactgcgcaccagccggcatacctgcttatataaatccggtttgaaagtaagatggccgttgacacccataaaatccctgaatagcggccggctggtaaccggtatggaatcggtggtggcgaggctcgtttgtgcaggaccatgttctgcacagcttatcataagagcagtaaagaagaggatggtggtaaacaaatacttccgtggcataatacaatgagcataaggagtgaaacaaaaacggcgaatggtaagggtgaagatatataaatatctttactcttaccatccgcctgtatcattgttcgctattcgcggttagtttctccagcccggcacctgtttgtacacaccgttgctctgcgcaattacatcaggattcatgggccatgccatatgtttggccgggtcaaaattacgtgccggccatacctgttttatttcgtaagacgataatggattcaccttatcgctgtggatacggccatgtaaaggcgcattgatctttgcataatcgccccatctcttgagatcctgcaggcggtctgtccattcgcaggccagttccacgcggcgttcatgcttgagatcctccatcgtaggatttgcaatacctgccagtcctacgcggctgcgcacttcattcagcggtgcagcggcttcgcctgccctgcccagtttgatcagcgcttctgctttaaagagcagtatttccgcatagcgcatcagtggtaaattgagtgcggtagttggataatccgggctctgattgatgttggtattggtggtaataacaccatctttaccgtaagagtaaggctccatatacttattcatctggaaacccgacaagctgttggtagaatagtaagaacgcaccaggccaaagaaagtgaacttatcaccaaatttcaggatggttacttcccttcttgggtcattcgcttcgtattcatcatacagttcttctgtaggctggaaatagccccagccattgaaaatagcccagccggtattttccagtactacgcctggaaattctgaaccaccctgcacaccggaagtaacagaccacatatattcagagctccagttattggcgatactgaaaacagcgcggtaattctgctggctgttttcttttcctttgatgagggcacggtggccttcatccctgatcttatcagcgagtgccgggatcagcgaccatttggaggcatcgtactgtgcccagtaagcgtatgcttttaccatatagccccatgcagcagctctgtgcgcgcgtccctggtcggaggtgctatatgtttcaaagaggggcagcagggaggctgccttttccatatcgctgacgatttgtgcatagttgtccgttacagaaggtagctgaggcggaatacgttttccgaattcaggattttccggtccgtcgaaaggaacgccctggtctttatgcccccagagataagccacccagaaatgtgcaaatccgcgcatgaaatacgcttcgcccaatgcctggttgcgtgctgcttccgtggtattttttgaggtgggtacattctggatcacctggttggcgcggttgatcattttatacagatccgcccatccgcttttcaggtaaccttcacggccacttggaataaagttcttgatattttcaccgtctgccttcgcccttcctacaatcaggtcgtcgctggcatcctgcacccagaaaaggtcgcgcccccaggtagattcattacgcatggccacatacatgtcgttggtagccttgcggagatcattgtcactttgccagaagtaagcagtggtaggtgcgccgttgggttttgtatctacccatttgttacaggcacttgcactcaacatcagcgatcccgcgagaaatatatgtttgaatgttgttttcataaaagcgtttggtttgatcagaatttaatatttgcacccagggaaaacacacgtgataccgggaactggccaccatccagaccgataccgcccacttcagggtccatgccggtgtatttggtgatggtgagcaggttatcgccgctgaagtatacgcgaagcccctggttccagctcattttcttaaaggtatagccgatcagcaggttctttaatctcaggtagttaccattttcaagataccagtcggagttggtctgaaaatttttattgggatcatttgcagagatacggggaatgttggatcctttattttctggagaccatgcatccaggattttatcccaacggttgtacccctgttcggagccgcttaaggtggtcatcttgaaagcgttgaacagctttacgccgcctacgccctgcataaacaggctcaggtcaaaatttttccaggtgaagctggccgtgaatccataagtgagttttgggaatgcattgcccatgtatacacggtcgccatcattgatggcgccatcaccattctgatctacaaatttcaggtcaccggctttcgcactgggctggatcatcttaccatctttctggtaggcttttgcttcgtcgtctgattggaagataccggcggtttttattaaccagtaagaataaaacggctgccctactttagaacggaaaggcgtgagcactcctctgaaagcatcattgtgtaccattacagaggagggatcagtatcgatatattccacattgttttttaatgtggccatattggcgctcaggctatatcccagctgtcctacgtgatcattccaggatacggcaacttccacacctttattgccgatttcccctttgttaatcaggggcgcatccagtccaaaggtattgggccaggcagcggcctgttgttggatcaggtcgtaggtgagtttatcaaagtaatcggcggtaatggacaggcgttgtttcagcaggctgatatcaataccgatgtctgtttgctgtgaagtttcccaggaaagtgaaggattgaaggctgctgtcattgccagggaattgcttcgtggcgcaccatcgccgatctgaaaggtataatccggtgtgagtttagcataaccataatagtgtgcgatagagcccaggttacctattcggccccagcttcccctgatcttgagcagatccatccattttacattatccatgaaagactctgagctgattttccatgcggcggttacacccggaaatcctttggagcggtaaccttctgctaacctgccggctacgtcattacggtaactggcggttacaaagtaccggtctgcccagctataggataatcttcctacgtaggaaactgtccggtctttccattcatcatcagccggcagattctgatcaaagatggtggcattggtaaaaaactgcgcccagtctgcctcattttcaaatccttttgcagcagcggagaaattgcggttggattcttcctggccggtcatagaggccatcacaccgatgttatgccggttgatgatcttattatagttaagggtattttcccagatccagttataacctttgtctgtagaataagttaacgtattctggtcatttggttttccgggttctgttcttctgggctcaaaatttttccacagtgcattttgctgacggtaagaaaaacgggaaaggtaagtgaggccagggataatatcagatactgttaattctgttaccgactgcagatcgtttcttttgttatagggtttgtttctcaacagggtagctaccgggttgatcacatctccataaatcccgttatactgagaacccctcggacccacaccgccaaaggtgccatcgctgtaatacggcgtagcagaacggggcatatacagggcggagaggatagcgccgctgtaaccgctggcagtttctgcgtccctgttatcgttgttattccagaagatatcctggcgcagtttaacgttcttagtaaactgataatttgcattaaatctcagggaaatatttttattataggtattgatcagcgtaccttcttccttctcataacgtgcctggaagagggtagaaaatttgtctgttccggcgtttacgctgatattgtgccgttgtacgagaccagtacggaaaatttcgtccatccagtcggtgcggtttaccaggccatccgggtttttagcaggattccatccttcgagcgggggcaatccggcattggtttgtgcgaggttggataccctgccctgttcttccgcggtgagcgactgcaacgtacgccatggttgcttggcgcctacgaagccggtatactgcacactgggcaacccttgtgttgcctggcgggtagtgatgaggataacccctgccgaaccggagaaagcgccgtaaatagctgcggaagccgcatctttcagcaccgtgatcgattccacatctgcagggttgtaaggggcgccgggtactccatccaccacatacagcacattttcactgttggccgaacccacgccgcgaatggttaccttgttggcattgctggtatgaccaccattacttaccacggtgataccaggtactttaccctgtatcatattggcaacatccagtaccgggcgttccttgatctgtttcatgtctggcactactgctacggcagcggagaggtcacctttttttgcggtgccataaccaagtaccaccacttcattcagtgcgttgttgctggttttcagtgtcaggttcaccgtatctgagctaccggcaggcatttccacggtttcatagcctacataactgaagctgagaattgctttatcgttttccagggtgatttcaaatttgccatcggcatctgtaacggttcttgttttagtgccctttacccaaacagatacgccgggaataggttctttatcttcggtagttacgcggccggtaattttgcgggcgactgcctggctggtttgtacttccggatctttttccgctttcctgagcaggattgctttgtcgcttacgctgtactctatacctgatttactacggagcatgttgagggcttcgttcaaactaatattatccggtttgtaatccctgacaataattttgtcgaagtcctgttttacataattaaatgtaaagctgctctggtgccccagtgcgctcagcacctgggaaagggaggcacgggaaatatccagtttcactttttcgctcaacccggtttgcctggcgtatccgaaggtagctggcaacagggcacatcccattagcaggaaacgtttgatgcgggatacagcaggcccgctgctgcgggtatgctgatcagcggaagtaaatgtcattttcatgtgttgaaattttcaggagcgttcacgtgttatttaatagatggtcacctgtttgtcggaaatacggaattgtttacggctgatgtagcatagattccccagcatttttacgaagctgtctttttggaagagcacagaaacatttttttcgatgccttgtgtgttctcccatttcacctgataaccgttgcgtgtgcacaatcgcattacggcatctttgaaaggcagatcggtagcgctgaatgcgccttctttccaggcggccactttgccggcttctgtagcggaaatattcagtgctttatcttcattattataagcggcggcatagccaggtttcagtatggtactgtcttttcccgtatgtacttttactttaccctgtaccagtgatacacgggttaatccttcgccggcataggcttctacgttgaactgcgtgcccagtacctggatcgcgagatccctggtgtggatgacgaacggcttgttcctgttgccctgtacttcgaaaaagccttcaccggtgagttgtacattgcggctttgtttattgtagtcctccttccatttgagagaagcggcggtattcagccagatgcgggagctatccggcagtacgaccagtttaatatcgccggtttcattggtgacctggaatgatttgttatctgcgaggcggacaggtggctgctgtgaataacggagccacataaatcctgcaccggcaaataacaagatgctggcggcggcagcccattgggcagcacgttttttccaccaggccaccggggcagccggcaacatgctgtgaaaattagccaggaattgctgccggtaaaggtttgattccagggcagacaaatctgcttcgctgtttaaaccgtcataccagttgtccagtaatgccagttcttcctgcgtacattttcctgcatgaaactttttcaacagggcttctgcccttggatatttttgtattgccatctgttaatgaatacccgcaacacaaaaaatgttaactcgatctaaggttaaggaattgtaaacagtaaaaaagaggagataaggctggcagacaaagccggatttgctttaatatgtgcctttacctgtttaagggcacggctgtataaaacgcgcgcggagccggcatctatacccaattgctgggcaattttctgataagaatagtggtggtttacgcgaaggataaatagttggcgctgactgggagaaaggatttccagcgcttcagagataatggtttcttttagtccgtgcagttcgtcggaggctattgcacccggtgactccagggtgtcgtttaatagtatttccagctttttcaggtgtgcctggtaacggccattggtgcgataatatttaaagatgcgcagtttcagggcatggagcaggtaaaactccagcgtttcatctttgggcacttcctcccatttcacccatagtgaaagcagcacatcctgtacaatatcaaatgcgtcgtgcggattggttttggccacggcgataccgagtaacttatcccagtaggaagctacagccgcttcaaagtcggcctggccggaaaccccggatgcatgatggaaagatattttcttaagcgcagacataagttgaaatataacagtccctacaaaagtaattgtctaatattacgtggatattaacgttatgaatccaggcttcttttcttttgaaaatcgatttagcagatcctcacaggaagaagtggtgttgctcctgtgctgttcattataaagttgttactgtactttgattgatattttaatgtggactgattggcctcaatcaaatataaatttactttttcaaacgggaaagaatatttataaagcgtacatcttacctcaaaaaaagtatctttctgcctgttttaaaaagtcgcctatgctcaccgaagatgcagctatcgccatacaggaagaattgcgccggcaggtaatcaccaccgatgaattgccggataccattaaaattattgccggcaccgacgtggaatacgacaaagattccaacctgattgccggcagcattgtattgctggattacaccacgctgcaggtactggccgtggctactcattgtatgaaagtcacctttccctatatccccggattattttccttccgggaaatgcctcccctgctgaaagcctgggaaaaactccccctgcttccggacctcatcgtttgtgacggccagggactggcccatcagcgccgttttggaatggcctgtcactttggggtaacggttaacaaacccgtgatcggctgtggtaaaacacggctatgtggtgaatatcatcacctcggagaagaaagaggcagtgttgcccccttaacagaagccggtgagcatatcggtaatgcactgcggacacaaaccggcattaacccggtatttgtttccacaggacataaaatatcgctggctactgccactgacatcgtactgaaattatgtacacagtaccgcttaccggaaaccacccggatatccgatcattatggacgactggcgctgcttgaatacaaaaaagaagggtgatagaaatatttggagaaatgattttattatttatatatttgcaaccccaaacggggaatacagaatggctgaaaggcttgcctgtaggaaggatcggtagttcagttggttagaatgccgccctgtcacggcggaggtcgcgggttcgagtcccgtccggtccgcaaagccactcttaaagagtggctttttttattaaaacccgctagaatcagggttttagcaagaaaagcatattaagtaataaacaaacattaccaaagagaaagggtacctaaaagggtacctattttatttccgaaactgggccccccggttagcccaatgtttcactcttccagctgactatcttgattttattaagaaatataatgggacgaaagagcaatcggaaataatcaaaatctgaaattgtggggtattgaggaacttgttaaattaaatacgtactatgaggtgtatcgctatgcatctgattatttcatttttggctctgatgtaggaggaacagcatacgctttcaataagcaaaattcgtcaatagtataagctgaccgacagaaaaactatcacggaatatgaaaattgagcaacacttatctaagaatgagttgactgacaagcagtttttggtgattgcatttgaaacggttaaatatcttggctggcgtatcagatttatctcagatgccggtgtcattgcttataccaataatggcgagcattcctggaacggagaaatcactgttaaactggacgcatctggtgctatggtgcaatgtgttaccatatcaagtctgctaactgacaacggacgcagcgaggccgccgtacgtgcatttgttttctcatttgaaaagataaaatcagagatcaacgaagatgaagtgcatgaaaaatataaaacctacaaaaaagattttgttcccgcttacgaagatactttaaagcccgatgtaaggccgaaattttcttacttaggtgggttgctgtctttttttaaaccggcaacaggctacttttttacccctattctaattgtactcaatattttaatctacctcatcatggtatgttcgggtgtagctgtattcgagcctgatgccgtaagcatgaccgcatggggagcgaatgcaactatttatacgctcgggggtcaatggtggagattaattacgagctgctttattcacttcggcataatccacctgctgctaaatatgtatgcccttgcttttgtaggattatttttagaaccgtttctgggaagggtaaaattcgtcacagcataccttctggctggcatttttgcaagtgtgatcagcctttggtggcatgacaataccgtgagtgccggcgcctcaggcgctatcttcggattatatggggtattccttgcactgttaagcacaaatcacatcgagcgttccatgcgcaaaggtttgctcacaaacatcggcctttttgtggtttacaatttagtattcggcagttttaaaagtggaatagataacgcagcacacctggggggactgcttgcaggcgtgatgatcggatacgcctattaccccgctttgcaaaaacccgggaatgtcttgttaaaatggcttacacagatattgtcgataactggtgtcattcttgtttcagcggtaatttacgttaaccttgccaaaagcgacaaggttacctaccagaagcagatccaggaattttaccaaatcgataccaatgcattaaaagtgctaagagggcaggaaaacagtacgggcgaagaattatttcgggcactgcaacaaggaaaatcagcctggagtcatggtattgaattgatcaccgaattggataaaatgaacctctctaaccggttacacctgcgcaaccaaacgctcatcaaatattgcagactaagaataaaagcttgtgaactaatcgcccaggacccggagcaaggtataaatagctattcatcagaaatgcaacagattaatatgcaaataggggaagttcttgacgatctgaaataagactaagggtataaatagactaaggagctgcaccgtggagtaggatatgcacttccccatccagggtaaccatatttagctatgcaacctttttattcaacagatttacgagttccatattacctactttttccgcaaaagataaagggcttgcaccagcgttgtttttatggtttggatccgcatgatggttcaaaaaaagttctacaatagcatgctttcttttgtcaccccgaacgtaaaaaacagctggccatagcggttggttaccaaaactatttgttgcggcaagattagcatgatgatttagcaataaaactgctatatcaagcaaattgttttcggctgcatgatgaagtgtggtattccctttatagtcagggatatttggatcagctccattttcaagcaataattttaccacatcataatgattaagcgccacagcagttgccaatgctgtaaaacctacgctatcttttatattgatatcaactgaggatcgggtcaataattctgctatcttttctatttttccgcctattgcgagttttataagattgttttccatttaataaaaataactatttgttgttgaaatgtatatttcaacgaagatggttcttccccccttttgttgaaatatacattattggcaaccagcaatacatgcaaccacgtgaaatcatgactttgcttttccagcctgattgccaccagattgccggttaccggctttctcttttggttaggaaaaagaaggctgaagctttgattattatagaataggtaaataatagctaaattgccgacgatctcttctgttccatgatgaacatacaggtatcagcaactaatgaatttaaagtctcttaccggaacgaataacacaaataacagacataatcctattcaaatgataaaacaatatcgattgttacttttagcagttttgctgataggttgtaaaaaggaaccagctatagaactggaagattttaacctgggcagcaatttatcgacatttgtatcggccaaaaacaagcacaaaacttatactaattattatcaaataaaatctgaaataattggcgcagacaccgttttagacggtgaatttataggaagtgagcagcccataagaattgactataaacagcaaatgttttcccagaaagatgttattgcaagattcggtgattttgagtttaatgcgatcaattttgccacaacggtaaccggaaaattgatggttttcaacgcggttgcggggaagatttctttgaaagaaacccaacgatttgtgcagctattgaatgacaaatatgggaaggcagttaagaccaagagcgagtttattaaaccatttgatatttattcctggcaattaaaagacaggatcattaaatattgtgtggtaagtgagaatgatagcaatgctttgaaagttggtactgataaggaccagcagaccataaaagaggggaagaacgaaacttatctgaaagcatttatatatattattaagaaggaatatgcagaccaggtaattggtaaaatgagtagcggcgacttactgtattgcgaataacataacaattcgttatttttccggggaaatggattctgttatatgaaaaaagtcaaagtcagccgctcctcctatattctttgtagcataattaaacaaagcaaaacgatagcccatgaaatgcgggaaggtataggccatttttaattgtgtgcccaatggtatccacgttttcccatcgagactataaaaaaaatctgctacatcttttctgtttgtaaaattgcattccgccttaaagtatactaccttttggtccagagggattttttgtgcttctacaggttggccggtgctggcattgatcattacgacagctttgttattcccggttattctgacaccagccaatccataatttttttgcaaaaggcccaaacccgcaaaatcaccatctttcatattagaaatgtcaagcgaaactgttccggagcataccgggccaatagtgcgttgtgtcaatgaatttcgtgccatcacaaaatcggtgtcaatcctgccggtggtgagtcgtaaataccctttccgatctgtaacagaccataaactattatccgggttgtggttccattgccaaaccagtggtaatgcccgttcgccttttttacgggtaaattcgtccgaagcaacaatgccggggatcaaacctttaccggccggcagatcgattgtatcgggcactttgccgttggtgcccaaaacgggccatccatccttccactttacagggaccaaatagggtatccggcctacagcgccataatcacggaacaaataagaataccaggttccatttggcgcttcgaccaatccgccttgcgccacgcccagatcctgtaacccaattcgtccttcgtacgggccggtgattttatctgcccggtgtattataacagtacgtatgctgccctttggccatgtaatattgaaaagataatatttgccgtttatcttaaacagctgagaaccctctggaccgaggccgcccgaaggagggcttgcattctcaatgataagcaggtctgttccgcctggctttatgcccgacaggtcctcatttaattcaaccaaccttaatttcccgcttccactaatcatataaaccttcccgtcatcatcaaaaaacaaagagttatcacccagatcgggggcaaatgaccttgccttccactggcctttttcgatatcttttgtagagtagatataagtttttcccgtggtttctgcaaatgtgcttacataataggtgccattatgaaaacgaatagaacttgcccacgaaccatgcccatatgcgtttttgccatttgtgagatttaatgcatcaacatttgctaaagtatcatatgcataattcaccagcttccagttcaccaggtcgttcgacttcataatcggtacaccgggactcatatgcatcgttgtgctgctcatgtaatagctattgcctacacgtactattgatatgtccggtacatctgcataaataatgggattagttgctttttgtgcgtataaacacggtactgcaagggtgataatgaaggccgtcatccataacctgtaaatctcatttctcatattcagattttttttcctggtacgcttacctgattttagttaatgtatttatttaaagcacgccaactaaatatgggtcgaaagtacttcgatagtgctttgagttcgaacattatccccttaatgataattcgaatactgaaatttacgaacaaacatcagatctatataatctgtaatcaaaggcgctaactcatcaactttctccagtaatttttcctccgctgcaggatcaatatcattatctcctgatatcttactcttaatttcttctttaaacaaacctatatataatgacctgatatttttatagcccggtaaactgtcgacaggatcctgacaatagagatcatattcaacataagccggtattctcttgtattgatgcccaaaatacgttcctccgtgatgtaattccccgtaaatctcattaacatatctatacaacctaagcaatctttctcttctcagatgctggttaacattcttctttttccaaaaataaccataaaggagatagaactcatcctgccctgcttcaccaccaaaacgggcatcttccggtgttggatgacaccaaaggtttgcataagcttctgccgggctggttggatatttctccatgaacaccggatttcgttttaagatatcttttagctcattttcagtatagacaagattagcgtcactatctattgtgattttagggctactatcttctttttttgcagtatcaacttttgtgcggtgatcaggtttgtttgcatgacaggcaacaaggcagaacagtagaaaaaaaagaaatcctttgtgcatataagtagggctagttatggtaaagttacccttctctgaattaaaaaagttcgaaacttttccttccaccgcgcaaagccactcttaatgagtggctttgcgcggtggagcagcagttctcaaatacattgctatgctacaacaaggataactttaccgtttacgccgccagccgttaagaaatcctgggcctttgctgcttcttcaagcttaaatgttctggaaacaattggtttgaattttccggctgctaccaggtccaggccatttttcaatgtttgaaacgataagtcggaagcgataaaacgcgcttccacatggaactgttctgccagctcctgtgaaggcggcaccacgatactcaatagtttaccaccctgctttaatacccggaaaagcccggcctgggcttcgccgccagccgtatctgcaaccaggtcaacgcctgtaacaatgctggtcacatcctgcaatttataatcaatcacttcgtcggcgccgaggctcttagctaaggccacaccttctccggatgcagtagcaatcacatatgcaccggcagcttttgccatttgcaccatagccccgccaactgcaccgcccccaccctggattaaaactttctggccttttgctaacttcccttctgtaaaaagaacagattgagcagtcccgatattaacacctatcgatgctgcctcttcgaaagacaggctttgcggctttggcacaacgaaattttcgtttgcaaccacaaattgtgcatacccgttttttaatgggatagcgatgacttcatcacctgttttaaattttgatactttttcgccggtggcaacaactattcccgccacttccccacctggtataaagggcattttcaccggacggatctgcttcataaatcccatgcgtattttcatatctatcgggtttacacttgctgccttcacctggattaaaacatcattttcattttggatagatggtgtcgaaacctctacctgttcaatcacctctgaattaccaaaggctttgtattgcattgctttcatattatttttattttttaaaattgtaaatagcttttttactgaagtgaactgtaaattggataatcaatgtaacctgtttcgccgggtgtatacaatgtgttgaagtcaacatcattgagggggtcgtttttttcgatacgcctcacaaaatcaggattagcaaggaatccccgcccaaaggcaacaaggtctgctgagttgtcctgcagcttttgctcggctgtctccattgtcaagccgttacagtatatgatagtattattaaatcctgtacggattgcatgatatgttttctctggaattgccggattggttgacaaatggatataggcaatccctatcttatccaattcactgctcagataggcgtatgtttgatgcacctcttctgtatcgtaaggctgttgatcgcttaattgggaaaacggggaaaaacgaatccctattttatccggaccgatagcagctgcgatgcccccggtaatctctacaatgaggcggctccggtttttaaggttacctccgtattggtctgtcctgttatttacatttggatttaagaattgctccagcaaataaccatttgcgccgtggagctccaccccatcaaaacctgcaaggatcgcatttttggaagcgcttacaaattccgctatcacacgcgtaatcccctccaggctaagagcttccggaacagagtgttgctgtaaaccaagcgagtcggtaaaatctcgccggcagccctgatattcgaaggacctacgggcagttgtccgcccggtatattggcaacatgcgcaatacgtccggtgtgcatgatctgcaaaaaaatctttgatccgttttgatgaacagcatccgtaacttttttccattccttcacctgttcatcagaataaataccgggaatacgtggataaccaagtccctgggggctcggtgctgtaccctcggttacaatcaatccggcgcctgaacgttgtgagtaatacgttgccatcagttcatttggaagattgccaatggccctgctgcgggtcatgggcgccattaccaaacggtttttgagttttagcgggcccttctcgaaaggcgtaaataactttttcattttgtatgatgatttaattctgcaaacaaaattagaagttatgttatgggtaaaataacccaaaagggcgtaagaatagtccaatacgacaagggtatatttaaacttaaaaaagttgtgaagtaaagatggggactatcctttgtaggaaaactttttgggggtaataccatattgcctttcaaacaatctgctaaagtggctcagattggagaacccgagctcataacccacgtcagaaacggagagtttggcctgtttcaataaaaaggctgcttcttccattcgtgcacgctgatagtaattgtatatagtaacgccaaaagtttgtttaaagagctgcttaagcttggtttcactcattgaagcgatcgtagctaattcctttaaaaccggcggagtactaagatctcgtaatatctcgctgcgtattaccaggagtttctcggcgtcggtactattaatatttttaaatgtggtgttctccctgagcgacagcttactaaaaagcaagtacagtacttcctgtaccttaatctgcacatagaaattgttcagggagttattcatatcgacagacacaatatttttaagcagcaattgcatttcagcatccaaactttcgaaaaagagaaaggaagcattttctgcggtaatggtttttattgtactgttagggttttcgatagatagaatgctgcgcaatctatctgcagcaacacccactactacatactgaatattgctgcccgctgggaaacggatttctgtgcgcaagtcgtttgtagaaagctgtatggcggaatcattcttttgtgagaacggtatgttttcctcgttattatatttaagttcaaaatcttcttcattattgtaaaagaaaatggtacgtatgttattgtatatgatggccggattacgtttaataacaaaatcttcttttaatttataccggtggatggttaacctgaaatcatccccaaacccaactttacgtacgtaaccttctcccagtcgcgctgggatttccaatacattatctctcacaggcacattaatctgttttgaaaaaaatgttataaagtcaaaatctggcgacgctgtaaattcaaaaatcatataaccaggtaagttattactcactctaaattaacgtaaataacctgtaagaaaccgaaaaaaacgactattttgttgattcaccttacatcacgtatgttcaagaaaaagaagcgttatgcggttccacttatgataacaaagttcctcttcctatttacgaagacatgcatcatcattttgctgatattgtggtaccccttgtccggaaaatcccaggccaaccccttcggcaatgcgcttatccccgacatgattgctgatgcaagtatccaggaaataaacggcacattctattgctatgcaactacggatggttacgacgatggcctccgcacatcaggaccaccggtggtttggaaatctacagattttgttcactggagcttttcggggacttattttccgtctgccaccaggcagttatattgggcgcccagtaaggcgatcagcgcaaacgggaaatactatctttatcccactgtcaacggatacatgtatgcagcagttgccgattcccccgacggcccattccgtttggctaccggagccgatacttttataaagccctactcacccaatacactgttacaactaaaaacgcccaaaggtcccactggtattgatgcggagatttttacagacgacgaccataaagcttatttgttctggcaaatgaggcatgcagccccgcttagtgtggacatggtcactgttgataccaatactgttaccataccaacaccccgcagcggctattccgaagggcccatttttttcaaacggaaaggcatttactattttctttacacgcttggcggagatgaaaagtatcaatacgcttacgtttcaggcaaggcatctccgctgggaccgttcgatgctcccaaaaacaacgacatcatcgccaccacaaatcacgagcgccagatctttggtccggggcatggatgcgttttcaacgttccgggtacagatgattactattttgcgtatctcgaatatggaagaggaagtaccaaccggcaaacgtatgtcaacaggttacgtttcaatgaagatggatccattcagccggtcgacctgaccatgacaggtgttggcgcactccatccggtgaaaacgggcgctcccaaaaaagttatgcaagccaccgcatcgagcacccgggctgatttgaaaatcaaaccggcaaaagattccctgcttcatcgtgttgaatatttcgtgccctcctttgcttttgatggttcaaacggatctcgttggatggcttctcccgaagactccgcagcctggatcatggccgatttaggtaaagtcacgagcataaaacgcagcgaggtttactttgtccggccaacagccggacacgcttacgttttggaatattccacggatgccacacactggtcgtcgtgtggcggtcacaatgatgttaaaatacaatcccctcattccgatgctgtcaatatcaaaacgcgctttttgagaattaaaattactactggaataaaaggtgtctgggaatggaatatttattaaaagatgggattatgaataatgtcaagctattgatagccctctggacgtgccagctgctatgcataaatgtatttggtcagcaaaccgggaaatggggagatcggggagatagaacctatattaaccccgtgctgccaggcgacttcagcgacctggacgcgattcgtgtgggtaacgatttttatgctatctcatccaccatgcagtattctcccggaatggttgttttacattcaaaggatcttgttaattgggaaattatcagccatgttgtaccagatcttacaaacatctcacccaatctcaactgggataagatgaactgttatggcaaaggcatatgggcgggttctttacgatattacaaaaataaattccgggtatatttcggtacgccggatgatggtttctttatgagtacggcagcaaatcctgcaggaccatgggagccggttcatcaattgtggaaagtatctggttgggatgattgctgctccctctgtgatgatgatggtcaattgtattttgttgccaccaactatgaaactgatccccaaaacaataaaaaatacaatatccatgttttcaaaatgacaccggatggaaaaaaattgatgatggaaactgacagcatcatccatcagtcacacggaagcgaagcaaataaattgtacaagataaatggcctttattaccatcttttcagtgaagtaaaatcagaaggccgggttatcatgatggagcgctcgaagagcatttatggaccatgggagataaagcaactaaaccatgtaaataaaacgctggataaagaacctaaccagggagggcttattcaattaaccagcggagcatggtatttctttacgcatcatggtacgggcgattgggaaggccgtgccgccagcctgcttcccgttacctgggtaaatggctggccaattattggaaaggtggggaatgataccattggttccatggtttggtcgggtcgcaaaccgatacatcttaagccacctttgcttaccatacaaaccgacgataattttaattctgctacccttcttccacaatgggaatggaattaccagccgagatcagataagtggtcattaactgaccgtaagggattcttgcgattgtacgctttcaaacccattacggctgacaataagaatatcctgttacaggcaggcaataccgttacccaacgcagcctacgcacaacatccaatgtagttaccattaagctggatatcgatggaatgcgtaacggcgaatatgcaggactgacacatttttcaacaccgggtacgagttgcattggaataaagcaggttaacaactcgcggtacctgacctatacacataatgaccaggactctaccgggtcaaccattgccgggcgtactatctggcttcgatctgcctggaactaccggggggagaacaggtatttttacagcgttgatggaaaatcattttcacctttcggaggtgtatcccggttagcctggggtagttaccgcggagacaggatcggtattttcaacttcaataccgaatcggatagcgggtttgttgatatagattcattccggtaccggtattcaaagtagattacctttcctcctaccgtttaaaaatatgctgggaaaacagatacaggttacgatcccactccgtgttgtcatgcccgttagtatccacactccaaacatgcgggacagatatttcgttaagatactgatgggccttttcactaatcccgaaaaggccgtctttattaccacaggccacccatagcagtttcaacttttcctgggcagttttaatatccggcacaaatttgacatctgtatacataccaccgaacatattcgtattgggcgccgaagaaaatccacctatataggcaaaagttcccaggttatacaaacctatatttaacgactgtcctccacccattgacaaacctgctatagcacgatgttcacggtcactgatagtgtaataatgtgaatcgatgtaaggaatgatatctttcaataaatcctcttcaaatggttttctgtaaccttcaaaaccatcggcccttccggaacggcttgctgttgctgtatctgtcactgtcagctttgaatcgcagttggggaaaaccaaaattacaggctgaattttatcatctgctatcaggttatctacaatgttatctgcctggcaccattccgtccattgccgatagtctgatcccaaaccatgcaacagatatagcaccggatatttcttatctgccgaatatcccggaggcgtatatacactcatttcccggcgtttcccaagcgttttggagtcgtattgaacaacggttaattttccgtgaggtacattattacgctgcacattaaatccggccgatggatcaggaaacgaggggacagtgtccgcgttaaaagaaaccttgcctgtttgtgccaggcagatatgactggcaacaataaatacaatcaaaacaaataaatacctgttactcattttatttttataatgttatttttattcgttccaaaccaatacgcctgctggttccaatactttattcccgatcaatattttggctccggctggcattttcatttcataattatcagaagaataatttacggccacataaaaaccatcgcgccaataaacaaatacgccgggaggataattctcggtggtagcgcccgcgccggtatagatctcccgcagtatatctgtctccagtttagcatcatctgtatctactccgatataggtaacagagcctttgccgattttatgcttcaccaccgctgcttttcctttataaaactggttatcgaataccgcaagggctgctgcatttttatcaggggcaagtaagtcggcccaattgttccagttgtaatgggttgaccccataaggatatcacctttggcgctgccagaaagcatatcggtcgcttttacctgcgctccaatcaaccctgatatgggagccgcccattcgccttcccagaaatggcccatgcgatctttggtggccgtgcggcaggtaataatcaaatgcccgccgttggctgtatattcccgccatttatataccagcgcactatccgccatttcgtaggcaggaacaatcacaaatttgtatttcgacaaatcagtggtttccggaattacgtctaccggtgcgccgaatgattttgctatctccaggaatttaaccgggtaattccaggtatcccattgccaggtttgtttttgccggtcaatcgtccagtaattttccaggttccaaaggattgccgttgaacgggccgccagtttctgaggtattgcagtattgggtttatattgttttctcaactcttttatttccttcatgaattgcatgtactcctcgccaccctgcgaaggagttacgccatctgtttttattacgccggcatgatactgttccgcgctataattaatctggcggaagcggtaggagcaggccagctttccgcctgctgcgaaggtgtgatagagccacatacgtacggtacccggcaaaagcagcgggttgtagcttccccagttcacaggtcccggttgaatttccatcacaccggatacaccgccaaccgatttataatattcagcagcaaaaagaattactttactatttcccaagcggaagccctggtctcctatattattggtaccaccattcggataggcggtgtaagtagcaaagtcgagtttacctgtacgcctgggatctgctccagtagaaacggctgtataattagtagtgatatattgatcttttgagatgtggttccgcagtatgcccgcctgaaaatcgagaaattcaccctgggcatctgcgcagtaacgtttaaagtcgagcaacgcatgaggattatttccccaccaaccaacgaggttagtatttggaatgatcacctggtcaaaattattgtaccactggctccagaaggcggttccccaggcgctgttcagtgcttcaattgttttgtatttttgttgcagccattgcctgaatgcttcctgcgaagacgggctgtaatcgggtttggcatcaggctcattatcaagctgccagccaatcacgtttttatttgttccataccgtttagccatttctgttacaatggtggctacaaacttcctgtaagcggggttaacgattgatcctaatccacgtgtgccctgctccccacgaatgtaatggccatccatcacaaaagtttccgggtaatttgccctcatccaggcaggtgtagttgcggaaggggtacacatcagcactttcaggttgtatttggtacagaggccaatcaccttgtcgagccacgaaaactcaaatttaccctgttcgggttccattttaaaccaggcaaattccgccaggtgcacaaattcatagcccatgccggcaatcttctttatatcccgctcccattggttttcgttccaatgctcgggataataatagatgccggtggtgataagatttttttcaggaaagaagtggttcacctcctgcgaggtggcattcaatcccgaaattaagattgttataataacaagtagcgagcgtttattcatctgttgatctgttttactaatttactgccgaaatttttaccggttttgaaaaattatattggtttcaacaccgctgcaaaacctccgcggcgaagcatcttaacctcaacggtactggatccgtccaccaccaaatactgtgttgtcagcgctttatcgtgtattccatccgtaatgagtgtcagcttgtatttaattccttccggcaggaaagtgaagctgatcgtttccttcttctcccactcctcgccattcatgccaccgatataccatgcatcgtttttgcggcgggcaagcataatatctttaccaggatagccactaagcaaccgaatatcatcccaggcattcggaacttcctttaaaaatgttctggcggcatccggtaattcatgatagccttccggacgatcggccagatgctgaatcccggattcaaacacaacactgagtgccagctcatgcccatatgaagtaatatgcgggtattgggaattggtgaaggtaaccggtgtgtaatccataggaccaaccacgttgcgggtaaaaggcagcgtggtattatgttctggcgcagcgggtgtaaaatccgggacattgttgtaccattcagcaccgcgtactgcctcgtatgtcatcaggttcggataggttcttgtccagccccgtggcaccaggcaaccgtgaaaatataccatcatttgaaattgagccgcatcttccaggatgtcgagataatatttgatcatgtcctgcttctcgctttcaaagaagtcgactttgatgcctgcaacgcccaatttcctcaacttcgtaaattcttccacccggctttcatgcgttaacaacttgtcgcggggagttgaggtaacgccggtatgagggccaccagaattgtaccacatcaatggcttcacaccttttgaatgaatgtattgaagggcatcttccaggcgtccgccattgctcattgcatcccattcccaatcgagcaacgtataaggccagttcatctcggctgccaggtcggcaaatgcacaaacaattttatagtcctttgtgccatggttacttgaccaataattccaggaggcgattcctggtttaatccagccggtattttttatgacagacggcgcagacacatcgtccaccaaagtagaggctactatatcagcaagggtacctgtaatcatcacacgccagggcgatttccacggcaacgtgatcgtaggctgcgatgctcccagtccctgtccatcccgcggatccggtaaagtaagtttgtatgttgcttcatcagcggcattgctgagtttagtgccgcaataagtactgtttacatctgcttcatgcagcaggaaccagcaggaattatcctttaacttaaaaagtgccgggtaacaccattcctgttgctgcactttgttatcgctcatggaagtgtataaccattcattggcagtattccatttttccatccagcgggttgtttcctttggaatggtgtaagcagtcagttcatcctttacaacaaacgtcccctgcttctccggaaattcataacggaaagcaatgccatcgttatacgccctgataacaatattcaattttgctttggaaggattctcaaaagaaaccatcacttcattggcagcattggtacaaacggatttcttaccatgcaacgcattgtattgctcctggatcaaaatgggtttacctgctttgaggaatttcagttcttttgaaaaatcctgatcactgcgcgacagtcctaaatcaatatgcggaacaacttccgaaaccttcccgttgttatggtaagacgctttgatgtaccagctcccaatatcactattttgcactgaaaacagttcaacactgattttcctatccggcgattgcaccgttgtcctttgtgcaaataacgacagtgagctaagagaaaaaaggacaacggaaacaaccgcaaatttcatattcaacatttcttcgtttaaattttatttaccgccggcaacaatggcatcaatagtgcgtttatccagtactgtgttatttcgtctgtccaaagccccacctgtatcccagaaaaaaggtttaataccactggcaattgcctgtttggttacataagtcaaccaataatccacggcatcattgtgggtggccagatctttgggaacattactactgctgccacgtctgtaagcgccgtactcgcccattataacagggatttgtttgtcgacgaacttggttttcatcttgccaaaggcggtgtttacgtcaccttcctctccccaggtggaattccggtcaggttcaatggtagaatgatgtcctgccccccagtagtaaaacattttaccccaggatgcatcgccttccaataaacagaactggaacggtgtataataatgtatttccaccatcatgcgatctttcacggcgtctgtgggaagtgtgttcatcagggtattggttttatcaatatccgttgacggcccctgtaccaccaacaccctgtagctgttgcgtccaccggtggatcgaacggcattgatgaaggtttgatgatagctggtgagtatgtccatctgctccgcagtttcagcaggaggctcattagcgctggcaaacatcacgtgctcatcaaaatcacgcatggtggtcgcaatttgctcccagaatgctttttgtttggcattgacagaatccttttttgcactgttgatattggcatccagccaaccaccgtcccagtggatgttgagtaaaacatagatgtcgttattaacacaatattgaaccacctcttttacgcggttcagccaggcatcctggatcttggcagtagttttgtctgaatactgattccatgaaactggcaggcggatggcagtaaatccctgctgttttacggcctgtacataactttcattgatcaacggatttccccacgcggtttccccgccaatagcttccagggtattgccaatgttccagcccagtttaaatttagcggctaactgcacggcattacttcccatgccggttgaattagccggggcaggcgaaacattgtagcccggataaatgccgctggcttgcgttactttaaccctgcgcgtctggctggttccggcattcacctccagcaccaccgaccggggggcaccggtggtattgggtacagtagtcaaccggatagcagccttgctgctaccggtcgactgacttacctgcaaccaggaagaagcgggattattaatattccaatttacattactggcaatggttacatcggaagtgccaccatccggctgaaaagtaacttcagataaagaaaccgacaattccggcgtaaccgtgctctttttactacagtatgtaaacattaccgtggaaatcatcaatccgataagtccatacaaatttctggttttcataatcatgatatttggttaaaatttattggtactatcttattttcactaccctgatattatctaccgcagcttgtaaaccggaagcagaaggagaagcagaaaagtttttggtatgaatatttacagatcccttggccgagctgcccagcaaagtggtcagatcggcagctgcgctacctttgccttcattagtcctgaatgtggataacggaatggtgactgtatgccaaccctttgtcttaaaggggacaacagtgccatcagcgccctgccacggctcatatcgggccatatagtcgaatgagttacctcttagtacataaatagaggtgcctgaccatgcggcggggacattgatctcaaacttaacggcatattgatcaataggaacgcttaaactgtcaacagggatccactgtacgtcgttggtattgatactccgttgccagttccaccagctaccctcgccggcaggcagaacatcattatttaacactgcataactgcccctgttgccgggaaaattaacactgctgttatctgtaccggtaccccagctgaaagtatttacattatcaaaattacagagcgcgccggttgtgggatcgtttacattaaaggtggtggaagcgttaccggattttgtgttgatcactaccggcccgccttgcgaaagcgttggcagtacaaacccgatggccgtaccatcgtcggctgtactataatcggtaattggtgtaccggcaaaagtcagctcacttataaaaaataaattcagcccatagatataaacggaatcacctgtgttggcattttcgttggaaatgctggtaatagaaggtggtggcgccacaatgccgaatgtaaaagtggtggacccgtgccgggtcacatagcggatcgtattcagactttctgccggcaccgatgggaatggtatcacagctggtaccagcacggcagcactggtatctgaaaacatgatgctattgatattagcgggtacgccgttgaaagagatctgcacagcatcctgcagattatgccccaccagcaccacccattgcccggtagtgagggaattgacaagcgtatcagcaggagaagctgcataatttctaacgctggtgataacaggagctgcttcagttacatctttcttgcaagcagattgcattagtgcaaaaacagcagcaagtgcaaaaaacggtaacctccaatagcgctggttgaatattattttattcacggtataatgtttttagtggttcttaataatatgacaccggaggttccagcaatttcgggttggcggttacctcagaagaaggtattgggaatgtgaaactttgaatggtggcaggcgtaataataccatatggatctccgggtgttataacaccattcgaaatggtaaatggcgcacgcttttctccatttaatttgctgatggccttgactgggttataataagacagtctgaccaggtcgatccaatattgtccttctcctgccagttcaattcttctctcattaatgacggagtccatatctattctgggagcaggagccatcccggcccttgtacgaacctggttaaagtagagcaacgcgtcgccgtcggcacttgaggcactgttaccaagtattgattcagcgtaaatgaggtaaacatccgccagtcttaataacgcattatgctcggtggaggacgtcagcgtcatcgttggcgcactgttatccttgttggtgccgataatatgcttcttcaacccggagctacctgtatatttaaatcctccgcctgccgcattcaactcagggtaatagtcgccgttaatcataaaagtggctttacgccttacggaatcctttgtttgataaagctggtacatatcaatggtcggactaatagcaaaccagcctgctgagccattggcagatatttccacacctcccggagaatatacctgcaacatatttccttccacccaacctcctcccggcgcccactgcaatgcaaacaatgactccggattgtcgttaaactgggttttgaacaggtcggcgtaattttttaccagcgcaaggccgctcttcttacacacatttccggcgtatttctttgcactgtccaggtaagcctggttcctggtgcctccctgctgatttaacccggctaccgtcagataaaccttgcttaacatgccttgtgccgaccaggtagttacccttcctgcagcatcagcagcggggagatggctggctgcaaaagtgaggtcattgattgcgaatttatatacgtcttccgtttttacccggttgatcaacggagatacaatcagttcgctgttatcttcaataacgggtaccgcgccccacaacaccgccaggttataataggcaaatccacgtataaaacgggcctcagcaatagccgcatttttgtccttatcaggaatggaagccggcgccttttgtgtgatggcattgatcgtaacattacagtgtgcaatgacattatacatccctttccaattggaaatcatgatgccgtttaagccggtaacggtgaaagtattcaactgcacagcatctccccagtaaccaaccgccatatttccactcagcacttcgccaacaggcaaataacaattgtagttccagtcagcccagggcgtaccagcatataatgcagctgttgccaacctgagatcaccagccgattgataaaaattatccgcacttatctgcgacaggggcggacgatccaaaaaacttttggagcatcctgttatagctatcgtagctatcaggaagacaattattttatccaatattgatctcataactatttatattaacagatgaatattttatttagtcagtttaatgttcgcaccaatggtaaacacgcggggctgcggataaaaaccgccatcaacaccagcgctcagcgggtcccacgatccgatctccgggtccattcccttatagtttgtaatgataaaggcgtttgaaacattgaaataaactctcaggtatttgatgctggctttactgatcagcttttcggggaaggtatatcccagggaaatattcttacatctcaaaaaacttccgtcttctacaaacttgtcagaattcctgttattatcattggtattatcattcctgattccgacaattcttgtttcagggttagttacctgtatattattaatatcagtggcgctgcctttcgggtcaatcagggttaatttcgcatagtcgtttaacgccttgaagtaaccaaagctggtacccggaaattccccatttacgcgaagctggttaaataccttattgccaacgttggcagcaaaaaatatattcaaatccacattcttataggagaaagtattgttgaaaccaatctggtatttaggtatgggggaaccgaggtaggtttgatcagattcatttataacgccgtcaccattaaaatccttgaatttcagatcaccgtaccagatgcttccaccggcagctcctaccgacagtggcacaccatttttagtgggcaatgcgtgggtttcaaagtcttttctcgtagcaaacacacctccgtcaataacataaccgtaaaactcgccgatagatctgcccactgcagttttgctgtactgcctgttcagtgaagcgccatccgtattgagtttaagcacttcattgatattgcgggaaactgtcacatctgttttccaggtaaaatttttggttttaatactggttgaactgatcctgaaatcaaagcccttgttattaacagtacctacattgacatacggagcttccatggcgcctggcgagtaaccaatcgccgttccggaatacagcggtaaagggatctgcaaaacaagaccatcggttttgcggttataaaaatcaacggagaaattcaatctccagttaaaaagtgttccttccagcccgatgttggcatattttgttttttcccattgtacataagggtttcccacattctgggtaagctgggcgatgcccgttagcccggtagccaccgtagccagtgtggaggtataggcataatcccggatgttctggttatttgttaacccataccccaggcgcagtttcaattcattaatatctttaacagactgcagaaaattttccttattcaatttccaggcaaatgctcctgagtaggtattcacccagcggttttcaggggcaaactttgaagagccgtctgcccggagattggcagtaaacaggtacttatcgttgatgccaaaattgatacggccaaagtacgattcctgggcgctttgccctttggagccgctattagtggcggtggttggatcaccgctgctgattacctgcacattatttgaagggaaatttgttcttgctgcagaagaaccttcatttgtaccgagttgcgcttcatgacccagtaacacatttacattgtatttatctttaaacagatgtgagtaggtaaggaagttcctgatggtggtaaacaaattttgcgaaaaattataagacccgctgttggtattattttttacaagaccaaatgtataggtaggattaaaccggtcttccgtcgccatggaaaaacttcctgttgcttcattccggagggtgagatctttggtaaaagcaatttctgcatataaattaccataaagctggtttctttttgcctcgtctttattaatgagggcgatcgcatacgggttcacggtactgttcacccagccattggggttataggctccgccccagctgccatcctcattctttacggcgatgtccggcgtttggcttaatgcggtattaattacattggagctggttgaatttacattttccttgatattcaccagttgcaggctggtaccgatctttaaccaattggttgttttattatcgagattcaaccttaatgaaatcctccggaaattggatccaagcgcgataccctcctggttaaaataggaacccgacagcaggtattgtgttcttgtgtctcccccgctaatggataaggtatggttagacatcggggcatttctgaaaagctctttctgccagttggtcccttcgcccaggtattttggatttacaaattcaggccgggtgtcaaatccccatcctaaccctgtattcctctcatttataaaggttgcatattcccttaaattcattacaggtaaccttttaggtatttgctggtagcctgtatacatttcataagaaatgcttggcggagcgacctgcccccttttggtggtgattactattacgccatttgttgcctgtgaaccataaatcgctgttgcagatgcgtctttcaatacatcaatggtttcaatttcagaaggattgatacctgccaatggattcacacctgcgcccaatgtggcggtgccgccaataatgatcccatctattacatacataggcgaacctcctccaaaagaagacaagccacgtatctgtatcgatacagctccgcctggttgacctgatatttgctgaaccactagtccgggcaccttaccctgcaaagcctggtcaaaggttaccggttgtgttttacggatctcatcaccggaaacagaagatatggcgccggtaacatccggccgttttactttgccgtacccgattaccaccacatcctccagttgtgaaatattctcagccatttctacttcaagggaagcagttttagccaccacttcttttttctggtaacctatcattgaaattaccaatgtactccccggggaagcatcgatcgtaaactttcccgctccatcagtaatagtgaagtggctggtgttttttaaggtaacagtggcgcctggaatgggggaattacttttactgatgattctaccacttatttttattgtttgcgcagagaggtttagggtggaaaggaatcccaaaagaatacccaatagcggtagtattcgcaagcgaatcattttggttgaattcatttttctaattttaacgtgggtagatgatgatcctcgcagttgttttcagcgaggatgatgtttcataaggccggaacattcgtgacaggagccatgcaatcgataagtgccagttctttttcagcagctttcgttgtttccaatagtcactttctactgtaattggtgacgacctcaagttgaaaagcctgaggtgaaggactaagtaaagggattgaaaaggtagacaggtggtcaggatctgcaacgtaggcagaaggacttgccaataagtctccatacgagacatgggccggcaagttaagtggcagcaattgtagtttcatatacgtggattgaatattgtaaagctattgttatgttctctgaatcaagggggtcatttgattcaaccaggaggcccaaatgttacaattcgttgaatatcactagcaactgtcaataaaccagggaaaaccggggccactatgttgcattcatccaacatccgcattgtctccctgcccggttctcctgataattaattagaacggccctggctcattaccaacccgcgttttgtttcaatacgttatccgataaagtgatttgtgtataaggtatctgcaccagcccctttgtttcgattaccttcgatgctaaaatggttttggtggtattcacgccgccattttgaacggtcaccgattctgcaatggctgaggcagcaacattgatgccctggcgaagaagatcccagtaacggattccttctcccgcaaattcaagtcttctttcatttataatatttgccttgctaaccggaacctggacaaagctggcgcccaatgcccttttgcgcacctcatccaggtaattctgtgccccaccggcgcctaattcagccgccattaacaaaacatccgcgtagcggatagacacataatcctggtactggctgatcatgaagctcgcgccccccattttttcagcaagacttcttcctgcctcatccgccatcggggtatattttttaatgcagtagcctgtatactcccgttgatcctttatgttctgaaaattgagcccctcatccactattgaaatgatagaggcgcttctccggctgtcaccggcagggaaagcattccaaagtttcgggtttacagtggctccaccccagcccatcccatacggataaatgctctgaacgcgaataccgaataacaccatccattggttaccatccacgtttccattccaatcgctggtaaaagtgtatttgatggcaaacaccgtttccttattatcctctcctacgtaattgttaagagaggcagcgggccataaattggcaaatttatctaccaacccaaatcctccattactgataacatcctccaggtaagcaagcgcctgcgattttgaaacagttcccaccaggtcggctttattgtaataaccggtatagcaaaggaacacacggccaagcagcgattctgccgcccatttggttacccgtccacggctggagggatcctggacgccatagccgccagcaggaagattggaagctgcaaataccaggtcgtcggcaataagtttataaacgctgtcggggctggcctgaggtacattatccgtagtaggctttgtaatcaacggaatattgccccataatctgaccatatcaaaataacaataggcacgtataaaccttgtttccgcttcatacgttctgcgcaaactgtcattgcctttccaatccaccccgtcaagatgcgacagaagcatattggcgcgatagatagccttgtagtacaggttccaggtatctccaaacatattctcatcagaaggcgaacggagtttatcaaattcgtccatcatctgataaccaaatccgtcggcattaccggtgcctccaaatgcttcgtcagacatgatggcagacgcaacaggaaaagcaacgccgcttgcccacacacgctgtaatccatcatacacgcctaccaatgccttccaggcatcgttcggtgttttataaaagttctgctcggtagcagacgttacatcttctgagtccagaaagtccttgttacaggccatcaacgacaacagcgcagtaaccagcatataaaattttaagtttttcatcgccaattcgtttttaatttaaaaccggatgtttgctccaaccataaatgttctgggcctgggataatatcctaagtccactcccgatgaaaagccttcattatatccaacttcgggatccataccattatatttggtaaacaggaaagcattcagcacggaagcatataatcttactttgcccaggtaattttttttgatcaggtttgagaaatcataaccgagggtaatcgtattgatacgcagataatttcctttatgtatgtacagatcagagaactgcgcccagttggcgccatcttctgtgaccctgggaattttattggaagttcccgggccatgccagcggtccagtatttctgaggtatagttaccaaacccgcccggtcccctgtacgactgaacaatttgattacctgttacgccggaggcctgtactaagagatcaaaccctttgtaatcaagcgttatattaaacccataggtaaaatcaggattgggatcgccgatatttgttttgtcgttggcgtcaataacaccatcgttgtttaaatcaacataccggacatcgccaggcttggcggtgggctgaatgggattacccgttttgcctttatacgccgttacctcatcgtccgattggaacacgcctgcggttttaagtccccagaaatagcctaccggttcaccgtttgccgcccggtaaaattcacctgcattggcatacagcacattggtattaccatgaagcacatgatcgtttgtaggaatattccctatcctgtttttattataggcgccgtttacgcccactgaataatggaaatttttgccgatgttgtttcgataattaagcgccagttcaacgccggtatttttcacatcaccgccattgatcagcggcgcatctgcgccggcagtagccagaataggcacggtaatcaaccagtcttttgtttttttgacataataatcaaaggttatatccagccgttgtaacacagtagcatcaaacccgatgtttgtttgctccgacgtttcccattttacatccggattggcaatacggcttggataagctccctgtgtactggctccttccaccggtccgaatatataacccgcattactgaagctgacaggagacacaaactgatatgccgctacattctggttacctacctgtccccagctgccacggagcttaaggaaattcaaccactgcacaccctccataaactcctccatagaagtcacccatccggcggacacggaagggaaatatccccagcgatgatccggcgcgaatttagaggaaccatcagccctgaaggtgaggttcagcaggtatttctcacggaaattatattgcaatcgtccgaagtaagacatcaacgcattctcagacgggccaccgccaagactcatatatggcgcacccttgttcacattctgcgcaacagaaaggtaggcatgctgcagatcggcaacacgcaggtcccagttggaaccattcataccaacagtttgtgttttcagcgaagagctacctgccattacaccaaaatggtgatcagcagcaacatcaaaatcgtagctgagtaaattgtcgaactgaatggtacgcccactacccattgactggctcaccttcgaagtatcattaaaggaataaatagaaagatgataaacgggtgtataaccatgactttgattcgcgtaatagtttaaacccaggctggaacggaattttaagcctttaatgggttccgcctgtatgtacacatcgccaaataaaccctggttactgttgcggttccgcgtggtatagtccatcactgcataaggattggcctctgtattgttccacgcctgatcaggttttcccgggtaccagccttttttatcgctgctgaaataactaccgtccgtgtcatacgtgggcaggaaagggcttgtagtgaaagcagcacgtaatgtattattatactggccgtctatcgcaattccatgattgttttgataattgaacgtaagatgttctcccagcttaacaatattctggtacaggttatgttcggagtttattctgaacgtgtagcggtcaaggtaagaaatgtccgatcctcctataatgccgccctggctggtgtatcccagtgacagggaataggtggaattgggactgcctccctgtacgcccaatacatagttttgagtcggcacattctttttgaacatctggtccagccaatctgtgcttaccggcaaattgttaactacctcgttgctgaaatacggcgctttaccggagttgacagcagcttcgtttatgatggtggcataatcttttgcattcaacagtttagccttgcgggcaagctgctgggcgccataaaaaacatccagggtaacctgcggtttctggttgacttttcccgttcttgtggtaaccaggataacaccgttggccgcctgtgaaccataaatagcagcagaggcagcatctttcagaatgtcgatagaggctatgtctgcggggttcaggtatgaaatgtcgctggtttgaacaccgtcaacaatatataaaggagaaaagttaccaacagtacccttaccacgaataatcacattcattcctgcgcctggctgtcctgaataggaagtgatttgtacacccggcgcctggccttgcaaagcctgcatggcattggtagtgttctgtttctggatgtccgcgccttttacctggatgttggctcctgtaacgagttttttcttctgggtaccataaccgattactactacattttccaattggctttcagcttccagcaattgaactttcaattcgcgtgaggtaacttttacctccttttcaacaaatccaacggatgtaattactatcacatcccccgttgatgcctcaatagtaaaccgtcctgcatcatcggcaacggtggatacacgggtgctttttacggtaactgatgctgcaggaaccggagcggacgtactttgactggtgatcgttccactcacctttgacgtttgggcaaaggcgttctggctaagggttaaggccccaagcatgccccacagcagcaatattcgcaagtaaatgattttgaatgaattcataattgtggatttaactgactactttttatatctatttttcttccatcgtaaaccacttccttgtcgcatttggcatcaggatccaggcgcctgggttctccgggcgaaatgatattaatgcgaagggctcttttctgtaacatgcctttgaacgatcctttccgctctccgacagtaacagttcctgttgcctgggtatattttattggaatgatggaaaatgcaccttcttcataattgtaattggtgccctcatcttcatacaggttgaaagatgcgtccgcaccagtgtaaatgttcaacgtaacagtgtcggcctgtttctccgctgcatattgtaactccggcccaaaaggcaggatagatccggcttttacaaataaaggcatccgttcataaggcgcttcagcagtaattttctgaccacctgcataccacttcccggaatagagatcataccatcctgcgcactcgggtaaatacaaggcacgttttgtttgccggtattcatacacggggtttaccagcagtgaagggccaaacatatattgatcagcaatgttcagcacggcggtatcttttgcaaagtccattgcaagtccgcgcatgatggtatagtcatcatggtacgtccaccctgccagcgcatagatatatggcagtaaacggtaacgcagtttatcgtaataaaggaaacttttataagcggggtgatcttcaggagctgtgttgaatacttcccggtaaggagattgcccatgggagcggaataaaggaacaaatgcgccaaactgcgaccaccgggtcatcagctctctccactcttccaggctctctgcatccgggctctcaaatttccttggcaccacaaagccacctatatccatcgtccagtaaggaagcccggacatagagaaattactccctgcagctatttgcgctttcatatcattccaggtggaaccgatatcaccactccatatcgccgccgcataatgctgcgaacctgcaaagccggatcgtgtcagcaaaaagacccttttatccggatccgttgagcgttgtccttcataaattccttttgcattctgcagcggatatgcattcaggaactctgccgcgctacccaaagcagtgggtgtcatttgcagctttcttttttccgggtttacgttggaaactatatccggttcgctggcgtccatccaccaggcgtcaattcctttactataaattttttcgttgatcagattccagaatcctttcctggcggcgttattgaaagcatcgtaaaaagtagaaacgtatcctttgcctatccaatctttttgctgatcggctatgtttcttttataaagccatccgtttttatcaaagttgttataggccggtataccgtcataaaattttggccatacagatatcataatctgcgtattgaattttttatgcaacaaatcaatcatgctgtcgggagaagggaaacgtttttcgtcaaactcctggctgccccattccgcttctctccaataattccagtccagcacaatgttgtcgataggaatttttcttttacggaattcatcaacagtattcactatctcctcctgtgttttgtatctctccctgctttgccagaaacctaacgcccactttggcacaataggtgccttacctgtaagcgtacgatagccggaaattacctcgtccatattattgccatacacgaaatagtaatccacctgtttgccggcttcggaacaaaaaccaaagctgttttgctgatcacggctcaatggctcctgccattttaaagaaaggtaggactcgcccccctccggtagccattcaattttcaccggtactttttctccttttttgaaatcccatggaatcaatgcagatgcggggttccaggcctttcgccaacgatccagcaccaattttccattcagccatacttttaccgaaccgccataagtgaagcggaactgatgtaaccccgacaggtgactggaaaggcttccctcccaggtcaccataccggaagctggggtaaattcccggggtagtagaatttttgaatctcccaaaaactccatatcaatatttccctctgctctttcaatatttatctcctgaggtttatgcatgttattggaataggaggcggtaagccagccggtttcacctttctttgaaaaaagttgcatggaagaaagcgggtgaagcggcctgatatcgccggccctggtgagggaataattatcccagagaatgccatagtttttattggagatcataaaaggaatggccacttcggtattgttctggaagaaggtaacctgttggccccggtaattcattataccgtcctggtgttgtccgagtccataccatgcgtccccgtcggccgtctggaatgtttgcgtaatggcgtaataacgtttaccgtcgaatatggcggattgaaaatccctgccaaacggctgtttttctgacaggatttttttacctgccagatccgtgaaagtaacggcgccggttttccggtctaccgtgacgattaatttttttgttttgagagtcaggttttctttagaaggaatgaaatcccaggtgagccctggttttttatgataaacagtaaccaggctggtaccggccactatttctttcccgggagctgccatcaccctgataatatcgtccgacactacttcaagtttaacagcatacgttgaacccgttagcagggaatccgtaaaaacgatcaccccatcaggaagagtaatataggcaggtggcgccgcaaataagttatttagtaacgcagaagccagcaggctaaacagcagtaatcgcaatttcatatacgtggattagatgctgtaaaactattgctatgctgtcagaaaccggggcgtcaaatgattcaacaagggggcacaaatgttacaaatgactgaatatcactggtatatttttgacaggcggtgcgttaaagacttttgtttttaagatttgccacgtattcggaaggggtagttttgaactcctccttaaataacttacggaatactttcggattattgaacccgacttgataggcaacttcagaaatggacatcccgcttttgtccagcaattgaacggctcttttcaaacggatggaacggataaaatccaacggcgacttacccgttaacgaatgtatctttctatataaagtaaccctgctcatatacatctctttactgaactcatccacagaaaactccgggttgtctatttgcttttcaataatttccaatgcctgttgaaggaatttttcatctacgggcgttatggtcacttctccggggttgacttcaatctgcttctgaaacctcttttgcaataatctctgctgcgccagcagattattgatgcgggaagccaggatctcaaaggtgaagggtttggtaatgtaatcgtttgcgcctgctttcaaaccttccagttgtttttcctcgcttcccatggcagtaagtaaaataataggaatatgagcagtgagtgtttcgtttttaattttcctggcaagttcaacgccgtccattaaaggcatcatgatatcgcttaccaccagatcggggtttaacaactttattttctcccagccttcctttccatttgtggcttcttcaacatgatattgccctttcaggttatcctttaagtaaaagcgcaggtcctcattgtcttccactatcattatcgtcttcttcttatcaccttttttattttcctccgccattatttgctccgtttcgcctgaaaatgcgggattagccagggtccggggagaagaaacataaatttttcttgcggggagcaataccgtaaaacaggtaccctgatccggttcgctttttacggtgacgataccattgtgcaattttacaaactcttttgtaatggccaggccgatgccggttccctggtttaccatactttccggaacatccgtctgaaaaaagcgttcaaatatcttttcgtgctgatcggccggaataccaataccggagtcttttacctcgatagcaagtgtgccatcggactcattatccgccggctccttatagatcaggccaacgctcaccgttccgctgtcataagtatatttaaaagcgttcgacaacaagttgaataaaatcttttcaattttatctttgtcaaaataaatttcgaggctatccgtgtcagatgagaaagagaattggatcttctttttctctgcaatatctgtaaaagaataactggtttccctgcaaaaccggacaatatcgcctatggaaggatgcaactttacttcctgcacctccatcttcctgaaatcgagcagctggtttaccaggtttaataagcgtttggcattacgctgtaccagccccaattgttttacctgctcttcatctgccgtatttttaatgatcttatccaatggtgcaatgatcaggcttaacggcgtgcggaactcgtgacttacattggtaaagaattttgtctttaactgctccagcgcatgcgctctctccgcttccctgcgctgttgctgcacttcaaaacgcatccgtatccggtctaatgtaatgcgccggataagcaggaacaacgctgcagcgatcaacagatatataatgtaggcaacaggcgttctccaaaacgggggttcaatattgatctgcaacgtttttacctcactccataggccggacctgttcaaaacttttaccttgaaaacatagtgaccgggatttagatttgtataagtggctctccgctggttaccatctgcatataaccagtcttcattaaacccttccagcatatatgcatatttgtcatatgcgttatgagaaaaatcaagcgcagcaaagtcaatggagaaaacattttccctatacttcagatcaatatgctgaagctgggataaagaacgtttgagcagcacccggttattgaccagctcgccgggttcaacatctttatttaatatctgaaaaccggtgaaaacaattttaggatgataaacgggtttaccaatagcagcaggattgataatattaaagcccgaagggccgccaaagatcaattcgccggtcttcgtttttagcgctgcattatcattgaattcgcggttctgcaggttgttggtggcatcataggtaaccacagaaataaccatatccttattttcctggtgcggagtaacgttacataacccgttaggtgtggatatccaaagcgcgtggtgattatcttccaggatattcaggatcatattatcaggaagtccgttggacatggtgaatgtatgaaactcctttttttgttcatcaaacaaattcaatccctccctcgttcctacccaaatccggcctttactgtcttccagaagacagataatcccattatcacttaaaccattttttttatttgttaccaggtaaaaaacactggtagttttattcttttccataacagcaataccgtaagctgtaccaacccataaattcccctttctatcatgcataatagcagaaacataatcggaaagtaaaactccccgcctggcgttataatggctaaactggcttgttcttctgtcgaaacgatccaggccgccacccaaagtgccgatccataagttctgatccctgtcttcaaatatctcccaaaccttgtcatctgccagacttgaggaatcattatcatgatgcctgaaccgggtgaacttcttcccatcaaaacgattgaggccacccaggtaagtcccaatccagagaacatcttcatgatcgatccataggctcacaatgacgttgttgctcaggctgttttcattttttggatcgtataagtattgtttgaaagtattattcttcctgtcaaaataaatcaggccaccgccattggtaccaatccagatgttacctgccttgtcttcaacaaaacggtttacatcgtcgaattgcggactgttttcatttagttcctggtgatggtaatatggaaactgaatgatgttactattataataatttatgccctgcttataagttcccagccatataatcccctggtcatctttatacaaggtggtgatactgttctgactgatgctcttgggatcattggggttgttcagcagataactggttttgaacccgttctttttgtcgatcagcgttactcctccgtgatcggttcctatccagatcaaaccattgctatcctgtacaacctggcttaccagttccgcattcaatctcgccggataagaattcttatcaaactgtttgatagtattatcttccgggtgaaaaagaaaaattccgaagttgtaactccaaagccagatgtcattatcatgatctataaaaagatgataggggttattagctttattcttcttcagtaaagcattggtagaaaaaattattttatccagctttatatcatattcctgcaaaaaacctgattggtataccaaccataacttcccatccgatgtttcacttacggaagtaattttcccggaagccggcggtgctttctgattaaatggttttacaattttatcgtttgctgaatacaggaacaaacccttatcatcatacaggaaccagtacctgttattgttccccttcactatattggtaacaccaccagatggcaaaccgatggaatgcaaatagtcatcagcgttgtcattaaacttctcggtatcggggttataaatacagggcccactcacggtcgacaaccacattttcctgcccggaagctcataaagtgacacaatattattgtcccttattgaagagctgtcattgtgatccttatgaaatatcctgcagaaatatccgtcataacgattaagtccatatgcagtggcaaaccataaaaaaccatcccggtcttttagcactgcatttacctggttatgcgacagacctgtgtatgtattgagcttcgaaaaattataatgctcactttgcgataaaacaacaagggactgcagtagcaaaataaccccaaaaaggtaacgcattactgtaggttttagataaaaaagtttacgcctcccaggcattcatacactagcggctgttgccgctttccctgccatcccgctgatcattaaagatgcccgataacgtttttacttttgcaaaaagcaaaaggtacttcattcctgtgagacagacccgatttggcaaaaaacggcaataaccacggtagtgattattgccgttttttttccaggatcatgacttactttcttaacaggcgtatttcatacacaggccctgcaattgatcctttgtccgccaggaatttaatccgcatagatccatcctctgcatagttaatatccgtaggcaattcgtaatcgatggtataaaatgtatcgctctgcccttcccggagatcgaccttagccagctgccggtcgttgacccatatggagaacttatgattaaattctttcccgaaataagtaacacgtattttcttacccgtcttgttcttatctgttaatttataactgaaccactctctcgctgaccgccaatgcctgttaaagctaacaccggcaaaggaactctcgtgtaagatggcgtgatccgattcgggttgctgttccccggccgcgatcacatcgatcgtattggcggcgaggcttgcttccagcgaatcttctttagccagttttgattgtaaagccgcaaaaccgctgctggattcttttcgccagtatacgatatagcgggcatcctgtattttatagaacggcaccagcttcaaatccttatactttgcaggataaattatttttccagccgtaaaagacatgggcgcatgcttgtcctcctcaatcatagctgcgtcatttgtggcatcgcttacaaaaacaggcatatcggtcattttgtagagttcaccgccggcaatgtgccccatccggctgtcgtcggcctcgcgtgatttctggaaaagcgtatcaattacagcagccagcaggataggcccgtgcaaaacagcctcataggcagatccgtcaggaagcgcttctgtgctggtttgcataggcgtctccactgtaataacatctcccttcttccatttccgttttaaatttatataagaggaaggcttaccgttgacggctacggatgcaccattgatctttaccttcagtgcgccttcttttacccacgaaggatacctgatgttcaggtcaaaactgttcttattaacacccactattttcagcgtggtaatgccctgttcaggaaacgcagtttcctgcctgaacagcagtcccttatctttccacttgagttcagatggaataaacaggttaacaaagagctggttatcagaatgggtgtaaatcatctttccatatttggcgtgattttccaacccgctgccaacgcagcaccacatactcgtttccggctgagagtaaacccggtaatgaccaggacgcatgggcgtaaaataaacaaagcctcccttcccgggacgctgggtagttagaatatggttgtacaaagctttttcgtagtaatcaatataagccacgtccggatctgataaatataaatcctctgtaagcttgagcatattgtaggtattgcaactttccggtccctctacgctggacatcatggtggagaaatcattagagggattaaaatgctccctgacgctattccctcctgttgctatagtgcggtgatgcacgaccgtttgccagaaaaactccgcggcatggttataagcggtgtctccactataatcggcgatccgcttaaacccgattattttgggtatttgcgtattggcatgtaagttatccagcttatcctggtccctttccaggggttgcaaaatagcctggtgcgaaaagctgtaagcggcgtccaggtattttttattgcccgtaatgccgtatacatccgccagcacttcattgacaccgccatgttcatttccaagcagctcctgcatctgcaccctgctgagtttggcagtcatttcacaaaaccagtctgcaaaccggaccagcatctcaccggcggttttattgcctgcataccagtaagcatcccggaggcccgcaaaaactttatgtatattgtagaaaggcacccatttccgcttataatccgcgaaatttccttccagtacttcttcccaaagttttctactgcccggaacgccgcccaggtaaccattggcgtttttgtcctggcaaagtttcaactcacctatcatataatccaggcggccggacattcttttatcacccgtggaggcatacatcatggctaacgcagaaagataatgcccgcagatatgaccatccagcccggagctttcccagtttccataacttccggatttttcaggaagaccagcttccctgcgaaacggcgccagcagcttgtccgggtttaaggcaaggatataattaatgtcagtctgctcctgctctttgaaaataccggggagcagccggacatcatttaaagaaaaaaattccagcgctttatggctttgcgcatgtatggacaatggaattatgaaaatcaataacaatatacgtttcataaaaaaacacttaaaatttcccgtggacagaattttaataagtgtcaaaataacaataataattgttaaaaccaatgcctgttttatattaagaggaaattaaatctgtaatcactccagttctataatagctttaatgaccccattagccggatccagtaaaccttcaaattcatttgtaatgttttcaaaagctatacgatgcgtgatgtaattggcaggctgcacccatccttttttaatagaggcgatgacatgttcaaagtcttcccgcgtagcattacggctgctcattaatgtggcttcccgcttgtggaattccgggtgactgaaactgatctcgcctttttgcaaaccaacaagcacatatctgccgccatgcgctatatattgaaagctgttattgatcgccttcaaactgcccgtggcatctattactactgcaggcatatcgccgttcgttatagcagccagttgctccgatacatctccggtggatacgtttataacatgctcaacgttcagcttttctttgcaaaattccagtctttttgcattcatatccatggcaattaccttcccgcccgcaatgcgggcaaactccatgatccccaatccaatagggccggcgccaataaccaatacaaactcacctcgctttacctctgcccgcctgatactatgtgccccgatagccagcggctccaccaatgccaggtcgtcgtagctcagtccttccccatgtattaacgaatagacaggcacattcaggtattccgccattcctccatctatatgaacgccacaaacattaattttaacacagcaattcggttttcctgacctgcaggcaacgcaaaccccacagttaaaataggggataaacgttacgatctccccatttgcaaaccctgctgctccattggcttctactaattctcccgaaagctcatgtcctaaaacacgcggataattaaaataaggttgtgttccttcgaacgcatgcaaatccgtaccgcaaacgccaattctgcggatcctgatctgggcgtagccttccccgggcagcgaccggctttcttctttaagcgttaatttcccgggctcatcacaaactattattcgcatatcagtattttaaagttgaaatatctgttccatcatcacccatttctcttctccctttgcccagggcaaaggctgctgaaacttccacattaactgctcccattcctgcactttgggattggcagcatctgaagcattttttgctgtctcattatagagatcattggtttccatgatcatcatcaggcggttacctgttctgtaaatctgcatgtccacgatccctgcatcaagaatgctttttcttacttccggccaaccatttccggccctgtgccaataatcatattctgctatcagctccggatcatcctttaaatcaagggctaaacaatatcttttcatagtgctaattaactttacaaatagctggcagcataggactggtcaatcagtccacacttttccatttctttccagaacccttccgggatgatggagtggggcaatgcaacattctgtgctaccctttctgcctgtgttgtattcaaagcgatactccttacgccgggtgcattcatgccaaaaactgcgcaggcggctaccggttttattttataatcctggcacaactggtaaaactgctgtcgccagtgatataaatttttgtctttttccgggtctgttaactgataattataataagcagatcctgttagaaaacctccgttaaaaacagaagaatttatgactgtgatgccctgttgctcaagttccagcataaaatccaccaacgccgcgggatgactgtgaatagtcatgctattcgcaatcattacccagtcgagctttacatccttaactatccgggctattacccgccagtcttttgcccccacgccgatagccctcaccctgcccgcggcttttaattcatgtaaagcacggtaagcatccaatatatcctggtagcgttgcttttgctcctgctcatcctttgatgcggcgaggtattcatcgggatcatgtacagataccagctgcgcgttatagttaccgagcagtttatttccctgctcatagcattccaggataccatcgtagcttatatgctgaatggcatcatgttccaggtttttccatatccccggttcaaaagtgggttcggctgtttttaattccgtgcgcaaccaacccagtttgttgctgatcagcacatccgaaggactgatcttcaattgttccaggctgcggcccagcgcctccagtgccaggccggcgccatatttaccggccgaatcaaatacaaccggctttggagagtgtttgatgctctccttaacgatagataacttcacttcatccggtagcgccacatataaatttcctaacccgctggtaccaaaaataactttgggcaatatgagttcctgcatataaaagccacttattttcaaagaatagttgaaacagataattgctcctgcttcatttttaccagatgacctttaaatccgaaataagccaccacagcaaaacaggccaatggcactgcgtaaccatattggatattaccggttacatcgcttatataaccgaatatcctcggtaacacggcgcctccaacaatagacataatgattaaactacttccgaattcagtatcgccgcgtaattcctttatgcccagcgcaaaaatggtagggaacataatggacataaaaaagcaaatgccaataaccgcataaacagtgatgataccggttccccagatggcgatcaaacaaagcagcatactgataactgcatacaccgccaataaccttgcggaactgtagtattgcattaaataagtaccgataaatcttccaattaaaaatgccagtccgcataaccctaaataatcagcggcctttacctccgatataccagccgcctttggtgcgtacagaataaacaaactaaacacacatacctgggcgcctacataaaaaaattgcgcaacaacgctccaggttaaatgacggtgtttaaacgcgtgaaaaatattcttactggccacatgaccttcatttgtttgaatagccggcaaacgggtaaaggcaaaaatcacggcgattaataccagtacacttccgagaataaaataaggcatttttacggtggccgcctcggcggcaagggccagcttccggccttcttccgtcatggcacttaactgcgccgctgtgtagcctttggttagtatcacacgcgcaccaatcacgggcgcgagtgtagtagccaggccattaaatgactgtgcgagattaagccgttgggtagaggtggcaggatctccgagtgaggaagcataaggattcgccgccgtttccaggatagttaatccgcaggcgattataaacagcgctatgagaaaaaacgcatactgctgcgtattggcggccggaataaataaaaatgagcccaatgcaaacaccagcagaccggtgataatgcccgctttatagccatattttttcatgataaaaccggctggcagcgccatcaggaaataagcgatgaacacagcagaatcaacgagcgtagcctgaacggttgtcagcgtaaatgatttctgcaaatgcgggataagtatcggatccaggttatgtgcaaagccccataaaaaaaacaggcttgtaatcaatataaacgggaaaagagtatgggactttgccatatgaacgtcttaaattttacaggtaactggttgggtgaaaaaacatctatacaatcgctccttcaatttttaacacaaatgcctctttgcacggcggttgttccggcaactgcaccttcaacccttcggatgtttgttcaaaactcagtcggtcatttcccaacaggcttacctggcttacttttccaacctgaccattcgctaatgttttaaccaatgcagttttatctgccggccatcccagcatcaccgcataaagcgttttgcctttcgccgtaaagcgaatatctcccggtccaaatggtttgccctttccttcgttaaagccctgtgcgctcaaagctaccacggattccatggcaggcccttcgccaaatactttccagggacgggtgctgtaaatggcttcgctgttgaccttcatccattctgccacctgttccactacagcctgttcttcactatcgatgctgccgtcactacgtacaggcacgttcagcaataggttcccattcttacttaccacatcggcaagcgtatgtatcaccgttttggcgcttttatatcccttgttatcatacaaacggcgatcgtagtgccacccgccaatacaggtatccgtttgccagggcaggggctctatctggttactttgtccacgctcaatatcccagatcatgcatttgcgttgctgttcgtctaacattttaccgaacaacgcagcctgcaattttccgtgttttttgatactggtgttataaagatgtgctgctactcttaatccggcatcactcactggccaaagcggcagcgcattatcatcaaaataaacgagttcaggaccatacttatcgatgaggtcaatagtcctgtttacaaaattatcgcagtacgtcttgtcaggcacacttgctccattcccccaataccagcggtcgcccatactgccatcattcaggctgtccttactcaacgcatgattttgggcatatagttcctgcggatcataaccattccaccatttattgctgccatcggctttagtcagtttgccatcataaggcacacctgcataaggaccggatttgtcggaacgctgcgccacctcataccaggtccacgcgtgagaggcatgaaccgttacgccaaagggcagcccctgttctttcgctgcttttgcccagcctccgataagatcttttttgggtcccagtttagtggaattccacttgtgatatttgctgtcgtacagatcaaaattatcgtggtgattggccatggccataaaatatttggcgccggcttttttgtataaggcaaccaattctcccgggttccagttctccgccttccagtcgtttatgacatccttaaaaccaaattttgaagggtgtccatatttctgcagatgaaatttatactgatcgccaccttcctggtacataccacgggcgtaccaatcgccgcgttccggctgacattgcggcccccagtgagcccagatcccaaactttgcatccctgaaccaatccggtacctggtatttccccagtgaatcccaggtaggttgaaatggaccgggcgccatacgtggaatagactgagatgttaacaaccggtgagcataaagattagatagatataaagatgacaaacctgtagccaggccctttatcagcgttcttcttttcatggaatttattttttattagctcaacacaagcctttaatggcgaatgatattgataaatcaaacttactccgaaatacttatcaaacatttggcttaataggacttttctttatacaaaaccgactatttgcttattattgcggtggtgaaaccgaaatattgggaaaaacaggataccggaaaagtgaaagcagctttccccgacaggccattcaacaattaattgcacggtatgattaaaagagcactaaaacatacattcacgttattgaacgttgatcacgtaaagctcgactccaggtggaattacaaaaatgtgatcagcccgtatttcaggctatattatatcgacggcggagaaggggaaatctgggatgtttctgcgaagatcaaacttgagcccggttttctgtacatcataccaagcttcacattatgtaaccttgtttgcccccaccatctcagccagtatttcgtccagttttttgaggaatcatcggatggcatttctttgtttgagaataacaggtccattcttaaagtaaaagcaactgaaatcgatatactgaattttgcgcgtttgctggaaataaaccccggcaggggcattaatcgctctgataatccaagggtgtatgaaaaaaatattttctacaaagaataccaggaattgaataaccggcaaagcatgtccacattcgcggaaacacacggtattctgctccagctagtttcacgctttctgacacaggaaatacttacacacaaagacggcggtcatgtgccggttaaaattctaaacgccatcagttatattcaattaaacctgaaccgcgatttatcggtcacctcgctggcaaaaagagcgaacctgcatacagattatttttcacgtctttttcatcaacacaccggagaaaggccggtaaggtacatccatgaaaaaagaattgaaagggcacagtacctgattgtaaccacacaaatgacctttgctgacattgctacgcaaacaggttttgagaacgtattttatttctctaaaatttttaaaaaaattacgggaatgtctccggggaattacaaaaaacaaatggatatgattggtttttagatattggagagtaaggcaatattcatcttctaacggcaactatatctttcggataaaaatccatgtccctgaaactgctatcatcaatattatacaatatagccacagcagccgtttcaaaactccagtatccttcaaaacctccttcacctttggctttgtgtgcatcatagttaataaagtccttcttaccctgataccagctgctcaaatattctttgattagagctacctgttctccgcccctgacctgcgtagctttgtaaagcagctcaaaagactttggataaataagttggtcagttgcgactctgtctgttagcttagttattaacagagcttcaatcaaagcatcctctccgttgctgtgaagatgattagctatttgctgaaacagcccaacaggcgcatcaaagataatgccccagctaataagggtaagcaccctgtagtaatcatgtgtcaataataaatgctttttcttatcccctgtactgatattccggttgtaggctacccatgcttctattagttgggggtaatcagctttgatatcctctattagacttccgccagagtattttaaagtgataagtcttttacaatcataatagagattttgggtgatgctatttttcttccattttcccgggaaaggtgtcacgttcagcttgccctgccgttcatgaacagcttcaatacaatcgtccatccatttttgccaataggcgctatctcttaacggttctctatgcatattttcattaactagcttagtttttccacctggtcatgtaactgctgatcccagataaactccatattgaatttaccatcggactccaatctaaaaatagctttgttccatttgttgttttcaccttcggtggtaatactgcggagttcaagaatatcaaatgtcaactggaaatcaaattcgtcgacatctatttgcttttcctcatgggaagtatttatgtaagtcccggtattactaaccattccatccagtacttccaggtttaatacggcgctttgccagtcttcttttattacgctggaaatattctttgccatggccaaataaatctcatctaccgtcataatccgttttttttgataattacatttaaaccgtcaaacagttcttgtaatttaaacattaaaaggattagtacaaacaataatcacggaataaaagaccttaaaaaacacaccttaccacgctaaataattttataccgcaaatttggaaagctgctgccagatgaaattgtaagaaaatgaaaacaagatttaaccgtcgataataaaaattgaaaaatctggtttaattaccctattttatgtatgtgctgcaccggcactttgttaacaggaacaggcaggctaccgatgccggggataccgtgagcgtgacagatcgcaaccaataaacccttgatattctgatttttattctatgacccaaattctatccacgatgacccacaaattgaacccttatttaacccgcagagcgttgctcttttctttattgatgctgatgacaacgacttccatggctcagataacctggcctgcgggtcagctgctgccttcgtttccggcaacggcaagcagcctggatttattttataataacggcacctctcaacggtcctggcgttgggaaggtgaaggcccgtctctcagccatcatacggggcgtttagaaagcgatggctggctttgccaggtaggaatcgatgcggcgaatgagcatatgatttacggtccttacgacaacagcgttacggcaggagcgaatattgccgagttcaggatgaaaacggataataatacagctaataacgactctatcgtcgatatcgatgtgagggatgctaccaccggtgcgatccttgcgtttaaggctattacccgtcagcaattccctgtagcatccaattacacaagttttaaattgcccttcaccatgccggccgatagccacgctattgaattgcgtgtattctggagaggaggcgcttatataaaagtggactgggtaggtgtacagcaagataatgctaccgcagaaacctatttattcacttccctgaaaggtatcgtcaaccgcacgcagccgcggctcttttcctatgaaggcgatgcctttgcagaagggccatacacctggatgcagtcattgggtttaacctggacagaatataccgaccggtgggcgcttatcaccaggtaccgtacggagatatccggcctgatcgtgtatgatccggcgcagacggccaccgttaacctggccactatgctggcaaaaaataaaaaggcgctcatcgcctccccatccttattatcacggttaacggctgccccttataatttccccgtattgatggatttacgtggccagtttaccagtaacctgcaggtataccaaacgttgtataacacttactggcccacactggatcaccggctgttaatcgggttaagcccggaagtgcatcagggttccctgcgggaatatgccactgccctgggcgccgcagtaatatggctggacccgcgggtggcaggtgaaagtgaattgctgaacaatttcttagcctccatgccggcgggggcaaatttcatgggctggtggcctgaagaaggctccggtgtaacaagagcatctacctatggaatagccaccattgccagcgattatgctactaatttaacggtgcatagcggtatgcccagaaccgttaatgttaaacctataccgccaaaaccaatcctgaaaaacaaaatttatgtggcgtttatattaagtgacggcgacaatcttcaatatgttgaacacctgatgcgcaagctctggaacaatcctgaccgtggctcggttcccatcgggtggacgctttctccggcgatgctggatgccatgccgggagcgctaaacttctatcatcaaactgctacggataatgataatcttatttccggtccgtccgggtacggttatgtataccccaataatttcccggatcaaaatacactcaatcaatttgttgctaaaaccgaagattataataaaagagcagggttccgggtggtcactatctggaacaccattaccggtggcattaaccaaaatgttggagagagctttgccacctacgcgccatcattacttgggttaacagcgcagaatacaggcggccccctcagcatctacaatcaaacactgcccgggttgcccctttcgtgcaattactgcaccggggaacaagccatgaaggatgctattgccgctgcctctgcagggtggaatggaacatcaccgaggttcatgattatacaggcgcaaccctggcaggatgtgaagcctacgaactttaagaacgtaatgaattcacttgattcaaaccatatcgtggtgcggccggatcatcttttccaattgctccgcgaaaaaaatggtcttccggatgttgattccaccgatagcctggtagcaggcatgaatcatgtgcgcatcaatatgatgaacaccgccaaaactgcaaaacagcacatttccctgtatcccaacccggtgggcaacaggctttatatcagggggctgaacaacaacgctaaccttgaggtgtacgacaacgacggtcagcgaatgaaaacggcattaggtatgtcaattaacatcgccgaactaatacccggcacgtattacttaaaggttacatccacagaaataaatcatacctataaatttattaaacattaattccggcccggccaggtttgaaggagcccgctcaatgagcgggcttttctttaaagcaaatcgttaacttagatattactactgacaggaaataagcatgacagacgacaagcaaaacatatacgacgtaatcattatcggcggcggacaaagcgctttatccgtagcctattatcttcgcagaaccacgctgaaatatatcctcctggatgccgcccctcttccgggaggcagctggcagtatacctggaaatcacttgcgttattttccccggcgcaatggagctcacttccgggcgtttttatgccgggaggccagcatcattatcccagccgcgcagaaaccatcaggtatttgcaggagtatgagttgaggtataaattcccggtagtgaggccggtaaaggttacatctgtagagaaagaggaaggaacttttattttaaccaccactgccggtccatatcacgcaaaagcaattgtgagcgccacgggcagttatgccaacccgtttattcctgctattcccggagccggctcttttaaaggtactatacttcattcggcgcaataccaggaaccgggaagcttttcaggaaaacgggtggccattgcaggcgaaggcaactccggcgcacaaatcctggcggaggtttccaaagtagcatctaccctgtggatcacaaagcaaccgcccgaatttttaccggataatattgatggcaaatatctttttgatgcggccactcaacaatatgaagcccggcagcaaggcagggattaccagcctccatcactgggacatattgtaatggtgcctgctgtaaaagaagcaagggaaagaggcgtgtacgaacattttcttcccgcatttgatcatttctatcccgatggaatagcgtggaacacaggccaacaggaacccgtagatgccgttattttttgtaccgggttccggccggcgttagcgcacctggcccctttgggaatcattcaaccggatgaacggattaaaacaaacggaacaaaagcaacagatattaccggtctttggctaaccggctatggatcatggaccggctttgcttctgccacgcttattggtgtaggcagaaccgccaggcaaaccgtggaagaactgagcagcttcctgcagtaataaacatccttctactctcccttaaacgacaatcctttttctttcagcgcattccgcaacttcggcagggaactttttcccatgccatgaagcgccagtatatcggcttcgctgaatttagaaagctgctgtacggttcttattcctttactctccaacgcgcggcgggcgggggcagccagcgaagcaaaaagctccccgggagcgctggtatgcctgctggtatttttctcctggctttctttcaccctgaactttactattttattgatcagggaaataggaagaggttgatccaatggaaactgcacggcgcctttggaattcttataaacggaaagttctttttcaaatgctttaataccagaaggagcaggataaaaaccgatgtgatgtttatatcctgcgaaatggaccaggttgccgtttaacgcaaaagttggaataccataacttatcttctcttctgcggcaggcgccattttcctgatagccgcccttatttgctgcaacagcgcctgggtttcctccggaaaaccggcgatatactgatcaatgtcgtttactgttttcatatcgctgaattctttcttaaaattagcataatccgggtgtttgcacaaggcattaacgcgacattatacaggggcatttgcgacttcaattttgcggagtgcagcagattttgtctttcccaggattacgctgattatattgattaaccggattttgttctttgggatttttttgatttggggagattgaagcggatgctggttgtagaacttcaatattttacccccggataaaagaaacacaatccaaaagaaacaccgatttttgatgaaattattcgtcatgaaggccatcgttattactcaaccagggggaccggaggtattgcagttacaggaatatgccacaccctcgccggggcaggaagaagtattgattgaggtgcgtgctgccggactaaaccgggccgacctgtcgcaacgcgaaggcaaatacccggcgcctcccggcgtgccaccggatattcccggcctggaagtggccggcacggtggtgagttgtggtacgggcgttaccatgtggtcgcccggcgacaaagtatgcgcactgctggcaggcggcggatatgctgcctatgtgactgtaaaggaagggcaatgcctgccggttccggaaggtatcagctttgccgaagctgccagtttacctgaaactgttttcaccgtgtggagcaatgtttttcaacgcgctaaattaatgccgggagaaacgttgctggttcatggaggttccagcggtattggtattaccgccatacaactggcacatgcattaaacagcaaagtatgggtaaccgtaggtacagaagagaaaggacaagcctgcatcaggctgggggctacgcaatatatcaattataaaaaacaggattttgaggaggaactggccacaacgggcatagatgttatactggatatggtgggaggaaaatatctcggtaaaaatcttactatccttaacccggaaggacggctggtgtacatcaactctatgggaggcaacctggcggaagtaaatatctccacggtcatgcagaaacgtattaccatcaccggtagtacactccggagcagggaatacagttataaaaaagcattggcggctgatatccgccagcatgtgtggccattgatagcagctaaaaaattcctgccggtgatatacgctacgttcccttttaaggaggctgcggaagcgcaccggctaatggccagcagtgaacataccggtaaaatagtgctggtaaatgaataaaaacaaaaggtgtactatgagcagtacaccttttgtttttattcattttagtaagatatcaaaagcggtaaccgatcgtcatcctgaagttacgacgggcctctactatataattataaaacccggtagcagtagtaggtatagaagcagcagtgagcaaccgctggttatcgagcaggttattcaccagtaatgaaacactgtactttcctttaacgtagctcaaaccggcatctgtacggaagtaattgggaatagagaacacttttgtggcgcttcctacgtagcgatcagccatccactgaatgccgcctgtaacaccgaggccattcaaaactcctttgccaatacggtagttcagccaggcattggtaatatgcgtagccgtattaggcgtgatattacctactgttttcgttgtggctgtaggtgattccttggagatctttgaatcggtgtaagcatagttcagcgtggcattcaatccaggtagtatttccccggcaatgtcaatttccacacctttggtgagtgtttcaccaagttgttcctgtacatcggcaccgcgactgtctttcatattcaggcttacgagcgagttttgcctggcaatacggtataccgtagcggatgctacccatctgccttcaaaccattccttcttcacaccagcttctacatccactcccttaataggtttaaatgcgttctggttggaatcagccccaggcaccggtacaaacgactgatcaaacaaaccgtaaatggtggtggatttatctacagaatagctcaggccaacgcggggagtaaacacattatccttaatagcaagcgccttggttttgccaaccgtttctgcgtaggtgaaacgcccggctaacgataaacgtaacctgttgttaaaaaagcccagttcatcctgtatgtaagcggaggtatagtttactgaactcacatagttactgccacctgctcttgtttttacactctggctgcggtctatagcaggcagggtaccgataggaatgctgtatacggggttatatacattgaattttttatcccccaccatatcgatattggccaatgttctgaaatctccccaaaactttttattccccatatctacgcccgccagtatcctgtgccgcaccgtacctgtatactcttcgccggaaatggaagcctgtgcaaaacggttctcacccgcttcatctgccacactgaaagttctgcccatattccctgcactatctactttggaagcccatatactgtttgcctccataccgaagttgaaataagctacctgcgcatgcgcttcccacttatcattcaccttatgatcaaaatacaggtatacgctgtgatccttcagtttacccggcgtgagggatggatctccgtaaaagaaatcattcgagatatcttcatccaacaattttttgccggagaaaacatagttaccattcgccaggtaagttgatccctggtaggtatattccagcgtaacagaagtacgatcgtctaccaggtattttaataccggcgcaaacaggtaacggttgttaaagttgtatttggtataataatccttttgctgaccggccacattgaggcggtacagcagtttaccatccttgctcagtttaccgtcaaagtcgagcgcggcgcggtaagtactgaaacttcccatgctgatgctggctgcacctttggtaatcccggtcggttttttggtaaccacgttataaaagccacccggctcaccacctgccagcataaagcctgccggtccttttacaaactcaacacggtcaatcatagcggcatcttctgctgtgggtccccagctggcttctatattcataccattacggaaagcggggatcttggaaccgcgcatcctgatattcgcatactgattatcccaatggcctacacgtgtggccccgcttacattacgggtgataccatctaccaggtcaaatgcctgctgatcggcaattacattggcagatattacctggatattctgtggcacttcgaggataggcgttctcagtcgcagtgatccggaaagactatcattcttataccggttccttgcaccgctcacaattacttctttcaattgtttatcggaagcttcgagctgcagtttcatctgcacaatctggtcctgttctactattacttcctgcgacattgttttgtacccgatcagcatcacctgcaaggtgtactttccgggcgccagttttttgaatacaaattcgcccttttcattggtgagtgtgcccctgtttttttctttgatctgtacagctacataagcggcaggcgttccgtcggaggtaactaccaggccgcggatagcggataagggctccgtatcagccattgcattcacggaaaagcaaacagtacatagaaagcataagtacaccgttatccggttgataaataaaaacatataggtcggttatttcggtttaaaattcaggcgcaaaattaatggcgatactccgggcgaggttatggattcgggaaaaaggtttacgcaatacggaaaaaacgttttagcgcaagccacataaagtaacaggaagcagttataaatacccgctatatctccctgaacaggtataaatacctgttttcaaaaacactcatttacgctcttattcaggccggcagatcaatggacatttgtggagaagaatgtgcagctgcagcacagaaaaaaacaggtctgcctagcttgacaataagcggggggtgaaaccgaaaaaccataacagagtaggaccaaaaaatacacttatgaatcttggattaacaatgcgctggggatatagcgcgcttcaattcaatgggacctcgtatgcttatttcccatccaaccaccttaacaacatgaggtcgtttacgcttgaagcaacgatcttttcaacggcatcaacagggaccattctttgcagtgcatcgccgactgccggcgcttatttcaacttcggcctttccaacggttttttgtatttggagaccatgaataataccggaaagccgtttcaggtaacggctacaaaaaagctacccctgctggaatggcatcaggtggcagctacttttgacagcgacaggaaattgatcacgctgtgcctggatggaatagaagtaggcagtagccccatacagggaattccttaccaggccataccacttcagactcatattggcgccggaaaataccaatccccatccggataccagaatttattctatgggcatatagcacgtatagccatctggaaatcggcccgggacatttttgagatcgcggaagatgcatttgcgattgttccccccgcggcaacgggaactgatctcgttttatggacagacttcaccgaaatgcccactgaagaccgttccggtaatggcattgagatctcctacagtacgcctccacccaactatgtttacagtatcccttcggcaggggtaacagaaaatggttatattgattgcggtgtatatccggagtataatttcggcggctatcagccttatactattgagggctggtttaatcccacctccacagcggatatggccgtattagtcgcctttgaaaaagacctgcattggcaatactatattcagtatgataaagtcaacagccgcctcattgcaaaacggaattcagatggacaagccatctactccaaggaacagatcacggaaggacgtttctatcattttgccgtttcctataacggagattcaaaaatgatgagcctctacgtaaacgggaacctgcaaacagccgaatactttcccggtggtgtagcgaatgttgcccagggaagactgataataggcggaatcggctttaccggttacattcaaaacgtccgtttatggaaagattgcctggagcaggcagaactccgtcaatggatactgaatgatgtgattaccgatccaagactggtagccaacttcgatttcactaccactccaccgatggattcaatgggtcataccgttcaactactgaacggtgctgccagcgcgctggcaacaacaacccttgaactggcagacagaaaagcccagctgggtgtttctatgcctatcaattccagctactttaatagcgtggaagaagcacctcttcctcctccaaaagtcataaaacctgctgatcagcgggaactatcctccgccgttctgaaggagaaaacgtttacagacctggttagtttctggaaggtggatggagaaaaacaacatgctttccgggaagaatttgaaaaagcatatgcacgggcagaagaaatgctctcagagaatgaaaatctccggaaagtttatacaagaacagatgaaaatggaagaacaaagatcatataccatgaccttcgtggcgacgcacttatttatgaccgtccaataggagaagtaactgactgcactatctggtggatcgtttttgtctacagcatctctgttaaatttttgggcatattcctcccgcttccggttttctctccctacaaccagattcccggtaaaattttcaatctcgctatcgcgaatgcaaaggtgttggcaaaaattactgctgtagtcggcactacgatcaccgttatgtccgggctggatattataacagaaatgcatcgtgaaaagattttatggcccattttaaaattcattgtagtctcggcgggttggtttgccctgactgctatccttgcgagagcttttacaatggctaccggcctggtagcagcagaaataatggcgaagtttattgtatgggctgcacagttgacgaagctgtcactggaatatgacgggaactgcgctgagcaaggacagggttaaaacaaaaggctgtatcaatagtcatttgatacagcctctttaatatagtaactctgcttcctcagtataatacccggaagctgatggtgtctttaatcttcttcagttctttcaatatttttttatcgtattcgctgctggtatcggtgatcacgtaaccgatagcggcattcgtcatcaggaattgcgacacaatattaatgcggtgatctgccagcacctggtttacctttgccatcacgcccggcacattgcggtgaacgtggataaagcgatgcgcattatttacttcaggcaattgtatattcgggaagttgctgcttttaaaggagtcgccattgttgataaacctggcaattctttttgccacagattccggcttgcgcatattatcaaagatcacgatccccatttctgtacaaagctcctgcgggatatgttttttactattacccaggtaaccgatcactttcaatttggtcgcctttttcagctgttctgcgctgagcttttctccttctcccattaacagtatacctgctgccgacagctgtttatcgtctgttccggcatgtttaatggtgaagccgtccttcttcaggtattttacggctgcttccggcacatcgcctgctacctggcaaagaatgcggttcttggggtaggagatggccgagggcaggttgttcacatacaggaactcatcaagactcggcgtgatatgatccgctttttcggtgacggacttgcgctctatattctctgtaaaggcataaaacttcttgatcatgccggactctttcagctgaaaatcggaataaccatcgccaataccgtgaatttcgccctggagctgcagttcatgcagcaattttactttgccgccttcgttggagagcgggtttgcggcatcatagccaactattttcccttcgtcgttaaacaaaaaggtattggcataaatattttcttttttgatatggaaaggcagtactaccggtgtaataaactctttgaatccgccggaaacgatcagcacatcctctgcatgatgtttaaaaaagtttttgttacgggagaaagaagtggataccagttttttcaaatgcttcaccaacagtttcagatggtctttattcgcctccagcagctgcacccgggcggcaaggctttccctgaaagaaagcttcccttccatggcgaggttggtcagatcttcaatttttttatagatctgttctctttccggatggtcctgcagggatatgcgcgccagttcatccaatgcttccacctgcgtgaaagtgctgtcaaagtcaattatatagtattttttgcccacggaacgatcaaatttggagcacaaaaatataagtttaaataagatttagcagacaatcttgtaattccggggaatttatgggggttaaagcctggactataaagcgtcccattcggtttcattttcctcttccggcgctttcttctccaccggtaaggtggccgttctcctttctcctatctgctggcgccacatggcatagtacaatcccttatgctccaccagctcgtcatgcgtgccggtttcagcgatctttcctttttccagtacaatgatccggtcggcgtgcataatggtcgacaaccggtgtgcaatgagcacggtgatctgttccctgcgggcggaaatacttctcaccgtatcagtaatcgcctcctctgtaatagaatccagtgcggaagtagcctcatcaaagatcagcaggcgggggtgacggatcaaggcacgcgcaatggaaatacgctgcttttccccgccggataattttacgccgccctctcccagcctggtgtaaatgcctttaccggaacgggccagcagggcggtacaggaggccttctccaatgcttcaattacttcttcatcggtggcgtcggattttacaaacagcaggttctctttaatagtgccggcaaacagctgtgtgtcctgcgttacaaagcctatttgccttctcagcgcattataccggatatcgccggaaggcacatcattgaaatatatttctcctgctaccggtttatacaaccctaccagcaatttcaccagggtggatttgccggaaccggagggtcctacaaatgcaatggtatcaccggtttccacggcaaatgaaatatggtcgatcgcattggtggtagccgttttatgcctgaacaccacatcctcaaaacgcatttgctgcaaatcgccgatttccaccggctcttccggacgctcttccaccgggcgttgcatgagtttatgaaacaactgcagcgacgcttctgcttcccggtactggataataatattccccaggtcctgcaacggaacaaaaatagccgtggtaataaactgcatggtgatcagctcacccgtggtgagtatattcctgaagatcagccacaacaggataaagaggatgctctgttttaagatattaagcgtagtgccttgtaaaaaagacagcgttctcacctgccgtgtcttttccatttccaggtcgaagatctctttggtaaaggttttcaaccgtcttatttccgggaaggttaaccccaggctttttaccagttctatattccgcaatgattctgtaatggcgccggaaagctgcagcgtttcgcggttgatcgcccgctgtacggttttcatttttttgctgagcaaaccggtaagcccacccaggaaaataatcccgatcacaaatacaggtatcagcgcccagtgtttggtaatggcataccagatcaggaatcccatacctaccagggaagtaaagaggatgttaataaaagcagtaataaaacgttctgtatctgttcttaccttttgcagtacggcaagtgtttccccgctccgctgttcctcatattcctcaaacgatagccggagggtttgtttgagcccgtcgttgaatacctgcatcccgaatttctgcactaccaggcgaagaaaatattcctggaaagattttgcgagccgtgccatcaaagccaccactacggcaacgcccagccagaacaataccccgtgcaccagatccttctccggcatactgtttaccttaccggcataatcgtcgatgatcttaccgaaaatcaacggatccgtcatcaccagcacctggctgatgccggccagtaataaagataaaatgaccagccatttgtgtggcttcaaatagttccagaggaccttcatattttaaaaatacgataaacgggtaacatatatcttcccggtaccaaaatgaaaagaggccggatcatgtgctgatccggcctctcttttccattacggattaattttttgccctgatggcctttacttccgcagcggtaaccgcactggctttgttgccgaaattatttctcacataagtcagcacatccgctatttcctggtctttcagaaaattatgcggcggcatattattggaataatactcgtcatctatcggaacagacgactgcatgccctttaatatcacctgcactaatgcgggtttatctcccagcacaaaagtggttttaatcagcggcggatttaaatgtggtacgccactgccatctacctggtggcaggtaagacaatattgctcatatacttttttaccgcgggccatcgcaggattggcgcccggctttttggtctgcgcagataaaaaagaaagcatggcaccaaatgcaacacctgttaaaatgatcctcttcataccatatcattatttaccactgtaggtaattttataaaccgttccttttacatcatctgttacatacagggaaccatcgggaccctgtgccagtccgcaggggcggtgctttgcctggcctggcgactggatatccggtacgcccgcaaaatcatctgcaaaaatttcccatttaccggatggtttaccatctttaaacggcacaaatgctacgaaataacccttctgtcctttctgacggttccaggaaccatgaaaagccacaaaagcgccattcttatatttggccggaaactggctgccggtataaaacaacaagccattaggcgccatgtgggcaggaaatgccactacagggtcaatggcgttttcaccaccggttttctttccgtcgccgccatattcgggcgccagcattttcttttgctgttgtccgtcgtagtaaatatagggccagccggcatcatctcctttctttaaggcatacatacattccgctggtaattcattaccctgttgcagcgtgtaatattccgggtacatgtcaaacaacccgtctctcccgtgttgcattacaaataactggttatccgctgtattccagtcgagccccaccacattacgcagcccggtggcatagcgggtaccatcgccataggtctggttttgtttatctgcccggaattgccagatgcctgctgccgaatcgcggatagggcatccttctatgcctttggaaccttttgcgcggtcctgttcctggcaggagttggaatacgcgccgatgttcacataaatgtttccttcgttatccagcgttaaagcttttgcttcatgctggtgtcggttaatcaatcctgttacgatcttttccggctgttcagggttgatcacttcaaatttatcattcagtgcataacggaatacttcctcatcggaggaggtatacaggtagtttcctttgattaccatgccggtaccgcggtaagtgccaaaggtttttacgtccttgccgtgtatcactgcaatggcttttcccggttttgaagtctggatttttacatagacatcccccagtggtgttaccgctatgtggcgggctgcgcccaggttttccgctattgcctgcgccttgaatcctgcgggcagtttcaaccctgcattgccgggatctgccactgtacggcgaacagcgctgctgtcgccgttattggccaggcattgaacggacaacagcgtcatcacagacaaacatcccaggagaactactcttgttttcatatttcttttatttacaatgattgatgaggggatatttaaacttaccgtgtaaaaatagtaatggtttttatggaattcctaatttatggatgaatggcatcagctcctggctaccagggaaatgtaatacttcatcaggtaatgataaatcaccagctcatgcaaacgggcgttggctgtaaacatgcggttcaggaacatgtgcaggtaatgcggcaccagttccgttactgccgccggctgtatgacccggagttccaggattatatccttccacctggccgcccgttccgccaatatttcgcgggcgccatccggtaacgtgtaatcgtttacgttatccgacagcacatccgtaatttgcctgctatgcgcacggtatttattattcagttgccgcagcaatgaagcatctccgtgatgctccgcaaagtactgctgttgtaaatgctgcaacagcttcattttcatcaacggcgtatagccgaaaccgtttaacaactcatctgctccttttaacgccagcagccagcgctcctggctttcagcgccgctgatggtcagtaacagtcttaccgccgcctcgctgtcgtggaaaaagaaagcctcgctatgttccatcagcgctggtccgtaccgctccagctcccgcacataagtatccagctgtatcttctgtacaatatcactgttaagataagggagcagtagtgcctctacttcctgcatcacggcggcactgtgttcccggtgctggggcaaatgaaagcggatacggatatgatgatccgggtcctggtaccggacaaagaaccagcgatccgttacccctgaggattgcagtctgacggtgaggggcagcaatactttcagcaacagtttatccatccatttgggcccacagtatatttttatatacatccattcgctgcccggggcaaagctgcgcggcacccctgccggcgcctgcgtggcgggcaattcagccgatggctcccacgcggcgttacgcagcggtattataatttcattgcagaaagcaccctgtccgttcgccgacaaacgggtagcctcgttaaataaacattcatataatactacatttcctttcttcagtttatctattaacagcattcgaccaaaagcacttgagaaatctattaacaggtcgttgtctccttcggataacagtacatgttccggcagccggcactgcgcttttaacagcagcaacgcctcatcttcggaatggacttccatgagtgattcaaacgcggcacgggtcaggtaccacctggccggcgccaggattacctcatggtataccaccctgggcagaaagggttcttcctgtaaaattccccagttccactgtaccgatagtgcgttctgctgttgcaggtcgcacaggaatttgtaggccgataagccgcggctgtagttatgggcgctggtgagccggggcatcacctcttttccccaccgttgcgaacgcagcactaccctgttgttacgcacgcttaccagcagatcgctcacgggcaactgatagttttccggcaggctgctttttcccaggaacggtatttcataatcgtacagggatggccgtagtaacacgttgccggaacggccttccggtaaatgaataacttctgccagtattttatctttctccagtaactgctcgcggcgtgtaaaatcacgtaagaggctttccagttccctgtttccggcagcaaaccggcccagcagggccagggcattggggccatggcatgctttcagcaaaaatttgaagtcgccgttatccatagcagcggccgaagcagctgccagcgaacccatgacgcaaaaaaatggtggtatttcctgtttatcggtatccgcggccagttcgtccaggtcagcatccgtgagggaaatggccatggctccggtggctccggcagcaagaaagcgtttcagcacaaacttcgtttgggcgttccagtgaatggtatcgttctttttaccggccggcattaccaggtcatctatgaggggggtatagctcgcgtcttcaccggataccaccccgtaccctattccggattcgctgtcgagggccatcatcaggggtatttcgcgctgatcatatttttgaaggaactgttctttaaaatgctgaaggtcgccgccatcaccggaggcgccaaataccagcagccgctccagccgttgcagcaaggtactggtaacggatgcagccaggcggacttccggcgacggaaaaaaaagatccacctgtaccggctctttcgcgtcgatgcccgggaaatttgaggctaatatatttttaacctcctggtagctgtttataccaatggcaggttgctgtaaaatctgccgcacttgttgcaatgcaggcaggcagtccggtgccggatgtaacgccagcaattcacggatcagtccctccaggttatcagtaccggcaatttccggagataatccggctaccaggatctggttccggatcaatgtttcgataaagccccgggcctcgtcggccgggatatccaggttggtgagtacgccggtgagccgggaaatgctggcccccctggcggctgccgcgaggatggcttccatatattcattttgcgggaaggcactgaggaaataatgccgcttcttatcccgcagctggtactcgaaataccggaaggcatcgccggaatgatataaactgctgttggaaaaataaagcagttgcgggccgatttcaggccgttgggccagttcgctcatcaagccggacaggtatcccatgtccagccgtgctactgcctggcgctgtgctataacaggggctggtaagcgggtaggcccggtacggatgtaaccggtgctgcaaccggcaaataagccgtaaggggtgcagcgtgtgctcattctcagcaggtaacggtaaagcgccagcggcagtttcagggaggtatccgccgatggcagccacttcagcatttctgcgtaaagcgttggactggccaggaaaacggcttcctgcaataacggttgggaatatattttccggagggcagatacaaaagagggctggtcattgcgggtgttacgatgcagttgtaacacttcctcatatgacaatagtggcattctcgataaaaagaaatcgcaggcgttcaacacggacatacgcgacaatggcatacttactttagtgggaaagctatgctttccggttctgtatgcttgaataaagataaaatgtttttaggatctcaggtaacagctattttgatacctggaataacccgttccatttcatctacaaacttcttgtaactggcaggtttacccaggtaaccttgcctttcttcctggcaaagatgctggacctcacggctggaataagcggtaacaagaataaaaacgcagtcctttttaaggaactttgctatgatatctcttgtattgcctctcaggttaacatccaaaaaaacgacgtctacttttctttcagcgatcaggctttccacggtgtccaactctgatgctttttttacgagttttagataggatgttctttggatatagctttccagtatatctaatgccagaggctcgtcatctactatggcacatctgtattgcatttcttaccaaaggggttaatcaattaggaataataaacaaatttaaagttctagcgtaaaaaacctgtccctgtcaaagtagtgggagtagtaggaacactcgaaagtattgatgttactccttcataactggacgcccttatgttctctattgtccttacatcagcttttgaaacaatttctttttctaaaattaacacagggcggcgattcacagacaatttgtttttcaacataaaacatgcatttaagatgatctcttaaacaaatcacaggccgaatctcgcccaatgcttataaatatcatattttattagacataattgcctttttcttcgaccaacagccctcattgttgataactattcgtcgtcttcatcattatagttggcaatgccaagcaagcgcttgaggtcctgccgcgacgctttggagataattacagactggccgttaacaacttccacggtattacccatgatggatttaatcgcctgtaatcttacaatgtaggatttatggatacgcataaactgatcgggcggcaaaatatcttctatagctttcatccgcatataggtaatgatatttttttccctgcatacaattttaatatagtctttcatcccttccacataataaatatcatcgaagaggatcttcgtcaacttgttattatcttttacaaacaggtgattggctggctgaactttcgacttagtagtttccatagctgccggttgccaacgctgactgatatgcgcacgcgctttatttaccgctttgaggaacctgtcaaatgaaataggctttaccaggtaatccactgcatccagctcaaaacccgcaatagcgtgatctcttgaggcggtagtaaaaataacaacaggtggattactcagggaacggatcatttcgatgccattaatattgggcatctggatatcggaaaacagcaggtccacaggctgccgttgcaattcattaattgcgtcaaaggcattttcgcaaaaggctacaggttgcagataaggcacccttccaatgtaattttccatcagatccctcgcaaacggctcatcgtccactacaaggcaggtaattacttgatccatattttctagttcaactttagtgtcaagacaactttgtaatattcgggattattttcaataaataaaatgtgttgatcaggatataacagaataagtcttttgcgggtgttcgttaacccaattcccccggatacctttttgccttccgggagttcccctttgctgttcgaaatttcaaatctcagctggttatccgatacatccatcgacgcatgaatccagcatttatctgctgtagtgctatgtgaatatttaaaagcattttctacaaaaggaaacattagtaacggcgctatctggtagctacccatcttttccgtatcgcaatcgaaatgtatactggcattttttccataacgcacactttccagttctacataatttttcaggaactccgcctccaggtgcagcggtaccatttctgtattcgaatcatagagcgtataccgcatcatctccgacaggtgcatgatcaggtccgatgccagcgcgtcatttctgatagacaatgaatagatgttattcagtgtattaaacaggaaatgcgggttcagctgggaacgtagaaaatcaacctccaggttcaggttatcccgctccagccttaacgtacgggtggtggtgcggataatgtccaggaccagtttcaacgacatgggcggcgctatggtcatcaatacaggaaagaagatcttcagcaaatggttaggtgaaaaagtatctttccatccgctgccaaccacccgccccaggaattccttcaccggaacatccgtgatctccagaaatgtaactacatacaaagagcataggtaattaataacagaccagaacaggaaaggtattattaaacatacaatcgtaagaaaaaaataccccttcagtaaaaccttcggtatcgtaaaataaaaaacagaataaaaaaagaacatggcgcccaacatgttccggataacaaatacaaggctggcgctggcggaaacagcaaaagtaccactcactaataaggcataaaacattgccatgcatccccacatgagcacatgcgcccatattcttactctccttcgataatacttatcagacaaaaaaaatgaaatccattccatgaatttccggctgatgtcaggcggctctccattggttttacttctgaaaaaagctagcattgtatccctgaatataaaaaatttacagtaagcagcagcaagtaaaataaaaatactttaccaatcttaattttcttttatcatataaatataaaatgatatacaaatagcctttttagtctataacttacacattatgaatgccttccgacagcagctaaagtacacgatgttggatacaaccgcattttcatcgcgtttataggtcaatacgtctaataagtttaacaggctgctatttaatgctgacttttgatatgcaagcctgaatatgttcgctggcttaagctctttgccgttaaaaattctacagaaacaaggatgaaacgtgcataaactgcacaaaagatactttcatccattgttgttaccattgtcacttaaatagattgacatttaatttattaataatattacaccaatctggtcagaaaacctagcgaattttgtcctttgtgaactccaaaaaaagattttagctgagggtatgaacatctacctgctaatactattctattctatggaaacactatgatttcccccttacagctctaaaagagataggcatcagtctatctctttttattatacagccactgcacccaccgccacaaaatcagcaaacacatcatcagcaggatcaggtagcctaccggcttcccgttatacactccctggcacaaccgggctaccccggcaaccagtaaggccatcaccatgcctcttgcaaaagggaaaaaaccggcatatttccggaacaataacgtgaggtaaccaatggtaataaacaggccatagaaaaccaggaatgttttccctttaatagcaaagggattccactgcgaggtaacgtggtaaacatacaggaagggtaacgagaaggcacagaggaccaggatggaaaaaaaaaggggccgtggagttgtttcgtttttcatgttatcatttttaaagatcaggaaccgcaaccaccacatccacctccgcaactgctgccacagctacttccacagctgctgccactactacagttgctgccgccggcatcattttcactcccggcttccttcttctttttgtcgcttttcgcaataagaagacccataaacagcagtaccattgtaaatccaaagaaagggccgctgtcggccgaacaaccggtaaagaagaagaaagaaatgaagagaaggggtgttataaagcgacggggaaacaagctaatacgctttatcagggagaaggaaagagagggggatttatttgaccagatggcttccggcggatcttctccaaagcattgccggtataactgcagcgtatcttcctgccaggcggcgtgtttttgctgttctgccttccccccgccggaagggtgatggtggatctttttacccagcgttttctcacaaaatgcctcccagtaattctgcgtgtaaagtaaatgctggtgccatactttatctacaatttcagaaggggaagcgcccgttggagaaatacagcagagataaataaagcgcttgtactcctgtatagcctgctgtgtaaagtcttcactccagcgctgttcccgggccagcttctttgaaaaggggaacttgatatccggttcatccaaatggaagttactgatctgctcccagagcaatttacccggtgacaaggctacaaattcattgtttttcatcatcataatttcattttttatttgttaataccaagatgaaattatttcagaatactaaagtcttgtgcgtatcttacatcgacctattttcgtattataatcgtcttattatgagtaaggaagaactgcttaacctggaacgattgatgaattatattgcttatcagtatctgaaaaaggtaagctgggaagatgtttcaaaaacagaatggagccacgtggtgcatgagttcaataccgttattgagaagcaacagcgcttcaggaaattagccacgcccccttcccttttcggcgacaattatttctatgaacacctggtgatccggaaactgaaagcagccaaaaacagtgcgggtattgcagcgctgagcagtcctaatttctccaagctgaatgtaatggccgtagcactgggctttaccagctacattgatttcatcaacaattcggcagaagtatacccttttcatgaactgaagatcggtatccccctgtcggaagtgaatcataaactactggatcacctggtaggttactggtattgctataaccggaaccttccgtttaagtcgggtaagaaagcggcggaacgcatctggaggtcttccctggagatctataagtcgggcgatgaatacctggtggagcgcaccggcagggacaatcatatgtattacggcaaaataacctcttatgccaactacatttttattatcatgaacagtactacgtttatccgtcaacgtcatttcataggccggctgaaagatatggaagacaatatcaaaagatccgggtatgccatcaacgaattaaactttgtaagcacctgtgtgagctttaatgaagaacctatagcgctgtatgagatctttcaccgggtggctaaagtgaaggacttccagcgaacgtctgtagacctggccttcgacagccccttgctgccaaagcatatcctggtacacctgaaagacagtgagcagaacaggatcatgcagcattagataactagctgttgaaagataaccgcacccaggggctttccggcgttatcaacaggtattccatattattatgcaggatttcgaagctgcccatttccacgccattccacacgcaacgtgcaaactggtaggaaacggagagatgtttccaggaggtataggtccttttaagcaggggcacacaagcctggatatattcctgcgcctccccgaagctgatgtaaccggccgcatagcccgaccggctcaggttaataatgcggccaaaatcccagatcagcatatccggctggaggctttcagttaccagtttcctttccctgaacagttccagcgctttacgggtgttgcggaaccgctccattaccaccgcctcttccagctcgttggttgcaatatgttcccttagaaaagctttactctcttttatggatacggcattgatcgcctgccagatgatgtcgtattctatccggtgaccgctttcctggagccaggccagcgtttcctgtagttcaccggcattgctgatatcccaccactccgacaaatgttcgcgggctgcctgttcattggcgcctgtagtcagatcgttcaggtattggcagtttacaaaggcgatatcagcgccgcaggctattgcccattgctgcggggtatccagctggctgtggggattcagtaatatggccagcggatgttcatctccatcagttacatctgcatcgtcaccggaaaataattggttaaactgtttgacgttatccttcaacagggcaggccagtcgcttaccgggctggtagtttgccgtaactgctgcttatacagggcaatttcttcttcgctgagtcccatattgcgcagttgctgctccatatagtgctgctgattcatcaggattggttaagggttcggttaaaatgagctaatacctggtatttacgcataaaaccaggttaaagtttttctttaggtataccgcacaaagatagagaatgttctgatacgagcgcatgataaagcaaaagcaatatcaataatagttaggggagcgatttaaaaggggattgccggcgcctggagggaaagtcaaatacacgtatacccgttaccggtagtgcttttgacgctgtagcacaaataaaaagggatgttgcggtacaacatccccatcactatgacgatcttctaatattaaaaagttctgtcgcgtttatccagttttcctctcctgttttgcggtttgggtcttcttggaagcgcttttggcatatccgggttggcgctgttggcttccatcagtgctgcttcttcaaacggatgcgacacggaaggaatggtttgccggataagtttattgatgctgtggaggaatggtctttcttctgtatcacaaaaagaaagggcaaaacctgccgcacccgctctaccggttctgcctatacgatgtacgtaagtttcagaaacatttggcagatcgtagttgataacgtgttccagtgagtcaacatcgatacctcttgcagcaatatccgtagctaccagcacacgcaggcggccatttttaaagttgttcagggtattctgacgggaagcctgtgatttatcaccatgcagggcatctgcatcgatgttacgtttcttcaggttttttgcgatcctgtccgcgccatgcttggtttgggtaaacacgatggtgcgttcgatacggtggtctttcaggatagtttccagcaaggattgtttatctttcttctttacaaaataaacggattgttcaatcctttctgcggtggaagataccggtgtaatggtaactttctccggtttgtaaagtaaggagttagccagttgcgcgatgcttggcggcatggtagccgaaaagaagagcgtttggcgctgctgtggcagttcccggatcacctttttaatatcgttgataaagcccatgtccagcatgcggtcggcttcatccaacacaaatatttccaggtggttcaggtaaatgtaaccctggttcatcaggtcgagtaaacgacccggtgtggcaatcaatatatctgttccattacgcagggcaatggtttgcctgtgctgcggaacaccaccaaagatcacatcgtgtttcagaccggtgtgtttgccataggcggcaaaactttcatcgatctgcaccgccagttccctggtgggcgtgaggatcagtgtacggatatgtttaaaaccttgtttttccggcgtactgttatgtaataactgtaagatggggatagcaaacgcagccgtcttaccggtgcctgtttgcgcgcagcctaagaggtctttaccttccaatacaatgggaatagattgtaattgtataggagtaggtgtagtgtacccttcagttttcactgcttttaaaatgggctcaataagccctaattgctcaaataacatgttgatatatctgatgtaataaatataaaataacgcttcttcatctttagcgttatcacaattgaggagagcagtaaagaaaagatttccggactggagagaatagatatttctgtgctttatgcttttaactcaacagacggaagcaaagatactgattttctggtgaagatgttgataaattaaaaaaaagccatatgaaaggggtattttaagtgtcaaaacagtccataattgccgttatgagggtttaaataaaaaaagccgctttccggcggctttttagaaatttactttgccgcttccggtgcagcatcaggtttggtttttggctcttcattcccgtggtgacaggtgtagcaggaaaccgccattacctcgctgcccttaaagaacttcttgttgatgcgtttggtcatcttcatcatatccctggcaacgcccttatgcggattagcgtcgctggcgaaatccagcttcttggcatcatctttccgcggctcatgacagaaattacattttacgcccaacgcagcattaaagccacgcattactttgatcaggtcgtcgtgactgatatcttttggcaatactttcagattggtagccttctccggctcctggggcagtgcgagtgaacatagggtgccggcagccataaatgccgccaccactacaaagcttttcctgattttcattgatcttgggtttaaataagtctttaaatgcttcctttaggaaggaatctacaaaaaagaacaataggttgtaggtgggtggggccgcttttttccgcggatggagcggagggtgagcggaggttatcggagcggaggttgtcttgagcactgattacgctgattttactgatttctcttttgtgatttttttttgatttggggagattggggtttgggttggagaaggttgttttgatgattagcagatgcttcgcatctgcttaatagatgcctggtacatgcttagtatatgcttaatgtatgctgatgacctggaggtgatgtggaggtgatgtggaggtgacgtggacttgaagctaagatcttttaccacagggccttacaggcgaaaaagtacagggtggttatacacatcagtgccatataagtaaaacggcgtgctgatacatgagggaaatgaatgccgtattcaactattgtaaaaccatcctaaattgactgaattttccggaaattctataaaaagacaaaaataattcaattttcagtaaccaatgaaggctattaaataaaaatctatcattgctcccatctttcaaaatcacagaaaaatcataaaaaaaatcacaaaagagaaatcagtaaaatcagcgtaatcagtgcccaagacaacctccgctcaagacaaccttcgctcgcaaaacaaccccgcacccagatggatgcgggggctttttataattatgaggacttagttattgtcaacacaaagcttgttgtagatcagttcgtctgaagagatcggccagatgtactgtgcaacggttggcgcaattaccggaacggtgctgcttttggcagggaatggaatacccaggcgggtaatttccatactcctgaagccttctcccagcagttcaatatgtttttccttggtgatggcggccagtaatgctgttacgttggcaaaatcagcaacggtataggtaatggtggcgtcagaccggtgtcttacggcagacaataatgctaccgctgtcggatccactgaattggtttgccgcgcccttgcttctgccaggttcagtaacacttctgcatacctgatcaccggaatataatctgtgaaggggcttggcgtagggaatttagtccagaaattcttcccgagggattgtacaataaacctcctgcgcgcatcggtagctggcttccaggaagaatcagcgatcacgccattaggatgcatggagtactctccgttgccggtgaatggctttgcagcaggtgtaaaatagtatcccagctgggtttgtgtgcccgggaaatcatccgtagacccggtaaatggcaatgaaaatatagattcctttgtagaatagggcggtgcaaataccttctgtacatccgcttccagcgcatgccctgcaggcgatacaaacggtgcactggcagacaccagttttgccgcttctgtaattactctatcatattgctccatatacaggtatacacgggttttataagcgatcgcactataggcgttggcgcgcgtaatggaggttaaggcgcctgctgccggtttggtcagtaacgcttctgcagaatcgagatcgcggataatctgcgcataggtttcattcaccgtactgcgggcgcgcgcataactgccaattttagcatgtccttcggtgtgaataattaaccctggcctgctgccggcgccatcccaatgcggacgtgcatataactgcagcaaggagaaatagcttacgccccgcacaaacttggcttccccggcgtacagctttgcgatagagtcacctacgatctggtttccaaccgcattcataccggtaaggaaaacattgacgttgttaatggtaatgtaaccctgcgaccagatctctttaacctcctgcgcttcgcctgtaggcaccattcgccaggtggcattcagcgttacgttgttggccttttcattcacaaaatcttcccctcttacttcgttggcaatggcatattttcctcccaggaacttgccgtgcttcatcacagagtacaagccattcgcctggctggcaatccgctctttggtttcaaaggccctgaaatcaggaatatctgtggaaggtaccgggtccagtaatcctttctgacaagcacccaaacctatcacggtaaccgccaatatatttaacacatattttttcatcttctttcaatttaaaagttaacattaagacccactgtcagcgttcttccattaccaagcgtgttacggtcaacaccctgaccggaagcattattaccattggaagaaacttccggatcggggccggggtactttgtaatcaacgcaaggttttgtccacgcacataaactttggcgccctgcaaacggatagcacttgcaacattatcagggaggcggtaagtgagtgcagcggtacttaattttacaaagtcgcctttgaaaacgttggcagcaatcgcaaaagaagaaccattggaaatattatcgccatatactacgcgcggcatatctgtctgatcacccgggttctgccacctgttcagcacatcggtactgttattccagtagcgttgatcccttaaccctgcattactgccgtagtacacataaaatcctgtttgataggtaagcaatacattcagctcaaaagctttgtagcggaaagtattctccaagccaccgagtattttcggattggtatttttataagccacagcatctttcacacctactgtaggagctgttttgccatcttcatacttatacttaacggcatccgcattattaaaatacaccttgtcgccgttggcattgataaagatccttctgccggttgcaggatccacaccatccgtacgcactacatacaacatactggcaggatagcctactttgttgatactggtttgttccaggctgctggtaacaaaaggaatggcagtaatatcgccggccagggatgttacttcatttttgttatgtgcaatattgaaaccgatgttccaggagaagtcgcgcttatcaatagccactgcgtttacgctgaactccattcctctgttgtacatgctgcctacgttggtaggaatggtagcaatggtagccgtgatgctggtgattggaatgcccgcagatggcatttgcggcacaaacaggattaagccgttaatatcattatagtaataagagaactcaccactgatcctgttattcaggataccataagtaaatcctatgtctgttttcttactggtttcccagttcagatcggggttacctgcctggttaaaataaatagaagaactgccaccgtaaggagcaggcttatacagtgataatgcatcgtagtcgcccaggcccgcgaagttacccactttaccatgactggccctgatcttgaaactgctgaatacattattaagacctgcattggtccagaaagcttctttcgtaatttcccatcctgcggaaaaaccatagaaagtacctttcttaaagttgggaccaaaagcggaatattggtcctgtcttacattggcgcttaaataatatttctcattgtaattataatttaaacgggagaaagcagataacaggtaattttccctgcgcagcaaataacgcgacaggtctgtgagccagccgccttcactattgttgaaatagttatccatttgtttctggcgacgcaaaccataccgttcgcgtgcatcccgttgttgctcaaaacccgccagcaggctgaggttatgattgccgaaagaacgatccagctgcgctgtatttgtccatacccaacgtttgttttgtgtataaatactgttaacatcaccgttagaagaaacgccatcgcccgacatgttattgagataaatatcgttgttcatcaggatgtaatcggcgccatactgggtttttaatgtcatccactcaaaaggtttcacctgcaggtaaatattgccctggatgtgactggcttctgtattggaatggtccatatccagcagtacctgcggattgtagataccgataggcagggtattttttccgccactcataccggaaccactgatattataacttccgtcattgttataggcggatactaacggggaagtgaggaaagcaagacgggcaagaccgccggagttaaaggcttctccttccagcgagccggaagatcccgagatcaggctttgttcattggagtaagacatccgcgcaccaattgaaaatgatttccccaattgctggtcaatgctgaacaggaggcttttgcgcgcgaagtcattctttttcagaataccctgttgtttggtatatcctgctgaaaaataatagctggtactttcagaccccccggaaacatttacgttgtgattctgcgatatggttttatcgcggtacaccacatccatccatttggtatcaatcactttaccgttggcatcgaggttggctacatagcgatcagcattaccggcatttttcagcgcctcatttttcatttcaagaaactgttccgtattcaatacggtgggcaggcgtgtgggcctggtagtacctacccagccatcgtagactactttcgggcggcctgcctttccttttttagtagttacaaacaccactccattggcagcgcggctgccgtaaatggctgtagcagcagcatctttggcgatatctatggaggcaatatcagcaggattaatgcttgataatggattcaacggagagttggaaatacctgcgcctacatcaccggaaaatgcaggtactccatcgataacaattaagggataggcgctcatggaaatagaattggagccgcggatccggaacaccggcgggttattcacgattccgttaggcaccgtgatctgcacacccgcggcacgaccgcctaaacctgcctcaaagctttgcaccggtaattcagcgatggcgctacctttaacggagacgatgctgccggttacatcttttttacgttgtgtaccatatcctactaccaccacttcggaaatagcttttgaatcgggcaacaggataacggtgcctgtggtattacctgtgacaggcagcgtttttgtttcgtatcctacaaaagatactttcaatgaattgatgttttcaggcacagcaagcgagaactcgccttttccgtcggtaacggtgcctgttttgcctccgggtaagctcacagaaacaccgggtaatccattaccggtatcgtctgttatctttcctttcacagtgcgggaatgctgtgccagcagcgaggttgctatcaatagcatacctgccagcacgagtagaagtttcctcatgtcagtttagatttaattgttgataaaaattacaatggtggtatcgggatttttggcaataaacatcctgctccggctcatgaaccggattggcatgcattaacaaagaccaggttattacttagctaaaagactctacagtcccgagttttaagattttagttataataattaaggtttagattcagaactttggttgctactacagtacaaatactcacaataaggtttgttgccagatttactggttacttaaaaataaaaaagaaatttaacttttcatcgcagtgataaatattactttgcgttcatctcttcaaaaacgattttccaacactctaacatttagctatcagcggcttatatattcaattaccgaccggaaatttttattctccccatccggttaacgtataggcataaccggtgtctttcggatgtgctttccagagaagcgtcagatcaagatccggatattttttttctgcgatggcagcaagttccaggtagccatctgcctgcatcggcttaatttgccggtattgccaggcggcgttaccggctgcgaatggaagcatccactggaaagccttacgcaggcttttcttaccggggctttcataattccagagatctacatctatcttttccgccatcagtgccagttcaaaaaatgctttcaggttaaagtaagaataattccaggaaagggtgcgctcgagttccagcggctgccggccatcggcttcaaattgttgttccatccgttgcctggtttgtgtgagcagcaattgttttgccagcgcctgttgtccggtgaacaatgccatggctactgcctgtacatcgtaccaggtaccatgattattttttgctgccaactcctccttccctattttactggtacgcatccaggtaaggaactggcggaaccagtcctgtatacttttgtattccaccaccggaaaggcgggcgaatctttcagcaactgcattccatccatcaatgcaattacagcatgtgtatctattaagccaataccccgtccttccgtaataccaggaatggcctggccgtagttgagattgggattcatccgggtagccggatcgaggaaccaggtatgtaataatgccactgctttggtggcgtattgttccttaccggtataaaaccaggcaagaccgagcacatttacatcgttgcacaaggcattgaaataagaatcatctttaatcgtatatcgttccggattggtcactccatcgcgacggatgtatggcaatccgtttgctttggtggaatccggccaccagtaggggcctacactcatgtaatcatgtttgtcgccactcggggggactttacttttaaaagtaaccgcatacggaccgtgttgcagcgcacggtcggcgcgcgtgagtaattcatgcagcgccttttcagctccgggctgatgcgttgcgatggctgctttctgcgccgtgagcacggcagggtcgaataaaaatgtgcaaggcgcggcttgttgtgcggccgtatgtacgggtaaacaggtgatcagtaaaataaagagggtacgggtcaggtgtagcatagttaatacttcctttctaatttaatcaattttcaactcttattaaaaatcttcttcaatcgcaataaccgggttttttaccgatattcacgaggctacctttgtttaaaaacattgaagctatgaatcattataacaccgttgccacggcaatagactatataaaagagcatttcaaaacgcagcccgacttacaggaaattgccgcggccgtacatatgagcccatttcattttcagcgtgtatttgcagaatgggcaggggtaacacctaaaaagttcctgcagtaccttacgctggattacgccaaaactatattgagagaagaaaaggtaaccgtgttcgatgctgcctttgaagcggggctttcgggcaccggccgcctgcacgacctgtttatcaatatagaaagtatgacgccgggagaatataaaaacggcggcaaagcattacgcattaattacagttttgcagagagtccgtttggtgatatcattgtggcatccacgtccaagggcatctgccatatggcttttgcagacgatcagcaactcgccctgcaggcgctgaccgcgcagtttccccatgcacagtttacccagatggtggaccttattcagcaaaacaccctgtatatttttacgcaggactggagccggctgtctgaaataaaactgcatttgcggggaacggactttcaactgaaagtatgggaagccctgctgaaaatcccgatgggtaatttaactacctactcacagctggcaacaacccttcaaaacccaaatgcttcccgcgcagtaggctcagcggtggcacagaatccggtggccttcctgattccttgtcaccgtgtaattaaagccaccggcgacaccgggcaataccattggggaagcacacgtaaaagcgccatcattggctgggaagccgccaaaaaaggaaatactgatggatgggagatataacctgcccggtattccggcagcgtccaaaaaaacaaagggctgcccgcttgtgtaggacagccccgtttttgcttatgaaaaaaaggaccagcactaaatagtgcctgccggttagacgaggaaaaaaagtttatcagaaaagtcaaaatatcaccattgtataaacgtcgtcaaacatgcctgcagggcatgagcattagttctctcacgaagatcagcgtccggtttagatgttaatcaagttagtttatcgtttgtgatacttctttttcagattttggttgctataaacacatcctcccgcagatgcttagtagtgcttaataggttaccttaaaaataaaaaataattttgcattttcatatataaatttcctgtttgtttagagtctgcattaaaaaacatatcgatatttagtatcaatcctttacatataccaatatccatgcgttttctgacctccccataaaaaacaatgaatccggaaagaaacctgccggtaaaccggtaagatggtgtgcccggagatggctgatcaatgtgtgctggaatgcccgtatatacttatcagtgagcgctggaatcttaccagataatacgcaaattttgccaaacaatctattttttttaagggtattataaggcggcgctccgattcttacacctaactttgctataccaaacaccaaagtacctacgggaacgcgaacttatgaatgtttacagtatagttaaaggaccccaacagccagagctgcttcatcatgaaacgctggccgatattttttcacaatcggtgcaggaacatgcccatcaaaccgcactgatattccagcaacaaacacttacttatcaacagctggatcactggagcgatgccatcgccgtattcctgcaatccaaaggaataggccccggcagtgtggttgggatctggtggccacgcagccttgaactgcatgcggctatactgggcatcattaaagccggtgcggcttatgttcccctcgaccgggagatgccggcagaaagagtagaaggtgtattgacagaagtaaaggcggcggcctgcttcagccaagttcccctccagctggaagcctcggtgttatcagtaccaccggtacctggcagcactgaaatattcacccttaacgccggaccgcaacccgaaaattttgcttacatattatacacttccggcagtaccggcaaacccaaaggcatcccgatcaatcaccggcagatttgccaccttatcagggcagaacaaaccgttttaaatatccgtgccaccgataaggtgtaccagggcttctccgtatcttttgatatgtggtgcgaagaaacctggctgagttactttgccggcgccacgctctgggtggccgatgccaccaccgccaaagccattgatgaactgggcgatgtattgcgccgtgaaaaaatcaccgtactacatgccgttcccagcctgctcgctatcatggacgataatatccccacgctgcgcctcattaatgccggcggcgaagcctgtacgccacaggtactatccaggtgggctgtacccccgaggcacttttataacagttacgggcctacggaaacaacggtaagcgccacttttgcagcgttaaagccaggagattatatcaccatcggacagccgctgcccaattacaacatggccgtggtagacgaaaaactggatatcctcccggtaggcgaacgcggagaactggttatttcaggacccggcgtaggcgacgggtatatcgaccgccccgagctgacccgcgaaaaatttgtggataagccagctgccatgacggaactacccggctcacgcctgtaccgcaccggtgatgccgccattattttaccggatggcagtatcgacttccagggccgcctcgatgatcagatcaagctgcggggatacaggattgaactcggggaaattgaaaaccagctccatgctattgccggcattgccgcagcagcagtggcggtaaaaaaagacagcaacgaccaggatcagctggtaggttatattgtacaggaagatcatgctccttttgatgaatccttcctccgtgcagcactcgccaaagtattaccaccctatatggtgcccggcaccatcgtagcgctggaagatatgccccgcctgccaagcggcaaaataaaccgtaaagcactaccactgcctgcggcctttgcacagataaccactcatgaagccattgatccggacgcccctgtagccgacaggatcagtgctatcctgtcaaaggtatttccggataaaatcatcgaccttcaacaggacttttttaccgacctgggaggacactccttacttgcagcagcttttgtatcacgactgcgccgtgaggccaatgtgcctaatgcatctctcaaagatatttatatacaccgccccctgcaggaactggtaaatgtatgggccgcacagccacagtcggctccaaagccaccccgcgtttttaataacgtgccgtggtggcgtcatctcagctgctggatagcacaaactgttgccatactggtgatcttcggattatttgccatgcagatattcctcccttacctgggatattattacgtggaacaggataccagccaccttggatatgcgatccttaccgctcttatcatgttttgcctgttaccgcctctcttttccatgcttattatcagtaccaaatggctggtaatagggaaaatgaaagcaggagattatccattatggggtacttattacttccgctggtggctggtaaaaacaatccagcgccttatgccttcacaattcctcaatggcacgcctttatacccggcttatctccggatgctgggcgtgaaaatagcaccggatgcgcaactcggcgcggtaaccattggcgcagaagatcttgttaccattggcagcgatgtaagtatcagttcacaggccgtcatcaataatgcatttgtggaagatggatggctgaaactacgcagcgtgtatcttggcgatcatgcatacgtaggcagcagtgcagttattggcggcgacacggtgatggaagcctggagtgaattacaggaccttagtttcctgccagccaacagtactgtgaaatctggcgaggtatggcagggtagcccggctgtactaaaagtaactaaaaatatcagtgagctgccacagcccctgccggtatcaaaagctacccgaagaaaatacagcgctatcttttcgctgttcctgctggtatttccatttacggtgctattgccgttgttgcctaccatcattaccctcaaccaaatggataatgccgcaccggattataacttcaattatatggtgatcacaccggcgctggcgctgagttatattattttatttaccgcgcaaaccgtgctgcttacccgtttactgcaatggggaattaagccgggcacttatcctatttacagcgcattttatgcccgtaaatggtttgctgaccagttgatgtcgctatcgctgattgtaatacatcctatttttgccacggtgtatatttcttcgctgttccgcgcactgggagccaaaataggccgcaataccgaagtatctaccgccagcagcgttacccatcctttactcgaaataggcgacggcgcctttattgcagatgcggtaacactcggcgaatctgatgtacgcggacaacagctgatactcgaaaaaacgatcatacataataccagctttgttggcaacagtgccctgataccacagggttatgaattgccggagaatatgctgataggcgtgttatccacaccaccctccaaagaacagctggcagctagtactgcccgcgactggttcggctccccggctattgcgctgccacgccgccaggaaagtcatttctttcccccggaactcactacccatccatcggcacaacgcaaactggccagggccacggttgaatttatacgtatcctcatcccggaaacagtggtgatctgctgcagtatcctgttcattgcctatgcccatgaccttgtaacagatgaaccctggtggatgatcctgttgcagttccccttctattatctctttttcctggggctgccggcattcttctttaccgtgctgctcaaatggattcttgtaggcaaatacaaggctttacaaagccccatgtggacatccaatgtatggcgcagtgaagcgattacttctacctacgaagcactctctattccattcctgctggaatacctgaaagggactccgtggctgccggtaatactccgcctgctgggtgtaaaaacaggccaccgcgtattactgaataccgcagatattacagaatttgacatggtggaaataggtactgatagtgtgttgaatgaagacagcggcccgcagacacacctgtttgaagacagggtgatgaagataggacccattaaagtaggccgcagaagcagcattggcgcaaggtccattattctgtacgatagtgaaataggcgatgatgtaaatattgcgccgttgtcgttattaatgaaaggagaaaaattacaacctggtaccagctggacaggcagcccggttaaaccggaataacgctatcaactatacgaaaatgattaacatccaatccatacaaataaaagatcactatgctctcatcaacaacatgatggagcagctgcatctttcggaaaaagcatttttcccgaaaacggccacctgggaaagcattgcatccaactatatgcaacatgtgatagaaatgcaggaaacctgcggtggcacttgcctgctggcctatgcaggtgataaaccagccggcttcatctttgcatatccggaagaaccggacgacagccggattgaagattatacgggtaacaccctctatgtatctgatggttatgtagcagatgaattccgccgccagggtatttacaggatgctgaatgaagaactggaacggatatacgtagcaataggtgttcgcaggatagtcagatatacgctggcgaacaaccatcgtatgcaacggttcctggcatcggaaaaatatgagccggtacggctggtatatgagaagtggctgacttaacagccccttctctaatagtcgatagcatggtcctttttcacagaagctccggcatatactttctttgaggtccatggctgcgccggatccgaccagaacggactgccgtaaggtaagcccaacgccaggaaaccggtgctgcataaataaaggctgccggtagaggtataggtatctgcaatctccggctgatgcccgcagaaaccaatctgcatccatccttttttatcaaaagtaccgggcacctcaaatattcgtttattcactgccgttagtgcacaccttacctgtgcgggcgatatttcttccggcagtttttcttccagtgcaatttgcgcaagtgcctggaaagctgcgttgcggtaaggcatagagcgacccactaccgggaaagttccttcaggagaaatttgcctttcaagaatagcggcataacgctgcattcgttttaatgccagctcatagtttgctttactcccctcttctttttcagccatcacctttagtacgtctaccagcatgggctggatcacaaaagagttgtaatagtcgtagtgaaaatgcgcgccgtcgccatacatactgtcacccttataccactccatcattttttgcacggccaggtcaattggtttgcggtcccagtcggcgccgaatttcagcagcatggcttcaatgatggcggagaacaatacccagttgttggtaaatgctttaatgctgcgtaaactgattaatccatctattacctgctgttgtgttttgggagtgagcctgcgccatacatgctttggtgcgcgtaataatccatgcgcgaggaaagcgccgtctaccagtggttgtgcatcaaatttgcctgtaaaattcatatagtcaggggatgcaggatctactgccatcgctattgctttgtgggtcatttccagcatggcaatacgcttgcttccctccatcgtgttgtctggtccaagttccagccagggggcaatgccggccagggttctgccaaatgcttcgaggtaggttactttctccaccggctttccatagttcggcgccacttcggtaggcatggtggctttcagttttcctttgctcagttgctcaataacgggctggcatatacgaatcatcagatccacattatactccctgtcatcgggtgcaggcttttcagccgccatcgctttcagcaatcccttttcagagcctatagtacttgccactcctgccataggaatagctttgataaaaaaacgtctgtccatgcaaataaatttacggcattattttgcccattgtttataccggagtaatgcttctacaaagtaataatcagcataagtgagcggtacatctacttccgatttattaggcaggtggcctacgctatgcatcagtataaaatcattgttttctccttccttcgccaggtatgccgggctgcaaagactggtcagcattttctctgctgcattccagtaacgtttaccatcggctttattggtgtaacggcttagctccagcaatgccgatgcggctactgaagcagcagatacatcacgcagtgcgttgggaatatccggcgcgtcgtagtcccagtaaggcacgagatcggccggcatatgcgggttatccaggataaagtctgcgatatgacgggcctgctccaggtaggctttatcttttgtatcgcggtacataagggtatagccatatagtccccatgcttgtccgcgtgcccaggcagaactgtcggccagtccctggtgtgttttacgttcatttaccgcaccggtagcgggatcgtaatccactacgtggtaagagctgtagtccgggcggaaatggttcttcatcgtagtgttagcgtgtatgcgggcgatttctgcaaactttttgtcgccgctttcgcgggtagcccagttcagcagttcgaggttcatcatgttatcaatgatcaccgggaacttccatgcgccgtgatcccatgatttaatacaacctacggtcgggttaaaacgggtggacaatgactttgcgctggtgagcaaaatggatttgtaagcggtatcttttgtgatgcggagggcattgccaaaggggcaatacatcataaagcccaggtcatgtgtgtgggtattgtactgttctttttgtaccagcgccattctcttcagggcttcgtttttaaaggccggatctttggtatattcaaaaaggtaccagttggtaccgggataaaaaccggaggtccaccagccggagttagatgtcatcaaactgccatctttgctggtgctgcgtggcagcaaactatcgggtacatgcgtcatcatcagcttgtactgcctggcggcgaattgcagggtggcatctgcttttgcgagtagggctttatctgctttacccgcctgcgcatacgattgcattataaatgccggcaataacaataccgtaaagaacaggttcttcttcataataacgtgattatagtatgatcatttcttttttccactgttctttgctgtaccagcagaagattcgcgggctatcagttgaataggtattatttcctgtgaataacgtgatacagtggaaggtgcggtactgatcagttccatgagagcggctaccacacgttctcccatcatggccgggtactggtctacactggtaacagccggcgttacgatttctgtacggggatcattggaataccctactattttcaggtcttccggcacccttacatttattttccggcaatactgcatgatggtaatggctgttgtatcgttagatgcaaaaacgccatcggggaatggaggttgcgagaatattttttcacaggtttgccaggcgttatcgcgggtgagttcgtgataaaatacgcgcgtttttttaaacggcagttttgattcctgtaatgcattcttataccctgctaccctttccacatacaggttacagctgagcggcccggaaatatgaacaatgtctttacagcctttttctatcaggtggttagtggcggtataacctcccaggtaatcatctcccttaattacttttacattgtaatccttcggtaccctgtcaaaaaatatcagcggaattttgttgtccttgaatacatcgaaatgggaaaagtcggtggtatataaagtggtagataccaccaatccatctaccctggcggaatacagcgtatttaccagtgctatttcctgttcgtaggaatcgttggattggcagatgatcaggttatatccatgttcctgcagcttgttttgaatgatggtgctgatggtagctggaaagaacatagagatacgcggaacaataagcccgatggttttgcttttgttgttgcgtaacccggcggctaaggcgttgggacgatagcccagtttacgggccatcttctttaccttatctttcgtacgtgcgctgatgttaggattatcattcagggcgcgtgaaacagtggatacggagagcttcagctcttcagcaatatccacaattgttttttcggtacgtttgctcatgtatagaggctattagctataatatgtcctgttatcttcccatccagccaccatccactgtaaggattgtaccatgtatgtaatcagccgcttttgaggcaaggaatattgctggtccggcaaaatcttccggttcaccccatctgccggccggaatgcggtccagtatagcgctgctgcgttgctgatctgccctgagggctgccgtattatccgtggcaatataacccggcgcaatggcattcacatttacaccttttgaagcccattcattggcaaatgcctttaccagtgagcctacggctcctttactggctgcatatcccggtacgttaataccaccctggaaggtgagcaaagacgctgtaaagataacttttccgcttccacgggcaatcattccttttcctatttcgcgggtcaggataaattgggcgttcaggttgatgttaatcacttcgtcccagtactcgtccgggtgctctgcggcgggtttacggagaatagtgccggcgttattgacgagaatatctattaccgggacgtcctgttccagttgtttaataaatgtatagaggctggtccggttggaaaagtcggattgataggccttaaaactacggcccaatgcttttacttctttttccacttcgctgccctccagctccagggaggctgaaaccccgataatatctgcacctgcggtagccagtgccactgccattgcttttcctatgccacgtttgcagccggtaaccagcgcagtttttccttttaactgaaataagtccatgatgaataagttggagttttccggcaggccagtggtggcctgccggaaaagttattgaatcgttacctgtaagggttgtttgatcttccgggcgaatgtttcgagataggcgaaccactcttcggcagaagtgatcctgccacctttgctccatgctgccccgaaatagtactcatatggctgctggctccctgctgttccgggactcagcaaatgtacatgatccgttttcattccgggtacttcccgtgcaaaaacacaacctatgcccagcgtgccatcgtcgccatgagcgggctcccaataacccattacgcctgttttctcatccagcaatacggtgccgggctctttgcgttttacaatacctgttaccacggggatgtcattccctttgaagctgtattgcacctgcattttattgagctgggaacctgcatccagggagatggttttagtaacggtaacggcggtgttgcctgcctgccaggtatcgtaggtgagggagaaagtggtgcgcaacggaccattgtcgagggttttcgactgccggtagttttttgggaaatagatggtatcctgtccggatggcgctgtgtcgcctgcgccaagtgttaagcccacgctgtaatagtccagcccctgcccgttatcgtggtgatagttgtccagtttataccaggtgtcaatcaccatatcggtggtacgcttggcccatacgtcaataccataggccatttcttttggtactttttcaagcgcctttccatacatgcgataagccatgcggtcgttttcccaggcgtaatcatctttacgctccggcacataacgcccgtatgcctttgcctttacgggcgccggggcgccttccactacccgcgcatacaaacttgcagcagcgggcagtgttacctgtaacaatatcttctttggcgatttaccgccttcataaatcagttgataaggaatttcctgtccgctcaatacgtccactatcttaaaacctttcagcgtttgtttggataattttgcactgaaagcggggtaaggaatttctgtcacttcttctatcctgttgataccagtgttattggagatgattacctgggcagcagcacttttccggagatcatatttgatcagttccgagcctgctaacaggaacgcacctacgccatatacttcggtatcattggcggttgcttttccgggtgcagcgcctatttcctgcacaaatcccagcttaccatccgggtgcacgcagccggtaagcgcttcccatcccttttttatcaccggtaaaaattccttctccggtaaaagaccgttattcactccccacatcaacgcatatacgtaaaagccggtgccgcttgtttcctttgccgggtagctttcagggtccagtaagctggcgtgccaggtgccatcggctgtttgcagggcttttatgcggtaagccatttgtttatacaactcctggaaacgtgcctttccggcgtagccggcgggcatattatccagcatacgaaccaggccgcccattacccaaccgttgccacggctccagtatacattggtcccgttcttttcttttttgccgatatagctgccatcgcggtaataaaggctgtcctgtttattatacaggtagtctgttgttttccaccatagcttatctgcggtggcgaggtaacgcggatcaccggtggccgtgcttaaataagccagtgccgggggccccatgaacaaggcatcacaccaggcccattcgcggtggtgaacaccatctttccattcgagcgattctgtatgcggcgctgccacaatgctatctgccagcttacggaatttatcggtcatcaccggatctttatacacactattcaattgtgaatagagctgacctacgcaatattcatctgcgaagaaacgatccggcccggtgttccagttattgtctttccctacctgtaccaggcggtccacaaaaaagggattggatgttacctgggccagcgacatcataccagcgtacatggcgccattagtccagtcggtaggcgcgtggttccagccattttcagttatatggcgccattgccaggaagccactttttccatttgcgcccttaccgcagctgcggtataggcatccgtgaaaaccgtggcatgcagaccggtaacgggttccgcagcatgcaccggtaagccggcatgcaggaaagacaagcccagcaagcttcctgcgataatttttttcatcatcatgatagcagctattatcagttcattaacgtagttccgtgatcttgcaatgatccatatcactgtagtcgaggttttcaccggccataccccatataaaagtatagttgctggtgccggcgccggagtgaatggaccagggtggggaaataaccgcctgttcattctgcatccagatatgccggctttcctgtggctgtcccatgaagtggcatacggactggccttccggtatttcaaagtaaaaatacacttccattcttctgtcgtgcgtatgtgccggcatggtgttccatacgctgcctggttgcagctcggtcatgcccatttgcaactggcaggtttccagcacgctgttcaccagcagtttattgatggtgcggtgattggcagtttccaatgtgcccagtgttaccacttctgcctcttttttagacactttacgggttgggtagctatgatgtgcaggtgtggaattaaggtagaatttagcgggtgttgctgcgtttttactggagaagatcacctgttgttttcctttgccgatgtataatgcttctttataggccagttcaaatttttcgccgtctacttccactacgccatcgccacctacgttgatcatgcccagttctcttctttccaggaaataggctgctttcagcaggtcaattgtgtccagtgttaccggtccttttacgggcatagcgccgcctgtgaggtagcggtcgtaatgggtgtgggtccaggcaatgtggtcggcgtcgaagattttctccattaaaaatgcctgcctgagttgtgcagtgtccatttgttttacttcagccggactgctggcatatcttgattcgaacgtggtgctcatataatctgcatgtttttatttatttgaaaaagcagctgatggttcttctcagcttactggtaatttacatcattatctttcccgataattttcgctaatcaggcggaaactctaaagtaatgcaaacgtttgcaaaaatcaagcatttatttaaaaaaatgccttcacagatggccagattcctttatttacggcgcatcacgaactccaccgagtgtttgccggttaacgcctgcttccgggccttcaggctgatgcgtgttacatactcgccccacactggtgataagcggccgtcttttatttcctcttgttccgcagttgcttcaaataaggcaggatcgtaggtcagtaacaggtcagctgtgctgcctttcagtaaaatcctccctggcgtatgggtatcggcatccaggctggtcataaaatgcagcaggaagggctccttccaatctttcaactggtatgtttctgataactgcagtgaagttttggcggggttgaatgtaaaggtgcgcttccaggattgcaccatagctgcctcgggatacgccgcggcaatgtccatactcagcttgttacggctgtattgcacagcagtagcctggaactgccggccatcgcgttgctgaacaccgttgatagtaggacagttatgccattgcgattgcataaaccatagcttatagcggtcggcactgaatgtttgctttgtataagtgcctacgcccacatcaataatggcgggtttcccatccatgtacagcacaaaatttcccacgtcgttgtgattatggctttctgcattatgtccgccctgtgcggcaaagaacaagcctttggatacgccggcttctgagcgaagggacaatacctgcaaatccgggagccagttttcagcggtataaggggctgctgctttagcagataacagggcgttgcgaagttccacgttatacacaaagaaagccagggaaggcgtcttcaccctattggtgtcggggctctccagccttgagagataagcggcgaagttgaccagcaatggatcatgaaaggctgctccgaataaatacaccgtatgtgcgggcggaatggtgctggcagaagcatctgcaaaattcacaaaccggctgctgtccacatgcattttataaatgtaggcgccaatgcggtgaatcagttcattgttgctccagctcagctggtgtgcagaagcactgttcagcaggtcaataaattcaataagtttacctcctgcatgtccccaataggtaggtccttcatcgcagccgccatcctccggatagccgttcacgaaattatccgcgctgcggatcgttttctcaattactttatttcgtatatccgtttcatttatgcccagtaacgcagtttgtaaaacattggtattgatccagatattccagttattcacgctgcggccggcccatcccatccaccagaaatcggtccgtttcaggtaaggctccacaatgcggtgctgtagttcataggtgatccgcttatttactaccggggaaaatttatccagctgatcgtgcagcaggaactgtgcccagctcagtgtggcggcagtttcccctgcaaacaggtctaccaccggctcttcagggtccggcaggtcgctgcctgctttctgtgccccgatatgtgccggcaatacccaggtgctttcttccaggatcagccataaaccatttacgatttgcggtatatactttcctttcccctccaccagttctcctgccactaatgccgctaataccttccggcgttcaaactgtgcattttcaaaatttacgcggttgccattatcacggtattgcaggtataaagtagccggcaatgaaggccagctgaacgataaatttttatccgcttccttcagcaatatggccctgctggcggccggcagggcggcaatttgttccacgatggatttatatcgttgctgcctccattgcacaatatttttaaatgcagcatcactacctttctgcctgtattcttcgtacaaataatttcttgttttaccagcatcctgggcaccaacgttgccgcctatactaatacctgaaaagagcaataccgtgcataccagttttttaacgtgcatttgacatttatttttagtaagatataagcaggacggaattataggctaaaggtgtggagaggcactgtcatgtatttgttacaatactgtcattcattgttcaccgggtgcttactttcaaacggaatcttgccgcctccggtaaatagtgcccataccggcatctttaaaaatattacctcttctcccatggaatttactggtttcatcgccggaaacccgcgccggtgaatcaaaaatatcaaaatataccagaattacaaacgtttgcatgaacattaccggataactacctgctcctatccggccggtgaaatcctactgatagccgattaacaatttataattcattcctgacctgctcccataaggtgttccagcggtataatcaaatagtcaaaatcttatcatggattaacattttactatcaccagccggagcagttatttactactttagctcctatgaacgcttatttacaaattcatcctgacgataatgtgctggtagccttacaggatataccggtaggaaccgatatctcatttaacggacataacattcaactgcaacaaaatatttctgctaaacataaattcctggtaaatgatatccgtgaaggggaccccatcacgatgtatggtgtgctggtgggcaaagccagtaaaagcatcaggaggggggaaaccattaccacggaaaatgtgatccatgatgccaacgcatttcatgaaaaagacagctccctggaatggcaggcgcccgatgtgagtaaatggaaaacccgcacctttatgggctaccaccgggccgatggccaggtaggcacccgtaattactggctggtaattccattggttttttgtgaaaacaggaatgtaagtgtaattaaaactgccttcgaaaagggtcttggtttttctcctgccgaagtatacaacgaacaggtaacagacctggtttcgctttacaaaagcggtgacctggaagccattaaaaactacgaggcaggcgcgctaacggaaacgagtaaacgtaacgtagttttcccgaatattgacggtatcaaattcctcacccatgagggaggctgcggaggaacccgccaggactcagacgctttatgtgccctgctggccggttatattcatcactccaatgttgccggagccactattcttagcctgggatgccagcatgcgcaggtatctatcctccaggaatcactgaaaaagctcaacccggcctttaacaagccggtattggtatacgaacagcagaaaagtgcttccgaatttgcgatgctgtctgccgccatcaaagacacgttcctggcgctggtggaagccaataagctgacccgcaagccaagcccgctctccaaactggtcatcggactcgaatgcgggggctctgacggattttccggcatttcggctaacccggctgtaggtcatacctccgacctcctggtagcgctgggcggcacttctattctttctgaattccccgaactctgcggcgtggaacaggaactgattaaccgctgccagacagaagaaatatccgataaattcatccgcattatgcgcctatatgaaagccaggcccagtcagtaggttccggcttttatatgaacccttctccgggaaatatcaaagatggcctcgttacagatgccatcaaatctgcgggagcagctaaaaaaggcggcacttcaccggttacagacgtactggattatactgaatatgtcaccaaacccggtctgaacctgctttgcacccccggtaacgatgttgaatccacttcagcagaagttggttccggcgctaacgtggtgttgtttaccacgggtctcggcacgcctaccggcaacccgattgcaccggtagtaaaactggccaccaataccaaactggccacccgcatgaaagatatcatcgacatcaacaccggtactatcatcagcggcgaacaaaccattgccggcatgggagaagaaatcctggaatacgttatccgtaccgccagcggcgaagtgcatacaaaggccgagcagcttaaccaggacgattttattccatggaaacggggagtttctttgtagcgaaggttgtcttactcaggattacactgattaagctgattactttgattttgtctttttgattttattttgattttttgaaattaagaaagatatattaagagaataatttttgatactcataagaataaaaacaaacgtccggacatctgcccggacgttttctatttaaaggaatttacaattctttcttactcttattaaatcttataaatcaaaataaaatcaaaaagacaaaatcaaagtaatcagcttaatcagtgtaatcctgagtaagacaaaatccgcttagttcaggttaaccgcctccattttaggcgcaaagaagtgcattacggtccaggctaccaggtaggctaaagcgcaaatggtgaataggatattgtagccaataccaatgttgccgattaatttataatgatccagcatagcgccgatcagcatggggaacagcgtaccgccaatagatccggccataccaccgatacccactacagaacttaccgcccgtttagggaacatatcagatgcagtggtgaatatagtggcggaccatgcctggtgtgctgcggtagccaggctgattaatgcaatagcgaaccatacattattggaatactgtataagcataataggcaatacacaaagcgcaaagatcaacatagacactttacgggctttgaaaaccggccaaccggatttgatcaggtgggaagataaccatccgcccccgatgctgccaaagctggtaatggaatagatgatgattaccggcagacccagcgtttctttcatatttacatggaaaatagattccaggtaacctggtaaccagaacaggaaaaaccaccatacggggtctgtcagtagttttccaaatatgaaagcccatgtttgcctgatacccaggagtttactccatttaatgggtttgggtttcagttcttccacttcctggtcggaatggatatgatcaaattctgctttggataatttcttgtgacgggcaggaatttcataatagatccaccagaatatcaaccagataaaaccgatggcgccggtccatacaaaagcatttctccagccatgattgctggccagccagtataccatagccggtcctataacagccgcaatattggaacctgagttaaaaatgcctgtagccagtgcccgctccttttttggaaaccattccgcggtggctttaatagccgcagggaagttacccgcttcactcacacccaggatagaccttaccacaccaaaccccagcgtggaacgcaccagtccatgtgccatcgccgacaggctccataccacaatagataccgcgtatcccagtttggaacctatcttatctaccaatgcgccaaagaaaagcaagccaatcgcgtaggaagcggaaaatgccattaccaggttgctgtacgccgtttccgaccagttaaactcggctgataaatcagttttaagcaatcctaatatctgtctgtctatatagttaatggttgtagcaacaaataaaagtgcacatacccgccagcgatacttacctaaagttgtggaattcattacggtttatttggaatttataaagtgcataagttacttcttagccctgagaaatgcaaacgtttgcactattttatctttcagcgcgccccagtccttactttcaatcagggacttagacagcaaattagaccccattcccacgcataccacgccggcatcaaaccaggcatccatactaatacgagtaggttctacaccgcctgtaggcataaacttcagttgcgggaacagcggcttaatggaatttacatagcccggtccgagtacattacccggaaacagcttcaccagccgggcgccattcttttcggcaacagcaatttcggtaggcgtcatacagccgggaatccaggtaatgctttcagcactgcaatatgtggccgtttccggatcggttacgggacaaacaataaagtcggcgcccataccggtatatactgcggcatctgatgcgtttttaatagttccgatacccaggtacaaatccggcatggcagccagtttcctgtcgcgcagggtagcgaagttctttcgtgcattttctcccctgctggtaaattcaaatacccgtaagccgccatcataacaggcttgcagtacttccaggcaaacattttcatcatcatgataaaaaaccggaataatcccgctttgctcaaatgctgctataattgtatcaggacttggtgccatatgctatatcagttttattatttctttctctgaggtagtattaaaatctcccatcacaaaaaatttggaatacgcggcagcggcggcaaaggaaatgatctgctgatcgtccagtccctgcagctgtgcatgtattaacccggccatgaagcagtctccgctacctacgcgatccaccacgtcgttggtatcgtattcacgggaaatactcatctgtccttcgttatagtaaaaagcgtagtacaaattatgagtaggagcattgctgaaacggaaagtgaacgccacccgcttgcaacgcttatacgtagcagtgatttctgctgctaccttttctgcctgttgcaggtaggtgtccttgctattggcttccagcgcagctgtatccagtgcggtatccagcatgttattggctgcccagatgttgcccatgattacatcacagtactgcaccagctccggcatcacatccaccggctttttcccatactgccatagcttgctgcggtagttaagatccgtggaaatgatcaaccccttccgggtagccgcttccaatacttccttgcaaactgctgctgcatcggggtttaaggcgggcgtaatagcgctccagtgaaaccattcggcatcaccaagcaaactgtcccaatcaaccgtgccgggggctatctggctgaaagatgaccatgccctgtcgtacaccacttctgcatgtttaaggtcgctgccctgtgccaggtaataaataccaatgcgcgcgccgccccacaataccctgtcggtatggataccgcggttactcagttgctccagcacgtctttcgacaagccgttttcaggcactttgctgatataggccacttctgtgccccagttggccaatgcagcggcaacgttggcttccgcaccgcctacgtaaatggcggcagtattttgtgccagctgcggcgacaagcgtaataatatttctccgaatgtgataacttttaccggcttcattagaatccaaaatatgcttttgcgttatagtaacatatatcctgtaccattttccctaaccaggcaatatcatttggcagctctccctgctccacatcgttgccgatcaggttacacaaaatacggcgaaaatattcatggcgggaataagacagaaaacttctggaatcggttagcattcctacaaaccggctcagcaggcccatgttgcttaatacgttcatctgcttttccataccgtctttctgatccaggaaccaccacccggaaccatactggattttaccggcaacggtgccatcctggaagttgcctgccatggtagcaaaaacttcgttgtaagaagggttgaggttatacactactgtctttgttaacttatctttcttatccagtgcatctaaaaatgcgctcatggcttccgcaacgcgccagtcgccgatagaatccacaccggcatctgcccctacccgttgcagcaggcgggaattattattacggatagcgcctacgtgaaactgttgtgtccattcccgttcgtggttccactcgcaaacagccagcaggatcgccgttttaaactgtgcattctcgtaaggcgttgctgcgcgatggtctcgggtattattgaaaatagtgtccagttcctttccggtagccggtgaaaaataaaaggtgctgatgccatgatcactcaggcggcagccggcttcatgaaaataggtatgccggctatgtaatgcttctatgagatcatcgaacctggtgatttctttattggcaactgctgccagctcgttaataaaacggttgaacaccccgggattgtccactgccatggccctgtcggggcggaaggtaggcagcacccgtgtgccgaaaggcttattggcaatagcacggtggtgttccagcgaatctaccgggtcgtcggttgtgcacagcgtgtctactttataatgttgcaggagtgtttgtgtggataaccggggtaattgtgcattacagtcgtggtatatcttctccgccgttttttcattaagcaggtccgttacaccaaaaggattttttaattccatgtgcgaccaatgatacaacggattccgcatggtatacggcgtagtagctgcccaatggcggaatttcgtatagtcgtcggcggggccggtaataaactcttccggtacgccgttggcacgcatggcccgccatttataatggtctcctttcagccagatggcatacaggttggcaaatgttttattccctgctatttcgtccggtggcaggtggttatgataatctatcaccggcatggacgcggcgtaatcaaaatataatcgtttagccgtttccgtttttaataaaaaatcttcagacagaaattccttcataacatgattaatttttgagcagctgcgattggataaatgctttcacgccgctgcttttcagcatttttaagatcccggccacctgttcagcaaaaccgggaatggccgacagatctgtttcccataaacgtttatcactgcagatcccggttaccatatcgcttatattggtgtgatcacgccaccaggctgcaaaaaccggggcgttatcgtcggtaataacatattcttccccgttcctgctgccgtaatatttaccggcttcttccctcaccggctgcaggaacagcagcatggcggcgaagcccaggcacagatgaggcgggagcgcgttgtatttttcgtagtaacgtaccagtgtgcgcacgttgcgcgcattcatcttggaactttcctgaaaagtgatgctgatgagcttatgcgcaataaacggattggcaaaacgatcgagcacttccggtgcaaacgcggccgccgtaggacaagcctcttcaatggtaggcagtatttcccggagcacgacttctttgaagaaatgactcatataatcgtcctgcatgcactcgtatacggtgttgaggcccgacaggaaagccaatggcactgccgcggtatgactaccgttcagtaaccggagcttctgttcacggaacggggtgatgctgggctcaatcaacattctttcatctgccttataaaaagataatacagaacgggtacgttcattcccttctatggcccacaacagatagggttctacttctatccataatttatcggtgtacccggccttttgttcaatttccgccaggttacggggtttaccgggaacgatcctgtcgaccagggaattgcagaattgattatcctgctggatccacgtgataaatgccggcggcagttcattataggcggccaattgcaatacaatatcttttaaaaggcggccattgtctaccaccagttccgtgggtacaatgacgaagccggtattggcgctacctttaaaaaaggtaaaccgctcccacagcaccgccagcaatttgcccgggaaggaggctggtacgccgtctgctattttttccggaacatattggattcctacttctgtggtattggagataattgtttgtaaagcgggctgatgaaccgcagctaatatttcctgccattctgcattcgattgcaaaacccggctaatagcggcgttgatcagtaactgatctaccagttctccctgggaaacacctttgatatgggtggtaaacaggctatcctgactggaaaaatcaatggtatcgccatcggtcgatttcactaccacaatccttccttcgtaaattccctggcggttggctttatctacaaggtagtctactaaaccgcgtaaaagcacgccggtaccgaattgaaggatcttttccgggaaggtgaatgttttttcatgaacgccggaatcctggttttttaatataagctctttgtttaatataggtagcattgcgactaatttatgctaaaaggtggctaaaactaataaatatataattcacaactaacaatttatagtgtttcggaaaataatcgccaaaacttgttaaaattataccggggatataatcagaatcaatcccgccattgtcaggatcaataaagcacagatggccgttggcttaaatttaagtaattttgttgctctaaacttttataaatgagcaagcatggtaaagtgctggtagccatgagtggtggtattgacagcactgttacagcgctgatgctgcatgaacaggggtatgacgtggtgggcatcaccatgaaaacctgggattatgcatctgcgggttccagtaaaaaggaaaccggctgctgtaacctggattcttttaacgacgcccgcgcggcagcggtgcatcatggcttcccgcactttgtgctggacatccgtgatgaatttggtgattttgtagtgaataattttgtcgaggaatatatcgcaggacgtacgcctaacccgtgcgtactgtgcaatacccatataaaatggcgcgcactgatgaaacgggcagacgcaatggattgtgagtttattgcgactggtcactatggccagatccgtcagcacgacaatggccgctatgtaatcagcaaaggcctggatgaaaccaaggaccagagctatgtgctgtggggcattcaacaggatgtactggcccgcacaattcttcctttaggcaaataccgtaaaacacaaatacgccagatggcttttgatttcggttatcccgaactggctaaaaaagcagaaagctatgagatatgctttgtgccggataacgactaccgcggttttctgaaaagaaaagtagagggattggaagaaagagtaaacggcggcaattttgtgctggcagacggcacgatcgtaggccatcacaagggttaccccttctataccgttgggcagcgtaaagggcttgatatcgccctcggtcgtcctgtttttgtaacggagatcatcccggaaaccaacaccgtggtgttaggtaatgaagatgaattacagagaagcgaaatgtttgtaagcggcattaacatggggaaatacgataccattccagatggcatggaagcggttaccaagatccgctataaagataaaggcgcgctgagtaacctgtacaatgaaaacggacaggtaaaagtaagcttctacgaaagcgtgaaaggcattgccccgggccaatcggctgttttttatgaaggcgacgatgtagttggcggaggaattatccagcggacgatgccggttttgtaaaaattaatttcataaaaaagggtgggaagacaaatcttcccaccctttttttatcttcaaaaactaagacaatcttactgcatacatggtatccgcgcccttgtcgtatccggcaattacgcctccttcctgcttccgcagatcactgatctcttctatatatttcaccacttcttcattctcctgtttaaaaacagagcaggtgatatagatcagcgagcctcctttttttacaaatggcgctacattatgggctatctttttctgtaactgctggtacttcccgatctcgtcttttttaaagaaggagatgctttccggggtacggccccaggtaccggagccgctgcagggcgcatccaggatgatgccatcaaactgctgacttcccatagaagcaggaaagttttctgctgtaagatctgccacacgtgcttcaaaatgcttgacccctgctatcgcaaaacgttgctgcagattttccaggatagatcttctcacatcagataccagtaattgtacaccgggctgctggtctttcagcaagatggatttaccaccgctggcagcacagcaatcccaccaacgctgctgcttctgcggatggaataattcaccggtttgttgactggaagcgtcctgcacctcgtaccagcttttttccggtaccactacttctattttagtgccgttgggcaatgccagggtggtattattgggaaacagttcatacggaatggcggccttatccaataatgacaatactttatcaagcttattattgcgcacgcggataaataaccgcggctgctttaagacagtataggcgtatgcgttagcatctattccgtccgacaggtcgggcagaaacggaaaaagtgtatcaggagttaaaggaacaggcagcagcgctgctttatcagtcagcggcgatgtgatctgctggttccaggcagggcggatcgctgccaggaaatcattcggtgtggtttcgcaaagaaacgcgccggtaatgatccgttcgcttacagaaaggcttttaccccagcttccgaggcggaagtaatgatataccagctgtgaaatccagcgccggtcgcggcctcccatgtagggatgttccttgaaaaaagatttcaggaaatggtgtaatggcaggctgccctggtaggcgccgataattttttctgcagatgctaaataattttcccaacgggtcatacgcgaagataagggctaatattgacgcggtggtgatcgcacaaaaaaatccggcctgataacagaccggattttattttattttctcagctgaaactagagtttcagcaatgctttcagcggatctttaccgaacagcaattgttcaggattttccagcatttcttttactcttacaaggaagctcactgattcgcggccatcgataatacggtggtcgtagctcagcgccaggtacatcatcgggcggatcaccacctggccgttgatggccatggggcggtcctggattttgtgcatacccaggatagcggattgcgggatattgatgataggtgtgctcatcagggaaccgaaaacaccaccgttggtgatggtgaaagtaccaccggtcatttcaggcatggtcagtttgttgtcgcgggctttggtagccagttccactactgctttttcaatacctgccatatccaggctttctgcattgcggatcaccggtactaccagtcctttcggagccgataccgcgatagagatatcgcagtagtcgtggtacaccagttcttctccgtcgatataagcatttacagaagggaattcctgtaaagcgaagcagcatgctttggtaaagaagctcataaagccgaggtttacctcatgctgctttttgaatacttctttatacttagcacgcagcgccataatttctgtcatatctacctcgttgaaggtagttagcatggccgttgtatttttcgcttccaccaggcggcgggaaacggttttacgcaggttgctcattttttcgcggcgttcggcacgggtaaacatttcctgacctattgccacgcctggattttgcagggcggcatatacgtcgtctttcatgattttgccatgagcgccggagcctttgatgctggaaggatctacatgtttatcggcaatcactgcggcagctaccggggatgctttcacatcattcgggatgctggtaacaggcgcctgttgcggttgtggagcagctttggcgggttgtgcggcgggagcggctgccggtgcggctttgcctgccggtctgccaacactggtatcaattttacaggcaacgtcgcctatttttaacgtatcgccttctttggctacggtaatcagtgcgccggcttcttctgcattcagttcgaaggtggctttttctgattccagttcacataccacttcatcacgctctacataatcaccattattcttcagccactttaccagtgttacttcactgatagattctcctactgtaggcactttcatttcaatcgtccctttatttgctgcaggtgctgccggtgcggcttctgccggagcaggtgcaggagctgctgctgctggtgcagcgggttcagctgccggtgcggcgtcggttgctggtgcagcggcgtctgtatcgatgctacaggctacatcaccaatcttcaaagtagctccttcctgagctgcggcggcaattttgagaacgcccgccttttctgcattcagttcgaaggtggctttctcagattccatttcacacaatacctcgtcctgctgaacataatctccgtcttttttcaaccactttgcaattgttacctcgctaatagattctcctaccgtagggactttgatttcgataaccatatttaatcagttgatggtgataccaggttttgcatttagcggttagcccttagctgaacgtaaaaccccgttattctgtttatactttgaatttctttagatgttaaaagccgtgtcaatgatctgttgctgctcacgggcatgaactttcgcataaccggttgctgtggaagcgctcggattgcggctgataacaccataattgatctgtttcaggttcatttgcaggaatgctgcagcgcccatgttcagtggttcttcctgtacccagaagaaggtagctcctttatacttctgcgcaatagcttccagttgtttaaccggcagtggatacagttgttccaggcgaacaatcgctacatctttgcgatcgtctttcgcctgtttgtcactcagatcaaaatacattttaccagagcacagtaatacctttttcaccacagcggcgtcgtcgataaacggatcatccagaacttccttaaagccaccctgtgtaaattcctgtatggcagagtaagcgcccacatgacgcagattcgcttttggagagaagttgatgagtggtttgcggaactgccaggttaactggcggcgtaacgcatggaagaagttggcagcagtagtaatattggtgatcaccatattttcttctgcgcattgttgtaagaagcgttccgggcgggcattggagtgatccggtccgccgccttcataaccatgaggcagcagcattaccaggccattctgcgtagtccatttctgttctgcactgctgatgtactgatcaatcactgtttgggcaccgtttacaaagtcgccatactgtgcttcccataataccaggttattaggattagccatggcatagccatattcaaagcctaatacaccatattcgctcaataacgagttataaattctgaatttaccctggttttcctggaaatgactgagacggctatacgtttcattggtattttcatcaaacaacaccgcatgacggtgggagaatgtaccacgttttacgtcttccccgctcattcttacgtcttttccttcgatcaggaggctggcatatgccagcagttcaccggttgcccagtccaccttgccttcttcctggtagagttttattttgtcctgcagcagtttgctcactttacgcagtggcacaaagctttcaggccatttcatgaggccgtcgaacagccgtttaaaatcttcttctttaatagcggttaccggggaagcctcgaaatcctgcggagtggctttgcgcagggcctgccaccactgctccggtttctggcttacataaggcagcggatgttgttttacatcatccaggcgggcctgtaaatcgtcccagaagcctttttccatttctttggccagcgcctgtgcttcagactctccgttattcaggaggaactgggtatatacttcacgcggatttgcgtgtttttcaatcagggcgtagaggctcggctgtgtaaacttaggctcatcgccttcgttgtgaccatgtttgcggtagcaaaccatgtcgatgaacacatcttcgttaaattcctggcggtagcgggcagcgagctgggatactttcaccactgcttctgcatcgtcgccgtttacatggaataccggggcctgtacaatagatgcaacgctggtacagtagtctgacgagcgggcatcatcaaaatcggtggtaaagccgatctggttattgattacaaagtgaatggaaccacctacgtagtatcctttcagtttgctcatttgttccacttcatacacaatcccctggccggcaacggcagcgtcgccatgaatgaggatagggagtattttgtcgtaatcgctgttgtagatcacgtctgctttactgcgtgcaaaccccacaacgatcgggtccaccacttccaggtgggaagggttgggcatcagttgcaggttaacgggtttgccgccgggagtggttacctgtgagcggaagccgaggtgatatttcacgtcgccgctacccatggtcatatccggtacggcgaggccttcaaattcattgaagatctgttcgtaggttttacccaggatattggccagtacgtttaaacggccacggtgggccattcctatcacggattcctgtacgccatattctgcggctacgttaatgatcgcatccagcgccggaatggtggattctcctccttccaggccaaaacgcttctgtccgatatattttgtgtgaagaaacttttcaaaaataacgccctggttgagcttctgcaggatgcgtttgcgctgttccagcgacaatggttgcagcatgattgactcaaactccttctccatccacttcgctttatcgcggtcgttgatgtaagtgtattgaagtcctacggaaccggcgtagatctgctgcaggtaggcaacgatcttctccagggtggttttacccacgccaatggtggttccggcgtaaaattctgttttaagatcagcgtcccctaatccgaaactggcgaggtccaggttggccttgcggtcttttctttcacggatggggttggttttagcaattaaatggccttttttgcgatacgcctgtatcaggcggtacacgcccagttctttcgccagctggtcgtcgttcacaggcaacgaagtgctgccccctgctaccggcgctgttgttgccgccttgccgtttacgttggatactgcaaaatcaaatccttcgaaaaatttaacccaatccgggtctacagagttgggatctttgcggaaatcctggtataacgattcaatgtaagcaggatgtgagttagtgacgaatgagaagtccttcatttacaacgagttttgctgatcttcagttcaaatacttttctgttgatcccaatatattaatatatgggattgcaaatatcgctcgtttttcgatacgctggttggaaaaaatgagaaaaaatcaactgattatctgtgataaaaggtgcttatatttgtagctcaccggaaaaactagatttagtttgttttgtaaagggaatatagttacctttgccgtccgaaacttgaaatttgaaaaatggcaaaccataaagcaacaaagaaagacgtacgtcaaagcagaaagcgtaatgagcgtaaccgttactatggtaaaactacccgtaacgccatccgtgacctgaaagcagttaccgataaagcaacagcggagaaagatttaactgaggtagcttctatgcttgataagctggctaaacgtaacgttattcacaagaacaaagctgcaaatctgaaaagcaagctggctaagagagtattagctctggcttaattgcttcagtaacaatatttatagctcttcctcgaaaaggaagggctttttgtttttccattttatcaagacgatgaaaaagatactcctgctgctgaccgccctgttccccctgctctccactgcgcaggatttcaccacgcgatacgaaaaaaccaatggccgcgaaaccgccacttataccgaagtgatccggttttacgaacagctcgccaaacgtttcccgcaaatccatattcaaaccgttggcgccaccgatgccggattccccctgcacctggttacctactcccccggccggaatttcgactttaaaagccttcaccggcaaaataaacgggttatcctcatcaataacggtatccatcccggggaaccagatggcatagacgccagtatgatgctcctccgcgaccttgcacaggggaaaatccatctcccggaaaatattatacccgctgtaatcccggtgtataacatcggcggaatgctgaaccgctccccctggtaccgggtagaccagaacggacccgatgccttcgggtcccgcggcaatgcccagaacctggaccttaaccgtgacttcatcaaagccgattccaaaaacgccctcgccttccagcaaatctatcacctcactgatccggatgtatttgtggataatcatgtgagcaacggcgccgactatcagcatatcatgaccctgctcactacccagcacaataaactcggcggaccaatgggcgaattcatgaacaaaacatttgaacccggattatacgcccttatgaaaaataaaggctacgacctcgttccttatgtaaatcactttggtgaaacgcccgacagcggctgggtagaatttgccgacgctccccgctactccaccggctatactaccctcttccatacctttggttttgtaccggaaacacatatgctgaaaccctatccattacgcgtaaaggcaacttacgccctgatggaatgctttattagttttactgcgacccacagcgaagagattaaacacctgcgcgaacaggcaaagcaaactacccttacacaaaaaacatttccactcgcctgggagtttgatatgaacaaatacagcctgatcactttccgtggctttgcttccgggcacaaacccagtgatatttccggcctacccaggttgtattacgaccgctcgaaaccctacaccaggcaggtgaaattttataactacgccaacgaagaaaactttgtggaaaaaccgcaggcctatattattccgcaaggttggtgggcggtaattaacctgcttaaaaataaccaggtaaaaatgcagccactgcaacatgataccaccatcctcgtagaagtataccatattgccgacttccagagctacactaaaccgtttgaaaagcattatctgcacaccaatattaaagtaaccagcagcaaagattccatcaggttccgtaaaggagattactatattcccatgaaccagaacgccaaccgtttcctgatagaaacactggaacccaccggtggcgattcgttttttgcctggaacttctttgatgctgttctcggacaaaaagaaggatattctccctacgtttttgaagataccggcgcggaatatttaaaacaacatccggagctgcaggaattgttagctaagaaaaaagctaccgataccgcatttgcaaacagtgccagtgcacaactgaattttgtatttaaaaattcaccttatgcagagccggaatatatgcgttacccggtgtatagagtaagatagaatatttttgcagatagaagcggagatgtaagcagggcttatgtctccgctttttttatgcatgctgttcatgataatgaacggatcatttcacccctgaataaaatgaacgggtttttattggaacatactttaaattcgtgcccgtttaaatgtttgttatatacttcagcgaaaatgaagtgggcataatccttccattataaaaatcatatcgacatgaattttgcaattacttatgtggattaaacataggagccattgcttcgtttgtcaaacactttttcaatcatctttcagataaaattacccgtattctttaaacaaaaaaccataaacatgtcttacaaggaattcgtacaggatttaaaacaaaacattgtccggagcagatacattgctgcaagactcgcaaaccaggagcaattaaaactctatttcaaaattggacaaatgctttccgagaaaataaatgcggagaactggggagcaaaagtaatcgggcaactctctgcagatctacagcaggcgctacccggtttaaaaggtttttccacaaggaaccttaacaacatgaggcagttttacgagacttataagacttttctaattatgcagtcagtgactgcacaattagaaaaatccttctatagtattagctttacacatcatatccttataataaacagatgcagtaatcctgaagtgcaacgtttttatattgatcaggccgcggaacaattctggtcagtaagagaattagaacatcaaatcaacgccaaccttttcaaacaccagggtaatatgccccacaacttcaataaaacactgccggaaaatatcaaatccaaggcgctggaagtatttaaagacgaatacctcatcgactttattaatattaatgaagatgatgatgaaggcatccttgaaaacgaaatagtgaacaacatcaggaagtttattatgagtatgggaaaaggatattcctttattggcaatcaatataaactggaagtaaacaacaatgaattctttgtagatctgctcttctataaccggcacctgcaatgccttgtggcgattgaacttaaacgtaaaaagtttaaacctgagtatgcaggccagttgaacttttatctgaatgtactggatgacaaagtaaagctgccacatgaaaatcccagcatcggtattgtactctgcaaacagaaagacaatatggtggtagattatgctatcaaatctatcgataaagcgatgagtgtaggtacctatacacattatcaggccaatagtatacctgaaaacatgaaagaatttttacctgatgctgaagcactgggcaaaatgctataaaaatgataatgaacaactcattttaataattcccaaagtcactgtatcagttcccgtttacacgtttgttatcattctccatttacaacaaaatggctaacataaaaccattatcaaaatgaaatttaaccatctgcttaacagcattgaaaccacacatgtacatttccaggaagttgctgccaaagctattaatcgctcccttactatccgtaactggatgattggatgctatattgtagagtatgaacaaaaaggtgtggacagggccagatatggcgcgcaattattggaacagatttcaaaagaacttcctgtgctaaaattatctgcaactaatctgaggctatgcagacagttctatcagtattatcctcagataggtcaggttgtttcagacgaattaaaaaataatcccattcaaattcgtcagtcagtgactgacaaatttgaaaaaatcaacatgcgaattcatcagtcagtgactgatgaattacaaataactgaaaatcaacaatatacaattcgtcagacagtgtctgacgaattgggaacttcaaacaatccaattagcccttcggcaataaccccgatagaaattggcagcgtttcaggaaagaaaattgtaaataacctgtcgtttacacacattgccagtttgctcaccattgaagatgatttcaaacggactttttatgaagtagaatgcatcaaaggcaactggagcgtacgcgaattaaaaagacaaatcaacagcctctatttcgaacgcatgggccttgcaaaagatccgcacaaactttcccggctgatacagcaatcaacagaaagtccggtgacacccgcagatctcatcaaaaatgtatactcctttgaatttctcgatctcccgcaaaaagcaatagaaaaggaaagtacggtagaacaaaaactactggatcatttacaggaatttttactggagatgggacacggcttctgcctagaaggccggcagaaaaggatactgataggacaggaatattattttgtagacgttgtattttatcaccgtatcctcaaatgtcatgtgctgattgaattaaaagttggtgatttcacttatgcggacgccggacagctcacaacatacctgaattatttcaaagcaaaaatgactgcgcctggtgataatcctccaataggtattctgctggtcaccaataaagatgaggcactcgctgaatatgccattccttccggaatggatcagcagatgtttatttctacctacgccgtacaactgccgacgaaagagcagctacaacaattcctggcgggcgaattaagaagatgtgaaagttaaaccctttccagtttcagcatgatatgctgttccccgtaaaaatgattgtaaaaaagaagagaatgcacaggcgcagacaactgctccgtaccgcgaaaccaggccacgggtatttgctgcgcttggataatctgcgcggccaaccataatccgaacgccccggcggtgtcatattcaccgcaaagatgcttgaacggcaactgtggtatgccaggaaaacactgatccagttcctggtaaaaatgttcgtagttactgtcgccattacggccagtaatgatcaggtcaggaggagtggtaaaggctttcagtgcggcagacaatttctccccggttggtttgtacagcatcctgaagtcggcaatagacgcgtaactctgcggtgtaggcgtgcccgttagtgtgaagaaagtagcgccttctccggcaatgctgccgggggagagatgacggtacaattcccggttgtcggtgggctggtctttccagaaaccgatccggcttttgatataaaaatgttcttttgtaatttcttcgaatgcgccggtaagcgtatgcgtggcgccttcctgcaacagcatcatactgtccagcagagcattttcaaacgaaaaaccgcggtgtacaaaagtgttgttgtaagcagtgcacttttgctgcaatgcaattaatccattcacagaattgtaagtagattgaataaaaggagtgggattcagggctgtttccttgtattcggcaatctctttgataaacttttccgtgtcttgtaaactgcctttgccggtaccggtaacaatagggcctggtgtggtgataccactttcctggatgcatttaagtgcagcggtcagtcccattttaagcacccttgtcatacgacgcaggctgttgccgggaatgaatggcttataatcgggttcaatacaggcaagcagattactatctgtatgtgccagctgtgccgaaaaaatatccccttcaaaagttggctgcggggagatggccgccattgcttgtatgtaacacttacccttcatatttgctgatcaccagggaagcattgttgcccccaaagccgaatgagtttgaaataacatgatttaccgggtatccttccatcagggtggtaaccggactaatattcaattcctccattctttcagagaaattgagattgggaaatattatcccatgttgaatggccagtatggaatagatggcttctattgcgcctgctgcagccagtgtatgtcctgtaaaaggcttggtagaactgaacaggggcactttatcgccgaataaacgttccagtgcctttccttcggaaacatcgttattcagtgtggcagtgccgtgtacattgatataagatacttcttccagtgagcacccgctcatagcgagggccattttcatggcctcataggcgccgtcgccatccggtgaaggagacgtggggtggaatgcctcgttagtattacagtatccgcttagctctgccaggatgcgactgttgttggccctggcaaaagattcactttcaagtacaaggtaagccgcgccttcgcccaggttcaagccggtgcgttgctggtcaaagggacggcaaaactgcttatccacatttttcagggaattgaagccattcagtgtaaaacgggtaagcgcttcagtgccgccgcataccatccgtggtaacatccccagcttaatcatgcgtgcaccaaacatcagcgcgttggcagaagaggaacaggctgtgctgatggtagcaatatgttcactgaaccctacggtgtcggctatacgctgcgtgcaatccgcacaatccagcgtatctatatattgtaaaaaggaacctgttttttcaggattgataatgtcaaaatataacttctcggtatcgcacatacctcccacggtactggcgttaataaagcctgtaggggccgattgaacatccgtaatgccggcatcctgcaaagcttcccacatagctgccagtccgagtaaagtggtacgtgtatacccttcctttaccggtacaccggccaatgcaaacaaggcatcgctggcatgttttacttctgcaacaggcagcacatttttgtagatggtatcaatgtagttgctgtaacccagtccactttgctgtaaccgcagatggtgcaaatttccggctacattatcaccaatggcggtgatcattcctatccctgttataaacactctttccgccatgtagccagtttacttatgctggttgttttgattggataaactccgccatagactgaacagactgcaggatcttgcggccttcgcgcgggtcttctactttgatatgatactgtctttccagcaataccatcagttcaagcgaatcgatgctatccagacccaggccatctccaaataacggtgcattgtcatcaatgtcttccggtttggtatcctgaaggttgagcgcctcaatgatttgttctttcagtttcttttttaattcttccataatgttgtaggtttatcacctgttgttcacaacaggcgaatgcccttgtggggagtaaaaatacagttttactattgttttgaaaacatttatcagttcattcttcttttttccacccatccggctatggccagcatagcgagtccggtgagtattaatctcaatacatttttccacacaaacctgacatctccgttgcgaaggtaaatatcgttaatagcatcgagtccccagcttaaaggcgacaaatgccccagcagctgcatcctggcaggcatcacctccagcggaatccatatgccgccaatggccgacagtatcacgatagagattgccccgaagttcagcgcctggttaggtgttttaaataccgtgccaatcaggatgccataagcggttgcggccagccctattccaccggctaccagcagggtagcccccggatgctgtcccattaccagttgtggtaaatccagcagtggcagcacataaatgccgaccagcatcatcaggtaaaactgcaatacacaaacccctacaaaaaacagcatcttaccagccagtatagccaggtaagaccccggtatcagcttcatccgcagcaggctgccatcctccctttcacggatcatattgcctgcaatgggtatcacaataaagaacatcgcaaaaatgctccaggcaggtacgttatgctgaacagaattagaaattacatccagttgttttgccgtacccgtgctttgctccttcaaccctaccgcctgcaaacggatggccagcgtatcagcaggagcaaccgtgctgtctttactcttcagctgttgtttaatacggcttagcagcaaatctgtttccacctgtgtgaggaaattatctactgattgatgaatagcgcctttaaatgctttcttcgcggcggggtcgaaatagattgttacgtttaatgaatcaacggttttcttaaccggcagggataccgacatgcccattcgatgggtgatatcatttacaatgcggttggcattgctcacaatagcggctgtagcgcctgcgggtatgataatgctgatcttgtatttcccttcgttcaccagttgtttggcacgttcggctgttacaggctggccatcaagagaatcgattatattgaattgcccgccggaagccagtccttcttttacagaccggcccaaacggccgtggtcattatctactgttaagatatcgaacctgatatcctggtaatctttgaagggcgcgtcctggatcagcgccattactgtaatcaataccacaggcattacaaacagaaggatgatccctgttttatcacgtaacagcaattgccactctttcctgatggttgccagtagtcttaacatcgcttttggcccttcgcttttagctttaaaaaattaatcccggagtgcatttccggtgaaatgcaggaatacgtcttccaggttattacagtcaggatgctgatggatcagggtttgcgggttaccctgtacgatcatttttcctgcatccatgatcactacttcttcgcataacgattgcgcctcttccagcaaatgggatgtatacagtatactggctccctggctgttgtaatcgcgcaggaactgtaatatcatactgcgcgactgcacatccacgccggcagtaggttcatccagcaccagcagtttggggttgtggaggatggctgcaataatgttggcccgccgcttcataccgccggaatatttgtgaatttctttgtgtgcgcttttctccaggccgaacagctccaggtaatgcataattttttgttgcagtggctttcctttgaaaccgtagagattaccaaaataagtgagattttctacggcagatagttgtggatacaaggctatctgctgcggtacgatcccgataatatgtttgatttcctcccggtgggcggcctgctgttttaagtcgtgtatgattacttctccgctgtcgcctctcacaataccgcataatattgaaatcgtggtggttttacctgccccgttggggccgagtaaaccggcaatcttccccttcccgaactgaaacgtaagtcctttcagtgtgggctctgcactacccttgtaggttttatatagatcttttacagatatgccggacataattcaattggatatttaattaccacttcacctgtgccagcttgcggaagaatgcgtcttccgatgccgcgcactccagtaacatctggctcagctctttataggaaacattatccgccgatctgcttttgcatacgcggccggcggcaaatgcaaaattacgccataagtcgccggtttttgtcagttcccctgcaagtctgctcaattcatctttcttcagtaaaactgctgcttcctgtaaaaaagcggcgtacaggaaacggaaacctgcgccaccggtgccgatctcttcctgcatgcggataatatttccaagatacagggtagctttcctgtcgccgggattttcagcatagttggcgacccttttggcaaggaagcggattccttttacgccgaacatgggaataggcactttcagcataaagtggcaggcctgttctatgccggctttgatcggtttctcaaatgaggcagaaggcggtacgtgtaccgggtaatacatttttcctttaggggccggaaaccctttggcaaagcgggcctgcgccaggctttcggggtcaatggtggtggcggtatccattacgggatcgcttaccaggtattgtccgtcctgtttgccgtaaacaaccaggttatgtgcgttaaagtgaaaccggtaagaagctggaaagtagggcaggtaataaacactggattgtaatccaacgggaatacccgcttcaattactttatccagggcctgcattcctttttccggtgtagaaaatttttcggattccatccgtacgcccagccgtttgcacacccgttgaaaaatggcgcctggccatatccggtaagtggtgcctggcacgccgttcacctttacaaaaggcaggtggccgaaaaagatgcctgcaccaatgccaaaagccattggttcactgatctgcaaaccataatgtcccagcaggtttgatattactccactttcacaatgggcggtctggtggtgttggaaaaaagaattagtcataatattttttgtggcagcatgacgaataacggatttgtgggaagatcatcggatatcatctacccacaaatccgttactattggtatgctttatctgatgtgcagcagatctgttaaactcactttgaaggcatctgcataacgctgcagcagtttaggactgagctttttgaatacgccgggtttcatgtgtctttttacctgccactggaatttaccgacatagctggccaataatggcaggtccatcaggtttttttccatgtaataggcaacaggactgatttcgccggcttctaccctggcgcgcgccgcttttactctttcgtttacttcttcccaggcctggtccagagcaatgttttccggctcccagcctgcgctctgcacctgtacataattgccggaattatccaccgcatacataatctgcttgaatgtaccttcatgcaggttatcactatcctgtggtacttcctcttttttcatgatagcagttttagaagtgattgcttataccacggtgatatgtgcataagcatatgaaaaacgtgcactttccggaaccatcattactactttctgacctttcttaaaacggccgctgttcatcagttcttccagcatcaggtaaggtgatgcggtgcctacgtttcctacctcggccaggttggtgaaccatttttccagaggaataggaacgcctaaccgggtaatttcctcgtctatctttaacctgaaaaattcagacgacaggtgaggcaggaagaaatctatttcatcgagattaatctggtggcgctctaccagctctttccacatttgtgctccggaaggaacaatatttttaccgagtaaacgggtatcttgtttaaaggagaacacgctatgctgcgcccattcttccggggtcatatcaatccatccggtggtgctgccatccggttgcttgatagcgccggcatacatacatgtttccagctcattggcgtaggagagtatttctacccagtctacccgcagggataagccgtcttcattgggtttatcctggaaaagggctgcactggcgccgtctgataacatccagcggagaaagtccttttcaaaagcgatgatcggattttcgtcgaggcttttcagattttctgcttccggctggaatttctgcgccagcatccaggcggaaaacttttcagaaccggtacttacggcattggaagtattaccgcagcggatggacatccaggcgtatttaaaagcctgcattcctgccgcacaagcacctgtggccgcaatcagctctaccggctggcatttcaaaataccatgcaccatcgcagcatgattaggcaacagctgatcaggagaagtggtaccgcaggccagtaactgtaatttgctgatgggaaactgctcatcaaataattgtgacacggcagttgcggtcatctctgcattggaatgcgtggatttcccttctttgtccaaagagtagtaacgggttttgattttgttgttacccaatatcttcaaacgcgcacgggaagcctttccatctaccatgccgagaatgctctccatttcctcattttctacaggcttgttaggtaaaaatttagacagcctggtaatataaacttccttcatttgaatttattcgtcttttaaggctacatgtaaaacctggtcaaagctgccctgccttgccagccagctcacagtgaaaaacatattttaatttaatatacgttgtatacagacgtaaatatagaattctaattggaattacaagtatcacgccactgcctgaaggtcgctttatacacgctttatgtacggctttgatacgcctttaaggtggacttgatcctgttatctcagggaaatacccttataataatctacttcgcggcgcagcttagcctttttcagatttaactgtataagagaagtaatcagggatattggtgttaaaacaaaaatacctaccagcagtaatccccggtacatagatacgcgtccctgacgggaaggagctcccggaccgcctttagcgctgatgaactttgcccagaagcggaaggccttcattcctttattttccagtactaccaggttgggaatcagttctaccgcatccagcgacagcaattgtgcatgcagggtgtcccattgattcctttgcagcgcctcggctatcggtgccgcaaaccggccggaagtaatgatctcgttttcctgtactcctgcctggggcagaaagcgcgtggcttccttttttcctttaaacgcccagcgaaggatggtaattacagaaatgaggttaggtgatttatccaccagtacaatattgcccacaagggtgctgcctgcctgctgcaggtaatttttcaccttttcctgtgcattcagccacatattccggctgcccagcagggtaaccacctttttgcctttcagcaactgtttggcagcatcactttgcaggaaagcggcggttggttgtgaaggagaaagaaaccagggctgataagccagtatcaccaggtcgaattgcgcattcacgtccactttcaatggttcaataccacggggggtggattgaacggtttccggcatggtatcataaaattgctgtttcccccatgggaaagggaaaggcgttacaggcaccagttgctcaaaagtaatatcggctttgccttccagcggagccagcacatgatcaataatcctcttcaattgccctgtctgtgtataatataccaccaggatcttcggtctttcgttcataaaaggaataggagttcaacaattcaaaacgtaaatcaaacagttcaaatagtaaaatctacaattcaagccgtaaacatacaaaaaaacggcaatgattcatgtgatttaatgataatttgacgcgaattgttgatggggtgagggatttattaagggggtaatgtcttgtgccccagccaggtacagcatcagcgggataattaaagcgaatgctgtacctggactcaaggacttgatattgttttcttcaaaacatctctataaactctctaacgccgccaaatatgatattgagaatgttaaagatttgtaaatgttgaagcttattttttactaatactgccagaacccgctacagaagaggaaatttgcggggtacccttgtaatttacgtttccggagccggcaatttttgcatccagctttacgctggcatatacatctgcatcaccgctacccgcaatatttacacttacattttctgatagcagctcatctgcctcaaaattaccgctgcctgcaatagacaaattcacatcctttgtttcgcctttcaggaacatatcaccggaaccggcaatggaggcttttactgccggggcgttgatttcgcctttgaggttaccggagccggacaggttgaacttcacatcagatcgggaagtaaacttaccatccagtttcaggtcgccggagccagccaggctggcctcattgatttccggggtggtgaggaatacgttcagatctttatgggtgctgatggaaacgccgcgtttcaatcttacaatgaggcggccgtcttcttctaccagctccaccagtggggcgatattatcttctgcctcaataacagccgctttagcagcgccctgtgtgaggtatacattcatgcttccttctactttgatcctttgaaaggggactacctgccgttcttccttgataacatggccgttaccttttacacgattttgtccgattacatcacaggaataaaagagtacagaaacagaagaggccactatggcctgacataggagcgattttgctgatatcatgggtttaaattataatagaaagatacgccagatttccgaatttcgaatttccaaatccgaaattcgtggaaggactttatctttgcaccaccatgacagaaaagatacttatcctcgatttcggttcccagtatacacagctgattgcacgcagcatccgtgaactgaatgtttattgcgaaattaaaccttgccttcagcccattgcctgggacgaaactattaaaggtgttatattatcaggcagtcctttttcggtgaatgatgagcatgcgcctatcattgatattgccgcgattgctgcaaaagtacccgtactcggtatttgctacggcgcccaaatgatggccaaagtttttggcggtgaagtggctaaaagcaatctccgtgaatatggacgcgcctttatggagcacaacgacaaagaggaaaagttattatatgatatctctgcaaaaagccaggtatggatgagccatgcagatagcattaaacgtattcctgaagctttcgaaattattgccactacagaaaatatcccggtagcagctttcaaaaatactacgctggccgccaacccgatgtttggtttacaattccacccggaagtaacccattccctggaaggtaagctgatcctccgcaacttcctgttacacatctgtaactgcagccaggactggacaccggcggcttttgtacatgaaaccgtagaaaagatcaaggcgcaggtaggcgataaaagagtggtaatggctctcagcggcggtgtggactctaccgttgccgctgaactgattcataaagccatcggcaaaaacctgttctgcatctttgtggataatggtttgctgagaaaagacgaatttgaaaccgtactggaatcttataaacacatgggactgaacgtaaaagggatcaatgcaaaagatcttttttacggaaaactggcaggcgtttccgatccggaacaaaaacgaaagatcatcggtggcctgttcatcgatgttttccagcaggaagccactcaccttactgatatctctttcctgggccagggtaccatttaccccgatgtaattgaatccgtttccgtaaacggtccttccgttactatcaagtcgcaccacaacgtaggcgggctgccggaaaagatgaatatgcagttggtagaaccgctgcgcttcctctttaaagatgaagtacgccgcgtgggtcgtgaaattggcatcagcgaaatattcctgggccgccatcctttcccgggtcctggcctggccatccgtatcctcggcgccattacccccgaaaaggtacacatgctgcaggaagcggataatgtatatgtagaaggactgaaagaagccggcttatacgacaaagtatggcaggcgggcaccatcctgctgccggttcaaagcgttggcgtaatgggcgacgaacgtacctacgaattcacagtagctttacgtgcagtaacttctgtagacggaatgaccgccgattgggcgcatttgccttatgaattcctcgctaaaatgtctaacgacatcattaacaaggtaaaaggcattaaccgcgtagtatacgatatcagctccaagccacctgctaccattgagtgggaataaaaaaaggaagcaataaaatactgagctatagttacggagttgtggatagacagataatttcttctatccataactccgtaatgctttatttcacattccccggaatgatttttgtaaattagcgccaattatgaaccacttagtttcaattaagcacctgttatccggattggctttattggttttgatcagctcctgctcatctaccaggaaaagtgccagtaaggtagacgggccaccaccatctctgagtaaacctacaccggccaaaaaaccggaggataataagaaagacgctgcaaaagcgccttttaatgtgcccgcatttgggaaagaagttaaaaaagcttcctataacattgccttcttcgcaccattatacctcgattccgtttttgccaacagcagtgaaattcccggccgcaccatgccacggtatgtattgcctggtctcgaattttatgaaggcgcgcaactggcactggatacgctgcaacaacagggatataacctgaaagtgaccgtatatgacagcaaagcaaggcaaagtgtatcttccctgatccgcagcaaagcgctcgatgaaacggacctgatcctgggtgctgtgagcaacccggagctgaaagaactgagcgactttgccaaaaacaaagagatcaactttgtttccggtaccttccccaacgatggcggtatcagcaacaacccgtttttatacatctccaacagcacgctgaaaacacattgcgacgcgctccagaattatatccaggacgcatttgccactaaaaacattgtgttgttccgaaggaacacggcctttgaaacaaggctggcagcagatttcaaggcatcctatgataaaatggaaagtaccaaaaaatcaaggatccgggaagtagtatggaatgaggccaccacaccagaagaaatttccaaatacctgctggcagaccgtaccaatgctgtcatcgtaactgccctggatgaagccggcgccaaaagcctgctgcgtaagctgagcatttctgccactacctatccgctgcagatctttggtatgcccacctgggacgtgattaagctgaaagaacccgagtttaaaggcttacaggtattttattcatctccctattataacgacaaaacagattactacagccggtatgtttccgattatttccgcagggtatacaaagcacgcccgtctgacatggctttcaaaggctttgacctgacctactactttgtaaaactgctgtataccaatggcgtttatttcaacaatatggtgagtacttcccccaaagtgatcaccaactataacttccttccggtgtatctgaaagaaggagaggaaacgccttcttactttgaaaataaaaatatctacatcatccagaagggcgacagcgtagacattaaaatgaataaatagttgctttgcaacaccacttacttcgtgccacggcggttgtcgtggcacgattttttttacgtacattccctatatgaatgtgctgcaatttaccgacaacggcatctactgccctgcaggcgatttctacattgatccctggaaacccgtcaaacgagcggtgatcacgcatgcacattccgatcacgccaggtggggaaatcaatactacttatgtgaaaatgccagtgttcccttattgcggttaaggcttggcaacgacatccaggtacagggcgtcgactatggagaaaccattttttttaacggggtaaaagtatccctgcatcccgcaggccacatcattggctccgcacagatacgggtggaacaggatggagaagtatgggtagccagcggggattacaaactggaaaatgacggactgtcggcccccttcgaacctatccgctgccatacatttattaccgaatctaccttcggattacccatttaccgttgggcgccgcagcaacagatttttgatggcatcacccaatggatatacgaaaaccagcaggccggcaaagccagtgtactactggcttacagcctggggaaagcacaacggctgttatatcacctgaaagataaagtggatcatttcctggcgcatggcgccatcgccattccccatgaggtgctgttgcaggaaggctgggcgctacctcccgtagaaaggataacgcccgaaacacctaaaactgcgtttaagaatgcggtaattattgccccgccttcggcggaagataatgtctggatgcgcaggtttcagccatactcactgggtatttgcagtggctggatgcaggtgcgtggtaatatgcgccgcaggaatgcggatgcaggatttgtattgtcggatcatgcggattgggccggcttgctggaggcggtaaccgctaccggagcagaacaggtatatgccactcatggcttcagcagcgtatttgcccgttatcttacagaaaaaggtattgccgccaaagaagtaactacttcgtatggcgatgaggaaattattaataatcctgaatcgtaaaccgtgcaacaatttgctgaactggtacaattattaagcaacagcaccaaaaccaatgagaagttgggggcgctgagccaatactttgccacagcgccggataaagataaaacctgggtgctggcattgttttcaggtcgccggcccaaacgaacggtcaacagcacacaactgaaaacctggtgcatgcaggccacggggttgtccgactggctttttgaagaatgctatcatacggtgggagatctcggagaaaccatcgcgttgctgctgccaccacgcaccactcctatagcggcgcccctgcattactggctggagcagctgcagcaactggagaaagcaaccgaagaaacgaaacaggcttttattttgcaggcatgggatgcattggacagcggggaaaggtttgtattcaacaagctgatcaccggtggatttcgtataggcgtgtcgcagaaaatgatggtgaatgcactcgctaaaacgtaccagattgaacctgctacgctttcacatatgatcagcggcaactgggatccgcataatgttacgatcgaagaactgctgcatcaacatactaccggcgcagacgcttcccggccatatccattttatctcgcttacgcactggaaggattaccggaatcactggggccggaaacagactggcaggcggaatggaagtgggacggcatccgcgggcagatcatcaagcgggaaggacaactgtttgtatggtcgcggggagaagaactgatcactgaaaagttcccggagtttacgccattaactgccgctctaccggatggtactgtactggatggagaaatactcacctttgccaatggcctcccactaccctttcaaacactgcaaaccaggataggccgtaaaaatgtaacccgcaaacaactccaggaagcaccggttatattcctgtgttacgatctgttggaatgggaaggaaccgatatccgggaaaaaacgctggcagaacgccgtgccctcctggaagcgctggtgcagaatatgcagatgccggtattgcagttatcgcccgaaattatttttgacagctgggatcagttaacgcaactgcggctccaatcacgcgataaaggcagtgaaggactgatgctcaagaaaaagatagccgcttaccaggtaggccgcaaacgcggcgactggtggaagtggaaaatagatccactggtaatagatgccgtgatgatatatgcacagaaaggtcatggccgccgttcaaatttatatactgattacacttttgcagtaaaagatggcgatcaactggtagcctttaccaaagcctattccggcctgacagacaaagaaattgcggaagtggataactggatcaagcgccactctattgaaaaattcggaccggtaagaacggtgcagccgcagctggtatttgaaattgcctttgaaggcattgccgcctctaaccgccataaatccggtgtagccctgcgctttccacgtatcaaccggtggagaaaagataagccggtagcagaaataaatacgctcgaagacctgaaagaactattgcgggtgaacggccataacgccagcagctgattgattgcgccggtaaaataccagcagctgtataatcgccgccagtgcaatcatcgccagcatggttaatcctgcgccatagctgctccaaccctttattgcagccagctgcatcatcaatccgaccaaagataaacccaggccgccgcccaacgcatttgccgtaccattaatgccagaagcaagtccctgctgtggttcgggcaccgactgcaccgccaggatagttacgcacgggaaagtaatagccataccaaatgaattgatacagcctaccgcgcaaaaaataaacagcaacctataatccgtgaagtagctcccgataaaaaagagtatgccgcatgccataaaagcatttcccagcatgcctgtttttaccacgcccagcctgctaaacaaacggggtaatataaattttgaaatgacacctgataaaatactaaaggggaataacagcaggccggcctgtgaagaggtgaagtgcagatcctgttgcaggtagatggtgagcataaaaatatagcttagaaagatactacccagcattactgctcctatattcccggtgatcaccccctgtaacctgaacaatttaaagtctactaacggagacggatgtacgcgttcacggcgtataaaaaacataccggctgcgaggaacagtaataaccacaggcagtattctgtatagtggtgagtgatattgccaagatcgtggatcagccatgctgccagcatcatcagtccggtaatcaataatgcactgagtaagttatgtgctggttttgccgcggtcttttcatcggcgggaatatatgccatcgccagtatcactgccagtcctattaccggtacattaataaaaaatacccattgccacccgagataattgctgattaatccgccgatagcaagccccgtggcaaatccaatgcccgctgtagcgccaaaaattccgaatgcgcggtttcttgctaccggttctttaaaagtattggtaataatagccattgccgccggaatggctaacgccacacccgcgccttgcagtgccctgcataccagcagccaggtgaagttttgggaaaaacctgctgccagggaagccagcacaaaacagcaggcgcctgttacaaatactttctttcttcctatagtatctgccagccggccgccaagcaatacgagtcccccataaaataaaacatacacggtttgtacccattgaatggcagctgcatcaaaatgaaaaaatgattccatctgcggaatcgccatgttgagcacagatacatccaatgcttcaaagaagatagccatgcaggcaactgttaatatgattcgttcctttttcacggtacaaacgtattaaaacatctcaaaaggaatttaaatcctaaaaatttagaacaaacggctataatcacgcaataaattagatatttgttccaaacacatatgcacatggcaagcaaaaaagaaaataatacggaggacatacaattgaacctggatgagaaagacctgggcatcctgaagttattacagcaggatgcaaaaatgactatccgggatattgcccgtcagctgaacctcagcactactccggtgtacgagcggatccggaaaatggaacaggcaggcgttatcaaacaatatgcagccatcgtagatcccaggaagattaataagagcctcactgtgttatgttatatcaccctgaaagaacacaataaaaagtgcggtaagaaattcatccaggaaatactcggtttcacggaagtaacggagtgcctgaatatttcaggggagtttgacttcatgatcaaagtacaggtaaaagacatggatgagtaccgtgaattttacgtgaataaactgggtgagttagacaatctgagtcatacacaaagcatatttgtgatttccgtgattaaagcaacgcaccaggtagtgttttaacaccagcaaacgggttagggatcagcagtacacgataaaattgatacacaaaaaaatatatactgtaaccttataacttatttacccgttttaaacctatgaaatacctttacctatccctgttaatgtttgtaactgctgctgtcactgcccaaaagaaatcttttcaatctgctgccggaataggcggtattggtggctatcattacggcgccctggcttttagttttgagccccgatttaatttttatgaattttctgagaaggagagtttatcagttggcgcctgctttgcgatgggcccttccattggttctgaccggcgtactgatcgcgataagatttccggcggccctatacagccaggatggatggtgaatattcccgttaccgttcattatacttttggcaatgctgccactccccgtagctataaatatattgggtactctgttggggcaggctacgcagcgcacaatggccgccgctatgtggatccgggtcccggcatcgatacggtggaagtgcatgcgcatggcctggtgctggatggcagcatcaatttccctatgggtaattcctcatggagcctgcagtcttcctatatgtttaacttcagtaataacaatcctgacatcaaaggtatattcagcatgtcgttgctctataatatcggcatccgtatacatcagtacagggagaaacggcactacgaccaccccagggaatactatcacgaactggaccgggaaatgagaaagaaaaagatggagagccggcgaaaaattatggcgccacggggttcatcaaatcaaaacccgcgtgaaagtcgagatagcctgctgcagattcccccggatcaaaaacaactaccatagaacataccggcttcctgctgcgggagttggttgtttcaaaagcaatgccctgtttcttatcctcatacaccacaatttttcttgccttattagcagattcataggcctgtgctttttgaacacccggatatgcttttttgatggctgcaatgctgcttcctggtcccacgcctttacgggttctgaacttcggtgaatttacgcggatctgttttacgtactgcgtatcctgtgtgcgcatcgcggtaaatacggccagcatatgcgacgaatcgatactgtcgtcttttctgcggctgtaccatatccgccaggctttcatcatagcggcatcgccgccatccggtttccccaatactgccaggctctgtgccggtgcttcgagttttatttgtccgattgattttccgggtgtgatgagccaggcgcttttctgggcgaatgctgcggaggtagcggataagatggataagaaaatgataaggaggcgcatagttttcgtttgggaaatgagttcaaaaatgttgccattaatagtaacgttttttttggggaaaggttaaaaatgggaaagaagcatgggactttgaaacacacatcggtgtattagatgtgaatgctaaaagttatcagtaaaatgaccaaaaccaattccgaagtaacattatctgatgaatctattatgaccaaaatattgctcataagaaataaaagaataatgatcgataaagatcttgccgagttatactgtgtccccacaaaacgattgaatgaacaagtaaaacgtaatataaagcgctttcctgatgactttatgttccaactaacggaaagtgaaaaggaagaggtggtcgcaaaatgcgaccacctcaaaaacctgaaattttcatctaatctgccttatgcgtttactgaacatggtgcagtgatgctggcaagcattttgaacagtgacagagctatagcggtgaatatccaaatagtgcgcatctttacccggatgcgggaaatgatattaacaaacaaggacatattgttaaaactggaacagatggaaaagcgggtatctggccatgacgagcagatagcgttggtctttgaatatttaaagcaattgttagattccccacaagaaccgcgagtgcaaattggttttgcacgccataaataagagcaaagtatttttctgaaaatcttgaatagataggcggcccatctgttgtcaattcgggactcaccgcgccccgaattgataattgagactgcctcaacaaattgcaatattgtaacccaataatcacatctcctggtatccaatacggacaaaaaggaaatgccgtacctttacccccatgttactcaaatttcccaaagatcagaacgggcagcagatcctcaaagcaggcaatacccacttcgccatgttaaagcaaaggagtaaggctgataaacgcaccatattcctgacggaaaacgtgatgatatttgtattggcggggcataaactactgcatttcgaccagcataccgtaaaggtggaagcgggttccgtattgctgatgaaacgtgggttttacgtaatgtccgactatgtgagggaagaaatacaatttcaaagtttgctgttatatttttcagatgaacaactgcgcaggttcctccataaatacaattatcttacgcctgtaaaagctgctgtcaccaatcatcttaccttgcccatcaccccgctgctggaagttttcggggaacattataccgcctactttgcacaaacaccgtctacgctggcggcgctgttatcggtaaaactatacgaggcattccttctattactggccacgccgcaacatgcttccgtgctggcgtttatgcaacagattgtatatgcacagccgcaggacattgcctttattgtaaaacaacatctgtttcaacctattaccctggcagaaatggccaggttgtccggccgcagtctggcttccttcaagcgggatttccagcagcaataccagtcgtcgccccggcggtggatcaatgagcagcgactgtcctatgcacacatgctcctggaaaccactacacagcaggtagctgaaatagctattgcctgtggctttgaaagcacgtcccacttcattcgcatcttcaaacaaacttatagtatcacgcccaatcatgtaagagccaaaaaagctatcatctgagctttttccgttaccggcgatgcgtattcggggataattttgcatttataaaaagaagaatatgcaaacattatctgaaaagaataaggcagtggtaaaacgcttcaatgaagaattcctggtgaaaggcaacctgcaggcttttgaagaaatagtagcaccggactttattaaccatactgcacctgccggcagcaacgaccgtattgccacccgcgattttatcttacagttactacaccctgcgatgccggatcttcagctggaaatttttgatatgatagcggaagatgacaaagtagtaacccgcaaagcatttacaggcaccttcaccgcaccttttatgggacaggcgcccaccggcaaaaaagccaccctgcgtattattgatatcatacagctgaaagacgggcaatacattgcccactggtctatccgtgaaatgatcaccacataaattatttgctgaaatatgcttattttaagcgtatgaaccgcaaacactttttgtctgctcttattaccaccggcgcgggcctgccggcactgcaaacactcgccggcattgggttatctgctccttcagataagaaggaaccgcttgttcctccttatctgaaacccggtgatatcatcggcattacctgccccgcaggatatatcagcagggaggagatccagcccgcaatccggattatggaaagctggggttttaatattcgtataggcaaaaccgtgggcgaccgggactatagtttcggcggtaccgatgcggaacgactcgcggatttacaagccatgctgaatgatgatgatattaaggccattatgtgcggccggggtggttatggtaccgcacggattgtggacaaactcgacttctcccgctttcagcggaaacccaaatgggtgattggtttcagcgacgctaccgtattgcattgccatattagccggcactttggtatcgcttccctgcattcaaaaatgtgtaacagcttcccggacgatttcggaaaatcagaagccgttatccaggataccatcatgtctatctaccaggcgcttaccggcaaaaaaatgcaatacagcgccttaccggatacccgcaacaggaaaggaaaggcgagaggggtgctcaccggcggtaacctgtctattattcaaagtatgtcaggcaccaattcggaaattgacaccaacggaaagatcctgttcctggaagaggtgggcgaatacccgtatagccttgaccgcatgttaggcaccctgcagcgctcacataaactcgataatctcgcaggccttatcattggcggatttaacaggattaagccggatgatcccggtgaagaatttggcagaaccgtgtatgatatggtactggaaaaagtgaaagattttaacttccccgtgtgttttaatttccccgtaggacatcagaaaaataactatgcccttaaatgcggcatgatgcattccctctatgttggcgacgacacggttactttaaaggaataattactttacaagaaatgtaatgataaacaatacggccagtacatacatgaccgggctgatgcttttgtattgcccggttaatactttcagcaatacgtaagacaacataccaaacacaatgccttctgctatgctatagctgtatggcatcattacaatagccaggaatgcaggaattgcttctgttacatcattgaaattaattttggtgaccgctcccatcatcaacatccctacaatgatcaaagccggtgcagtggcagcttgtggaatcatagcaaaaacaggtgcaaagaaaagggagagcaggaacataacagctactgtaagcgccgttaaaccggttttaccaccggcggcaattccgctggcactttctacataagcggttactacgctggtccctaataagcctgccgccgtagtacccaccgcatctgccatcaaagcctgcttggcgcggggaagccggccctgctcatccagcaggcctgccttattacaaagaccaatcaacgttcccaccgtatcaaacaagtttaccattaacaaggtgaacaggatcatcaccatatccagggtgaatattttatcgaattgcagcttgaaggcgattggcgccagcgaaggcggcagacttaccaggtgaccattggccggcaaatgcgtgatgccaagcggaatacccactaccgtggcggccaggataccaatcagcaacgcggcattcacattccggtacatcagcaccgcgctgacgatgagtcctatcagcgctaccaggggcccgatgctggtcacatcgcccattttcagaatcacaccatccagctttccacctccgacatgatgcatccccgtttcaataatacctgcgttggccatgcctatcagcgcaatcaataacccgatacccactgaaatagcatgcttcaggttttccggtatgctgttgatgatcgcctcccggatcctgaacatcgacaaaaaaataaaaataatgccttccaggaaaaccgctgtaagcgcaaactgccagctgtagcccatagaagacacaatggtgtaggcgaaaaatgcgttcagtcccatccccggcgccacgccaataggcagcctggcatataatgccatcaccaatgtgccaatggcagcggccagggcagtggcggtaatcaacgcattaaaatccattcctgtacgcgacaggatactgggattaacggccaggatatacgccatggtggaaaaggtggttaaccctgccaatacttctttcttaacagtagtgtgatgttcggagagccggaaaaattttgcgagcatgatgcaaaaataagcgtttcacgatttatcattttatcctaatttcattcctatgcaacaacgttcgggtggatggaaagtgattaataattggttgggcgaaaaagaactgaagcccttcaaattccaggaggatgcctggaaggcttacctgcagggcaaatcaggaatcgtaaatgcacctacgggtttcgggaaaaccttctccctgttcctgggcgccgttatcgcctggatagatgcgcacccgaaagattatacccacaaaacaaaaaacgggttacagctattatggataacgccgttgcgcgcgttggccaaagacctgggccgggccatggaaagcgccctgcaggaactcaatgttccctggcaggtaggcatccgcagtggcgacacacccgttgccacgcgggcggcacaaaaaaagcaaatgccggaagtacttattattacaccggaaagcctgcacctgctgctggcgcagaaagaatacccttccgtatttaaatacctgcacaccgtggtggtagacgaatggcatgagctgataggcagtaaacgcggcgtaatggtggaattgggtctcagccggctgaggggactgcgacagcatcagctaaaagtctgggggatttccgctaccatcggcaacctcgaggaagcgctggaagtgttgctgggcccctatcatagcgatggccttattatccgcgccaaactgaaaaagaatattgccctgaaaagcgtgatcccccacgaaatagaaaattatccgtgggcagggcatctcggcatcaaaatgctgccacagtcgttacccattatcaacgacagtcaaaccaccctgatatttaccaatacccggtcgcagtcggagctgtggtaccaggcgcttctccgcgaagatcccatgctggcaggcgcactggctttgcaccatggctctatagatatggaactgcgtatatgggtggaagaagccctgcacaacggtatcctgaaagcggtggtatgtacggccagcctggacctcggggtggacttccggccggtagacagcgtaatacaggtgggcagcccgaaaggggtggcccgattcctgcaaagagccggccgtagcgggcatcagccgggagccatcagtaaaattttcttcctgcctacccatgccctggaactggtagaagcggcagcgctgaaagccgctatggaacaggatcttatagaaagccggatgccggtgctactcgcttatgatgtattactccaatacctcatgacgctggcggtatccgacggctttcatgccaatgaaatatgggaagaagtaagacataccttttgctatcagcatattaccgaagatgactggcagtggctcctctccttcctcaccaccggcggcgaggcgctgggcagttatgatgaattcaaaaaagtagagcgggaaggcaacttctacatctgccgcagccggatgatggccatgcgtcaccgtttacatataggcaccattgtaagcgacgcgatgctcaaagtgaagttcatgagcggaggctacatcggtgtcatcgaagagggtttcatttcccgcctgtcgcccggcgattcctttaccctggctggccgcaacctggaatttgtcctgatcaaagatatgacggtactggtccgcaaatcaaattcaaaaagatcgattgtgcccagctaccagggcggccgtattccactttcttccaacctgggacggatgctgcgcgaaaaatttaatgaggcgctttcgcgtaatacaaaagatccggagctgattgccttacaaccactgttcaacctccaggaagaactgtcgcatattccaaaagccaatgaactgttgattgaacagatagccaccaaagatggttaccaccttttcgtgtatcctttcgaagggcggttggtgcatgaagtaatggcggcgctgctggcttaccggatcagccgtattcagcccattactttttctatcgccatgaatgactatggttttgagttgttgtctgatcagcctattccgctgacagccgaaaacgccaaacagcttttttctaccgaaaacctgctgatggagctgcaaaccagtgtaaactctactgagatggcccggcgaaaattccgcgacattgcggtgatagccggtttgatattccaggggtatcccggtaaacacaaggctaaccgtcacctgcaatcgtcggcttcgttgttgtttaacgtgttcaaagactacgatccgcaaaacctgctgctaaagcaggctttcaacgaagcgttcttttaccagatggaagaggcccgtttgagggaaacgctggaacgcattgccgttagcaggatcgtgatcaccacaccacaaaagctcacgcctttctgcttcccgattaaagtagacagtttacgtgacaccatgaccagcgaaaagctggaagaccggatcaaaaaattgatcacggtgaacggttaagaaatctctaatttgcacctcattaaaaaacagttgatccagtggttgcggaaatatttcactttcaggaacagcattggcatttatcacctcagcgggcaattttctgggaagaagaaaaagcgctgatcctttcagatctgcatctggggaaggcggctcatttccggaaggcagggattgccgtgccggcgggtattgtacaggaagacctgttccggctacagcaactgattacccattacctgccagacaggattatcatagtgggagatatgtttcatagccgggagaacaatgaagtgcagtattttaaattatggcggcagcagttttccaggatctccttcgacctggtgaaaggtaatcatgatattatggctgatgcggtgtatgagcagctgcagatcaatgtacaccctgcacttactttgcgtaatattcattttatccatgagccttgtgaagacaacaatggcttcgcctatactttttccggacacctgcacccggctttcgtgatgcatggagccggcaggcaacggctgcgtttaccatgcttttattttggccggcattgcggcattttacccgcttttggccactttaccggctcagcgaaccttgaccccgaggaaagggatcctgtgtttgtaatagccggaaaatcgattatacgcgcccaatgaagattgccagtcacgatatatatacgcatcctttgccggcagatcatcgtttcccgatgctcaagtatgaactgataccagcacagctgctgcgggaaggcattatcaccccctggcagttattcgctcccgaaccggttacagaagaaactattcttttaacacatactgttgagtactggcataagctgagagaccaaacgctggacccccgggaacagcggaaaataggcttcccccaatcgcctgcgcttaccctgcgcgagatggtgattacacagggcaccatcgatatttcgctgcatgcgctcgatcatggtattggttttaatgtagctggcggcacccaccacgcgtttgcggatcatggggaaggtttctgcctgctcaacgattttgctgtagctgccaattacctgctgcaccggcaacgtatcaaacaggcactggtgatagacctcgacgtgcaccagggcaacggcaccgccgcactgtttgctggtaaccctcatgtatatacgtttagtatgcatggcgcacacaattatccatttcataaagaaacatccgactgggatattcccctggcagacggtatggataacggcacttacctgcagctgctggaagaagccctgccagtgctgattaaccgggttaaaccggatcttgttttttatctttcgggggtagatatcctggaaacggataaattcgggaagctgaaggttacgcagcagggctgcctggagcgggatgaaatggttttccattcactgaaaaaacatcacatcccctgtgcagtggcgatgggaggaggttattccacccacatccgcgatatcgtaaatgcgcactgtaatacttttaaggcaggcatccgtatttacggttaaataattttcccgtctttcattaccagctggcggtcgctcatgggcgccagttcttcattatgcgtaacaatgataaaggtttgcttcagtttatcgcgcagttccatgaacaggtgatgcagttcccgcgcgttacgggagtcgaggttaccggtaggttcgtctgccattaccacgtcgggatcattgatgagggcgcgcgctacagccactctttgttgttctccgccggagagggcgttgggtttgtgctcaagccggtctttcaatccgagcgtttccaggaggaacaccgctttttcctttacctggcttttgcgggtgccggcgatataaccggggatacacacattttcgagggcagtgaattccggcagcaggtgatggaactggaaaataaagccaatatgacggttcctgaaatcggccagggcgtttccctttaaaccggtcagattgacatcattaagccagatactgccagcagtaggcgtatcaagggttccaagaatgtgcagcaaggtactcttaccagctccggaggaacctacgatggttacaatctctcccttactgacagtaatgtctaccccttttaatatgggtaaattggaataatttttggtaacattgcgagcggttagcataacccaaagaaaagtaattaaccgataaaatagtaaaagttgtttatttcaaattaaataatacttttgcggaaaattaaaaagtaaaaattttaataagatgtactggacattagaattagcttcatacctggaggacgctccatggccagctactaaagacgaacttatcgactacgccattcgttccggtgcaccgatcgaagtaatcgagaaccttcaggagctggaggatgaaggggaaatttatgaggggattgaagatatttggtctgattatccgtcgcaggatgacttcttctttaatgaggatgaatattagccagtatcgctgaccgcactcccgttcaactatgacaaataattactaagccgctcctgataaggaagcggcttttatttttggtattcagagatccggcgatgtggcagaaatgattgtttctgctgcatcgccgggctcaataaataactggtttatttttccatctggtcgatcaccggtttggaaacgccggtgaaggagaaacctccgtcgtggaacaggttctgcatggtcaccattttggtgaggtcagagaacatggctacagcgtagttagcgcattcgtctgcagtggcattacccagcgggctcattttctctgcataggacataaagccatcgaaacctttcacaccgccacctgcggttgttttaaccggtgactgggagatggtgttcacacgtacttttttgtgggtaccgtaatggtaaccgaagctgcgtgcaattgattccagcagggcttttgcgtcggccatttcaccataatcggggaatacacgctgagacgcgatataagacaatgcgataacagatgcccattcgttcagtgcatccagcttgtaggctgtttgcagcacgcggtgcaaagacatcgcagagatatcaaatgttttgtgattaaaatcgtaatccaggtcggtatagcttctgcctttacggatgttcatacccattgctacggagtggagaacgaagtcgatcttaccaccaaagtgctccatggatttgttgaacaggttggccagatcatccatattggtaacatcagccggaataacaggtgccttacaggtttccgccagtttgttgatctcacccatacgcagggcaataggggcattggtaagcacaatttcagcgccttcttccacgcaacgcagtgcagttctccaggcaatagacttgtcgtccagtgcgccaaagatgatacctttcttcccttttaataagttatgagccatttggtcaaaaattaatttcggcaaaaatagtcgttatagttgaaaaaaaaagctgttagctgtcagcgaccagcatttagacggttagtctttaactaaatgcagcctgctaaaggctaacagctattatgagatagcagtttattaatgtacggccagcatttcgcgggcgttctccagcgcagcggcagtaggccgttctccactcagcatctgggcaattttattcacccgctcgtcctgcgacaataaacgtacgctggtagttactttatccgctttagcgtctttatatacaaagtaatgtgcatctgctttcccggctatctgtggctgatgggtaatacagatgatctggtgtgatttggccagatctttcagaataacacccacctggcgggcagcttctcctgaaataccggtatcaatttcatcaaagatcagggtaggcagcgctaccgactgggctaccagcgacttgatgcataacatgatgcggctcaattccccaccggaggccactttgcccactggtgcaaactggttgctcttattagcgtcaaacaggaattcgatggtatcctgtccgtatgaattgagttctccgggtatgatgtctactttcaggcgggcgttaggcatgcctacctgcgccagtaaagtgtttacatgtttttcaaaaggaccggcctgctcctggcgatgcccggtgatgactgcggccgcttgctgcaggctttctttcagccgggtttgttcctgctccagtgatgccagctgttcgtccaggttcagtacatcctctactttctgtgtcagcacttcttttatggccagcagttcggcagtggtatgcaccccatgtttcttgaacaaacggtaacccagcgccattctttcattcaccagttctatccgttgcgcatcatattgtacatggtcgttgatgctttccacctcaccggcaatatcctgcagttcgagataagtggacaatagccgttcagataccgcgggcatctctttatggaaggcagataaggcctgcagcgatgactgcagctgtttcagctgttgaagaatgggttgttcatcttccttcagctggaaataaacccggttcagggtgttctttatttcttctgcgtgactcaatgtttgcagttctgcttccagttcttctatttcgttggtgttgaagcctgcttccgccagttcatcaagcaggaagcggttatagtccagctctttgttggcattgtcgcggttatccagcagctgtttgtatttcttctgtacctgtgtgtactgaacaaatccctggtggtactgttgcagttccgttggtttgtttaccagggcatcgatcacttcgcgctggaaatcggcgttaccgagcgccagtgtatcaaattgttgatggaggtctaccaggtatccgctgagttctgccagctgggagatgttcaccggcgtatcatttacaaacgcccttgatttaccggcagcactcacttctcttcttatgatcagctgatcttccagatccagctcatgttgctggaagaaggccgccacctgtgatttctttactttaaagaacccttctatgatgcatttgccggttttatcgaacaatactcccgggtctgctctttctccgagtatcagggaaagggctccgaggaggatagatttacctgcaccggtttctccggtgatcacattcaggttccctgagaagtctacttccaggtgatcgataattgcgtagttcttgatggttagtcgctgtaacataagtaaggaaattcctttatgatgttgaaagctcaggttccgtttacccgctgcatgcctgctttggcgcgctggtcaagggaattcttataatcgtggcctttcatgttcagacaacgctgataacattctatggctttggctttttcgtttctcttttcataaatgtaacccatttggagggaagcccgtgcagcataatattccggcctgttggtgcccactttcacggttacctcgtacatggcaatggcctgatcatcctgcccgctttcatcatatatgcggcccaaacggtaggcatattccagcttatcttccatcgcagggaattcagccgcttttttggtaagcagcaatgccagcgctttattgaaatatccgccatcgctcagtaaacgtacgcgcaacaggaatgggttgggccatttaccggttttggcttctttcagtgcctgtttgtcggcgtccgtttccagtcctccttttgtgaggatcagggcgcggtatttatctgccgcagcctggtttccttccaggtaataataccagctgagtcgctgcaaacactccttcacataaaacttgcctttaaaattactgacaaaccgctccaggtaaatatgtgcatccggatccagccgtgttaatttcagtaatcccattacataattgtaatactgcatgtccgcatactccgctgtatcattccgttcctgcaacacttttatgccggtagctgccctttggttgtttaaagaaaggttcgccaccattaaagcaaacaggtagttatttttagtatccagttgttttttttgtaagaattcccacgtttcttccggtttattcacaataaacaacatcaggtagcaataatagtagtaagattcttcccggaacattctggcttcgggcgcattgctctcaatgaacttattcacatttgccatcccttctttcatactgcccttaaggccaaggatattggtgatccacttatagccttccggaatagtgccgaatacggtttgcatggcgcccagcagcaggttgttgggaacaaagcccggaaaccgttgctgattttctttcagcatgatatatgctttccggatctcccaggtcgcatcccatttttcatcaaactttattttgatcagggcccactggaatttgatggccgcctgtgtgtacaggtaataaggcgagtccggggaaccttctgccattttattcagccggaaggaacgcaggctccttttctttgaatactctgcagggtcttcattaaagaagagtgggaaaaaatctgcatagttatccaggaaatagggcgccagattatccggatgctcttttttttctgcttccagcaaagccttaccggtgtttaacctcagctgcataatggcatcatatgcctgctcgcagcgggtgttaaaatcaaatactttctgcctggcgctcacgttaaatcctacactcaacaataacaacaaagaaaaaataatacgcatacggggaaaaattccaaaattaaaggccaaatctctcataacatcctccaaatcccaaataacacttcacattttttaaagttgcattgttttagctaaatccctgccacaaaataaaagaactactacgcaaggtacctgcgcaacggcaatatacacaaagctaatataattagtaaaacaaaactaaataaattagtatatttttttatgcacatacaccaatagaaaaaggacatccggagatgtccttttaaatacttattgctgagggactatattttagatagtcacagtcgcttcgagatcgttatccaccaggatacgtccgcagtgctcacaaacgatgatctttttgtgctgacggatttctgcctgacgctgaggagggatcgcattaaagcaaccaccgcaggaatcacgctctacagttactacagccaaaccgttgcggtagttcttacggattttttcgtaagcctgcaataagcggggatctaccttggttttagcatcttcactttctttgcggaatgctctctcttctttatctgtttcgccgatgatcttttccagttcgcctttcttgtgcttcaggttcgcttccttatctgccaccgctttcttggctacttccagtacgcggcttttttccttgatctcttcgttagcgtccttgatatgcttttcagccagcttgatttccagcgcctgcatctccatttctttggtgatggcttcaaactcacggttattcttcacattatcctgctgcttctcgtacttcttgatcagcgcttccgcttctttgatggcgtttttcttgctggcaacaaagtcttgtatacctttcatttcattctcaatgtgagactgacgtgtgttcaggccttcgatctcgtcttccaggtcttttacctccatcggcaactcccctttcaacacctggatcccatccagcttggaatcgatcttttgcaatctgagtacagacgctaatttttcttcaacggagtattcttttacggttgccatgtattataaataatttaccgggtttgttttaatcgtagatttaagaggcgcaaaattacggaatttttcggtcaatatatgataaaataattccactgtgaactgctcactctcaaaatgtccgatatctgctataattaattgattgtcagcgtcaaaaaattcatgatacttgaaatcagccgaaatataggcatctgccccggccgatattgcctgtttcaacaggaaactgcccgctccaccacacaacgccactttttttacgggacgccctctcaaaggagtatatttcacacaaccagtccggaactgctcctttacaaactgtaaaaattccagctcttccattgcctccggcaaagtacctatcaatcccgaacccacctgctgataagcattttccaggcttactatgtcataagccacctcttcgtagggatggctgctcaacagcgcctgtaaaatttttccttccaaatataccggaaaaattacttccaactttatttcggcctcaaaatgtcgttttccgggcgtacctacgtaaggatcagtgccttccgcccctttaaacgtgccttcccccgcgccgttgaagctgcattcactgtaattgccaatatggccggcgcccgcttcaaacaaggcagcccttaccgtttccacatctgccgaaggcacaaatgtgaataacttttttaataatccccgcttaggctgcaatacccgcgtttgctccagccccagtttagccgccatctgcgcacataccccgttccgtacattatccaggttggtatgcgctgcatacacggcaatatcatgtttaatggctttaatagccacccgttctacataattattcccattaatcttcttcaatcccccgaaaacaatgggatggtgggcaatcaccaggttacatccggttgcaatggcttcgtcaataacagcttcagtggcgtccagggtaagcagggcgttggtcacctccacatctgcccgcccgaaaataagcccggcattgtcgtagctctcctggtactgcaaaggcgcgaactgttcgatggcctgtatgatctcttttatcttcatatctgcaaaaattaatggttcattcccggcatctgctaaatttgcaaaaaaatatcttttatgcccggaagcaaatctacagcagaacagtatgcggattacaaaataaaaatgcaaaaaattgcggacgtaagaaatgccctggcggtacttggatgggaccaggaaacctatcttccggaaaaaggcgcgggattccgcggtcagcagatcaccaccctcagctccatagctcacgaattattcaccgccccggaactggaagccatcctccaggccctgaaagggaataccacactgaatcctgtagaacagaaaaatatcattctttccacagaagactttgaaaagaataaaaaatacccggcagcctttgtggcagaaatgtcgagagtgaccaacgaaagctatcacgcctggataaaagcccgcaaagccaacgactattccattttcgccccggcgctcgcccggatggttgaactgaaaaaacaggaaacggatatcctcggctatgaaggacatccctacaacgccctcctgaatgaatatgaaaaaggcgcccataccggtatgctggataccattttcaatgaagtgaaaaccgccctttcaccactgctcagccaaatagaacaacaacccgctatcaataaggatttccttcatctgcattataaccgcgatgtacaatggaaatttggcctcgccctgctggaaggtatgggatacgacctgaaagcaggccggcaggacgtttcagaacatcctttcaccaccagcttcagtccacttgatgtaagggtaaccacccgcatcgatgaaaatgattttggtaacatgacctggagctgtatccacgaaggtggccatgccctttacgagcaggggctccctacagaacaatacggccttccctgcggagaagccaccagccttggcatacatgaatcccagtcgcgcctctgggaaaacaacgtgggccgtagccttcttttctggcaatatcactatcccagcctgcagcaactcttccccgaaaacctcggaaacgtgtcgctggatgcgttctataaagccattaataaagtgcagccttccctcatccgcacggaagcagatgagctcacctatcatttccacatcatgatccggtatgaaattgaaaaaggactgatcgatggcagcattgatgtaaaagatctgaaacacacctggaatgaatactaccgtcaatacctgcacgtaacggtacccgacgatgttcatggcgtattgcaggacatccattggtcgcacggcagcttcggctacttccctacctattcactcggcagtttttatgccgcccagctttttgctgctgcacaaaaacaagtacctggtttggacgcacgtattgccggcggtgattaccagccgttactggaatggctgcgcaccaacgttcacccgtttggaagattttatacctcaaatgaattgtgcgagaaagtaaccgggaaacaactggtatttggcgagttcctggaatacgcgaaagcgaaatatgccgggatatacggtttctaaaataaaagtccggaacgatctgtgaaagatggttccggactttcctgttacttgtagtatacttcgattacaaccccgccagcttctccagctctgccagctccatcacaccctgcttccgcgctatttctttaccatccttataaaaaataaaagtaggcagcttagttgcatcaacagatttcattacgtcctggtcgttaccgccatctaccaataccctctttacctgcggatgtttttggaagaatttttccagcaccggctccatctgcttacagggaggacaccacgcagctccaacatcggtaagtaccattccttttgcatgaacggcgttgttataatccgctatagtaagctgcggcttcttttcagcgacgccctccaattgtttgcctgcccgcttccacgcattgatgccgccatccagctccactacctccgtaaaaccatgctctctcatccatttggcggcggcggtgctgcggccgccgctcaggcaataaatataaacggtctttttcttgtccaggtactgcacccggtccatgaattcttctttctttgtataatcggcctgtaaggcatgcggcaaatgcccggtactgaattccccggcggtacgcacatcaaacacctgtgcatccggctgttgaatatccttttcaaattccgcggcatccacttcctgccgctcctgtgccattacggtaatgcctgtgagcatcaataagatggctaagaaaactcgtcccatatcttctttattttcggcataaaattaataaacaactctgcaccttgcctggccggatgagaattataacagggctgtaacgtttttatatcaaataagtgagaaaacaacttggtgtattccgctgctgtaccaccgaagggcggcccgtcctgcgtaaaatgacggttaaataacacccctgccaggtgcccgccaggtttgatcagcgaatacatgtggtccacgtaatccatccggaggaaaggaggcaacgcgcagaaaaatgtttgttccaataccaggtcgtaactgcctttatgcgcaaaaaaatcttcttccagcactttcacacgggtacgggcaaacgtttttttcagttgttccaccaatgccggtgcaatatccagcaccgttacatcgctgaaagcctggcctgccaggtaagcagcctcgtaactgttgcctccaccgggaatgagtatacgaatatcccggtccaccagctgatcaatatactctttcaggggtggcgacaccgctcccatatcccagcccgtatctcctttcagatagcggtcattccaatactgactatccatatccggcattgctttttatgctaagttacggccattcagccacatacataaatgcatcgcttttccaaacattattactatttttatgctttgaatatacctgtgaaaaggccttaacgccaacctatgccatgaaaagcctacacaattatttgtggattgtcacaaaacatattttgctttgtctgctgccggtgatggccctggccgttgctgcccgtgcgcagtcagttgccatcaatgcagataaattagcaggctgtcctcctttcctggtgaactttaccgccacattagatgcaggctaccaacagatagaatgggatttcggacttggcgccaatgtgaccaacgacctcaccccctccaaaacattccaggaccccggcatttaccatgttaaactaacggctacctacggcgccaataccatcgtcaaacaacttgacatccaggtatataacaaaccccttgtcaacttcactatccccaacaccaccggatgcgcgcccttcatggctactttcagggaccagtctgccccgggagacggcagcattgcagatattacctgggatttcggcgacggcggaggcgccacaggcgcaaatgttacacacacctatacgcaggcaggcacttataatgtactcagcgctgtaactaacagctacggatgtacggcatttaaaggacccgaaccagtgaaaatacaaagtgcgcctacgccggctttctcggccgacaaaacacaaagctgcaccacgccattcatggtaaatttctttaacaatacggtgaataactcgcccgatccggtgacctatacctgggattacggcgatggcactaccggcaccgccaaccagcatacctataccagggaaggccgtttcaccgtaaagctcaccgccactacctccggtggatgctccactcctcttactaaaacagcgtatatcgtcattgaaaaagtgaaaccagcgtttactttttcagcaccctgtgctgatcaaccggttaacttcaccaataccacacaacctgttccggaccaggtgacctgggcattcccggatggcactactcaaaccactgcaaacgcggtaaaacaatttgccacgccgggcgactatgtcgtgaaaatgcaggctaccctcggtacctgcatggaagagatccagcaaacgattcacgtaaatccctctccacaaattaacccggtagctacgccactcagcgcatgcaatacgccttttaccacgcagttcaacgcgcaatccgccaacgctactgcatggaactggaactttggagacggcactactgctacgctcgaaaacccttcacatacctatacccgcgaaggatcattcacggtaagtctcaccgccaccaatgcttcgggctgcaataaaacagtcaccaatcctggttacatcaacattgccaaacccaacctgagtatttatcgcagcgcaacgaaaggatgtatccctttgccggcagacttctacgtagaactggatgttaccgatcctattgtcagttatcaatggaacttcggcgacggcagcacttctaccgatgcaaggccccatcatattttcaccacacagggaactttcacggttaccattaccgtaaccacagcaggcggatgtactgccagcggcactaccattgttatggcaggaacaagaccagtagtggattttgttgccacccccctgaaatcatgcgctaaagacccggtacagttcaccaacctgtctgttccccgtggtacttcctggatctggacatttgtacaggataacagcaccagtacggaagaaaaccccaaccacaccttcaacgaaatcggcagtcatgatatcattctcacagtaaacaataatggctgtattgagcagttaataaaacggaattatatccagatcattccacctattgcacggtttgaaactgcaccggattgcttggatccctatcaccgtaaattcacggacaattccacctttgggcctattcccaccgcagtaaaatcctggctttgggaatttggcgaaaacggcgctacttccaccgatcagcatccggatttccggtaccagacaacaggtctgaaacaggtacggctcaccatcgacaatggtatctgtacttctaccactacgcaatcggtgaacatcattgatgaaaagcccgttattactgctgataagcccaggatatgcaaaggagaaaacatccacatttcattaggaccgctgaataatgccaatatcaacgaatataactgggattggggcgacggcagcgccattcaaaatataccggcttacaattttaatcctgccaatggtatcacacatacctataacaaaacaggcacctttaccattaagcttaccattacagataaaaacagctgtatccgcgaagccccaccctttagcattgatgtaaacggggctacacctgattttgattataccggcaagagatgtaaagatgagattttcagcttcacggataagtctaccgtaaacagcggcaacagcatactcaactgggaatgggatttcggggatcagagcagcaaagagaattatactacacaacccattgacataaaacatacctatactaacgcgaacgattacacggtatcattaaccgtcaccgatcagtttagttgtgtagtgaaaatccagaaagtgattcgtttcgaccgggtgaaggccgactttatggtaccatccaatatcgcttgcctggataagtcgtttacatttatggatcagtcgcagggtactatccaaaactacgcatgggatttcggcgacaataccaccggcacgggaaacagacctgtaaaggtttacagcgcccctggccaatataacgtaacactcaaagtaaccacccccgcgggttgtacggatgaaatcaccaaaacaaatgccatcagggttcctgatccgaaagcatctttcacgataccggataacctggacctgtgcccgccggtgaaagtattatttaccaatacgtctactgattttgtaaactccagctggaattttggtgataacggcacttccgccaaaaatgatcccgatgtgcatatatacgcacgggcacgcacctacgacgtagtgctcactgtatattcagaaggaggttgctccagcactgccacgcttcctattaccatcaaaggaccggacggcaccatgaaaaccacgcctacacagggttgtgtgccgctggcaatcagtatcagcgctacctctgttaaaaccgacagctatatgtgggacttcgatgatggtaccgtacttacttctaccacaccggtatccccggcacacacctataccaaggcaggcatatattatccgcgtgtatctttactggacaatcagggttgcgtggtaaaagcggcaggcaacgataagattattgtagatcaaacaatagctgattttgctaccaatgatttccaggtatgtggcggtggtgaagtaacttttaccaacaagagtaaaacgttaaccaaagattcacttgcacttgatttcaccaatgcctgggactttggcgcaccgggtaatcccggcaacagcgctgccaccgtgaacggcttgtttaattatccgcagcctggaactactcatgttaaactggtagtaaccagcgcctatggttgtatagatgagaagatcctgccggtggtaattccgccgcaaccggtggccgtcattgctcctgttttaccgctttgtgtgtctggcaaggtacagctgtccggcagcgacagcaaaaatataccaggcaccaagtggcactggcagataggaaccgggcaaacatacgacgtacctgttccgccggaaatacttttaaacagcaccggcaccataccggtggtattaacgatcaccaacagtgatggttcctgtccttcagaaactactattcagatgatcgtacatccttcaccggtattaaatccttctccggtttcggccactatctgccgtggtgcggcattacagttacaggcgaataccaccgccaatgtagcagtaaactggactgattacaacatctccgacgtaaccagcgtatcgccgcaggcaatgccggatatcgataccttctaccgggttaccgccactaacgaatacggttgtacgaatactggtgaaatagccgttaccgttacgcagccgttcaaaatttacgcgcaggatgccgaaatatgtgcgggagaaagcgtaaaaatgaatgcaggcggtgccttacgctaccagtggattcccgccaggggcttgaaccacgcggatattgccgatcccgttgccagtccggatggcaatatcacttaccaggtagtgggttataacaacagcacctgcttcacagatactgcgttagcaagagtttacgtacgtgcggtaccggtagtgaatgccggtccggatatggtgatagctaccggctctgttattccattgccggtaacaggcagcggcgatattattaaaactgaatggacgccggtaactggtttgagctgttacgactgcctgacgcctacggccacgcccacagacgatattacttaccatgtaaaggtaaccaaccagtttggctgtgtaagtaccgacgatgtagctatcaagctggtgtgcgatgaaggtaatgtattcatccccaatacattttctcccaatggcgatggacagaatgatgttttctatgtgcggggccgcggtatgcagtccatccgcattttcaggatcttcaaccgctggggacaactggtatttgaacgtaccggagtgaataccaatgatccatcctcgggatgggatggccgttacaaaggcgccatcctgaacccggatgtatttgtatactatgtggaagtagtgtgtgacaaaggtgctgtaaacctgttgaaagggaatattacccttatcaggtaaagacgaatttttgatacggatgttgttgatttgcagccactctgctgtattccatcttttctttatcaaaatttccgaaaatcaaaaagtttatatatgtaatttttattaatttgtgtagacatttagtcaatggaaaacctgtgtaccctatgaaataccgacaggcaaagtgtttttggacattgctgctccttatatcccttttgcaggcaaactgcttactggcacagaaggcggactttacctataccgcttcgccgggcaacctgtgtacacccgtaacacttacattgagaaataccagcaccggcactccgcttacctataactgggatttcggggatggcagaacttcacatgaggagcatccacaggtcacctataccagtggcggacccgtaaaaatcaccctcgaggcagtatataaagtaagcggcggaacaaccaccagtacttattggcgtagcctggtagtaggtgctaccccacaggtaattttttcggcagatgtaacaaaaagctgcaaagtattcaccgctaatttcacggatgccaccacaggcgcggccagtcgtacgtgggatttcggcgacggtactgcaccggttaccaccagtaatgcttacataccacatcaatacacccgcgcaggaaaatttgatgtaactcttaccgttactaacaccaacggctgtacggccaccttaaagaaagatgcctatatcgatatctccctgcccgagattacaatggctacgccactatcaggctgtgtgccttatactgctgcgttcacggctacttctgccaacgatatcaatgatccggtggtatcctgggcctggaatttcggggatggcaacacccaatccactaccaacggaaatgtaaatcatatctatacgcaaaccggaacttataacgtaggcgttaccgttactacccaggggcaatgcgtggtaactacaacgttcgataagtttgtgcataccggcaatcccccgtccaatgtaagcttcactgtatctccggccagtacctgcaccggcgatccggtacgactgctcgccaatgccagctttgcggacacctacagctgggatttcggagatggaaaaacggaatcaggcagcagtaacgatatccgccattcgtttaataccaacggtattcttactgtgcaaatgaaagcgggcagtaatggctgcttcacagctgcgccaccagctactgtaaacgtaaccggtccggtgtcacaattcagcgtggttcgcgattgtgccgataaaagtaaattcatctttaccaacaactccattggtaccagcgctaactctacctaccagtgggattttggagataattctcccctggtaaacaccatggacgcagtacataattatacaacgcccggcaattataccgttcgtcttactatcggggaaataggcaataactgcaaccatagcagcttccagacaatctactattttcgggccgattttacggccggcgtcaactccatctgccgcggaagcaaggctacctatggtgtgctgaatgtaccattgggactggtttccagctacacctggcaatttggcgatggcaccacttttaccaccactgaccaaacctatataaaaacatgggccgctgcgggtacattcgataaccagctgaccattcgttataatgatcccgcttattgcgacgacattgtgtataaaccggatgatattgacatcctcgcaccgcaggccgactttaccaccggcccggttacctgtgcaggccaggcggtaagctttatcaataacaccattacttctcccaatatcccgattgccaactggtactgggatctgggcaatggccttagttccaccgctcaaacaccgccagcgactaagtacagcgcttccggcggacaggcggtgaaactagtggtgacagatgcccgcaattgcagggactctgtcagcaaaaccatcaacattcatcccaccccggtgttgaaagcatcggcacaacaaccaaagatttgcgagggcaacagtgttaacctgaatgccttatcagacggtacggtgcaatggctcaccaccaaccagctcagttgtgttttctgtacagatccggtggcatcgccacttacaaatacccgttaccgcgtgcaggcttctaacgtatacggatgtacggtatttgattccactgatgtagtagtagtgccgaaagtaaatcttactgtaagcaatgataccattgcctgctacggcacttcggtacaactgaaagccgccggcgctaccatctataactggacgcccgttaccggtctgaccaacaacactatcgctaacccggttaccacacccataacagacatcacttaccaggtaaccggcaccaacgacgccatttgccccatgagtgcgccgcttgctgtgaaagtatccgtaaaaccggtaccacaggtagatgccggcaaggaccagacagtgatggtgggagatattgtgcggctgatggccagcggaagccctgacattgtgaagtggaaatggagcccggatgattacctcgataacaccagttctccttatgtaacggctgccgtacgtaagcctatcacttacagcattaccggtactaaccagttcggctgtacgaaaagcgatatcatgaacgtggacctcgtttgcaataccgacgtggtatttattccaaatactttcagtcccaatggcgacgggcaaaatgatatattctatccacgcggaaagggcatcagcctgataaagtctttccggattttcaaccgctggggacaggaagtacatcatcgcgaaagaatcaacattgatgatatcagcaccgggtggaacggctcctttaacggcaagccgcagccttctgatgtgtatatctactttattgaggcttactgtgataccaacgaatttttccagatgaaaggcaacgtaacattactcagataaatatttttaacctggctaacatgaaaaccatataccgcgtattactggcgatagtttgcagcacgcatgcagcaccgttgtatgcccaggatatacatctgtcgcagttctatgaaacgcctatcctccgcaatcctgctctgataggcattttcaacggcgatgtgcgcgtgcaggctgtatatcgtaaccagtggaacagcgttaccattccttaccagaccggtaccgtgagtggcgaaataaagttccctgtgggtcgcagcaacgactatgtgactaccggtttgcaggttacctacgaccgtgcaggcacttccaaactgcagtccacgcagatcttcccggctatcaactatcataaatcgctcaatgaagataagagtagtttcctctctgtaggattcatgggtggctttgtgcagcggcagttcgatcccaccaacatgacctttaacaaccagtataccaacggccggtttgatcctgctaccgctaccggggaagaaggcaaactggcgctgaaaggctacagttacctcgatgctggagtgggcctgagttacaacagcgtgatcggagaagatgtgaattactttatcggggccgggtacttccattttaaccgagccaaaatatccttctataacgatcagaatattgagttgcagccgaaacttacgtttaacgcgggtatcacaatcccggtagatgagcgggtaaaagtaattgcacattacaaccagttgcaccagggcacttatacagaatatattggcggtgctttaatcggttatggtttaatggaccagggactggaatcgacccgggccatttatggcggcatcttcctgcggtggaatgatgctattatcccaaccatcaaaattgacatggataaatacgagatcggaatgagttatgacaccaatatttccaaactgagaacagccagccagacatttggcggcttcgaaatttcattggttttcaaggggtttcttaacagccggaattcaacgctggaaagcgtaaactgtcccagattttaatctattataaatcaattaattatgaaaataaattaccaagcgttaaaaattacataaaatatgcggaaatgctaacaaaatggcctgtggtttgttatttttatgtagaaacataggcgctcgaatgagccgaatttgtcaaacaaaaattaggaaatatttgaaaaaaactttatttttataatactatgtggaaaacctctaccctgattctcataatggttttcagcctttttaccagcataggtaaggctcaaagcgaaaaatcccaacctgccacggaggggggtagcaaaatcgtgaagctatatcccaatcccgctactaccgtcataacatttgaagttcaacaacataataacgatcgcttatacgatcttattgtatataatttcctcggaaaaaaaatagatcagttaaaaggcatcagttccaagacaacggtgagcctggataattattataacggtttgtatattttccagttaagagaccagcggggcaacctggtggaatccgggaaattcaatgtggtcaaatagcttagatatatctggcatcaaaataaaaaaggaaaagtcacgatttacatcgtgacttttccttttttatatcttctgttatcaggaaacttctacaatcaggaatttcaggtaagtagtgttctcaatattccgcaggatgggatgatcctgggcttgggtctggaaagtaacctgccgcagtcttttcttcgcatcttttgcggccgcatctatggtttgcaggaacagatccggcgataccaggttggtgcaggaagctgttaccaggaagcctccgggtttcagcagtttcattccacgaagattaatttccttataaccggttactgccttcgaaatattttcgcggcttttggtaaaggccggcggatccagtattaccacgtcgaacttcttctcctcctttgtccattgcttcagctgatcaaacgcattcaccgcctggaaccggcagatatcctgcaggttattcagctcggcgtttttgcgggcagtagcaaccgctgtttcggaaatatcaagtccaagtacgcttttagcgccataaaagccggcatgacaggagaaagtaccggtatagcaaaaggcttccattacatcggcgccttttacaatatgcttgatttcgcggcggttgtcttgctgatccaggaaatagcccgttttctgaccgtttacgatatccacatgaaaccgcaaaccattttcattgatgatcaggttggtgtcgaaaggctcgctgagaaagcctttctgctgggtcatgccttccagttcccttacaggcacgtcatttctttcgtaaattcctttgggtgaaaaaatgcggttgatagcatctacgatggcatctttccatttctccatacccaacgcgagggtttgtatcacgaaataatcgttgaatttatcgattaccagtgccggcaggtcatctgcttccccatatacgaggcggcagttttccacatagcccagtttttggcggtattcccagcacttgaggagacggcggtaaaagaattcagggttgatttcttcgttcttatcacgggtaagaagtcttacaagaatctgggattgagggttgatataaccacgacccaggaaaaaacctttatgcgtatatacatctacgatatcaccggcatttacatctccttttatttcggccacttcattgccaaaaatccagggatgcccttgtaataccctgttctgtatctgtttctttaaaaaaactttagtcatttattgtatttcgaggggcaaaggtagctatttagcggttagccttggggatttcactttcaattctgcctttttgtcggcaaaaccgctgttggcaaagaaattgactggatacctgcgcagacaattattacttattatgacagaaaacgaaaaagacatgcagacaaacggtcaggctaacactggtagcgaaaacgaaggcatgccagaagaaaatataagcaatagttcaaatacgaataatgaatcaggtgaagtgagtgagctggagaagaaagaaaaggaagtaagtgaaatccgtgataagtacctccggttacaggcagaatttgacaattaccgtaagcgtactgctaaagagcgtatagaactgatgcaaacagccagcaaggaggttatcatatctttgctggatgtgctggatgataccgacagggctgaaaagcagttggaaaacacaacagatgttgcggtcgttaaagacggcgtaatgctggttttcaataaactgagaaacactctgcaagcgaaaggactaaagccaatggagagtatacataccccatttgatccggatctgcaggaggctattaccgaaatccctgctcccacaccggagctggttggtaaagtagtagatgtgctgcaacctggttattacctgagtgacaaattgatccgtcatgctaaggtaattgtgggcaaataaaatgacgatgtggcataatctctaaggatgccctatgctaaaagctgacgtaaaacaatattttttaccggacaagagctggtgcctgcaccagcattaagtgattattataatgtctaccaagagagattattacgaaatactggctgttgccaaatctgcttcacaggatgaaattaaaaaagcctaccgcaaggtggcgatgcagtttcaccctgaccgcaaccccaataacaaagaggcagaagaaaaattcaaagaagcagctgaagcttatgaagtattaagcgatcctgataaaagggcgcaatacgaccgctttggccatgccggcatgaatggcaaccgtggtggcggcggatatggcggtggtggaatgaacatggacgacatcttctccaacttcggtgacatttttggtaacgatgacattttcggtagcttctttggcggcggtggcgcccgtggtggcggtggaaaccgccgtggacgcggtacccgcggctccaatctccgggttaagatccgtcttacctatgaagaaatcgccaaaggcgccaacaaaaagattaaagtaaaaaaatatgtaccctgccagcattgcggtggcctgggtgcaaaagataaaaacgcattccagtcatgtaatacctgcggcggttccggccaggtaagaaaagttacccaaactttcctcggacaaatgcaaaccgttaccacctgccccacctgtcatggcgaaggccagatcattaccagcaaatgcggccactgtaaaggtgaaggccgtatgtacggtgaggaaatggtgagcatcgacatcccggcaggcgttcaggaaggcatgcagctgagcatgagtggtaaaggtaacgccggcgaaagaggcggcgcacccggcgatctgctgatcctcatcgaagaagaaccacatccagagctgcaacgcgacggactcaatgtagccttcgatctgcacatctccttccccgatgcagtgtatggcacttccctggaagtaccaaccatcgacggaaaagccaaaattaaaatccctcccggcacacagagcggtaaaatattccgcctgaaaggcaaaggattcccttccgtaaattcttatgaaaaaggcgatcagctgattcatgtgaacgtatggacaccacaacacgtgaccgcggaagagaaagaaatgctcgacaaattacaatcgtccgataacttcaaaccaaatcccgaaaaatctgataaaggattcttcgaaaaggtaagagatattttcagctgataatgcagcgggttttgtcttggctcaggattacgctgattttactgattagctggatttttactttttggattttttgattttcttaagatataattaagggagataaaagcgaatatccgcttctatctcccttaatcctttataaaatcaaaagtaagaatccagctaatcagtaaaatcagcgtaatcctgagccaagacaaaattcgcgcggtaaacactacaccatggaacaaaaactgcagatgttcgaaaaccggctgacgaaagttttccggcatacctccaaactggccagacgacaaaacatcacctgctaccgggtgtatgatgatgatattcctgaatttcccttcagtatagaaatgtatgaagaccatgtttacatcgcagaataccaccgcaaacacggcatggaagaagatgcacatgaagaatggctcgatacctgcctggaactgattagcaaagtactggaagtagcacccaataaaatatgggttaaacaacggcaacgcaaagaaaacaggaaaagccagtacgaaaaactcagcctggaaagccatatcatgacggcttacgaagctggactgcaatttaaagtgaacctttccgattatctcgataccggcctgttcctcgaccatcgcattacccgcagcatggtaagggaagaagcaaaagacaagaaagtacttaacctgttttgttataccggctcgttctccgtatacgccgccgccggaggcgcaacagaagtaacttctgtggatctgtctaaaacctacctggcctgggcagaagaaaatatgaagctgaacgggttcgataacccgaaacatacttttgtacatgcggatgtactgcaatacctcgacacccttaaacttaatacctacgacctcgtgatcatagacccgcctactttctccaacagcaaacggatgaaggatttcctcgacgtacagcgggatcatgcggatatgctcaataaagtgctgctggctacaaaaaaagatggcattgtttacttcagtaacaactaccgccggtttgtactggaagccgataagatcagcgcctccagcataaaggatattaccaatcaaactttaccatttgattttcagcagaagatgatcaggaagtgctaccggttaataaaataaaagatcaatgctttcctttgcgtaccatttttaccatcttcaaaaactctgagcgatagttgcctttgtcggcgcccaatgcctggcgggcaatatcgttcaccatttctatattgcctttgccgcagtaagacgacttgcgcagcagcatcccaaataaagccacgccggcagcaaagcggcaatcatcggaggccttatcaaaatttttcatttctgcggatataacaccgggtaaatattgcatcgccgtatcctgcggatcccgccaggatatttttacctttgccagcactgaatccacagcagcttccggtgtgggaataatttcatacaatgccacagaacaatgcccgctgccaatgatccctccgctaaattctcccttctctgagctgtcggcaggtagtattttattttcataaccgataagcctgtacgattttacgagggctgggttaaaccatacttccgactgcacatcgcgggcaatcgtaaacagggtgctgccgaattcacgggcaaatattttattggcttcttccaggtcatctatataggcaaaattaccattccctttactggacagggattgcagctttgaatctttataattcttcatcccaaaacccaaacaggtaagcaatactccgctttccttttgctgaacgatcagctcttccatttcattatcactgctgaggcctacgttgaaatcgccgtcggtggccagtatcacgcggttattgccctcagggatatactgctctgatgcgatccggtacgccagtttgatggcggcttccccggcagtggcgccgccggcactgagattatctattgcgttcaggatcttctctttctgatcgccgggcgtagccggtaaaagaacaccgggttcgcctgcataggctactatcgctactttatctaccggacggagattattgaccaggatgcggaaagctgcctgtaataaaggtaatttattgggggtacccatagagccggaaacatccagcaggaaaaccaggttactggcgggaaaactatctgtctccaatgcgcgggccctgatggcgatctgtaataaccggtgggtagtttcccaggggcaggtggtgtaattactatacatagccatcgtttcgccggctaacggtaacggataatcgtagtgaaagtagttgatcatctcttcaatacgaacggcatctaccggcactgcttctttcagccgcaggaagcggcggatattgctatacgcggccctgtccacatccacggcgaaggtagatacgggatggttggccgtacggacaaatttattttcgtaggtggctccgtaagtttcattgtaaaaggagtgtactcccatgccggtattaccgtaattgggattgctgctatgcaacagttttgaccgggctttggcaagggccaccggatctgcatcttttcgtagaggcgataacgttattaacagcctgtcgtatttgcgcaccgttatctctttggattgataaccgttttgtataagcaataacgtggccgatgccgtggggattgaaattttaaaaagaccgaaagcgtttgtgaccacatggactgtgtcatccatcaccttcacctgtactcctgcaacggggcggtgggataaactgtcttctaccgctcccgatacccagattgtttgcgcctgcagccctccaccccacaaaagaaagagtaaaaggtacttgagcatgtattaagttaagattttttccgggcaagcgcccggaaaaaataattactgcccggattccaccagttgataaatggctggcaggttccggcccaggccatcgtaatcgaggccgtatcccagcaggaacttatcgggaacggaaaagcccaggtaatctattttgataggatggatcatcgcatccggctttgtgagcagggcggccaccagtaattttttcggttgctgatgctccagctggggcaggaactggctcatggtccggccggtgtccacaatatcctccaggattactacggtgcgtccaaagagatcttcgtccaggccaatggcctgtaccacattacccgtagatttggtgcctttataggaagccagcttaataaacgagatctccgcctcaatagtgaggtatttaaacacatctgcggcaaacataaaggagccgttaagaatggcaataaataaagggcgctctccctccagatccttattgatttgttccgccatctccttcacccgctgctgcaacgccacttcatcaatatagggctggaactctttgtcatgcactttgatcaacgacataatacgctcatttccttatttaacaatcatcagcaaaaaaagatcgctgcttatttacttaccagcaaacgctggccgattttaatatcaaaaccctgcaggttattccattcctgcaactgtgtaacagaccggttgtacattttggcaataccatacaacgtttccttcggctgtacatcatggtactgcatacctgatttctgcactggtgcaggtgtagcaggccgcggagccggttgcggcacagatgtttttggcgtacctgtattcccggtggtggttacctggccggctttcttcaggtcttctatcatggctaccggcacaccaccctgttgcggggctggttttgtttccggtacagcaccagcgcctgctgcgttttgggctacttcttccttaataccctccagtgctttacggggagagaaatcttccggtggctcctggtcttcttctttcagtacccgggtatttttagccagccgtggtgcggcggaagcaaaaccatcaagcgttaaccgctgacccgcagcaggttcttccccttcgttcattttattacggcggcgtaaccatcttaactgtacgccttctgcctgggctacgtcgtgcatggtttccccgttaacaacgctgtggtattccctgcttcctcttttgcttttcttttgtaagaaaacgatcatatcctttgcaggcgggttatcattttccaggtcgttgtaacgtaccagcttacgcaggcgcatattacgctggtcggctacctggatgagggagctgcctgcctttacatacactgctttgcggccgttgatttcaaagatacctttcggatagctggcggtttgtttggtgcctgtactttgatttttccttccgggagatgttttgcttcccttttcggttacttctgcatacatcgttccatcggttgctgcgccaccggcagaaggatctttccccatagcaatcatcgtatattgctgaaggttataatcttcaattactttaatcagctgttgcgggtaagttttattagtagcgtatccggcttgtttaagaccaaaagcccatgatttataatcctcgccatcaaactggaagaggaaggcatagcgcgggttggcgtgcagaaaatcggagtgatcacggtaggaatcggtggcggattcatatacacggaaacactcctgggctgcatcgtcatcgtatttgatggttttgccggtccaggtatttttgcatttaataccgaagtggttgttcgattgtaaacacaaggtgccgttgccggactgtgtttctataatcccctgcgccagtttgatggcggcaggcacgcctgagcggcgcatttcctcaatggctaagtttttataggtggcgatgtactgctgcgttgtgatgttctgtgcgtgcagtacggtaacgaagccaataagaaaactgactaccaataagaattttcttacttgcatgtatgttcggatttaatgggcgttttatttcttcctgatcatcagtacaccatcccgcatggtgagtaatacctgttctgcacggtcatctgccaacactttttcacaaaaactgatcatggcttttgcctggcgtccctgttcgttttcaggcagcagtacctggccgtgatacaacacgttatctgccaggataaatccgccgggacgcagtttatcccaaaccaggtcgtagtactgttcatatccggatttgtccgcgtcaataaacaccaggtcgaatacttcatccagttgttcaatgacatcggccgctttgccgatatgcatttttattttatctgcattcccgcttgccgagaaatattgatgacaaagggcttccagttcttcgttgatatctacggtgtgtaatatgccatcgggtgcgaggcctgcggccaggcaaatcgctgagtacccggtgtaagtgcccagttccaggatgcggtgcggccggatcatatggcttatcatactgaggaactggccctgtacctgcccgctcaacatatgcggcaacgctaccttcagatgtgtttccctgttcagctggtacatcaattcactttcccggctggtatatttttctgaataggcctctactgctgccggtatgagctccatatattaaaatttctgcaaagctaaggaaaagcggctaaccgacagcctgttgctttcaacagaaaaagcggatatatccataaacgctattctgccgggttttattctctccgggcgtacgttcacgcatatccgcttttccggcctgaagggaggctttattagaaattcggtcttaatttattggtagtatagaaaacacggaaatattccactacttcatctgctgtgtcaaataactgcagcaggtcgaggtcctgcgggttaatattgctttccttttccatcattacattacggatccagtcgagcaggccactccaatactctttccctaccagcaccatcggcgtttcctccattttcttggtttgaataagggtggctacttcaaagaattcatccatcgtaccaaagccaccaggcatcatcacaaagccctgggaatacttggtaaacattactttacggacaaagaagtaatcgaaattgagactattctccgggtctatataaacattgggatgttgctcgtgcggcagggtgatattggcgcccactgatttgccatgtgctgcctgcgcgcctctgttggcggcttccataacacctggtccgccaccggtgataatgccaaagccttcttctgccagcctggtggatatttcctgggccaggtcgtaataacggttgcccggtttggtgcgggccgatccgaatatggaaatacagggtcctattttagccagtttctcaaatccttcaacaaactccgccattatcttgaatatctgccagctggaatgcgctcttgtttccgtccagtctctttctttaagattctttatactactgttcatgcaactgcttttttattatgctataaaacaccttcccccgtgcaggcacgcggaatgatgtaatttatataataattggcttacagtaacagctttacgcataaaaaaagcaggtaactatatagaaacctgctttacatttaacacgttatgaacgtgcagcgatgttaaataaacatcgctgcagaaacgttgctaatgctggcaatcaaaaaaataaataatgttgaaatttagtaagatagtactaccgttttaatcaacagatgttctcataacgcttaatctccattaatttattaattatttaagcaataacctaatttaaatttatcaaggttacgcaaaggtatgcgcgcctgccactacttcttcggccagcccgaaagacaatgtcatcccggctccgccaagaccatttacgatcgttacatttttttcgggagagaataccaggtccgttttgccgttggttagttttgggtagatgccatgccattgttcctggatggtatactccggcgcctgtaaaaacgtatgcatatattgcaggatgagttcattgataaatgctttatcaaatggttcgaagtccggaccatattcatgtgagtcaccaatggtgagttcgcctgcgccattttgagaaatcagcaggtgaatgccccatttcacatactccggcatttcctgtgtgaagcgctgcttcagtggttccagggttttacagctttcaaaggccgcatagtgtcccagggttaagcctgcgcatagtgcgggacccagttgccagttgcccggttgcggaatggtacgcatcatctgcagtttgcattttttcagcggtgcggccgcaaattcagcagggtaaagcgtttcaaagtcagcgccgctgcaaacaaatacttcttccactttccagcgctcatctttggtttcaataaagggcatgctgatgccatttaccgcggtgccgaaacgaaccgttacgttcaggtgttcctccaaatgctttgcgatagcggcactggcctggcgtgggttcacggtcatttcggaggcactccacaatgcacctttcaacccgtttgttttaatcgcgctggtatattttcctatttgtgagggagcaatcagctcacagctgtaaccgttgccgggagcggcctgtacaaattcttccaataccgccagttcatctttttcatacgccaggtgcagtgatccggtttcctggcactgcaacccggcggcagcagccagctctttccaggtacggcggctgcgcatagcgcggtcgtacattttacctgccgtttgcccgatgggccataccagtccgaaattgcggatagaagcgctgatcgctttactgttacgttcaaacagcactacttttcttcctttttttgccaggtggtaagacatggccaatcccactattcctgcgcctattactgctacatctgcctgttgttgttgcatgatatcaaatgtaaagtgtgattaaaagatagacagtagttcatccagggatgctaccaggtgggtatgcggacctttctccagctcttcccgcgtataagcgccggtagtaacccctattacatagcggcaacctgcattggtgccttcttccaggtcggaaatggtatcgccggttttagcgaccgacgctatactgcggattcccagctgttccatgatccggtatatcatatacgggtatggacggccgaagggtacttcatcgctggtagccacggcatcaataagtcctttttgctgccagcccaccctttccaggatcacgttggtaatggccctgtcgaagcccgtatccagtgccactttaataccttttgccttcagtgcggcaaataccgctgataccccttctttttcccttaccgcaggatgtgtggcataatgcactttcatgtccgccacaaaacggctgtgcaggtcaacaataaaggtttcatcgctgtagcggctatccttctgctgctgcaacaggtaacagatagcatacggtttggcgtaccccatcacctcgttcacctgttccagcgttactgtaacacccgccagcccgatcgcttgctgcaacacctttgctacattggattcatcatgcagggtagtgcctgcaatatcaaaaacaactaattgtattcccatcttttcccattgttaataggtggcaaagataaggagttactaaaaataagtttagcatttataaacatttaacatgcgcgtaatatgcgcgtattttgtcttggctcaggattacgctgattttactgattagctggatttttacttttggattttcttggatttttagattaataattaagggagataaaagcggatatattcgcttttatctcccttaatcctttataaaatccaaaaagtaaaaatccagctaatcagtaaaatcagcgtaatcctgagccaagacaaaatccgcgcgcttaaaagccgagccccgcgcccacccggtatatcaggctgttgttatagggcgagcggtcgtcctggattacatcatataaaatggagatgccgatgcctaccctgccgcctacgttttgggtgtaacccgcgcctaccagtaagctgggaacgccatagttggttttgtaggtttgtttttcgttgttgtcgaggtaaacggtagaattttgtgtaacgaaattatattccggctgaacatgtataaataccatcgggagcggatatacacggccccagataccaccgccaaaaatagtatacttatcccgctgcattatctggtcatagttccacactttatactggccgtattgcgcattgatgttaacacccgcagcgatgtagtcagagaagcggtaaccaaccagcggagagatatccacgttggtaacatcgccaaacaccattcccagcgaaccgcctaataccaaacgggaaggatcaaagcccttacgggtaacggtgtctgttttataatactgggcgtgtgccagctgtacgccagccagcaggaaaatacatatcaataaacgtttcatgatcagctttattaagtttaactatttaccggcagaaaggtttaacaatcgaaaattttaccccggtttaatatattctttggatcaaagatctgttttatttgcttcatgagttgcatggatgtgtgatcaaaaatgatatccatatagtttttctgtaccaacccaataccatgctcaccggagatggtaccgcccaatgctttcaccagctgaaaaatttcccgtataccttccgtgagggttccgttccattgttcttccgtgagggtgccgcggataatatttacgtgcaggttaccatcgccggcatgcccgtagcacactgaatggaatccatacctgttcccgatttctttcacgcctttcagcaataccggtagttctgcgcggggtaccacggtatcttcttctttatatacagaatttgcttttactgcttccgccacccggcggcgcagtttccagagttcttccttctgctgggaatcttctgcaaacaatatctccccgatatcaaaaccttctaccacaccggcaataccttccatttcctgcatcagcacttccgggtaattcccatccacttctatgagcaggtgtgcctgtatatcgtcttctattttaactgcgctactttgtacatattttgttacccagtcgatggcgtcacgctccataaattccatggccgaaggtgtgtaacccgcccggaaaatagcgcttactgcttcacaagcgctttcagcagagcggaaaggaaccagcatcagcaggtctgttttgggtagtggtattagacgtaatactattttggtaacgatgcccagggtgccttcgctgcctactaccagctgggtaagattataaccggtggcatttttcagcacattggcgcctgtccagatcacttcaccgctgggcagcaccatttccaggttcagcacataatcttttaccacgccatatttcaccgctttggggccgccagaattttccgcaatattaccaccaataaagcaggtaccgcggctgctcgggtcgggcggataaaacaagcccttttcttttacggcgttctgtaattcttctgtgatcacaccaggttcggtgattacctgcaggtttctttcatctataagggtgatgcggttaaaccgttccatggatataagcacgcccccaaactgagcgagcgctcctccactgagccctgtaccgccaccacggggagttacgggcaacaatgcttcattgcataatttcatgatacggcttacctgttcggtggtatccggcttaactactacttcggggagataatgcagatcctcggtttcatcctgtgcataacggctcatactttcttcgtcggccaatacatattgcgctccggctatttcacgtaatgccgctacgtgagcggcagttactttattgaacgttgtcatggaacaaaaataatcataatgccggttaggtggtatatccggactgttaaaaagagggacagatcgtagatcttctcgcattgttaaaggtgcggttgctgtaaagtcctgtataaacgatgcctatctcataagcgccacgccggttgttggcggcagagagactggaggtagtgatatcgtagttaaacatgagttttatggcgttgatctggtagccaaccaggaataccgccgcatcattggcgcggtaataaacgccgccatacagttgttgcacgccgtcgccggaaagattataggcagcattggcgcccagcatcagttcccgcgcgccggcctgtgtggcataatacgctgcagggttcaggatcactttatcgctcattttcaaactcgcattcaggaacccgatataccgccggggaacggtgttattgccatcaaaaaaggtttccctgggtgtgttgatatgttgtacagaaaagcctgcatttacataaatattatcggtaggaaaataagcataattcaagcctgcctgcaggtcgaaataattgacgctgctttgggtgatgggttccccggtggggatctgtgaatcaaagaatttaccattccactggtcggcgaatgtgagcttggtgatatccacccgtttgccggcggagcctacattgaaccctgcggatagcaggctgctgaaacccaggagctggtgataagcgatagaagcgtatcctttggtggaggtgaggtttcctgcgccggccacgtcgcggagcaatacgcccccgatgcccacccagccatattccagctgatcgcggaatagttggaagtcgccatatgccgacatcgtccggtaaggtatcggaacgctggtccactgatcacggtaattaatgccaatacggtaattgccgtccggaatgaacccggtattggcagggttagttgtcaatggcgaattaaaaaactgtgaaaaatggaggtcctgtgcgtacgccccacccattgaaacaattaataaaattgccagacatgttgataatttaacgatctgattcatggctcatcatcttaacaaggttacacttcctgatctgctgcctttggtgccatccgtaaactcgaggtttacgatataggcataagcatccatgggctgaatatttcctttaaaccggccatcccatccgatttgaggatccgaactttcaaaaaccaattgaccccaacggttaaatattttaagattgaatttggtcgctccaaaagcttttacataaaacacattgttcttaccacccggtgcaaaggcgttgggcacatcaaacagcggtaccacaatagcgcttacttcctcacattttgtatccgtacagccttctgcgttagtaacagtaagacacacgttgtatgtgcctgtgcgcaggtattgatggctgggatttggcagggaagaggtatccccgtcgccaaaattccagaggtaatgtatcacgtttgccgaggaaccattcaggaactgtatcggcgtattttcaattgctttggtgggtgaaaagtcgaagtctgctacaggcggcgctgccacatttatttcctgcgtaatcgaatcccgtttgttacaggtattaggatcgtctacctccagcgttattttccagcggcctgctttattaaatgtatgcaccgggtaaggatcgtgtgaaacggaaccatcatcttcaaaggtccaggtgaatgtttcaccgccctcggtggtattatccatttgtatttctgtgccaacgcaaaccgttcccgggtcggtaaatttcgctataacgttctcggctacacgcagggtgtaggtaattgtttgcggtgcattacagaaattagtatctaccagtgtaagggtagcattatagatgcccgcattctggtaatagtggaatagcgggaaggtatctaaaccggtatagaatggaggtgttccatcgccatagtcgaggataaatgagctgtccctgaaatccgcagctggtgtggattcattgacaaacatatacttcaggctatcgcatggatcctggcgccgggcttcaaaatggagtatcgcttcattgttgcccagtttcacagttacgtaggcggtatctgatccgttacaactttgcggatcgtattttaccattctcacgcggaaggtgccaatccttgtaaagatgtgcgtcaccgtatctccctcaggtccgaaattcagcgtggtgccatcatccgggaagaaccactggtacgatttacctggtaaacgggtggtatccacgaaggtgatggtatccggtacgcagtagttggtgcgcctgtcgagtgttttggcgcctgctttcaccccatcgaggttaaaggcaattttcagcgcgccaagattacaggcggctggcggtgtgctggagtaggcgcccggcgtagtcgggtaccgcggtttgaagccactgttgctcacgttgcaccaggcgcagatgccctggtagataataccattgcggtcgaagcggctggtaccgccatctacgtgttcatacaaaccggagccgccaaaatagctggcatacaatggaccctgggttggactaaaccgtaccgcatcgcgttgcagcacatagaaataaaaatccatcccgtcggtgctgcgttgcagcgcatccggggtggtagttaaaccggaagttcctgaattcgggtagtgcagggaggtattgatacctccgccccatccggacacgtatacgttttcgcagcggtctaccaggaaggcggtgggagaaatattaggggaagaaaccagtgttcttctttttccgaaagtagtggaatacacgaatgcggacaggtttgcctggagcttcgagataaactgcagtccgttttcattgtatccattggcgcttacttgtatgatgggccatgctccttctgtggtgcccattacatatacaaatccgtttttatcgagctggataccgtatatctggtcggctgcggcattatccgaaccgaggaaagtactctggataatgtttcttccgtcgtttgaaatgtgcgcaataaacccatcgcatacgccgccgcggtactgggggtatatggtgcctgcggtaacggggaagtcgtcgctggcggtgcctccggctacatacagggtattcaacccgtttaatgcaattacataagccgcatcttccttgctgcctccgaggtaactggcccataccaggtcctggcagagcgggtttattttcatgatcacaccgtcctgcgagcctttgttggttccctggaatacgccggctgttacgggaaaattggtggaacgggtgcagctggccacataaatatagcctgcattatccactaccacttcgctgcgggcgtcgtcgccatagttgcgcagcagtacccagtcgccggcctgacggtcggcccgcatatttacgccatcatcttcgccgccggcaatgatcagtgagccgatgatagcggtgcctgtggcgtttattttagtaatggcgatatcccatcctccgcgggttccttttacgttggtattgggatagtcgctggaagtagttctgccggagatcacaaggttgccctgctgatctacaaataagctatgaggttgttccaggccgctaccgcccatgtaggtggcgtataccagcctggttccgttggcactgaatttggaaatggcgatatcaaactggccaccgccataaacgctttgtactgccccggttgttacggggtagcccggattaaacacaataccgccgccgtataaattgccggcatcatcgtaggtggcagtgaagccccagttatccgagcgggcacccgatacggtagaaaaaacgtagatcggatctatgaccagcgggtaggccgcgttatattcaccggatattttgaagcccagtttattaccatttaaccggtaagatacctttacggttacacgttgattattgatatactggtaagcaaagggcagttgttcaatcacatcccccacagaggtgtgcaccagcaactggccttttttcagttccatgccggtagcgccttcatataccatctggatattatccgggttagcgcccggatgcacaatcaggtcatatttcagctgggaaccttcagagtaaacgtgcgcatcgatgccggaataaagggagttataattaacgccctggaaggaacccaccccggttgcccatttggtgcggtcgtttccgatgaaatagctgcttttggcgtcctgttctttttcgggtactatttgtacgtcaggattggcgttcaggaaagtaacgttatacgcatgcccgcgtacatcaggaattttgccgggccgtggagggggctggccattccctggctgggcaggtgctggtttaaagttgcttttcggaacgtataccgtatcactccggtgggagtgtccgtgcacatattcgttcaggctccagagatcctgctggttcatcatcaggaaagtgaagcctgtttttttgaggaagatagcggcgccatccagttctgttctgtagatgacatctttatcccactggcctttgttctcaataaaattcagcggtgtgaagttcgcatgttgctgctgcgcctgggcggatcgtccggtgaacaaaaagcaaatcattaatccaataaggccggtcgggaaggtaaatttcaacgggattagattttattttattcttaaaaaccaatataatactattaaacgcagaagccactcaaattgttacggtcgggaaaggcacaaaacttctgaattgaggaataacaggctaaatgggaaacaaggtgaatctcagcttcagcagctttatacttttttaattcatccatcagttaataaacgtaaaaaccatcaggaaattttactccagacagatttacttctctgggcagctaaaaattcttttagtgcctgattttcaggcaaaagcagatcggtgtcttcttccaggatcttttctgcgctggcgcgggcggcgtcgaggatgggtttgtccgcaacaatatccgccagtttaaagtcgagtaccccgctctggcgggtgccttcaatatctccggggcctctcagttccatatctttctccgaaataataaatccgtcgttggtttgcaccattacgttgatccgttcgcgggaatcctggcttagcttattaccggtcatgagcacgcagaaggactgttccgctccgcggcccacccttccccgcaactggtggagctgcgacagcccgaaacgttcggtgctttctatcaccattacagaggcgttgggcacgttcacccctacttcaataacggtggtggctaccataatatgggtatcgccggttacaaaacgctgcatgttggtttgccgctgttcggccggctggcggccatgtaccatactgatataatactgcggttcggggaagaaagctttcacctcttcatatcctttcatcaggttttcatagtccagcttctctgaatcttcgatcagcgggtatacgatgtatgcctgtcgtcctttctttacttcttcctttataaaatccattacctgcggccgttgatattcggtgcggtgcacggtagtaatgggtttacgtcccgggggcatttcatcaataacggatacatccaggtcgccgtaaatggtcatagccagtgttcttggtataggcgttgccgtcataacaagaatgtgtggcgggatggtattcttttcccataggcgtgcccgttgtgccacgccgaagcggtgttgttcatccacgatggccattccaagatttttgaacgccacttctttttccagcagggcgtgggtgccaacgaggatatcgatgctgccatcgagggcgccggccagtatctgcttacgtgccttgcctttgatgctgccggtaagcagtgctacctttacatccatccgctccagcaattcggagatgcctttaaagtgctgctgcgacaggatttccgtgggcgccataaggcaggcctggaagccgttgtcttttgccagcaacatggatagcagtgctaccattgttttaccgctgcctacatctccctgcaggaggcggttcatctgccgtccgtgaacggtatctgtccttatttctttcaatacccttttctgcgcgcctgttaaggaaaagggaagatgattgttatagaattcattaaaagattcgcctactgcaccaaacacaaagccgtgtgattgcttgtgtcttttgagctttaaccggcatatacggatttgtgcaataaacagttcttcaaatttcagccgtcgttgtgccagccgtgcgtcgtcttcgctggcgggcaaatggatcctgaaataggccatcgcacggggcatgagccggtattgctgtaatacttctgcggggatattttccctgatttccagtggagataattgttccagcaggtttttggtcaattttcctatagcctttgccgttagtccgcgggctttgagtttttctgtggtataataaaccggttccaggaattgtttaccggtagcaatttcttctgtgagcaggtccacctccgggtgtgccagctgggtaacgccattgaatacggagatcctgccgaatacgaggtaggccacattttccttcagtgatttctgcatccattgccagccctgaaaccataccaggtcgatggtgcctgtttcatctttaaaagtagccaccagtcttttcgacctgttctctcccattaccaccatgttgatgatctttccgcggatctgcacaaaatcttcatacccgctgagggaggcaattttatcaatcctggtacgatctacataacggaaaggaaaatattgcaggaggtcgccgaaggtatatactttgatttctttacgcagcagttctcctttctgcgggcctactcctttcaggtattctatcggatttgataatatggcagtaaaagtagaaatggttatttcgttttttgtgaacaacaaaaataaaaaaggcaagtggtaaaaactcaccacttgcctcttttactaaaaaaacaattataaaactattcggctattgcatctacttttccttccacgaactgtttcatccactcggtggtaacagatttcggtctttccagggaaagtccgagtgccctgtcccagcaaagggaagccagtacgcctaatgcacgggatacgccaaacaacacggtatagaattcatattccaccaggccgtagtgtaccagcaatgcgccggagtgagcatctacgttaggccatggattctttaccttgcccaggtcctgcaggattggcggcacggtttcatacacttgccatacaattttcacgagttcatcgtttggcaggtgttttttggcaaactccatctgtgcggtaaagcgtggatctgttttgcgtaaaaccgcgtgaccgtaaccgggtactactttaccatcggctaatgttttgcgtacgtaggattcaatttgttctttagttggaacgccaccacccagttcttcacgcatctggagtatccatttgatcacttcctggttagcgaggccgtgtaacggacccgccaaaccgttcatacccgcggcgaacgacaggtaagcatcgctcaatgcggaacctaccaggtgcgtcgtgtgtgcgctcacgttaccaccttcgtggtcggcgtggatcaccatgtaaaggcgcatcagttctttgaaaccttcatcagagtaaccgagcatgtgtgcaaagttacctgcccagtcgagcatgccgtttggctgaatatgctggccacctttatatttacggcggtaaacatatgctgcaatacgtggcagacgggcaatgaggttcatggtgtcctcataggtatagctccagtaatcttttttattaattccttctgagtaagcctgtgcgaaagcagattctgtttgcagcgccatgatacccacgttgaacatggtcatgggatgtgcagtgatcgggagagcttcaatagcatcaaaaacgtggttgggtacatgagaacggcggccccacatgctggacagatattgtacatctgcctcagtaggcaattcgccgatcagcatcaggtaaaataaaccttcgggtaaaggttctgcgccacctggtgcttttggcaggtgttctcttaattccgggatggaatatccgcgaaaacgaattccttcattggcatccagcagggaagtttctgttaccaggccggttataccgcgcataccctgataaacctgtgccagtgttacctcctcaattttcttggtgccgtgattctttaccaggtcttttacttcaatgttaagttcatctgctttaaccttgaatttctcttttatgtaccccattttactgctattgttattaatgaaaacaaaatcgatcaatagtcaaaagtaatgatttgttaacgaagttaccaccctttcgtggtatttaatgccaaattaacaacgattcccggatgaaaaagtaaggcgatatagtcgcagcgggcttcattaacagtatatttataagccgattacgaatataatatataacacatctatatagacgttaaagaaatgtaaaattttcagaatgaattgaaaatattgaaagaaaaatagcggtgattttagcgaaggttgtcgtggaggttgtcgcggaggttgtcgcggaggttgtctttctcaggattacgctgattttgctgattgacttttttgagatttggggagatggaaacggaggttgtagcggaggttgtcttgagcactgattacgctgattttgctgattgacttttgagattgggggagatggaagcggaggttgtagcggaggttgtcttgagcactgattacgctgattttgctgattggcttttgagattgggggagatggaagcggaggttgtcttgggcgctgattacgctgattttattgattggatttttgtgattttgagggaagtttggaattttcagggaaattgatgggtaaattttattgaatgaaattgggggaggatggtggttgaattaggattgaataaaggttgaataagatgggactgatattgactgtggaatacttcatttttactttgcatgggcttagcatatgcttgaaagatgcttgatacatgcttaatgtatgctgatgacccggaggtgatgtggaggtgacgtggaggtgacgtggacttgaagctaagattgtttgtggcagggctttacagacgagaaagtatatggcgcttagacgcagtgcaaccatataagtgaaacagtgtgctaatataactgtgaaaatgactcaccagcattcaataaatctttaccgttaaatactatccgcctttttaaattatctatggaataatgagggtaaaaagcttttaaattcattgaattttccgaaaaatcacataaaagcgaaattaaaccaattccccagagaaaaaccaatagacgaattaaaatctaaccagcgtactaatattcccaaatccctgccaaaatcacgaaaatccaatcataaaatcagcgtaatcagcgcccaagacaacctccgctaaaatctccccaaatctcaaaaagtcaatcagtaaaatcaagggaatcctgagaaagacaacctccgctacaacctccgtttccatctccccaaatctcaaaaagtcaatcagcaaaatcaagggaatcctgagaaagacaacctccgctacaatctccgcatcatttgggggcctggcgatacaggtagaacgccagggcgccgaacaaaatattggggatccacaccgccagcagcgggttcaggtctgcttttacagaaaatacggtggcaaattgcaggaatatgatgtagctggcgctgatcacaatacctactgccaggtgcaatccacttccgcccctcaccttcttggcggcgataatgccaccgatcagggtaaggatcactactgcgaaggcggcggaggttctcctgtaatattctacccaataggtattcagtccttcggcaccacggatgctttcccgctggatgtatcgcctgagatcgggcgtggtcatggcttcctggatattcttttcgtcgaccaggtctttggggaccaggggtattttaagcagggtatcctgtttgctggtccaggtttccttcaggccgttcatggtgcgcatggatacgtagtccagtttccactttttggcggtggaatcccagctgatacggtcggctttgagtttgaaagtcatggattgtttattcacaacagacagtacaaaattgctcccgcttttatagttgggatcgtaagtaccgaaagttacataggtaaagctatcgatacgggtggtgcggtcgtattgtgatttctcgtcgtcgtgactatggaggtatttattttcaaagctggtacggatgcggttggcgttgggaactacccagtagttggcgagccagagtactcccccgaacaggaaggcgcccatccagtagggacgcagaaaacggcgaaagcttacgccggcagccagtatggcgatgatctccgagcggtaggccatcttggaagtaaaaaaaataactgacaggaatataaacagtggaaacagtaacgccaggatatgcgggataaagccgaagtaataatccactatgatttcatgcagcgacaggtgatgcttcatgaagtcatccaccttttccgtagtgtcgatcactacagaaatcaataggaatatcatcagggagtaaatgaaagtacctatgagcttgcgtaaaatgtaccagtcaattttagtcatgaccccaaagatattagtttattttatagtccggacttttacaggcgtgttttcagctgattgatcatcccggttttccaggtggcgaaagtgccggccagtatttgcctgcgggcttccttcacgagttccaggtaaaaggccaggttatggatactggctaatgtcatgcctaaaatttcgccggctacaaacaggtgtcgcaggtaggcccttgagtaggtgctggtagcaaagcaggggctgttggcatccacggggctaaagtcggttgcccattttttgttccggatgttgataacgccgttccaggtgaacagcattccgttacggccgttgcgggtgggcattacacagtcgaacatatcgatgccgaggctgatgttttccaggatattccagggggtgcccacacccatcaggtaacggggtttgtcggcgggcagtgattcgcataccagtccgcacatttcgtacatttcattttccggttctcctacgctgaggccaccgatggcattaccggcgcaattgcgggaggcaatgtattccgcggaggctttgcggagatccttataggtgctgccctgtacgatcgggaacagggtttgttcatgaccgtaggcaggttgggtgtcgttgaggcgtgtgatgcagcggtcgagccagcggtgcgtgagttccatcgacttgcgtgcataacggtattccgacggatagggcgggcattcatcaaaggccataataatatcggctccgatggtgcgttggatatccattacattttcgggcgtgaagaggtggcgggagccgtcgatatgcgactgaaaaaccacgccttcttctttgatcttgcggttggctgccagggaaaacacctggtatccgccgctatcggtgaggatgggccggtcccagccattaaatttatgcaggccaccggcgagcgacaacacttccaggccgggtcttaaataaaggtgataggtattgccaagaatgatctgagcctgtacatctgcacgcagctgttcctgtgtaaccgcttttacgctgccaacagtacctaccggcataaaaatgggcgtttctatttccccgtgggcagtggtgattttcccggccctggcattgctgccgctatctgtagttatcagttcaaaattcactcgtcgatatttcaggccgcaaagatattgaaatgaagcgaagatcgaagctggtggattttgctgcgggaggcaatctctccaatgttcataattaattcttttacagataataaaaatattatatttttgcggtcattatgctagaccatctaggtgaaattgccttatactcttttgctgccatagccgggatacagatcatttattttctttttgtgttttcccgggtagctttctatagacgtaaatttgacctggaccatgcaccggacgggcctttttcggttatcatctgtgccaaggatgaagaattgaacctgcagaaaaatctgccgggcgtattgcaacaacgctatcaccagcacatgaaacccgaatacgaggtgattgtggtaaatgataactctgaagacgacaccaagtactacctgcgctccattgagccaggttatccacattaccggcatatagagatcaagcaggcggctaaattcattcccggcaagaaatacccgctttccatcggtttgaagggcgcccagtttgaaaaggtattgcttacggatgccgattgcaaaccgggcagcacctactggctttcgctgatgagccagggctttaccgataaaaaggaaatagtgctgggatacggcgcttatcataaaaagccggggttcctgaataagattatccggtatgaaacctttttcagtgcgctccagcatctttcctttgccatgagcggtatgccttatatgggtgtaggccgtaacctggcttataaaagagagctgttctttaaacacaaggggtttacaagccaccagcatcttgccagcggggacgatgatttatttgtgaacacggcggccaaccggaaaaatgtgggagtggtaatagacaaacaggcttttacctactccgagccgaagctgagctggagaagctggttccagcaaaaaacccggcatatgtctaccggtaagcattaccgtttcggtcataagtttgtgctgggattattttcgctgacgcatttccttttttacccggcgtttattttcgctttatttttcccgccgcccatactctggtatgtgctgggaattttcgcggggaaagtgctgatacagtccattattacttatgccgccatgcgcaggctggatgaaagcgatttgtttaaattcagctggctgatggatattttcatggtattatattatatcatttttacaccggccttgcttttcaagtcaaaaaataaatggtaataagcagcaggcaatagctttctgcttatttgcttttgctttacttttgccgcatggaagttattttaaagtatttcagcgacttcacaccgggacagctgtcgcagtttgaggcactgcagggattataccaggaatggaacgaaaagatcaatgtgatatcccgtaaagatatagacgccttatatgaaaaacacgtattacattctctcagtatagccgctatagcggagttccagccaggcacccaaatcctggacctgggtaccggcggcggattcccgggtattcccctggccatctttttcccggaagtacaatttcacctggtagattctattggtaaaaaaatcaaggtagtggagggggtagcggaagcgctgcagctgaaaaacgttactgcggcgcacagccgcgtggaagacattaagaaccggaagtttgacatcgtggtgtcccgtgctgtggctcctttgggagacctttggcgctggagcaagcatgtattaaagaaatccaccgtacctggtaagcagtttgagaaggggctgatttgcctgaagggcggggatctggcccaggaaatttccgacagcggcttaaaaccacgcctggtaaaggtgtatgatattttcccggaagaaagttttaaggagaagtttgtggtattggctaagagctaaacccggtttccagtgtagtgtggtggatgcccaggtgttccagttcatggcgcagttctttcttcaaagcttctgtgccggcagcgtccagctgcggatctatggttacctgggccgttaaagcgttttcggtagtgctgatcgcccacacatgaatatgataaatatctttcacccctttcacggccagtgctttttttcttatttcctgtaagtcgatgtctttgggcaccccgtccatcgacaggcgcaggctgtcgcgcagcagcccccaggtaccgattacaattactaccattactattatactcagcaggggatccagccaataccatttggtgtagatgatcaggataccggcaactacggttgccatagataccagggcatcggcagccaggtggaggtaggctccttttatattcaggtctctttctttgtctttgaaaaacagccaggccgtaaaggcgttgatgaaaatgccgatgcctgctacaacggcaatgggggttccgggtacttcgtaaggctgactgaagcggcggatggcctcgtatccgattacgcctaccacaataagcagcagcatagcgttaaacagggagataagaattgtacttttgcggtagccataggtatagccggggttggaggtaattttaaccaggcggaaacccagcagtgagagggccaggctggccacatcgctgagattatgcccggcatcggccatgagggccagggaatgggtgaggaaaccggcgataaactcggccgccacaaaagccaggttgagggaaataccccatataaaagccctgttaacctgggcgttgttaagtgccggcgtatgagcgtgggcatgatcatgcataaacgactgatttccttgtacgtaatttaagaagattttttttcgtccttataaaatatccgcttcgctgcttcgtcatccttattaagatgaaacagctggtccttacaaatagcattatggccatagagcaaaacgaacgcatacaggcaaccgtgaagcaggaacgcaagcgattgctgcattttatccggcaacgggtaaataatgcgtccgatgcagaggatattttacaggatgttttctatcagtttaccgaatacctgcgcctgggaagccaggtagattctatcaccggatggctttttgccgtaacccggaataagattaccgattggttccgtaagaagaaagaaactcctttttccgaattcacgcgcgagatagaaggcgaagaagtgctatttctccccgaactactttccgacaaaaacatggaggcagacactccgatggcgaaaaagattatgtcggaagccatcatgcaggccattgatgagttaccggccgatcagcggcaggtattcctgcagcacgaactggaggggaaatcctttaaggaaatgagtgaagaaaccggcatcggggtaaatacccttttgtcacgcaaacgttatgcagtgctattcctgcgggaacgcctggcagagctgtacaacgaattacttaacgactgatttaattaaaaagatatgagaaacaattttggcagaagaagaggactacaggtgctcaaatttgtgataatgggagcgctgtttgttacagttgtgggatttgccaccatgctattatggaactgcctgatccctgaactgttccacgggccggtcattactttctggcaggcgcttggcctgatgttactgggtaagttactttttggatggcataaccatcacgataaatttaaccgtggccgggaatggaaatcccgcctgaaagacaggatggcgaacatgacgccggaagaacaggaaaaaatgagagaacacctgcgcaaccgctgcagaaccgggtttggcgcatggaaacgtgacgactggcatcgtgatccggacagcagatgggatcgtgaccgtgaccctgaacaacctaaaaacgaagaaaaagaatcacactaaaaacatttgtgcgatgataggaatattcaaaaccaatataggcagcctggaagagcgtcagcagatgatccaggccattgcttccagcttccccgttgggtcatgccatgtagacctggacgactgcgataaagtattacgcattgccgacttacaggtggaagagaatattattatagaattcgttcaaaaacaaggttttgaatgcgctgtgctggaataatctgagatttttccacagcaaatcaatattcccgggccatgtggcggttttattatacataaattcattttatatgtaatatgctattggccggttcgcaaatctgacgtaacttcaaagagaatgcagcggcccgggtatattgtttacaaagccaggtattgtgtatctgaaaccctctaaattttgtttcctatgtacctgaaccagcacgagatcaaatctctcttaaataccagtttcgataacttcgtggattttgtgaatacgttgccggatatacgttttaccgcatccccttacggtaagtggtctgccggccagcagctcgatcatctcaccaaatccatcaggcctgtaagcagcgccatgggatttcccaaggtaaccctgctgtatttcggcaccagcgccatgccatcacggtcgtacgatcagctagtggctgattatgagcggatactggatgccggcgcaaaggctaccagggcctatcagcccggggtgatctatcctgcgcagcgaccagcgttactgcaaggttttcttctccagaaaaataaactgatcaacaaactggctgcctggtcggaaagtgacctggataagtatcgcctgccacatcccctgctcggaaaaattaccatccgcgagatgctgtattacattgcgcatcataacgaacatcacctgaacaaattaaaggaccaggaattacagggccacacctggcagaaccaattacagcagctgatattctgattttttaggttaaattgtttctacttaaaaaatcatcatggctacaactgcgttagtcatcagcggcggcggctccagggcagcttttgctgttggcgccctgaagtacctctattcacaacaaccagccattgcattcgactttttttgtggcactggtatcagcgcattaattgctccgcttgcagctttgggagaaattggcttgctggaaaaattattcaccagcaacaccaccgccgacctggtaagcaccagtaccatgttgcaacgcttcccccaaaacaactctctttacaacgccaccgcccttacccataaaattaccaacatctttaccgacgcccgcttccgggcgctgcaacagctgaacaaagaagtatttgtgaccgcgcgctgcctgcaaaccaatcgtatcacctacttttctccatcgggcacggatatggtgaaaaaggattatgaggttatatcgctgcacgacaattatacattccgtgaagccatgcaggcatcctgcagcatgccggtgtttatgccaccggtggaagtggcttcccttcccgatcatgtgcagcagttcaccaatgcaggaggcgcacactatcatcccgttaaactggccatagaaaaaggcgccgccgaaatctatgttatcctgctcaccccggaaacacccggcgaagatgatatcttattcaaaaatttactcgatatcctcgaaaaacaggtggataacagcaccaatgaaatagcggccaccgacctggaaataacacagctcatcaaccagtcgctgacttatcttgatacagtaaaagatcacctgaaaaaaaagggcatccctgccgccgacatcgatgcgtgttttgatcttcccgccgctaacccgttcaagggaaaaagaacagtaaagctgcatgtcatccgcccgaaaacagcgctggatgtagctatgggaggactcgaatttataccgcaggcaatgaaagaaatgatggaagccggggaacagcgggcagcagaagtgttgcaactgctgtaaaaaaataccgggatgctgcttttgcaaacaacatcccggcgcatgctttattactggtgtgtgttaagacactgctttgttattacttctgtccacatcggccatacgctgactgggatctatttccagctccttaatatctccgagcggggtatccagttccacttcataaacaggattagtccagtaccaaacgggatcgactatacgctttacatccgggtattcgttaggtttttcgccatacatgattgacaacggaatatagtgcagcaccttattaccgctcttatctgttaccataaaatcaatgggcatcggcatatatcctaccctgcgcaaacgcactattgttttatttccctttgcaaaaacactgtcgataccatagtcgatatgttttaccgcattgataaaatattgtttgtaccaatccagttctatcccgctttctttctccattacccgtacaaaatcatttacgttcggatgtttgaaacgccactcgttataatagcgtaacaggccgttgtcgcggtttttagcgccaattacataacccagctgttccaggaacacagcgcctttggagtaagcggtaagactgtaaccataattggtattaaagtgatcggcatgtgtggtagcgggttcttcgaacggacttcttgccagcgcaaaatagccggcataagcatcttcctgtgcatcgcggcctttcagtgaatcgactgtgttaaagatcacattgttttccgcgaaggtggtaaagccttcatccatccagggatacaggctttcgttggtagccagcattccctggtaccagctgtgcatccattcgtgcatggctacaccgtacaggccatccattttaccgttgcccatgatgagcgtgcccattggatattccataccgccgtcgccaccttgtatgaacgaatactgctcatacgggtaagcgccgtaatgtgctttgatataggcataggctgccggcaccattttggccagctgaggccaggtattgtgcgtgtattcgttgtcgatataaaagaagtgcgccgtaaagccatccactttctgtgtgatgtgtttgtaatccgggtcggcggcccacataaaatcatgcacattgggcgcaatgaaatgccaggtgagcgttttgccggtgggaggcgttactttgacgcctggtttctggtaaccatggccaatctgatcggggttttgcaggtagcctgtaccgccaatcacatattttttatcgatggtaatctttacgtcatagtcgccccatacaccataaaattcgcgggcgatgtaaggggtggcgtgccatccttcataatcgtactcgcacattttaggataccattgtgacatggagaagtccactccttctgcgttattgcggccactgcgacggatctgtaccggcacctgtgaggcaaactccatgtcaaaaacggctttggaatgcggaagaatcggcttatccagcggcacttccaggatagtttccactactttgaagtcctgtggttttccatcgcgtttcagggagatgattttctggtaacctatttcatctggtttcagttgggagatgcggtcacgtacgcggttatcccagtcgcggcgttcgttccctttcttatcttttcctattacaattttgcccagttcgcggctgcgtacatccatcatgctaccgggctgaaaggcgttccagtagaggtgataaaagactttctttaatgtatcgggggagttattgtaatattcaaggtgttgttgtcctgtgaactgattagccggcgcatccaccttcacatccatcgtatactttactctctgctgccagcggtctgactgagcgcttagttttaaccagctgcccgccagcaaagcgatggccagacagctacctgttgtaacccgatacttcattccgtttcatttggtttaaaacagctaaaataaggatgatttggcgattttgccgttgatatttgatgaatgcgggcggtggaagtaaatcaggagaaactgtggagggtgagtccgagaaagtccgcgtactgttgtgcggctggttcaaaagttttgagtgtggctttttttagtggtttaaacggatcggtagtgatggtgacgctgtcttttttaaagctgcgtttccaggtgccaatgatttgcccgttttgcaccatgatggggttgaagatcccgttgatcgtcattacttttttggcaaactgcatgtctatcagtgtgctgcggtctttataaccgatgaaatattcatcgaaggcgggcagcagcagggcggtgtcatgtgcggtttgtttttttccgggggccatccaataggccgtgccgcttacatccagtggttttaatgcagattgggcgccttccagtccggttttagcatctgtgagcgacaggccggcccattgggcaaagtccggtaaagtagccgggccgtggctgatgaagtagcgtttggccagggtaaccagcgacgtttgtttgttaaatgttgctgtgccgggcagccattcatccaataaggtgtaggtaaattgttttccgctgagggggccgttgcaaataattccgtctgccgcagcatgataaatgatgtggttcatgcggtggtcgtcggtattaattcctttttcctgcagcagggtgatgagttctttgcgggtgaggtggttgcctccctgcagtgctttggcgatgtattgattggttttctgcaggagggcgttgtccatgtccagtttgcgcatcatgctgcccatgcgggcttttatagtgggggcaatgagttggagtatccagcgtacatcggcggccgccaggaggtgcagggtaccgcggaaggcggtagtgcggataatggatttattgctgatcgctttttcgatgtctgcatcagtgctgccggggagccgaacgccaataccccatttgctgttggcatgctcctgtgcctgcatggcgccgaagaaggctactatgtcctgtggttttttgaaagatgttttgagcaactgctgatgctggagtcttaatgcagcaatatcaataacgggcatggctaaatgatttgttatacaaaacaacagcacgggtgtgacaaaggtatgtcagcaaccaacctgaagttaaagataattattcaacgccctgaaccactactacgatttctccttttacacctttttcagcgaagtaatcgtgtacttcctggagtgtgccacgtttattttcctcgaacattttggtgagttcgcggcatacgcagcatggacggtctggtccgaaatactggatcaggtcggagagggttctgagcagcctcatgggcgactcataaaaaacgatagtccgttcttcggtggccagttttgtaaagagggtgtggcggccttttttgagggggaagaatccttcaaaggcgaagcgggtcatagggataccgctgtttaccagtgcgggtacaaaggcggtggcgccgggaaggcattccaccggtacgccggcgcgggcgcattcccttaccagtaaaaaaccgggatcggaaacaccgggtgtaccggcatccgtgagcatggccattgttttaccaccctgcagctgttgcaggaggtgttgtactattttatgctcattatgctggtggtagggcgtaacgggtttattgatctggtaatgccgcagtaatacgctggaagtacgggtatcttccgcgaggatgagatcagcttcttcgagtacttttacggcccggtaggtaatatcggcgaggttgccaatgggagatggaacgagatataatttcataatttaattacgaattacgaattacgaatgtgtggggagatgcagtccggagactttaccagtcatctccccacagctccgttatccgcaattcgcaattaattattgtatttgtacttcaaaagattccattacctggtttgccaacagtttctggcaggcattttcagcgatctgccttgcttcttcctggctggcggcttcaatttgcagagtaatgtgtttaccaatacgtacatcttgtacctggcccaggccgaggttcttgagaccactcattaccgctttaccttgcgggtctaataattctttcagtggcatcacattgatatgtgcagtaaaagtcattgtgctagaaattttgccgcaaacctacatcaaaaaatccagaatgttaaaccgcttctattttgggcggcgccactaccgataatattacgtaacaaataaatataaaaggaacggcagcaaacttcaggagcggtatgctcaccagggtgagcccgatcagtaagaagcggggccagttgtgtgccaggcttttgcttttgaacttcaggctgatcatgggtatttccgccaccatcaggtagcagagcacggcaatggtgatatataatacccagatattctggaaccaatgtgccaggttgaagggattaaataaaaggataagtgggaaagaggccaccagcaaggctactgccggagtaggcacgccaatgaaactttcggattgacgggtatctatattgaacttggcgaggcggtaagcagcgaaacagggtaccagtaaggccggcgccaggttgagaatagatacgtcaaatacgtcgggttgctgaaaataagcgctgcgcaggaggcggtataacatcatgccgggcactacgccaaaggtaactacatcggccagcgaatcgagttccttgcccataggccctgatactttgaggaggcgggctatcatgccatcaaaaaaatcaaaaatccctgcaatcactaccagagcagatgcccagtatacaggttcagggctgataatcgtatagtcggtaccgttaatttccgcgcggtattcaggcgcatgcagtatgcagataatggccagtgcaccgcagaagaggttacatagggtaagaatattcggtatttgtttcattaactgtgattatgatgattttgtgattatcctgatgagcgaagatagaatattgacaattatattatatcatctatcttttaatctttgctaagcaggataatcacaaaaaaacacctttattttttcgccatcagggcttcaatttcatctgccgtgataggaatattcttcatcaggtctacattaccatcggcggtgagccagatattgttttcaatgcggatacccagttgttcttcttcaatataaatacctggttcgatggtcattacagcgcctaccgggataggttgatggaaagaagggccgaggtcgtgcacatccacacccaggtgatgggaaataccgtgatacaggtatttgcggtatgccggtgtttccgggtcctggtttttcacctgttcttctgtgagcagaccgatttttatgaactgtttagtggcttcctctcctaccatttcgtggtatttggcgatggtaatgcccgggcggaggatggatttggcgtagttatgcaggtgcaggcaggcatcatatacctggcgctggcggggcgaaaacttaccgtttaccggtacagagcgggtaagatccgcattgtatccgccgtattctgcaccgaagtccatcaggattacttcaccatccttacattcctggttattagagatgtaatgcagggtgcgtgcgcggtcgccggaggcgatgatagaactataagcttcaccggcagagcggttacgcaggaattcgtgtaaaatttccgcatggatttcatgttcccatacgccgggtttaataaatttcagcaggcggcggaaagttttttccgtgatgtccattgcttcctgcatcaccttgatttcttccggtgtttttaccgcgcgcagttctttaaagataacggctgcacgcaggtagttatggagcgggtagcgtactttcatttcctgtacatagcggtagtcttttaccggtacctggtttgccttgcggttattttcgttggaattcaggtagatgttggcggcttcgttgatccactgttgtaaaagcgcatccaggctatcgagccatactacagtattcatacctgacaccgcatatgcctcgtctttgcgcagcctgtgcccatcccacttttcctttaactcgttgggccgtaccagcaccagtacttcgcggtacttcgggtcggggttatcgggatatagcaccaccatcgtatcctcctgatcaatgcctgtgagccaatacagatcagcattctgtttgaacttgtacaacgcgtcgccattggtgggcagttcgtcattggagttgataatagctatagactgtggctgcattttagccacaaaacgctggcggttcttcacgaacagctgcggatccaagggcagattcttcatatcgcttaatttcaaatgaggcttcaaacctatgtaaaattcgggaggtagaaatatgaaaatggccggaaccggcaaatcggtcaatatctgcaccattaaatgacaaaatcgtactaatatttccttacaattatttaatagtatattctctcaattgtggttagataattccgcaatgaaaagtagacattctgaagatatcgcaacaactacctcaaaccgctatttaatttctaaatttcaatggtataacacctataaaatttgacaatatcaaaaaatcgctagttttgcttttacaccaaaacaatcttgcttttatgcaaatgagtagcgtaaggaatcctgttgctgacttacggggacttggcatagagaacgtaacgaacgtctattaccaactttcacccgagcaactggcggagcaaacggtcgcccgtaaacaaggggtatatgccgattcaggggcattagctgtaaataccggcgaatacaccggccgctcacctaaagacaaattcattgtaaaagacaacatcaccacagacactgttaactggaacgattttaacctccccatttctgaagaaaattttgatcgtttatatagcagaatcacccgttatttcagcgggaaagatgtatgggtacgtgattgctatgcgtgtgccgaccaggattaccgggtcaacatcaaagtaattacagaactgccctggtcaagtctgtttgcctacaacatgtttttacgtccttcggaagatgaactggattacatgcaccccgactggaccgtgatccaggcgcccggctgtttggctgatcccgccactgacggcacacggcagggaaatttctccgtcgtgaatttcaccaaaaagatcatcctcattggtggcagcgcctataccggtgaaattaagaaaggtattttcacgatcctgaattatgaattgccgcacaacaaaaatgtgttaagcatgcattgctccgccaacgtgggcgatgacggcgacacggccatcttctttggtttgagcggtaccggcaaaaccacgctcagcgccgatccttcgcggaagctgatcggcgacgatgaacatggctggactgcgaccggcgtctttaattttgaaggcggttgttatgcaaaatgtattgatctttctgaagaaaaagaaccacagatatttcatgccgtccgtgaaggcgcgctactggaaaatatcaactttttccccggcaccaatactgtgaactatgcggattgccggatcaccgaaaatacccgtgtatcttatccgttgccgtatatcgacaatgccatggagccttctatcggaggtattccaaagaatatattctttcttacctgtgatgcttatggcgtattaccaccggtttccaggttatcgcccgggcaggccatgtaccagttcatttccggttacaccgctaaagtagcgggtacggaagcgggcattacagagccgaagtccacattcagcgcctgtttcggtgcgccgttcatgcctctgcacccggcgcagtatgcacagatgctgggtgaaagaatgcggaaatacaacgtaaacgtatggctggtcaacaccggctggaccggcggcgcttatggcaccggcagccgtatgaaattgtcgtatacccgcgctatgatcactgcggcattgaatggcagcctggataaggaaacattccatacgcatcctgtattcggtttttcaatccccgaccgttgcgccggcgttccgtccaacatcctgaacccacgcaatacctgggaagacaaagccgcttatgacaagcagttgagagacctggccgggcagttcatccgcaattttgaaaaatatgcgggagctgcagcaccggaaatcctggctgcggcgcctaaaatttaataaataaagtactgtgatccggctcttccgttgtatacatcaacaagaagatttatatttaagttttgccttataatttccactgaacaactcgtaagttcctgacgggcgcaatgcctgagcaaagcaagttcctttacaggagcttgttttgctggatcttcggaagatgtaagtccatagctccccgctccttctgacagcgcttccctaaaaagctgattcccatagctgattacatacagctttttcttacctttgcacatgcaaattttagacggtaaactcgtttctgaggctataaaagcccaattagccgctcaggtggctgaattgaaggccgctgggaaaaaggtccctcacctggcagccatattggtaggtaataatccggcaagtgaaacctacgtagcatccaaagtaaaatcatgtgcagaatgcggttacaattccaccctcctgcgttttgatgcgcagatctctgaaaagcatttgctggaccagatcattctgttgaatgagaatccggatgtggatggtatccttgtacaattacctttaccaaaacatattaatgaagagctggtgatcaacaccattgatccgagcaaagatgtggatggtttccatcccatgaacgtaggtaaaatggtaagcggtttacctgcctttattcctgcaaccccttatggtattatgctgatgctggagcattacaacatccctaccaaaggaaaacatgcagtggtgataggccgcagccatattgtaggtacgcctatgagcattttgctgagccgcaataccaatcccggtaactgcactgttacccttacccattcccagacgcacaacctggctgaaatttgccggcaagcagatatcattattgccgctatcggcagaccggattttgtgacggcagatatggtgaaagaaggcgctgtaattgtggatgtaggtattaaccgggtggaagatgccaccaggaaaagcggattccgcctgaaaggggatgtgaaatttgacgaagtggctcctaaatgcagctatatcagccccgtaccgggtggcgtaggtccgatgacgattgccgcattactcaaaaatacctatcacgccactattggtttgaaaggaagtatgaattaaatatagccggaactaaaaaaaccggacctttgtgaagtaagtcatgtctgtaacaacgataaatattagtaccgataccctcccgctgatggagcgcttttacactattcagggtgaaggctatcatcaggggcgggctgcctatttcatcagactgggtggttgtgatgtgggttgcgtgtggtgtgatgtaaaggacagctgggatgcagataagcatccgcaggtagccgttgccgatattgtaactgaagctgcggcttatccaggccgtattgcagtggttaccggtggcgagcctttgctccataacctcgatgcacttacccgttcgctgcataagcagggttttcatacgcatattgaaacctctggttcatcgccgctcagcggaaagtgggactggattactttatcgcccaaaaagtttaaggcgcccctgccggaaatctgcaaggccgcgcatgaactgaaagtggtgatctttaataaaacagattttgcctgggccgaaaaatatgcagccttagccggcaaatactgtaagctgtacctgcagcccgaatgggaacgcagcgcagaaatgacgccgctgataacggagtatatcaaggatcatccggagtggacaatgtcattgcagatccataagtatatcaatgttccatagcgcggattttgtcttggctcaggattacgctgattatattgattttaaggatttgaacactttggattttaaatgatttggggagatataagcggacatttttcgcttatatctccccagatttttataaaaaagtaaaatcaaattttcgcttatatctccccaaatcatttaaaatccaaagtgttcaaatccttaaaatcaatataatcagcgtaatcctgagccaagacaaaatccgcgcgcactattttcacagtattttcgttaattacactgcgaatacatactatgaaaaagacctccctgttaatactgatttgcctgctgggcttcggactgctgttacaagcccagacagttacctatgaaaatgcccctaaaaaagccaaagccagttttgaccgcgctattgatgccgtaagaacttaccagacaaaagctgctatcggatttctgcaggatgctataaaagcggcgccgggatttactgacgcatacggacaaatgggtttgtgttatgtagagctgaaagaatatgcagcagccacttccgcatttgagaaattaaaacaactggacagcagcgggctgcgaccggtgatggtgccctattctaaagcgatggcaggcaccggtaatttcgtaggtgcgttacagttaatcaatcaatacattgcgtccataaaatcgaaaagtgcaaacgcagagaagctgaaagttaattatgaatttgccgttaacaacaaccgtcaggcagtgccattccacccggaaaacctgggtgatccggtaaacagtaaagatccggaatactttccctcattaactattgacagtaaaacattgatcttcaccaggcgcgtaaatggccgcaatgaagatttttatattacgtaccgggacaacaatatctggtcagcggcacaaaacatgggtgaacctgtaaactcctctttcaatgaaggcgcacaaaacatttcacaagatggtaccatgctggtattcacaggctgcgaatttccggaaggcaaaggcagctgcgatctctactactccgaaaaaaccgcttcgggctggaccgccccaaagaatatgggatcgcccattaacacacgcgactgggaatcacaaccctgtctcagcgccgacaaacaaacgctttattttgcacgtgaaacaccagatcatggtgcagatatatttgtaaccagccggcaacccaacgggcaatggagcgtaccacaaaaaatgggacccaatatcaataccaacggcagggaaaccacgcccttcatacatgccgacggacaaacactgtacttcgcctccgacgggcatcccggatatggcggcctcgatatcttttactcacggcggcaaccggacggcagctggggaccagccaccaacctcggttacccgatcaataccatcgatgaagacgcctcgctggttgtagaagcaaatggtaaaacagcctacttcgcctccgaccgctccgatacccgcggcgcactcgatatttaccgctttgaactctatcccgaagcacgccccctgcaaacactctacgtaaaaggctatgtgtatgataccctcacgcagcaacgtttaaccgccagcatagatatcatcgacctccagggcggatataacattgccaccgtgaaaaccaatgaaaccggcgactacctcgcgccattgcccgtaggaaaggattacgccatgcacgtaaacaggaaaggatatctcttttattcagataatttttcactgaaagaacataaccccggtatcccttacgaaaaaaatattccattgcaaccactggctgccaatgccagcatcgtattgcataatatcttcttcgacagcaaacagtataacctgaaacccgaatcggtaacagaacttaataagctggtaaacctgctaaaggataaccctaccataaaaatcgagatcgccgggtacaccgataatgtaggtaccgacaaagacaatcaactgctttcccaaaaccgcgcaaaagcagtagtgagctacctcgttgaaaaaggcatcccgctggaccgccttacggcgaagggttacggcgaaagcgacccggtggccaccaacgatacagaagaaggaagagccgttaacagacggacggtgttccggattatcagcttgtaagcggagggatcggcgcgtaggttgtctttctcaggattacgctgattatattgattttaaggatttgaacactttggattttaaatgatttggggagatataggcggatatttgattttactttttgattttacttttttgattttacttttttgattttactttttttataaaaattttgggagatataagcgaaaatatccgcttatatctcccaaaatcatttaaaatccaaagtgttcaaatccttaaaatcaatataatcagcgtaatcctgagaaagacaacctacgcggcaaacccctgcatcattagtagttgcattagtagttgcgcaaccggctttgcaggatggagtctttttgttgggtggttagtttgtattggaagttgtacaatgccccttcccagtcgccgtacattgggttgggcaatacgatatagcggctgccgaagttgggggctgcgtgtagggcagcggtatttctttcttcaaaaggttttttatcgaaggtggcggagaagtcgccgaggttatcgccaaacagcattacaatttcgtattgctgtaatacctgttgccggcggggttctttgccggaggtggtggttttcagcagcaggtgctgatcgtcggcatcgggaaactggtagcgttgcaggttttgcaatgtaacggctcgttcgctttcggccctgttggtgatgtaaaatacttttacgcctttagaggccgcatacctgaaaaaggaaggggcgccgggaacggtgtctgcggcggcttttgcggtccattccatccagcttttatcatcgtaggttttacctgccagcgcctggtgtacggagtaggggctgttatccagcacggtttcgtcgatgtcggtaactactgccagcggtttgtttcctttggcggcgaggtattgatcgaggcgaagtgccgccagttgataagcctgcagacacaacgccttgtattccccggattgttgctgccataatgccgcccatgccggtccgcccgggatcagtggcgatccggtggttttctctgctgcgggccgggtagttttgcaggcaaacaatcctgctaccattacgcctgtcagtatccatttcatcttcataaaaatatccgttggtagctgcaaaaataattcatgcagtgcagaaaaagtgccgcaggaaaattgtaaattatgcggaaatattgtttgttatgccccaggaactcatgtatcaactggcattaacccgtattcccctgatcggagatgtaattattaaaaaattgctcgagcattttggcagtgccggcaacattttcaacgcgcggaagcaggagctggaaagaattgaaacggtgggcgccatcagggccgccgccatccggaatttccgtgattttacggagatagaaaatgaaatcagttttatggagaagtacaggatacaaccgttattttgtacagacccggcgtatccgcagcgattgcttcattgctacgacaatccggcgatgttatattacaagggctgcgcgtcgttgaatgccccgcggatgatcaatattgtgggcacgcgccatccatccgcctacgggaagagtgtttgtgaaacattggtaaaagggctctctgaggcggggattaccattgtgagtggtttggcctatggtatcgacatcattgcccataaaacggccttaaaagctcaaatacctactattggggtgctggcacatgggctggaccggatttatccgccggcgcataagcaggtagctgtgcagatgctggaacagggtgggctgctgacggacttcccgagccaaacggcgcctgaccggcagaacttccccaagcggaaccggatagtagccggcatctgcgacgccactatcgtgatagaaagcgggatgcgcggcgggtcgctgattacagctgatctggccaatggctacaaccgggatgtgttttgtatccccggcaggcttcatgatctccaatctgccggttgtaattacctgatcaaacaaaacaaagctgccctgctgacgggagcggaggatgtgctggcactgatgggctggcaggagaaaacagctgctgttaaggcgccggtagtgcaaccggggctatttccggaattaagcgaggacgaacagctgattatgtcgcttttccgggaaaaatcgcagcggcacctcgaagaattgtacctgcaaacccgtttatccggaagccaggtggccaccgctgtgttcaacctggaaatgcaaagtgtgctcagaagcttacccggacagctttacgagctggtttgttaatgatttattaacaaccggcagcacctggcgggaagtgattattttatttattgggtaattaggtgtacatttgcgtgcaattattttttaactgattaatagttgcatcatgcctgcgggaaaatctaaacccaaatttgtagctgacggacttacatttgatgatgtgctcctggtaccggcctactctgaagttctgcctaaagaagtaaatctctctacgcaattaacaaaaaacatacgtctgaatataccaatggtatctgcagcgatggatactgttacagaagcaacgctggccattgcgctggcgagggaaggcggaataggtattctccacaagaacatgagcatcgaacggcaagccgaaatggtaagacgtgtaaagcgcagcgaaagcggaatgatcattgatcccgttacgctgaaggtggatgctaccatcggagaagcgctgcgactgatgaaagagaacggtattggcggtattcccatcattgatgaccacaacaagctggtaggcatcctgacaaacagggacttacggtttgaaaaaaataaaaaacgccttgtaaaagaagtgatgaccagcgaaaacctgatcactgctccggaaggcactgacctgaaaaaggcagaaaaaattcttcagcaatataaaatcgaaaagttaccggttgttaacaagcagggcaaactggcaggactgatcacttaccgtgacatccttcagctgaccagctatcccaatgcagtaaaagacgaatttggccgtttactggtgggtgcagcattaggtattactgccgatttactggaccgcgcacaggccctgattaatgtaggtgtggatgtagtttgcctggacagctcacacggtcattctattgccgtactaaacaacctgaagaaattaaagaaaacattccccaaactgcaggtgattgccggtaacgtagctaccgcagatggtgcgctggcactggcacaggcaggcgccgatgcagtgaaagtaggtgtaggacctggttctatctgtactacccgtattgttacaggtgctggtttcccgcaactgtccgctgtaatggaagctgctgatgcactgaagaaactgggtatcccggtaattgcagatggtggtatccgctataccggcgacatggtgaaagccctcgctgcaggcgcttctaccatcatggcaggatctatttttgcaggagtggaagaaagccccggggaaactatcatttacgaaggacgtaaatttaaatcttaccgtggtatgggttctattgaagccatgcaggaaggtagtaaagaccgttacttccaggatgaagatgatatcaagaaactggtaccggaaggtatcgttggccgtgttccatacaaaggtatgttgtcagaaatagtacagcaatttgtaggtggtttacgggctggtatgggtcttaccggttccaaagatattaaggctttacagggagcgcagtttgtaaaaattacagcagctaccgtaaaagaaaaccacccgcatgatgtggtgatcacaaaggaagcacctaactacagcagataagcaactgtttagatataacgcctggtatgaaagtaccgggcgtttttgttttcagtaattccccgcttatcttcgtcgtaattcgtaattcataatccgcaatgcttacatgaagaagccttacctgttgctgagtatactgagtggtttgatttgctggcttgcctggcccaccctgccgtttaccccgcttattttcatcgcctttacgcccctattatatatcagcgataaggtgcagcaccgctggaaatatttcgggcttcttttcctggctttcctcgtttggaatgtggcatccacctggtgggtgggcaataccacccttccgctgagcggcgtttttgccaattgcttcaacgccctgctcatgagcattccctggctgggtctcaaaaacacgaagcggaaattgccggaatctgtggcttactttgcattgatcgtatattggttaacgtttgaatacattcaccagacctgggaattcagctggccatggctggtgcttggtcacgcctttgcactgcggccgggatggatccagtggtatgagtataccggtaccagcggaggcactttctgggtgttactggccaatgttgttatttacaatgtatggaaacgtgcccgcctatacgattttacgtggaaacagatcctgttgggggaaagctggaaaccgctgctggtaattggtttaccgttgattatttctgcctttatatctgccccggtggataacccttcgcagaaaacagaaatcgtgattgtgcagccgaatattgatccttatgatgaaaagttcagcgcaggatcggcgatggagcagcttggaaagtttttacatctcacggaagaaaaagcagatagcaatacccgttatattatatggccggaaacggcattgttcccgcagggcgcctgggaacatgaactgaactatcagccggaaattgtggccatccgtgaaatgctgcgcaaatacccgaaggcgaagcttatcagcggtgctgccactatgaaacgctacctcactaccgatgaaatacccaccaccgcccgcaccatgaatgacggcacccgttgggatgcctataacagcgcgatccaggtagatacttcccgcaacgtccaggtatatcataaatatgagctggtacccggcgccgaactggtgccgtatgtaggctacctatcgtttatgcaaagtgtggcgctggattttggcggtattaccggcagttatggcaggatgccgggtgtggaaatgtttacaaatcccgccgacagcattaacgtgttccccgtaatctgctatgaatctgtgtttagcaattacatggccacccatattaaacccggtgctaatttattagtcattataaccaacgacggatggtggggaaacaccgaaggtcaccggcagcatttacagtatgcccggatacgcgccattgaaacccggcgctggatagcccgctgtgccaatacgggtatatcggccgtgattgacccggcaggaaacgtgcatcagccacaaccctattggaaagaagctgtttttaaagcaactgtaacaccggaggcaggtattacgttctatgtaaaaaatggtgatctggtttcgaaagcggcactaatattttgtatcttgtttgtggtacatgcttttatttcacgatttattcccggcttaagacatgcggaaatcaatcaataacggaaacatcacctggctcgacgaaggcaagggtgcagcgatagtgcttatacacggtttttcagaaaatgccacgctttggcacaaccaaacaacgcgactaaaggagcattaccggattattatccctgatttgcccggcaccgcattatcgccgctcactactccgctgaccattgaatctatggcggagtacgtatatgccatcctgttagcagaaaatatcagtgaagcagttgttatcggtcactcgatgggtggctacattgcgctggcgctggctgaaaaatacccggcactgctgaaaggacttggactctttcattctactgcaaaggcagacagtgaagagaaaaaagaaggcaggcgcaaatccatccggatgatggaacaatacggagcagaaacatttttacggcaaacattgcccaatatgtttagcccggctaccaaaagtaaacataacgaattaatagacgcctatgtaaaactaggcatggaatgccagcttcctgcgctggtagcgtattacgaagcaatggcagtgagaccggaccagacagccgtattgaaaacccttcgggtgccggtattatttatgatcgggaaagatgataatgcagtgccgctggataacgtgttgcctcagataactttacccccggttagcagcatacatatttttgaaaacgtgggccacatgggtatgtgggaaatagcggaagagagcaatgtgatattggaacagttcatcgcattttgtcaacgataatctaaaaacacctgttgtgaaaaaacttcttgtcatcctgctatgcatggtgtgcgccctggtggcgcaggccagtcatattataggcggacaggtatattacaagtttctcgggcagagtggaaacaaccttcaatattccatcacactgaaattataccgcatctgcggcgatggggagcggattgccaaaatgccctctgctgtgtatctttcttcttttgacagaagtgattaccgggcagtaggccagtacaaaatttcacgtaccagctttgaagtaaaaaatcttgcgaagatagatccttgtatcgttaacccaccggtgatctgttaccagatcggaacttacactaccactatttccattccggtaaacgcctcggggtataccattgctttccagagctgttgccgcgatccatatatggaaaatatagtggcagaacctattcccggcggccgtcccggcgacctgggcactggtgctacctactacgcggatattcccggcagcaactccggcgctaccaataattccagtcccgtttttaataaagaagaagctacccttgtttgtgcagacaagaaattcacgtatgatttttctgcgtcggacccggatgcagattcgctcagctacgagttctgcgatgcttataaaggcggtcagaccagtgaaggagatgtaccacctgcagcggtagcgcctccctacagtttcgccagctatgtgtcgccattcagcggcagcagtccgctgggatctaccgtaaccatagatccgcataccggcattatttccggtgtggcgccggcggcgggtaagtacgtggtaactgtttgtgtaaatgaattccgccgcggccagaagattggaacgttgcggaaggactttcatatcaacgttacctcctgcgtgaaactggccacggctgccatgcccgaaaaatatgcagactgcaacagcttaaccgttaccttcaccaataacagtacgctcggaaagccctaccactgggactttggagatggcaccacccttgataccactactgccaatcctattcagcatacctatgcacggcagggcacttatactgtaaaactttatgtagataaagccagcaattgcggcgacagcgccactgctatcgtatatgcgtacccggtattcaagccggcatttaccaccgccggcgcctgtgcgaataaagaaacgaaattcaactctgctcctacccggtccgatgccggtggtattgcgtattataaatgggattttggcaacggggatacttccaacctggcaaatccgccttacacctataccacgccgggcacttataacgtaaagctgtatgcccgcaatgtgaaaggatgtgagcaaaccattacacaaccgctgatgatttatgataagccgccattcacggccaccaacgataccttgctttgtgcaaaagacagtctgcagatgcgggcaggcagcgcacttgccggcagttattcctggacgccggataattactttatcctgaatcccaacgcaccaaacgccgttgtatttccgccgaagtcggctgtttataaggtaacgtttacggatacacagggttgtaccaattttaaagatgtaaaggtagatgtaagagataccatccgggtgcggacgatttccgacagcaccgtatgtaccggtgatgaggtgcatttaccgtccgttacagatgggttgtatacttaccgctggacggacctggaccgcaaccaggtagtgtcgctggtggccgatgcgtatgttactccggctccgcccaaacaaagctatgagatacaggtagcattggggaaatgccgttctgccgataccgttacactcaaagtggtggatccgcccagggctactgcgtctcctgataccacggtttgttttggtattccgctcacgctgcgcgctaccgggggcgcttattataaatggacgccggcttattatgtggataaatccacatcggcagttacattggcccatccgccggacaccaccttgtttaccgtaacggtgacggatacactgggctgccctaaaccggttactgccaccgcgatggtaaacgtggtgcctaaagtaaatgcgtttgccggcaacgataccatcatcatgctgaacacgccgttccagctgaatgctaccgggggcgtgcgatatacctgggcgccgccggacggattgaataaccgcaatatttataatccggtaactacgtataaccgtgatattacatataccgttaccgcctatacgcaggagggttgttccggaaccgacaacatttttgtgcgctttatcaaagggccggatatttatatacctaatgcattctcacccaacggggatggtttaaatgacctattccgcccgttaccggtaggtattgtgcagatggaattcttccgggtgtttgatcgctggggtaagctgatgttctccagtacggcgtatctcaagggatgggatggaacggttaacggcaatattgctgcagtgggtacctatgtttgggtagttcaggggaaagatattaacaataatactgttcaacgtaaggggaccgtcacacttgtaagataaagttggccgaattgaaccgtatatgctctttttgtgttaaattcagagagcagtatcccccatcatgaagagagcagttttactgatattgagctgctgtttgttccctgtttttgcggctggatatcatatcattggtggcgaaattttttataaaacattaggaatgactgaagataactcccgctaccgttatctcatcactctcaagttataccgcgacgcagattttacctgtggcgaccgacaaggttgtattgacagatttgagaacccggttactgctaacgtgtttagttccaatggttccaaagttttatcctccgtttacctctacatcgcttttacccgtccgctgatagataccctgaaaaatccttgtcttgctccgcaggcgcaacaccttgaagtggctttttataccgccaccatcgagctgccacctgttgccggggggtattatgtttcctcccaacgctgctgccggggcgaaaaactgagtaatatctatgattctgaacacgaaggatccacctattatactgtgataccgggaattgagtcgaggcccaataataacagcgcgtacttcgaccgggatactgctattgtcatttgcagtgccatgccgtttaaactggattatgcagcgtatgatgaagacggcgacagtttaacttataacctctgcagcgccttaacggatggttccgacgccaatgaaagcaactccaccacaccgccgccttataattctaccgtaagttatatccctccttattcgggcaataacccgatgggaggcagcccgggaatctccatctctccgcagggactgattacctgtactcccaacctggcgggaaagtatgtagtgacagtatgcgtaaacgaatttgacccggtaaccaaacagttcctgggtacccacagcaaggatatcttactgaccgtatttaactgccagacaaaaattaccgccatctttccatcggtgctgaataactgtacagaagaccctgccttacacgttcctattaccaattccagcgtagccggttatacatctacctattactggacctttggtgatggtaccgatacgctcacggacaccagaacaatgttttatcatcaatatcccgacaccggtgtatacaaagtaaagatggtggtaaaccccgggctggcctgtaccgatagcagcgaaggggaaatatttaactacccgggattaacggcgggctttaccactaccgggcactgcaggggtgatcctgttcagttcaatgatacttcctcctaccggtatggaaacattacaggctatatctgggacctgggcttgctggacagtgtgattacacctgggacacaacggtctatgagatatgtttttcctaaaggtgacgtatatacgatttctttgacgttgctaacggataagcagtgcgtaaaaaccgtgagtaaaaatatcaggatatacgaagtaaatccctttgccggcaacgacactatcctggcgaaggggcagcaaatggtgatgcagggcagtggcggcgagttttattcctggtcgccggcagacgggcttgataatcccaatattgcgcaacccctgttaaactataataaggacatctcttttgcgctgcgtgtatctaatcaacagggatgttttggtttcgactcggtacacgtaaaatattacaccgggcctgatatgtatatccccaatgcgttttcgcccaatggcgacgggctgaacgattatttccggtttattcctgtgggcattactacctataccttcttccggatcttcaaccggtggggagcggaaatttactcctcaacaaatttccgcacgggctgggacggcaccttcaaagggatgccggctccggtggatacctatatctggatattacagggtaccgatttcaatggaaaagagatcatgaaaaaaggaactgtgacgttggtccgctgatccttagtaaattgcacaaaaaaataaccactcatgggaattgttcttatcaccggcgcaactgccggttttggtcaggcatgcgctattacttacgccggcaaaggttatgatgtgattattactggtcgccggaaagaaaggctcgaagcattgcaaacccagttaacgcaggaatttggtatcaatgtgctggcattgaattttgatgttagaaaagaggaagaagtgaaagccgttttaggcactattccggaagattggcgcaaaattgatatcctcgtgaacaacgcgggccttgctgccggtttaagcaccatcgacgaaggcagtacggacgattgggatgccatgatagacactaatgtaaaaggactcctgtatgtgtcgcgcaccgttattccatggatgcgctcccgcacgatgggacatattatcaatatcggttccactgccgccaaggtggtatacgccaaaggcaatgtgtactgtgccaccaaagcagcggtagacgctatttcccagggcatgcgtattgatctgctgccttaccggataaaagtaaccgctattcaccccggtgcggcagaaacagagttttcgatggtgagatttaaaggagatgaagataaagcgaaagaagtgtacaagggatttatcccattaaccgcccaggatgtggcagacgtagtatactactgcacatcgcttccaccgcatgtttgtatcaacgacctggtaatgacgccattacaacaggccaacgcatattacatagataaaaaataacacataggtgtgatttcattacttgatgatagtctttatatttggaaacatttatatattttctgtacataccttaccgtttcgcagaaatcaatgccaatgcagactatcctaaactatgaaaccatatccctatgcttacatttatgactgtgtacttgctgcgtctgtactatccccggtggaaagaaggctggcgcttctatttcggtaattcccggaaaggcaattatggccgttgggcatcgcgtaaagattgggccggacaaaaaggcttttccctgggttacagctgaaacaggtttttaaattttgggatttagttatttgatttcccctttttgattccgggaaacaaacagctaaatcccaaaattattttacggcatactcaacaggcttaccactacttcactcctgttacctgctcttcttttataagccactagtgttttattatcctttactccgctgatcaccgggaaattagcataggtgctgtcggcagtaaggttgcctgcctccatcgttttaccatctgctgctttatactgaaagccgatcctgctattgaagtcgcccttccactttaccggttcatcccatacaatcatgatatgatctgcgatggtagtcatttgcggatgctttgccataggtgatttactcagcgattccttttgcgtataggtgttaccgttatcaacagagcggcagtaaaatgcgccctgtccaccgcccatggtaaaccatgcaaagtgaagaccggtgctgttggccgtaagcgttggcccggtatgcgggcagccatttactacccagttatctgcactgatgcgcacgggagcagaaaaggtgcgaccaccatctgcagatacctggtgtaccatatcacggatagagtcgttgatgatatcgcggtaggccaggtgaatattgccgttttctgccacatacattttagtgcggcagcactggcaaatggtggatgctaccggcattgcatgctgaaaaccgttacggccggcagtggtagcgaagtaaagcgtagagccttcagcgttagtatccttgcggttatccagccagatggcagcagcttctcctcccggcagtaatgccatatcaaaataccgctggtcgcagccggcggtatctgttaccatgggtgcggccggctgccaggttttaccatcgtcgaacgactgtgtgtacattactttgcctgcatatttattccgcggatcattggcttccacaccaaagagcgctatcaccgtaccaccgggcttaaacagcagcttgggtaaattttcatcatgcgggtatacgcctgcagaagcaggaatagcaacgggatctgaaaacgtataaccattatcgttagacactgcatagtacatcaaaccggtatctgcaccactgtttgtttcctcccagctgatcaccgggcggttatctgcatcctttgtaataaacgggcaggacgcatctttcccggcgtgcgacaccactattgccttaccaggttgtaaggcgccggagcggcacgcggctattccaatcatcattaatatccatactgctgcttgcttcatttgtttatttttttccggtgaaggtatatgccacgccgaggttgaaagtttgacgcggacctaccctgtatgttttaccataggcagattgctctgcggtagtggcatacaactggtctccaacgttcatgcaattcagccagcactcaaatcctttataggcatagcccaccctggcattaaaaaggttatagccattgtataaagaagtgttggcaggatccatataatacttactgatatgctgccattcagcgccgagcctgaaaccatttaacagcgccggtttccacgtaacttctgtattcgtcatccacttaggcgcaccgctcatctggttgttattgtacactttactgccatctgcgtaagctttaaaaatatgttccgcgtaagtgccgctggcgcggatgaacaagctacgcaatggtgtgtactttacgttccactctaccccactgtgcgtggtggcgccggtattccggttttcatacacaccatccgcatttcttacgctgataatttcattggtgccattcatgcggtaaatgctcacatcggcataacccttctgctgtgcaaaagcaaaccagccgccggcttcatagttctgataagtagctgatttcagcaccggtacttttacgcctgtatacaattctgaaatattgggcggcgcaaaacctacactataatttgcatacagaccgcggtttttaccgaggttgtaagtgagtcccagcttgggcgtaagcgcattaaagttattccgttcgctgggcgcgccggtataggctgatggtgtaaggtggttttcaaaattataatccatgcgatcgtaacgtaaagcagctaccaccctcattgccggccatggagaaaattcgaattgcgtgtatacggcgctgttaagtaaacctacacggtaatccgtgagcagagaatctgtgttccggtagctcatataatagccggcagcatcttttgtaatatcaatataattggccacgtaggtagcagggctgtaatcggcgcttacccccgcaatgagtgccgcctgtttccagccgaattgttttttgtgttgcgcaataatgccatagctgttaaagccgtcgctgttgatttgtccgcctgctttgagagtacctcttatatccctgatggcataaaagggattttgcccaatggtattattacggaagaaggcggtaaaggtagtatggttgctgttatcccattcatgttccagcgtactgcgtacccgtaatgcctttacttcccggtaggtaaatgtttgaaagctgcggtaatcttttgcaaagaaatgggcgctgtcgaggccaccggtttgatctgttttatagttgatgagtgtagcggcattggtccatttactcttttcattgacctggtaatccactttcgcggtaagtgccagtttatgaaaatcgctgtgatccatataaccattggcttggttggcgtaatagccactcactgcaaatccaactttctttacggtattggatacactgaaatctgttcttttgtatccccaattgctgccttccagctgtatccgggcggtaggcaccaaggttggcgaagcggtgatgaaattaacggcgccgcctaccgcttcgcttccatacagggaagaggccggaccgcggatcacttccactgttttcaatgcggccatattaatttcaatcagcgcattgtggttaaagtcgccgatggttctgatgggtataccatcttccaggtaaaggaacaggcttttatacccgatgggctgacggatcgccatggtatgctgttcgttgcccaggtctaccatgtatacgccgctcactttattcagtactttatccagcgtggtggctttggtttcactcagtgtttgggcagatatagtgctgatagctaccggtgcttccgagcgttgctgcttatcgcgcgaagatgatacgatgatctcattcaggctggtagtgctctggcgcaggtagatcacgggcattccggccgctgattcagcgggtatttgcacaggaacgtatcccacataagatatttctatagagtctgcagcagtggctgttaattcatatttcccttgtgcgttggtattacatccgttgccggcatgcagtagtcttacgttcacacccggcagggcttctttcgtttgtgcatctgccacgcgcccatgtatctgctgtgcataactgttagcaacagccatgcatgcaatgaggagtaaacaacattgtttcatgtatgtatatgtcattgactgttcgccggtggcgaacagggttagtcaggtagtataagttccaaaaatcaggctactaccagctgtggtgggtggaaaacggaaagaatcagtgtatgcgggtggggagctttataatacgagataaaaacgagctgattaacggggggcgtggtgtggaaagattgtaacgtttctacgaacatcacctcatatttatcttttccggtattattatttttgtcttgttgggcgtcccggtcgagctcttttttgagatggcagcggccgttacagtgcatctggggcttattcttattttcacaaagaacgctggcgatataggactggttcactttaaactgcacaaaaaccacacttctgctgaagttttgcagcagaagacccagaaatatgcatataatacccaatcctttcacgccgcaaacctagtaaataattaccattcccctgccaggaaaaaacggatttatagttagataaacgggacagttgctgcctttgttcatctaactataaaatatttttattacctactgtgataatacaaaccggaaggtaataccaccgctggtgctggttatcgggtaagcggtggagataaccggtatggtttgccgacggtcgtagaagaagcgtaaattcaggcggttattcaccacgtagtcgatagaaggcgaaatgcccactactttctggccgctggtaggaatagacaggtcggcatccaggcggttattggccgttttatcgtcccggaaactcagatccagccggaagttcatatcgttttgcagttttttgccaccatttttactgaacgagaatggcatctgaacacctcttaccctgtagcctgctccaatgatgatttcgctggagcgtacttctgtgagctggtaatcgatgaggctcaagctgagggaacggctctttctgaattccaccctcgcattcaggctgttcacaaaagtgaggtccacacccaataacggggagaacgattctataagcgtgaggttaggtaccaggaaataagggaaataatttccggatatagtatccctgaacgccgggaacccggtgagacgcggatcttcaaaatacatggatgtattataggagttcatgctcagcgtaccggtgtaggcgtgcctgatggtaaaattggtgaggaaggaacggaatggttccagcttggttaaaccattgtaggtaatactccagttcggttttggaatataattactgaatggattgctcttcacattatcattgccttgtttcagcagtgataccttatccgggtcggcgccggtatatgccgccaggaaagctggtatcagcacgtcctgcgcataccttgtataaccgtatgcataagccggatctttaggatcggtggctggtacgcctggatctttattgtatggattggcggcgcccagtcgttttgaaatggcgttgcggtatgattcaaagttgcggaaggtttgtgaaataccatccgacgtattgattttaccgaacatggttttgatggcgatgtaagtaatttcaaaaccaccggcatcatatggactcaggtgctggaagtctgttggatctgtgagatttttgaacagttccgtatgtgttttggtaaacgacttcgtcatggtcagatcaatacgcagatcgtttagcggttccagctgggcctgtaagtcccatctttgtgtaaattgttgttgtgcctggatattaaacatggtatccggggtaatgagtcctttctgcgcaaacctgtcgagccatttcctgtcgggctggtaaccaaatacgaagttaagtcccggcgccatggtggcccagttcataccaataattttggtactgtcgatataccctggcaaacgggtaccggcattttcattgtagttaaacccgattcgtttcagcatcatcagtggtttcagcagtccttttacccacggtgaaatttcgctggaagaagcggtctggttctgattggactgttgattgccgttgttgtttttgttattgttgttattattctgattgttgttattctgtggtttcctcgcatttatttcgcgcaggaatttcgatttattatacagttccgtgaatttgaattccgccgtcagtgttttctgctgagagttttcgatcgcgttaccgaggtacaaggccagctgggaggcgcctgtccaccggtattccgtgctgtaaccgaatgcgatgttggtccagctgagtgcggggaacttcgacgtaggcaatgtgtacgtgaagttggcgttgtgcatgtagttggtattacgcccgcctttgaagaagttactgcgtacggtatctttcttcgctgagttattgatacgtccggcgggttcgtcgatgcgggcgttatttactgcgttgaattcaaaattgatactacgggtaagatcccatttaacggtgtagtaccggtcgaacgtaaagtatttattataggtttccgggagcttgtatttcacgtcgccgcctacattacgtacgcgggtaacgccaaactgcctggaaatatctgccctgaagctcaggatagaaggtacatagttgacattgaaatcccgtatcaggtcgagccagtgcgttttacttttgatcagtttcttaaacggttccaggtaatgcggctgaccggcataattatatcccaggcctcccctgtgtttggtgagcatatcattttcaatcaggggattgtgccgcaggatctgggaaaaggagtagctgatatcaaaattttccacatcccacaggtgtcgttttccgccgccgcccaggttgagtttccggacgttggtgaagttgagacttttgatagaggtgaagtcctgtgcatcgcgccggatagaatctttttcccgccggcttctggccagggcaattttatctttcagttttatatccaggtcgtaaggatcatactccgggttgctggccgactgtgagtaaccggcatatacgggaatggagatacctgctttctttggcagcagtttacccagatccaggttggctgcggcatcgtattgcaggaagttatcgcggaaccgttcatttacgcgctgatcaatatttccgaagccggcggtatgcatgttgccggaaacagagatggatcccaggtcggagagttgcacatctacccttgccaatgcagcgtatccgcctttctcatcgaaatcggagagacgcagttcatccagccatacttccgcacaacgtggctgaccgtcatctttcgggttctggataccgatcatcatggtacgggcatctcccaggctggggttaccgattaccgtcataaagtttccgtactggtcggctaccgggttagcaggataaggcaacagcggtgaacaggaatcgcacatgttgcgttgctgtttcagggtgctgagctgcgacatgagcaggtcgagattattacgttccggccagatgtcgagcgctgttttaggaccgttccaatccgttactttcagcgggatgcggtattcataataattgcttacaaagtcgctaccaatgcgaattaccgcctgcacctgtccatctttcagggcagtagcggcgcctaccgcttcggcgtgaatatacatctgcagttttttatactggcggagatccatattcagtgttttgtacaatgcgcggatttccccatcctgcagattacataactgaacagacaacgattgttcattcagttgcagggtggtgttattggtgctgatggtattttgccttactactcccggtggtaacacgtatggtattggtgtacgggaagagttttcttcaatattaacagcagatgaattaaaggtagtggtattatccaacgggataggatcaccgggacgcagttcgtacatataacggcgccattggttacgtaccagttccagtttaccaaaacgcactacgatggagtcgttaaagttggtaaggaacatacgcataaaccggatggatttaaaatccggtatgctgcctattttagcgttgtattggttcaacggtactttgaactggtaccaggtttctgttgttttctggttattgggcaatgtcacatctgcctctactttatccacaataaagttggaacctaccgccatattgggtttcaaatctaccctatactggaaatattcctctgtttcattcatggtattatccctgttcaggtcttctgattcaggaatattggtagcggcggaggagaattgtgatttcgggtcagacaccggggagttaccttccgggttgctgtagttcttatagcgctgcagaatggtgagaccattatataccggatcgcggtaatgcttgtagtcatcattggccgggtcctgtaaagcgtggttatataccgggctgccgccgaaattttgtctcaacgtatccatgtatcctttaaagaaggccccttcgtcctgtgacttcaagccgtcgtagcccacatcctggtagttacggatattggggtcgttatcaaaggcctgggtgatctgctgctggaatttaggtacgcggccccatttggaagagtcaatcttattcggatcctggcggggatcgggcattccgttttcaaagaactttttggagtctttgaggatatcttccgacacgttaccgaggttgaaatacagggaaccgccggtgctgttaggctgttttataaaggggtcctgtatccagaattcgatgtattctatattggctgtttcgaaatcactgttgtcgatagccctcatgataccgccccatttaccctgtggccgtgccaggtgaccgttattgtccatggctatgggggtattggtaaagttataaggacctctttccgtaggatagtaagccagatcgagggtgctcagctggctttgcccgaaatcggtagacctgttcttgaacacttctttctggtataccagccttacccgcgggtccgactgatcatctaccgaaatacctgccggcaggttgggtgattttggtaactggagggtaggttcgatgatataccaggacagttttgccctgttttttccgtaatccagtatattattcaattctgcttccgggaacattaccctgccgctggcgtctgtagcgccttttggcgtagaggcgagcgcccagctggtagcagggaacttcaggtcgtagccactttttacaccttcgaaatcgtcgatataagcagtaccgcttttgctgccgggttcattaaccagtttgctgtggcccgggaataagcgggctacctcaccggtgaacaggatattggaaggggaagtgctgttatagttgggtagtttatccaggaagcggttaagtcctttccattcggaggcgtagtttgcgtctacgcccaccattgtatttttaatggggtcttcgccgtagttcaccttttggtaatagggccgttcgctcatacgcaccacagtacctccgaggcttaacttatcatttaccagatagtccaggcgggtaccaaaatagttccggacctgttgcccgaacagggagttattttcaaactgcacgttgataggtacgccggagttgagtacgcctccattgataattttcagacgtccgaggttataatcaatgatatagtccacattttcgcggagttgctggccgccggcggttactaccactgaccctggcggaatggtggtgccggaaccaaggttgatttccgagctgctggctgatttataggagcccctgatcacgtaccggttcaactgcgggaattgttgggctataactttgatggaatcgtataatacgttgtagagatattgtttttccaggctggcgtcgccgttaaaggctttcttcaatccgtcggcaaagggttccagtacggggaacatgattttacccgacagggagttgatcgtatagccttccacgtagtcgaacacgccatccggctgtggatccagctggttattgaggcggtcgaggctaaggatggtgatgatgggtgcgccggcgtagtcgcctttggcatcggggatataccgcttatcgctggggggccttccttcagcgcccggatctttataatatacgtccatgcggaagtcttccttatttacctggaaggcgccggtagcataaatatttttcatcatcaggtcccataccgggagggtaggacgggcggacgtggctttaagcaatttgaggaacagaacgggctgattggcgctgttgttctggtccggcggtacatcctgggagaactcacccacctggtacacccttccgttgtaggtatattgataggctacagccagtacttcatccggttgcagctgttggttaagggagataaagcccagttgcctgttgtagatgtattcggtagaatcgagtttacgggcgaatgttttttcgaactctgataccggctgcaagccgatattgagcaggcggctcaccactgtcccggtattccggctgcccggatcgctgatcagttttgaatagaggtcgttggttcctctatccggcagcttggagctggtgagtacagtgatatcatccttattataaggctcctgttccgccaggtccatcaaaccaacgatgtcgcgggtttgggtggtggccccggttttattggtaacccatacttccagcctggtgatattgaccagtgacttgatcaccggcaggttggacatggcgctgttgaaattattgcggaagtattgtgccagcaggaagtggcggttatcttcatattcgtcggccctcaggttatagtcctgtacctgggtaccgcctttgagcatgaggttttgtttctgcgacttctgattggagagtacactggtaacggttaagcggccgaactgcaactgggttttcaccccgaaaagcgactggataccggatatgagggtactgcgcaggggaaagctgacgttaccggcttcaattttctttataatttcatcgttgtagccggtgtattccagttttacctggttttcaaaatcgaactgtgactgggtattatagttggtgatgagtttcagtttatccccgattttgccgactacgttcatgttgatgcccatatcaaaattaaacccgccatttttcctggcttgttccaccagcacggggtttttgatattctggccctggtatccgaaagtgaggtccaggctaccttgcgggcggatatccactttgctgcctccgaagatacggtcgaacaggttgttgccattgtacagggtgggtccattggcacgttggttcaggttaccaagtgcgctggctcttttctgccagtaatcctgttcactttgtttggattgcagtttatagaactcgtcgaagttcatataggtagggttacggtaatactggttacctattttttcggtaacggtgtattgtttggtaaccggatcgtattctactgacttgttgatattggaagggtccttgagatcaatagcattccctgacccctgatccgttattttggggccgcgtctgtcttgaagggggtatttcaaggtatcttttttcccggtagtatcgattttggtttgaggagtaatggtggtatccggtttccatctacttctcgataatttcagattcccagaacgatccctagcggcagtatcaacaatgataaaagatacaattgctgtcactacaaatgcaccatagtatgtctttcttgccaagaaaaataggttttatagaggattttatttacttcttataacgttttcagagccttctttatcagttcttccaaattttgcaatagcggctcggttttcatgaccttctggatagatgattctgccataccccgggctatccccagagttatcagagcatttaacgcatcttcgtggattgtattgttcacgtttgcagataaatgtataccggtatccttatgcttcgtcaatttgtctttgagttccaggatgattcttttggctgttttcgcaccgatccccttcacgctttcgagcattttttcattttccatcatgatagcgcgttgtacatcttccggttgtagagatgacaacatcatgcgcgcggtacttgcgcctacccctgaaacactgatcagcaggagaaaaaggcttctttctgcttcttcaaaaaaaccatataacgtgtgtgcatcttctttaatctggaggaaggtcaacagtttgcaactttccatattctgtatacgggaatatgtattcaggctaatctgtacttcataaccgattccattcacatccatatgaacaagagcaggtgatttatatgctaatttaccattcagataagcaatcatacgaggtaaaggttcagtaaattaattaaacttttggaaaatggttaataatgtatccgggaaaaccggggcaaagatgctaacttttaacggattgacaatccctaatatttgtcatatgcgacttttttaggaaatatacgtttatatcgtatttttacgcctcgttttaaacacatatttagtttatatgaataaaataacggccgctattacagcggtgggtgggtatgttcccgattacgtgctaaccaaccaggaattagaaaaattagtagatacaacgaacgactggatattaacccggacgggcatttcggagagaaggatattgaagggagaagggaaaggtacttctgatttgtgtgttccggtagcattggaaatctgcaaaaagagaggaatttcccccgaagaaatcgatctgttgattgtggccaccgtaacccctgatatgacttttccagctactgccaacgtggtaaccgacaaaattggcgctaaaaacgcttttggctttgatatcagcgctgcctgttccggctttttatatgccctggaaaccggcgcccggttcattgaaagtggccgttacgccaaagtaatgatcatcggggccgacaaaatgagttctatcattgattataccgacagaaccacctgtatcatctttggcgatggcgccggtggcgtattgctggaagccaatacagaaggtttcgggttaattgacagcatcctgaaaagtgatggtcacggccgtgaatacctccatatgaaggccggcggctctgtaaaacctgccaccattgaaaccgtaaacaaccgcgaacactacgtataccaggaaggtaaaatggtgtttaaatacgccgtttccaacatggcggaagcagcgaaagatgtaatggaacgcaataaccttacctcaaacgatatttcatggctggtaccccaccaggcgaacaaacgtatcattgcggccacttcccaatacatcaatgtaccggatgagaaagtgatgatgaatattcaccgctatggtaacactactgcgggcactatccctttatgcctgtgggattacgaaaagcagcttaaaaaaggcgacaacgtaatgatggctgcctttggcggcggattcacctggggcgccaactacatcaagtgggcgtacgacggcgatcaatacggtaaataaccttactcccgatattacaacggataacagtgacggatcacccgcagctgttatccgtttgtgttttttacgccttccagcacggccgtaaacaccaggtaccgtccttcactggcggtagccaatacagtccctttcatcttttccataaaatcccgggtaatagcgtagctaagggcatacatatcgtactgccagcagaccagttgctgtaagatctcttctgtagcagggccggcatcggcaatgatgcggatatataccgccccttcgttgttccaggccgacaggatcagcaggctgcccggctgtgcatactgtatggagagccgcagcaggtgcaactgtgcaatacggagcatttccggatccgccattaccaccgccccttccggcagcaggttaactaccaccagtattttttcctttacagcagccgctgtttgttttaatacctgccggaagatatcactcagctggcaatgtgttccctgataagcaaaccccgacaactgcatgcggatccacattaagatgttgtcaaatacatagagcgtgttaccggataccgatgcaatttccctgatcaaagcagccatggcaggctggccggcctcctgattccgcagcttcatggccacctccgaaatataatacagcggtgcgcggaagtcgttggcgatgatggtaatcagcttgttcttaaactcatcatttgcccgcagggccacatttttaagcgatacctgtgtataactgtctgaaatagcatcttcctgttcctgccaggtgatgtattgccggtatctgctgtaaagcaggataaacagcaggatcacaataataaacaggcccgctattacaaactggctatgctttttccgcaactgcacctgttccagctccagttgttgctgcctattgctgcgcgacagctgttgcagggattgttcttttaagaaaaaggccatgtaattaatagggtcctttccctgctggtagcggtgttgcgcggccagccgcatgatttcccggctgtaataaccggttttcacaacgttgttatgccgttggtagtagtcgtacaaccccgccagcaccggcaggttcagctcaatgcatcctgctttttttgccagctcataagacagctcccggtaacgggtagaatctgtatggtagccgagccggtgatagtcttccaaccggttataaatatccatggccacatagggcagtcccctgttcaatgcagcagcagccaggctgttgatcctggcctctgcctcttttccacgtccctgtattaccagtgtatctgctgcgtaagcgtcgatgtacaacggcaaccggctttgcggatacttcttactgatacgcgcagctgtttgtaatgcccattgtacggagtccttacgggtactatccctgtaaaaacgcatcgcgtaatttaccaatagtatactgtagacagaatcctgcgatgccgggagcctggcagccatatgaaaggcttcatagaaatagttattggcatctgccggccggcccatattccggtaatagagatacaggttgctcagcgttttagcgatgcgggcactgtctgatgacgctttatgcagccgcagggcttcgtacccataaatgccggcaacattaaaatctgttctcagggcgtagcagaaactcattacatcgcaggcgtctgccaggccttgtttatactgccatcgtccggccatttcatattccctgatggcatagataaagctgctgtcgaggttaatcatcatgtacagcgccccgagttttcccagggtgttgatataagcgatgctatcctgctgaacagacaactcatgcagcaattccggcagctgcggactttggggaacagcgcgctgtgcagcgcacaacaatgcgagcgccagcaacgtggcggatacccagcgttggtaatatgagttgtttatgctgcgcgtcatgctgtttccggtgattccggcagctgataataaaaggtgctgccttcctcgtaattgttttccgcctttatttttccgttcattttatctataaaatccttgcagatgatgagtgccagcccggcgcctttccctgcacgttcgggctcgctggtgtggctgttccagttaaagagatgcggcagtacagcggcatcgatgccggaaccttcatcaataaaagaaaccgtaagccagttatttttacgtatagccttaattgttattacgccatagtcgggcgaaaatttaactgcgttatgcaaaaaattccggtggatgaactgcaacatttcataatctgcctgaacggtggtacctgcaggaatgtcgatcgataaccggatgtctttcgcggcaagtaaatgctgcagggcgtttgccgtggcgctgatcatttcttccagcaggaatatcttcggatggtacacgaagccggacaattgggtacggatccatcgtaatatttcttcaaaaataaccagggtgtctgaggccgtatgttccacctgtacaatcatgctggcggcatctgttacggtgagcgctttttcatctataaacccggtgatattgacgatgttatacaggggcgttctgaaatcatgcgcgatcatggaaatcagtttattcttaaagtcgtcgctatcctggagcgctttattacccaggcggatctcctcctgcagcgtggccatactggcggcatttttccgggaaaggcggtgggcgcgcacatagtaagtgaggaggatgatgagcaggatggcaatgcccgcaataatcagcagctggtaataccagaagtgatttgcggctttattagaggccagttgctcccgttgtgagtggtgttgcagccggagagagtccagccattcatcgccaaaggcataggaaagataatctgcttcgccggccagcatatcttcctgttgctgctgcattacgccgagggcgaggcggctataactgttggcgttgggagtgtctcgcgattgtaggcaggtgttatacagcccggtgatcacgggaagcattaacccggtgtatccgcctgctactgcatagtccactgatttacgctgatatagcaacgaatctgcctttctttgccagatacaatagcctgttagttgcatgcaggcatacatggcgatgtagttaaaccctgcactgccggccgcggccattacttctttcagggtttcttctgctttccgggtttcgcctgcgcgcagttgttcgtgcgctgcaaataagcgggtgtataaagtacccgggacgtcgttatacctgtgtgtgaggttgatggcctgtttcagtgctttctgtgcaacgggcaaagcggtggaatccgattcattaataaggtagtaactaaccagtacccatgcccgcagggagtctaatcctgcatcccaggcgactttcagtgccttgttaatatagtgctgggcttccgcatgtttttgctggtattgataaaaggtgccaatattcatcagcgatacggtaacccctgcggagtcgccggcagcgcggcaggcagccagtgcattgtcatagaagagaaaggaaagataccggtggggtctcagcgcataataccggcccatgccccgtaatgcgtcgcgttgccctttgctgtaatgaatacgctccgacagttcgttggcgcgcctggcatatgccccgctgctgtccagctgttgcggcagatacaacgatgatatcctgtttagcgcatctgcatagtcagcactgtccgttaaccgtggtaacgcatgcttaattgctacaatatcattatgctgggcgcacaatgtccgcgaaataaaaagcagggcacacaggcccatacggcgtaaacatgacataaaagggaatcagcggcctgtaaaataattttatttacagtcccttcttccatccattttgttcattttaccacctagatttcaaataccaatcccttacgtttcagggcttcatatttttcaggatcgaagcgatacaggtgagccccttttttggaggaggttttgtctttttcctctagtttttccatcacatccagcgacaggatcttcttccggaagttacgtttatcgagggttttctggtagatctcttcgtagagacttctcagttgtgagagggtaaatttctccggcagcagttcaaagccaatgggatggaactgtgcgttgttgcgaagtgcggccagtgcatcttcaatcatctttgtatgatcgaagatcagttccggtatttcgtggagttccagccaatgcgcaccatgttcacgggccagtggcttatcgtggtttttaatacgtatcagggcataataggcaacagatataaccctggcgccggtatcacggcctacattaccgtagcaatgcaattggttcatgtaaatatcattcagccaggtggtatgttccagcacgcgggcggccgcttcatcggtactttcatcttcctgcacaaagccgcctaccagcgaccattcaccggccataggggcaactttacgttgcatgatcaataatttcaggcggccctcatcaaaaccgaagatgatacaatctactgccaccaggtgtttcggggctttagcataaaaagaagcagcattcatataggaattttaaaaggcggaaaatctatcaaaaataacaaaaccaacctattttttcggcttaaaacgactgtattccgtagccggtatcttacttatgcccaacaactctaacatatatacgagttgaccacggtaaaaggtactactgttgcacacctgcatgatcacatcctgcaccgctattttatagtgctcactctttttgagggtgtaggcaacggtgtggttcagctttacctcgctggccttttgtacccattcttccagttgtgccgactgtgtaagccaggcagcgcaggctgacgcaaagctcccgctgaagcccgccgtaggatcggttgttttctccgtgagctgtaaacgctgataccagagactttccgtatgccacaggtgataaacggcagcgcgcaatgtagaaatccctcctcccaggtcccggtccagctgttcatccgttagtttaagtaacccctttgccagctgctggtttgcccaacaattgtaagcagtataatgcgcaagcatatttttcatgtaagaagagattaatgccgtttccatcccaaacaacctacaaattacaatattgtttgtcattttaacccaccgatatttagttgccggtacatgggcatccgtgtaccggaatgcatgacggcgacggacttcgcaattttgattaatttgcagcctgcggccggaggccgttcctgcaaacgggtgtgtataaacaaacggccagggtacctgattaatatatacagatatggaagatataacgttaagggttgcacgaagagaagacagtgcccgattgatggaactgatccgggaactggcagcgtatgaaaaagcatcggaagaagtaacggtgagccaggaacattttgaggaagccggatttggccccaacccggtgtggaaggcatttgtagcctccacagttgttaacgggcaggaagtgattcacgggtttgcgctgtattatacccgttactccacctggaaaggttgccggatgtacctggaagatattattgttacagagaactggcggggccggggcatcggcaagctgctgtttgatcagctgatcattgaagcaaaggaaaagcagttcagcggcatcgtattccaggtgttggaatggaatacacctgccattaatttctaccaaaaatatacggataaatttgatcctgagtggattaatgtcagcatagaactgcaataattttccgctcatacaattccggaacggtatgtcgttaatcctcgttaatattgatgacataccattccactatgatttttatccaggacttccggacacttcacaacgtatccacacccgacctctgcgacactttcaacgcggctttcagcgattatatagtaccgttgcacctcactccgtctatactggaacaaaagatgcagggcgaaaacctgctacgggattattctatcggcgcctttgccgggaatttgcttggcggcttcattttacatgctgtggacgacaaagtgcatccaacggtgttatacaacggcggcaccggcattattccccaataccgcggccagcacctcgtgcagaaaatgtatgatcagtttattcctgcataccagctgcagggtatccgtaaaataatactggaagtaatcagcaccaaccttcctgccatcaaagcatatacgaatacagggtttcataaaacccgcactattcattctttcaaaggcaatataaaaacgcataaaaacccggcgggcatctccataaaagaaaatacaacacccgactggcccctgctggctacctttatggatatgatgcccacctggtccaacagcgtgaacagcatacagcgggaagcgccttttacagtgacctgggaagctactgtggacgggcaaacggcgggctttatcagtgttcacaaagatacccgcagaatcaggaatatagcggttcaccccgggttccgcagaaaaggtgtaggcagcgccttattgcaatacgcagccgatcagtttatgggtgcggcggtgagcattattaatatcgatgaacattttccggagatcgacaaattcctgcaacaggcggggttgatgcattatctgtcgcagtacgagatggagatcgcgttataaaaatgcagcggattttgtctttctcaggattacgctgattttactgattttactttttggattttttttgattttaaaagatcagggagatataagcggatatattcgctcatatctccctaatattttaatcagttataaaatccaaaaaatccaaaaagtaaaatcagtaaaatcagcgtaatcctgggaaagacaacctccgcggcattaattaattccgtttaccaccgtttccttgttgattttctggatcagtccctgtaatactttaccggggcctacttcggtgaattccttgccgccgtcggccaccattgcctgaacggattgtgtccatctcacagcaccggttaactgatcgatcaggttttgtttgatctgtgcaggcgctgttacggctacggctaccacgttctggtatacggggcaggaaggattattgaaggtggtggtgttgatggctgcctgtaactcttctttggcagaagccattaaaggagagtggaacgcgccacctaccggcaggatcagcgctcttttggcgccggcggccttcattctttcgcaggcaatttccacgcctttgagggtaccggaaattaccagctggccgggacaattataattggcaggtactactatttcgcccgtttcggcggtaacagcagcacatatttcttctactttagcatcatccagggccagtactgcggccatggtggagggttgcagctcacaggctttctgcatggcattggcgcggatagctaccagtttcagggcagcttcaaatgacagcacgccattggctacgagggcggaaaattccccgagggagtgacctgccaccatttcgggctgagaatgttccgtgcagaggaaggcgatcactgcatgcaggaatacggctggctgtgtaacgttggtttgtttcaggtcttcctctgtaccattgaacatgatatcagaaatacggaagcctaaaatgtcgtttgcctgttcaaaaagttcttttgcttttgcgttggtgtcgtacagatttttgcccatacccggaaactgggaaccttgtccgggaaatacgtaagcatgcttcatgtggatataaattaatattttttcaaatataaataagaattacggatttacaggtagctgataaatataaattactattatcatctacccataaatccgtaatccgtaatataaattattttatttgctgatcagtttcatgaattcggccctggtggtaccatgttcgaactggccactgaaagcagacgtggtggtaagggagttttgtttttgtacaccgcgcatcatcatacacaggtgctgcgcttcaatcaccactgcaacgccctgcggctgcagggtttcctggatagcatctaggatctggtgtgttaaacgttcctgtacctgtaagcggcgggcatatacatccaccaccctggctattttgctcaggccggtgatatacccgtttggaatataggctacatgggcctttccgaagaagggcagcatgtgatgttcacacatagagtataactcgatgtcttttacaatcaccatttcactatatgcttcggtaaacttcgctccttccagtatttcgcgcgcgtcctgctgatatccctgtgtgatgaactgcatggctttagccatccgttcaggtgttttttgcagtccttccctttcagggtcttcccccagcaggtgcaggcattctttatagttttctacaagaccggacgtgatcttttcatcgtaactctcgttcttattatacgccattcttatatgatttaacaaatttcaaaggccggtaatatacaggcattacttgccaccatagtactccacgtagatgcgcggggtttcatacagtttgatacaatgcagctgcacttctgcaggcaggtgtttggccagctgatcccagatagcgatagataaattttcagcggaagtgaatttatctttcataaaatcaacatccatattcaggttccggtgatcgatcttttctatcaccgcatcccggataattacccctaaagtcttggcattaaatacaaaacccgtttccggatcaggattaccttttatagtgacgtgcagttcgtaattatgaccatgccagttctcgttggcgcatttaccgaaaacttcttcgttcttttctttgctccagcccgggttagataacttatgcgcagcattgaagttctctactcgcgttaaataaatcattattgcaaaaaatttttgcaaaaataccactattaagtgagtagagccaatttatcctaattcctgtcaattgttttacatggggagcaatcatttttgctgtatttttacgggatgaaaatattggtgaccgcggctaccacgctggaaatacagccttttttacagtacatcgaccagcacattccggcccttaaagccgcgaactgcaatatagacatactgattgcgggtattggcatgatgcacaccgctttcagcctcgggaggcacctggtggtaaaccggcccgatatagccatacaggcgggtattggcggtagtttccgccacagctgggagctgggacaggtggtactcattaaacgcgaatacctggccgacctgggcgcggaagacaacgatcagtttaaagatttatttgatatacagctctggcagccatcacagccgccctttaccggtaccagcctggtgaatacctttgccggattgcccgaagtacctcccctgcccactgctaccggggtgagcgtaaacctggtaagcggcagcgagcctaccataacaaagctggtgaccaaatacaaccccgacatagaaagcatggagggcgccgcctttcactatgcctgcctgttggaagaaataccgttccttcaactgcgcagcatctctaactatgtggaaatcagggataaaagcaaatggaagatccccctggcaataaaaacactcaacgacgaactgataaaaaccgtggaaacactggccggcatttaacgacagactataaaattttgatagctatgcatttatctttaggtttttcaccttgcccgaatgatactttcatttttgacgcactggtaaacaacaaaatagacaccggggaatttaccttcgatacccacctggaagatgtggaaacactgaacaactgggcactacaaggcaaactggccattacaaagctgagttttgccgtatacctcaaggtaaaagatcaatacgaactgctcaacagcggcagtgcactgggacgtggttgcggccccttgctcattgcaaagaaggatattccccgcgaagagataaaaaatctgaccatcgccattcccggagaaaacacgaccgccaacctgttgttctccatcgctttccccgaagccacgaataaaaaggtaatgctgttttcagaaattgaaaacgctgtgctgaacggtgatgtggatgccggcgtgatcatccacgaaaaccgcttcacttaccagctcaaaggcctcgtaaagctgatggacatgggcgagtactgggaacaaaccaccggtaatcctatcccgctgggaggcatctttatccgtaaagatgtgcctgaagcgacccgtgcacaactggatgcgctgatccataaaagcctgcaaaacagctatactacttaccctcagctgtctgactatgtgaaatcacatgcgcaggaaatggatgaatccgtgatgcgccagcatattgatctgtatgtgaatgatttcagcttggacctgggcgaagaaggcaaagccgccgtagtagcgctgatggaagcagcggaaaaaatccgcccgtaaagcagccgattttttcgttcttttgttgcggtatgatcgagaataaggatacagacctgtggaacaggttccggcaaggagaggaacaggcgctatataccttgtatgaaaagtattatcacctgctccttttcctgggccttaaaatatgcgcaagaagcgaaccggtaaaggattgtatccaacaggtgtttctttatttctgggagaagaaagaaggactggataccgtcaccaatgtacgcagctacattatcacctcctttaaacgcaaactgttattacatcttcagcaggaaaaaaaggacaattgcctgttgtcgctatggatggataccgaaaccggcagcgacattccttctgctgaacaattgctgatgcagcaacaacaaaacaaagaagccatcggacgtatacaggaagccatatctttactgagtccgagacagaaagaactaattaacctccgcttttacgaaaaccggagctacgacgaaataacagatatcacgggccttacgcaccgcactgtttacaatcacttgtacgaagcactgaaatcactcaaacaatcactggaacaggatcttaaatccggcaacctgcatttgagaactttactgctgttacttcccttataatttccctgttagattattttcaataaagcctctttaaaataaaatttatcaaaatctgaaaatttaccggtccgtacccggtaaaagagcaatgattgtcgctctactttaaaaatagatggggaatgctgccaaaggacctgactgaattagacctgctgctcgacgacacctttctgcaatatatccggcgaaacaacgacacggctattgctaaatgggaaagctatatcctgttgcatcctgaaataaaggataaggtggcagcggcagtggcgctatattataacatcaatacggttgaggcggaaaaagacaggacggtacagctaaacaggctgcaacaggcgatcaaagccactcacccagcgcgtatccggcggatcaactggcggcaggtggcctggcgcgcagcagcagtactcctgctcgtgggaggcgctaccctgttatggccccggctaaagccacggaagcccgcaacggcccccaacaccttcctggtgtattccagcgaatggggacaacggaaattgctcaccttaccggatggctcttcggtaattctcaacgccaatacaaccgttaggattccttctgattacagtaaccggcaccggcatgtagaactggtaaagggcgccgccctgtttgatgtaaaaacaaattccgatgatccctttatggtaaccagcaaacagatacaaaccactgtgctggggacttccttcttaataaaatcttatccgtatgagccacagtcgaccgtttcattactcagcggaaaagtaaaggtaagtgagcaatcgggtaaggcagatccgctcacactggcgccgggggaacaggcgcggtggaatgaatctacccggaaaatgagcaggtcaacatttgataccattgcattacgcacctggaaatcaggaaaattagtgtttaacaatgccagtgcttttgaagttatacgtgaactggaaaattggtatggaatacctttcgaggtaaccggaaattcattatatgccaaacggttctccggagccttcgacaacgataaattagaaaaagttttgaacatcttttgttttacagccggatgtagttttcaaatacaaccggacaaagtgctgattcaattttaataacaaagcgtttccaccaaaatcgctgaaaccgggatcacatgcaggctgccggcgcctgtagtgaccatatcaaccatcattaaaaaatctgatgcatgacttttaattatgcgcgcctgcgtgcgccgttaagcactgcagtaaaatggcagttccctcttttggtgttgttaatgctgatgatctgtatgctatcatacgcccagcaaagaaaatcaatagcgctccgggatgtgacaatttctaccgccttcaaaaaaattgaaagcacctaccaggtaaagttcttttatgacgccgccaccctacccatccggcatgttaccctggccataaaaaacaggagcatccgcgaagtgctggcagagctggaagatgcttccggccttcaattccgggtaagcggtaacatgatcggcgtagtaaagccttacaatccaaccggcgttacaaaggccctacccatgataagaggaagggtaaccgaccgtcagggacagccgcttcccggcaccaccgtgcgggacattattaccggcaaaggcaccgtaacagatgccaacggcatgttcgctgttagtgctgaagaaggccacccgctgctgatcagcagcatcggctaccgccagaaaacgcaggtagtatccgggaaagaaaatcatatttcgatggaggaagatgctaccagtcttggcggcgtagtagtaatgggctataccaataaacaagcggctgaactaaccggcgctgtgcaaaaagtttcgggcgaccagttgcgcagctctgtttcttcttccaacatcctctctatgctgaaagccaaaaccaccggcatgtacatcgtggaacccagcgccgatgccggcgcaaggggacaggtattgctgcgcggcgaatcttccctcccatccggtaccagcgcttacttcggaccgctgatcgttatcgacggcgtgatttccaattcacagaacctgcaggatgtagtaaatccggctgatgtggaaagcgttactatcctgaaagatgctgcgtctacggccatctatggttcacgcgcggcacagggagtcattgtggtaaccaccaaaaaagctgccgccaacagcggggtgcatgttacactcgatacccgttacggcgctattaaacagaaccgcgccatccgcatgatgaacaccacagaaagtactgcgctgatggataaagtaatgcaacgcagatgggaggaaacaccttctcttcagcaacaatttcctactgcagcagattttattcagcaaagaaggatttatacagatgaagataaatccaagaacttcgactgggaaaaagccatgtttgatgatggtgatttttctgatatcagcctgggacttaacagtggcaatgataaaacaatggtgtacgcaggtgtaaactggtacaaggagaaaggcattaacattggtaataccttcgatcgccgtaacctccggctcaaccttgtccagaacttctccaaaaaagtttccggcggattgaacaccagtgccatcatcgataaaaccatttcccgcaatggtgtgccggcactttatatgactcagccttttgtaacgccttacaatgcggatggtacactggccgacagtatcccggtgaggcaatccaataattttggtgttccttataccacctggtcacagaattttttagccgaaaagaaattcgataataccgcggttataaacaaccagcacttcactggtaccgcgtggcttagctatcgcgtattgccctggttaagtcttaaaaccaccaatactatcgattatatcaatacccaccggaactcatacctggatccccgtagcttctccgggaaatatggtggttatccttacctgtttgctcctggcgctgctactcctaatggaacccttaccattgcagataccaggttctttaattttacctccacaaatacactgaatgcctccaaacagtttggacagcacagcctgaatttcctggcaggaacagaatgggcaaggcgtaacagtgaaaccagcagtacagatatgtataacctgctgcccggtgaaagaaacatgggcgcagcgaaaaatttcggtagcgctatcaatgtggcgtacaattccccctaccggccctccggcgggtatacagaaagagcgagcttctccgcttttagtgaattaaactataactacctcgctaaatattatgcagcagcctcccttcgtaccgatgcctttaccaactttggccgtaataaaagatacggtactttttatgccgtaagtgccggatggctgatcaacaaagaagctttcctggcagatgtgaaagcaatagacctgctgaagctgagagtagtacacggaacttccggcagggatgtaggcgatggatacctgaaccaaaccctttatgctgctgccagcaactatacctacgacaacgttaatagcattggctccgccatcacacaactggaaaacccggatatcagctgggaaaccactgttaacaataccgccgggatagacctcagtctatggaaacgcgtggaactcacggcggacctctactccaagctcagtaaaaatctgctgcaacaggtattcgtaggttctgcacaaggatctttccaacagtatcagaacgtgggagaagtattgaacaaagggctggaactgatgctgaacacccggaatatagatgcccggaatttcagctggaccaccaacctcaatgtgagctttaataaaaatacaatacagaaattatacagcgattctcttcttgataactacaaccgcgcctattaccgttatgaaggagaagacctgaacgtgattaaagcgatccgctatgcaggggtaaatcccgacaacggcgctccactatttgaaaattatgacgcatccggcaagaagcaggtggtggaaggcattggcgccatgtcagatatccgcaattaccagacagtgggttctgctacacccaaattctttggaggtttcaccaacacttttacctacaaacaattttcgctgagtgcagagatgtggttccaggcaggcaactatactgcgatgagccttatcaacaacttccaggatcctggtgcgccgtttctcggcaggaacaatgtcaactggcaatccagccagaaagtatggcaacaacccggtgataaaaatgccaactaccctgacgtgtacagcagcaagatgaatacctggcgggcattcgacagccgctcatcgctggtgtatggtaacgccagccatatccgcatgcgcaacatcaggatcggatacgatcttgctcagaaaacactggcaaagatccacgcacagcgtgcaggcgtgttcgttagtatggacaatgtttttgttatcaaacgtaaagactatgtaggcgcagatcccgaaggtgcctccatcggcacgtccacttcctatggaggagtaggtatcgggaacgcaaatccacggcgcattactgctggtcttaatgttacattctaaactactgaaaaatgaagcgtacaataataatagccgccgtcagccttatttcattaagcgcctgcaataaacaactggatgaattacgtccgcataacgtcatcaacgaagatgcccagttcagtactcccgaaggattttcccaggcagcactgggtttgtatccgatgatcacctcgggtgttgccatggaaaacagcagctttggatatggtgatgttacgatgttcctttcggaaacacacggcaacaatatccattcactcgatctgggtccgaaccgttactccgatgcgttcgattataccaattcgcccgataaagaccacagctggacttactacttatggagagggagttactttaccatcctgcacgccaacaagctactggataatgtaaccaaagaggaacaacgtcctgccgttttacaggcgaaagcagaagcgttgtttgtgagggcgtttgtatactttaacctggtgcgtttttatgcaaagccttattaccaggacgcagcaggatcgcccggtgtgatgcttattaccacggcggccaacggcaccggctataagcccgcgcgtgccagtgttaaagccgtgtacgagcagatagtttcagatctggaaacagctatccccttgtttaaccaggaaaagtccaacagcttcgccggtaaaatgagcgccgctgctttgttgtcacgcgtgtacctttatatgggtggcacgttccaacaacccgacgccacttttaaccagcaggcagtgagttatgctgaccaggtgattaacagtaacaagtacaccctgctcaccggcaacgactaccgggcctactacaacagcagcaatgccgccaataaggaagatatttttgcaggcaatacggattatggcagcacctctatcagccaacagtacgcctatccgccgcagatcaattatacgggcggttactaccgtccttctcccgatttgctgacgcggatcagcacaacagatctgcgcacatcgcactataaagtaaacgtaactcccggctttccaaacgacagcattgccacggccaagtacatgtacctgtacaccgccatctacagcaaatcgccgttccggtacatccgcctcgcggaagtatacctgaaccgcgcagaagccaatgccaagctcggcaaaaaagatcttgcactggccgatctgaatatcatccgtaaccgcgcagggcttgtctccgtagatctttccgggcaggcactgttggatgaaatcctcctgcaacggcgcttggaactcgcctttgaagggcatatcggttttgattttttcaggaatggattaccgatggtacgcaactatgcttctgccagcagcggcgccatgacgattgccgccaccagcccgaagatattactgcgcattccgcaggaagaaattatcctcaatcctaatcttacacaaaacgaacaatagcattatgaaaaaaataatttgcgtactatcgttaccgttagcattcagtcagctggtaaccgcacaacagaaattcagtataaccggtaccgttaccggcaatgcgcccgcgaaatactacctgcagtatagcaatggcacgaaatacattaccgatagcgctgaagtaaaaaatggcaggttcggctttgcgggtactttatcgcagccctcacccggcgtgttttctgcagcgctgatcaacaacatgaccggcaacaaaaaagagcaggcttacctcttcctggaacccgccgccatgacaattactatcacaaacggtgacctcagtaccaccgttctgaaaggctctgtaagtaatgacgaaaatgtacaactggagaaagaaagagaaatcgctactgcaaaataccagccattactggaagcactacggaatgaaaaggaccacgacaaagccggcgctatccgcgagcaactggcgccttactttgaaacaaacaaccagttgtccaggaaatttatccgggaacatcctaattctttcctgagtatttatctcatgcgcttccaggtaggcagcatgacactcgattctgccaaatattattacaacggcctaagcaccactttaaaacaaagtaaaaatggtgtggagatagcgcaggagattaaaaaaattgaacaaggttcgccgggcagcgttgcctttaatttcagtaaagcagatatcaatggccagccactcagtttatccgatttcaaaggaaaatatgtattggtagatttctgggccagctggtgcgtaccgtgccgcgcgggtaatcctcatctgctggaactatacaaacaatacaaggataaaggttttgaagtgatcagcgtgtccgacgacgaccgcaatcatgatgcctggaaaaaagcggtagaaaaagatggtattggtgtatggaaacatgtactgcgcggactggacatgaataaacgcctgaagaatgaacctaacccggatgatatcagtgaacacttcggcattcattctttgcctacccagatattaattgatccgaaagggataattatagcccgctatggcggcggcggagaagaacatgaggcattagacgttaagttgaaagaagtatttaaccactaacattcaccataaaaaagcagtggagatgaatgatcatctccactgctttttttattatttcttcagtgcttttccatatacttccaatgcgcgccggcgtgcttcttcatgcaacacgatcggtttagcatattcaaatccttcaaattccggcacccacttacggatatattttaaatctttatcaaacttctgcgtttgcagcgtgggattaaataccctgaaataaggcgcagcatcacatcccgaaccagctgcccattgccagccaccgttatttgcagcaagatcatagtctaacagtttagctgcaaaataagcttccccccaacgccagtcgatcagtaaatgcttggttaaaaaactggcggtgatcatgcgaacacggttgtgcatgaacccggtagtgttcagttcccgcataccggcatccactatcgggtacccggtttgtccttcacaccatttctcaaactccgcttcattattacgccatactatcttatcatattctttcttaaaagaatttcctactacatgcggaaaatgccagaggatcatctggtaaaactcccgccagatcaattcctttgcaaaagtggcattgagctgcatggcctgctgcattaatgcgcggatgcttaccgtaccaaaacgcagatggatccctaatttggaggtaccattcacagaagggaaatcacgggtttcatcgtagtgtttaatcagtgcttctttcaggtcttttgccggaaaatgtttttcacccgctgtaaatcccatctcttttaaggagggaatttttacaggggattgtttaaaaagatgctggtaatattttttacagggataaggtttcagatgaaaaaaggtgagggtgtcgtgccattttctgctgtaaggcgtaaatatcgtatatggttcaccgttatctttcagcacttctcctttttcaagaatcacctggtctttgtagttgtgaaaagaaacaccctgttcgctgagctgctttgctatggcagcatccctgtttcctgcatagggttcataatcatgattggtgtatacgttggcaacgttgtatttggcggtccagtgcgcaaaagcagcctgcggagtaccataaaaaatgtccattgaggaacccagctgttgcagttgctcctgcatatcctccagtacttcgtgaataaaggtgagcctgcgatcgtgtttatcttccaggtcattgagaatgtgggtatcaaaaacaaatacgggtactaccgggtttccggcacgtaatgcataatagaaagcggcctggtcgtccagccgcagatcacggcgaaaccagcataaactgattttttgttccatgttaacggtgatttttacagcatgctttcatgtaatacttcgtgcaaaatagcggcggtggcgttaccatagctgctgtcgcggaagaggcccacccaacggatgccatagatggcgttggttaaaaatatttcatccgcattttcgaggtcttctatattgagtggtttttcttctattttgaatggcagttctgttttcagcaggaacttgcgcattacaccgcacacaccgccttcagacagcggtggcgtataaagtactttatcccgcacaataaatacattggcgatggtgctgtcggcaacccttccatatggattaagcaatatcgcttcattcagccggtgctgcttggcatacatggcagccatcacataaggcaggcagttatttgatttaatagcggataatttatcacagctcttttttacatccgggaagatgtctgttacgagtccgttatcgtttaattccaatactgttctgcttaattcccagcattggataatgtagtttggtaagttattgatgggatcgtataagccgccatcggagcggaagatagccagccgtacgcgggccatctgggatatatcatttttattgcagagttccagtatctgcttaacaaaatatgctttggtaaaatgtgtggggatatcaaaatgcagcaggtgtaaactggcgagcatccgttcaaagtgcaggtcagccagcaacacttgtccctggtatactttcagggtttcaaaaaagccatccccgtatctgaaagatcgattatctgccgtaaaaatcgggtcggctgcgggaatatatttaccgttataacagagaaatccaacttgcacctcgaactattttagcagtttgaaaggtaccaattatttaggtatttttaagtttagagatttagacattttgtttcagtgaagtatgtattccaaaaacaaaacatctaaatccctatacaggttacgtattatttacggagttgcaatcctccgaaatgcagacatacaaagccatccggccgatgagaagatcctatgcttcagctaaattttcatctccgggatatctccttcaatgatcagcttaccggctgttttagagcggatttcctctacggtgacaccgggtgcacgttccaggagcttaaacccatcgggcgttacatccagcaccgccagctctgtaacaattttctttacacagttgacaccggtaagcggtaatgtacatgccggcagcagtttactttctcctttgggattggtatgcatcatggctacaatgatgttcctggcagatgccaccaggtccatagcgccacccatgcctttcaccattttacccggaattttccaattggcaatatcgccggtatcggaaacttccatggcgcccaatacggtaagatctaccttaccagcgcggatcataccaaagctttctgcggaatcaaagaagctgccaccgggaagcagggtaactgtttcctttcctgcattaatcaggtctgcgtcaacgtcatcagcggcaggatacggtcccataccgagtatcccgttttcagactgcagcataatagaaactccggcaggtatatagttggataccagcgtaggaataccaatacccaggtttacatacataccatcctgcagttcctgtgcaattctttttgcgataccatatttatcgagcggcataaaatatcagatttgaagcgtggagaattggatgaactagatcttaacggttctgcgttcgatccgtttttcatagttgccgcctttgaaaatgcggcgtacgtaaatacccggcacatgtacctggtctggttccagctctccgggttgcaccagttcctccacttcggcaatagtgatttgtcctgccctggccatggatgtgctgaaattcctggtggttttacggaacatgaggttacccaacgtatctcctttccaggcttttacaatagcgtaatcggcgtgcagcgccagttccatcaggtgaggcttgccatcgaatacccgaacttcttttccttcagcgatctcggttccgtagccggcaggcgtgaaaaaagcaggaattcccatgcctgccatctggatacgcgtagccagtgttccctgtggaatgaggtctacttccagctctccggccagcagttgtctttcaaattctgcattttcaccaacataggaagacatcattttcctgatctgcctggttttcagcagcaggccaagaccaaaatcatctactcccgcgttattggaaatacaggtcagatccttcactcctttttttaccagggcggtaatacaattctccggaattccacacaaaccaaaccctcccagcatcagtaccgctccatcccggatatcttgtatggcttcatcggcatttgctactactttgttcatgttttggtgttttatagattagggctgccgcttgataaaaggccggggtgtatccgccttcggcagcaatagtacgctgtctgcataggggaaaatgcttttcatacgaaaccggagcggtgcattttcatcgattggattgggcaaccgttgtttcctggaagcaatatctgtttgtaccatctggaaaacttccttcagcctgttgggatgactttcgtaataccggtagctctccataaattccttcacgcttactttgtgcaggtccagtatctgtttgtaatagacctttactttctcctgccggagggaatcgaaattgggcgtataagtaacctgcatttgttgctcattgctgtaggcatctgcaatagacatatctaccaggatacctgtcatacgttcctttgaaatatatttacccgacacctggtcgctgttggcacaggcaaccaggaataccactaacaaagccagggaggcgtatttcatcatcatgttcatcatagcgttacttcatctgttgatacttctgtgcattgggcacatccatctgggagagcaattccgctgcacggcttttctcctgtggtgtggcacgggagaatatttttaatagctcctctcctttggagaggaagaaggtttgcatcagcatggaattggggatatcctggtggatggaatagagcatattcaggcagttcagaatggctgcacggccttttatcacatcatcatacatcaggtccaacccctgccggtgatactggtacattacatcatggaaccggaggaacttggcgttcagcaggttatcctgtaaccaataacggttgcggtttccttcgaaagctttccatccggaaatctcctttccatccggtgcattatttacaatattaagcgctttcttaaaatatacatctccgcctttgggggagaaggaatcataatcgagcccgaggatgatattaacataataggccaggatagcggttaagttggaggccagcggatcatttcccaccaccctggtatcgctgaactccagctgctggaattccacgtaccggaacaccacattgggatcctggatattcagcaaactcgttacatagctggcgttatataccggcctggtggcctgtatggtcagggtagccttgtaactgtcgttccctgaagtaccggtgatgttcagcaaaaagttacattctatccgttcagccggtgtaaaggcatcgtttgcccaatgccggttattgaggaaatcccggacggaattctgcagggtagtaaatatttttttgtctacgccctgtatctgttgggcaactacagacacattggcccttatttcctgggctttaacggccggggagcagcatagtaaaaaggcgcctgcaagcagcaggaacaacgggaaacgattatgcatgttgcaattcgattatagcggaaacaatatcctgggccacggcctgtttggatttgagggggaaactgcgttcattcccgtttttgtcaaacagggttactttattggtatcatagttaaagcctgcaccagtatctgccagtgaattcatcacgatcaggtccaggtttttatcacgcagttttttcagagcatattctttttcgttgtttgtttccagggagaatcctatgagcaattgccccgggcttttattatcgcccagcgagcgtagtatatcgggtgttttttcaagatcgatatgaagctgggcttccccttttttaatctttttgtcggccacatttgccgggcggtagtctgctacggcggcggcggccactactattccggcgccggaatagcgggccgttacggcatcaaacatttcctgggcggtttgcacatgggtaatggtgataccggggtgggttgttttctgggaggtgggacccagtaccagctgtacatcagcgccggcatctgccagggcttccgcaatggcaattcccattttgccgctggagtggttgctgatgtagcgaaccgggtcaatatgttcgatggtagggccggctgtaacaatagcagtggtaccgttcagggctttttttccgtttttctgctgaaaatgctgttgcaggaaagtcaggatctgttctggttctgccatgcggccttctccaaagagtccgctggccagttccccggattccacgggaatctgctggtgaccgaaagaaatgagcttttccacattgctgcgggtagccgggtgatgccacatgtcttcatccattgcgggggcgaagagtacggggcaggttgccgaaaggtataccgccagcaggaggttgtcgcacaggcccagggccattttggcgagggtattggcagaagcgggtgcaatgagcataatatctgcccagcggcccagcatcacatgattattccagctgttgtggtcgctgatattcaggggaacctcgtttttagagagggtggccagggtgaggggggtaataaagccggcggcggcggtggtcatgaccacttttacttcggcaccttcctttaccagcaggcgtatgagggtagcggacttgtaggcggcgatgctgccgctcactccgagcaggattttttttccttgtagcattttgatagcgtccatggacatatataaaaacaaaagcggcagaaatcattctgccgccatgaaattaatatttttatttttcgcaatcacgcacctcacaaaataatgtgtggcggattagctaaacaaatcgtcgtcgttcttgcggaaataaattttgctgtccaggaactcctgagtagcctggatggccggatttgccagtctttcataaaaacgggaaatctcaatctgctccttgttctcgtgcacttcttcgaggttgtcagtatgactggcaaactcttccagtttggaatggagctcctctttcacggaaatattgatctgattggcgcgtttggctattacggcaatagactcatataaattaccagttctgttcttaatgtcggtagtatttttagtttctacccagggattaaggctactggttagacttcgctttaatttgctcattatccagtgtttttatgttgttttgtgctaaggtataaaatttttcggcatctggctttaatttgctgttcgggtagtgatccgcgaagtccaggtattcgtcgagaaccgttgcgtagcgctctttttgtctctccggaatactgtttttagcataattatagtaagatctgatggccattactttgtaactgtcgcttttatcagagtcggggtagttgcgcatcaggtttttgaaggcaataccggcggctttgaagaagcccaggttataatatagctctgcgctggagaattctttcttttccagctttcgtctgcacaactcgattaccaggttggcttccgacactttatctgcggtagggtagttattaatgaaggtttgcatggcagcaatggccttcatggtattagtttgatccagtgatacctttggcgactgcttatagtagcaataagcctgcatataatctatttccaccgctctcgggctgttcgggaacaggtccaggtagtttttaaactggaaggctgcctgaacgtagtccttaacgtagtaagagcaatatgcgaaattgtaatacatgggctcaaacttctcagttcccttgtacacctgaaccaggtcagtgtagagcgttattgccgtattgtattttttcttctggaacagctgattggcgtagtccaacttcttttcaaagttgttacttttttctattctccgtaactggttgttacaggaggtagttacgacaaccgcaagaacactgatgtacaataaaaatttccgcataaaagagtggcaaaattaagaattaaatgtaaatgtaaggcagagagattttgattgctgttaaaattttgcaaaagagggaattaaatcgccgaaagacgggttttccaccaccgccggggttgctgacatttttcccaccccgatgtggaaaaattgatttcaggtaacggatgtacctgaaaaaagggctcagattataaaaaaaatccactcataacgatttcttcaccccattttcccacccgctatgctattcgggaatgtcttatcccatggggcatctgcaagatataaacacataattcacacttataaacacgttatccacacgtattattgtttaatgcaccgtaagggtgcataaatgagggtaaaatggctctgatgcaggcgcttgcatctgtggaaaaaatttataaagtattttttcgttaaaaagtgggaaaaagtgttattttgtgttagaaaaaggattttcaaggactttgcccccatggtatgacaggatttctcggtgaatatgaatcgacgctggacgcaaaaggacgctttctgttacctgccgggtttaaaaagcagttgacagacggggccggaggacagtttgtgattaaccgtgggtttgaaaaatgcttatccctgtatcccatgaacgaatggcagcctatttttgaacgtatcagcaagttgaatgactttgatccaaaagtaagggaattcaggcggtacttcttaaacggggccaccattctggagttagacagtgcaggaagactgctggtaccgaaaaacctgctgtcgtacgccaatctggaaaaagatatcgtgctggcagcagcatccaataaaattgagatctgggataaaggtaaataccaggagttctttgaaaatttctcaccaggggcgttcagtgatctggcacaacaggtaatgggaggaggagataataacatatcaatttaaagaggggagcatatgggcgaacaacaatatcatttacccgttctgctgcaggaaacgacggagctgttacagataaatcccgatgggatctatgtagacgctacgtttggaggcggaggacactcaagagccatactggagaaactgggtgaaaaaggacggctgatagtatttgatcaggatgaagatgcttaccgaaacaggattatagacgaacgtgtcacttttgtacaacaaaatttccgtcatctgcaacgctttctgaagttacataaagcagaccaggtagacggcctgctggcggatctgggcgtttcatcgcaccagttcgatacagcagaaagaggattcagtattcgctttgatggcgacctggatatgcggatggataccagaacggaatttactgccgctcagttgctggcaacatggggagaagcaaggttacaactgattttccaggaatacggagaagtaaccaatgcaaaaaccctcgcccaaacaattgtaaagcagcgcaaaacacaccccatgcgcaccatcgcagcatttaaatctgtgattcagcccattgtaaaaggcaatccgcaaaaatacctggcgcaggttttccaggcattgcgtatagccgttaatgatgaactgggcgcactgaaagatttactggaacaggccaccaatgtgctgaaacccggaggaagactcgccgtcatcaccttccattcgctggaagacaggatggtgaaaaattttatgaagaccggaagttttgaagaagcacaggaagacccgtttgcaaaagaaacaccccctaaattgttcaaattaatcacaaaaaaaccggttaccgccagtgatgcagaattgaagcttaatggaagatccagaagtgcaaaactgcgggtagccgaaaaacaagcgtgacaaggttgtaaactgcctgtcacatcctaccctatcctatacacacccgttttgaatttgcgttcagattaatattgtcaatttttaaaaagacatagcgcgtgggagacgacttagatacaatccaggaaaatccggctgaagaaagtacccttcccccggagcaacgtaaagaatggcgtctgcgcatcaactacaaagcgttggtgcaaaacatgccgtttatcggtttcctttccctcctggctttagtatatatcgccaacagtcacctcgctgaaaaaaaaatccggcgcattaacaaactaggcaaagaaattaaagagctgaagtgggagtatatcaatgtgaaaagtgagctcatgtttcgaagcaaaatgagtgaagtcagtaagtcagtagagccgctgggccttaaacaactcagctcccctccgcaaaagattgtgctgaaaaaggatacagaaaaatgaatttaatattgatgcctgacgctgcccgcctgacccatcactcaggccggggatgctggtaaatcaaatcaatggcaagcatctcaattataaatgcagccagtgtcaggtatcttcttataagttatcagcctttagccgtcagctatctgccccagggtaaataactgacagctaaaggctaaaggctaaaatgctaatacaacatcgtggatgtaaaaaaggacatattgtggagagtgtatctgtgcctcatcggcatggcgctgttcagcgtcgccatcctggtgaaagtgttctatatccagaacgtgcagggcaactactggcgtagtatggccgatagcctgcacaccggctacgtggcactggacgcagaaagaggcactatttactcggaggaaggcaggatgctgtcgacctccatcccttatttcgacatccggatagattttgcagcagatggcctccgggataagaacggactggtgttcaaggaaaaccttgactccttatcctatcgcctgtcccagatattcaccgaccgcagcaaagccgcctggaagcagcagctgcaggaaggatataaatcaaaggaccgctactttttacttaaaagagacgtaccctttaatcaataccaggaattacgcagcttcccgatgtttcgcctcggcaaaaacaaaggcggcatgatcgctgaatccaaaagtaagcgcatcaacccctttaaactgctcgccaacaggaccatcgggctggcccgcgaaaattcacaaagcgtaggacttgaaagaacctacaacgaatacctgaagggcgttaccggtaaaagactgatgcgccgcatcgcaggaggtacttatgtacccgtagacggttacgatattgaacctgaaaacgggcgtgatatagttaccactatcgatgtaaacatgcaggacatcgtggaaacagccctcatgaatatgatggtgcagaatgaagccgaacacggcacctgcattctcatggaagtgaaaacaggcaaaataaaagcaatagccaacctcggcaaacaacccgatggcaacggctactgggaagatatgaactacgcactgcaggtaggggaacccggttccacttttaaactggctaccgttatcgcagtgctggaagataaatacgccaccatgaactctatggtaaacatggatggtggccgctggcaggtaggacgcagaaccgtattcgattctgaacctcacccgggcccgcaaaatgtaacgatcaaacacgcatttgaactcagctcaaatgtgggtatggcaaaactggcctaccagttctataaccggcaacctaacaaattcgtcggccatctgaaaagattaaggctcgaccagttttccggtatagacctgataggcgaaggaagaccggttattaaaaccaccgcttccaaaacatggagcgccacatccctgccctggatggcattcggatatgaagtgcttatcagcccgctgcaaacgtgcatgctgtacaatgcagtggctaacaacggtaaaatgatgaaaccctacctcgtcaactccatacaggaatatggccaggtagtaaaacagtttgagcctactgtattgctggacagcatctgcacgcaaagcacgctgaaacagttacaggccatgctggaaggtgtgcccattgatggtactgcaaaaaaactgcgcagccagttttacaccttcgcaggtaaaacaggtaccgcactcgtggcaaacggcaaccgcgggtatgcagataaaatttaccaatcgtcattcgccggttatttcccggcaaatgatccgcagtacacctgcgtggtggtgataaaaaataaaccgcatgcattgcacttttacggtgcaggcgttgcgggtcccgtgtttagagaagtggcagataaattatatgccatcgcggtagaaagacaaaaacccatgcaggccaccatgcaactggataccctgctgtcactgaaaaatggcaaaggcagtgaatggaaacaaatcctgggtaaactgcagctgcccatcggcaacgcccccgctaataacagctgggtaagcgccaaggtaacagaccgcaaaattgccttccagcaggtagcacaaacaaaaggcgcagtgcccgatgttaccggaatgggcctcaaagatgccctgtatctgctcgaaaatgccgggttacgggtagtaataaaaggcgccggtaaagtgaaaatgcaatcactccccggcggaactaaaataggaaacgaacaaacaatcgtaatagaactgagctagatgaagacgctgcaagacatattgtataatgtaagcatcctggcagtgcatggtaatacagatattgccattcacgcactcgccatcgattccagatccatcgggtccggagatgcttttattgcagtgaaaggcgtacacacagacggacacgcgtacattgaaaaagcaattgcgttgggcgccgcagcagtgatctgtgaaacattacccggacaactgacagaaaatgtttgctatgtacaggtaaacaacagcgctgtcagcagcggtatcatggcaggtaacttctatgataacccttctcataaaatacaactggtaggcgttaccggtaccaacggaaaaacaaccatcgctaccctgctgttccgtttgttcaccaaactgggatatcactgcggactattatccaccgtgcaaaatcagataggcgataccgttatacccgccacacataccacgcctgatcccattaacctgaatgccctgctggcacaaatggtggatgacggctgcctgtatgtgtttatggaagtaagctcccatgctattcaccagcaacgtattgccgggctaaaattcgcgggaggcatcttcagtaatatcacccacgaccacctcgattatcataaaacttttgatgaatatatccgggtaaagaaatcattctttgacaacctgccctcctccgcttttgcactcactaacctggacgacaaaagaggaatggtaatgctgcagaatacgaaagctaaaaaagcaacgtacagcctgcgcacactggcagattttaaaggaaagatcctggaaaataatctcacaggactggtaatgctgacaggagatacagaagtgcatttccgcctgatcggtgaattcaacgcctataacctgctggccgtttacggcgccgcagtgctgttgggcatcgataaagccaaaacattacaggccctcagcgacacctccggtgcagaaggcagatttgattatatcatttccgataaagaacagatcatcgctatagttgattacgcacacacgccggacgcactgaaaaatgtgctggctaccatcaaaaacctgcgcaaaggcaatgaacaggtgatcacagtagtaggctgcggcggcgacagggataccaccaaacgccccgtgatgggagatgtagccgtggaaaacagcgatcgcgttatccttacttctgataatccccgctcggaagatccggcggaaattatccgggaaatggaagcaggcgttcctgttcacctgaaaaagaaagtcatttccattaccgacagaaaagaagccattaaaacggcgctgtcgctcgccaaccgggaagacatcatcctggtggcaggtaaaggacatgaaaagtaccaggaaataaaaggcgttaaacatcacttcgatgataaagaagtgctgctggagctgatgaaaaccctggagaaatagactaaaactgaagatagatacttaataatccaatgacttaaaagcctgtactccccggacagcggagaacaggttacgactaaaacatatgttatattattttttaaattacctgaaaacagaatttaagatcagcgtcatcggcggtggtatgtttcagtatatcactttccgtgtaacgatggcattactgctgtcgctggttatttctttgctgttcggtaaaaggattattaaatttctacagaaaaaacaaatcggcgaaacgatccgtgaactgggcctccagggagaaaacaccaaaaaaggaacccctacgatgggtggacttatcatcttatctgccatcgtaattcccactttactttttgcacaactggcaaatgtatatatctggctgatcctgttatctaccgtatggttaggaatgatcggttttgtagatgattatatcaaagtatttaaaaagaataaagaaggactggcaggacgtttcaagatcatgggacaggtgggacttggtttgattgtgggctgtacactttattttaatacagatgtggtggtatcccgtgaggtaataggcgcaaaaacactggcgccttatgaaagacaggtgactaatcacccggagcgtgtaactcgcgacggacaccgttttgtggacgttaaaacgccgattaccacgattccgttcgtaaaaaatcatgagttcaactactccaaactgatctcctggattcccggcgcagaaaagtacacattcgtactctatatcctggtggtcatctttattattacggccgtatccaacggcgctaaccttactgatggtttagatggactggcaacaggcgtttcgggcatcatcgggataggactgggcatctttgcctatgtatccggtaacatccagtttgcggaatacctgaacattatgtacatcccgaacctcggggagctgtcaattttcattgcagcctttgtgggcggatgtatcgggttcctctggtataatgcctatccggcgcaggttttcatgggtgacaccggtagtctcgcgttgggtggcatcattgcttcactggccattatagtaaggaaagaattactgatacctatcttctgtggtgtattcctggtggaactactgtcggtgatgttacaggtatcttacttcaaatacactaaaaagaaatatggagaaggcaggcgtattctgaaaatgtcgccgttgcatcaccattatcagaagatcggttaccacgaaagtaaaatatcagtgcggttctggattattaccatcatgtgtgtggtagtagctattgcaacactgaaaatgagataaaacaacactaaacaagaagataaaacgaatggaatataaactcgtcatattaggagcaggagaaagtggaataggtgcggctttgctgggaaaacagcaagggtatgatgtatttgtatctgatggaggaacaataaaagataattataaacaggaactggcggtaaaccagatctctttcgaagaaggacatcattcctgggatatcatactggatgcaaacgaaatcgttaaaagtcccggtattcctgagaaatcggaattgatgaaaaaggtgcgcgaaaaaggcatacccgtgatttctgaaatagagctggcctaccgtttctcgacaggtaaaaagatcattgccatcaccggcagcaacggcaaaagtaccactacggccctcacctatcacatctttaaaaacgcaggtttggatgtggcgatggtaggcaatattggcgtgagctatgccaggcaggtggcaaccgcaccagcggagtattatgtgattgaaatcagcagctttcagctggatgacattaaggacttcaaacccaatgtggccatcctgttgaacattacgcctgatcacctggaccgctacgactatagcatggaaaattacgtagcctccaagttcagaattgccatgaaccagacagctgaagactacttcatctactgcatggatgatcctgagatcatgcgacatttagcgcagcaacccatttattcagcatcaataccttttaccatcatgaaaccactgaaagaaggcggctctattgccaacgaccagttgcacatagatgtcaacggagaaccggttatcatgtcaatgtatgacctgtcattaaagggaaaacacaatctgtacaattcaatggcagcagcaattgcaggcaggaccatggatataagaaatgagaaaatccgcgaaagccttgcatcgttcgagagcctcgaacaccgcatggaatatgtgacatcggttagaggcgtggattttattaacgacagcaaagctaccaatgtaaactccgtttggtttgcactggaaagttttgacaagcccattgtgctgatcatgggcggcgtggacaaaggcaacgactatgatgccatccgcgacctcgtgaaagaaaaggtaaaggcaattatttgtatgggtgtggacaacacccccatctttactgcgttatcaaaagacacaccggtaatgatcaacactaccagtatgcacgacgcagtacaggaagcatttaaacaggccgcaaaaggagacatcgttttattgtcgcccgcctgcgccagcttcgacctctttaaaaattatgaagatcgtggcaggaaatttaaagaagaagtaaaagcattgtaacaggtgttgataaacagaataaagggttacatcttaaaaaataaatgaaagcaaaacgcagctaatgatgggattgctctatagaacaaaaggcgataaggttatctggacggtagtattttttctatcgctggtaagcctgcttgctgtatatagtgctaccggctcactcgcttaccgcgaaaggggcggccatacggagtattatctcctgaaacagctcacggtactggtaatgggattgctgatcatctattttgcacaccgcgtgaactatacgatttattcccgcgtggcacaaatcggtttcctggtatccataccactgctgatgtacacgctggcctttgggtctaatatcaatgaagccagcaggtggatcaagctgccgatcatcaaccttacctttcaaacatccgatgtggctaaactcgccatattcatgtatgtaagcaggcaattatcaagacggcaaaacctgatcaatgatttcaaaaaaggatttctgcccatcattataccggtaggcattatctgcgcgctgatcatgcccgccaatatgagtaccgcacttttgctgggtgccagctgtatgctcctttgctttattggcagggtgcctatccggttcctggcctctatggtggccgcgggagcggtaatggtagtgctgctttttggaatcgccaaagtaaccggcatggagatgcgtacgaaaacatgggaaaaacgtatcgataacttccttcatggtgatcatacagaaacgccctaccaggtgcaacaggccaacattgccattgcaggcggcggtattttgggaaaaggacccggcaacagtacacaacgtaacttcctgccacacgcctattccgattatatctacgctactattatagaagaatatggcatgtttggcgctttcctgatactggcggcttatatgattttattactgagaagtatcaggatttataaaagatgtccatatgctttcggggcattcctggcagtaggactcagtgtaacattggtcatacaggcgttaaccaatatggcggtaaacgtacagctgttcccggttacagggctgccactgcctttggtaagtatgggtggttcctctgtattatttaccagtatggccattggtattatattaagtgtatcccggaacgtggaagagatggaaggtaaacaggcagagaaagagcgattggaaagagttattgcgcaatcggaaaccgctgcagtcgcttaatacgtatttataacaataattgtaatcaggaatagaacatgcaacgcaaagtgatcatagcaggtggcggtacggggggacacatcttcccggcgatagcgatcgcgaatgcgttgaaaaaaatagagccggacatcaacattctttttgtgggcgccaccgggaaaatggaaatggagaaagtgccgcaggcagggtatccgatcgaaggacttgaaatagctggttttaaccgcagcaatatttttaaaaatatcctgctgccgtttaaaatttggaaaagcctgcgtcgcgcaaaggccatcctgcaaagctttcagcctgatgtggtagtaggtgtgggcgggtatgcgagcttccccatgctgaacagggcacagaaaaacggtacgcctaccctgatacaggaacaaaattcctttgcgggtaaaacgaataaaatactgggcaggaacgcgaaaaagatctgtgtggcatacgatggtatggataaatttttcccgtcagaaaaactggtgatgaccggcaatcctgtgaggaacagcatttcccagtcggccgtaacacgggaagatgccttgcagcatttcggactgagtacggcaaagcaaacggttttcgccgtgggaggaagcttgggcgccaagtcaataaacgaaggattacaaccactgttaaaagaattagtggctaaggatatacagctgatctggcaaacagggaagccttattacgaaacagcgaaagctgccgcggcgccttatggatcgcatatcaaggtatacgatttcatcaacgtaatggattttgcctataaagcggcagatgtagtgttatcacgggccggtgcattggcgattgctgaattatgtgtagtgaaaaagccggtgatatttgtgccttacccgttcgcggcagaagatcatcaaacgtccaacgccatgaacctggtaaacaaacaggcgggcctgatcattaaagacgaccaggtgccatcacaactgggcaacgtgctgttcagccttttgcaaaataaagcgctgatggaacaactggaaagcaatatcggcaagctgggaaatccccacgcggatgtgacaattgcgaaccaggttttaggaatcatttagaagagattttttagaagagtatatggatttgaacaacatacaaagggtttatttcatcggtatcggtggtattggcatgagcgccattgcacgctttttcaatgagaaaggggtgcaggtaagcggttatgaccgtacctccacagcgctcacaaagcagctggaagcagaaggtatgcaaatccattatacagacgatattaacttaatcgacaaaaccattaacctggtcgtatatacgccggcgattccggctactcatacggagttgcagtggctgcgcgataatggttatgaagtagtaaagcgcagtgatgtgctgcaggaaattacccgttccctgtttgctatcacggtggcaggtacgcatggcaaaaccacggtatctaccatgatcgcccacctgcttaccgacagcggttatggctgcaacgctttcctgggtggcatcagcgtgaactataataaaaatttctggagcagcgataaagcggtagcagtaattgaagcagacgaatatgaccgttctttcctgaaattaagtccggatatcgcggtgttaactgccatggatgcagatcacctggatatttacggcactccggaggcaatggaagatgcttttatccagtatacgcacaatattaagcccaatggcacgctgattgctaggttcggcctgcatcgcaacaaagagctcaatgcaacaaacaagttgttgtacagtttacaaaacgatgctgccaacgcttacgcctccaacatccgcatgatcaatggcggatatgagtttgatgtaatgcatcaggactggatgatcgataacatttccatgcacattggtggtatgcacaacgtggagaatgcagtagcagctattacagtagcacacctgctgggaatagatgcggctaaaatccgtgcagccattggtaatttcaaagggatccggcggagatttgaatatgtggtaaaaacggatcagcaggtatatatcgatgattatgcacaccatccggaagaattgcgtgcattgatcaccagtgcaaaggcattgtttccaggtaaaaaatgtaccgttatttttcagccgcacttatttacccgcacccgtgacctcgcggatggctttgcagaaagcctttccctggcagacgaggtgatattacttccgatctacccggcgcgtgagctgccgatagccggtgttaccagcgaaatgattgcagataaaataacagtacctgtaaagattttaccgaaagaaaaagtagcggaatacctgggcaaacaggacgtgccattactgattaccgccggagcgggagatatagaccagttaaaagaaccgttggctcatcttcttaaaaataaaacaacacaacattaaaaataaaaagcttgtctaaaactaccacaatattaaaacgactgggtgtcgccgttctctggggaatggtgctcacaggctttacagtattgctggtggcggctatacaggacaaggatgccggtaaatgtaaaagtatacaggtaaaatttgaggggaaagatgataacttttttatcgaatcaaaggatatcaaatctttgatcacgaaagataaaaatctgaacccggtcggtaaaagtattgccgatatcaatatcgctcagctggaatccattgtagaccaggatccctgggtaaaaaatgcggagatctattttgataacggccagcagctgaatatcaaagtaacacaacgcgaaccggtagcaagggtatttactttctcagggaacagcttttacctggatggcgccggcgaacatataccggtatccagtcgttacgcagccagggtgcccgtattcacagggtttcccacggatgcagaaaagctgcagcaacccgacagcctgttggcagcgcagatagtagatatgggtacatacattggtaaggatcctttctggatggctcaggtagagcaactcatgatcacgggcgaccgcaggtttgagttcataccgaaactgggagaccaggtgattgcattcggagaaggtatagacatagaaaaaaaattcaccaaactgctggctttttataaggaaggattgaataaagtaggctggaataattatacacgcatcaacatcgcatttgaaaacgaagtggtgtgtacccgtaaggatggcgttgttccattgcaaccagtgatcaaaacggatagtttgaaactggccgatgcagatgaaccgccgatagcggacagcgaagattcaacgacggtagcaccggtagtagcaaaaccggtacattccgaacctgccaaaccggtaactaaaccggcacatgcagcgaaagaaaaggctaaaccgcagaaagcaaaggtgaagaaagaaaaagcagctgcgccggccaaacaacaacctaaagcagtgtataagccagggaataaatctgttaacacatcaaaaaaacaaaaaacgccatgaatcaggaagctcccatcattgtaggactcgatataggtactacgaagattgctgccattgcaggacggaagaatgaatacgggaaactggaaatcctgggattcggtaaagctacatcgtttggtgtacagcacggtatggtgctgaacattgaccaaaccattaaagctatcaggcaagcactcgagaattgttatgcatccaaccctaacctggaaattaacgaggtatatgttggtatagccggtcaccatataaaaagtttgcaaacccgtggagatattgtacgcaatgacactgatgcggaaatatcccagaaagatatcgaccagctgatcaacgatcagtacaaaacagttattcccgcgagcgatcagatcatcgatgtgattccgcagcaatatatagtggacagcctgcagaacatcacttaccctatcggtatgtccggggtaaaggtgggtgcaaacttccatattattaccggcgacaaaaacgccatccgtaacattaaccgcagcgtggagaaatccggtctcaaaatccgcgacctggtgcttcagccactggcttctgctgcagcggtaatgtgcgacatggattttgaagcaggtgtagccattgtggatattggtggtggtaccaccgacctggcagtattttatgaaggtatattgaaacataccgccgttattccgtacggtggtgaaaacattaccaacgacatcaagaacggcctgggtgtattaaaaacacaggcagaacagatgaaagtacagttcggttatgccctggcagatgaagccaaaacaaatgcctatatcacgatccccggattaagaggtcaaagccccaaagagatctccgtgaagaacctggcacacatcatccaggcacgcatgagtgaaatactcgatttcgtggtatatcatctcaagcagatcggtatggataataaaatgttgaatggcggcatcattcttactggtggcggttctcagctgaaacacctcatacagctgacagaatacaccaccggtgcaagcgcccgtataggattccccaacgagcacctcgcaagcggccacatagatgaattaacaaaacctatgtatgctacctgcgtgggcctgatcctgaaaggctacaacgattttgaaaacgatcgaaaagcactcgaagaaaattatgtaaaaattaataccagctatctggccaaagaacaggctgctcaatccgtagcttcagccgaagactggatagaagaagaaacccccagcagtcaggaaatacaggaccggaaagcaaaagaaagaaacgcctcattgaaaaacttcctggacaaaatgaaaacaaaaatcattgatatgttcaccgaagaagaagatgcaaaactttaaaagtttaatggcgcaattgttgcaaaaagcaaacgtttaatataataagaattaagaacgataattaataatgacaggacaaatgaaccatagtaacatacaagcatacacgcacttaattcttaatagttcattattaattattcgtactaacccataaaagtatagagtcatgatacattttgatcttcctaaggaaaaatcttccatcatcaaagtcatcggtatcggtggcggtggaagtaatgcggtgaatcatatgtatagccagcgcattgagggggtaaatttcattatttgcaataccgatgcacaagctattgctaatagcccggttcccaataaaatacagttgggcccgcacctgacacagggacttggcgccggtgcaaatcctgaaatcgggaaacaggcgacggaagaatcctttgaagaaatcaaaaaaatactggaggtaaataccaaaatggccttcattactgccggtatgggcggtggcaccggaaccggtggcgctcctatcatcgcgcggatatgtaaggaacttggtattctgaccgttggtattgttaccactcccttttcttacgaaggaaaaaagagaatgctgcaggctgatgaaggcgttaaccgcctgaaagagtatgtagataccctgctgattatctccaatgataaattacgtcagaaattcggcgacctgaagttcaaggctgctttcgaaaaagcagataacgtgctggctactgccgccaaatgtattaccgatgtaatcaactctaccggtcagatcaacgtggattttgccgacgtttgtaccgttatgcgtaacggtggcgtagcaatcctcggtgcagcactggcagaaggcgaaaaccgggcgcaaagggctatcgaagatgcattaacttctccgctgctgaacgacaacgatatacgcggtgctaaatggatcctcatcaatatctcttcttctgaaggtgaatttgaacacaccctcgatgaaatggatattatccaggcatatgtacaaagccaggcgggtgaagattgcgatgtgatcctcggtgttggctatgatcaaacactcgacaggcaattgggcgtaaccatcattgctaccggttttgaacaaaaacccattacacaacagaaaatcacaccctccaacccggagcgcgtagaacctaaaattgtaatgcagttaggtaaagatggtgacgaaaaaaagatgagcgtacaacaggcacagggcaccttattccaggagccgcaagacctgatggcgccacgcctgatggagccggtagtaagtcatcctgagcctgtaatggcttatacgccaccgcagccacaacaacaggcgcctattgctcctgcacgtcaaaactatgtgctgaacatacaacaggtaccacctgcacagccacaacagccagatccgcagcagatacaacaacaaatgcaacaggcgcaacagcagcagatgcagcaaatgcagcaacagcctgttcaacaacagcctgttcagcaagtgccacctgcacatacacaacagcctggtgtaaatatcattcaaccgcaaacaggtaatgcggccggaggatatttaaacagacctgcacatatttacgtggaaccaggcgctcctgctcccgaaatgaaaatggtatttaaagaggaagaagaaagtgcggtaaacgtacctcctgctcctccggaagtgcctatgcaacaggcttacgaagacctggaagaacagaaacgcaaacaagcggaaagagtggccaaattacgcagcatcagtttcaatgtgaaaaacatggacaacaacgcggaactggaaaacgtacctgcttacctgcgcagaaatgtgaacttggataatggtgctggctctgctgaacacctctactccaactatacggtgagtggtgatcagggccctaataatcatacggaaatcaatacgatcaatacctttttagatgggaaaaagcccgattgatgaacacatttgattgttttttagttgtgttaaaaaaagtcctccggttccccggaggactttttttatgatacttttattcaattaaagttcgttcaacccttgcttggctgtattcagtatttgagctgccggtgtggttttcagcgtttcttcctcgaaaggctttactaaattatccagcttactcaaacctgccgcgttgccgctttttgtaaatgcttcgcgcaatattctaatcttttcatagtcctgtataccttctatcagtctttcataacggatagaagatctcggtcccggatatacgaaataggtatctcctgcagcccatgagcggaaacgggaatcatgcagcggatctgcaacccagcagttgaaagcccagcgcaaatacccgttatatcctttgtttgcagcatgccagcccataaaagctgcttctgcaggtggggaaaaagtaaaagtattggggaatccttctgtacaacaggtgtaaaaagtagtgggcaatcccttctctaagcgggttttcatgatgttggcaggaaaagattctttcagtgcaatacagtaatcatgtatttcattggccaatggttcatgatagctacccgccagtgataatttgaagtcgctgctcgcaccacggatcactttcagtgtttgcagcatgtcttccataggccgctcatccatagcgatagccgtaatatcaaaccagccctttgccttcaggtgctttacaaaatcagtcagcataggctgccagtgttttgtatattccgcagagccaggcttcgctacaataaaagtatcctttgcagctgcctcatcataataatagaacttcaggttccaggggatcatgctgtagcagttgatttccttccggatgccctggtccatcataaactgcacccatttatcaaagatgctgtagtcgtatgtccagctgccatttttcttctttgtccattttaccattgtgccataaatgtcctgtgtctggctattccagggatcataaataatggtggcagtgatcactttctgacctgcatttgccagcattttcatgtaaggtttcatagcttcgaagtgtgcattactccagggctttacgccatatacgcgtgctattgcataagggctctgccacaaatcaagatgaaattgccagtctttcggagcaggcagggtatgttccagcacggttactgcaaaaggcatatccaccgtggtaacgcctgattttacactcaccgagcctttatatgtgccggctggtgtgtttgccggcacctgaacgcttagccataccggctgtgtagtattggcggcaatagtgcttttattgatgatatcaatgccatctgccacgagcgaggagtcgtaatccttcgggttgcggtgcccgcagccgccgccgtctttattcaaaccatctgtgagtacatatctaacaaaaccggtggtgactgccgaagccgcaattttattgcctttgttgtcctgcagtacagatgcccggaggcttacttcgggctgcacagcggcagaccagatcaccaactgggtatggactctctcacctttccaggctttcgtttcccaggctggcgttaatctgctgttatcgggtgcatttcttttttcataacgggtatctgcagtaccgaatgcaacgtgaagcctggtgtcattaacagccgcccaggacgctttattaacgggtttgggatcgggcaggtccctgtagccagcggcgggagatatttgcgcccatacgttttgttgcagtgccagcattaccagcacgccaaaaaatttgttcaccatactaaaatttagcgttttcagatattcggataacgtgatttgttcactgatcaccgtcatcccgaaacctcaatatctataaaaaaagtggatttttccctttaaagaggacgatcggttatataaaacagaaaagccggatcataataagatccggcttttcttgttaaagatttatattaatgtacgatccgcttcagctgcagattggtgaccggcgctaccaccaatgggtatttctcgatggtcacatagctggaatccagtccaaagcccctttcttctgacaaactgatctttttcaggaagaaatacatcttcatcaccattctttcatacaaaggcaggtcgttgtcgtgcgacaggaatttctccataacaataaactggaagtcacccaccacgttattcttactcagtgattcatagcggctggtgatatttacttccttgttacgaaccatatcttccaccaccattctgaacatcaggttaatacgttgttccactttgaagcccagtcgaaactctacgcgtatcacttcgtttggaataattgtttgtacagagtattcactcaggtaaggttcgtctaccacatccacgtgtacaaaccagtatatatccgcccgtttgggttttttattgagaattgaatagatgatcttatgttctatttctttcggattatcggcactgctcatatacaccaggtgggtagcgtattttggaatggaggtatcattgctcagttcctggatgataggcagataatcttccagtcgcacaaattccacgtaacggttcttgatcttacgcgatttgaaccatacaatcatcacgaggaagagtgcgccggctacaataaccgttacataacctccgtgcatgaatttaatcacattggcgaagaggaatgaaaattctatggtgaaataaacgatgagatatagcagtatccaacctacccatacccgctttgtataaaggtaaaaagcgaagaggcaggaggtcatgagcatacagatagtgatggagaggccataagccgcctccatattcgacgattcccggaagatcagcacaatggaaacgcaacctacaaacagcatggtattgataccgggaatgtagagctgtcctctttcttctgtaggatagtttacccgcattttgggccacaggttaagccgcatggcttctgcaatgagggtaaaagaacctgatatgagtgcctggctggcaattaccgaagccagtgtggcaattaataccccgaaaatgatgaaccattccggcataatggtgaagaatgggttctgatcttttggcaggatctgacctttttgcgtgagcagccaggcaccttgaccgagatagttcaggataagacatgttttaacgaagatccaggatacccggatattgcctttaccgcagtgaccgagatcagaataaagggcctccgctccggtggtacaaaggaatacagctcccaggatcaggaatccccggggataagtagttaagagttcaatggcataatggggactaaatgcttttaaaatgcttaaatcatctgctacatgcgaaataccaaggattcccagcattgaaaaccacaataccatgatggggccaaacatccggccaatggaaacggtaccgaactgttgcataacaaagagtcctgtaataatggtcagcactattttgacgatggtcaactggcccaggtctttaaagacttccagcgtccggagaccttcaatggcggcagtaacagtgatgggtggggtgatgataccatctgcgagcagagcggcgccgccaatcataccaaaaatcacggtccatctggcgtggcgtcttacgagtgcatagagtgaaaagattccgccttcccccttattatctgcccggagggtgaggataacgtatttaacggtagtttgaagggttagtgtccagatgacacaggaaatacctccaattaccagcagatcgctgatggggttccctcctacgatggctttgaaaacatagagtggagatgttccaatatcgccgtagataataccgagcgctactaccaggcctgccagggataccctgttgatgttaattcccacgtaataataagtttattaaaaaagcctccaaaattaggggtaataattgacacttcaacaatatttcgtacaggagtgtttgcttcaaaaaaaagtcctctcccgaatgaacgggagaggactttttttaagttatcatcttaatgagtgatactgattagttagcaggagctaagtcaacagtgccagactcaccaggagtgttttgtttgatgaaacgaccgcggtcgataccttgtttgtcagccaggtagtcgattactgagtcaacacgacggctgctcaggtcaacaccacctttcttacctttagcacctgcgtgaccggtaaccagtacgttgcaggaagggttagatttcagggaagctgcaacagaagccaggatagcttcctgatcgttacctattttggtagagctgcctttgaaagaaacgctaggcagaaccaggcttgcgcaaggcgcaactggaggattcttgcagcattctggatctgggcatttaccaacaccatcagcatcaactggctggcagtaagtaggagtgatcagttgtttgtctttgtaatcaggaacaccgtcaccgtcagtatctttagcaacaccgtgaacatccactggtgcacctgctggggtgttaggttcgcgatcgaactggtcagttacgccatcgccatcagcatcaggcagaaccggagttggaagcttcatgtgacgtgggttgctcagctcgctgtaagcatattccagtgggttgatccaccataatggctgtacacgtttagctgggttacccaggttgaagttcagacgtacgcttgtgtaagagtagaaatctttagaagcaccgcctggtccagcatagccgtccatgtatgcatcgaaaggcatagttactttttcttcaataccgatgttgaaacgtttagaaactttaaacgcaacgccagtacctacatccagtgcatgacggagtaactggttgtcgtcgttacggccgatggaaatacggttaccctgagaaggagcattttgctcgtatttatcatctctcagatctttgatctgttttctgatatcactgcgttttgcattgaaattaataccggaatagttatagccatttccgcttgcatctaatgcatcaacgtcaacgtcagccattacgatagagtaaccagccagtaaataccagttaaccttaggttcagctctgtagaacaggatgttgcttaaagaagcgatcacatccaaagacagctgatggttttgagacttgtagttaggaacaatcatgccgccgtttaaagctgcagttcttccccatggattgataccacctgcagcctgagtaggacgcagtttgtagtcctgacccttatcgatggaaccgatgtactcagctctcagggagaaagtatgtcccagtgcttttctcagggaaacaccgccaccaaaacctggttgaggaggaacggttccgctgatcaggtgtaaaccaccactaaaacccagttcccacatatctctcggtttagccgggaaatttgattggtggttcgtgaagttattttgttgtaccatacgcttgctagacactttggagctatccagagcatcgtagccggttggttgaacctgtgcaaaactagtagatgctgatagtaaacccacagcgcctgccagtaataagtactttttgcttgccataattgttttttttattaaaaactgttaaaaatttactaataacccgttttttacctagcaaaggtaaatatcataaatgaatatacaaatttttcttgcaatattattttcattgataagtccttcaaaattagagcttaaatgaaagtatttatataccttaattccagttaagttaaagatctgtataactcgtgttaaaggattccttaactcgtgttaaaggaatgttatactccttatacaaattaaaggccaaaatgttaaaatgtgatttataaaagttagcttagcaatccttttttatttaatacatggacgatattaaacacctgataggtaaagaattacaggattttgaaagtaagttcgcagattcagtaaaaagtcatgtgccgttactggaccggatcatgcattatattgtaaagcgaaaagggaagcagatcaggcccatgtttgttttattatccgccaaacttttcagtgacaatatccaggaaagcacttatcgggccgccgccctggtggaactgctgcataccgccaccctggtacatgacgatgtggtagatgatgccaacgaacgccgtggcctgttttccattaatgccctctggaaaaataaaatagcggtactggtaggcgactacctcctttcaaaaggactactgctgtctcttaacaataatgatttccgaactttacagatattatcagaagctgttaaagaaatgagtgagggagaactgctgcagatcgaaaaaacccgcaaactgaatatcaaggaagatatttattttgaaattatccgccgcaaaaccgcttcattactggcttccgcatgcgctgccggcgcatggagcagcagcaacgatgaccataccaccgaacaaatgcgccttttcggcgaaaaagtaggcatcgccttccagattaaagatgatctcttcgactatggctccgccaaaatcggtaaacctaccggcatcgacatccgggagaaaaaaatgacccttccgcttatctataccctggaacatgcttccactgaaacacgcaggaggattattaatatcgtcaaaaatcataatacagaaaaagaccgggtagaagaagttatccggctggtaaaagcatccggtggcattgactacaccaggaaaaaaatgtttgaataccgggatgaagcccttaccatcctgaataaattccctgaaaacgctgtcagaaacggattagaatccctcgtacgatttacaactgacagaacattttagtaagaataaaaaataatgtaatatgcggaagaagcgggaagcttaagcctttaaaatataataatgcaaaaacgctggacagtaaaggcatatcaaccaaaccaggaacagttactacagtcatcattacgcatacatccgttgttatgccggttactggtacaacgcaatgtgaccaactatgaggctgcccggcaattttttcgacctacactggaagatctgcacgatccctggaaaatgaaagacatggacaaagccatttccaggattgaactggcttttttccagcacgaaaaaatactgatctacggggattacgatgtagacggcactaccgctgttgctaccgtgtacgcctttctgcaaaaactctacagcaatattgaattttacattccccaccgctaccgcgaaggatatggtatttccatacagggaatcgaatacgccagggataatgattttagcctgatcatcgcgctcgattgcggcattaaatcaatcgaacatatcactactgcaaaggaatggggtatcgactttattatctgtgatcatcatttgccggatgcaatactgccgcctgccgtggcgatcctgaatccgaaacagcacgattgtccctatccttataaagaactgagcggatgcgggatcggatacaaactgatctgcgccttcgcacaaaaaagaggcctcccccagtcggaagccaataaattcctggacctggtggctaccagcattgcagccgacatcgttccgatgaccggtgaaaacaggatactggcttttcatggtcttataaaagtaaatgaagatcctttacctggtatcaaagcactgattacactcagcgcgctgaaagaaaaactgaccattgccaacctcgtatttgtaattgccccacgggtaaacgccgccggcagaatggacgatgcccgcaaagcagtgaacctcttcatcgaaaacgacgtggaaaaggctgctgccatcgcagccgtactgcacgccgataacttcgacagaaaagaaatagacagcactattacccaggaagcaatcgttctgttacaaaatgatgtggatattgcacgcagaaaatcaaccgtgctttaccaggcccactggcataaaggagtggtaggcattgtggcttcccgcctgatcgataaatattattatcgccctactatcatcctcacccagtcgaatgataaagtagccggctccgcccgttctgtgatggggttcaatgtatatgaagccatccaccagtgtaaagatcttctcgaaaattacggaggacatttttatgcggcagggatgaccatgaaaacagaaaatgtaaaagctttccaggaacgctttgaagaagtggtagcccggaccatccacccggatcagctggtaccggaaatagtgatagataccgaaatccatttcacggaaatcactgctgcattttataatattctccggcagtttgaaccactgggaccagataacctacgccctgtttttcttgccagaaaccttgttgacaacggctactcgaagattgtgaaagatgaccatattaaattctccgtcaaacaggggagatatggtcccactatgtccggaattggcttttatatggcggagaaatttccgttgatggcagataaaaagcctttcgatatggcatttacactggatgaaaatgaatggaacggacaaacgtccctccagctgaaagtaattgatatcaggactgcagctatccagtagctttataaagagagatgaaggcagttacaagtgttgcttcagcagccaggtataaacatcctggttggcgtaagcccttgtccaggcatcatggccgccgtttggatattccgtatactgcacattattacccaacgctcttaatgcctttaccaggacacgtgaattctccacatttacagtaggatcgtctgctgaatggaaaacccatataggcatggttttcagatttttcatacggtttatatcacctcccccgctgataggaacaatggcggcaaatttttcggggtgtgcagaactccagtcccaggttccgtagccgcccatgctcaagccggtcagatacacccttttgggatctacatgatatttgctgatcacttctttgtataatatatcaaggtactgtggattccaccatccgctcaggcattgtggtgcaattatcacaaatggctttcctgctgacacttttcccaatccaacattccttatcatatcaatattgttccccatttcccctaccccatgaagaaatatcacgatcggccatttgtaatctttcttctcgttatatccatcagggatataaagcaggtagttactgatgttgcctcctttggtgtctatttttttcgcagtgatgcctgtttgctgtggaggaaaagtatcgcctggcggcggcgttaccggtatggtatcccccggccgattagttaccggattagtcatttctgtttttgaacaggaaaaaaatgcgagcgcactcagcacaaagacatggcacaaaattttaattgctctttttttcatataactagtacaaactaaagtcccccggccatacgccgggggacagttttacaatatttttcgtttcagtttttctattgcaacaactgcaaataaaagaccaaaagagcaaacaccgttaattttttttattgtgcccgtcttattattttttctcgcccatcaattccacacttctattcacaaatgctgtaagatctgcacctgtcaataaattctgggacaacagcgccaggtctgccaggttctttatctgcttctgttgcaatgcgttgtctccttccttaagaatttgtgtgtataccgggtggttggcgttgatggtcatatttatttcatcaggcatactcgcataccagctcattccgccgccgcccatggctgccatatctttcatacgacgcatcagctccggacgggttacaattaccggttgcgcttctgcgctgagtcctttcatttctactttgatattgggttgcgttacctgggagccaaacaactctttcaaagcaccctcctgttcttcagataatacggtagtggtattttcttctttatcaatcaggttatcggcaatatctgcatccacacgggtaaaggaaacgttatcccatttgatctccatgttgttgatgaatgcagcatccaccattgtttccatctttactaccaggaaacctttattttttgcggcctgcacatagctgtcctgctgcacagggttggtagcatataataccaccagtttctgttctttgttggtttgcagggctgctgcggcagtacggtattcttcctgtgtatagaatttaccgccttccacatcttccattatcaggaacttattggctttttccatgaacttgtcgtcggtcatcataccatacttcacaaacagtccgatggaatcccatttatcttcaaaggaagcgcggtcgttacggaatatttcatccagtttgtccgcaacttttttggtgatgtgagcattgatcttttttacgttaggatcaccctgcagatagctgcggctcacgttcagcggaatatccgggctatcgatcacaccatgcagcaacatcaggaattccggaacaatatccttcacttcgtctgttacatatacctggttggaatacagattgatcttgtctttctgcatctcatagctcttgttgattttcgggaaatacaggataccggtgagattaaaaggatagtctacgttcagatgaatccaaaacaaaggaggttctgcatatggatataattctttgtagaaattctgataatcttcagtggtcaactcgcttggtttctttgtccaggcaggagtggtgttattaatctgcgtgccttcaaaagttaccggaacaggcaggaatttacagaacttttcgaggatagtgcggatgcgtccatcttccaggaattcttcgctttcctcgttgatgtgcattacaatttcagttcccctgtcggccttgctgatttcttccagttcatactcagggcttccgtcgcattcccaacgtacagctggagcttcttctttccaggattttgaaaagatttccacctggctgcttaccataaaggaagaataaaagccgaggccaaaatgaccaatgatattggtaccattttcctgtcctttatattttttcagaaattcttctgcaccggaaaaggcgacctggttaatatatttatccacttcttctgcagtcataccgatcccatgatctgcaatggtgatggttttcttttccttatctactcttacatcaatagcaatgtctcccagttctcctttaaattctcctacactggccagggttttcaatttctgggttgcatccacggcattacttaccagttcgcggataaaaatttcatgatctgaatacaggaacttcttgataattggaaatatgttctctgtctgaacacgtattgcacctttttgcattgatatctgatttttttggtaaccttttttcaaagtgtgtgccagcgggatgagggctgacaagatgacaacacacaagttgaaaaaatattaaatatgaatattgtggctgtgaatatacactacctgggtttatccatcattgtaatttaattctgaaaaaagggcagtgcagaaaatatctataacaaatatgaaaataaaatcatattacattccgtcaaattaacaaaataatcatattaaaaaaaccgccgaaagggtttattcagtagatttattgtatcgaaacccggattccccaatttttcaaatattactatggaaagacctctactcatcttcttatttatggctttttttgtttgtggtaatgtaagcgcacaaaccaatccggctgtgcagccattaccgtatgaacaaaattttgacgcgttaccatcgactgccgtgatatacccggcgggatggcagggatggctgctcagcggcgctccttccggcagctttaatacagcggcaccggcatccgataaaccactgatcagtaacggcagtgcgtcggctaccgccaatggtgtttataactacaccggtaaactgggcttcctgaacagcggcagcgccgacaattcactggtgctttcccttagtaccagcggacagcagaatgtacgtttaagctacgatgccatgaccatcaggaatccttacgatggcaactccaatacgaggatcaatgaaatggttattcaatatcgtataggcgtaaccggtacctttaccagtatcaatgaaacggcctatcagaatgacaccattccgcaaaccggttcaggtgttacctcaccgcagcacctggtgaatatgtcagtgatactgccgccggattgtaataaccaggcaatagtgcaactgcgatgggtaaaccgccagatcagcggcgcgggctccaggccgggatttgccattgataacatcactgcatccggcagtggcagagataccactcccccggtaatcaccctcctggcaccggttaacgcggcagcagacgtgtcgcctgtcacatctcccgaaattatattcagcgaaaacataaaagccggtaacgggtacatcaggttgcacaacagtaacagtgggataacagacagttttccggtaaccggtaacgctattgtaattaataacaatagcgttaccctgaaacaaatcctgcaaccccacagtcattattacatcacgctggacagtggattagtaaaggatctgtcggataataatttcgcaggtatggcagataccacgcaatggaatttcactactggcagccaggaactcagctataacttcaacgactgtacgccaattggcagcagccagttgagcgggggtttcacacaatacagtgtaactggcgcgcagctatggggatgtacaaatttcggtcagcagaacagcaatggtgtacagataaatggttacagtggcggagctgttgaaaatgaagactggctgatatctcccgtatttgatctcaccggtttgcaattcccgctgttacaattcagcagccgcactgcgtttgccggacccgcacttagtctgcgtgtttccactaactacacgggcagcggcgatccgcgcagtgctacctggactaggctgaatggccgttttcctgaacccggcagcgacgtgtggacgctatcttccggtattaatctcgctgcctacaaacagacaggcgtttatattgcttttgtttatacatccggccctgccgttcaggcggcacgctggacgattgatgatttcaggctgacggataccaccgctgcgccggcgccgagtttgaacagcagtcctgttgctattgacttcgactacgtaaaatccgggcaaatatcagaagcacagcgtgttagtttctgggccaatgattttaccggagagctgaaaatcactgccccggcaggtttcatggtatcaggtgacagctccagttacagcagtcaggtcattttcactgcagcagcattggctgccggtccgcaggaagtatttataaaattcgctcccacggctgctgatcaggcttacagcggccaacttaccttcagcggtcccggtttccccggccgttccattgcactcagcggcacatcgttgcggtcattaaaagtggtgaactggaatatagaatggtttggcagcccggctcaaaacccggccaacgatagtttacagcaagccaatgtaaccaccatcctgaaaaaactggacgccgatatttttgcgttggcagaagtagtggacactgcccgtttccgtgcggtggtgagccagttaccgggttatagctatgtgttatctgactttggctcttatgcagatagtaccacggatgctgattatgtttcggcgcagaagctcgcgtttgtgtataaaacggctgtgatccgtaaaatcagcacttacggcatattaagacagggaggcagcagcaatgcttattataactggtcgtccggcaggttcccttatgaaatggaggctactgccaaactgggtaatgactcggcgcgtatccggttcatattattgcatgcgaaggccaatacaggaacaaagcccgaaaagattacttcctggaatcgtcgcaaagatgggttgaaggagttgaaagatacgctggacgtgcaatatccgtatagcaatattattatgctgggagattttaatgacgatctgtcaaaaactattacaacggagttattaccggatactactacttcatatattgacttcatccgcgacagtatcaattaccggccgttgaccctgcccttgagtttatcgggtcagcgttccaccgtcagctacgcctcggtgatcgacaatgtgatcggttccaacgaggtgggtgttgcttatttaccggcatccgcacggatacaaacccaggtagcggggctggtaagcagttatggtactactaccacggatcattacccggtattaagcaggtataatctgggtattttgggtaatcctttaccggtagaaaacttcgatgcccgggccgatggcggtaaagtgctggttagctggcatatgccttatgaaatcaacagcagcaggtttgtgatagaacgttcccggaatctccggacttatgaggcggtggacacggtggctgctcatggcagtaccgcggaggcatccgattatatttcctatgatgagcaaccctggccgggattttccgcttaccggttaaaaacaattgggctggacagcagcgtaaggtacagtccggttaaaatggtattggtaacggacaaggacttctggcggaagctgttatggtgcatatttggccaccagttgcagtattggctggattggccccgcagtggtgatgctaatataacgttgctggatgtgcagggtcgtgttcgttaccagggcagaactacctttgtaaagggccggaactacagaactatcgctaccgaccagttacctgcgggcatatatttcctgagagtgcagtcgggtgaattggtgcaggtgaccaagattcttattaatcagtgatcttttttgaaaaaaccatgcaaatgagacgccgccctgtttaccggggcggctttttatgtatgggtatcaagtaattacgcattattctctataaaaggcaagatatttagggaaatcggcctttcatgcgtggaaataaggaatagttcagtatctttgcggtcctaattttttaattaaaccatttaaaacagggaattatgaactacgaattgatggtgatctttacccctgtgctttctgaggacgactacaaagccgcccaaaagaaattcgctgatatcattaaagataacggcggagaaatcacgcacgaaaatccctggggattaagatcactggcgtatcctatccggaagaagactacaggaatgtatgttgttctggaatacaatgcgccatccgacctcaatgagaagctgaaaatccagctgaatcgcgatgaaaatgtattacgtcacatgattactgcgctggacaagcacgctgttacttacaacggtcgcaaaagacatggcgtaaatgctgaatctaaaaccactgaagcttaaaactatggcagttaaaccgaaacaagaaatcaagtacttaacggccgtaaaaaccgagaaacgtcagaagaaatactgccgtttcaagaagttgggcatcaagtacgtagattacaaagacgcggagtttttgaagaaatttttgaacgaccagggcaagatgttgccacgtcgtattacgggtaactccctgaaatttcagcgtaaagtagcccaggctattaagaaagctcgtcaaatggctttattgccttatgttactgaccttttaaagtaagaagttatgcaaattatcttaatacaagacgtagataacctgggtcagaagaatgaactggttagcgtaaaaaatggttacgccaggaatttcctgattcctcagaaatttgcggtagaagcaagcccttccaacatgaagcagcttcaggaacgcctgaaagtgcagaaagtgaaagaagagaaactgctggctgaaattgcgaaagtagtagaagtgttgaaagcttctcctgttaaaattggcgctaaaaccggtacatccggtaagatcttcggtagcgtaactggtgttcagattgcccgtgcaattaaagaacagaaaggttatgaaattgaccgtcgccgcatccacatcctggatgatgttaaagaactgggtacctacaaagctcgcctcgatttcggtaaaggcaacgaaaccgaactggaatttgaagtagtagctgagtaatattccaacttgtttggaaagaagaaagtcccgggctgaatcagcccgggatttttttgtatcaatatgattgcatttatgtttcattaacgaatggcaactgagttgttgatagatttggttatatttgtaatgtaaccacaatgaaaccagcaaaacacatatcaacacctgatcctaaagtcatcactattctgaagaagatgatagcggataagaaattgattcatgattacattacgaacggccgtgatttatctgaattaaaatctaaaggtattaagtttgttcagcccttataaactcacagaattaaaagtcgggttatatcaatttacaactgatcaagaggttgtttataatgtatattttggggatggcatctgctattttcaggattatccggaattttccgatgatgtaatgacattcggatttgacaggattagtagcccccactctaaatcccgcgccgacataaaaatccgctttacaattacccatcacattcttaatctccttaatgaaaagcaagacaaaatcttattttttgtctgcgatagtgcagacagcagaggaacggccagaatgagaatgtttgagcattggtaccagcagcaaaaaatcagttttcttgaaaaatataatgagtctatcaccacatcagaaatagatattcactgttccatcattcttcattcaaaaaacgttatgaaggaacacatcatttccagctttcgcaatctcagtaaatccaccgccgaaaaactcaaatcttattagtattttcataccaatattccgccatgagtatgaaaaaaattatcttcttctttatcgttgttgttaccgcctcggcctgcagcaccagaaatcacaggcccggacttccccggctgaccaccatcagcatccagggagaaagcatgccccagtataccttccggtatgatcagcagggcaatctcgctgaactggtacatcaccggccattaaacgataccatcagcactttttcctatgatcattcccaccggattaccggaatggtattatccaaccgggaaaataacgtcacagcagtaaaagagcgcgctaaagtcacttcctgggataaagatggtaacatcgctaccgtacaatactttgatgcaaaggaacaactgctccgcgttaccaatgttcgctggaagaacgggttacctgctgccatgaagtactccgattccacacaggcagtcagctggaattatgatgccgcaaacccagtaagaaaagatatctgtatcgatagtttctcaggcaaaaaagaagataccttagttactttgagaactgcaaaatacgaatgcgaagattctattaaccccctgcatcccctggccaatcagttgctgctcagtcatgctgtggctccggtcgtcaacctttctccccagggtgacttatcagacgcttttctgcacctgaatacccataatccttttcttatcaagattacagaaaaagaaaaaacacgctgccagcaaggtttactcgaatatgaccgcactaccactgttcaatatgcctactatttcaacggcggccgccaatatccggctggcgcctgggtgcatttacacagtgaaggatataccaaattgggaagtgacaaccattttgcacttgaatatcaatacgaataacgcgcaattggggatttttcattaacttttaggagatgaaaatcacagaccgattaaaggagatgccggttacactggtgttgatcggcataaacgtacttgtatttctttacaccatactaacaggaatgagtatatggtggggagatggaacccacctgctgcatgctggcgccaactattggtcactgaccatagagcaacagcagtactggcggctatttgtcagcatgttcctgcatgcaggaatgggccatcttttcacaaatatgctgggactgtttattggaggcattttcctggaaccggtattgcgtagtttccgttatggccttgcctatatgatcacaggattaatatccgactatgtcagcatctggtatcataaaggcgcagtgggtgtaggcgcttccggtgctatttttggtatttacggtgtattcctggcgctgctcaccactcccctcttcccggcggagataaggaaagcgtttctggcttatattggtttatttatagcattaaatgtaatagctgctgcggtttcacaaggagtggataatgcagcacacctggctggctttctgagcggcgcccttaccgggtatcttttcttttttacactgacaaaagcagatggggaaagacttacccgctaaacctcttccgaaattctaaatacttacatttgtacacttaaatgcaacaaaagatgatgaataagttatggtttctgctgtgtgtatgcgcaataatgatattgagctgcaaaaacaaaacagcagataacaccaacgccactgccaacgattccacaccgcctgctattaataaaactcccgatgataccgttcagctgggtaataaaaccttcttcgtgtactttatcgaaaaaacagatttcgataaatttccgcttgctcccccggattccagcgaagcagatgtactggcaaaagacagcctcgtaaaaagggaaggtaataaactaaccatccagctggaaaatggaaagcaaaagatcatggcgaataacaacaacgacggcgaagattatatcggctatacctatgccggcagttatccagctatcaaaagaaaaggattttttattacctactacgaaggcagtgcctttgagctggtaaataccctgaatggcgattctatggtaacctggtcggcccccgccgtttcaccggataaaaagtatatcatcaccgcatcaatggacctcgtagccgcttttgatcctaatgggtttcaactgttttctgtaaatggtaacgacataaaagccgtgggagaagccagcctcgacgactggggtccgggcctggtacactggatcaataacaaaaccattctatctgaatacattacaatagacgaggaaggaaatacacaaatacgctatgtaaaaatggtaatgcaataacagtatttagtatatttagtgagatatcgcatatcaaatccacgctcatgaaaaaactgttcaccgctggtttattaatagcactcacctcttgctataccgcttttgccgcgctctccccagttaatacaagatttcaggcgcctaccatgaatgtggagggaactgccagttcaatcgtgagcaaactggataaatcgttgatccttaccgaaacgcaaaagcccaaactacttaatatcgtaactaattacctgcgacaaaaagtcaatatccaaccactgcaacaaagtaacctgaaagcttatactaccaagatgaacagtatgcaaaatggattgcatgcaaagctgaaacccctgctaacactcacacaatacacagagttcctggggctaaaacctaaatccttcgacgacacaaatgttttgtcgcaattatattactaagcaacgcggattttgtcttggctcaggattacgctgattatactgattagtttgatttttacttttggattttttctgatttttagattcaataataattaagggagataagagcgaatatatccgcttctatctcccttaatcctttataaaatccaaaagtaaaaatcaaactaatcagtataatcagcgtaatcctgagccaagacaacatcaaatgataatctgccggtcgcgcgctacgatacgccagttggcgaccaccgcattgcgctccgctacatatgctttttcatatagcgccacggtggggcatatatgttttggtactccatacaacactgtgcccacgggatattgggttgcatccgctactttcaataccaggtgctcttcactctgcgataccggttctgctgccggtgcattcaggaattgcacccttggctgcggattctctgctgctacggatttatgcccgagatcaacgcaaatatgctgttcatcgataacagaaatcacgcggctgatcaccaacgcagcccatttaaacggctgctccggcaggttagctgcgtagcccgcatcccagaaaatgaaagtacccggactgcaagtgatacctttccttgctgcatgtaccgggaacgtgggtgtgccacctgcaacaatctccggctgtggtaacccactatttgttacagccgctgccagtgcagcaacaggtgcatatgcttcatcacaacgccgttttcgtatatccatatccgtatcatgcaggtgaccgtcgtatgcgtgtaaccctacaggcactactcccggcaaagtgttaagatattggtatacctccagcgcgttgggcccgggcctgacaccggtgcggttcattcctatattaagatccacatatacgggcaaccggcgcccctgcgcagcgaaaacagtactgatagccagggcagcatcagcgttgtcggtaacacaggaaaaaacggtatgcggatatttctgtaccagttccagcaaacgcacaatcttcggtcccaccggctgataagccattaaagcatcagctgcatttaccatccccagcatctctccttcggcaatggtggcaaacttaaaacgtcttattccctcttccatgatcagctgtattacctcagcgatcttactcgtttttacgtgtgggcgtaaccgttgtatgtcatcgatcattgtttttagcaatgagatgttatcctttatcctgtctttataaataacaattgccggagaatcaatctgcgcagcatttgtaagttgataccattccatgcagggaaatttaaactatactacgtataatcatacacgttatacaaacaaacttaggatcaaacagccaattaaacctgttactgatacaatagtttccattatcgaccaggttttaatagtgtctttcacagacaagttaaagtattccttaaacatccagaaaccggcatcatttacatgggaaaacatcaggctgcccgcaccggtagccagtaccatcagactcggatttacaccggatgcagcaatcataggcgctacaatcccggcggttgtgagtcctgctacagtagcagatcctatacacacccggatgatagccgcaataccccatgccaggattaacgggtgcaggtgcatattctgaagcgtggtagcaatgtaactgctaactttgctgtcgtgcagcaactgcgtaagcgcaccggagccgcctattaccaggatgataacggctacatcccgcacggcatcatccattattaccattactttttttgcgggcattcctcttctcaatcccaataaatacatgccgttcaacactgccagcaacatcactatcaacggctctcccagccagttggccagtctgaaaagaaaagtatcttcaggtatccataacttgaccaaagccgtcaccgccagtaaaaataccggtaacaacgcagcaaagagactcacaaacatacccggcaattgttcttccggaatcggtggcgccacaaacatttttcccgggggattggtgtagtgtttcaggaaacgcgaaaataccggtcccgccagcacaatagccggaatagccaccataacaccgtacaacaaagtaagccccatgttggcatgaaactgctgtatcaacgcagttggagagggatgcggcggcaggtatccatgcgttactgataaagacgcgagcataggaataccgagatataccaccggtaactttgtacgtgccgccacggtgaagatcaggggcaccatcagcacaaacccgatattgtaaaacaagggaatccccactataaaaccagtgagcatcaacgaccattgcacatactttggtccgaacaggttcattaaaccgccggcaatcttttgcccggcgccgctttccgccaccagctttccaagcatgctgccgaaaacaatcaccacaatcagggaccctaacgttttacctatgcctgtttgaatagactgcgtgatgtctgttacgttcatatgtaacgccagtcccatcagcaaagacactataaggaaagagaggaaagtatttaaacgccaccaggcgaccagtattaccagcaagaggatggccgcaataacaattaataagggcatacagctgttgttttacatgaacatggaaaacaacaagataataaaatattattcgtatctcaaggctataatcggatctaatttggaagccttataggcaggatataaaccggaaacgagccctactgcagcacagatagttactccaataatgatccagaaccacggtacaatgaaagcagagctcagtaatacggaaacaatatttcccaggagcatgcccataattacaccgatcacccctcccattacactgataataatagactcatacaggaattgggtacgcaccacgtgactagtggctcccaacgctttggtaacacctatttcgcgggttctttcggctaccgataccagcataatgttcatcagtccaatagcagaaccaaagagcgtaataaaggcaataacaatagcaaagaggttcactttgcccaaactggaaaaaagcatttctgcaatactatcgctcttgctgatctcaaaattatcttcttcattaatattcaatccgcgtataatacggaacaggcctgtggcctctccctgggcggcgtccatttgcttgatatcttttacggctactgctatctggtaactggcgttgggccggttaaataccctgcgggtattattcaccgtggtgatcaccacgttatcggcgctcatcattttgctgctgccttttgatgccagtacccctactacgcggtaccggatgtctcccacgcggatcgtactgttcaccacatttttaagctgtttgccaaatagtttctccgccacatcaattccaagaatagccacatttctgccggactgaacatccagctggttaaaatcccttccctgtgaaatctcataattggaaatctgcaggtagtgttcatctccccctatcacctgtacattgggattcgttttcttatcatctttatataccgtggcaataccggtggcctggaaagacacactcaccacagccgggaagtgataacggtcccggaaggccactgcttcctggtaacggataattttattgctgttggatttttttaccttttttacatgcttgtttcccttggaagctttattgttatcatccccgatatgcacctgcatcccccggttacggatagagaaactgttagcgcccatgctcgcaaagctgctgtagatgctgttcttcatactgtcgatcgccgtaagaatacctaccagtaccgtgatacccaatgcaatgatggacacagtaagaccagtacgcaacttgttgctggttacagaacggtatgccagggaaaaaatatctcttgattgcataataacgggttacctataaagttaacgtaatatagctatttaatccattcaatttgggatgaacggcgggtaacggcgatcagtataaaagagaagaccgaagcggatcaggtaaatcgcttcggtcttctccctatgttataagctcacagcttttacatccagcataataaaaggttcgggaacaggcccaataccagcaccagtgctatggccaggatcagggcagccttaaaaccgcctgaaacaggttctacttcgggttccccctgtttaaaatacatggcaatgatcacgcggaagtaatagtacacgctgatagcagcacacaatactgctatgatcaccagccataaaatatgaccatgttcgatagccgcggctaaaacaaaatattttgcaaagaaaccagctgtaacagggataccagccagggaaaacaggaacactgccaccgctgccgccagcaaaggctccttgcgggccaggccgttgaatccttcaaaggtataatccttcagtttcatcagtaccgcaaaaacgccgatagtggcaatactgtaggcggcggagtacaggataattccctgcgcgcccctgttattcatagccactactgcaaacagcataaagcctgcctgcgcaatactggaataagccagcatccgtttcacactctgctggaaaactgcgctgaagttaccaagtatcagggtcgctgctgtgataatagaaaggatcagtgtccagtgtccgctgatgctgccaccggcaaagctggtgtggaacatccgcaggaaagcaacaaatccacctgcttttaccacggtagacataaaggaagtgaatacagtgggggaaccatcgtatacatccggtgtccagaagtggaatggtactgcagatactttaaaagacagggcaaataccatcaggatgatgccgcataacgccaacggatgcacgctttctgcaccaagtcctaatgctgcaatatcaaaagtgccggcggcgccataaatcagggtaatacccatgagcaggataccggtagaaaaagaccccatcaggaaatacttcagggatgcttcattgcttttgaggcttttcttatctgctcccgcaagaatatattgcgggatagacataatttcaatcgccaggaacaacatcagcaggttactgaacgaggtagccagcgaaatacccgccaggataaagaataccagggcgaaataatcagctacatgttctcctaccttttcaaattcactgcccgacaacaggaaatataacaaagtggcgcccaatgctacagcgttgaacaacacaccaaatttggtcacttcaatcatgccatacatgatatacccgccctgctctacagacggatattgcgccagattagcaataaatgctatgaggatggccgcgatggcaaaaaatttaatatgctgcttattgcgtacaaataaaccaacaaacatcagtacaacgcccgataaagcagtagaaattagtgcattcatatttttgcgttacaaaaccccgttacaaatttttccattccggtattcagtttttggctgaagatcagaataatttacttaccacatcagacgtgccgctcaccagatccagcataggtttgggataaacgcccaatactatgatcatgatcaccaccaggctcagtgccagtgtttcacccggctgcagatctgtagtagtttcggttaattcatttccttcgccaaatatcactttctgaatcatacccagggtatatacagcagagagaatgatacctaatccggcaaatgccataaaccagtgattatattggaacaatccgctgaacatcaggaactcaccaatgaaaccattggtcagtggtaaaccgatgttagccagactgataataacgaggaaaatagccatgcgtggcgccttctgtgccatgccgcccatctggtcgagatttttgatccctaaacggttctgaatgacttccacgatgatccacaaaccaataatattgataccgtggttaaacatctgtaccattactccctgcaggctttgttcgttattggcgaaaatagcggcgcacatcaaaccgatgtgggcaatggaagagtaagcaatcaggcgtttcaggtcgttttgtaccattgcaatgcaggaagcatagatgataccgatgatacataatacaatagctacatcagaccacatggcagcgccctgtggcactaccggcagcagccagcggatcaccccaaataaacccattttcaccattaccccggaaaggatcatggtaacaggggtgggcgactgctcgtaagtatcgggctgccaggtgtgaaacggaaataccggcatcttgatggcgaatgccacaaagaacagccagaacagccatttctggtcgtccggatttagcgccgcacttgtaaaggaagcccagctgaaggaatgatccggtgtttgaaagtagatatagataatacctaccagcatcagcaacgaaccgaggaaagtgtatacaaagaatttaaaggtaacggcgatccgtttttcaccaccccataaagagcagaggaaataaacaggtatcagggccagttcccagaatatgtaaaactgcagggcatcgaaagcggtgaatacaccagttaagccagcctgcgataataacatcagaccataaaaggcattggccttttcgtagttgcggttataaatagtaatgaaaacaagcagagaagcaatcgctgtaagtaagcaaagcatcacacccattccatctaatccaacacggaattgacttcccagctgcggaatccagtcggcaacaaagttcaggctgtcgggagcagtacgaaagcggcaccacgatccaattgccaacaccactgttgccagcgatgagatcatgcccagcacttttggcccggaccccttcagaccaaatgcaataaggcccgctatgaaaggaatcaatattaataaaactgtcaacataatttatctgcgcttgtaacttctgctattggtttataataagaatccgatcacaaataatacgatcataccgatgaccatggcaaagatgtaaaaacctacctgcccgttttgtaccaggcggatctgctgacctccccattgtacaccgcggcctacaccgttcaccagcttgtcgatacccgccttttccaccgtatcacggaagaaacgggacgacaattcatacaatggttttacgataatagtatcatacagttcatctatataccatttgttttcgagcacttttgccaaaccagtactttctgtacccgcatcttcaaacttcgtaaatttctgacgcgccagcaggataaatacaatcaccagcacactgctcacacccatcagcaaccattctgtactgtgcgacaggtgatgttccactgcaaaaggtgcagatggtgcaaacaccggcgccaggtattcggccagcatattctttgttccaaacacttcgggtaaaccaacataaccacctatcacggaaagtactgccaggattaccaaaggaatggtgatagcagaaggactttcatgcaggtgatgctcctgttcgtgtgtgccacggaatttaccagtgaaggtgatgtagtataagcggaacatgtagaaggcagtcatcagtgcgcctaacaggcccagtacatataataccgggttgttggcaaatgcctgcgccaggatttcatctttggagaagaagccggagaaaccgggaatacccgcaatcgccaggcatcctaccaggaaggtccatgcagtagtaggcatgaattttttgaggccacccatcttcctgatatcctgttcgccacccattgcgtggatcacggaaccggaacccaggaacaggagggctttgaagaaggcgtgtgtcattacatggaacacagccgctccataagcgcccacaccgagggcaaggaacatataacctaactggctcaccgtagaataagccagtacttttttaatatcgttttgctttaaagcaatagaagctgcaaacagggcagtagccagaccgatgatcgcgattactgtctggatatgcggcgcgagtgtataaatcacgttgctgcgtgcaatcatatagataccggcggtcaccatcgtagcagcgtggatcagcgcagacaccggggtaggaccagccatcgcatccggtaaccaggtatataaaggaatctgtgctgatttacccattgcgccaacaaacatcagcatggcaatagcggtgataacgccattgttcattcccagcggcgccgctttggcaaacacgtcggggaaagtaaccgtaccaaactgcaggatcatgaagaagatagcaatcaggaaaccaaggtcaccgatgcggttcatcacgaatgcttttttagcagcattgttatagctggtatttttaaaccagaaaccgatgaggagataggaacaaagaccaacaccttcccagccgataaacatcatcacatagttggcgcccagcaccagtatcaacatggaaaacacgaagaggttgagataagcgaaatatcttgcaaagctttcgtcactttcctcatgcatgtaagaagtagagtagatatggatcagggtacctacgccggtgatcaccagcaggaacaaggcacttaactgatctacctggaaggcgaaaggaatctgcagagaacctacagaaatgaaatcaaacaggtgtactgtctgagcagaaaatccgggagctttaacttccaggaatattaataagctaatcacaaaggacgccagaactgcgccactgccaacaaatcctaccagggacttggataaaaatctgcgtcccaatccattcaccaggaaacccaataatggtaaaaatggtaccagccaaactagattaatcatttatcaattctatttacgacgtcgaaaaatttaataattaagacagcagaattattaatttttcagcctgttaagaatgttaatatctactgagtgtgtgtttctgtagaccatagtaattatagccagtcctactgctacttccgcagccgctaccaccataataaagaatacaaagagttgtgcagaacctgcatctacccttcctgcatctgcccacattttggaaaatgacaccatcaacaggtttactgcattcagcatcagctcaatgcacataaaaataataatcgcatttctgcgcatcagtacacccatcacacctatgcaaaacaaggcgatactcaggaatatgtaatattgaacaggcataaaataaattacgggttaggaattacgaattacaacaggcaatccgtattactattcttttttaccaattaccacggcgccgatcattgcgctgaggaacaaaatactgctcacttcaaacggcaccacatattgtttgaacaggatcataccgagatttttaattaacccgatatcagtagcatttgtgctcaatgccggcatgctggcatcgcgtaatgcagctaccagtaccaccagtaaagcgcccccgctgatagcgccggcgtatttcagccagttgcgtttctgcggttccaggtcagcattcaggttcatgagcatcagcacgtagaggaacaataccatgatggcccctgcatatacaatgatatgcactactgccaggaactgggcattcatcataatataatgcccggctatggtaaagaatgttacgatcaggcacaacacgctcgttacaggatttttactcaataccacgcccaacgctgataccagcgcaacgaccgacagcaccatgaaaattatttgttgtatactcattcccatctctgctatgtttgactattgtatttttagctaaatgtgcgctgtgaataatattatttgccttctttcggatgaggaatcagcagatcatcttttccgtagataaagcctttacgctgatagtttgcaggagcaaaagtttcagacatatacactgcatctttgggacaagcttcttcacaaaaaccacagaaaatgcaacggagcatattgatctcatatttcgctgcatacttttcttccctgtacaggtgctcttctccctctttcctttccgctgcttccatggtaatggcttcagcaggacaggctactgcgcacaatccgcaggcagtacatctttcacggccttcttcatcccggttcagtacatgtaaaccacggaatacgggactgaaatcacgtgtcttttcaggaaaactaacggtagctttcttctgaaaaaggtgcttaaaagtgatccccatacctttggcaatagcagggatgtacatcttctcggcgaatgtcatcggccggcggtctactgctttcgccctgttagttaatgcttgcataatgaatgctttatttaatccacacgtttggtgtgtatttaatcagataatattaatgttgacgagccaataccagtgccccggtgatcagcatatttaccagtgccagcggaatcatgatcttccagcccaaacgcatcagctgatcgtaacggaatctcggaacggtccagcgtacccacataaagaagaaaatgaaaaacagtgttttcaggaacagcgccacaaatccgaggatggtgaccatgttcggatccagtcccagctgatccatatacgggaaggcatacccgccgaagtacatggtagagatcagcgcagaactgataaacatgttgatatattccgcaaacaggaagaaacccagtttcatggaagaatattccaggtgataaccaccgttcaattcgttttctgcttccggtaaatcgaagggagcgcggttacattcagcaaaagcgcataccaggaagatgaaaaagcctaatggctgatatactacgttccataaaccatgacgctgttgttccacaatatcctttaagctcagggagccggtcagcatcagtaatgcgatcagggccagtcccattggcagttcgtaggagatgatctgcgacgcggcacgtacagatgccagcaaagagtatttattattggaagcccaaccgccaatcataataccatacacccccatgctcactacgccgaagatgaaaaggatcccgatgttcacatctgctatctgcagggaaacgggacggccggcaattaccagggtatcaccccagggaatcacggcgctggtcatacaggccaccaacatcgcgatggaagggcccagtacgaagagaaagcggttagcgttggtaggaataatttcttctttgaagaagagtttaccaccatctgccaatggttgcagcaatcccataaaaccggcgcggtttggacctaaacggtcctggatccaggctgccacctttctttcaccccaggtagaatacatagccactaccaatgaaagtaccagtacccctgatatcaggagtactttttcaattataaaaaaccaatctatgcttaataaggtcatacttacacgtaattacgattgttacttcttaaaatcatcagagtgagccgggccgtcgatcttcgacaaatcaatgtccggtctgtttacctggctttcagagtgaatattaaacaacagtttgggttgtcttccgtccaatacatccaccagcggatctttaggttttacagtattcacgtaatgcccctgggaaataacgctgttacgttctattttgcgtggaccttcaatgatccagtcttttgcttcttttttttcaaagcggcaaacatcgcagataaagtcttccacttcgccgtatttatctttacgggcggttacgcggaatacttcgtcgccgcgcatccaaagcacagttttaccgcagcattttggattttcgcaattgcggtgtgcatctaccggtttcaggaaccatacgcggtttttgaaccggaaagtttgatcggttaaggcccctaccgggcaaacgtcgatcacgttaccgatgaagtcattatcaagcgactgggagatgtaggtgctgatttcagaagcatcaccacggcccaggatgccatgttcgcgtttttcggtaagctgatcagcggtgtacacgcagcggtagcaaaggatgcagcgcgtcatgtgcaatttaatatgatcaccgagatctactttatcaaaagttctgcgtttaaattcgtagcgggtgctgtcggcgccgtgttcgtaactcagatcctgcaggtggcattccccggcctgatcacataccgggcaatccagcgggtgattgagcaacaggaattccactactcctttacgagcatccagtacttccggggaagtgatgttggctacttccataccatccattacagtagtacggcagctggccaccagtttaggcatggggcgtgggtcggcatcggaacctttggatacttttaccaggcaggtacggcatttaccgccgctgccctgcagtttggaatagtaacacatggccggcggcactacctctcctcctatcttccgggccgcattcagtatggttgtaccgggttccacctccacagagatgttatcgattttaaccttaaataattttatttcctccgccatcttaatatcttttgtgctcgcggggagcaacgtttattttatatattgattctttatttcagtatatgcatacccgttatacagcagctggtgttggcgccggcaatgggtctgcgtaatgagccagaccgaaattgcgggtctgtgattcttcaggatttgccacatgccattcaaattcatcgcggaagtggcggatagctgctgctaccggccatgctgctgcatcgccaagcgggcagatagtgtttccttcaattttgcgttgaatatcccacagtaaatcgatgtcgctcattttgcctttaccatactcgatgttctgcagcactttcttcatccagccggtgccttcacggcaagggctgcactgaccgcagctttcgtggtggtagaagcgggcaaaggtaagggtattgcgcacaatacactggtcctcgtccattacaataaatccgccggaacccagcatagagcctgttgcaaagccgccatcggccaggctttcataggtcatcatacgggtttcaccttttgctgttttcagcagcaggttagccggtaacaccggaacggaagaaccgccggggatacaggctttcaggcgtttgttatttttgataccaccgcagtattcgtcggagtagatgaattcttctacggagatattcatttctatctcataaacgccgggtttgttgatattaccgcaggcagaaatgagtttggtgccggtagatttgccggtaccgtatttaatatattcgtcgccgccgatgttgataataggcactactgcggcgagtgtttccacgttatttactacggtgggcgattgccataatccttttaccgcggggaatggtggtttgatgcgcggattaccgcgtttcccttccagggattctatcagggcagtttcttcaccacagatgtaagcgcctgcaccacgttgtacgtatatttcgagatcgaagccggtgccctggatatttttacccagccagcctttattttttgcttctgcaatggcctgttccaggatgtccggaatccaggcgtattcaccgcggatgtagatgtagcaactgttagcgccgagggcaaagctggagatcagtaatccttcaatgaggaggtgggggatgaattccatcaggtagcggtctttgaacgtacctggttccgactcatctgcattacaaaccaggtagcgcggaacgccttccggtttggcgatgaaactccatttcaggccggtagggaaacccgcaccgccacggcctctcaggccactcttcttcacttcatccagtacgccgtccggccccagggttttcagcgctttttcagctgcagcataaccgccgttgctccggtaggtgtcatagtaccggatgccttcaatatgtgctttatctaacagtaatttgcgtcccattgtcttccttatggtgtaatgttaccggtattcccggcgccattatcagatttgtgtatatcttttatgccttacgtatgccgtgttgcgaaatgcgttctgccagtctgtaaaacaggagcccggcacttacgccacaaataacggaaaccagccagttatcgatccgccataatgcggtgagtaacgccatcagcagtattgcttccactacctgtaatttgtggcgctgatacatttccttaaaacgcatgatcaggttattttttggatgcatcagttggcgtttgctttagatctgcattctgcgatgatttcatctactttagccggtgtaaggtgctcccggtaatgttttcccaattgcatcatgggagcataaccacaggcgccgaggcattccaccgttttaagggtaaacagcccgtcggcggtagtttcacctacgccgatacccagcttatttttaatgtaatcaatgatctgatcagaaccacttaccatgcacgggcctgtttggcacacctcaaataaataggtgcctaccggtttcaggttaaacatgctatagaaagtagctacctcatacacttcaattgattgcagttgcagtaaagttgcaacgtagtccattgtttctgcactcagccatccaccaaatgcttcctgagccaggtgcaacaccggtatcaacgcacttttctgcttcccttccgggtagcgtgcaatgatttcttttactttattcagtttctcttcagaaaattgaaccacagccattattttattcagctttaatcttcgaaatattcaatagcgtaactacgcatccagttcacctgcgatcaggttcagactactcatacaaacgatcgcatcgctcaacatggcgccttccaccagctcggcgtaggcctggtagtaaatgaagcatggacgacggaagtgcagcctgtaaggactacggccaccatcgctgatcaggtaaaaaccaagttcgccattggcgccttccactgcgttgtacacttcacccggaagcatgtctgcttcacccatcacaattttaaagtgataaatgagcgcttccatctttgtataaacatcctgtttttcagggaggtaataagcaggtacatctgcgtggaacacatctgccggcaggcttttcaccttatccatggcctggcggatgatactgagactttcccacatttccgcgttacgcacctggaaacggtcgtagctgtcgccggtagtacctaccggtatggagaagtcgaaatcctggtaagagctgtaaggattggctacacgtacatcgtaatccacgcctgctgcgcgcaggtttggaccggtgaagccgtagctgagtgccctttctgcagtaatagcacctacgccctgtgtacgttccatgaagatacggttacgggtaagcagggtttcaaactctttcagtacagcaggatattcgttcaggaagcgttctatttttgcgaaagctgcgggcgtgaaatttctttcaaagccgccgatacgaccaatgttggtggtaagacgggaaccgcagatctcttcatatatttcgtatatcagttcacggtaggtcatcacgtatacgaaaccggttaatgcgccggtatctactcccattacggagctacagatcaggtgatctgcaatacgcgccagctccatgataataacacgcagataatccactcttttaggcgtttcaatgcccaggagcttttctacggtcagtaaccaacccatattgttaataggggcagagcagtagtttaaacggtctgtcagtggcgtgatctggtaatagggacggcgttcagcgatcttttcaaatgcgcggtggatataccctacggtagaaacagcgctcacaatgcgttcgccatcgatttccagaatgttctgaaatacgccatgcgtggccgggtgtgtaggacccaggttgagcgtggtcgtatctttttctatagagccttccggcagctttatatgttgtttctgatctaacataacctcgttgtattaaagatttcctccccttccaaacatctcatcatctttatcaatacgcatggagtcttccagcggaaattcctttctcatggggaaataggtcatttcgtccacattcagcacacggatcaggttgggatgtcctacaaagttgatcccgtagaagtcgtaagtttcgcgttccatccagttggccgatgcgtacagctgggtagcggtaaaaacgtccggtttggctacgggtgtgaatactttcagacggagcctgatgttatcctgcaggttgtgtaggtgatatactactgccagttcttcgtttttcctgtcgggataatgcactgcggtgatatccgttaaaaaacgaaaacgcaattcctcatcatcaaacaggaattgcattactttcaggttataatctttctgtgcggtgagggtaagcagcccaaacggctcttcaaagccggttagcacatctccaaacttctccgtcaggcgttgctgtatgcgttcgtttgttaaagacattaacaatttgaaatttacgatttacaattaaccattcccctctccttacttgataccgtaagactccatcagttctttatacctgtcggagttacggcggcggagactttcctggcctaccagggcctgtattttcatgaagccatcgatgataccttccggtcttggagggcatcctggcacatatacatctaccgggatcacctggtcgattccctgtaatacagagtacgtatcaaatataccaccgctggaagcgcaggcgcctacggccattacccagcgtggctctgccatctgcaggtatacctggcgcacaataggtcccatttttttggaaatggtccccattaccatgagtaaatcgcactggcgtggcgtaaaggccatacgttctgccccgaaacgggccatatcgtaagtagccgccatggtagccatgaattcgattccacagcaggaggtagcaaatggtaaaggccagatggagtttttacgcgccaaacctattaccttgtcaaaagaggtggcataaaatccttcaccggaatatccctcggggatttccaccatcttcaccttgttattatattgaaccggacgagccattggttttaatttaaagagttaattaatcttcccatttcagagcacccttctttgtgatatagataaatccacacaaaaagaagcccacaaacatcagcacggccgtaaagccttcccatcccaattccctgaaattaaccgcataagggtagaaaaagattacttctacatcaaataacacgaaaagaatagcggtcagaaagtatttgatggctaccggctggcgggcgttacccttttgctcgataccactttcaaagttgataagcttgtcgctggttttgcgtttaggacctaaaaagtgagtagctaacatcgtgatcccaacgaaacctaaagcagcaattaattgcagtactatagggaaatagctaaaaggagtagtcgttgctgacaaaaatacagtttctgtatacataagcttcccgataaaaacattgtccgaatgcgcaaaaatactgtaagttgaccaattatcaaatctattaagagttaaaatattatcttttttcaccaaccggaaactaaaaaacctcctgcgggtacaggaggtttttagcaattatatgtaattaataactatttcttgttctgaccctgctttgcagctggtttggcggctggtttttcacgggcagccatattttcattgatctgtttaacagcggtgttattcggatctaaggcagtcagtttatcagcatatacttttacattggctttatcttccttaaagtagtagtataacagctcataagtgtaagcgttgatcagcgtacccctgtttttagcaggatcaacttcagagatttctatgtatttatcatagaaaggttttgctacaccggcctgggcctgtggatctttagcaaaattgctctggcctctccagtagtaaccggtacccagctcaggttttgcttcaattactttctggaaagcagaatcggctttagccagcaaagtagtatcgaaaggcttaacatttacggcaccgtagtagtagttgatacctacgttgaagtaatcgatcgcctgcagttgctctttattagcgagagataattcgttcgcttttgcataccattctgccgcagcagtatagttacgggctcctttcagctgctctgcgatctggataaaggtttccggatcttttgtagtgatagaacctgcatatttttccaggtaagccagggcctttgtattgtattggttctgggtagcggaatcagaagatttcagcttcatgtagatggctgacaacagtttgtaatccgcagaatccagtttgctttctcccacctgctgcacataagtatccattgttttctgggcgttcagggaatcacctttctggaggtaagagtccccgatcagcagtaccaactggttcttataggcgtcggtggcatttggcaatgctgcctgacctttactgatagcggcatcataatctttcttgaagaaagaaatagaagctgacagcagttcattcttggttttatcagcaggatcggctaccgccatatatttctccaggtattgcgctgcattttcccaggaaagctgatcttttttaggagtggtgtagaacaggaacagttcatataaggccggaccatatttcggatccatgttggtggctttcgtataatctgctactgcttctgctttcagcctggcgttatagttcaccaaaccctgtttcattactgcttcagcgttgtttggatcgagttccagtgctttttcataagtggtgatggctttaccgccgttttcaccaccgaggaagcggtaagcatctcccagctcaatataatcggctgcaacgggagtatattgttcttttttcttacggccttcgttgttcaggagtttctccattacagtgagggcataagcgcggtcgccacctttgatttcgctgtttgcatcagcaatagcgcgggcaacatctccatcgcggccctgtgtggcggcgctggcggcatcaaatttctgttttgcggcggcggcattaccattgatcagatcaatacggcccataccagcctgcagtaaagcagatgtgggtactgcctgtaagcctttctggaaggtagcagcagcacctgcagcatcatccattccgagttgggctataccgaggtaataatacgctttgtcttccgtaggctttgctgcgatcactttctctaaattctgcttggcagacaggtacttaccgtaatacaggtctttcagtccgtcctccacagattgggccatcacaccgcttgaggcggcgcaaagcaatgctacgattaaacttttccgtttgttcatgcaatctggttttttagttttagttgtgtttttcttctacttaaggttggcttccctgaatactacattcaatctcgccgggaataaacggaactgcttcattaccagctgtccctcataactaccgagaaaggttgcaaatccactgccaagtccatgatatggttctttcaggcaatagaagaagccgcgttttaacggataggtgccaataccaatataggcctggtatggcttaacaaattctgaaccattgtctgctcttagtctgactacagatacctcacgtgtaaaagccatagacaatgaatcgttcggatcagagatccagctaacacctataacaccaatcgcgtctttgttttttgtcacataatccaccacttccgggttggttttcgcagccattgtattggttggcagaggtttacccttgttgatggaatccatgatataccgcacggtgcttgagttggcattgtcaaacaccagttgccacttcctgtctttattggtgccgtccataatctcacgtacctgattcatattcaacacagaatcaggattctccttatttaccaccagcgcaagcgcgtcccaggcaagtaaaaggctgttaggcgtaattttgatttgcttgaagtaatcgcgttcctgctggttgaaatcgcgggtaacgattaccaggcgggcactatcatttaaaagatctttaaagcaatcagcctccggtttataggtagggatgatatgtgcttttggatacagcgattgaaaaacttttatttccgaatcaatcagcggcttatatgtctcatccacacttatatggatggtgccttctgtagctgtatctaattttttcgcatttggattctgtccgcaagcggccatcatcaatgtaatagctgctaaatatacagcattcattctttctaaactgaaaaacatattacacctctttagttcctgttaaaaaaaagttttctcactccattataaaccctaaagaggccgtaaactattaaaaccgcaccaacaatactcatcatctgtggcgatattctgaattccccgaatcccagtttctccgcaaagattgcgaacaaaccaaagaggataaaaaatattcccctgatcagctcacccattggccgatacctgttttcctgccgtctgcttgtttgttcttcgtgtgtttccatgttgcgaattacaattatacaaaaaataattttttaatcggtcatagagaattttagaggaatgttaaaaaactgacttaaaaccgcacccttttgcttgtccagccgcaatttgaggcattttttcaacatgttgttattttttgatttacaatatgatcatttactgactattacaatttgcggcaaatacttctttgtaactcataaatccccgtttttttcttctaattcctgttaaaagatgcaaatacacccacatttccataatatcttgtaggtttgcggcctgatattcaaatattcatccgcatgaagatattgatggtttgcctgggtaatatttgccgctccccccttgcagaagggattatgaggcacctggcagcaacaaggggactggactgggaaattgattctgccggtaccggtaactggcacgtgggccattcaccagatcaccgctccataaaggaagcccggaaaaatggtgtggatatcaccggcttacggggcaggcagttccagaccgccgattttgatacctttgaccgcatctatgtaatggacaggaataattatgccgatgtgctacgcaaagcccggaacaactcggataaagcaaaagtagccttcctgctgccggatcagcaggatgtacctgacccctggtttgacgatgccctgtttgcacctgtttataaaatgatctatcaggcctgtgaaaacatcgcagaccagcaaccataaaacttttaatatttttcagagatgataaagcccggtattcctaaaggcacccgtgattttggcccggtggtagtgagaaaacgtaattatattttccagaccatccgcgaaacctttgaggtatttggtttccagccgttggaaacacccgcgatggagaatttatccaccctcaccggcaagtacggagaggaaggagataaactgatgttcaaagtactgaacaacggagagatctataacgaagcccatcaggctaaagataataaggaactcgtttccgccattactgaaaaagcattgcgctacgacctcaccattccattcgcacgctacgtggtaatgaaccaacacgaactggcccttccctttaaacgctaccagatgcaacccgtatggcgcgcagacagaccacagaaaggccgctaccgcgagttttatcaatgtgacgccgacgtggtgggcagcaattccttacttaatgaagtagaattactgctgatatatgataccgtgctaacaaaacttggcttgcagggttatgaattacgcatcaacaaccgtaaaatattattcggcctcgctgaagtgatcggtaaaacggaattactcaccgatattaccatctccatagataaacttgataaaattggtgcagacggcgtaagaaaagaattacaggaacgaggtttaaccactgccgatattgataccatcgaaaagttcctggcgattgaagggagcagcgaagacaaactggcacaactgaaagaactccttcagtcttcttccaccgcgttaaaaggtattgaagaattgtcgtttgtgctcaactccggctatgctaccttcaataccactcccatcattgatgtgacgcttgcacgtggacttaactactacaccggattaatcgtggaagtaaaagccccggctaccgtgaaaatgggcagcattggcggtggtggcagatatgatgacctcaccggcctctttggcctgccaggtatttccggcgtagggatctcctttggcgttgaccgtatttacgatgtgctggaagaactgaaactattcccgcaaacggcgcagcaatctaccaaagtattattcctcaacctgggagaagccagttcccgcgcagctttcagctatatgatgcaattacgtcagcagggcgttgccgcggagttattccatgaaccagcgaagatggataaacaaatgaagtatgcagataaaagagcgattccttatgtcattatcctcggggaatctgaactgcaggaaaacctggtaagcgtgaaaaacctcaccacgggccagcaggagaagatcagcggggcggaattgattagctacgcattttgattcaagcaataaaaaagaaggccgtttgtatgatacaaacggccttctttttttataacaacctgtttatttcgcgtgacgttttgcaaactccgctttggcatcttcaagatactttacgaaggcgtctacattttctttcggatcatagccataaccgatgttcagcagtgcattaccttccaggtctaccggaatgtagtatggctgcgagttacggttaaacttggtgatctggatatcctggttcttcaacccaacatcctttacattcaaccctgaagttttagactcatacctttcctcatcggaaagctttgtcttctcatcggtgtacaaagaagccacgataaaatcgttgcgcaggatcttcatcactgcaggattggataataccgacttttcaaacttacggcagtttacgcacgtatgcccggtaaagtcaatcatcaatggcttgttagccactttagctgctgccagcgcttcttcataatcaaagaaaacatgctccacgccgggaatttcagaatgcaggatatccaccagcttcttcggttttacagtgttggcattgttgccgccgccagtaccgccaccttcgccgctttccagtgctgcctgtatatttaccagtgatttgttgagattaaaatcctgagagccttcatgcggcaggaatccactgattcctttcagcggggcgccccacataccaggcaccatgtacaccgtgaatgtaaacgcagcaatggcaaaacagagacgggttactgtgaggaaaggcacatcgctgtcgtggctcagtttcagcttaccaatcaggtacagcgtgagcaacgcaaaaatggcaatccacagcgccaggaatatttcacggtccagcaggttccagtgataagccatatccacattagacaggaatttcaacgccaatgccagttccaggaagcccagcgtaactttcactgcattcagccagccgccggatttgccgatcttattcagcaaactcgggaacagggcgaatagggagaatggtatagccaatgccagcgagaagccaaacatcccgaccagcgggccggagtttcctccttttgccgccagcaccaacaggttacccaaaataggacctgtacaggagaaagacacaattgccagcgtaagcgccataaagaaaatacccgccatactacccatgcccgctttagagtcagacacattggcccaggagctgggtaagctgatttcaaaggcgcccaggaacgagaacccaaacaacaggaagatcacaaagaagatcatgttggcgatgccattgctggccagtgagttcagcgcactggcaccaaatattttggtgatcaggaaacccagcagggtgtagataacgatgattgacagggaataagtaaatgcgttcttgataccttctgcccttgtttggctacgtttggtgaagaagcttactgtaatgggaatcatggagaatacgcaaggcgtgatcagcgcaatgaatccaccgccaaagctggcgataaagatccaccacaaagatttgttagatgcgtcgtcgtccgctatgccgccttttacagcagcggtacctgcagtatcagcgcctgctttcgcggcggcaggatctcctgtaggcacttcaaaagtggtttcttcaggtaccgcatcctctcccttcagcaccatgtaagtaatggtgccggaaagtttggaaacgggtccggtggcttttaccgctgccaccagttctacctcattttcaaaatatttgatgtccagattatcgaataatggttctttgcggttttccagtttaccattctctgtgatacctgtaatagtggcttttacgctgctatccagtactaccctggtattaggatcatcgtttcccattgtggtggaaaaaagcaaccagcctttttctacagtgcccttcagatgcagcacatattcctggtcagttttcttttctgcagaaaactgccatttaacaggcttcgggcttgcgtcctgcgcgtttgcactaagtgcgaacagggcaaagacaggtattagaaatgaaagcaaatgcttcatatagtcaataggctttaaataatataaatctgagaaaacaagaaacgagttccgttgaggaactcgttttgcaagtattgttatcagttaccggattcaatttattttcctccaacacttactgcaaattccacttctttcggtggcaggcactgatggtcatcacaaaccatgtactccacagatccttttactttggtagcggctttgccttttaccgttactttttgtacaaagtctacagagctttcgtagaatttcagttctgagttaaagtttttgtcgaatgacttatgcagtttacctacttcttccaccttacctacagcggcagtcagtggatttttggtgaacttaaacgaggtagctaccggaccttctcccgcttcctgtgcgtacagatgccagccggcatcaatcgtagcagtagcgtgtacttcgtaggtagtggcattcaccttcttcgctgtaaagctccattttaccgggttctctatctgtgcacttgccaggatgggcaaggcgaataaagccagtgctgttaataattttttcatgcttttctttttaattggttggttgattttaatctatctagttgttattgatcagactttgtaagatcagctgcccgtccgtattacccagggccaggcttgtagccctttccgggtgaggcatcataccaaaaacatttcttgctttgttacagatgcctgctatgttacggatggcgccgttatggttagcagtttcaataatgttgccaaactcatcgcagtagcggaataacacctggttgttcttaaacagctcatccagggtagcgtcgtcggcatagtaacggccttctccgtgtgcgatcgggatcattaatggtctgccggctacatctttggtgagggatgcagtggtattttcgcttttcaggtatacatttttgcagatgaactgctggtgctggttctgtaataatacgcccggcagaagacctgcttcacataatacctggaaaccgttgcaaacaccaatgacacggccacctttgttggcaaattcaatcacactctgcatcatagggctaaatttcgcaatagcgccgcaacgcaggtagtcgccaaaggaaaagccgcccggtaatacgatacaatcttctgtgctgaatgcgctcaggtctttatccttatgccacagttctataacttcctgtcccaggtcattacgcagggaatcaatcatatcatgatcacaattagaaccgggaaaggtgacaacgccaaatttcatctgaaaatgttttgtgtttatgtgtaaataatgcttttaaaaaacgtttttttccacatttttgccaccatttatacgaatgacaaaactaatgggaaaggacaaaattacttcgccgttcgcaattttccattgccgtttgtcctgatttaacaaattactggtaatcaggcccttaaaatgggggaatcagctgaaatattgcataacaatcacatatgccagtgcaaagaagtggataatgttggcaaaagtgtcgttggtaaccgaccagaatacgttaccggcgaacatggaaatcggcaaaactgccagtacccagtaggctgctgaaaagtgaacattaaagaacggtatcatcatggctaccagtacatatatgatgagtgccgcccatattttacggccctgtatcagcatttttttaagcgggcgctgcaacagcagccatcctatcacgaaaaagagcaaacaggcgatcatggcgccccaaaccttataatcggtgatcatgggcaacgaggcgcccatattcgggattttccaaagaagggtcatctgaccggtgaggaacaggtaggtgcccatcaggtataacggacaaatcaggcccagcagggcaatgatccattccgccagccggaaagcccgcataatcagcatgctggacagcaacaaagaacagaatataacagaaggaaaataaaagagcccgcttatccccagtgcaaacccgatattaaacactacatcacgggcggaggtacgtgtatacaactccgttatactggtaaatacccacaacatgatgaggtttacgatcagtgccggagaaaatacgttccagctttgcagcatggacgtaaacagcaggtaacacatggccggcaggtaagtaggccgcggaaataaccggtgatgattaatgatacgggtgaaaagcagggattgcagaaacaacagtaaaactgccatcgacgtaaacaccagcgggctgccgcctgtaaacgtatgcatccatttcaccagcaggtgatacaaaagcccttctgatccgtctgccatataggtagatgggtggatcagatagtaaaacttaacaaccagcgtgtatattaacaacagcaataccgttagcggattgcctgagcggaaaaatcttatcacagtgcaaaggtgtgattaaaagtcaattttagcaaagcaaatataattcctgtaaatgcatggtatcactaccgtacggccactgatttgtttgccataccggggcatccaggtgaaacccttatccaggttacgcagcgtaggcatgcggttcactttacctcccggggccagacttacatccgtcaacatataattccttctgtccagttcattatacagaaaacgtaattcgctgcccacgtttaccatcaggtaagacaggtacaggtcggcgttatcgtcatactggctcttatgaacaaagttattccactgcatattgccctcatcgtcgaaagacaataccgctacgttatcatagtgataacgcaatccctgtgaattattccagtagtagggattgtagtacatggaagagtaaggcgagtagtaatagggggcgtacatgccgccgtaaggactgccgtacatataattccaccggttccagggctggtagcgggaagaggtggagaaagattctgccgtaaggaggaatccaccgttactggtattgatgatcttacggatgaagtagtcgttaaaggccgcggcggtgctggattccccacgggcgttcattttcaggtcatcggggaatacctgcgatttctcatacaccgttttatgattggcgtagtcgtacttgtacagatacaagccatctacatttccccttttctgtttataataaaaagcggtgaccagagccgtttgcttattattatcaagcttcattttcacttcatccagcagctgtgctttgaaggccattacagaggtttcaaagctgtcgaccagcgaacgtttcacgaccatactgccgctcaccacatagtcgcggttggacgtgcgttccagcttattaaagagcaggtcgccggtattggtaagattaaagttgctgaggaactgtttcttttgcatgggcatggataaacggctgttgttcaccaggctcatggcactgtcgtacaggaaggtatagaatacgttgttgttttcgttatcctggttgatcttatacaccatgatgcggttcttatcttccgatacttcaacagaatatactttgttctctttggagtagataccgatgcgggtggagtcgatcaggatgggtgcatctgcaaatttagcttccggcgacatggtggcgcagaaactgtataccgcatccttgcgctggaattggtagatcatcagcactttatccggataggccacaaaatccatactgatcaccttacggggcaggaagtccagtttaaccctttctttcagctgcatcgcattgtcatatacagacaccacatagtcgccgcggtctgttttatacaccagtatattccctgctaccttgccaataatttcaaactcggtgcttttatagtcgtccttctccggttcagaataggttattttctgtgccgttgctgctgtgccggcgaaaagcagcaacaataataactgtaggcggtatagcgtatgcatgcggttatatagatttcagatatttttgtgataatgcagatggcccatttgcatgtgccattttcaaacttacattaaaattcagaaattaacttgtcaatttaaagccggtaagtcctgcttttacataaattccaaaaggcccgatttattgtgtatttttaataaattattttaaaaaagcagctattattggatggaaaccgttattataaccggtggaacaggacttatagggacggcattaacccggctgctgctggagcgcggctataaggtgattattctcagcaggcgtcctgataaacgcagcaacacgaatgtaacatatgcccactggaacgtggaatcccaaaccatagataaagaagttattcaacaggcggattatatcgtacacctggcgggcgccaacgtgggagagaaacgttggacagcagcgcgtaaacaggaaatcattgacagccgtacccaaagcagtgaattaattttcactgcacttaaaaacttccccaacaaggtaaagaaggtgatcagcgcttcggcaacaggttattatggcgactttacagaccacatcttcaccgaaacagaccctcctgctaccgactacctggccaccaccacccatacctgggaacaaagcatttccaaagtaactacacttgataaaaagctggtgattttccggaccggcattgtgctcagccccgatggcggcgctttaaaggaattctacaaaccattgcggtttggatttgccaccatacttggatctggcgaacaatttgttccctggatacatattcacgacattgtacggttgtacttcaatgctattgtgaacgaccggctggaaggcgtttacaatgcagtggcgcccaatcctgttaccaaccgtgaactgatactcagtatggcccggatggccaaaggacgcagctttatgactacctatgtacctgcttttgccctgaaactggcattgggggaaatgagtgtggaagtattgaaaagcgtgaaagcgtctgccgacaaaatacaacgaaccggtttccagtattcttatcctaccattaacgatgcaatggagcagctgtttagccgataacggttttctccatagcagcagctttcagtaagcattcttcccattctttttccggatcactgtaaaaagtgatggcagatccggtctgaaaagagaggtagcggttatctgcgttgtacagtatgctgcggatcaccacattaaagtcgaaatcacctgccggcgtaatatatcctatggctccggagtaaagtccccggcgggtttgctcatattgttcaatcagttgcatcacccttaattttggcgcgcctgtcatggatcccatcgggaaagcattccgcaatacttccgtgaagggcgtttcgggagataattgtgcggagacggtagaaatcatgtgatgcacatgggcaaaggaatagatgccaaacagttctgttacttccacggtgccctgcaaggcagtatgggataaatcgttgcgaacaagatctactaccattacattttctgcacgttctttcgcactgttcagcaggtcctgttgcagctggcggtctgttaccgggtctgcatctttccggctggtgcctttaatcggctgggagataacggtgttgcctttcttttgcacaaaccgttccgggctggaacaggcgaggtaacggtgatgcaggcgataatatgcggcaaaaggcgatggcgacaaggcattgagccgggtaaataaagccggtggatgtatgctgatattttccatgaagttttcgcggcagaaattaacttcataacaatcgccctgcaggatgtgttgttgcaggtttttcactgcagcaatatagcgttggtgatccaggcggctttgcagcggctgcaccagggaagtaactacgggtgatgtatccggcggcgtgcgcaaaacggctgtaaggacttcctgcgcgtcttccctggtaaaggcttctccaccgatatgcacctggtttttttgcagttgtatgatgatgcggggcacaaaaaagtgcatatccggaaaaccgataccatcgtagtggtgtgaatgcagacctgccgtttcgtttttgagatcataggcaaggtgcccgaagagccagccggcgtgtgtttgatggaattgctgtaaagcggggaatgcgttgccggcgtttacttcgagggtatgcagtgcatctgcagcgagtatggcttcatattgatgccagggagaatcgtaattattattgtctaaaaaacaacaaatgttgaactggtttccccaatccaacatttgttgcttaaatattttctgattatcaaccggaaaagtgtgaaatatcctgataacaatcgtgtttagtgcttaaaaatcatcatcgtcatcatcaaaacgatcgttgaacagatccatgtctttgaattcatcatcgatacccagatcgtcgtcatcatcggcttttttgctgccagtgctgggacggccgcgtttacctttcgacttaggcatgtcaaactcctcaaaatcaggatcataatcatcatcttctcctttctcccacgcatcatctacatcatcctcctcatctgcgtcgtcttcttcctcatcatcatctttacgttttgatttggatgcagacttatctgatttctttgaggcagatttggaaggtttcacatcttcatcctcctcctcctcatcatcatcatccacctctttcttaggcttggccgcagctttgggagcttcttttgcagtcttaggagaagtagtttttttggtctctttctctttatcagattttgatttcataataggttaccttatttctttgccgtaaagttttaatagttttttttattcgccaaattttttttgctgttttttttccttactttttggttctacttttcaaggatctgatcgcgcccaggtccgttggaaacgtatttcacgggaacgcccagatacgtgtctactgctgtaacaaatgctttcatctccgctggtaactcgttgaactgctgacaggtagaagttttatcactccatcctttaaatgtttcccagactggtttaatgtccagaccgttaatctggaaaggcagttgctttgtttgttttccgtcaatttcataagcggtgcaggcgagtacctcgtcgaattcgtcgagcacgtcgctttttgtcattaccagttgggtaacgccgctcagcatacaggtataattcagcgctaccaggtcgatccagccgcaacggcgtggacggccggttaccgcaccaaattcatggcctgcagaacgcagtttctcgccggttgcatcatgcagttcggtagggaaaggaccgctaccaacgcgggtgcaataggctttggtaacaccaatcacttctctgatccactgtggagcaatacctaaaccggtacatacgccggcagaaatggtattggaagaagtaacaaaaggataagtaccaaaatccacgtccagcatacttccctgggcgccttcagccaatacttttttaccggctttcagtttctcattcaggaaatattcgccgcttaccacattcatttgctgcaggaaagggatggcttcgaagaattcagcttcccagttggcaatatcttctgaaaattcatttatatcgtactgacataacagctgcaggtgtttctgcttcagtttttcgtacagtgttttaaaatcgggggataaaacatcacctacgcgtaaaccatttctgccggttttatccatgtaagcagggccgataccttttaaagtagaacctattttatcatttcctttcgctatttcagacgccttgtccagcgcgcggtgtgtaggaacaatgatatgggttttttcagcaataaacagattttttgtcagatctactcccagggctgaaatatcttcgctttcttttttgaaagctacagggtccagcaccacgccgttaccgatcaggttgatggtcttatcatgaaatacaccggatggaatggtgcgcaatactactttctgaccgtttacatacaaagtgtgaccagcatttggtccaccctggaaacgggcaatcacgtcgtacctgccggcaaaatagtccacaatcttacccttgccttcgtcgccccattgcaggcctaacaaaacgtctaccataatgatttaattaaatatcggaggtttgttgctttaaaagaagtcgcaaaattaaggcgaatattaagaattacaaacaaattactaattacacaccggaattgcggataaaagggaagatttcatcaagatcttctgaaatcttcccttttacccgcccttctttatttgctgtttgtattttttactttaagattcttcgaggcgctggatagattgtattccatcgagcgttttaagcctgtccacgagctcgtccagttcttccttatcgtgaacatatactttgatcaaaccctcaaataagccttcttttgactcaatgctgagggcggagatattaatcttcagttcaccggaaataatgttggtgattttgtggatcacccctacatcatccatcccgataatgcgcaagcctgtcaggaaggaaatttcacggttcttcacccatttggtttttaccacgcggtggccataattagccagcagctgtgcggcattggggcagttggtacggtgtatcttcaacccctcgctggcagtgataaaaccaaatacgtcatctcccgggatcgggcggcagcagttcgccagtttgtaggcgattttatccgagctttcaccgaaaatgatcagttctgcatcctttttggaaggcagctggtgttttacatgttcttccggtacgtgttccggtactttcaccggttttgggggttccagtttatcgcccagtacagaaaactgcttgagttctttcagatcaatgttgcggaccgccacctggtaatataaatccagcggggacggttgtttatagaactgtaccagttcattgatattatgctgactgaaagaaatattcatgtgcgacagcttacgctccagtgctgcctttccgtccatcgccactttccgcttttcttccttcagcgcatccttgatcttggatttggctttggcggtgagcacaaagttcagccagtcttccgaaggcttctgtttattggaggtaatgatttccacctggtctccgctgcgcagtttatggctcaggggcaccagtttgtaattcactttggcgccgatacatttgttacccacggcactatggatagagtatgcaaagtcaagcgcagtggagtttaccggcaatattttcagatcccctttgggggtatacacataaatttcttctgtgaacaggttactcttaaaatccgcgaggaagtcgagcgtattggaatcggggttgttcaggatttcccggatctgggtgaaccactgatcaaatttagattcctgctgggcggaggcattgctgccttccttgtaccgccagtgtgcggccacccctttttccgcatagtcgttcatgcgtttggagcggatctgcacttccacccatttaccactgggacccattacggttacgtgcaacgcctcgtacccattggatttagggttgctgagccagtcgcgggttctttccgggcttgggtggtaaaagtcggtaataatggaatacaccttccagcaatctgccttttccttatctatcgcggaatccaggatgatacggatggcaaaaaggtcatatacttcttcaaaggcaacgccttttgttttgatcttattatggatggaatgaatggatttcgggcggccataaatctcgaattcaaatccttcatcctgcagcacctctttgattggcttgataaactcgttgatatagcgggtgcgttcgcgtttggtttctttgagacgcttggctatttcacggtaggtttgctgctccgtgtatttcatggccaggtcttccatttcggatttaatattgtataacccgagacggtgggccagcggcgcataaatgaacacggtttcagaagctattttcagttgcttttcgcggctcatgctgtcgagcgtacgcatattgtgcagcctgtctgccagcttgatcaggatcaccctggggtcatctgccagcgtcagtaatattttcttgaagttttctgcctgtgcggtgctggtactggagtctattacggtagatatttttgtgagaccatctacaatgtgagcgatctcattcccgaactcgcgggacacatcttccagtgttacttcggtatcttccacggtatcgtggagcagggcacatatggcggagcgtacgccaaggcctatttcttccacgcagatctgcgctacggccagcggatgcaagatataaggttccccggatttacgccgcatttccttgtgtgcatctgctgccatttcaaaagcagtacgtaccagctccctgtcgccttttttcaaacggggcttcaacgccctcaataaagcacggtaatgccgaacgatttccttcttttcctgctcttcgtctaaattatatttttgtacaaccactgtttccattgcaataaagttacgatttaatataatctgaaagaaaaaacagggtgctgcaaaaaaacacccaccctttgccgggataaaccggaaagggcgggcaggttgattatcaggcgggaaaaaaatgctatcagtgaagaggcacggtgatctttaccggcaggatgtcttccggcacattcaggcggagcccaacgttgtaaacggtttccagctctatgcgcggcaccagccggagcagcctgcgtacgcggccgataaatacgtccatactgcgactggcataaaaatcttcttttccccaaacccgcagcaatacttcatccttttggacgatgatattgggccggctgaggaaataacgcagcatttttgcctcgatgggagaaattttgcctttggccagtttgctgctggtttcgaagatcttgagtttccggtaatggaaggtgtaattcgccactgtgtgccctaccagcaactctgttctgttgggacgggtccacttcagcatcaccttcattctttttaccagttcctcaaagctgaatggctttacgaggtaaccatcccctcccagctggaatccgctgatgcggtcagcttcgtccgtcttttctcctgtcaggaaaaagatcggcgtcagcatggtcacattccggatttccttcgccagttcaaatccgctcattttcggaagaacgatgtcgataagacagatatcatatttggaccttgagtaaaggttccaggcatctacgccgtcgaagcaatgttccacactgtagccggcctgctccaggtgctgtttgacgataccgccgaatgccttgtcatcgtcaacaagcaagacttttggatttctgttcatatagctaccatttgtgatcagttcgactataaaacaaaaaagagatgtccgcgggtaagcgtccatctcttttttttatttatcaacactaattcacattaattcacactacaatcacagcttttccacagccggtattttgatagctatagcatgctgaaatcctttatcacggatagatgcagggatctgcacttccactcctgctgccgtagttttccacaccagcttattattggcccccagcacctgtaaacgggcgcctttaaccggcgttaatcctttaaatgaaattactgcgggcagtttctcattttgatccaggagatagatcgcatatacgctgccgtcttttttacgggtgaaacacactttcccgtccttgtaaggcgccaccgcacgggtgccgtaaatagcgtccccgttgatatggatccactcgccaatatgcttcatggtagtataagcatcgttatgcagctcgccatcagggccaggcgccacattcagcaggtagttaccgcctttggctacaatgtccaccaggttgtggatcagtacattcacggacttatatttatcgtccggcacataagaccaggagctgcccatggtcatgcaggtttcccagggatagctgagcggcttgtcggggatctgctgttcaggggtccggtaattttcgtacgggccatgcacactgcgatccactacaatcaggccgggctgatggctgcgggccatggtggcaattttgcccatgtctatatcctggtcctgcggagcagtttggctccaggaaagcgattccttggtttgctgcttcagcgggcgcacccagccgccatctaaccagaggatatccagtttaccataaccggtcatcagttcttcaatctggttataggtgtattgcttgaactggttccatctttccgggtatttcttcagatcataattcggattgcggtcctttggcgggaagtagctccaccagtagtattcggtgtgccagtcgggcttggaaaagtaagcccctgcgtgaataccttcctcacggaaagcctggaatacttccttcgccaggttggcgcgggggttcttgctaaaagcgccgtccgcagcggttattttataatcggtttgtttggtatcaaacatacagaagccatcgtggtgcttggtggtaaacaccagatacttcatccctgcgtccttcgcggctttcgcccatttttcggggttgaagtgaacggggttaaaggttttccctaatgcctcgtactttttcaggtaatcgtaataaggaatacctgccggcttacgctgtgtccagccttcatcttccgggcaaatgctccaggattccaccacgccccattgggaataaggtccccagtgcatgatcatcccaaatttccagtcctgccactcatccagcttcttcaccaccgcctggtctgtttcaggtacataaggcggttcttcattctgtgcgtgcagactattaaagcccagcaacgcaaatcccaataaaaccaggtatttctttttcattgtcagtttttataagacgatactaaagtagttactttcaaagcctggtggataagttcgggcagttgtcctgtccgcaaccggatggtccgggtttctcccggcaacaaatcaaagtaattatcttcaaaatgatcggttgcagtggcattgtcaagcgacaggtaaacatttcttgccagcttatccgttttcaggcggatataaacaacgccgttatctttggccaccttgctggttaccacatccaggtgcggcacttccaggttcatatctttcgctggagcaaagtaaaagatattccgctccatatccttactgtctattcgcagttgcgcatagaatattacccttgccgggttatttccctgtaaaatagcggcggtatctatgctgtgcagtttttcgctggtatttccttttacagcgatatccgttaattccttttgccagatcaccttgccattcaggtccacggccttcatcaataaatcagctttgccttcgtattcgtctgttacgaggtaggtacacagctgtccgttttcaatgacgctggataccagtcgcggcttgaacgcatcttttacataatactgcaatgctttccagcggccatcgtaatccctgcccgaccaggaagctcccggccagcaatcgttcagctgccagtacagggtgcccatgcaataaggcatagccctgcgatgggcttctatggctactttcataccttctgcctgtaatacctggctgaggtaaacaaaggagggaaagtctttcggctcgcggtagtaatgcagcatatatgttttgatcgccgtatttcctttcgcaggacttttctggtgggcctgcattacattggagaagatatcgtaatcttctttcgcagcaaacgtgcggatcgtttccatagatgggaaggactggaaaccatattcactcatgaagcgtggtatatgtgtattgaatgcttcaaaccattccatgccatgccatacgccccagtagtgattgtctcctttggtaaaatcttccggcttgccccagttgctgatgggcgaagaatggaaataaaaagcgcccggctgataagccgctacctgttgtggcagcacttctttaaacagtttatcatacccctgctgcaaactttcccactgcgtattcgtataggcgtaaccgctttgccagccccagtttttaatagctacggccacctcgttattgccgcaccatagcgccagcgaaggatgattgcgcaaacgtttaatattatcggctgcttcctgctttacattgtccaggaacgcctgatcggaaggataaagggtacaggcaaacataaagtcctgccacaccagtatcccgtgctgatctgccagtttataaaaattatcatcttcataaatacctccaccccatacgcgcaccatattgaagttggagcttaccatatcctggaacagcttttcctgtttttccttggttacacgcggcagaaaattatcctggggaatatagttggcgcctttcataaacaccgggcggccgtttacttttacataaaacggctccccgaggctgtctggtttattcactacttcgatggtacgtagccccaccctggcgctttgcgcagccagtacttttttattgctgagcagatttgcctgcaactcgtaaaggaacggtgtgcctataccggcaggccaccacagcaccggtttgggtatggagaaaggtacttttattacgtttatccccgcctgcaggcttaccggcaattttgccagttcgcgcatagctttccctggcagcacctgcaaggtataatcgcctgcggcagcggcttcaatggttatttccgcctgcatgtctgccttcgcggaatccagctgcagctgttgccagtacacatcgcggatcactgctttattccagctccgcaatacaattgggcggtagatcccggaggtaaccagccgtggtccccagtcccagccatagtgatacggcgctttacgtgcataaatacttaacggcatatcgctggcatcattaccagcgggatagatgatgctgtcctgcaaaaatttgggcatgtctgttttgatgggacttttaaacaggatgcgcaattcgttgtcgcccgctaccagccattctttcacagttaccgtatgcgaaacaaacatgttggccgattgcaaaattaaatggttattgagatatacatctgcataggtatccaaacctttaaactccagttctatcacctctgcattcagctcctgctttttgatatgccatcttttccggtattgccagtttttcttatctacccactgcacggccttttcattggttcccacaaaagggtcggggattaaatgctgtgccagcaaatcggtgtgaaccgtgccgggtacggtagccggccgccagatgccttcatcggcgcgggaaaattcccaaccggtgagcatagggttattttgtgctattccattggtaaacagggtaaaaaacagtcccactgttaacagtaaatatttcatgtcctattttttcagaagaaccaaaaatagcactgatttacgatctttgggagatgaaaagtatctggcaacaaatattgaggtatctgtatataggcaagaaggatcccaatgcaccaaaaacacgttacgtggctatgatgcatgggatgaacagaatttcactgttactttttatcatcgctattattatcatggtgatcaagctgatcaggcggcactaagcgatagcgtattcgtagatcacttctgcagcgcggcgggaagcatccttttctcccagcttatgccacaattctgcatagtctttcatgacgcggcttctggcagcttcatcattcaacagcgcatttaattcctttaacaggttttcttctgtgaggtcgtgctgaattaattcttttaccaccagtttgtccatcaccaggtttaccagggagatatattttactttgatgaggtgtttggcgaagaagtacgaaataggatttcctttatagcatactacttccggcacgccgaacaaagctgtttccagcgtggcagttccggaagttaccagtgcggcttttgcctggcgcaataacttataggtttgtccttttaccatggacacgttgggatgctgaccggtgagactttccaggaaatggtcgtccaggcttggcgcctgtgccactacaaactggtattgcggaaagtgctttgccatggtgagcataatcggcagctttacgctgacttcctgtttacggctgcccggcaatacggcgatcacgggtttatctgataacggcgcatctgcgggttgttccctggcagctttgattacttccaccagcggatgccctacgtattccgttacataattccatttattgtaaaagtcaggttcaaacgggaggatgcacagcattttatctacatactgcctgagtttttttaccctgttttctttccaggcccatacctgcggggaaatataatacactattttaaatccctgttgtttgccccattcggcgatgcgcatgttaaacccgggataatctaccagtaccagcacatctggtttaaaggcagcgatatcttttttacacagttctatattctttaaaatggtgcgcaggttcatcaccacttccacaaaacccatgaaggccagttctttgtaatgctttaccacatgggcgccggcggcttccatcaggtcgcctccccagctacgtatatccgctgacgtatctaattgccgtaattgttttacaagattgctgccatgcaaatcacctgacgcttctcctgcaataatgtaatatttcaatattcttcgattaaaaattatctgatcagtttgagtaacaatatgccgatagcatacagcatggtcatcaggaaaatacctttggctgtaatatccagccgttttcttgtatacaggaaaaacaccagtccgtttaataacaggcagatgctggtgagcttcggaatcatctgtttattatctttcagaataccgagaaactgtcccagtcccacgttattatgcggtttgatgacaaaaaagtaatacaggaaaaacgcaagcaggggtgttaaaaaccccagtaaaatccctaacggaagattgtctttttttaacatactgtaattatgatggcgatataacgaatgtttacaggtctttccaatcttcttccagcttctttttcaatgaatagttcgtcaggtcaaactgcactggtaccatagaggcgtaattattttccagtgcccacacatctgtatcctgtccggtatcgcggtttttaaattctcctgtcagccagtaatattttttaccgtgcgggtcgcggcgttcatcaaattcttccacccattttgcgtctgcctgccggctgatcttcagtcctttgaaatccttttcactcactatcgggatgttcacattgaacagggtgcccggtggcagatcggattccagcattcttttggtgacactgtgcgctacttttttgggcagcgaaaaatcagcatcatagctgtattccaggaacgagaagcctacggaaggaatgccttcaatggccgcttccattgcggcagacattgtaccggaataaattacgttgatagagtgattggcgccgtggttgatgccgctcacgcagatgtccggtttgccatgcaggattttgtcgcgggccagctttacacagtcgaccggcgtgccggagcactgccatgcctctattccttcaaagatatccaccttttccaaacgcaaaggaacgccgatggtaatggcgtgtcctttacccgactgcggactatccggcgctaccaccaccactttgcccaaaggtttcactgcttctatcagcgcccggatgcccggcgccgtgatgccgtcatcgtttgttaccagtataacccgctcttgttttgccataattcaccttttttctttgctcaacaaatttaagctctctgccaaacatttcgctttaaaagaatgtgaaatatatggatatttctacagatcggattttaatattttcctgaaaaccaggtagatgcccaatgcgatataggctatcatggcggttacatacacgtacgcttcgtactgatcgccggtggataccattttgcccaccagtggaaacggcagcagctcgtcgccgctctggagcggcagcaggccgccaacggggccggcatttcttttaacaataaaagacaacagctgatccagcatcatattatacgccacaaaaagcacaatggccagccccgcccgtttcaccaacacgctgatcagcagggcgatggtcagcatcacattaaattgcaggaagtaatacagcatgtaatggtatccatccaggctgaagggcttgttgccataaatgattcccaccagggcgccgctgatagtagccaccactagtgtgagtagggaaatagccaccagccagaataactttgcgtatacaaactggcttctttcccagccgtcgattacgttctggcggttggtgcgatacgtatattcattggttaccagaatgatcaggagcagtccgaataatgcggagatatagctgttgagcgaagccatggttaaccacacttcagggaagctgaagggattgccaagcattttgcttatctgttccaggtttccgctgagtttgtcggctaccatgaaattgccggcggggataatcaccagtgccagcagcagcattacccaaaaggtgcggtagttccttactttgagccattcggtatagatgatctgtttcatgatgcggcgatgttagtgatttccaggaatgcagtttcgagacttttcttgcggagttgcaggtggctgagccagatgccctgttgggcgcagtagctgttgatggctgcggcatcgggggattcagcgaaagaagccctgacaatgttgccctgtatgatggcgccggtgcaaccggggaacctgagcatggtggcctgcagctgcgcgttatctgctgccgccagttccacgaagtcgttccggctgatgacggtgtttaccggtcctgacagcaataacttcccgcttctcaaaatagccacgtgtgtgcatactttttccacttcatcgagcaggtggctggcgaggataatggttttaccgctatctgccagtttacgcaccagttcgcgcacttccgcgataccggagggatcgaggccgttggtgggttcatccaggatgagtacatcggggtcaccgagtaaaacagcggcaatggccagccgttgtttcataccgagtgaatacgttttaaaggccgagtgctggcggagtgtaagaccgcagatctccagtaccctggcaatatcgtctttcccgcgctgtttgatagcagcggagatttccaggtttttatacgcgctgagatagtgatagaagttgggcgtttccagcaacgttcctatttgccggcgttctgcggcggaaggcgctttatcaaaaagggtgaagctgccggtatctgctttgagcacatcagtaacaatgcccagcagggttgttttgccgctgccgtttgggcccagtacgccgaacacgctaccagccggcacatcgaaggatacaccggacaatgcctgcaccgttccgtatcgtttggaaatgttttgtaaggatagaattggcacgggagtaagtctaaaagatgaaaataaaaagggaaatgcagcgaatgatcttatggctaatcttcactacatttcccatacattaaaataacagtttctaatttcgtacgggtttgcccgttttaatcacgctttgtaagcgttccagcgttttgcgttcaccgcataaactcaggaaggcttccctttcgagatccagcaggtattgttcgcttacaaaagaggcttctgtaagatcgccgccgcacatcacataagcgagtttatttgcaactttctgatcatgttctgaaatataattaccaaacttcatggcgtatacacctgccagtaaggctcccagagcgccgcggcccattactttgatgtctgttctttccacggggcgggtatagccttcgtcggccagtgcaattacgctgcgtttggcatcggcaataaggcggctgaggttcatggtaatttcatcgtgtcctttctttagcacgcccatatcaaatccttcaaagccggaggtggctactttagcggtggctacggtcatgaagtaatccttcaggggttcttcctcgatgcggccttccttgtattccaggctggcgcggagcgccatttctttggtacctccgccgccggggatgaggcctacgcccagttccaccaggccgatatacgtttcggctgccgcctgtactttatcggcgtgcaggcacatttcgcagccaccacctaaggtgagggcatgtggggccaccactacgggtaccgatgaatagcgcaggcgcatggtgctgcgctggaagaggcgcactgccatgtccagctcatcaaactcctgttctgctgcgagcatgaagatcatgcccacgttggcgccggcagagaaattggtgccttcgttgcctactaccaatccgcggaaatccttttcggcgcggtctatggccttattcaatccttccagcacttccccgccaatggtattcatttttgttttccagtcgaaacaaaccacgccatcgccaatatcaatcaggttgcaggcgctgtttttccagactacattattggagaagttttccaggataatgaattgtccttctcccggtaatggtttgtaggtttgggtagctacgtcgtaatataatttcttgccgttgtctactttgtagaagctggtgattcctttcgccagcatatcttttacccattgggcaacggtgagtcctttttcttcgatgagttttacggatgcttccacgccgagcaggtcccaggtttcgaaggggccgatttcccaaccaaagccggctttcatggcgtcgtctactttatacaggtcgtccgctatttcgggaatgcggtgcgacacgtaggagaacaggaatgcgtggaactgtttatagaagtcgccggccttgtcggaagctcctgccagcgctttgatgcgttgtttcaggtcttcgatgggtttggctgcgtcgatactggaaaacttagctctttgctttggtccgtattccattgactggaggttcagcgtaaggatttccttgctgccgccgtctccttttgttttcttgtagaaaccctgccctgttttatcgcccagccagttgttttccactactttctggaggaagggaggtattttaaagatgccgatggcttcatcctgcgggcagttttccataacgcctttggctactctcaccagggtgtctatccctaccacatcggcggtacggaaggtagctgatttagggcggccgatgaccgggccggtgagtgcatcaatttcgtctatcccgaggcccatttcctgcatgatgtgaaatatggccatgatagagaacacgcctaccctgttggcaataaatgccggggtatctttacatagtacggttgttttgccgaggaaaagatcgccgtagtgcatgagaaaatctatgacagcgggatcggtatgtggtgttggaattatttcgagtaaacggagatagcggggcgggttaaagaagtgggtaccgcagaagtgtttctgaaaatcttcgctgcggccttctgtcatgaggtggatcgggatgccggaggtgttggaggtgatgagggtaccaggtttccggaactgctccacctgggtaaacacgcttttcttcacatccaggttttccacaactacttcaatgatccagtcaacatccgcgaggcgtttcatatcatcggtgaagttgcctgttttaatgcgtttgatcacatctttggtaaaaacgggcgacgggttggattttatggcggcctgcagggcatcattcacaatccggttcttcacagcgggactatccagtggcagattctttttcttttctgcctcgttcagttcctttggcgctatgtccagcagtaaaacctgtacgcctattcctgcaaaatggcaggcaatccttgatcccattaccccagagcctaaaacggctactttgttgatgtgtctcattgctttggcttttggctgtcagcttttattcattacgcggagcttccagcatttgtaacttaaatttaccgatccttgaatttagcattttttggagttccatcatcagggggcacccgatttctgtaaaatttgcggatcggagcgtagtttgtctttctcaggattaaacttattacactgattgcgctgatttgatcacttttgattttaaaagattcagggagatataagcgaaagtatccggttaggggatttgacctcttttgattttaaaagattcagggagacataagcgaaagtatccggttaggggatttgacctcctttgattttaaaagattcagggagacataagcgaaagtatccggttaggggatttgacctcttttgattttaaaagattcagggagacataagcggatattttcgcttatatctccctgaatcttttaaaatcaaaagtgatcaaatcagcgcaatcagtgtaataagtttaatcctgagaaagacaaactacgctccgatccgcaaattataccggctttatgaaggcttcgccattacttcgtattcgctttgcacctgctttacacccggagtatccgtgcagtgtacacggaggggacgtggaggtgacgtggacttgatctggaaacaagccactctgccgggtttcagcttactccgctgcccggctttacaccttcggcggggtttacgaaaatcagcttgccattgtcttccgccatcaggatcatgccctggctttcaattccgcgcattttgcggggggccaggttggctaccagggttacctgtttgcctacaatgtcttccgggttgaagtgcatagcgataccggaaacgacggtacgttgttcggtacctatgtctaccagcaatttcagtaatttatcggctttggctactttttctgcctgcaaaatggttcctacgcgcaagtccagtttagcgaaatcgtcgtattgaatttcgggctttgccggggcgggaggcgcttcttccacggcgggcgcagctgcagcggcggcatccatggcctgttttaaacctgcatggagtttttccacctgagcggttacctggtcgttttccacctgcttgaataacagttccggcggacgcagggtatagcccacactcagcagtttgtcgctgccggcgttgtcccattccagcatacggtccaccactttcagcatgtggcagatctttttcgcggtaaacggcaggaacggctgggagaatatcgccaggttggccgtcatctgcaatgcgatgtgcaggcaaatgtcgatgcgaccctgtaaaaatgcgatgtccttttcttcgtactgcgggtatttggcgtgttgttctccattcttcaacttttcaagtacgcttgccagtatccagggttcatttttctggaggtattgattgcctttccgggcaaattcaatcacttcagacagtgcttcccggaagcggtatgtttcgatgctggtttcaatcttctcttttgccaggccgaactctttcagcatttcggtatcgccgtcgttcatgaactcaggatgcagtgaaggtacttttccaccgcacagtttatgcatcagcaccattgcgcggttaacaaagttaccgaaaacggccaccagctcgctgttattacgatcctggaaatccttccaggtgaagtcgttgtcttttgtttccggcgcggtagcacaaagtacataacggagtacatcctgctgatcggggaaatcttcgatatagtcgtttacccacacggcccagttacgggaggtggatactttttccccttcaatattcaggaactcgttggcgggtacattgtccggcagtacaaatccgccgtgcgccttcagcatggccgggaagatgatacagtggaaaacgatgttgtccttaccgatgaagtgcaccagtttggtatcgtctttacaccagtagtccgcccagttttcggtcagctcctttgtagcggagatataaccgatgggggcgtcgaaccatacgtacaatactttaccttccgcatccggcaggggtactttgatgccccagttgctgtcgcgggtcatggcgcggctttgcaggccactatccaaccagcttttacactgaccgtatacgttgttcttccactctttatgaccatcaatgatatattctttcagccacggttcgtagttctgcaaaggcatataccagtgcttggttttctttttcaccagcggtgcattgctcagcgcagaatgtgggttgatcagttcatccgggctcagggttctgccacagcgctcgcattggtcgccataggctttatcgttaccacaattaggacaggttccgataatgtacctgtctgccaggaacatttctttctccggatcaaaaaactgttcgctttctttttcttcaaacaagccgtcgttgtacatcttcaggaaaaaatcctgggaggtctggtgatgtatgggagcgctggtacgggcaaaaatatcgaaagagattcccattgcagcaaagctgtcgcctataattttatggtatttatctaccacatcctgcggactcacgccttccttcattgctttgatggtgatgggaacaccgtgttcatctgtgccgcaaacaaactttacatctgccttttttgcacgtaaataacgcacataaatatctgcaggcaggtagcagccggcgaggtgtccgatgtgcaccgggccattggcatacggtaatgccgcagttattaaatatctattaaattttgccatattctcttaaagaatgcttaaataaactttaaatcagtgattgtttttggaatcaccataacaatttatcaccttagtcagcgaataaagaatgaatttacgctaactaatctgcaaaggtaaacaaaaggaacaatggtaaaaattccgccatatttgaaaaaaggtgatctgatcggaattacctgccccagtagcaaaatggatctgcaggcagcggagtatgcacgtggcgtactcatttcctggggttaccgtgtacacctcggtatcacggtaggaaccagcttccataacttctccgcgccggatgaactacggctggaagagttacaggatatgctgaacgatccggaaataaaagcgattatatttggccgtggtggctatggaatggtgtgtatcatagataaactggatttcacccgtttccggaagcagcccaaatggctttgcggttacagtgatattaccacgctgcatgcgcatgtgcagcggcattttggaattgccacgctgcattccgtaatgtgcagcggtattacccccgatacatttgataatgaatatacagaaagcctggcaacagcgctgagagggaaagcctaccgctactccgcaccagcgcatccaatgaacaaggaaggcaaaaccaccgggatactggtaggcggcaatttatctatcctggccaacctttccggcacttcgtcacaaatcaacaccaaaggaaagatcctgctgctggaagatatcggtgaataccggtataacatcgaccgtatgatgtataaccttaaacgtgccggttggctcgacaacctcgccggactggtagtaggcgcctttacggatggcaaagaaacagatacgcctttcggccagtcggagtatgaaattatcagcaacctggtgaaagactacgacttccccgtttgctttggtttcccgagcggacaccagacagccaactactcgctcaaacttggtgtgaagcacgagttgaagattggcgccaaaaccgtgcttgcggaggtgtagcagatggatcggcgcggattttgtctttctcaggattacgctgattatactgattagtttgatttttacttttggatttataaaggattaagggagatagaagcggataattcgctcttatctcccttaattattaattatttaaaatctaaaaatccaaaaaaatccaaaagtaaaaatcaaactaatcagtataatcagcgtaatcctgagaaagacaaaatccgcactaatcctccacgtctggcacgatctccagaccgtattcttctgcggtgaggacaccggcagcgcgggtgctttctatcagtgcggtatccggttgcaggtcgtgaacctgggtttgattgtggaggtagtcgatgccatagaatttgccggcgatgcccaggggaacaccgatcaggtatttcactacttcgcaaacgatttgggtgccgagggcgccgtgggtagcgccaagggcgccagcatcgaagttgcggtagccttccgtgagcggtaatgcacaacggtaggatgctgaagtggtgccgtccggcatgggcatattaaagccggcgaaccaggccatccagttatgtacttctccggtgatataaggtttgttgtgtaccaggcaggcatcgttgatcaccaggtgggtgggcaggtgctgggtacaatctatcacgaggtcgaatcctaccagcatcaggttgatgctgtcgggttttacctgcatgaggatggggtaatgttttgtatatgggttgactgcccaaaggcggctggcagccatttttgctttgtgtttgcggatgtcctgcatctggtagatgggctggcggtgcatgtcttcatcattgatcacgccatagtcggcaatgccgattacgcctactccgctggcgctgaggtattgtactaccgggcttccgaggccgccggcgcctactaccagtacgcgggcttccttgagcttctcctgcatggtgatgcccatgcccggcacggcaataggatttttgaaatgttgtatttctttttcgctgagtatcatatgctttatcctttatccagttcctgtggaaattctagggtaaacttgctgcctttacctactacgctttccactttaatttttcctttatgtgcgtctacaatggcctttacatacgtgagtcctaggccgaagccttttacgttatgtacgttgccggtatgtgcgcggtagaacttttcaaagatacgtgaaatagtgtcgcggctcataccgataccgttgtctgcaatcacgatgaagaggcttttgcgggtattgtaagtttgtattcttatctccagctgatcattggaatatttgatggcattatccatcaggttgaagatgaggttggagaagtgaacatcatccgccatgataatggggttgatggcatccagctgaagatccaccacaccatttttggtggccagctgcaactggaggttatcggcggtactttgaataacgttgtgcacatcagtcggctggagtttcagcgttatttcatctttctcaaggagggcggattgcaggatgctttccacctgtttgttcatacgtttattttcttctttgatgatgccggagaaatactggattttttccggttttgacattactttctcattcctgatagcatcgatggccagcgaaatagtggccagtggtgttttcagttcatgggtcatgttattgatgaaatccgattttatttccgagagttttttctgattgagcagggtgcggatggtaagtgcaaatgcggtgatgatgatcatggtaaacaggacacctcctgatatcatgatacctaattgtttggctaccgaatcatcgttgggcatgatgatgtaaagcttttctgcccgtggattaaaatcattggattccgacaggaggatcacctgtacgcggtagtctttcttctctttaatgctgtcggcttcattttgctggaacatcttttcaaacccggccgactgcatccggatggtaccgaattccgatccgggaacagtgccgatgatggcaaattcgaagctggaactatcgaggtgatttttcctcatattgttctggatgcaacgtttcacttcctgcacagtaaagaagtcgctcacggagggaacgctgtattggggtacccggttaatgtcgagattaaatcctttggtagcggctccttctttgttatcgagcttaaacataatggcagcctggcggcggtacatcatatcgttataaacgtccctggacatactgacagcgcgctgaaagagctggtcctgtttgatatgcacggcactgatgatccagctgacctggatataaatgattccaagcagggacaaagtgatcaggataacgatgacggggaaaatcttcttcagtggtatcatgtaagtttttgtcaggctttaattatctcaaagataagtgcgaagaaatactaaaatatgttaaaaaagatgtttgctatagcaactatgatacaaaattccagacgggatattgcctctgtacttattctccgcaatacaacatcactttaacgtaattttaactgggtactgctgtttttattaatgcttctttccttacctttgcttcagaatcttggtactaaatttgattagttcaggatcataacaaagtaattaaactttctacatacatcgatgtggattcgttccataagcgatttagattttggttgataaaatggtaaggaggttttctagcctcctttttttatttttcctactttcctctcatttttctttttactttactattcaatgatttagttaaatttgaacaggctataaaattgtttgtctatggtaactttgtcgcccggcattttgctgatagctgatccatttttaaaagatccaaattttgcgcgcacggtagtacttctttgtgaataccaggaaaaaggcagttttggctttgtaatcaataagttgtttgatcaaacgcttagtgatcttgtgcccgaggtattgataggcaatgtcccggtgtactatggtggtccggtacagatggataccattcactttgtgcaccggcatccggagctgatcagcggggggcaggagatattgcctggtgttttctggggtggcaggtttgaccaggtagtggctgccatcaataagggtttgctggagccggacaaggttaaattctttattggctattccggctggacagagggtcagctggacgaagaggtaaaggagaaatcctggatcttatctgacaccgacacttcactgatatttgagcgcagggagcagcaaatatggcagcaatcccttaaaaatcttggcagtacctttgccatgatggcaaattatccaattgatccttccttaaattaatggtaatattctgagacagaaggagatgggctgtgcccggtatttaaagtgaaaaatgaacaggatgaatgctgtttatttaaaacaaattaaatatcttgctaaagtaattggggaatcaaaccagctacatagcccgttttcaggtaatttaataaccgataagatacacctatgaaggcaaaacctatgaacattttgctccttctatagaccgataccagcatttacctgatcactaactgattattgtcaaaggcattcattaggtaatataaacagccttgatgaggctgtctattgatgtacatgtagttactgcggatatctcgtatagccgtgcaggtaatgtattgtacataatgaataggaggaaatcccggtggacagtcctgtccttaaccgggtcatctaagattggaatagttaggacaaaacgaaggccgggtattcttacccggcctggttattatattttagctggtatgctttatttttccactgctacagcgccttctacgagtacggtagccttattgcgcaacacttccacaaatccgccgctgatggtatagaactctgcatgagctttatctttcagcactttcattttaccatttccgagggctgcaattaatggcgcatgtttatccagtatttcaaaagaaccgtcaatgcccggcagttgtactccgtacacttctccggcatatatttttctttcaggtgttaatacttctaatagcatgttatgatcgtaaatggtgaagggtaatgatcccggcggaaccgggatcattgacttaattagttattcgctgcttccagtaatttcttacctttttcaatagctgcttcgatgttacctaccaggttgaaggctgcttcaggatactcatctacttcaccgtccatgatcatgttaaagccacggatagtttcttcgattggtaccagtacgcctttcagaccggtgaactgttctgctacgtggaatggctgggacaggaaacgttgtacacggcgtgcacgggatactgtcagcttatcttcgtcgctcaattcatccagaccgaggatggcgatgatatcctggagttctttatagcgttgcaggatcattttcacgcgctgtgcacagttatagtgagcttcacccacgatagacggagacaggatacgggaagtagagtccagcgggctcacagccgggtagataccgagatcggagatcttacgatccaatacggtggtagcatccaggtgggagaaggttgttgccggagccggatccgttaagtcatccgcaggtacgtaaacggcctgtacggaagtgatggaaccatttttagtggaggtgatacgttcctgcatcagacccatttcagtagccagtgttggctggtaacccacggcagaaggcatacggcctaacagcgcggatacttcagaacctgcctgggtgaaacggaagatgttatctacgaagaacaggatgtctttaccaccacctgcagtgccatctccatcacggaaatattctgccagtgttaaaccagacaaggccacacgcgcacgtgctccgggaggttcgttcatctgaccaaacacaaacgtagcctgtgattgtttcagtaattctttatctacagcggtaacatcccagtcaccgtgttccattgattctttaaacttgtcaccgtatttaacgatgtttgcttcgatcatttcacgcatcagatcgttcccttcacgggtacgttcaccaacaccggcgaatacggataaaccttcgtaaccttttgcgatattattgatcagttcctggatcaatacagttttacccacaccggcaccaccgaacaaaccgattttaccaccttttgcatagggttcgatcaggtcaattactttaataccagtgaacagtacttctgtttcggtagccagatcttcaaatttaggcggctcacggtgaatagggtaaccgtttgaagcatcgatatcacctagaccgtcaatcgcctcacctaccacattgaacaaacgtcctttcacctggtcgccaaccggcattttaataggcgcgcctttatcaactacagccatgccacgaaccataccgtcggtggagtccattgccactgtacgaacactgtcttcacccaggtgctgctgtacttccaatactaccttctgaccattttcgcgggtaatttccaatgcgctgtagatttcgggcaatttgtcatcaaagtgcacgtccaccacgggaccgataatttgtttgatcttacctgtgttaggcatatttttaaagaggtttataaaaatactaaaatgttactgttccaaaaaccgcacacaattgcatgtatacagtttccaaaatttgccgcaaaggtaagagttaatgggtgaaaatcaaaacgctaacgatgaaaaaaaaccttttcccaccgcatttttcgccgattttatcattaataaagttttataccccggcaatgcaaagcggagcctgtcaaattatatattttcattattcataaataacgtgaagctacaggcgccattcatataaaaatagcttccttttcttaattcctttactatttttaatcgctatcctgatatatacaatatataaatatgatgaagtcaaacagtgaacaatcccgcaggtcattcctcggcaacctttccaaagcaggattactgggcgtcaccggcattgtaccggccgccgccaaagctggcatcttgtcagcaacatccaccacgacagctgctgaacacgcttttctctgcaaaccgtacctccagtatcctggtccacataccatttcagtgatgtggctcaccagccgcccctgctacagctgggtggaatacggaacagacgggcagctggataaaaaagcccaccgcgttacaaacggactggtagacgccaacaaccgcctccaccgcatagaactggaccagctggaaccgggaaaaaagtatagctataaggtatgctcaaaagacattgtttcctttgaaccgtataagctgacctatggcgaaaccatagaaagcgccacctacaccttcaccgctcctgatccgaaggcgaaagaagtgtcctgggtgatcattaacgatatccacgaccggccggcttccatcccacacctgatgaaactgaacggcaaggatccttatgatttcgtattttttaacggggatgtatttgactaccaggccgatgagcaacagatcattgatcatatgctcactccctgcggtgataccttctccacacaaaccccgttcatgtatgtaaggggaaaccacgaaacccgtggcaaatatgcccgggaatggcaccagtattttgacaacccgggccacaacaactatttcacctttaatatagggccggtatcggctattgtgctggatacaggagaagataaagaagatgagcatcctgtatacgcgggcatcgttgacttcgacgcctaccgggaacagcaggcccgctggttggagcagcaactgcaaagtccggccttccggaaagcgaaacataaagtagtgatgatgcacattccgcactaccactccggcgagtggcatggcgtaaaacattgccgcgaaatgtttggcgatctctttaacaaacacaaaattgatatcctcatttgcggccatacccacaaatacggcgtgtatgccccggcaaaaggagagcatgaatacccgcttatcattggcggcgggccaaaagaaggtaatcgtaccctgataaagataaaagccgatcagcagcaactggtattaaccatgctgagagacgacggcaccaaagtgggtgagtacaccgtgtaagtacaaaagaagctgtctcataattaattgagacagcttctttgttttagccaaaagatggcctaataatcattatgatgatcaggtgttttttaagagaataaatagttaatgtcagcttgctttagcaa

SEQ ID NO: 2 - DNA, 1040048 bp, Chitinophaga pinensis
  source 1..1040048: mol_type = genomic DNA
actaacggattgataatcattctcaactgccatcacaatggctaatttttgctcaaaactgtattttctgcgtttatccataaaaatgccccctaaaagtgtctaacttttagggggcagtacatatatccgcttctatctcccttaatcctttataaaatcaaaagtaaaaaatcaaagtaatcagtataatcagcgtaatcctgagccaagacaaaatccgcaccggaggcgattacaccgctgctttataacgtttctccacctcatcccagtttacggcattccagaaagcgtcgatgtattccgggcgtttgttctgatgtttcaggtagtaggcgtgttcccatacgtcgagcgccaggatgggggtgcccttatctttcacaatattatgcatcagcggattgtcctggttaggtgtattgatgacagccagtttcttatccggggttacgatgagccatgcccagccggagccgaaaacagtttttgcggcatcattgaattttgtctggaatgcttcccagctgccgaaagcgctggtgatggctgatttcagcttatcagaaggcgtcttttttgtgggagacaataatgtccagaagagggagtgattataatgtccgccaccgttattgcgaatggctttatctttgtccgtcactttgttcatgatttcttcgagcgacagtgttgcaaacgctgtaccggcgaggttatcattcaggttcttcacataggcagcgtggtgcttatcgtggtgaatttccatagtgagcttgtcgatatgaggctcaagggcgtcatatgcgtaaggcaacgcaggtagaacaaagggggctttaggatcggcaaaggccggctggccggatacagaagaagtagccaggctgctcaatggcccactcaggatggcggcgccggcaagactggtaagcttgagaaattctctcttatccatgttttattatttaaatatattattgagtaataaagatcgagtcaggccgggaatgccgcaaatattaaaccaaatctcgttggtggagagagatgaaaactaatattaaaactaaggtaaaagtataaaaacgatgatttaatatcaaaataaagggaaacttttactttgttttcatattaaattactattttaccttacattcatatcatttttgtaatgaaaagttgcaattaattgtgtgattgccagatatatttatcccgggcctggcaggcaaacaaaggaacctgttcattaacccgccaatgcgccaacgtaataaccgatcagatataattaatattttaagcgaatactaaagagcaacaggaattgctttacacacgataatttagcgtcattcagtgcaagcaatcctggtccaacctcgataaagcaggaaacatgatacaagagtacctcaggaaacaacaggataagagcaatgactacaagcctgttttttatgatttgaagcgcgcacaagaccttcagtccttcgagacccttctggaaacccatccgcacctacgcatcaacgaccatatcgactctcagttaaaggagctgatgaaaatcaggaatcctaccaaacgcttgactgcagaggaatacgaggaaaaagtacaggcacatcttggtggtgtttcccccgaaaaatatggcgtgtgggtatactatccctggaatgaccagctggtgcacctggtaaatgaagcggagtttattgagttacgtaccagcaggaaccagcataaaattactgcggaagaaattgcggtattgtcaaaaaagaagatcggcattgtcggcttatccgttgggcaatcgatcgcattaacgctggtcatggagcgtatctgtggcgaactgcggctggcggacttcgaccggctggagctgaccaacatgaacaggatccgttgtggtgtgcacaatatacagttgccgaaagtggtgatagccgcccgtgaaattgcggagctggatccgtttattaaagtgagcatttaccaggatggcatgacagaagccaatatggatgacttctttaccggcggtggtgtgctggatatttttgtggaggaatgtgatggcgttgatattaagatattaagcagaataaaggcgaaagcgctgaagataccggttgttatggaaatgaacgacaggggcatgatagatattgagcggtttgatcttgaaccagaccggccgcttatgcacggtttgataccggaggtgaatattgataccttaaagggtttaacggatgccgagaagctgcccatcttcagtcccatgctggcgctggacaaagcatctgacaggatgaaattctccctgggtgagattggtaaaactattaccacatggccccagctggcctcttcagttgtactgggaggagccctggttgccgacacctgccgtcgtatcgccctggatcagttaaagagttcaggcaggtattacatagattttgagcagttgattgtttaacatacttatgccttgtataagcgctattccgcaatgtcatgattaatgtaagggtatttagggctccggatgatcctgaggcttgcatgagattttataccggtcacctcaagttgctggaaatttattttggtattgcccaggtaacatccggcagcgctgactggatgcaacatgaaaatacaatagtgatcatagtggaggacgatactcgtaccaaaacatatggtggggcacgtgtgcagattgctgacggcgtgttaccactgcccattgaaacggcgataggcaaatacgatccgaaaatatattcatatgtaaaaaaaggcagtgcggagatctgtggaatgtggaattccaaagaagtggccgggatgggaatcggcagccaggtattggcaagagtaggtgttgtattgggcgcacagttaccgatagacacctatcacgtgttatgcgcacccatcaccacccgggtagggaaacgtgtaggttttgttatagatgaatcactggggaataacggtacgttcttttatccgaaagacgacttcctggccaccgctatggtgatcaacgattgctacgagctgccacatgccgatcccaaggagaaattactgatttcagatctgcgtgaaaatccaatgcaatctaaaattgaagtaggcccaaagggttcctacgaggtaaactacagcctccggatccctacacacgcccactttaccccttaaaacaattaatcggggccggtatttctgaaaaaaacatataaattcaagcctgatactaatctattttcgtgatgctgtccaagattgttggtttatggtcaatctttaccctgttagtcctgtttcatgtaacggcacaacctgttgtgtttaaaaacagcaaatcgctgttacagataggtggttatcttgagctatacactgataaggcagacacgctcactattgcctcggctcccatgcaggcattcaaggcttccgggcaggacgtaccaaacctgcagatcacgccatatacccaatgggcaaggttttccatcaataaccagtcgaaagcggagaagctgctgctggaggtggaatatcctattatagatgacatcacgctatacgaactgttgccggatggcactatcaggcaaacccggctgggggagtttactgcttacaaaaaccggggatacgaccaccagaattatcatttccctatacggctgctaccgaatgaaacccgccagttctatctgaaagtaaaggcaggagaacagctacagctgccgatttacctgggcaccccggaaagcatctttgaaaagaacaacaaacgggagctgatttttggtatatacgtgggcgttatcctggccatggctttttataatctctttatttacatatctacccgtgacaacagctatctcatctacgtgagttatattatatgcgtagggcttacccaggtaacgctgcagggttattccttccgtttcctgtatcccaacagtccatggctggctatgcacgccacggtgctggtgccggtgttcaacgggcttacggcgctggtgtttatccagcagttcctgtctaccaaggtaaactacccgctgggacataagctgatgaatgccgtgattgtactgtacatgctttgctttatacctaccttcctggatatgtataattatgcgcagatacttgtgcagctggatgctttcctcgccgcggtgatggcctttgttgttgcctaccgtatcagtatgaagggagtgaacgcggcccgtttcttcctgttggcatggtcaatattcctcatcagtattttcgtttttgtactgcgcaatttcaatatcctgccgtataacaactttacctactatgcgctgcagattggttccggcgtggaagtactgctgctgtcgtttgcactggcccataagatcaatgtgttcaaggcggaaaaagaagcatcgcagcagatggccctggctatttcccaggaaaatgaaagactggtaagggaacaaaacatcatactggaaagtaaagtaaaggacagaactgaagacctgcaggctaccaacctggaactgaacatggccttaactaacctgaaagatgcacaaacccggctggtggaaaaagagaaaatggcatcgcttggtcagctgacggccggtatcgcgcatgaaatcaataacccgatcaactttgttacatccaatatcaaaccgttgaaactggatatcgctgatctgagggagctgttaaaccgctatgatgaattacctgtgagcacagatatatccaaatcgctggcggatattgccctgttcaagaaagaaattgatattgactacatccacgaagaaatttcctcgcttatcaagggtatagaagacggcgcttcacgcaccgccgaaattgtgaaggggttacgtactttcagccggctcgatgaaagcgaggtaaaatccattgacatccacgagggactggactccacgctggtactgcttcgtaatgccataccgccttatgtgaacatcataaaggattatgcaggcttgccgaagattgaatgttacgccggtaaaataaaccaggtgttcatgaacattttcagcaatgcgctgaatgctatcaaaagcaagaaggagcaacacaatgaattcatctccattaccaccaggcaggagaacagcttcattgttattaccattaaagataccggtattggcatgtcggaagcggtgcgggaaaagatctttgatccgtttttcaccaccaaagatgtgggggaaggtaccgggctggggttatctatcgtattcagtatcattgagaagcataaagggaagattgttgtgaactcggcgccgggtgaaggagcggaatttattatatatttacctcttagtatcgcaaatcatttatcctaataaccataaggcccttcaatgaaagaaaaccgcataagaatattatacatagatgatgagattcataacctgaacgcgtttaaagcaagctttcgcagaagttatgaaatctacaccgctacttctgcgcaggaaggcaaactgctgctgaaggagatcatggtgcatattatcatcgccgatcagaaaatgccagtagctacgggtgtggaattcttcaatgaaataaaggatatcttgcctgacccgatgcgcattttgctgaccggttatacggatgtggaagatattattgatgccattaacaagggccacatctactcctatatcaagaagccctgggatgagcatgagctgcacaaaaccattaacaatgcctacgaaatataccgcacacgaaagcaactccgggaaaagatagaagagctggaaaaaacgaatgatgaactcaaccggtttatttattccacttcccatgatttgcgttcaccattgatgtctgtgctgggaattatcaatctgtcgaggctggataattctgtggtagatcccaatggttatataaacatggtagaaacctgtgtgttaaagctggacgatttcatccagaagatcattgagtactaccgtaattcccgcctggagatagaatatgagagaattgacttcaataccctgctgaacgattgcatcactgcgtttaaaccgcagaatacccagatccgctttcaaaccaatgtggaccaggccgttgatttcaggggggataccttcaggatcagtgttattttgaacaatcttatttcaaatgctgttaaataccagaagccggaggaaacaaacccgatggttaacctggcggttaaagtagagccacacaaagcaactatctgtatacgtgataatgggatcggcattttaagcgagcatctgaacaatattttcaagatgtttttccggtccaagaacaataataaaccgggcagtggtattggcttgtatattgtaaaggaagcattgagtaaaataggcggtaccattaatgtggagtccaaatatggcgagggcacccaatttgaaattaccatccccaacagaaatgaattcgatacctgacctgcgagtcatattgattgatgacaatgaaattgatttgttgctgcatgagaagttgatcggatttcaacaaatcagcagaacggtgatttcgtttgcaaatgccaataaggcactggaattcctgtcttccaatattgccttgcctaaaattccgcccactgttatcctgctggatatccagatgccggaaatggatggctttgaatttctccaggcatttgattcttaccccagtaagattaagtcccaatgtcatatcgtaatggtgtcttcttcccttgattatggggatattacccgtaccaacgcgaatcccatggtaattaaattactccggaaacccttgctgttaaaagatctcaaagaaaccgtggaaggaattttcaaagattttttataaaatgttggtgtttacaggaaaaaatatatttttgcatcccgaagaaagcaataaacgggggattagctcatctggtagagcgcaagcatggcatgtttgaggtgaacggttcgagcccgttatcctccacccgtaaagcctgacacaatgtgtcgggctttttttatggctgtagccggcgatcaggccagtacatcagttaagccagctgccacaggcctggtttgtttcaggggtaatacaatgatgaaggtagcgccctctccttccctgctcctggcggtgataactccgccgtgtttatcaatcacttttttggcaatagccagcccgatgccggtgccctcatagagttccgaagtgtggaggcgctggaagatggtaaatattttagaaagatatttttcattgaacccgattccattatcgcggataataatgcggcagtaatgcccgccttcaaagctggcactgtcggggtttagatccgttacaacatctgcggtaatatgtatctgaggaggtatatctttccgtgaaaacttcaacgcgttgctgatgatgttttgaaacacctggcgtatttgccccggcacagcttcaatctgaggcattttctccacagtaataaccgcatcccgttcaacgatcatcagctccaggtcgaccaggatctcctggatgattttattgaaatcggtaacttcgtttatgcttgacccggataaacgggaatagttcaacaggtcgttgatgagccttgccattcgttctgaggagcctacaatcctttccatataggaaagggcgttagggtccgtgtgtagaaacttatctcttaaaatagcgccgaaaagctgaattttccgcaggggttctttcaggtcatgggaagcgacggatgcaaactgttgcagatcgtggttgctggcttccagcgatttattaatctctctcagttcttctgtcctttcccttactttctgttccagcatatcatttacctgttgttgatgtgctatcagtgcttcctgtgcgagttttcttacctctacttcttctttgagcgactgatgcatttgcttcagttcctgcgattgctgataaaggcgggagaatgtctttactttcatcaggaggatatccgggtccaccggcttggtgatatagtcgataccgccggagtcatatccttttacaataaaccgtttgtctttattcacggcagacaggaatataatcggaatgtccttcgctttactgtgccccgacagtgcttccgccacttcaaagccgtccatgctgggcatttgcacatccaggatgatgagcgtgtagctgtgtttgagtattttcttcagggcttcttccccggatagcgcggtatccacttcgaactggtatagttcgagggttttcctgatagacagtatattttccggcttatcatctacaattaagatcatacgacatactcgttataacagatgggcaacgggtggaaagcggcccaatgttattcttttaaacttttaaacaatgacagctcaataatcatacctctgccattcggtttatgaaggcagccatttcctgtggctgcagtatagcgtcaacgggcgcctggaggatggcttgccttggcatgtaatccacatctgctgtagccgggtcctgcacggcggtggtgcctcctgcctcgtgtacatctttcagtccttcggtgccatctgtgttggcgccggaaagcagtatggcggtcattttactgccataggccagcgccgcggaagtaaaggtaacgtcaatacttggtcggctgaaattcactttctccgaatcatccagggaaaaagtatgatccgattctatcagtaaatggtaatctgccggcgcgatgtagatggtggccggtagcaggggttctttttcaccagcttctctgaccggcaggatggatttaccagacaataactccgttaataccgactcataatggctttggcggtgcaatacaattaaaatggctgcaggaagtgaagcaacaagtcctggtaacaatgtcaggataggttgcaatcccccggcagaaccgcctattacaattaaatacggtgctgtagtcatatgcctcttattttgttattacagctgcaccttccgccagatcttctcccggttttccagttgtttaaatttaccggtcacgctggtaaagttaagtgtttccttacttcccagtgccaggaagcccagctgctccaaactgtcactgaataacgttaataccctgtcctgtagttttttattaaagtagatcaatacattgcggcaaatgatcaactggaattcattaaatgagccatctgttaccaggttatgcggggaaaaaatgatcttttccccgaggtcttcccggaacttggcatattcataattggccgtataataggaagagaaatcttcccggccaccggcctccatatagttgcgggaatactgctgcatttgtgaaagccggaacattcctttgcgtcccttttccaatacgcctgcattgatatcggtagcatagatcactgccttgtgcagcagtttcgcttctttgagcaggatggcaaaggaatatacctcctccccggtggagcagccggcatgccatacccggatagacggataggtggccagcaccggcaatacctgggtacgcaatgcctggtagaaagaagggtccctgaacatctccgttacatttaccgttatttcttccacaaaacgtaatgcgtatgccggatcggaaataatacggtagcggtattcggcaaaactgggaaagcggtctacctggtacagatggtttacccgccggttaatagaggcgggcgcatactctgtgaaatcatacccatacctttccagtatgtcattcagtaacagcaacacttcctgttcacttatcgggttcctgctcacgtttgctcagataaatattgttgtagctgcaacagtagctcatctacatcaattggtttggaaatataattatcggcgcctgcttccaggcatttttcacgatcgcctaccatcgcttttgcagtaacggcgatcagcggcaggcggctgttccagggcatggcgcggatggcggaaatcgtttcatagccatccatatccggcatcatgatatccatcaacacagcgccgattgcatgctccggcgataatacccgtaatgcttccgcaccggtgccaacagccacgcatgggatattcctggatcgcaatactgcctttaacgcaaagatattgcgtgcatcatcatctacaattaatacctgtttctgttccataaaagttatttcatggctttatcgtataaccatacccgtaataaggatagcaactgatctatatccactggtttggaaatataatcagaggcccccgcctgcaggcatttttcccggtcgcccatcatcgctttggcggtaacggcaatcactggcaaacctttgagtcccggttgtttgcggatagccgcaatggcatcatagccgtccatttccggcatcatcatgtccatcagcactacgtctaccgggtgctctttcagctgctgcagcgcttcgttaccgtcgatagcagacagtactttcatctggtgtttttccagtgcttttgttaaagagaaaatattgcgtacatcatcatctgctaccaacacggttttatctttcagcacttcattcaatacgcccatcttcccacttccaccctgtgcagctggcgcgttttcagataccaggtgcaggaacagggatacttcgtccagcatacgctgataggaatgcgccgtttttaccacgatggaatcagcatactgccggatccgttgttcttctgcctttgataaacttttaccggtaaaaatgataataggaagattttccagtccctttatttctttcaccatttccagcgcctgataagcccgctggtcaggaattcccatatcaaggattacgcagtccacatcttgctgttgcagcagcgatacgccatcttccacggtattgctgatttcagaacttacgtggtagttactgaggaaataggccagcgctttggcgtgcttcgcattttcttccaggatcagtacttttttggtagatcgttgcaatacaaactccatcttttcaaagatcagttgcatgctttgcacgtctaccggcttgctgataaagtcgaccgcacctttcaggaggctttctttttttgcttccatggaagacatgatatgtaccggtatcggcctggtggccggatcacttttcagttcttccattacctgccagccgtcttttatgggcagctggatatccagcaggatacccagcggtttgtagatgcgtgccagttctgcggcttcatcaccgcgtacagatacaattcctttatatcctcttgcatgggtaaagtctagcaacgccttcgcaaaatgcgtatcgtcttccacgatgagtattacggaatcgccgttttcaatgaggccacggtcgtcgtaaacgtcttccggaacggtgggcgacaggtatctctgtttcggaccggcggctgtttcttccactaccggtgacggcagtacgaaaggttggcttacgggtgctcccgttttacgaaccaccgggatcgtaatgacgaattcacttccctcattgttggtactgctcaccgaaatatgtccgccgagcagcttggccagttcccggctgatagacagccccaggccggtgccgccgtatttcctccgggtagatccatcagcctgctggaaagcttcaaaaatcacctgttgcttttccgccggtataccgatgccggtatcttttactgcaaagcggatggtttcgggtgtttctccttccagtatttccatgcggacaaatcccctcgcggtaaatttcagggcattggacaacaggtttttgaggatctgttccagtctcaactgatctgtttcaatactggccggcaccgcagcgtctttatgtatcaacagctgcaatcctttttctttagccattggttcaaacaacgcctgcatattggaactgatatcggcaatggatacctggctgaattccagttccattttgccggattctattttcgagaggtcgagtatttcgtctatcagcgtgagcagcccttttccggagctattgatcacctgtgcatattcgatctggtcgccgttaagattggtgtcgtgattttcagagaggagccttgataacaataagatagaattcagcggtgtgcgcagttcatgcgacatattagccaggaactctgatttgtagcgggtgctgagtgccagctcttctgctttcttatggatatccaggttccgttccacgatgatctggtttttttcttcgaggaggcggcttctttcttccagttcagcgttcgactgcatcagttcttcctgttgtactttcagttcttcttcagacacctggagcttttgtgtttgggcttccagttctacgttcaggctttcgagttcggtgtgttgtgtttgcaattcttctgcctgcgcctgcgtttcctccagcagttcctgcaggcgggtgcggctccgggtactttgcagggcaatggcgattttcacagcagcctgctgggcaaagtcgatcacattttctttaaaagggaacagggaacctagttctactacgccctccgtaacacctgcatggatcagcgggataatgagcacgtgaccaggttgtgcggaggctgcagcgccggcgatatgcaggaaatcatccggcgcttcgcggagatataatggttccttttgtaacacgctttgcccgagtaaggttttccctacttcaaccacccggggggccggatgggccggcgacagcgcatattcagcggataaacgaagttcaccggagtaccggatatacagcacccctgtttgtgcgccgatgtattgtatcacatccgttaaggcatctttactcagtgcctccatgtccttttcaccgagcaacgtttcgctgaggcggttaatacctgtttgtatccatattttctggtcggcatgatagcggaatgttttcaggtctgcggccatttgtactattgcatggccgagtatatcattttcgctgcggggttttacatcaatattaaagttgcccttaccgatactgtcggccgcagtagccagttcctggttagtttggtcaataacagtaaaagaacgccccaggcttccgatagcatcttttgtgtgtacttcgggcgccgatcccggtacgcctttcgcgatatttacagccgctgcccgcagcagttccaggctgtcggtgatgcctttaatagtaaaggaaataaataccaccaccaacacgatgatacctaccaatacaagcaggtagcgggttttcagatcattttcttttttagagataatttttgcatccctgcctactttatccattacggcgcgctgcaacagcttcagctgatctacggccagggtagaattgtcccaccaggagtctgcattaaacagggtatcaattttacgggaggcgatggtgcttttaataaaatcgtttgtgataaccatttcattggaggattccgttttaagataatcctttgacacggcgggagaagctttgtctaccagctctgcacgcagggctgcaaacatgtcggcgttattttctatgcgggcaaaatcttccggccacacttcttttttcagcatgaaatagtaaatatccatacggatcattccctggtaagctgccatctgtgccagcaggtattgcgcgttcatatcctgctgaacggcttttaataccgggatatccggggtgttggtattggccaggtcgttcaggcggaaaataaggttggaataatagtccagtacctcccgttgcggcatgcttttactatcaatatcttttctctttttggggagtgtatttagcagtgagtattggaagaaacggctgtcgctggccagcaacctgcctttcaccgcatcgatggccagatcagttttggcgcgttgggtgagcaggtcattcaggcttccggtttgcagtacatagtttacgctgttcctgcgttccatatgaatttcatcggccactttcatgatagtggtggcagtcgtaattttctgcaccaggttatcaatagtatctatatcttcagtctgtttattgaatacggctataccaaaatatacgagacacaccagcggtattacagcaactaacatcagcttcctgggaagagggagctgcataaagtatttcttcatttgcctgagcttgtttaatttttacaggggcactattctgcaaactgtgctttcaacgggttttaacacatttcgttccaaacagtaccactaaaacgaataatatgataataaaataacaacaaaatcttagatttgtctctattccaaaacgatatatgcccgatagttgtaaatatacctcagtacttttaattgacgatgatatagatgacagaatgatatttggtgaagtattaaaggagctggcaccggatattatttaccatgaagctattaacggagaagacgcactacttaagctgaataataacctggcgccggatcttatcttcctggacctaaatatgcccagggtagacgggaaacagtttcttgcagaaatacggcagcaggagcatttaaaacatatccctgtagttatctattccacgtcttcacatgaatcggataaaaaagaaacccgcgaactgggggcctcttattttctgacgaaacctaacagtcttcatgagctgacacatatactgggtcatcttctacaacaaaagttattttaatgaaaaagcctcacaaagaattgtgaggcagcttttctaccattgttactatttttaaacccttatatgctcacgcatatgcttatacctcaaaggtgggttttaaattatgttcaagtgttaaccggatcttaacgactcctgcattaaaattgtttcactacttcttcgagccatcctgccgaatggaaatttactttcaccgctggctgaatgcctttattgtcaataccctgccctgcagcaatcctgcgggagcgggtaacgggatagtctattgaaaaatcaggcgctgaaaaccttaccctggctatattagagtaatccagcgcccctgccgtgggagctcccatgagcttcactttctgactttgtaccgcttccagtaaaaactgttctgcggtattgctgcaccggccattaatgagcaccgctacttttgccggggctggcaaaggagccggcaggatcatgttttcatccggccccatacttaccagccggccttgcaaaccactaccctgttcaattacagtgcggatctgctctacatattcgccgggtagttttccggtttgttcgtccagggtatggcgccatgcagcaatgttatccggtgtagcataaaagtcggccccggtaatccttacaggttgggtatacagcaagggccgcaggcgttcaatcagtttatcagcgcccgcaccgttgttgcgtacatcaatgaccaggttggggtttctccgcagatactcgtcgctggcattcagcacagaatcggcggccggataggacgccgcgtcaaagctgcttatacgcagatagccggtgctgtcgtttatttgccggaaaaagaaaggcgccgtcatatcggcgaaggcgggtatttccgccggtgtattgtcactcttcttcacgcccgtgaattgctgcggcgatgccgcagcgggtttctgccaacccaatgcagacaggccatcgcgttgttttccgatggtgagggtatcaaagttcacttcctgcgcggcgtagctgatcatatcaaatttatccggcccggtagcggccagttcaaacaatacgtctccgggtttccaatccggcgaggctgattccatgattacgccggcgtaagtgcgcaatccccgcaggttctttaccagggccactttatagagggagtcggcctggtaaataccagccacaccgcttacgggctgtttctgcagcaaatccagctgctgtggggtgagggtgattttttctctgaggggcgtgtagccaatgtgcagggcgagatgctggtctttgaagaagcgcaggtagcggtttaccagcaggagacaatgcgtggcgcccttgatggtagccgcctgtaaccgtagttttgccagcatggcagtataagcctgctccgtaaccggggttactttgtcgataaaccctgcataattcttcctcagatagacctgtacgctgtcaaatttcttcctgcaatcgcactcctgcgcgtttacaactgtattacacaggagtaataacaatactgctattgctttcatggcaaaggatttgaatgtttctggctgataataaatggtctttaaatatatatattcgggaggacactaccagaaaatatttatcatcctccaccaatattaataaattacatgtcctaataaagcgcatatgcattttgacgaactggaaaggctgtataatgaacaggcatatactgaagcaattaccaaactggaaatatacctgcaggataaccccggcgaggcccggggctggcaactactgggcttatcccagctggaaaacgccaaggccactgataaccgcgacctggccaccgctatgtacaacgaggcttacgaggcattcagccaggtgctgaccattgaccccgcacatgtgcaggcccgtgtacaccgcgcctatatgggcgccaatgtgatggcagacaaaggagatgaaacgatcggcgattgtgatatcctcattgccggcggcgatgaagaactgactaccaaagcattactgtaccgtttccaggtatgggtgctgaaaaatgaaaccgaaaaggccctggcagatatgcaccgcaacctccaggtatatgaatcactgtacgccgacgatctgccacagctgaatgtggcgcggttccagtgttttacccgtatcggcgatgtatattatcacacggaaaacaggcccgccgccctggaatattacaaacaggcctttgaatgtacggtgtttaacaaccgcctgctctctaccacctggttcgcactggatatggcggattatgattttgcagccagcatgctgcagatcatgatcacggcaggagaaaatacacaggaagacatgctgcgtttgctccggcatatccagcaactgcttgcggatggcgtgcggaatgccgcgctggcaagggagttctgcaaaggcactaccgaattctggcagcagttttttggagatgatgatgacgaaggtaccctggaacagatttccaccggcaaacactttattgctgagtaccccgacgaagcctacttctatcattataccgctacggcgttcttcaacattggcagttaccaggaggcattgccctggtatgaaaagtcgatggccataaaaccttatccgttcagcatggtgaggtggtattttacgagctataaagtgaacgggcaattccccgaaagctggccggatgtggagcatcacattccgtacgactggtacgcagcgggtgttatcttcagtgaaattattcaactggaaaaagacaacggcgtaaaacaggcgtccaccgcgctgaagcgcttcctgtataaaaaagcatttgatatctatcatgcctactggtatgaaaattcaggtaactcttatgcaggccatcctcatcattttgccatgtgctgtaacaactatggcattgccttgtatgaaggcggcatttttgtggaagcagcgcatgtacacaccatcggttacaatatgtcgcccttctgggaacagctggaatccagggctgatgcgtatcacagcatgggtaagctggccgaggccatcgccgaccgccataccatcctggaaaatttcacagaagtattgccgctgatgtactatgtgtctatccatgaacgaatgatcgacgacctgtgtacgttagagaaacatgccgaagcattggatctctatgaaaaaatactggcggaatacaatacctggattgcaaaggatatgcaggaactggatgactacgaccgggaaaccattacgtataacattgaccgtattaaaaccggccgcgcatttatccgtaccaacagcgccgatgatttatctgaacgcatactggcgctggaaacgcacctggtggaaaaaccggatgacagtgacgcctatttcaacctgatgtacctgtattttgataatgcccagtacgaacattgtattggcgctatcaacaaccgcatttccattggcggcatcaccaaactgccggtgatttcgcaaatgaagatctattacttccgtggaaaggctgcgttaaagcttggccgctacaaagccgcgattactgatctgctgcatacgctgcagattatgtctaacggcgacgctgcagacaatgcccccaactaccggtttggggtatacgcttttcttgcagaggcatatttgggagagaaagaatatgacgagtgcctggcatatgccacgcagtgtttgaatatttatgccggcaacaactgggcatgggatacagaggcgtctgccgtaagatatacaatggcgctggcttatgaagcaaaagatgaccccggtacctgcaaaaaaatcattgacctgattgtggcgaatgatccggaattcaggcctgcggcagagaaaaaaaatgaactgagaggaggaggattattttcttttttcaggaagaagaaataataattcagctgtttactttctgcacaaactgcagcaggtaaacagctgaaaaaagatcttggtccttttacatgggcttgttaaagctcaccatccaggggaaaccatatttatcggttaacatgccaaagcggtgcgcccagaaggtttctgccaggggcatcgtaactttccccccggcggataacgcattgaataatttttctgattcttcgtttgattcagtgcccagcgccagtgtaacgttgtcaccatttttgggcgcctggcctcccatgccatcagaggccatgagctcgaaagaagatgttttcaaaaacgcatgcatcaccaggtctttggacgcagtgggtacgttttcgctttcaggcgcctcgcccattgtcatgataaacaattctcctccgaagatgtctttgtaaaagttcatggcttcgcggcaattggttccaaaagtgagataaggtgttaatgtggtggacataacaatctttttagggtaagaaaatggaatttgggtagctcctaaagttaggcaaaaactaacttatcaacaccttatttcttaccagcaggcaggcgccgatgataccggcgctttcaccgagcctcgacattttcagtttggaatcgttgcttaccaggctgagggaatattttttcatagcgctttttatgggcaggcggatgtggtcctgtgtagcagccagggcgccgccaagtatgacgagttcggggttgaagatgttcatgagcagggcaacgccgcgacccaggttctctcctactttggcaataagttctatggccagcatatcgtcgttgttggctgcgtctataatatcgtgcaggtggatatcttcgggggattgatgcgtgcggctcagcatagaggaagaacctgcggcgagcttttgccggaacatattcaccagcgcccatccggaggcttctgtttccaggcatccttttttcccgcagtggcagatgatttcattgtcgaacatcgggatatgccctacttcgccgctgtagccggatttaccgtagtatagctccccgttgatgagtacgcccatacctataccatagtcgaggttgaggaacagcacgttacgttcgccgttcaccaggtccgaacaaaattctccgtaggccattgcccgtgagtcattttccaggaaaacgcggatgcctactttggcggcgatgactttgctgaggggttcatcgtcgaaatagaagaggctgtagttgtagccggtggcgtaattgatgcgtccctggatattgataccgatgccgaggatcttttctttgggaacggtgaggccatcgataaagttgttgatcaggaggcacaactgttccagggaagctttggtattatccagttcgtaggggagtccttccacggtggtgaccaggtttttgtggaggtccgacaggcccaggttgaggtgatcctgttttacatccaccccgatgaagaaggcggaatccggtaccagtccgtacaggttgggtttacggccgccggtggattctattttgccatagtccattacgaggccgtcgacaataaggtcattcaccaggttggtaactttgggtgtgctgaggttgagctctttgcacagatcggcgatagtggcgttgccggtattggcaaaataggccagcgccgcctttttcaggttgatattcttataggctacaccggtagcgtttgcgctgttgagctcttcaaaaaaggttttagccatagccatcagatagacttttacagtaattgctcaccaatttaacagcttaattctgattttttaaaatttaggggtagaaacaggggaatgtttctctatataaatgattttgttaattcgcaaaaaataatacctttgcaatcctttttgagttaaaaaggggctcttgtcatgtatagccggatagggtttccgggccggttgaacactgggaagagtaagttctttttatttattgcggatgtgatgaaattggtagacatgccagacttaggatctggtgccgcgaggcatgggggttcgagtcccttcatccgcacatataatattatgtggcaatgcgtcaatatggcaacgtgataatgctatgctctccctcactttcattgtcactcctgtcttattcagacacagtttcacctgattttattcaaaaacagtttcctgccattcctacttgccgttgtgacttcatggcagaaaaataaacaaggaatcattattgcttcttaaagaacactttatacaattcaattatggcaaccgttacgagagaaaacattggtttattgaacgataagatcactgtgaaagtgagccaggaagactaccttcctaattttgacaaagcagtaaagcaattcagcaaaaatgcgaacataccaggcttccgtaaaggaatggtacctgcaggtatggttaagaagatgcacggtcaggctatctttggcgacgaaattctgaaaactgttgagagagaattaatgggttatgtgcagacagagaaactggagatcttcggccagccgctgtccctggaaaaacaggcaaaagacctggatttcaacaagcctgctgattatgccttcgaatttgaagtggggctgaaacccagcttcagcgttactcccctggaagataacaaaaccacccttacaaaatataaagtaaccgttaccgacgaaatggtgaacgatgaagtacagcgtttacagctgaaaggtggaaaaacaacagaacctgaaacaattacttcagaagataacgtgattaacgttaaattcgaagagtctgacgagaaaggtaatgtagtggaaggcggtatcgtaaaagaaaacgccttactggttaaatactttgcaccggctatccaggctgaactgcagggtaaaaagaatgaagacagcattgtattccaactggctacttcctttgacgagcagcgtttgggctggatcctgaaagatctgggctttgaagcaggcgacaaggaagcagcaaacaaatatttcaaactgaccatcacgaaagttggtttgattgagaaaagagaactgaatgaagaattcttcaaagaagtttatccgggagaagaaatcactactgaagaagctttccgcgctaaactgaaagaagaaatcggcaaatactgggattctgaaagccgcaaccaccttcacaacgacctgtttgaagtactggtacacgaaacgccgattgaattgccaaaggatttcctcaaacgctggctgcaggtaggcggtgaaaagccaaaaactgcggaagaagcggaaaaagaattccctagttttgaccatcaattacgttggacactcatcagcgataaactggttaaagaaaataaactggaagtttctttcgaagatctgaaggaaaatgccaaacaaaaagtattaggctactatggcggcgccgctgctgatggagcagaatggttagacagctacctggatcgcctgttacaggatgagaaatttgtagaccagacttaccgtgaaatgatcactgccaagttatttgactgggctgaggctaaggtgaacgtgaaagaagaggaaatcaaagcagaagattttgttaatttacctcataaacatcaccatcatgaacattaataatgaattcagaaaatatgccatccagcatcggggaatcagcagcctggtagtagacagttacaccaaaagccaccagatcaacagtctgactccttatatccttgaagaacgccagatgaatatgacccagatggacgttttctccaggttgatggctgatcgtattattttcctgggagatcccgtgaacgactacgtagcaaacgtgattactgcgcagctgttgttccttgagtcttccgaccgtaaccgtgatatacagatgtacatcaatagcccgggaggaagcgtttacgccggcctgggtatttatgatactatgcagatcatttctcctgacgtagctactatctgtaccggtatggcggcctctttcggcgctgtactgctggtagcaggtacaaaaggaaaacgtaccgcgctgaaacatgcacgtgtaatgattcaccagcctcatggcggtgcagaaggccagacttcagacatcgaaatcactgcgcgtgagttcgtgaaactgaaaaaggaactcaacgaaatcattgccggccattgcggacagccactcaaaaaagtggaaaaagattctgaccgtgactactggctgactgcggatgaagcaaaagaatacggcatcattgatgacgtactccagaaaaatccaaagaaaaacctggaaacacctcagtaaagcttaaagcacaaggcataaataagctattgtagcgaagattacagcgatacatattaaaaaacgctattatcttcgctacaatagcttttgttttgtgagatgataagctttactctattaagacttacgctttcggctatttagtgtaaatttgtaaccctgcaataacagtgcaggcaatgatagtttcgtagaaaaataatctattccgaaatgaaagaatctaaaatccgatgctccttttgcagccgctccaaagaagaagtgcagatactgattgcaggcgctgaaggacacatctgtgaaaactgtgtagccaacgcacaggagataattgaccaggagttattcacccccggcaaaaaagcagctgcagccgtagcccccaactttgcacccaaagtgtctaaaccaattgacatgaagaaattcctggacgaatatgtaattggccaggatgatgcaaagaaaatactggcagtagctgtatacaaccactataaaagacttaaccagcagattggtgatgacgaagtagagattgaaaaatccaacatcatcatggtgggcgaaaccggtacgggtaaaaccctgctggctaaatccatcgccaaacaattaaatgttccctttgctattgtggatgcgaccgtattcacagaagcgggctacgtgggtgaagacgtggaaagtatcctcagccgcctgttacaggtatgtaactacgacgtggaagctgctgaacgtggcattgtttacatcgatgagatcgataaaattgcccgtaaaaatgataacccgtccattacccgcgatgtaagcggcgaaggcgttcaacaaggcctcctgaaattactggaaggcaccgaagtactggtacctccgcagggcggccgtaaacatcctgaacagaaactgatcaagctgaacacgcagaacattctctttatctgcggtggtgcatttgacggcgtcgaaagaatcatcagcagaagggtacagacccactctatcggttttaccgtaaacaaggaaaaagaagaggaaaacagaaaacagatcctgcgttatatcaactcccaggacctgaaatcctttggtctgattcctgaattactgggccgtttaccagtggttacctatctcaactcgctcgacagggataccctgaaactgatccttactgagcctaaaaacgcgctggtaaagcaatacaagaaacttttcaaggtagaaaatatcgatttacagatagaagaagaagcaatagattatatcgtagacaaagcgatggaatacaaactgggtgcgcgtggtttacgctccatctgtgaggtggtactgagcgatgcgatgtatgaactgccgtctgccaatgaaacacactttcatcttaccagggaatatgcacaggcaaaactggagcagtcaaccctcattaaactgaaagtggcataactgttccggtaatccgttaacagcaatactatcgctaactataaaacgctatttatgcaggaactcattcagcaattacaggaaaaagccggacttaccgccgaacaggccgcacagtccatcgatgtgatcaaagaatatgtgaagggcaaattacctccgtttattgccggtacagttgataactggtttgcaggcatgtcggataaagccgaaggaaaaaaggctggtctgatggatcaggcaggtgattttctggataacgtgaaagataaagcggaggattgggccgaagaagcaaaggataaagtgtctgatttcttcaacaaagataaaaagtagtttaatatacagtgaagaagggctttccggaggtatttcccccggaaagcccttcttctttttagaggcttctgagataaagatacaacgcggttaactcttcatccgtgtactgtgcagtcatgttccacggcatatcctttaccagcagctgctttccttccggcgttttgccggtacgcagcgtggcaataaaatcgttttggctccattttccgaggttcccggtagaggtgatattggctaccggcacagcgcccggtaccgggttatcgccgccggtcaatgtaggcttgtggcaaccagtgcaggaaaccgccaggtactggccgtactcttttgttgccgcctttgccacctggttaggctgttcccggtgatgatctattttttccacggggaacaagggtattttacccattacagacaggacttttcccatcggtcctatttttatgggaatggaaggtgcatctacttttggctgtgccctgcaaaacgcaattatagccgcaatatcgtgatcatccattcgggtgaactcctctgaaggcatcagcaataatggcttatttgcggtgtttaaaccgtgccgcaatgcctttagccagtcagtgttatcatagctttccggcaaccctcccaggccataggtgatattattacccgcaatacggccgatagccgggtcatccaccaccatttttccgcgcaggtctgtcccgtggcattcgccgcaaccctttatttcatagaggtgccggccctccgcaatagtagctgaatcggtggggatgggaatgtttcttactgtaactgcatattttttgctggcatgctgatggaagagaaaagtaaaaacgccgtatgccgttaatacgatcactaccaggcccaacacgatacgtgtggcccacttaagacttttggagaacataacaattaaggaatatttcagctgtaaaagtaatagggataaatattacaggtatcagtagaactactgaattaaagaagaatcataacgtggattacaggcttcacatttttactaagcatctttatacgggataaaccagttcagacccggtatagaaaagcacccgtattacagggtgcttttcattgcgtaaaagtgtttcaaatctttcttgattttgtgtgttaaggttgataaacggtaaagagtgatgaattaacccaaatttaacgttccttttgcaatattcaataacactaaaggggtaatattcaattattttgaaaaaatgatgaacggcttataaatactcttttcataaattataaaaatcctgctatctcaatagaatcagtatcaattgcaaaatcgttattctatctcagggcttcccgggcaattacaatcttttggatctctgaagttccctccccgatggtacataattttgcatctcgataaaatttttccaccgggaagtcctttgtatagccataaccgccaaaaatctgtacggcatcgttggcaacccgcacggccacttccgacgcataatatttagccatagctgcctgctgggtcatttttaccttgcggtttttcatatctgccgcctgcatggtgagcaattctgcagcagctatttctgtggccatatccgccagtttaaaggacacgccctggaaattagagatgggctggtcgaactggtaccgttcctttgagtatttcagggcagcgtccatagcgcctttggcaatgccaagcgataatgcggcaatggaaatccggccgccgtccaatactttcatggactggataaagccgtcgccttctgcgcccagcatattttctacaggaatgcggcaattgtcgaataccatttccgcagtttcggaggcgcgcatgcccagtttgttttctttcttgcctccactgaagccgggagtacccttttccacaatgaaagcgctcataccatgactgtcgcgcacgtcgccggtacggactattactaccgccacatcgcagcttttcccgtgggtaatccagcacttcgtgccattcagcacccagtcgttcccgtcttttttagccacgcatttcatattcatggcatcggaaccggtattaggctccgtgagcccccaggcgccgatccattcaccggtagccagcttaggcaggtaacgctgtttttgcgcttcattggcaaactgcatcgtatgaccggtacacaacgagttatgggccgccacgcttagccctatcgccccgcagatgcgtgaaatttcactcaccacggttacatattccaggtatcccaacccgctgccaccgtactcctggggcaccagtacgcccatcaatcccagttccccgagctgtttgaatatatgtaccgggaactcctgctgctcgtcccattccatcacgtgaggctgaatatgtgttttcccgaaatcccggatcatttgtgcaatctgttgttgcatctccgtaggcgcaaagttcataaacgtgtggctttaatatttgatctcaatgtaatgttcaattttacgataaataatctcatccaccaacggcaggttgcggaggtccgatactgccctgaaacccgcgtggctactgcggtactgcacaatgagacgggccagtttatagcgtatgtatgggtgagctgccaaagatttttcatctgtgaggttgaggtctagtttttttagagaactgctacctatctgtaagaacggttgaattttttgaaatgtggagtcgggtaagccataacattccgccacctgctccacggcataaaaacctcccagccgctcacggaaggcaataatccgccgcgcgaagcccgctccgatgcccggcagcgactgccaaacgatgctgtctgctgtgttaatatcaataggtacagccggggctttcttacgataacgggtaaacgacgtatcattatacctgacaaatgcgctgtcccggtaatagtgatgtccttttttaaatctttcatgcagggcattgctgtccccgtagtatgattccctgccatagtttttatttccgggtccgctccgcggaccatatctcccggaaaaccggttattgtccttacccgcaatgcgcacataaggtatcagctgtgtgcataagacgggaggcaacccatatatcttgcccagatcagccggcgtcctgaaatacccgcccctggccaggtacttaccaatagtaacagcggtgcgttcgcttacacccagctgctgccagccgcttgccggcaacgtgttgggatcgaagtaaaacaggctatctgtgtgtgcattactccgccgggtaaaagccggttctttctccactgctgccagcctggcttcaaaggccgttacggccgctttcaggttatcactaccggcaacgggcgtacgctgaaaataaaaaaccaggttggggatatagctggttaatatcatgagcagcgccagcgttaatatgcctagccgctctttccgggaaaaccgcagatattcgcggacaaatgatttccacatgggtcaacaacaattttgaccaagctaggattatgtatgctgtgttttgttaacagaaataaaacgcctctaaatttcgaggctaaggccgtcgtaggccaggtgggtacccgcaggcagctccgctgataccgcttcatgcagcccgagctgatggctgatatgggtgaggtatacttccggcacctccagctcttttcccagcgcgatggcttcttccagggtaaaatgagaaatgtgcttttcgcgtcgcagggcgttcagtacgaggatcttagaaccacggatcttttctttttcctccggcgcaatgtagttggcgtcggtgatataggtgaaatcatggatgcggaagcccagcacgggcatctgatgatgcatgacatgtaccggtgtaatggttagtccgtttacatcgaaaggatcggcggcaatggtctgcaggtttatttccggaatgccagggtatttaaaatcagaaaaagcataggcaaactcacgtttgatcacactttgcgagaactctgtggcgtatatattaatggcgcttttctgaaaatagttaaaggcgcggatatcgtccatgccggcgatatgatctttatgggagtgggtgatgagtactgcctccaggtgtccgactttttcgcgcagcatctggtagcggaaatccggggtggtatctactacgatattaccggcgggcgccgagatcataatactgctgcgtaagcgtttattttttttatcggccgaggtgcaaacttcgcaaccacaagctataaccggaactccctgcgacgtacctgtacctaagaatgtaactttcatcccaacatcatttgtctgtttttgcctattctgctgcgtgttcttccgaagccccgccttcttcctcccccgcttccgggatcggtttgctggcctgtatctgtttgtagagcttatgcgactctgccgtcagcgcttcttcatccaacggcagcgtcgttaaaatatcgatcagcgtattgatacgcccttcgaggttcaggaatttgttgatcactaccaccttcttgtgttccaggatgcagtaaccggacaggaaactacctttttcgaagcgcaatacatatttggcctcgtcgaagatcttttccagtttagtcaggttattaggtgtgattttgatattcatgtcgcaaaaatagcaaaaagctgttgttactttgttaccatcctggcaaaaggcacaatcatttcttccagggaaataccgccgtgctggaaggtattccggtaatagttcacaaaatagttatagttgttgggataacagagatacccatctccttttgcaaagatgtaggaagagttgacgttgggctttggcaatccggcatcacggggatcgcggaaggccagcacttctttcggctcatagttcaggttacggccgtgtttgtagcgcaggttggtagtggtttgtttatctccgatcacctttacaggtgtttttacccttacgctgccatggtctgtggcgatgatcaggtttatttttttatcgctgatacgtttcagggcctggtgcagcgggctgtgttcaaaccagctggcagtgatagagcggtaagaggcttcatcgccggccagttccttcagtacttccatttcggtgcgggcatggctgagcatatccacgaagttgtatacaattacgctcagcgggtaatccagcatgttatggatattattgagcatggtttgggcatcggcgtgattggtcaccttggtgtatgaaaaccggggatccattttcatctgcttcagctgggctgcaaaaaaatgctcttcatacagatttttcccgccttcttcatcgtcgttcttccattcctggggaaaccggtgttcaatatctatgggcagcatgccggcaaaaatggcattacggctgtattgtgtgctggtaggcaaaatgctgtaaaaagactcttcctccaccagccggaacgattcctggaaaataggctggatcgccttccactggtcgtaccgcaggttatcgatgagcaggaatacgttgggcacgttggggtccaggttaggcactaccttatcgcggaacagggtatgagacatcaccggggcttcttttgtttttggatggagccagtcgctgtaattacggctgatgaacttggaaaactcgttgttggcctcggttttctgggcattgaacacttccagcatttccgggctgttggtttttgtcatttccatttcccaatacaccagtttcttgtaaatgtccatccactcgttaaagtcggggttggagctcagcgccataaacaggctgcggaattcctgctggtaggcggtagtggttttttcggccaccagtcttttgttatcaattatttttttgagagataataatacctggtttggatttaccggtttgataagatagtcggtgatctgggagccgatagcatcgtccatgacattttccgcttcatttttggtaatcattaccacgggaatctgctgatcaatttccttgattttaccgagtgtttccagtccggtgatgccgggcatggattcgtccagtaatactacatctaccacctgttctttcaaaaattcgagtgcgtcatatccgttggtaagggccgaaactttgtagcctttgctttccaggaagataatctgcgatttcagggactctatttcatcatctacccatagtatatttatctgactcataataagatttaaggttccggtaaaaaaaggaatttacccctaattttttgcaaatatcattccccgtctatcatttgccggtaattatatgttaaaaagggctgaacacggtaaaatcatagcaggaaaaagtgaacaggctgataaagttatttaccttcgcatccataactttaattacctgtaacctaccaattgttttgaactgtcataggggtatcgtggatgccgcgcgtcattataagtaaaaaaattacatataattaatttcgggtgtagttttgcatacaggcaccagggattcagacgcggacgcccccgtctgaaatcgtataattaaatgcaatgaccgaacgcaagcgaaaaattgttaatgatccggtgtatggctttattaccatagatcacccgttgattcttaacctcatttcacatccatattaccagcggctccgccgcatacaccagatggctttggcgcacctggtgtatcctggtgctatgcatacgcggtttcatcatagcatgggcgcctatcacctcatcagtatggcgctgctggagctccggagcaagggggcagacattaccccggaagaggaagtagcggccaaaatggccattttactgcatgacatagggcatgggccttattcccacgctttagagaatggcattattgaaggggtatctcatgaagagatttcccagtggctgatggaggcattgaacaaggagatggatggcgccctgtcccttacactggatattttcaatggacgttatcataaaaaattcctgcatcagctggtgtcgagccagctggatgtagacagaatggactacctgaaccgcgacagcttctataccggggtggccgagggcaccatcgggtacgaccgcatcatcaagatgctgattgtacataagggggagctgatggtagaggaaaagggaatttattctattgagaagtttatcatagcccggcggctgatgtactggcaggtatacctgcataaaacggtgctcagcgccgaaaacatgctggtaaaaatcctgatcagggctaaagcgctggcacaggagggaaaggagctgttttgctctcctgccctgtcatatttcctgtacaataccattacaaagaacaattttgaatgcggaccggaatgcctggaattattttgccaactggacgactatgatattatgggggcgattaaagtttggacaacacacgaggacaaggttttgtcccttttatgcaagtggctgatagacaggaacttattcaaggttgtattaagtaatcaggcgtttgacggaagtgcagcactattattgaaggaacaggtcagacaaaaatgggggattgaaggagcggatctggactacttcgttttttccggtgcggcctcgttaagggcttataacgttaatgacgagaagatcaatatcctatttaaagatggaactgtaaaagacatttcctctatcgacaatgcactgattagccatacactggcgataccggtaaaaaaattctacatttgtcatccaaaaattcaggctaacaacgttttataaggaataaaatgttaaataaataagttcatactatccggtgtagcctggaaaacattacaattttaaactatgcagtttagcgcattacaattagctaccatgttagatggtaagctggagggaaatccggacgtaaaggtgagcaacatcgccaagattgaagaagctggcgagggcatgctcagtttcattgccaatcctaagtatgaagaattcatatataccaccaatgcctccattctgattgtgaatgagagcctggtgattgagcgtccgatcaaatcgaccctgatccgggtgaaggatgcctatagcagctttgcgttgttattggagcagtacaggtacctgaccggcaataaatccggtattcagcagccatcttacattcctgcatctgtgaagatgggggaaaacgtgtttgtgggtgcttttgcatacctgggtgaaaatgtggtgctgggcaacaacgtaaaaatataccctggcgtatatctgggtgataatgtgatcgttaataacgattccatcctgtatccgggcgtaaaagtatacgacaactgtattgtgggtagccgcgtaatgctgcatgcaggttgtgtgataggcggcgatggctttggatttgctcctcagccggatagttcctataaaaaagtaccccagattggcaacgtggtgatccacgatgatgtggaaatcggcgcaaacactactatcgaccgcgctaccatgggtagtacggtgatccgtaagggtgtgaagctggataacctgatccaggtggcacataatgtggacatcggcattaatacggtgattgcggcacaaaccggggtttccggcagcaccaaaatcggccagaactgcgtgatcggtggccaggtagggatggttggtcatatccacatagccgacaataccaaaatcaatgcacagagcggcttatccaagtcgattacagtacccaatacctctctgacaggctctccggcgtatgattataaaagttcgctgaaaagtcaggcaatttttagaaatttgccggaccttgaaaagcgcgtaaaggagctggaagagatggttaaacaactgctgcaagagcgggcaggtgtataaatgattactggttaaatagttatatattagttaccttattatggaaaatcaacagttgcaataccagcataccttaaagggtgagatcaccttgtcgggtattggcttgcatacaggcgcctatgttaatatgacccttaaaccggctacgccggggcatgggattaagtttcaacgtgtagacctgccgggacaacccatcgtaaaagcagatgtggattatgtggtagaaacaacccgcagcaccacgctcgagcacaacggcgccagagtgagtaccgtagaacacattatggctgctttggcaggaaccggtgtagacaacgtactggtggaactggatggtggcgaaattcctatcatggacggaagcgcctacgcgtttattgaagcgatagaaaaaaccggtctgcaaaaccaggatgccaagaaagtatactatactattgataccaacatcacttactatgatgagaagaaaaaggtagaaatggtggcgatgccggccctggattaccgcattacctgtcttatcgacttcaactcaccggtattaggtacccagcacgcgaaaatgaagggtatcgaagagttcaaaacagagattgcaccctgccgtaccttctgcttcctgcatgaactggaataccagctgtcgctgaacctcattaaaggcggggatatcaacaacgcgattgtggtagttgacaagccggttaccgaagaggagctggaacgtttagcaaaggtatttaaccgggaaaccatttctgtacagaaagaaggtatcctgaacaatatagaattacgtttcccgaacgaaccggcacgtcacaaactgctggacgtggtgggtgatctggccctgatcggatatccgatcaatgcgcatatcattgccaaccgtcccggacatgcctccaacgtggagtttgcccgtgcgatcaaagcgtatatcaaaaagaacaaacataataaagacgtccctgtttacgatcccaatcagccacctgtatttgatacaccacgtattgaaagaacattgccgcaccgttacccgatgctgctggttgataagatcattgaactgggagaagaaaaagtggtaggtatcaagaatgttaccttcaacgagcatttcttccagggacatttcccttcaaatcctgtaatgccgggcgttctgcaattggaagcgctggcgcaggtaggcggtattcttgcattgaaccgcgtacctgatcctgaaaactatgatacctatttcctgaagatagataattgtaaattcaaacagaaagtagttccgggcgacaccatgatattaaaaatggagttgctgagtcctatcagaagaggacttgtggaaatgcgggggacagtattcatcggcaacaaagtagctactgaggccgacatgatcgcacaaattataaaaacaagagaaggcaaataatagcaatgatccacccgcttacatacatacatccggacgccaaagttgcgcctaatgtaaaaattgatccatttaccgttatacataaaaacgtagaaatcggtgatggtacctggataggttccaacgtaactattatggaaggagcccgcatcggcaaaaactgccgtatttttccaggcgctgttatttctgccatcccccaggatttgaaatttgcgggtgaagaaactaccgttgaaatcggcgacaacaccactatccgtgaatatgtgacgatcaaccgcggtaccaaagacaaatggaaaaccactatcgggaataactgcctgatcatggcatatagccacattgcacacgattgcgaagtaggcaactactgcgtattttcaaataatactacccttgccggtcacattaccgtgggcgaccacgtggtactggctggaatggtagccattcaacaattctgtaaagtaggcgatcacgcatttgtaaccggcggttccatggtgcgtaaagatgtgcctcctttcgtaaaagcagcacgcgaaccactttcctatgtgggcgtaaattccgtaggattaaagagaagaggtttttccctggaaaagatcaactctatcctggacatttaccgtgtcatctttgtaaaaggttataaattatcaaaagccgtgaatatcatcgaagcggaatttcctgctaccgatgaaagagatgaaatcctgtcgttcatccgtgaatcaggacgtggcatcatgagaggctatacttccaggaccaatgacgatatctcttaaccagacaggtaagcgttttaactacgactggattttccgtcgggtaaccctcacctttagtgaaggacaacgttatgccatactgggtcccaatggttcagggaaatccactttattacaggtaatcagcggcgccattcaacacaatgaaggcgccgttacctatagcacgccggaaaaacccatcgctcccgatgcgtttttccagtattgcgccatcgctgctccttatcttgaactcatcgaagagttcaccctcacagaaatcatccagttccatcaacagttcaaaagcttcctgccgggaatcactcccgccattgccatgcaactggtaggactggaaaaagccgccaacaaacaactccgcaacttttcttccgggatgaaacagcgtatcaagctggccctcgccatcctgtctgatgtccccgttcttttgctggatgaaccctgtactaacctggatgccgccggtatcgccgtataccagcaactcatcaatgaatatggcggcaaccgcctgattattgtaagctccaacgatgaacaggaatacttcatgtgccgcgaacatatccatatcctggattataaatagataaaatcaccgggaatattatcttcgtgaaaagctaaaagctatatgaagactgccagtaagaaagtgattaatggctgggccatgtacgactgggctaattccgtgtacaacctcgttatcaccactacttttttccctatctattttttagcggttacaggtgaacatgtttcctttctcgggatgaactttgtaaactccgcactgtacaattattccatggcagccgcttacctgctggtggcccttgcctctcctatcctgtcctctattgcggataccaggggtaataaaaagaatttcctgcgcttctttaccatactgggggcactttcctgctgcgccctctactttttcgacggggatcatctcctgctgggcgtgatttgctttatcctttctaccattgggtattgcggcggcctcgtattttacaactcctacctgcctgaaattgcagcgccggaagaccgcgaccgtatcagcgcccggggttacagcatgggctatgtaggcagcgtgattttacaactgctggggtttggcctggtggtattgggtcccaaaatgggcatgggtaaaagtcagccggtgcagcttaccttcctgctggtaggtatctggtggtttggctttgcacagatcacctttgcccgcctacccaaaagcaccgtgatcaccaaacacacagttaacgcattcacagaaggatttacggaattacgaaaagtatatgcccaggtaaaacaactgccggtgctgaaaagattcctgcgtggatttttcttttacagtatgggggtacaaaccgtgatgatggccgccaccatctttggtggcaaggtgctgaagcttccggatgaaatgctgatcgttaccgtggtgattatccagattgtggctattgccggtgcatggagcatggccaggctttccacaaggtttggtaatttacgtgtattgattgccgttgtcatattctggataggcatctgtattgccggttacaaaatgcaaacggctatgcatttttatttactggccactgcggtaggactggtaatgggtggtatccaatccctcagccggtctacttatgccaagctgatgcccgaaacagaagacactacgtccttcttcagctattatgacgttaccgaaaaactgtctattgtaattggtatgttttcgtttgcctatatagatgatctcacggaagacatgcggaattccgtgctggcactggtggtattttttgtgatcggactgatatggatcatttccgcattgcgcaagcaaaagcagctatcgcagaattaggtatctttcaaaatagaactatccaacaaaattcaaggataatgaaattatacaccatagaaacaggattctttaaactggatggcggcgcgatgtttggcgtagtgcctaaaaccatctggaataaactgaatccggcagatgaaaacaatttatgcagctgggccatgcgttgcctgctgatcgaagacggcaaccgcctcatcctggtagacaacggcattggcgataagcaggatgcaaaattctttagtcattattacctgcacggagatgcgaccctggataaatcgttggcggcacatggtttccaccgggatgatatcaccgatatgttccttacccacctgcacttcgatcactgtggcggcagtattatccgccagggcgaacagctggcgcctgcttttaaaaatgcgacctactggagtaatgaagatcactggaaatgggctacacaacccaacgaccgggagaaggcatctttcctgaaagagaatatccttcccatccaggaaagcggtcagctgaaatttattaatcatcttgaaggcgtcaacttcacggataatatttccatccggtttgccaatgggcacaccgatgctatgatgctgccgcagatcagctataagggcaaaaccattatatacatggccgacctgttgccatccactggtcatataccactgccctatgtaatggcgtatgacatgtttccactgaaaacattgcaggaaaagaaaagctttttacaggaggcggcagataaagaatatatcctttacttcgaacacgacccggtaaatgaatgctgtgtactgcaacaaactgaaaaaggtatccgtgcaggtgaaactttttcactcagcagtatttaaattcctgtcagtctgtcacaattatggctgctgcattatatttgatagcaatcctgtatggctatacacataacaacagataataaattgaaaaaactgatcgttgtgggcgaccgcgtgctgataaagccagctacaccccacgagcgcaccagcagtggattatacctgcctcccggggttcaggaaaaagaaaaggttcaacgtggctatgttattaaaacggggccggggtatgctatacctgtgcctgtggacaatgacgaggcctggaagcctgaagaagagaaagtaaaatatattccgttacaggtgaaagaaggcgacctggctattttcctggtcagtggttccaccgcggtagtgtacgaggaagaaacctattatatcgtaccacaggctgctatcctgatgctggaaagagaagaagatctgtagatcatcttctgttatcttataaataaaaaaatctgctaacgaatagcagatttttttttgtctatcatgtatgaaaaagcaatctattctttgtattccagtatatcgcccggctggcattccagtacccggcagatctcttccagtgtggaaaaccggatggcctttgctttgccactttttagtatactgagatttgccatcgtaatacccacctgtacactcagctccgtcagcgacatcttcctttttgccagcatcacgtccagattgacgattatccccattgtatattgttatttagatcattaaatggtcaacgcctgttcttccttcaggctcaccgccctttcgaaaacgatggccagcgccaggatcaccatgaaagccatcagcagttcccaggaagcgcccaatacgctcagcagccggaaataaagccggttgttgtacacctttatgctgtcgcccgctatccaggcaaaaacgattttagtgagcagcagtcccgataacaccagcaggatcccttttaccgcgctgagatttttacgggagataatatcttcactcccggcgccgatcaataaccggaaaagataccaggtcattaccaggtacaataaacccagtatggtattttgaagaacggctgcttttaaaccgggggtatcaggactgaaacgtgattgaaaaaaagcaacaccattaaagatcgtgatgtaaacactgatcaatacagaaatgagcagcacgattttcaacgggagaagatacttactgattttcatgttacgccctgtttaatagctcaaaggtattttcattttatcgaaaatcaaaataattttatcgtttatcaataattaatgatcgataatcggtatgtatagacggataataatttgaagctcaaccgcttgttgctttttattatcttcataaaaaaaattacgtcatgcccaatcaggatgcatttctggaatatatcaaaagcggctatacttttaaaggcgagcatttcaagctgggatgtgccatgctgaacggcgaagtagtagccggggcggatgttttcctgccactcaaaacacttaaccgtcatggtttgattgccggcgccaccggtaccggtaaaaccaaaacgctgcaggtgatcgccgaaggactcagcgatgccagcgtaccggtattgttgatggacatcaaaggagatctgagcggcattgcagctgccggcagcgacaacccgaaaattgcggagcgttatcagaaaataggtggcagctggagtgcagcggcctatccatcagaactgttatccctcagccaggaaaagggcgtgcgcttacgggctaccgtcagcgagtttggccccatcctcctgtcgaagatcctggaactgaacgatacgcaggctggccttgtagccatgcttttcaaatattgcgatgataacaaactgcctttactggatctgaaagactttaaaaaagtattgcaatttgccggcgatgagggcaaagtagcactggaaaaggattacggaaagatatccactacctcgaccggcaccatcctgcgcaaagtgattgaactggagcaacagggcgctgcattgttttttggagagaaatcttttgaagtagatgacctgatgcgcatcagcgacgatggccgcggtatcatatccatactgcgcgtaaatgatatacaggatcgtccgaaactgttttccaccttcatgctcagcctgctggcagaattatacgcaacccttcccgaagaaggcgacctggacaaacccaagctggtgatgttcattgatgaagcgcatcttattttcaatgaagccagcgacgccttgctgaaacagatagacaccatcattaaactgatccgttcaaaaggtgtcggcattttcttctgtacccaaaacccgatggatgtacctccttccgtgctgggacaactgggtcttaaagtacaacatgccctgcgcgcctttaccgccaacgaccgcaaaacaatcaagcaaacggcggagaactacccgttatcagatttctataaaacagatgagttgctaacccagataggtattggtgaagcgctcattacctgcctgaatgaaaaaggtgttcctaccccgttagccgctaccatgctggtatctccacggtcacgtatggatgtattaacaccggcggaaattgacggactggtgaacaattccaaactggtaaagaaatacgggcaggaaattgacagcgaaagcgcgtatgaaatcctcaccgccaagctgcaggaagccgccgagaaaacagccgctactgaagctgcgccaaaatcttccgggaaacaaaaacaggaaaaaggcgttcttgagcaggtgatggatagctctgtagcgcggcaggtgggtcgtaccgctgccaacatcatcacccgtagcctactgggcgcattgggcctgggtggaaaaagcagtaaaagtaaaagctggttttaattatgcaacgacagtcacgctgtcagtttacatcaatatatcaaaagtatgagtagaattattaaaacgggcgtatgctcgtacggcatgtctggacagatatttcatgccccgttcctgcacgtaaacccgggatttgaatttacagcggtagtagaaagaagtaaaaacctggcgcagcaacgctatcctaacgttaaagtatatacgagcgtggaggatatgctggcagacaaagacctggaactgatcgtagtcaacactcctaactacacacacttcgactttgtaaaagcagcactggaagcaggaaagaatgtgattgtggaaaagcctttcaccgtacacgccaaagagggtgaaacacttgcagccttagcggccgagaaaggtttgctgctcagtgtttaccacaaccgccggtacgacagcgactataaagtagtaagagaggtattgcagtccggtcagctgggtgatgtactggaagcagaaatacactacgaccgcttcaaggaagagctgagttataaaaaacataaagaactgggaggccccggcaccggcgctttatatgacctgggctcacacctgatcgatcaggccattaccttgtttggcatgcccaaacgcatctgggcagacatccgcgtgatccgccgcgactccattgtagacgattattttgaactggtactttactatgatcatctgcgggcgcgtgtaaaatgcaactacctggtacgcgaagcccttccagcctaccagctgcatggccgtatcggctcctttatcaaaacaaaatctgatatacaggaagcgcagctgcaaagagggcttttccccaacagccccgactggggcgccgaacagccgcatgaatggggcctgctccacacggaaattgatggcaaagtagtaaagaaatatgttcccggtggaagcggcaactacatggactactaccagggcatctacgaagccttagtaaataaagctgccaacccggtaccaccgcaggacgccattaaagtgatcaaagtaatcgaagctgctttcgagagcagtaaggagggcagggtgattgatctttaacgcggatgttgtcttactcaggattacactgattatgctgattacctggattttcacttttggatttttatatgatttttaaagagattcggggagacaaaagcgattaaccaggatattgattttaaaagattcggggagataaaagcggttaagctggattgatcaccctgggttttaaaagaatttggggagatataagcggttacattcgcttgtatctccccgaatctttttaaaaatcatataaaaatccaaaagtaaaaatccaggtaatcagtaaaatcagtgtaatcctgagtaagacaaactccgctctcaccgtgcgcaagacagccgccccgcctcatcccgcaccacgatgccttcttcgttcaggaactggaggacttccatcaggtcgcttctttttacatcgggtagtttggtttgcagcatgttaaacagcagtggttcttctttcagcatggtgataacgtggtcggatatacgcttgaatccggcggcgtccataggctgtgatttcttttttaagcagatgtcgcatacgccgcacggagtggcatccttttcgccgaaataggctaccagttgctgcgtacggcacatatcacggttacgtacatacgcaaacatggcggcgagcctgtccgcataaactttcttgcgtacttccaccctggccatattgatgcgcaggttttgtgaggatacccgttcctggaggaaacacagctgtggttcgtcgcggcggggctgataatgcaggatgccgtattggtgcagctggtgcagctgtgcggcaatatcatcatcttccatcagcatgatgcggcctatctgccgttcataaatgggtacggcattatcgaaaatcccttcgtaggtacgcaacaaagttttgataatttcttccaatgcaggatacgcattttcaaactcgtacagtgattctttattggtaacgaattccgcccgggaggggaggaatacgctttcgctgagctgcagcacgccttcctgttccagcacgcgcaccgcgctgtaagcaatggtgaggttcaggtggaaggtgcgggcaaaatcgttgatgtcaaaatcgaagtacatgccttccgcgctgcctaccggcacctggaggtagttaacaatgccctggtatacttcacggatctgctccagcgagggaaactgcaacgcaatccgttcatgcatatccgttagttcctcttcgttatagagcaacacggcatatgctttctgttcgtccctgccggcgcggcctgcctcctggtagtaggcttccagtccgtcgggcatatcgtaatgcaccactatgcgtacatccggtttatcgattcccatgccgaaggcattggtacaaaccatgatgcgtgtttcattattgatccaggcttcctgccgggcggccctttctgcctgtggtaaaccggcatggtaataactggcagggatgccctgtagttccagcagggaagcaatttccttggtgcgtttacgattacggcaataaacgatgccgcagccgggtacgcggtccagtatatgttttaccttatcaattttggtagattcttccagcacgctgtaagaaaggttggagcgggcaaagcttttggtaaacacccgggcgtccttcatcagcagtttctcacagatatccgtttgtacccttggtgtagccgaggccgtgagtgccaataccggcgcttccgggaagaagctgcggatatccgcgatctgcaggtatgccggacggaaatcgtatccccactgcgagatgcaatgcgcctcatcaatcgccagcaggcttaccgggaggccatcacaataggtttgaaaaagtttgctttgtaatctttcgggagatacatataaaaacttgcatccaccgcggcgggcggcttccaggaccctttccacctcctggtaaggcataccggaatagatggagtatgcagtgatccctctttttttgagattggccacctggtctttcatcaacgcaatgagcggggtaatgaccaggcatagccctggcttcatcatggccggcacctgaaaacaaatggacttaccaccacctgtgggcagcagggccagtgtatcctgtccttccagtacagcattcacgatatcttcctgtaacgggcgaaactgttcgtatccccagtattgctgtaatatggctacgggcgtactcaaataaaaatttaatggttagtgcgaagatacgcgattagagcggattttgtcttactcaggattacgctgattatactgattagccaggattgatcatgttggatttttaaaggattttaaaggattagcgaagatataagcgaatgatatacccgcttatatcttcgctaatcctttaaaatcctttaaaaatccaaaaagtaaaatcaaagtaatcagtataatcagcgtaatcctgagtaagacaacatccgcttagatcacgtttttgtagcgcaggcgtatagagtttactgccagcaccacatcggagaggcccattatgccggcgcctacgatgggattcaggaatccgagggcggctaccggtatcgccactacgttataaatgaatgcccagaaaagattctgtttgatggtgagataggtatgttttcccagtcccagcgccagtggcagcgagcccaggttgttattaagcaatactacgttagcgctttgcatggctacctgggtggcatcgctgagagagataccaatggtggctttagccagtgcgggcgcatcattgataccgtcgcctaccatggcggtaggggcggttttcatgagggcgtctatcttttgtagtttttgttcgggcgactgttccgcgtatacttctgtaatacccagcttggcggccagttcccggcacttgcgggtggtgtcgccacttagtaagatggatttgataccggattgctgcagttgtataattacctgtgcggcttctggccgtatttcatctgtaaaatcgatccatcctgccagcaggccgtttttcaggagatacaggttatggctgtcatcttccgtaataccatttgccatgcggaaagagcctaactgccactggttacctgctttatcgctggcacgcatgccaagacccttgtgttcgcggacctgctgcagcggcacttctccggcagatttccagagcgaagcaatagagcgggcaatgggatgggaagaatatttttccaggctgtatactatctgtttaaaatcttcttccggcatatcaaaaaagtggtattcgcccaattgtaatttaccggtggtgagggtacctgttttatcaaatactacctgcctgatatccttaaacatttccagggtgtgacctcctttgatcaggataccattgcgtgcggcgcgtcccagtcctaccatcacggcggcgggtgtggccaggcccatggcgcaggggcaggaaataaccaatacggctacactgcgcatcatggcagtggccagcgtggtatgccctataaaataccatccaaggaaggtaaccagggctatgccgagtaccagtggcacaaatatggcgctgatgcggtcggccagtttctgcatgggtggcttatccgactgcgcctgttttaccagttctatgatataggacaacacggtgtctttaccggtggccgtgatatatactttgatgctgccgtcttccagtatggtaccgccaattactttgtccttttcttttttgctgacaggcgcgctttcgccggtgatcatggcttcgttggcatggccgctgccccagtagatggtgccgtccatgggtattttatcacctgtattcaccagtacgcagtcgcccgtacgcagggtacggttatccacttcatggatatgttcgtggccgtgatcggtgttaataagccgggctgtagtgacctgcatgcgtgccagttcggcaatcgcggaagtggtttgttttacggacctttcctccagcatatttcccaggaataccagggtgataatggctgccgtggtttcgtagaacatataatcggggttgccgtacacaacggttcctacaaaactgtatacaaaggctgcggtggcgccgatcgataccagcacgtccatattggccatgcggttgatgacggaacgcaccgcgctacggccgaagtgccacattcccacgaggtatactggcagcgtaagccagaactgtacccaggggtggtgtaaccacgaccagctgacccacatatgcaggagcaggggtaacgtaaatatgagacaaaaaacaaatttgaatgtaagggtggtatatattttcttttctgcgggtttgtcttccggcaacactacgcgatatcccatttgggtaataccgttgagtatttccgttgagttggcgccttccggtgcgttgaaactaacttcttccgtggcaaagctgacgttaacgtcctgcattccctttttctccaggtatttggaaacgccgagtgcacaactggtgcaatgcattccttccaccttgcaattaatggctgtcatctgacatctttcctcctgcatacaaagttagcagcggatgaaataggcaggtaaaatattaatgcaacgaagcggcagaagtgccatacaggtgcccggaaacaggccggacaagggccttacccgatttttgacgcagtgctgcaacttttgcaaaatctggtgacaatcgcttttgctttccgctttctccttatttttggggatgcaatggacatttacgctggatcaactgccggaaacagcccggcagttctgggatcatttcaccggtaaacaggttttcacccttaaaggcccgatgggggccgggaaaactaccctggtaaaggctttatgcgccgccaaaggcgtgcaggatgctactgccagtcctacgttttcaatcataaatgaatatgcctacaccgacgcagcgggaacaccccgccgcattttccacctggacctgtaccggctccgggatgaagacgacgccatcagcgccggcgtggaagacacactttaccaggatgccatttgtttcgtggagtggccggaaataatagcgcatatgctaccgccggataccattcacctccagctggaggtacaaccggatcaaaaaagggtcctgcgcgaaatcgcttcatctctcaaatgatgtatctttggatacttcgatttaaaaaaactgaacacgcatatggagcagaggcaaaaacctgtagtaagtgctgggtttacctattcaccgctggaagaaacgttggatattccgcagaaaaattcccgtttgtttataggtatcccgaaagaaacatctttccaggaaaaccggattgcccttacgcccgatgcagtcagcattctagcggcacacggacatcacatagtggtagagcataaagccggcgacgggtcgcattattatgacaccgactattcggaagccggggcggaaattgtatacgacaaaaaggaggtctttaaagcagagatcattgtaaaatccgcaccgctgaacgatgaagagatagagctgctgcacccgcaccagatcgttatttctcccatccacctggctgccctgaaagcgccacaggtagaaaaaatgatggataagcgtattacgctgttatcttttgagaacctgaaagacgatgcaggcacctaccctattgtgagggccatgagcgaaattgccgggggcgcctgtatgctgattgcgggacagtacctgagcaacgacaacaaaggaaaaggtatcctcctgggaggtattaccggcattcctcctacgaaagtagtgatcataggcgctggtatcgtgggtgagtttgcagcccgtactgcacttgcattgggatcttccgtaaaagtatttgataataacatttataagctgaaaaggctgcagaacaacatcggggtacgtgtattcacctccgttatccagcctaaagtgctggcagagcagctgcgcaatgccgatgtagcggtaggcgcattgtcgtcacaaagcgggcggacgcctattgttgtcagcgaatcgatggtgagcaacatgaaagcgggttccgttattgtggatgtgagcatcgaccggggcggctgttttgaaacctcggaaatcactacacacgaaaacccggtatttaaaaagtacgatgtggtacattactgcgtacccaatattccatccggttttgcccgcaccgcctctgaagccatcagcaatgtgctgatgcccttactcgtggaagctgccgacgacggcggattcgaaaaccttgtatggattaaacgcggcgtacgtaacggcatctatctttataaaggcgcattaacgaactaccacctgagcgaaaagttcaagcttaaatacaccgatttggagttattgctggcggtaaaaggatagagcggatgttgtcttggctcaggattacgctgattttactgattacctggatttttacttttggatttttctgattttcttaaaataataattaagggagataagagcggatatccgcttctatctcccttaatcctttataaaatcaaaaaagtaaaatccaggtaatcagtaaaatcagcgtaatcctgagccaagacaacatccgctctacacttcgagttggtagcccatcaatatggccgctatgatgataatgcccaccacgatgcgatagtatccccacattttaaatccgtacttttttacggcccctataaagaatttgatggcgcccagggctactacaaaggccacgatgttgccgattagcaggagcttcaggttttcgggatgcgcggttagcaactcccgtccttttagcagtttgtagccggtggctgctgccatggtaggtactgccaggaaaaaagagaattcggctgctacgctgcgggacagcttttgctgcataccaccgatgatggaggctgcactgcggctggtgccgggaataagcgccaggcactggtaaaagcctatgcgtaaagcggtaaaaacgtctattttttcttcggtggtaatagtgggttctttaaaatagtcgtctacaaacaggaggatgataccacctaccagcagcgtaattcctactgttagcgggctttccagcatggcatcgatcttgtcgctgaagaggaaaccgaggatcagcgccgggatcacggcgatggccagtttcaggtaaaagttaaaccggtttttatcaaataccaggaactttctccaataaaataccaccactgccaggatcgctcccagctggatcactacttcgaatagcttggtaaattcgtctttaccaatacccagcagtgcgctcacaatgatcatatgcccggtggaggaaaccggcagaaactccgttagtccttccacgatggcaataatgatagcctgaaaaacattcatcgaatttaatatggttaaaagttaaaaaaaaagcgatgagggatcatcgctgttaaaatacttttatagaagcaattatgcctttggtttcggacggtgcataatagcatatacttctatcaccaggcccagtacaataacgataggcgccagggtgattctgcggaagctatatacctgttccggtttaaagctgttgggatcgctggaatctcctcccatcatgaagaggaagcccaggataatcaccacaataccagccagcataaatttgtagttttcttttgggaaaatagggcggctgtcggccaatgtgttttctgcctccttatttaaagctgttttagccatagtgtttggtattatatcctcgttaaagatttaaagttaatacagatcgtccagtttcaggcgcaggtatttcatgacggagcggtgtgtgctcaccaaagaaatactgattccgatgaggatcatgcctataaagaggaacgctatcatcaggttatcacgcaatcctgccagttccggcaataatttatcggataccgacataataccgatcaggcctgcgatggcgattaccgcggcgatagcgccattggcaatgctgcgaaggtcaaagggcttggcaataaaccagcgggtagctcccaccatttgcatggttttgatcaggaaccggttgctgaacatggccaaacgaatggtattgtcgatcaggaaaatcaccaccaggcataataatccgctgatgatcaggataattaatccaatcctgttaacgttttcgttcagtttgctcaccagcatacgctgataggatatttcccttacgatgctttgctgtgacaggttattttcaatgatcttcaaactgtcattgtttacataattggcgtttgcctttatgttaatgctgctgtacagcgggttatattgcagaagggtgataaagtcctccccgaaatcctttttgaaccgctgtgccgccatatctttcgacacatattcaattgacttaatatatggcctgtgtgccattgaatcgcgcagggccgtggcctgtgcttctttcacgttatcccggaggatgacctgtatttctatgctttccttaaaatacacactcagcttgttagcatgtattaccaccagacccaatgtgcccagtaaaaacaataccagtgctacaccaatgatggagtacaggtaggatggtttcgacttctttgctgatgatttcccggattgcgccattaatctgcagtttatcggcgaaaataataaaaattagtagttatgtgtttaattttgccaacccggtcaggtaataaaccctttccggccaatagaatggcaatatatagagatgttggggaatgacattggagtattaatgaatttaacattattttgctgaacaggcattatagcaactttttaaattataactgataacgccttaatgaccggacgtattgtttatatccggacaattaaggttcatctacaacagatatggaatacaatttcagggcaatcgaaaaaaaatggcagcaacaatgggagcagtcgcatgcttaccgtgtgagcaataacagtccaaagcccaaatgttatgtactggacatgttcccctatccttcaggggctggtttacacgtaggccacccgctgggatacattgcaacggacatctactcccgctataaaagactaaaaggctttaatgtactccatgccatggggtacgatgcatttggcttgccaacagaacaatatgccctcgaaacaggtcagcatcccgcagtaaccaccgaacagaatatcaaggctttccgtgaacaactggataacatcggcttttgctacgactgggaccgccaggtaactaccagcgatccctcctactataaatggacgcagtggattttcctgcagatctttgaaagctggtacaaccgcagcacaaagaaagcagaacccatcacttccctggtagctatttttgagaaagaaggtaacgccggtcatatctgccccggcgaccggagtatacaattcacggcggccaactggaaaagctatagtgagccggaacagcgcaacatattgatgcagtaccgcctcgcctacctggcgcatgcggaagttaactggtgcgcagcactgggcaccgtactcgccaatgacgaagtagtgaacggcgtaagtgaacgcggcggttaccctgtagtaaagaagaagatgagccagtggttcctgcgtatcaccgaatacgctaaccgtctcctggaaggactggaaacagtatccttcagcgatgccatgaaagaaatgcagcgcaactggatcggcaaaagccagggagccgaaattaagttcgccctgaaaaactccaccgaacatgtggaggtatataccacccgccccgataccatcttcggcgtggacttcatggtgatagcgcctgaacacgagctcgtatcccggatcaccaccccggatcagcaagctgaaattgataagtacctcgaatacgtgcaaagccgctccgagcgggagcgcatggccgatgtaaaacaaattaccggctgctttaccggcgcctacgccatcaacccgtttgatggccgcgaaataccggtgtggattgcggaatacgtactggccggctatggtaccggcgccatcatggcggtgccctgcggcgatcagcgcgactttggctttgccaaacatttcaatatccctatcaccaacatcattggcgacgccttcaacgggcaggaagccaatccaaccaaagaagccaaactgcaaaacagcggcttcctcaatggcatggacatgaaacctgctatggatgtggtgatcaccaaactggaagaactgggtatcggtaaacgccagatcaattataaaatgcgtgacgccggctttagccgtcagcgctactggggcgagcctttcccgatcatttataaaaacggtattccttacgcgatggacgaaaaagacctgccgctggaattaccgcatgtggaaaactataaacccggtgaagaaggtgaaggcccgctggccaacatcaccgattgggtgaacgtagcccccggcgtaaagcgcgaaaccaacaccatgcccggctatgccggcagcagctggtatttcctgcgctatatggatccacataataacaacacctttgcagaccgtaaagccaccgattactggaaccaggtagatgtgtatgtaggcggcaccgaacatgccgtaggacacctgctctactcccgtatgtggacgaaagtgctgtacgacctgggacatatcggttttgatgagccatttaaatcactgatcaaccaggggatgattggtggcagctccagactggtgtatcgcgtacgtggcacccaccaatatgtttcacatggtttgaaagatcagtacgaaacagatgaactgcatgtagatgtgaatatagtagatggtgtagaacttaataccgctgccttcaaaaaatggaagcccgactttgcagatgctaccttcatactggaagatggcaaatacatttgcggcgtacagctggagaaaatgagcaagcgcttattcaacaccgttaatccaaatgacctggttgagaaatacggcgctgatactttccgtatgtacgaaatgttcctgggaccagtagagcaatccaaaccctgggataccaaaggtattgaaggcgtacaccgcttcctgaaaaaactgtggcgcctgtttgccgatgagcaaaaaggcatcctggtaaatgaacaaccagccacgccggaagaactgaaaatattgcataaaacgatccagaaaatagatcacgatacttccagcttctcctacaatacagcagtaagccagtttatgatctgcgtaaatgaactcgctaccctgcgttgtcacaaacgcagcatcctggaaccattgctgatcctgctcaccccctatgcgcctcacctgtgtgaagaactgtggcagtatataggcaataatgaaagtattctgaatgcactttacccggtgtatgaagaacaatacacaaaagaaagcgctttcaattaccctattgcgatcaacggtaaaacccgctctgaaatgggcttttcactggacgccgctattcccgacattgaaaaagaagtactggccagcgaagtagtgcagaaatggctggaaggtaaggcgcctaaaaaagtgattatcgtaaaagggaagatgatcaatgtggtgatataatgccgcgcggaggttgtctttctcaggattacgctgatttaatggattagaccttttgtgatttgcggagatcggagcggaggttgtcttggacgctgattacgctgattttactgattaatctttttgtgattttgggagattgatggaggagttggggatgaataaagattacttaaagagtgactgggaaatacttcgttcatacttagcatatgcttaatacatgcagatgacccggaggtgatgtggaggtgacgtggacttgaagctaagatcgtttatcacaggcccttacagacgaaaaagtgcagggtgtttagacgcggcactaccatataaatgaaatgtgtacccgatatagcgtgagcggcatttaatagcaatagcttattaaatgccgcttaactttttaaattatttaaggaatactgttggtaagagctgctgaatttcacggaattttccaaaaattcaatgaaaagccaaatttaaatcaattttcaatagagaataccgatgctgaattaaaatccggccaatgcactcatctccaaaaatcccaaaaattaatcagtaaaatcagcgtaatcagcgtccaagacaacctccttaccgtatactcaacccgcttaaaataatcccgcacgtggacaaccccaccagcaaaataatccccgacgataataataatacttttcctatgtggttcttattggcaatgatcagtatcagtccgattataaaataaccccctaccaaaaacattgctatcagtcccgcagcaatgatcccttcatcgccggctacgcacatcagcaggaaaatgcccagtggtatcagggtaaacaagagtacatctttgaaaaatttattcatatacaattatttaaacaataggaataaaagtccgttcttcctggagttgttttaaataggcttccttatcatcacggtaaaaaaggttcatggtttcaaatgggataatgcggccatctttatgcacaatatgcacgcacgactttttaatggcgcgcacatcaaaatcataagcatcgaggaagcgcatgatcacaatgcggaacaggttcgtatagtcgagaccgggagcctgtacctgtggcaggcagcaaagcagcgactgcatatcatttaccgcagcatcggtggagatgccggtactgaatattttcaggatgtgctgatgcagtctttcgtcctgttcatacacgatggtgttttttgaattattcagcagcacagcaggatccacgtagcgggtgagcgggtatacctgtccttctattttgagggcataggccattgccaaagcgtccgggttgcagggaacgggaataatgtcgtgatcgttccagatgggtgattgctccaggatacgttgccgtacttctgtaagggtgatacgatccgtagcggggtcgaagccatcggtgcggccggccacctgtaccggctgaaacgtaacaccgcgaacgcagggttgtttcagggcatagtcgatgatagcgcccatttcgtcttcattcacgccgcgttgcagggttactactaaggtagtactgagatttacttcattaagattttccagcgcctgttttcttacatctgtcagatcctttccccgcatacgttccagcgcttccggcttaaagctgtcgaactgaagatatacctcaaaatccggcatgtaggtagcaaggcgtgcggtgaattctttatcttttgcaatgcgcacaccattggtgttgatcatgagatgccggatcggctttgttttagcgatatccagtatttcgaagaactgcggatggatagtaggttctcccccgctgagttgcactacatcgggctgaccttcgttttccacgatgatatccagcatctgctctatttcttccagggtacggtgccggccgtaatgcggcgacgacatggcgtaacacgtaggacaggtaagattgcagcggtctgttacttcaatgacgctcaggcaggaatgctgctcatgatctttacagaggccgcaatcataaggacagccatagtgtgtgctggtattggttttaagcggcgcttcagatggtttgttatagttgcgggtatttttgtaatagtcgatgtcggtagcgattaacaccttttctttcccatgatgcgggcaatgcttgatcatgaaaaccttttcatcttcaaatatcaccttcgcgtctacacggcgcaaacaggtactgcagatgctgagtgtaaaatcgtagtaggtgtaatttttttcaggcatattgtttttgtgttagtcgtgacggaaaaataatcaccggtgaataatagagtaacccggccaaacaggccagctgtatagatcccagcccgaaagcgaagcgatatcctggtttgataaaatccagcccgaaacggaacagcaggtaggcaatcatgaaaagtttaaaccgtgcgccgtttgccagggaatagcggcggctgatgccggttaacatctgccataataatattaaaaaaataatttcatagagagataccggatgccgggggatgccatcgcccagatccatgccccagggcaatgaagtgggcagcccataggtttcttcataaatacccatcgtaaaacaacctatgcggcctatgatcatggccagtatcagcggataaacaaacaggtcgccggtagaatctttttcgccgatggccttcttgatcagctctactccggcaagacctcccagcagtcctcctacgatggttttattctgatagatataaaacagcaggttatcggcgtgatacagccccggcgggttctccagcgctcctaacagccggctgccgaacaaagcgccgaaaatggcgcctataatggcccagagacggttactgctttctatccggtcgccctgctgcttccgcaggtataaaaaataccggaagccgataaacatacccagggtttccgttactgcgtgcagcggaaaatgtaaggaaaacaaattgatataaacggggaactgcaaaggaccagcattatttaatacacaaattaatatttatatttagacgaaagtcaagcactacaaaatatgttacaggaggtattaaagaaatatcagtccacctttaagccggttattccgcttctgggagatcatgagcccctgctggtaatggatttcaccgccaataacacgaccctcaccaaaaacatactgcaggacattaaccgcttcagccggtatatcgacaatacgctggaacaaagtggctgccggctgggaattggcggctatgcggagcatcgtactatttatgcggtaagtccccattttgacgccggggaagaaccacgccggctgcaccttggcatcgatgtatggggagaaacgggcacccggctgtatgcccctatgaatgcgcatgttcatagcttccgttttaatgatcatttcggtgattatggcgccaccatcattttgcagcaccagctggacggatataccttttacacgctgtacggtcatctcagcatttccaacctgcaggggttgtatgaaaatatgcccatcactgccggtcaggcgctggcccatttcggcacacctgccgaaaacggcggatggccgccacatctgcatttccaggtaattgaagatatgcagggtttccgcggcgattatcccggcgtatgccgctacagcgaaaaagagaaatacctgcaaaactgccccgaccccgatataatcctccagctcaaccagtacacccattaaataaaaaaggctgccggcaatataccggcaacctgtggtaatggttggttttaatatcttactttgaattctgtatcagcccttcgccatacgccatcgcattcagcgaaaacggcataatccataaatgggaatcaggcgtaatggaataggttttatcaccttcctgcttcgtgatggtagccctgaattgcggatcgttgttaaacctgcgcaaatcaagatataccagcccggtgcccctgtattcacacttcagctccctgcggatcagcgcaatggcgccagccaggtcagtggcagttacatctgcataaaactccggcaggatacgtttacggcgcacagtgtttagtacgttcatggcttctgcaattttcccggcgcgggccaggcattcagcctttacatagtacatttccggcgtgcgaagccctgcagcatttacatcatcccttctgcggtaggtccagatggtttccaaaccaaaggcccgcttcgtgaaattaactttaaaccgggcgtctcctttatcatactgcgctgaatcggattcccgcagcatagaaatatacatgccctgtacctgcatataagagctgccgtagtgaaagttataattctccgggttcctgaattcatacttcgggatattgatagaagggctcgtaccatctgccaatactttattctcgttataataattcacatagtcaaacagttcgctgttctgttttaaggcttcctccgcaaaggaagcggcggaggcatagtctttcataaataaatgtatcctcgacagcaatgcgtaccccgcgcctttacctgagaagtaaggattgtccggatgtacaggcaaataaggcatcgccgcattcagatctttaaggataaattcatacatctcttttaccgatacctgtttcatagatgcttccacattatccgatgtattcaggaatacgcccggatccgtggcagcagtggccggatcatacattttagcatagctggtgatcaggtagaagtacaacatacttctgcctaccctcgcctgcgctattaaacggtctttatccgcctgggtaccggtagtggcgttctgtacattattcaccagcacattataaataaagatgccggtgtaggcgccattataccccgcgtcatcagaagtatattgcaaccggtcctgggtttcctgccagttgaaattaatactggttaaattaagcgtagcctgcccgttggcgattaaatagaaatcattggctacctggttctgattatcgtaatcgaaagaatgcgctttggcattttccaccaatgctttgtaatcttcaaaactctgcggaatcttttgtcccttcggcacaatctccaggtacttcttacaactgatcgttccggtaatcaccaatccgcataatataaaatgaatgatccttttcatatacaaatctttacaacctcatgaattaaagtgaaatattaaatccaacattataggttggcatgatgggcagcgtaagccctgaaccattgtagccggtagcttccggatcaatatcttctccgttgaacccgatgtagaacaggttatcggcctgtaaacggatcctggcatctgcaattttcaaccggtgtaaccagcttttcggaagagaataactcacggagagatttctcgccttaatgtaagctgcgcttacgattgtctggtcgccatagatataataactgttcctgtaattgttaccatttttatcatagtcccatgtaatacgcggctcattggtgatcagttcatcacccggtttcttccacgcgttggtattgcctgccggcatcaccgcattcgggaacctgccattgatataaggcacattcattctcattacatgacctgcgttgtatacaaacaggaaagagaactggaaacttctataccggaaattattgattaacgcaccgctgtaaacaggtacataggtaccactgtaacgcactgcatccggcgtagtgatcagcttatccgtcagctcattcttttggttgtagatctgtggttcaccgatgctgtttaagccgccatatgcgtagctgtaaagacttctgtacggatcgccctgcacatagtatccgtttgcattcggcaccagttcactggctgttctgggcttatagtctaccctggtaacttcgtttttattgaaagatgaatttacggtaacatcccagtcgaagctacgacggcggacgatcagtcccttgagcatcagttccactcccctgttctgcatagcgccgttgttcacataagcagtggcaaagcccagcgcggggttaatggtcacggtactcaggaggtcattacttttcttattatatacatctactgatccggacagcctgcttttcaatacgctgaaatcaatacccacatttgtggtagcagttttttcccaacgcaggttagggttcggcggattattaatagagccggtggtgttgcctgtcatagtattgatgccatacgatgccaccataaaaggaccggcgttccttgccacgttgccattaattccgtaagatgctctcagcttgaggatatccagccacgagataccttccataaactgttcccggctcataatccagctggcgccaacagaccataaagggcggtactggtaggtgggattggttccaaacaggttcgacaaatcataccttacgctaccattcaccatgtatttgtcgttataggtataagctgcatttccatagaaagaaaaataacggttggttacttcattcaaatacgccagttcagaagggcttaaagatgctggtcttccattgagaccaatgaagcggttactaagctccagtgcattaaccggcatgtagctcagcgtgagcggatcatacccgaacatgccactgaagtcgcggttgttcttcacttccctggtttcagaaccggcgatcgctattatttcgtgacgttcattaaatgttttgttgaagtttaactggttgcggaatgtataagcccgcaggtaatcacccgtgttgcggaatgcgtttcctattggtaacttataggtagtgttgccccttgtatccaatgcggaaaatgtgttgagtttatcgcgcatgtaataggaagtaacatccattaactgctccgttttgccactgttcttttcatactggaacatgatatcatagttgagccacgaagtaatttttgcattcagtttaccataagcccgggttttaatagaacgggtgtagagcaggtttttgttcatttcctgttccggaattctatcgatagaatagaggccatatttgtcataaatagccttgtcgtcagcagtttgggtgttccttaacggcaatgcatttccttgtgcatcataaatggattcaaagggcatcatgctattaaataaaccggtagcagacattccatcggcgcccgtacgtttattatcgccataattcaggtatatgcccgcggtagccgtgagccatttgttgatggtgagcgtgttggtaaaattcaatcccagcgatttatttacatcctgtttgttatacccctggtcattcctgaaagtggcagagaaactgaaagcgttgcctgcggaggctttggacaccgacaggttgtattgctgattagctgcggggcgtaccaggtgatccaggatctgttgattgaatacgttttgatgacgcatttcgttcagctttgcatctgcttctgcacgggtaatttttccttctgccacctgtagcaggtagtcgagtgcaggcgttactattcctgcgccggcgcggaggcgtgcggcttccgtgagcggtgttgttttaaatgcagggtcattatcaaagtaatcgtaggtaaggtctattatttcgttggcgtcggctctcttcaggtaggagagatcatactttggcgtcatggcaaaatcaccggaaaagctgatgcgtgccgggccggacttcgcttttttagtggtgataacaattaccccattagccgccctggcgccgtagatggaggcagccgccgcatctttcagtacggtgatattttctatatcttccgggttaatatccggcacataatccctcagtctcctgttatcgtcgtaggcgatgttttctaccgggaaaccatcaatcacatacagcggtgcgctggtagcgttaaaggtgctggttcccctcacattgatatcgcctttataacttactacgccgggaagtgtaccttccagtacctgtgcgagactggaaatgcggcgtttctccaggtcggcggcttttacagtggcgaatgcgccggtggcgcgttctttcgacagggtttgataacctgttaccaccacttcattgagcactttgttttccattactacctgcagcgtattacttctccccaatgctaccttctttgcttccataccggagtaagaaaataacaggacgccggcatctgcgggaatggtgatcaggaagtagccattgttatcggttactgtccattttctttgtccttccagttggatggtaacgcccgggaggacgctaccacgctggtctttcactgttccattcaccgtgcgggttcctgtttcctcaaaggaatcggcgcttgcagccggtgatgactgtaccaggttactggcctgcatatcttttctttgacggggtacaatggtgtagtgatttttatctacatacaaaaacaacaaatcacggggatacaggatacttttcagtacatcctccaccggcctgcctttcatggcagctacatttaccgtggtggttttgtttttcagcagcacgccttcatacataaaggtagttccgtataatgccgttaccttatccagggcttctttaacagaaacaacaggcgaacgtttaccggctggttgttgcgctattgcccgggaactgcccagtaacaatatgcataggtacaggaagccatacaggctttgtttgatacaaatcctcatcgatcttggtttttgataatatgtgtttaaaagccgcgctgaccggcgctcttaaaggtcagcgtatcattgttcttttcaattttcatgttcagtatggctgacaattcaaacaatacattgttcacgttattcagcggtaacacgccatctattgtacggttggccacagtagtatcttctattataatagtaaatccatatgtatcctgcagtgtattgataatatcttttacagcggtttgttgtagctgcattttgctttctgtccatgccagcgctacttcttttttagcaacagctttccgcagcagtcctttaccggcatcataatccgcttgttcttccggttgcaggatcagtgaggcggtaccttttgcagctgatacttttacctttccttctttcaggaatacttccactttatcccttctttccttcacgttgaatatggtacccagcacttccacctgtacttttcccgcatgcactgtaaaggagggtgtagccctgcgggaaacgttgaacagtgcttctccctgtaaccatacttcccgtttcccatctttccagttataataactcagctccgaatgagcatttaagatgactacagaagaatccggtaatgttacccggagttgttgaccataggcactgaccaccttattcattttctccggacgaagcaggaaccaggcggtgacgatcagcagcggcagtaacactgctgctgccagccggtaccagcggcggttccgggtaatgggcacgacctgttgttgctgcagttgttgctgtatcctttcccatacaatggcttttacccctgttgccggcgtaattctttgcaggctaaggatagcttccagtgcgaccactgcctgctcaaacgcttccctattcggaggcgcactgtcccggaagcccgtccagaaagccgttgcggccggtgtggcatgcttcacccattcccggaagaacgcatcttccaggaaatcttcttttgtaaataaatgataaccggtctccaattaaatatccattagctcctcaaaaatcatcacaggaaagtaaaaaggaactttgctgctccagtacagaacacaaagaattcgcaaaacaccccacttttttccaattattttataatttttttattaaaacttatagaagtattgattttagtgactttatatgcagataaatttttcatatttggtaatacccctacctaggaggagtttgccccggcgctgtactatttttttgtacatttagccgatcaactgggagatggatttttctgcaactaccgacgccacaatctgggaagcacttcaacagggcagtcaacaggcctttgctacaatttatgaccgttactttgagcggttatatgagtatggtatgcggttacatcctgatgatgacctggtaaaagatgcgatacaggaacttttcataaaattatggactaataaggatacattgagcacccctgtaaatccgcgtccctacctgcttgtagcgctccgaagtactatttataaccggttacgtccacataagaacagaattgtgatctccctggaccaggagcaacacgacttcctcgcccacttttctcctgaatcggcctatataaagaaagagcaattacaggcgcaacaccagcagctgctgaatgcacttaaccagttaaatgcaaggcaaaaggagatattgtatctccgcttttttgaagaactggattacgagagtattgccaccatcatgaatatttctgtaaaaggcgcctataagctctctgcgcgtgcgcttcagaatatgagagacatcctccaggtatcttccgcagtgcttattacgctgcttaccaatttgcgtttggagatgatgaaatagtaaattatctccgcttcagtaggatttacgcttcaccgtattatttttacaggctaaaattgaattggtatgagaagcatatggctgacagttttttgctgcctgcttgcaggcgcactggctgcacaggttccattgaaggtaatgactttcaatatccggtataataacccggacgacagcgccaatgcgtggccgcaccggaaagataaagcggcctccgaaatcctgttcctgggcgcccatacactgggtgtacaggaagcgctgtatgaccagatgcaggaccttcagcaaaggttaccacaatataaaacgattggtgtgggcagggatgatggaaaaacaaaaggagaattctccgctatattttacgataccacccgtttgcagttgttaaacagcgaaactttctggctgtcggaaacgccttccgtggcgggtcatatcggatgggacggcgcctgcgcccgtattgtgacctggggaaaattcagggataaaaaaacaaacaagttattttatcacttcaatactcactttgatcatatggggaaaattgcgcgcagggaaagtgcgaagttattgctgcaacgggtacatgatattgcgggaaaagatgccgccattattaccggcgacttcaacgctgttccgtcagatgaacctattcagattgttatgaatccaaatgatccgctgcatttaaccgatagtaaagccatcagcaaaacggcgcactttggccctgccggtactttcaacggatggaatatcgcagaaatggataacgagcccattgattatatctttctgaaagggaagatggatgttttaaaacatgccagcatttctgaaacgtgggaaggaagatatgcttccgatcattttgcggtgtattcggagatcaatatcaggtaataaaaataaacaacggatctgtggggagatactaacagtgtatctcctacagatccgttacgttaaaagccgttgctacttagtcgtgggtatgttccactgacatgctgttttccagtgcattcaccaccttgttatggaggttgccgttaatgtctatgctgatctttaacttgccatcagcaaaggagccggtgaagtcgccgatctgcagtttggtgaggatgaggtccatagaaattttgagggaacctttccaatcaattttggtgtcggttaccactacatcttttccatgtgcctgcagttcaatcttgccggagagcaggatttcaacgggaattttcttgctttcccaggtaataaaacctttcagtcttactgccggatctttcttatccccttccactctcgcatacacttttacctgctggtaagttcctttgggaattttaatggcgccaattacagcaggtacttgcttaaggtcaatttgcctgtctgtttttaatttgaattccacttcatctttaccacgtctggcatcgaagcggatttctcttaaacgggcggttgctgtgtcccaggtgatgtcgaaaccaccagacgctgcttttgccatggatgcatcacctgtgatagcagataagcgtcctgaggcatcaggagataacgtggcagttggattgatggctgagatttcgtagttcacgctggcagcgtccgcgtcgtcgattggttgattagtatctggtcctgccatgtccgtattggagcaggaggatagcaagatactggcaatgcctatggcaccgcagaaatgtaggattccggttttcattatcgatatggttttaaatgactaattggggaaattcgtggggtaaatttaacaaagaatttggagaaaaaaataggttcactgttaatttaaaaagaatgatccggctgagcttcgcttcaaccggatcaatatatgaggttacttcttcagcgatgccttctcaattcgtgtaggcgtgtccgtaccattcacaatggtgccggcgctgatggcaattgccttaataatatctgtgatatttttaatatccagtgtcgataattcatctcttactgtatgatagaaatggtctttatctatttgcgtggtggaaatggtgtgtgccggaacgccttgcctggcgagggtagcattgtctgaccggtaaaacaggttctgctccggatacgggtccggatggaaagtaaagctggatcctttcaggttgcgctggaggatagggccaaagctggatctttcataccccgtaatgaaggcgctgttcttaccgaatttggattccttaccaatcatctcgatattaaacattgctaccactttatcgggatcctggtgttctgaaaaataacgggacccatgtccgccggattcttccgctgtaaaggctacaaaaattacggagcgtttgggtggatgtttcttaaaatacttcgacagcatgatcactgctgtggtgccggaggcatcatcatctgcaccattggcgatactgtcgcctgcttctgaaggcaatatacccaggtgatcgtagtgaccggagaagatcacgaactcatccggcttggtacttcctttaatcataccggctacgttggcaaagtgctggctggtaacttcacggcggagatgaatgctccaggaggcggtatctgctaccggctcttttccgaataccagtatgatttgtttttcagcaggcggtactgcttccagttcactttttgtatcatagctccgttctgaaaacgaggcagcgatattgctgatgtaaccggccatatcagcgcctacccatacgagggtattcttttgcacggctgcagggtcacgcaatattttcatgagttcagcaggttcatttgcataagcaacattgtagctgctgtctttttcccaatcgaagctgcgaccggtgcctacggcaacaacgggccagtctttcagttctccactaacggtgagggatacactggaagtttttaaactgaacttgccgaattcctgcagaaaggttttttcgccgggcagcggctgaatgcctgctttctcaaactcgctgctgataaactgtgcagccttttcaataccgggtgtgccggggtaacgtccttgcatgtcgtccgcagccagggtaccgataacacgtgctacttctttctctttaatatcctgggtgtagccggtagcagcaagactgccggcagccaataataataacagtgatttcttcatataagcggttaatcctttttgttgttgtctattttgatggttgacggttgttctttttcctgtgtgaaataggcattgctatatgtctgcaggatagcagcataatctgctccgaactgcaagtctagcattttcccatcaggcgaaactaacactttggtaggataaccttttattttgtaagatttttcgatcttatcatcggcatgggcggccgggaaaacgtatttattggcggttataaagttgcgtgatgtttccatcggctcctggcaggaaatggccaggacagcgtttcccgggtacttcccggcgtttatatcctgggccagtgtattaaggtgaggcagatctttccggcagggtgagcaccaggtaccccagaagtccagcagcaaccattttccccggtaatctgccaggcggatgttctcattgttcattcctttcagtgtaaaatcgggtgcatcctcccattctttcagcaatacatcgcggaagtaagcattgaaagatttgccggggaagtgcgcattaaagaaggcccgtgtactatccagcatatccggctgggcggcaagttgccgcgacagcactttcattgcttcttcgggcttgccgagtgcgtccagttctttggcaaaacgggcgctgtaattttcttccgagtgaagaaaagcgcgatcataaaaactctcatacgctttgtccgcattgcttttcggggcagtgccagcggccagtgccaggtagttcagcgccgcttttttatccgttgtctttgtctgttcgtatttaaggtaataagcgtgtgaaaggatgtttttatttgctattttcttgctttgcaattccgggtgtgctgtccagaaggcggtgtcggcctggttatttttaagatcgctcaatgccttatccagcaaagcatccgcggcagccggcatattggatttgcgaaggatgtcctgtaccagcaattcataacgggcggccttacccagtgtcatttctgccgggcttatttgcccgaaatctgctgcaatactttttaatatagccgtatccgttgtatgcattgctttattccataacgacatcggccttacagatacctggaaaatactgtcgttctccgccaatatcctggtcagcagcaactgggcgccggcaggggctttcctgctttcttcaaatatttctgcaatgcgtgcttcactgacgcctctgctgcgaaactccttacgtgcttctatagtatcaaagtcatgctgtggtagatattgtgcgaaggattgatccagccaggagtcgagtgaccttccgtcggccgacaggagtttcagcaataccattgcactatctgggttttcataataggtatgctgtaatttattaaacagatgggaggatgatccggccagtgctgctgaaggaacctctttcagtgcattctggtattgctcatacatgtattccgaaccgctgccatagatactcagctttgccagtttaaaggccaggcggttaccatacagaggagcactcactgccaggaaccgggcaatttttgctgaatcaggttctccgtttacttccagccagttactcattctgctcatacgcatcagcgtattgaaccaggccgtgtcggccggtaatactttagcggtggcgggtgatacggtgacttcccgcgctgttaaagcggtaccgtttgactgcacctgccggctcagcgacttaaaggtttgtacatttcccttattacggatcaggctatacgaaattccaccggctacccgtacactatctgtcttattttcttccggcgtgccggttacttccaccagttctttatcgccgcttgtaacccggaagttccagggactttccttccattcgctatttgcagtaagtgccttgggcgcagccgggaaaaagcacttcagttcaaagttcaggtaattccagttgttcgctatggcagccagtgcatcgtcagtcagggcgagggaggcgccggcctcgctggcaatggctgcaatattcacgggagcgctgatactatcattggaatatattttaaacgccaccggccggtgcatcagcagcatgagactcatcatttgccaatcctgcagataggtatcgggatctgctgaattaaatcgggcatctggcctccgtgcggccgcactttccagctcgtaaacaaggttggcgctaccatccgggtttatgccggtgatggtgatcctcattgttttgtttatctccatctggtagccaccctgaagactatcctttaatattaactggtagcgccaggaatcattctttttaaactttaactgggctatggtggcaagggggctgcaagcaacggtcaggtaaacaaggagcaacaggaacttacgcatataacggggtgattttaatctattaaagtaaacatataaaaacgaacaaacaatagctgcctgctacctttgaatatttgtgtatttttggcatatacaattatgtccaatcagcctttaagaccagaagataataagctcagtgccgctgagaaagagttcgagaacagtatacgtccgcgggagatcgttgaattttccggccaggaccaaattatcgagaacctgaagatattcattaaagcggcaaaaatgcgtggggaagcgcttgaccacgtgttgttccatggtcctccggggcttggcaaaaccacgctgtcgcgtattgtggcgaatgaactgggtgtaaatatccgcgaaacttccgggccggtgattgaaaagcccggcgacctcgccggtctgctcaccaacctggaagataaagacgtgttgtttattgatgaaattcaccggttaagcaccgtggtggaggaatacctgtattccgccatggaagattaccgtattgatattatgattgatacgggtccgagtgcgcgcgccatacagattaacctgcagccgtttacgctgataggcgccactacccggtcggggttgcttactgccccgctgctgtcgcggtttgggatcaagtcgaggctggaatactacaatgccgccacactgcataagattatctggcgggcagccggtttgctgaatacaaagatcacttctgacgccgccaccgaaatagcgcgccggtcgcgcggaacgccacgtattgccaacgggttgctgcgccgcgtacgcgactttgcccaggtaataggcaacggggttattgatatggaaatagcgcttttgagcctgaaagcgttgaatgtagatgaatatgggttggatgagatggacaaccgtattctcaatacgatcattgaaaacttcaagggagggccggttggcatcactactattgccaccgccgtaggagaagaagcaggcaccctggaggaagtatacgaaccgttcctgatccaggaaggttttattaaacgtaccccgcggggcagggaagtaacggagaaagcttatatccacctggggaaaactcccttcaggggtgggtccaatatgttgttttaatgccgcggattttgtctttctcgctgattacgctgattttactgattacctggatttttacttttggattttataaaggattaagggagatagaagcggatattcgctcttatctcccttaattattattttaagaaaatctaaaaatccaaaaaaatccaaaagtaaaaatccaggtaatcagtaaaatcagcgtaatcctgagccaagacaaaatccgctattctttcactaccagcctgaagccgttaccatgaatgttcacgatttcgatattgctatcgtctttcaggtatttgcgcagtttggcgatgtatacgtccatgctgcggccgttgaagtaggtatcgctgccccatattttcttcagtgccagttcgcgtggcaagaggtcgtttttatgttcgcacaacatgtggagcaattcgttttctttaggggataacgtatgtgtttcaccgttatgggccagggtgcgcaggcgggaattgaaggagtaggagccgattacgaattcgtgaatttcttcttccttattgttcagttcctggttgcgtttcaggatggcttttattttcagcagcagcagttcgctgtcgaatggcttggagatataatcatccgcgcccagtttgtagccctggatgatatcttccttcatggttttggcggacaggaagaagaggggaatatcggggtctacgtccctgatttcttccgccagtttaaatccgtccatattgggcatcataatgtccagcagacagatgtcaaatttttcgcggcggaaggctgccagggccaggataccatcgcggcataattccacatcatagtcattcagctccaggtaatttttcagcaccatacccagattggtatcatcctcagccaataatattttcggtttacgttcttccataatcataaagggttgattacaacaaatataaagtttttctgcggcacgaaaggtcggtaaaatttgggcgccggctctcaaatgatttgttaaacttacggtggcgggtcgggctaaagtcttattatttcttgtttaacagcgaagtgaagggataacggagattggtataattgatcatatctaccacgatattccctacagatatggggctttcgatgcgtagcggtactttgttggcgtcgtcgcttacccacacggtcattttttcgccgccttcgaagatggtgcctttaatgaggaggggtttgaatttaatggcccggaacttcccgaacttggtatttacttcttctttccccatgtacctgatgtagatgttatatacctggtcgtcgaggaacatggcgaaggggattttatcgcctgcgttgtatttgttgaagtcgatgttacgggcataatagatagcgctgatcacgtcctgtacgcaggggggtacggtaaaggtgccgtttgtgctgatagcctggtggccggcctggttaaacactacattattaaagatcttgtacccgccttcgtttacattcctgacaaatttgaggggttgcagggtggcggtatctatgtagctttcgtatttgtcgcgtactttaaagatccagtcgtatgcacggtaggttttgccatcgcctaccacatgataaacatcgcggttggcgaagcgttccagtgccacgttaaaagtggcttccccggcgcctacgtacattttaccaagattatagaatactttcagggtaatactttcaccagcattgaagctgctgttacggatggagcagaaatcggtttgtgcttcaacgggttgaatacaggaaagtcctaaaattatgagtagcaaatacttcattgatggaagctatttttccttaaaaatttttactcctaacaacagcacacttcccaaaacggccggtattaccaggttaatcagccagatacctgcagtggcagctacgatggccacggtattggagctaagcaacccaagaaaaaagatacttactttccccctgactcctaattctgcgatagcgatggtaggaactcctgccattaccaggtagatgacgctgttcagtaagaaggcctgccaccataggaattccatgccaagtgcgtccaacaaaatcaaatactgtgccgagaagaccacgtaccgcagggctgaaagcagcaacaggtaacgtaaatcgccggatgagtacttaacaatgatctgcacaaacaccttcgctttacgaaggaaaggtatcttttcaaatacagacagaatgatttgtaaccgaaaatataacaatatcgtcaggccacaaattactgtaccggtaatcaggactaatttctgccataaagaaggtgtaaggaagccgctttcttttgccagcgcatagttgttgatataatagagcaaaccaattaacccaaaaataatagtgacgatcagctggctgaaacttcctactatcgttgccgcaatggctttcagcttattatggtttttcaggtaaagtatgcgtccaccgtattcgcctacacgattgggggtgtttatagacagggatacgccggaaaggattgcactgaacgaccggagaaacgacacttcttcgaggggtttcaccagcttctgccacttacgggcttccagtccccagttgaaaagcatcagtaccgtaacgaggaagatgcccacccagcctttctcctgcaaggctccccacatgtgccgcacggattgttgcaggttatcacggtggatgagttgcgagtagatagagtatgccagccaagtaaaaagccctgcccctaataagtaattgagaattattttggtacttttgttcagacagtcaaattttggcaaaaataaactcctgttggcaaacaagtcaaaaataattctcggcattgaccctggcacccttgtaatgggctatgggcttatacttatcgaaggaaaaaaggccagcctcctggagatgaacgtattgaaactctctaaattcaaagatcactacgaaagactacagctgattcattgcagggtacaggaacttattcaagagcaccaaccaaccagttttgccattgaagcgcccttttttggcaagaatgtgcaaagtatgctgaaactgggccgtgcccagggcgtggctattgcagcggctatccaggccggtctggaggtcaccgaatattcccccaaaaaagtaaaacaatctgttacaggcaatggtaatgctgataaagaacaggtttggctgatgctgcaacgcatcctcagtatctctgaacgccctgattaccttgatgctacagacgctctcgcagtggcagtatgccacttttaccaggaaggtaatccgctcgcaggaccaggcaaagcaaaaggctgggagaaattcctgcagcagcacccggaaaggatttccagataaaagttaccgggttaaaaggttatttcataaatccgtaaattgtagttactttggtttaaattcaataacccaattaaagctaacggccatgcgtccggacaacagcttaactatgaaaagtgaccatcatttgttatatggaaattgtataacaagcttttttatattaatcagcatcaggcagatatgaaagcaagaatcctattggtggaagatgatcaaaatattggtgcggttacgaagaaacgattggaagaagcgggctatgatgtagtgcacagtatagacggccaggcggcctgggaacagttccagttacgctcattcgatatttgcctgctggacgtggtaatgcccaaaaaagacggcctacaacttgcgcagcagatccgcgaactcaatgaccatgttcctatattattcctcacttctaaaaatgaaaaagaagacagaatagccggactccaaaccggtgcagatgattatatcagcaaacctttcagtatgcaggaactgatcctgcgcatagaagttttcctgaaacggacgatgagccgcgggaaagacaaattgaacctctatacaataggtcagcttacctttgattatgaagatctccgcctctatacttccaatggagatatatccatttccgttacacaaaaagaagcggacctgctgaaatacttctgtaataatcccaataaaacactcaaaagagaagatatactttccaatgtatgggggaaagacgactatttcctcggacgcagtatggatgtatttatcaccaaactgcggaaacacttcaaatcagatcctcaaatcaaactggaaaccgtgcacggtgtgggattccggtttaatatcccttccaaataaccgttacattgcggcaataatctgcgcctgtattgccttaaattcttctacagacagcttcagcttactgcgggaaaaattcatatcatctgccgaattaatcgggatcaggtgcatatgcgcatgcggcacttccagtcctaccacgctaatgcctatacgattacagggaatcactttttctatggcctgtgcaatcggcttggcaaacaataaccactcctgcaacaggttatctgccacgtcaaagaacttatccgtttctgttttgggtatcaccagggtatgcccttttaccagcgggaaaacatccaggaaagcataaaaatgttcgttctctgctatcttatagctcggaatctcgcctttgataattttcgtgaagatggtcatagtatgtagttcttagtaacatgataaaaaaaacaggggctgcaaatgaatgcaacccctgcaaatatcatgaaaaagtaggcttatgcagttatattatcgatcttaaatttaatctgtccgtttggcgcctgtacttcagctacctcacctacctgcttacccaacaagcccttgcctatgggggaggttaccgaaattttgccagctttcagatctgcttcggtttcagaaacgatctggtaagtaacagtcttcttattagctacatttgtaatagttaccttacaaaggatagacacttttgatgtatcaatagcatctgcactcactatccgggaagctgcaatcgcattttccagtgtggcaatcctcgcttcatgcaaaccctgtgcttctttagcggcatcatattcggcattttcctttaagtcacccttttcccttgcttctgaaatagcacgtgcaatctctgcccttcctttggttttaagctgggtcagttcgctcatcatttgatcaagggtttctttcgtaacgtaatttatgccagacataacctgttgtgtttttttggttataagaaaaaaaaatcaacgcctccatttgcacagaagcgttgtttactggtattattgcaaatataatgaaatttgtataaagaaaaaagccccttatttcggttataaataaattgataatcaatcatttatatccgaaaaacacacctgtttgaccaggtttaaagtatatttaatttctctaatacaatacgggccattttgatgcttgcctgatgagagtaaccggcaatatgtggggttactactacattatcagccttcagcaaccaggccagttgttctttttcttcttcgttataagcagatagtttttcattttccagcacatccaggcaggcccccgccagcacgccattactgagtgcggcaatcaggtcgcggttattcaccagcttgcccctggccacattcatgaaccacaccggccgggcaaaagaagcaaaaaacgccgcattgcccaggtatttcgtttcggtggtcagtggcaggtgtaagcttaccacgtctgcctcccggaatatttcttccatggtcgactcctttaccgcagccgtaccaaagcctgttttatatttatcgtacgccagtatgttaacgtcgaacccctgcaacttatgcgcaaaggtgctgcctgtattaccatagccaaggatggccaccgttttgccattcagctcataaccccggttgccgtcgcgctcccagataccctgccgtaactccaggctgcttttcagcacattgttcaacaggcacaacaacatgcccaccgcctgctctcctaccgcatcccggttaccttcggggctgctcacacaacggatgcccttactttctgcataaggtacgtcgatcagctccattcccgaacccaggcggccgatccactgcaggcgtttagcctggtcgatcaactgcttgtccacatgaatacgcgtggtaacgatcagccctgtgcattcaccgatctcacgatatacttcatcatacgtaacagccggcaggtaggtgacttcgtaccctttgctttccagctgttcaatcaaatacggatgtgtttttgccgtaactaatactttcctggtcatatcatcttatgggataatgctgcaaaatcagccacactcagctcctcggctctttttgtaaagatggggtcctgtgccaacagttccttgtcaaacatcgttttcagcggattgcgcaattgcttgcgccgttgtccgaaagctgttttcaccaatacaagaaatttacgctcagaggcaatatctaccggttgttccagccgggtgaggcggatgacggcagattttacttttggcggcggattgaagcagttttcatgtacttcaaacaaatattcaatcttataataagcctgtaacagcacgctcaggataccatattccttatttccatgcggagcggcaatacgttgtgccacttctttctggaacatgcccactaccacatccacctgctgacgccaatcgagcagcttaaacatgatctgggtagaaatattatagggaaagttgccgatgaggcggaacgggccttcaaaaggcagggcggcatccaggatgctttcgttgatcagcttccccctgatagcggggtacgttttttccaggaactccaccttttccctgtccagctcaatagctttgaaatgaatgcctggcagctgcaacaggtattttgtgatggcgcccccgccgggacccacttccagcacttgctggccttcgattacaggtagcgactccacaattttcctcgagatgttctcatctgtgaggaagtgctggccgagtgatttttttagtgtatacattgtgaagcgcaaagataaagcatttattagcttttagcttttgaaaatgcccccggctaaaagcgaaaagctaaccgctaaatactttatatttgccattcattgaggcaattcagcatgagtactattcagatcaacaaaccggtaatcggcatcaccatcggtgatatcaacagcattggcgccgaaattatcatcaaaacgtttatggacgcgcgtatgatggaattttgtacgccggtgatttttgcatccaacaaaaccatcaacttttaccggaagctgatgaatgaaaataattttaactaccagagcatcaaggactttacccgccttaaccataagcaggtaaacgtgtataactgctgggaagaagaagtgcaaatcacccccggagtactgaatgaaaccggtggcaaatacgccgcacgggcactggaagctgccatcaactgtttgaaagacgggtatatcaccggcctggtgacagcccccatccataaaaacaatattcaaagcgaaacttttaactataccggccacacaccttacctgagggattccttcaatgcaaaggatgtgctcatgttcatgaccgccgacaatatgcgtgtgggcctgctcacagaacatgtacccctggcggacgtagcaaaatatgttaccaaagaaaatatcctgggcaagctgcacctgatgagagacagcctggtaaaagactttggtgtggaccagccgcgtattgccgtattgggacttaacccgcacgccggcgacgaaggactgattggccgcgaagaaattgaacacattgcccctgccatcaggcacgcgaaaggcaatggtatcctgtgtttcggaccgtatagtgcagacgccttctttgcaagggaaatgtttaagcaatttgatggtgtgctggcgatgtatcacgaccagggcctgataccgtttaagtcgctggccagcggcaacggtattaactatactgccggactgggcattgtgcgtacttcaccggatcacggcacggcattcgatattgccggcaaaaacctggcggatccggattctttcagacaagcgatttttgcctgcctggaaatactggaacaacgggaacgctatgccgagaacacccggaacccactcaagaaaacagaactggcatcggaatagctcagggccttccggctttcaggtaagattgtatggaagtaacgtagttttcaaaggctttcctgccggtggaggttatcttgcagatggtttgcggataattatccttaaactgttttactacggaaatatattccgcatcgcgtaatttattaatctgtacactcagattacctgctgtggcatttgttttttctttcagcagcgtaaactctgcttctttttcactgatcaacacggacataatagccagcctcaactgtgaatgtaataccgggtccagatctttaaaatccatgagcttaattttcttatacagctattttaatatttagctattttgtttcaatggttttatcacggaaacaaaataactaaatatctgaataaatactacctgattattgctggctttgttccagcagcttgcgggtatatggttctccccaatgcggtgctatactgctttccggcttgaaggccgcgaacttttccaacgccagctccaaggttgttttagcttttgatttactgccaccccattgttcaggtgtaaataataatgattgtccctgtaacatgtagattctcgggttctccggattaaagctcttcgcctgttccagcagggaagctgcttcagggccatacttcatgccacggctcataggatccactgttaaccgggcggtggccaccagtgaacggatacaggcaatttcagagttctttggactcagcgcttcggccttgtcgaggttggcctctgccttgtcggccagcggatctatctggcttttatctttcaacgtaagtgcctgcattacctccatataggcagcataatagtaaggcaaccactggcttttttctgcatccgcaatacgctcaaaagtattggccttttgttgcaatccatcaggcgtgaaaatgctgctgctgtccaggtcagacgtttgcttcgtcatggcctctgtgtattgggcgctttgcgccatgagggtagtagttatgctaccggtaaataaaaaagcaagaaataatcgtttcatatttattatgattagaggttattaataacatcctgtcttctgtcgataccaaaattcataaacatgccgaggtaaataaatctcggtacgttgggtactacttcatccctgcgtaatccatcggtagaataatggtatccgaacacctgtttattgcccaatacgttgctcaccgacaacacaaaaatggtgaatgccttccggatactggtgaggtaactggcactcacgcctacggagttgtaggtcattgtcctgtcggacatgaacttgtcagtggactgattgggattgtaataaggacggcctgtggcaaacgaatacgttaaccccaggttggtgctgagctttggcagaaaatgcttgtatacaatgctggcagtatgattggccgcaaagtcgggctgtacccggaacggatagttcaggtagtcgcgtttggtatcaaggtaagagtacgacacccagtaatccacgttcttaaacgttttccggtcgcgccagaaaagctccactccctgcgcatacccgctgccattgttgttatacgccggcgttgttttcaccaggtcggtatacttcttataaaacacctcagtacggaacgtataatccgttgccacccgctgatagctgaggatgtaatgggtggccttcatatagcccaggttgcggttgaagcggatatactgcggctccggcttctggtaataatcgccataggctacggaaaactggctgtagttattcattttatatgccagcgatacacggggtgcaaaattcatttcccccaatacagaactgtattccgcacgacctcccacacgccctacgaagctgggggtaaaataaatatctccctctgcaaaagcagcggtgtagttgtctgagaaattagctttattttcattaaaggccgatctttcttccgcatactgatactctcctcccagccgcaatacagagaagcgcccgaggtttttgtaaaacatcacccgcgtctggctcaggtccgatcgcactttaatcagtgagggcgccgggttctttaacagggtatctgcattgatattgtccgtgttgctgctgaaggaagcgccgatatataagtgccagtcgtgaccaatattttcccggtaggtaagattcgtatatacgttattgttatgcagcttaaacgactctgtataacccgggtactccaggctgttggagttaaatcccattttggtccagttgccatacccgtaaaatttgagcatgcctgtacgggaggttttatgccggaaatttacggaggtgccgatgatttccggtcccaggttcggtgcgtttttaggcttaacgatattaaagtagggcgacagattggtataatctgcttctataccgtaggaagtttttttatcttttgagagattgtccagccccgcgctcacacctattaccgataccccgacagaagaagacgaacgctccggcagatcgatggattcaaggatcagtgcagaggacagtccctgcccatattgcgcggaatagccgccactgctgaaagtggttcctttaaacaggaagggagaaaagcggccgcgtcccgggatatcggggaggctgctgtaaaaaggattccttacgagcatgccatcgatgagggtttgtgtttcatagccggtaccaccgcgtacaaacaggccctcgcggtcgttggtttgctgggcgcccggcaatgttttaatggcattggcaatatcggcgccggcgccagctgtggttacgatatccagcggcttcagcactgtacctttcttatcatcgctggcttcaaagctgccggcagaaatggttacaactcttagtgcattcaccgcacttttcagcacaatgttcagttgttctcctgcggcggtatttattttcagttccagtgcctggtaattggtgagcgtggccgataacagctggtcgccggtggcggtggtggtaaaggaaaaagaaccatctgctgcggtggtggcgccatcgtaggagcctttcactgcgatgttcacaccgggtaaaggatgcttctttgtatcagttactttgccgctgattttatgctgcgccaaagagaacaggggtgtaaagatgaagagacacagatagcggttgatattcgacatattcagggattaattacataacaaatgtaaactagtttattttataaaccaaataatcccaaagaaacggataaacgctggtttctccggtattgacctttgattaatttattacagtacatgcacaaaaaagcaccctttacctgacggtaaaaggtgcttatatttttagcgatgaacgctgttatttatgcgaatcttggcttcagttcatttgccagtgtaaccattttcttcaggccatcttccggcaggttacctttcttgaattctccgagtacttccggtaagcgcacctgcatttcattcaggaaagcttcttcaaaagcacgtacctgtttaacaggaacatcacgcagtaaaccgtttgtacccaggtaaatcatagctacctgtttttctacggcgtacggactgaactgtgcctgtttcaggatttccacgttacgggcacctttatcgataactgctttggtagcagcatccaggtcaccaccgaatttggagaaagcctccatttcacggtattgtgcctgatcgagtttcagggtaccagatacttttttcatggatttgatctgcgcattaccacccacgcggcttacagagatacctacgttgatagcaggacggataccggcgttgaacaggttaccttccaggaagatctggccatcggtgatggagattacgttggtagggatgtaagcagatacgtcacttgcctgtgtttcgatgataggcaatgcggtcagggaaccaccaccttttaccaggtgtctgatagattcaggtaagtcgttcatctgttttgcgatggcatcattgctgatgattttagcagcacgctcgagtaagcggctatgcaggtagaatacgtcaccaggatatgcttcacggcctggaggacgtttcagcaacagggatacctcacggtaagcaactgcctgtttggacagatcatcataaacgatcagtgcagggcgacctgagtcacggaagaattcaccgatagcagcgccggcaaatggagcgtagaactgcagcggtgcaggatcagcagcgttggcagctacgatggtagtgtaagccatagcgcctgcttcctgtaatgttttcattacaccggcaacagtagatgctttctggccaattgctacgtatatgcaataaacaggtttacctgcttcataaaattctttctggttgatgatcgtatcaatacagatagctgttttacctgtctgacggtcaccaattaccagctcacgctgaccacgaccaacagggatcatcgcatcaattgcttttacacctgtttgcagtggttcttttactggttcacggtacagaacacccggtgctttacgctccagcggcatttcatacaattcacctttgatagggcctttaccatcgataggttcacccagtgtattgattacgcggccaacaacaccttctcccacgttaatggaagcgatctttttggtacgacgtactttatcaccttctttaatacctgctgactgacccatcaataccacacccacgttgtcttcttccaggttcagtgcaattgcttttacgccattgctgaattcaaccagttcaccataacctacattgcccaatccgtaaatgcgggcaataccatcacccacctgtaatacagtacctacctcttccaggtcggcagaagcattgaagttgcttaactgctggcgtaaaatcgccgaaatttcatcaggtttaatatcaaccataattatgattttaaaaaaagtcgttagagaaaattagtataacgacaacagctttgcgtgtacgcagcggctgctgtatagattaacgtaagtcagatacgtaaatattcttgttaaactgttgtttaatatctttcagatcacgcaggatagaagcatcgaacaactgatcatttgcttccagtacaaaacctccgatcaggtcagcattcacggctgtttccagctggatctgctgtgttgtttcgctggcaattttctgtttgatcacgtccagggtagcattatccaaagcaacagccgtggtgatcttcaccgggctgatgtttttcagtaccatgtactggcgtgcaaactcagtggtcatttcagccagtgcgctttcacggcctttggtcaccaacaggttgataaaggaaatggtagtagcactgatgcggctttcaaatatggcagccagtatcttctgctttttatcggcctttatgatagggcttttaagcaaactcaccacatcggggttgcttttcatcacctgttgtaagaacagcatgtctgtatgcaccacttccagctggttcagttcctgagccagacctatcaatgattttgcataccgggatgctaaacggggattctgcatattaaaaaagcttttagcttttagctgttagcctttagagctaatggctaatatcttagttcaatttgatttctcctgccagttgtttcacgtaaccttcctgtgctgttttatcagccagttctcttctcagcactttttcagccacttcaatcacgaggttacctacctggttctttacatccgttaacgcagccattttctggttttcgatagcggtgtaagcttcactgatgatcttctttgcttctgcctgcgcttgtgttttggcttcgctgatgatcatatccttcgcgtctttcgcttctttcaggatcttgcttctttcagctttagcttccgccagcacatgttcatgttcagctttcatctgggccatttcttcctttactctttctgcagtggcgatagagtcagtgatggaaccttccctttccttcagggtagcgaggatgggggtccaggcgaattttttcagaatcaggaaaacgacgatgaaaatgaataatgaaataagaaacaagcctaacgcgggttgcaacagatccatataattagaattttattattttttgatgttgatattttctgatttcaggtagtttgacggtttgtctgtaacaaaagattactgcatccattgccctgtgcgccggatgcagtaaaaagtttggcttacagaactaccgccaacagaccagcgattacaccgaagagagcaacaccctcaaccagcgcagcagccaggatcatgttcgcacggatgtcgttagcagcttccggttgacgagcgatagactccagcgcgcttttaccgatgttaccaacaccaataccagcagcgatagccgcgataccagcaccaacagcaccaccagctttagccagaccagatgcagcagcagcctgcaataaaatagacaaaagtgccataatgaatatgtatttgaattataaaaaatttcgatttaataaagcggttggcatttaacttttggcaaaggctaaaagctaattcctgtatacttagtgatgagcttcgtcatgcgcaccttccattgcctggccaataaatacggctgtcaggttagcaaagatgaacgcctggataaatgctaccagcaattccagcatcatcattacaatgttgaacagaacagtgataggcaggaagccgtaaccagctaccttatttaaagatccgaagatgaacaccagggatataatactcaggatgataatgtgacctgccaggatattggcaaataacctgatcatcagtgatactggcttggtaaatacgccgatcaactctaccggcgcgaggataaacttaaccccaaacggaaccggaggattgaaaatgtgaccccagaaatgtttgttggtactgaacatggtagcaataaagctgatgatggccagtgctgccgttactgccaggttacccgttacgttggcagaaccaggcaacagacctaacaggttgtttatcaggataaaaaagaatatagtcagaataaaaggcgtatacctttctgcatgtttaccgggaatattaggctttaccacttcatcacgcataaagatgatcaccggttccatcaggctctggaaacctttaggggctttcttggaaccacgtaccctgtaagccttcgctacattcagcatcaggattaccagcaatacggcggcaatgatcatggaagtgatgttcttcgtcatggagaaatcatagattggctcaccggtaggattgccattggcgtctactgcgatcactttgccatccatgtatttggccggatccagtcctttttcgtgcaggtagtgcgcgtttaccagctggtaaccatcgtacgctgcatgaccatgctcaaatttagaagacgaaaatactgacgtgccccgtgcaggattgtaaatgatcactggtaacggaacagttacatggttatctccaatgctgaacaggtgccagtcgtgggcatcctttacgtgtcccagaataacttccttagcatcaaattttttaggctcaccttcttctccccccttaccttcttctccttcatgaggtgcagctgctgccgtttcatggtgggaaacttcctgtgcaaaggaaaaattactaaaactgtgaaggcctaaaaccaacacaagtgctaccattctatgtttgaaccaattgaaagaaatcaccgttttctgaaattttgcgcaaagatactcgtttttatcttcaaaattaagcgactacggaaaaaaagtaagatatatcgtaattatactgataaccagatgcttgtaattaaaaaacgcccgtttttttccacaaaaaaaggccgttgaaatcaacagcccgttaaagtatttcatattaatatttttctaattcattttacccttcttataccttactcacattaaactgcatactatgcagtttgaaataaaacccttccagcttcagtaactcttcgtgggtacccatctccttaatttcccctttgtccagcacgataattttatcggccttgctaatcgtagaaaggcggtgggcaatgatgatggcggtacggtcggctatcagcttgtcgatcgcctgctggatcatcatttccgactcggtatccacagaagatgtagcctcatccagcaccaggatagccggatcatacagcaaagcccgtacaaacgaaatcagctgccgctgccccagggaaagggtgcttccccgctccatcacctggtaatcatagccgccgggcagctgcataatgaaatcgtggatcccgatcagccgggaagcctcctctaccttcgccctgctgatattgctgttatgcaacgtaatgttatcataaatggacccggcaaacaggaacacatcctgcaataccacgcctattttgctgcgtaacgactccagggagtaagccggcagatcaatatcatcgatcttaatacttcctttctgaatttcatacaacctgttcaggatactgataatggtggttttaccggacccggtatgacctacaatggccactgtatcgcccgggtttgcatgaaagctgatattcttcagcacataacgatcatctatgtacgcaaagcttacattatcaaaagtaatggcgcctttcatcttctcagcgctctggtgacctctgtccgggatataatcttggttatcaattaccttaaacacccgttcactggctaccatacccatctgcagcgtattgaacttatctgccagcatccgcagcgggcggaacaacatattcaggtacatgataaaagcgatcatcactccctgggtaacctcgtagttcagcactttattagcgccccaccagaccattaatcccaatgaaatggccaggataatttccacaaccgggaagaaaacggaataggcaaaaatagcgtcaatattcgctttacggtgttccttgttaatatgtttgaaacgggcaaactcccttttctccgcggtaaatgcctgcaccaccaccattcctgtaaggtgctcctgcacaaaggcattgagcgccgataccgcattacggacccggtaaaacgacttattcacactttccttaaaaatataagtagcaaagatcagtatagggaaaggtgaaaggctgatgagcgtcagacgccagtcttccataaacatcaccgccagtatggcgatgatcatcagcagatccgccactatagaaataatcccttcggaaaacacatcattgatcgcctcaatatcattgatggtcctggtggtaagcgtaccaatgggggttttgtcgaaaaatgccaggttcaggtgtacgatctttttatagacagttacacgcaggtcctttactactgactgccccagccagttggtgaggtaggaaaaatagaagcggaccactgtttccagcaataacaaccctatctgtacaatggtcaccaggatcagcatctgcatcagctgccccgctatatacttatctaccgttacctggatcaggtacgggcgcagcggggaaatagcggccagtacaaccgttaatatcatggagatgtaaaaggatcgtttgtaaggagccgcgaatgagaatatgcgccgtaataaactgaaatcaaatactttctttaccgcaagattttccaatgtgccaggtttaaactactcaacaaacctacgataaaaaataattacgccggaggtttgcaggcaacaccggaatacaaaaaaagaaaggcgcaggggtcctgcgccttccggaaatatgctgataaataacttacttcttttcgtccttcataatttgcttgtaagccttaatgaatatagctccaaggtttttatgaggtggtacataatcgctgaaaaggtccttgttgcgggcatctcctgcaaatttctttgtcagctgggcccacatgatcacccaatccacatttttaccggaacgtacctgatcttccaggctgtggatgatcggttcatttacaaaccgggtacctacctgtttggaagaaatgatatgcgcttcgggtgacttttccagtacagtagccaggttatgataaccgccgcaggaaccgagcacgactatcttagcggagctctggaggttttccagggtggtattgatatgataactgtggccacggtgaatgaaaatggtagggtgaatatcgttttcatccaggtattccgacagtttggatattgcttctttatccgcaggttcatcggtgggcaggttcgcataaatagtagtggctttcccttttagcgaagtaatggtggcccagtatttatttttgctcactttccagtcggacgaagggaaattagtcatgaagctggcgaaagattcctgcccgtccttatctccataaaaaaacacctgctgatataccctgccactgtcgctttccaatgtgttataggtaacgtagttgataggcggcagctggagcttggcagccatatcggtggctttggaagaatcgttttctgattttgactccgtttcaaacaggctgctgagcagttgataaatcactgtaccgcgtttatcactgtgtttttttacatagttcaggttcttctttacttctacacggaggaattccagcagtttctcatcgcggatactaccaaaggagttggccacgtctaccgcatcttccaggtcttcggttttttccaggttctgcacatatttctgcatgagataattggaattttccggcgccatggatttcaggaaatgatccagggtattgaaaccggccgccatggcaataaactttttgaagcggtcgaaattcactaccatcagtaagctgtcgccgcgcggaggtttcatgcgaagcatcatctggtcatataaaccggcgttgctgtgattggtgtagctggaggtatacagttcttcctggccgttgatgatcaggtagtagagttcttccggtgtgaaatttttaacgatggcaaacctcactggggcgggttcttcatgcaggtcgtttaccgtacggatatacagtaatgattttgcctgcatgttttccatcatggctttcaggccgaatgggttttgtccatcagctttcagcttctgcagggcgatattggacttcaccatttgcttgaaatactggtagtcgttatccacaacggcctccagcttctcaacggtagtggtgcctgccaggagctcatctatgaagggtaatatcttggtgctttgggacgactgcccaatgcgtacgatctgctgtacaataggatcctggttacgcttgacggcattagccattggcgtataggaggtggcgtaggtaagtacctggttggggtatttacgggctacggcggctacaatggaatcggtgcccggatagttgagatagtctcccagcttaggcattacagtttccaggttattgaaggcatatttagtgaatacctgtcccctggcttctttgtagccgggattatcctggaaggattcgatgatcttttcggatgcctcgaaggaaagattgctgatgtagggcaaaatgctctgacctttgatatctgcacgcatcatattgcggaaagccgctatcatagcaggcgcttcttccggatcgatgttacggcgcgaccgtttctgattataatctttcagcgttacgtagatagcagaaaggtattttactttcagccggtgatccagtgaatcgttatcctctatctcctgctgcatatcgtccacttccttgatcagggcgttggttacctgcaagttggtggtttgatcatcagatacttttacgagatcgtctgctttaccatcgaacttggcggcagcggcctgttctttatcgatgttatcatgaaatccctgtctgctgattggaatcggatggtggctgctttgtgcctgtatttggctgactgccaggaccgtcagcgtcactattaataaaaatcttctcatactaaatggatcttttcgcaaggaccagatagcaaatttacaaccaaatacagagtttgccagcacttcgttgctatcttttgttttttagcgggaaatatatcttaattattctatctataactaaaactgttatccatgaccagcatctgattgaaaataaacacgaaaaagaaggccgttgttcagcatgatcataatcaccttcctatggatggcggataattgacatattaatacagcattgttatttgacgtaccttgccgtggagcgcggaaaaccagtctgatattgaattaacaatttcataatgttaattttccattaatcacggagatggctttataattttgtcccgtctttttaaaagcaaaatttatgatagaccaagcggttgcaggaaaaattctggtagtagatgacgaattggatattctggaaatcatcagttacaatctcaaaacagcgggttacgataccgtaacggcgaaagacggcagcgaggctatccagaaagcaaaaatattcagaccggatctgattatgctggatatcatgatgccgaacaagaacgggattgatacctgccgcgaaatcaggaaaatccctgagttcaaagatacaatggtattgtttttaactgcgctcaacgatgagaaatccgaagtagacgggctgaacatgggagccgacgattacatcgccaagcccattaaacccaaattgctggtaagccgcatcaatgcgcttttccgccgtttgcacaaacccgaggaaacccgcgtaacactgggcgacctgatcatcgaccgggaaaaatttacggttacttacaaaggacaggaaatcatcctggcaaagaaagaatttgaattgctgcagttgctggcatctaaacccggccgtgtattcctgcgcaacgaaatccttaaccaggtatggggtaccgaagtgattgtgggcgaccgtaccatcgatgtacatatccgcaaaatacgccagaaaataggcatcgacctgatcactaccgtaaaaggcgttggctataaatttgagatgtagtcatccgccctgttagcctttggctgttggcctttcagtgccggcagcccgtccggatcccaccaaaacattgttctccggcagctgaatgctggcggtcaaaagccattactgttgtcaagtaaaaaatttaaagtaatttcccattattaccttaattactcactttggagtatgtttaaagcaaaaaacctgtccccccagaagttagcgggatttacagcccttgtgatatcagccgtcatcgcattgggcagcctggtgatagatggcaattggaaagtagtagtgggagcctttgtgctgactttcctggtatcctattacctctatctttataccctgcagaattttatttacaggaagataaagctgatctataaattcatttaccaaacaaaagcgtccaagagagaggagtttttccaaaagaatattcttcccctgaaaaccattgaagaagtaagtgaagatgtggaaaaatgggccagccagaaaaaagaagaactggacaacctgcgccggaatgaagagttccgtaaggagttcctgctgaacctttcccatgagctcaaaacgcctatttttgccgttcagggctatattcacaccctcctcgatggcgcattggaagatcccaatgtaaataagctgttcctgaaaaacgccaccaagaacatcgaccgcctttgccggctgatcgacgacctggacgaaatatccaagctggaaagcggcgaaatgaccgtgaacgcagaagtattcgtgatccaggacctgatcaaagatgtatttgataccctgtcgctgaaagccaataccaaaggcattaagttcagtatcaaaaagggctgtgaagcgccgcagccggtatacgccgataaagaaaagatccgccaggtactcattaacctggtagataactccataaaatatggcaaacccgacggacataccattgccagcgtttacagcatggatggaaaaagggtgctaatagaaatttccgatgatggcatcgggatggcggaagaacacctgccgcgtgtatttgagcggttttaccgtaccgacagggcgcgcagccgcgatattggcggcaccgggcttggacttgccatcgtaaaacacattgtggaagcccacgaccagtccattaccgtacgcagcaaacctgaaataggcagtacgtttggatttaccatggaatccggaagagaataaaataatcagaaacggtattgcatcctgcaggtaagcacattatcctttaggtcgtccttgtacccttccagttcagtgctttcgttggtcacccaatcgtaatacaccatgaacttcaggtgttcgtttgcataatacaggtagccgatgcctacggtattgtagcgtatatccgcgggggtaagtcctgcgcccggagcgccgatatctttaccttttacttttgtattgggatcgtaccagtcatacttcaatacggcctggtgttttgcgttgccgaggttttgaatataatagagataggccccgtcgaaattgcggatataaaggggcagcagtcttccttccggtccaaccggtataacgcccggcgtttccgtggtaagtgcagtagctgtttgccgtccgcggagatactccgcccggaactgggtgaatcccttcccttccccgttggaaattttccattgcacatccgcgccgtagtaatgccggggcgcaattttcccgatattggatacggacgaatccactgtaaagacgggctgcccattggcggtacccatggtatggatctgttttgtaaactgctgcatgccgccgtacagtacagatgcaccgcccgataactggctttgggtgccctttattttccgtggcttaatagatatgcggcctataaagtctttatgactgtcgaaatcagtggtagctgtaagcccctgcccgttgaaagcacccgcatctattttcaggaagcgcagcggatgatccttgcggcggggttcaaaagatatcatggcgccaagatcgcgctccgttctcatcaggatctgtgacatccgcccacgctcaggggtttcacgatccgccgatgacaggttcacctcataaccaaaaggacgggcaaacatccctcccaccagcgagaataaattgaatttcgtctcaaaaaaacgaccatagaaatcacggatgttcactccccgctctgttccatcaaactggaaagcaaactgcactatcggcatatcctgtttgttgtagcgctcataatccacccggatacgcccccgccgcagggtaaagcgattatccactgcggtggggaaatttcctgccgcatacccctgggcacccctcgactgcgccatctggaattcgggctggatatagccgctaaaacgcaatgcatcgtacttcatgtacatggatatcatcccctttcccatttcagtggtagtgtctatcatatccatcaggaattgcgcacgggcagttcccgtgaaacataacatcaaaataacgatcggaataattctggcagtgcgcatcaggttctgaaattattgcgcaaaagtatagaattagcctttatttaatccagttgtttaaaccggaagggcttaaatcgttaatagctcgttaatccgctcccgttccggccggctcacctgctgccggcagactttcgtgtaaattagtttactccaaaaatatgcgtccatgaaaacatcaacttttaaccattgggaaaagaaaatacaacaggcgattgccctttcccatgacgatccgcagggggatcgcggattgaaagaagtagctgcgctgatcagcgaatctgttggcaacttctcgcacaagtttgtagaaatgtatgggatgtcttatatccattttactaagctaagaagattggaagcgggcgcagggtacctgcgtcacagcgattacagtgtaggaatgatcagtgaattgtgcggatacacgcaatccagctttaccaaagctttccgggaattctttgacgaagcgcccatcagcttccgcaacaggctttacctgataaatgaaaagaataccctggcacgcacaaaaattgcttctactccacatgatgatccgcagcatgttattttcaccccggaccggaccgaggacataaaactgcaggattaccagctgtattataatatcctcccacggacgggcgacccggtaaaaacaatggtggactacctggggatttaccagaagcagctgtatgccattaaaacttccctggaactgcccggcgccatgatcatcaccggcacactggatatcgtacctgttaccgactattcaaggatgttgatgtatgtaggtattatgattcccctgcaaaatgaatacgataaagcgcataaccaggtacggagttcattccaggagcccttcagtctttttacgaaacgtgttccggcaggcaactacaaaaagctaccggtgcccatgagctttgcagccgcagggttgcccatgtacgagttcattaacaacagctgccgggcaggatatttcaaaatgagcggtaaccatttctttatttcactcaccggcgaaaacgaatctgaaatctacatcccctggcaaaaaagataaatcatattaaaactggaagtaaatcgggatcataggttgcgtgcttttcacctgcaccagcaaccagatgaaagctaccatgatagctacgctcccggctacagggatgcgtcccagtattttctctacagaaaactccacttttgaaggcaggaagtgcaggatgaaacccagtaccattacccagaatacagcggtataaccattgtataactccagggcaatttcaggctggaagtcgtataccacctggtggatcagcgaccatgcatcgtggaaggtagatgccttaaagaacacccagcagaaacacacaaagtggaacgtgatgagcactcccataaccttcaggaaactggctttccatccggtgatcactgttttacttttcttcagatagtcgatacgcactttatccagtgccagcgcaccgccgtgcatcgccccccagaaaatgaagttccagctggcgccatgccagaagccaccaatcagcatcgtcaatgccaagttaacatactggcgcaccctgcctttgcggttaccacccagtggtatatacaggtagtctctcaaccagctggacagcgagatatgccagcggcgccagaactctgtaatggaagaactctggtaaggagaatcgaagttaggcggaatcttaaagccggtccaccgggcaatacccagcgccatatcggaataaccggagaagtcgcaataaatcaccagcgcataaccatacacacctatcaaacattccaaacccgtatgcttgctgggatcatcaaatatgtattgtacgaagttctggtaaatgaaatctgagatcacaatctttttgaacaatccccccatgatcaggtacatccccttgccaatgtcttcagaactgagacggtaaggcatagagatctgcgggataaaatctgccgcacgcacaataggccccatcatcagtttcgggaagaaagacaggaagaaaagataatccatgaaattatccaccggcttaatttcatcccggtaaacatctatggtatagctcaggttttcgaaagtataaaaggagataccaatgggcaggatcagcttcagcgtggaaatatgccccgctgtaacgtcgttgatcatccctataaagaagttggtgtatttgaaataaaacagcaaccctatattcaaaaagatgctcagtatgagcaacgatttcttcacttttttgtcggggctttcatggatccatctcgacaaattaaaatccacaatcgctgaaagtatgaccagtcctacataatagccgcaggctttataaaagaagtaaagcgagaatactgtatacacccatacccttgcggttttactcctgcttaccagcaggtaacacatcaggaatagcgcaaaataataaaagaagaacccactattaaaaaggaccgggtctgactcatggtacgacagttcgtataacagtttattaatgtcgatcatcggaggttactggatttttctttgtttgctgtagataatgtgtataagaacgttgcagggcttcatacaatagttgtccctgtaactgatatccccgtgcattaaaatgaatatggtcgggcgcccatgttcctgcaaatctacctttctgtgctttattcaccgcattaaaattccagcaggcaataccatgttgacgggcatagcccatgatttgctgcgtcaccatagagatatatgggttgggataatacgcggtatgatatattgttctgtatttctttttgcctattttcttccgggtggctttccgcactgcgcgcatacaatccggtggtgtggtcagcaggatatttacggaaggatcttgttcgcggatgagtgttaccgttttatctatttcatccctgaaggccagcgggtccattctgccgccataggcttcattggtacccagggaaatgatgaccagttttggtttcagcacggccatttgtgccagcaggatgttgctgatttcgttgtaatgttgaaacatcgcaccgttgatgccaacgctgtgatacagcactccgttgcggctgttttccataatggcgccataaaaccggaaaggaccgctccctgtgccttcccaccttgcctggaaagattgcgacgtttgtaaaaaatcgagggtggctttgctcagagtggaagagccgggaaaaggtgcaggcgttaccgttacagtagcatccggtactaccaatgtgttgttggtatttccggcatcatacagcagggttactttacggaagttattgtccatagatccgtccgttttgccggagaaagacaatgtgggcgcatcgttctgggaaatgatggtaatagcgccaggacccagcacatcagatttattgcggtctaccacccgttccgatgcccatctcgcagtgctgttccacttgaaatcttccgggccattggtgccggccaggttatatggaaaaacaaatcccctgcccgcataaccaaactggttctgcaacagggacgccaccgttagtgaaaaaaaacctgcctgcacgtgggaatcgcccagatgcagaatggatattacgttactatctgcctcatggagcagggaaaatacattgtacaaggcagtgtcctgctggatagccccggcatctgctgattgttgcgcataagttctaaacccgctgagtatcagtaaaagcactgccacccattttgtgctaaggttgttgtgcctgactgtattcattcataatagctttgtaaagcagcgatcccactttggctgctcccgtcctgttaaagtgtgtatagtccttgttggccatcaccgtgtctccctctacccactttaccatggcgccttctccgcccatagcggcaaaaaggttccagtaggctgtaccatgaccggcggccaggttatgctgtactttcagcaatgcttccacaccgggtgcggtaatatatttatcagcttttctgtaagatttatcggcagtaccaatgatcaggaatgaagtcgccggcaggtcctggcgaagtgagtccattactttcttcatcggtcgctcataccagctgtagtcagtgagctccggtcggaacaatacattggcgccgtaatgcattactaccaggtcgtaaggacgttcctgctgcatgcggcggaccatactggcggacaagcggcccagttccacgccgctgatacctctgaacgaataattatccacataaacaccatccccgttttcaaaacaaacaccataaaaaggcatagcgcttccggcgttgcggagcgttaccgaagtagcgccggtatcctgttgcaggtcaagccggttcaccggtgctgcgccagaaagcgtgtaggctttgtcgttaatagtaaccgcgccggcttcagcagggccgtacagtatggagacctcccggaatttgtcgagcaacggttttttcacaggagaatacttcacccagctgtttccgcccggataaaaggtatgccctgataaacccagggtaacgttggatggtggtgaattcttgtagtgataatctttccagtcggttgaaaaggtatgtgtaatggtagttctgaaagatgctaccacagaggttacgggaacaaaccccacgccgccgccgccgaagtaatgttgcaagctgtcgcgcaggtcgccggtaatcaggtcgccttcaatcatggagtctccgaaataggcgatccttactttgcggcgtttaccggctttcagttctttgagggcagcgaggaattgtttcattcctacaatggagtcgccaggtacgggggaagcgtattccatgatacctgtatacgacataaagtcgtgggtatggtctggattaggcacatgcggattagcgccggtgctgtctaaaccagaaagcttactgctgtcgttgccggctgcagtaagcttttgttggtccggggaagtagcatttgttctcagatctgacaacatatccagcttccggaattgaaagtctttgtatgaaaaggtgtaattgagctgtgacagccctactacgcaaactaaagttccaagaataatatagaacggataggcagacttatttttgccggacatagtttatgatctgttgcacatcactgatcgcctgctgccggcatgcctacggttaaccatttttctgattccgttgccacgctatccatacctgcgtccagcttatacaatttatagcggttaataatatttgtcactcgtctgatccattcatggccggcagatgaataaccgctatggttcattttcttgagccacagtgtaaattcggggtttcccttcatttcgccgaaccactttttgcgtgccagtacttccacaaaatgctcataggaagccatgtctgacacatattgtttgtacacggaccgtgctcctggctttgccttggaaatgctatttttccctacaattccaaaatggttgtgcaacaactttgcgtttctacttgttccggtgcctgattccagcatcgctattccgagaataacgcttgccgggataccagtttcctgcattaattctacagaaaccggtttaaatttctttaaataactgtttgtggattgttgtgcaaacccaacattgctgagcattagcaataataacaccgcacataaccatactgtcctcttaaagaatgttgaaattctcatggtagtattttttgatacaggtgatagttccttctttgttttcagcatcatttcttacctcacatatcaacgatgatcacaccgcaatattactttaaaaatttaaataatacgtcgttctctttttcttatctaacccgttaatctcttgttaaaaaaaattgtacctcatatttgtgtcaatcccctttgatgcggcagttggccatatcaaaggggattttagcgacaaaaagcattctcttttgcaaagaccatgccggcaatagcagcttctgccatttaatcagtggcttattgctttaccaggctgatcttcaattcgttaagctgtacctggtctatcgcagcaggcgcatccagcattacatcgcgtccggaattattcttcgggaaggcgataaagtcacggatactttcactgccacccagcagcgaacagaggcggtcgaatccgaaagcgatgcctccatgcggcggtgcgccatattcaaaggcgcctaacaggaagccaaatttatgttctgcctcttcccggctcattcccagagctgcaaacattttctgctgcaggtcgcgctggaaaatacggatggagccaccacctacttctgtgccatttaaaactatatcgtaggcgttagccttaattttagcgtattgtgaaggatcatccatcagcgagatatgttccggctttggtgatgtaaacggatggtgacgggccacccagcggttttcctcttcggcgtattcaaataacggaaagtctattacccacaacggtttaaagtcgtttttgttgcgtaaaccgaggcgttcacccatttccaggcggagttcgctggctgctttacgggtacgctcttccttgccagccagcaccaggataaggtctccgggttgcgcctgacatttttgcgcccataatttcagctgttcttcgtcaaaaaacttatccacagaactcttcaatgtaccatccgcgttataacggacatagatgagcccgctcatgcctatctgtgggcgttttacccagtcggtcagttcatccagctgtttgcgggtgtactcggcacaacctttagctgcaatcgctaccaccagttccgcgtcgtcaaatactttaaagcctttattctttgcggtatcattcaggtttaccagcttcatttcaaagcggatatccggtttatcgttaccataatattccatggcatcatcgaatgtcatccttgggaaagcatccgggaattcgattccttttatttccctgaagatatgcttcagcatatgctcaaaggtagccaggatatcttcctggtccacaaagctcatttcacagtcgatctgtgtgaactccggctggcgatctgcacgcagatcctcatccctgaagcatttcacgatctggtagtagcgatcgtatccactcaccatcagcaattgcttaaaggtttgcggcgactgtggcagcgcatagaactcattggcgttcatgcggctcggtactacgaaatcgcgggcgccttccggggtagatttgatcaggaaaggcgtttctatatccataaaaccagcggtgtgcaggtagttacgtgcagcacgtcctacctggtagcgcagttccaggttttgtcttacgatgttacggcgcagatcgaggaagcggtatttcatccgcagctcatcacctccgtcggtatcatcctgcaaagtaaagggcggtgttttagccgcattgaggatggtaaaatcgctcacggtgatttcaatatcaccagtgggaatgtttttatttttactggagcgctcggttacggtaccttttacctggatcacaaattcacgaccaagtggctgtgcatccagttttgcgttcaggctttcaccgaacagcagttgagtaataccataacggtcccgcaggtcaaaaaaattgatgctgccaaactttcttactgtctgtatccatccggccaaagttacttcctggcccacctgttccattcgtaattccccgcaagtgtgcgtcctatacatgcgtaaatagttgatttagttagttttatggttgaattacgggacaagtaatcatcaattggcgaccactatccagttgttcacttatacccataaggggggcaaagatacggtttggatcgggcattttatgcccggtgtatgttaaaaatatcgtacgaggtctatttccggcatcagtggcgcatcagcaacaagcacatccctgaaatgcgccgccataaaaggcgccagcgagcatccctttgtgcctagcccgttaaataagcccacagacggtaacgcagggtgaaaacccgctattggtcgccggtcgtttcccgatggccgcaccgacgataactggtccactatttcataagggaccttcagcagctgtgcgaggcttttttccagcacttcccgctgctttgccgttgggtggtcatcctcgtaatcccatacgaaagaagaccccgcccagaacaatccattgtcctgcggcaccagcgtaatacctttctttatgatgtccccggtttccagcccaggtatcttcaccagtaatacttctcccttattgggtaaaaattttatctccttaaaaaaaggaagcctggtagtacctactccatcgcagaagataactttagcggcggcaatatctttataggtaaccccatcttccgtaatttccaggtccgccacatccaggtgagtttccagcagcgcctcctgtgcctttaaatactgccggtaagccggcaacaatgcacggaggttcaccgtagcgccatgtacaatggctgcaccatggggctgatccaggaacgcttcatatttcagtgccgctggcagctccgtatattcattgccggtagtcttgtttaggaaagcttcccgcatttgcagcgaagggaaaaccgtccacagctgacgttccgtgaaaaccggcacttgcagcagatccgacagcgcagtgtatgtagcttttgcgaaaggataaatggtatcatacatccaggccggttcaaacctgcggcccgataccgggttcatgatcccgccagctaccctggaagcgctgtttggctttgcatcatcaataacaattacttttttccctgcctgcaagaggaaccagcttaacatggttcccgcaattccctgccctatgataaggtaatctgctttcctcatagcctcaaaattagcaataaaaaaagggctgatggagatgtccaccagcccttctgaactatattactgttattactcggttacttttacattaaggccgctgctatgtgcggaaaattccggcgcatacatacactgggcggtactgataccgttggaaaatttaccctgatgggtaacaaacaatgtatattcaaacacataagttcccttgggcagataactgaaaaagaaatctgtagaggcatcccgggtgctttcataatagctcaatccatcctgccacttgctagcgctgattacattggtaggctcaaaacaagccgcccgcatgtctttcaggtgaatgtattccatctgcctgtcggcgcgcagcacaatccgcacttttactttgtctcctactttcagttcgttgccatcggtgattttagtaagtaccggtcctttgtcgctgttcacttctttgaacagttctttttccagtaccagcggcgtggcggcagcagtaattttatccaggtcttcaaagtattgccagtacacggcgccccaggaaggctgtcctttactgtcgctaacggttacgctgatgttgcccatatccggcttcacggctttggcgtctatcctttctttaaaatagccggtaccggcttctttggcagcgggtttcaccgtagtatttccaagttgaatggatacttcgggagaagcagccagccagttagcgccctgcagcagcatggcgtagcaggcgtctgcggtcgctttggtggtatgccagttattagtttgcttgtttttcagcaaccaggttttcatatctgccactgccccggcgtcttttcctgctacctggaaggcttcaatcagtaatgcctgtgtttcaataggcgcctggtaccagttgtaaccaccggttacatctttccaatacatacccatctctttactgttcatggcattttccttcagcgattttaatatagccgccggcgttacctggtcattctttttgaactgcgataatgcaatcatgccctgtgcataacggctttgctttgtccagtatttctgctgctgggcgtagtaaaagtcaaacgacttcttcatggcagccggtacgggtttgtcgaagaagctgcgggcatacaggtagtggatctgcacctggttgatctgctcctctttcaggttagcctttgctttgatcaatctatagtaatctgcatcgagctctttatcgaggtagtcgatggccttcatggccattgcggtagctgccggatctttttctgaagtcagctgctgcaaatgacctaagcctgcaacaatatactgtgtaaggaaacggtctttccacatgcctgtaaaccatgggaaagcgccatccggcaattgtttcgctgccagctgatccaacgctgattttctttccttctgcatccgttgcaggtcgaacagcagcgcgatattctttttctgctgcgcttcattttttgcttccagcacccacggcgtttgttgcagcaacacggatttcaactcttcgttctttgccaggttgctttgcaatgcggccgtatcggtgatcttccatttatcaaagatggcctttaaaccaggagtagcattggtaatgtgtgtagccaatgcgttggcataatagcggttaaatacctgctcagcgcattcatacggaaattccatcaggtaaggcaacgcctgtacagcgtaccaggcgggattactggtatattccacggtaacgccatgctgtacaattgtttcggaagaatcgctatgcagtaatttattaaaggtaaagtcgtgtttaccatcgccgcgaaccggtaatggaagcgattctgtgaccagcatccggttggttaacacgggcaatgcattttcttctccatcgctgaaattccctgcctgggcagtaacccggtaaatgagcgcgctctggaacccgtgcgggatctggatcgggaagcttaccacggtactttgtcctgctttggccgtaaaatgttgcagcgggaaaatgttctggaaccatccatccaccggttgcatggtagtagcatccagcagttccaggtgtgcctggcctatcagctgggagtccgacaggttactcactttagcggtgaattccattttatctccttcgcgtacaaaccggggcgtattgggctggatcatcagcactttctgtgtaacaatactggcgttggtataaccgaaggccagatcctttgtatgtgccagaccctggaagttccatttggtgagggcttccggaacagtaaactcaaaggtgatattgccgtccttatccgtgcggagatcggggaagaagaaggcagtttcctggaagtttttacggatagcaggagcgattggctcctcgccgcctgccggcgctttttctttggccgattgggtgtcaacggctttataacccatggcgtcgtcggccattgctgctgccggggctggcgccatttcctgcagggctacaccgggcgcgaagccacctaccggggcagatgctttcattctttttgtagtggcagccccccgtatcatgatctgtcctccgccggcgccgtccatcatgttccagtcgaacaggttcagcatttcatagttcttttcctccgccggatgtacttttccatcacggtcatacagtcctgtagacacatccattttgaaattctcccccccgttaaacctcaatatattatttacataagggtagatagccggctggtaccatttgtgtggcacaaactcatccagggatgcatcatacatggaagcaagcatttcggcggctgctttttcatttttatacccggatatctgtgcggtccatttttctttttctcccggtaataatttatcgcgatgggtacccagttttatctgcaggtctttattgtcccaggcaactgttacggttggctcaacggtaaacacccggttatcttttacaaacacataggccagcgatatatttccccggtcattttctgtaacgggaaaatccagctgcttcacaccggagagttccaatgtggaaagtacttccggcgcaattaccgttttctttgtttgaatcaggtgcacgctacctgcagaagaacctagcaggatggtggccgttttacccggcgacactactgcagcagcaggataggaccacaaatatacaggcgctggtaacgttttcggatgagcgtctatcaactcgaaggttgttttctgaacaaccagttcgttgtttttatcttttgcacttacttccagttcataaaatccaggggccagttttttggtatccagcactactttcccttcgggattacctttaaccgtttcctgtagaactgccgcctgacggggccagtttttatgatcatcttccgatttatagatatctatcgggaacgcctgtacgtaactggcttcgtccattacaaactgatcgggcgcttcccagtagcggggacgcaacaggcgcttgttgggagtgagcggttttatctgcaccgtaaggttagctggttcaaatgcgccgttcaggttgcgggaataaatccttacgtccttgaaatcatcccgttgcaggcgagccggcgtgtttaccacaatttccatcgactggtagcccacacttactgtttggtcgccactgcgggtttcgccgttaagatctgttacatcggcatgtactacgtaggtaaataccggtttggtggcaggatctacggatttatcgttgagcgcgggaaactgcacctggaaggcgccattggcgtcggtagttgtttctccatgaacaatttcacgggaagaaccgtacggagcggctatcttgtaaaataaccacgggtaaggataacgtacccgccgctctacgcggtaggtgactttggcgccgtcgatattattacctgcaaaggccagggcttttgcactggcggtaacggtgtcacctatacgataagtgctttttatggtatcaaactgcacatagaattttgggcgtttgtattcttctacctggaaagcgaggtatccgttgcccacctcatctctcaggctgtaaccaccgttcatgcggccttccggcaatataaacgtcccggaataagcgccgaattcattggtggttactttaatcgaatccgctttatcgccattggcgtcgtacaacgacaaagtagttttgtaattagtgagtatgtcactgccggtttcgttggtgcgtttctttaaaacaattcctttaaagtagatggtttgcccgggtcggtaaatgctcctatcggcaaacaggaatgtttgagccttgggttcctctttccgctcatagttggtataatagtaacgatgtgagtcgatatacagctcatcctgaccatttttccaatgcaaccgcaggttattattttgctttatgggagccggctttacgcggccatcgttgccggtagtaaggttttccaccagcgtccattcttctgtattgttgttcttatttcgcagcaactgcaggttgataccagccagtggcttaccggtggtacgatgcaaggcataataggtagtaccgttttccacatagctgatgttggatacccaggtcatttgcatggccataggattatttttcagtgcaaacttcggatcagcgctggacaacagcatgtaatggccggttggcagcgcatctattttgatttccgctttgtgagtgatataatcctccggatcgggcagggcctgttcccaggatttgatgaccgggcgcgacagcatcagctgccagtaagtattgccctggtcgcggtagttactctgcgccttgcgtaacagcttcaggaaggtttcatctattttaaaaacacgcaggtagatcttattaatattcttatacctcaccagtgttctgaacggcagctccggtacattcaccgtttctgttgccagttccaggaattgctcgttaatctggtccagcatataagcgcaggatgcgccaccgcccgattccggcgccaacgccaccgccttttcgcagatagctttcgctttccgcatattatctcctttcccgttttccgtgtcatctgccttttgcatataataagatgcctgcattaccattacagtggtcacctctttttgcccctcgtaggctaatgccatctggtcgagcgcctggagataaagcgcctctttattttccattactgccaccaggtttatccaggccattctttccacatccacatccagtagggcggctttatcgccggcatgcaaacggatcagttcctgcaggatcagcagggcttgatattgcagggaagtgctgtcggcgctggtgaagtgatgtgccgcaaagctagcggcgggcgcaaaggcagcagggtccgtaagttcaaactggttggcggggttggtaatggtagcttccccggatttaaaataatccagggcgcggtgagccagcagatcgtacagggttggccgcagtggccgggtatttcctttaacgataacgggttcaaaggcaatgaggcttgttttttccagtaattcccggtcagacagcgacgcctggtaggcggcggtaatttcctggtgcagccggtcggctccccaggtgcttacatctgttccttcatcgccggcgatggcggtgcggttgtagaaccggtaccggttattctgaaaataccggtacagcatttctgctttgatgctttgcaggatggccttctgcgcgccggcagcagcggcgatttccgcgtccattttctgcatattgagcagggtgctgctgtcgttgatctgcgcgttgtacttcatctggtagatgagcgctttgatttgctgtgccgttgccttgtcttttacggcgtgggcataaatatcgttgactacttccagggctgatttaggtaatcccttatcttccagtgttgtaattttcttccaggagttatcgtagttgaactgggccatcatcttattgttgctaaagattaaaacaatgaatattccgatgaataaacgcatatgggatcgttatttacagtaagttaattcttttactgaaggatgccggtgcaggcatggtttccataaaggggaacaaaaaaggtgaaaagtgttggaataaatccccttcacttttcaccttatatatttttaccggcagataattatgccagggctgcagttttgcttaatacttctgccattgttttaccaatgttagcaggactttccactacgtgaacaccacattctgccatgatcttcattttcgcagcagcggtatcttcagcaccaccgatgatagcaccggcgtgccccatacggcgtcccggaggcgcggtttgaccagcgatgaaaccaactacgggtttagtaccgtttgctttgatccactgggcagcttccgcttccatgcttccgccaatttcaccgatcatgatgataccttctgtttcaggatcattcatcagcagttctaccgcatctttggtaggtgtaccgatgatgggatcgccgccaataccgatggcagtagaaacgcctaagccggcttttactacctggtcggctgcttcataggtcaaagtaccggatttggatacgataccgattttaccttttttgaagataaagccaggcatgatacctactttagcttcatctgccgtgataacgccagggcagtttggcccgatgaggcgggtagttgtaccctgcaggaaattcttcgccttgatcatatcctgtacaggaataccctctgtgatacataccaccagagcaataccagcttcggtagcttccatgattgcgtcagctgcaaatgcaggaggtacaaaaatgatagaaacattcgcaccggttgcctttactgcatcggctaccgtattgaacaccgggcgttccaggtgtgtgctgccacctttaccgggtgtaacaccacccactacctgggtaccatattcgatcatctgtgtagcgtggaaagtaccttctgtaccggtaaatccctgaacaatcactttactatccttattaactaaaacactcatcgcgcttgttttattggtttaatattatatgtctgattcttctggacggcaaaaataagccgatttccataattctgcaatttagtgcctttaagataaagctaccaattggtttggaaaataattggcaataaataaggagagtacccgggcaggtagtgccaataacaacagatttaaatactatatattatctttttaactgacaatcatatacatataaacattactgttctccctgttcctttttcagctgatcccgccactttccatctttaaataattccagctgccgcatttcttttgcttcccgcaggaactcggaggcaaaaatgaagtcgtttaatttctggtccttgctgaacacgatatctttattgctaccctcccactgtttctggccctggtacatatatacaatatggtcgccgctttccattacggtgttcatgtcgtgggtattaatcacggtagtaatgttgtattcctgggtgagttctgtaatgagcttatcaataagcagggaggtttgcgggtccagaccggagttgggctcatcgcagaaaaggtatttcgggttgagcacaatggcgcgggcgatgcctaccctttttttcatcccgccgctgatttcagcggggaatttctttgcggcttctttcagctgtaccctttcgaggcattctgctaccctggccttcttttctttcagcgtgccttttccaaacatttccaggggaaacatcacattttgttcaacggtcatactgtcgaacagggcggaaccctggaacagcatgcctatttcctggcgtattacctttttctctttttcatccatggcggtaaagtcctgcttatcatacagtatctttccatcatccactcccatcagtcctacgatgcacttcatcatcacggttttaccgctaccgctggcgccaatgatgagatttaccttaccgggttccattatggttgatacgcccttcagtatttccttatccccaaaaccctttcttatgtcttgcagttcaatcatgattacagtaatatggccgttaatgcgtagtccatgaataatatcagcacgcagcttaccaccacggcagtagtgctggctttacctatttccagtgcgccgccggttacgttatagccgtaataagctgatacgctggcaataataaacccgaaagtataggatttggccatcgcaaaaaatacgttgtatgccttgaactcctggcggagcccctgcataaactgctcggaagatataatgcccgaaagcacgcctgcttccttgccaccccagatacccaggaaacccgcaatggctaccagtaccggtatcatcagtatggcggccataattttaggcgctatcaggtatcctttggtattgatccccataatttccagggcatcaatctgttcggatatccgcatgttacccagttccgaagctatttttgatccgattacgcccgccagtacaatacaggtaagcgttggcgcaaattccaggataatagtatctcttaccacctgtgcgatggtactttttggaatgataggacttaccagctgataggcggtttgtaaggtagttacccctcccataaacagggaaataataaatactatcccaaacgaccctacgccgatatccacacattgctgcataaattgcttccagtacatcttcatgttttccgggcgggaaaacatgcctttgagcatgagcaggaagtttccgaaatgatagaagaatttgaactccataactgatcaaagataggaaggattttttcaatcatatcctaatttaagatttaatgcagggcttagcgtaaactacttaccagcaaacgcttcaaactgcgttcaatgatctcccccattgttttacaacgggaaaatacggcatcatgataatattctgccagctcatcgcccagctgctggatcttttcggggaaagaaacgcggtcggtcataattacatccctgaggtctttgatgcgatgccgctgcactttaatacggcgggcaattaccgcacgttcttcctgctggtactgttttaccacttcggcattgagatgtttaatggcaaggtctacaaatatccggttctctttgaagtactgcggcatatataaagtacgccggccttcgtaaaactgctgatcaaaatcaatggcacggatacggaactgtacatcatcaaaatccggggtaatatcaaaaatgaaattataggaacgcatgtcgcccagcaaccgtacaaagcaccgttcattgaactttacaaattccttggcaatacgtttcgggttaaattcgggcctgttcaggtagtgaagaataaactgatcaccaggcaccccggcaatatgttcttccacgagggtattaccatcgatcagaaagttcatccagtagggagataaaatatgctccagttccaatccataaatacgggaggcatcggcgatcttgatataaaaataatcgtatacctcgttgtaattattaacaatcttaatccggaaaggatgggaattcccaaaggtgcagtagtcgatccgctcaatatgcaggtgctcttccgccgtttggtcgccaccggccttcagaatggaatacacccgttttaaccccgcatgaatggaccctaccatactctgtggataaaaaacggtttcccacaaagtatctttcccttccttgtcgtacaccgatatcgcctgatcgtaataccgcagttcctcgtaagatatcggcagcttcacttcccgctcatacattttaaggtaattgcggaaagcagagttaatcggaaaaaatatcttctttcgggagatggtttgcatgggataaatatagcggattttgtctttctcaggattacgctgattaaactgattagctggatttttactttttggattttttctgatttttagatataataattaagggagataaaagcgaatctccgcttctatctcccttaatcctttataaatccaacagtaaaaatccagctaatcagtttaatcagcgtaatcctgagaaagacaacatccgcgttacttctttttcttcttgtccttcgcgttcttctcgtctctgcagcatttctcctgggcgtctaccacggcgatgtttaccatgtttacgatttgccgtacggtgctgcccagctggagaatatgtaccggcttcttcattcccaacaggatgggaccgatggcatcaaatccggccacttcctgcaacaggttgtaagcgatattaccggcggccaggttagggaagatgagtgtgtttacttcttcttccagtaattccgtaaacggataattatctttcagaatttccttattgaaagccatggcggcctggatttctccatctacaatgagggaaggatcacgttgcttcactatttcgcgggctttgctcatggtttgcgcttccggcgtctggctgctgccaaagttggaatacgacagcatggcaatacgcggtgtcatattaaaatgcttcacttcctttgctaccatcatggtgatatccgccagttcttccgccgttgggttgaagtttacggtggtatcagcaaggaatagcggtccgcgtttggtttggatgatatacatgccggctacacgctttgcgccgtcttccataccaattacctgcagcgccgggcggatggtatcaggatacttacgggtgaggccggaaatgagggcatctgcttccccggtttccaccatcatacagccgaagtagttacgttcccgcataattttacgcgcttcgtagaggttcagtcctttgcgctgacgtttcttgaaaaacaggtcaccgaagcggtgacgcatttccttcatatgttcgctcttcggatctatgatcaccacatcatcaatttcgatggcgttttccagcatcagttcacggatgcgggcttcgttacccaacaggatcgggtaggcgataccttcgtcgttcactacctgtgcggctttcagcactttcaggttatctgcttccgcaaaaacaacctttctcgggtcgcggcgggctttggtaccaatgatcctgaaaagctgattgtccagtcccaggcggtgattcagttcattccggtatgcttcccagtcggtgatgggctggtgcgctacaccgctttccattgccgctttggcgacggcaggtgctactgtgctgagcaggcgtggatccagtggcttgggaatgatatatttcggtccgaagaaaatatttctttcattataggccaggtttacgatatctggcaccggcgactttgccatatcggccaaagcccttactgctgccagtttcatggcctcgttaatttgtgtggctctcacgtcgagggccccacggaaaatgtaagggaagcccagtacgttgttcacctggttgggataatcggagcggccggtagccataataatatccgggcgggctgcgatcgctgcttcgtaggcaatttccgggtccggatttgccatggcaaatacgatcgggtttttagccatgctcctgatcatttcgggtgttaccacatttcctacagacaatcccaggaacacgtccgcgcctttcatggcttctgccagcgacttaactttcgtgttggtagtgaattgtttatgtctgtcggaaagatcctggcggtctttgttcaatacaccatctttatcaaacatgataaagttttccggtttggcgcccagtgccacatacagcttaacacaagccatggcagcggctcctgcaccattcactactatttttactttctctattttctttttaaccagttccagtgcattcagcagggcggcggaggaaatgatggccgtaccgtgctgatcatcgtgcatgatcggaattttcagctctttcctgagcctgtcttcgatttcaaaacactcggggcttttaatatcttccaggttaatgcccccgaaagttggctccagcgcctttacagcggccacaaaggtatccggatcttttgcattcagctctatatcaaatacgtcaatgtcagcgaatatcttgaacaatactgctttcccttccatcaccggtttaccggcttcagggccaatatctcctaaacccaatacagcggtaccattgctgataacgcccaccaggttgcctttcgcggtatatttgtaaacgttttctacatcattgaaaatttctttgcatggctctgccactccgggagagtatgcgagggagagatcccactgtgattttgtgtctttcgtaggtatgacttctattttgcccggcctgccctttgcatgataatccaacgcatcctgcttattcagtttctttgccatataaatataagattgttattgggcgtgcaatatacgaagtattgaattaagggcagccacccaaatagtgggatatcctctcataattaagcatgctaaccattaaaattacttacttttacagcgttaaacattcgtaaatatcatgatacaacgcatccagagtctctatctgctattggctgccgccgcaggcgctgctgctctgtctttcgatttgtggagagctaccctttccaatggtgtaaaacaatctgtaaacgcctccagcaactatctcctgtttgtactgtatattattattatcctgctggccctcgttaccatttttctttttaagaaacgtaaactgcagttccggctgacaatatttaatattctttttggttttggagcactggcctatcaatattatgtagtgcagcaaacggcgaataaactgaataccggcggcattactattacctccgcatcttatttgccggcctccttcttaccgattgttgtcattatacttttattcctcgctgccaggggaatttataaagatgagaaactgatcaagtcactggacaggctcagataacacaacattattcccacaaaaaagccattgcctttacacacgtaaagacaatggctttttttatgtacatcattatttcaggaacttcccggtataactttcttttactttcttcagtccttccggcacgccggcatacagcaaattaccgccaccagcaccaccttcggggccaagatctattacccagtcggcactcctgatcacatcaaggttatgttcaatcaccagtaccgtatgtccctgttcgatgagggcattaaaggagtccagcaattttttaatatcatgaaaatgcagaccggtagtaggctcatcgaaaataaacataatatgcccctgcgcctttcccttacccaggaaggaagccagctttacacgctgtgcctcgccgccgctcagggtatcactgctttgtccgagttttacgtatcctaatcccacactgctcaacgggcgtattttgttgcacacatctttttcatccttgaaaaagtcgagtgcctcgtctacgcccatatccagtacttcgtaaatattcttccctttataggttacttcaagtacttcgtctttaaagcgtttaccaccgcagctttcacaggtaagatgtacatctgccaggaactgcatttccacaatcacctccccttcgcctttacatgcgtcgcagcggccgccatctacgttaaaggagaaatgttttggctggaagccgcgcatcttgctcagcggctgtttggcgtacaaatccctgatctcatcatacgctttgatgtaagttaccgggttggaacgcgacgatttaccaattggattctgatcaatcatttccacctgtgtaacatcatccagtgcccctttgagcgctttgtgattgcctaccctttccgcaaattcgcctttcagcttcatcagcgcaggatacaggatctgcttaaccagcgtggttttacccgatccgctcacgccactgatcactgttagtacctgtaacggaaaatcaactgtgatgtctttcaggttatgctgacgggcgccttcaatggtaatcgcttttttccatttgcgtactttcgccggcggatcaatggtaaactgaccgctgaggtatttaccggtgaggcttttactatcttttaagatctgcggataagtgccttcaaaaataacttcaccacccaaatgactggccagtggccccatatcgatgatataatcggcttcctccatcatctgctcatcatgttccactaccactaccgtattaccgagatcgcgcaattctttcaatacggcaatcaagcggtgtgtatcccttgcatgcaatcctatgctcggctcatcaagaatatacatggaattggtgaggttacttcccagtgtgcgggtaagctgaatacgctgactttcgccaccactgagggtattggccacccggttcagggtaaggtatcccaaacctacatccagtaaggttttaatccggtggttaatttcaagcaggatacgtttcccgatctgttgttcaaactcattgagttgcaggttatcaaaccattctttcaggttggataccggcatatctaccagttcggcgatactgcggtcgcctacttttatataaagcgcttctttgcgtaaccgtccgccaccacaatccgggcacacggtgcgtccgcgatagcgggcctgtaacacgcggtattgtaccttatataggttctgttccaccattttaaagaactcgttgagtccataaaaatgttcgttaccagtccagagtaatttcacctgttcatcggtgagctctgcgatgggcttatgcaccgggaaaccaaatttccgcgcagttttgatcagcgcttctttgtattctcccatcttttctccgcgccacggggctacagcgccttcaaatacgcttaaccgtttatcggggatcacgaggtcggcatcgatgcccagcacctgtccgaatccttcacaggtaggacatgcaccgtacggattgttgaaagagaagaggttgggaaccggttcttcaaactgaataccatccagttcaaagcggttcgcgaaatgctgcatctctttaccatcaatttccacgtagcaatcgccttcactttcataaaaagcggtttgcacgctatcggctatacgatgtttatcatcttcctcaaaatcctttgctaccaaacgatctatgagcacccaggcgtcggcgggaacagtgatttttttctgttccagcagttcctctatgcgtaccaacccggtgccttcactaccgggcatatataaacgggagaagcctttctgcaccagtatgttcagttcttctttcacctctcttttggcatgcctgcggaagggagcgagcagtaacacttttgtgccatttttcagtttagtgatataatctaccacatcacttacttcatgtttttttaccagttttccggagatgggggaataggttttacccactcttccatacaacagccgcagatagtcatatatttccgtcatcgaccctacggtggagcggggcgtgcgtgtaattactttctgctcaattgcgatcgcgggacaaattcccttaatgtaatctacatccggtttgttcatccgcatcaggaactggcgggcataagaacttaagctttcggcatacctgcgctgtccttccgcgtacagggtatccatggtgagggaggatttcccggaaccggacacaccggtaacaactaccagtttactgcggggaatggagacgcttacattcttaagattatgtaccctggctccttttatgaaaatctggtcctgtgggctaacttcctgaggatcaattatgcttgtttgtttctttacttttgttgccatgacagaacaaatttaagggaaaagatgttagctcggtcgcttgctttttacacgcgtctgcaatacgctaaaagctaatacctaagcccggaaagctatttttattatttgttttattgaactaatcttctatatttgcataggaccagatctatctcgctggatattccaaaaatcatcattaactaaaaactgttcgtatcgcctaaactctacttaattaaaacaaccaaactggctgtaaagtctgtaatttatttactaacccgcctagttgtagaagtttatgcaagtaatgtacaaattgtgcgatgagcagttgattaccctctttaaaaaggggcattcttccgcattagaagagttggttcaccgtcataaagataaggtgttcacctctatcctgttactggttaaagattcattccttgcggaagatattttccaggacactttcattaagattattgacaccatcagagctgaacgttatactgaaaagggaaagtttttaccctgggcaatgcgtattgcgcataatctgtgtgtggatcatttccggaagatcaagcgtacaccaatgatcaggaccggagatgacaaagacatctttgatgtactgggcttcagcgacagctgtgcagaggagaagctgattacccgtcagagtcacgaccgcgttcgcagaatgctggacatgctgccggaagagcagcgggaagtgattatcctgcgacactatgcagaattaagttttaaagaaattgccgatctcacgcaagtgagtatcaataccgcactgggtcggatgcgttatggtctgatcaatctccggaaaatgatgacggagaagcaaatctgtctatgaggaacccttttttttgcttgccagcaacgagcggccggatgtaatgtccgaccgctcgctattttaggggggtgcggattttgtctttctcaggattacgctgattttaaggattacccggatttttacttttggattttataaaggattaagggagatagaagcggatatattcgctgttatctcccttaattattaaatctaaaaatcttaaaaaaatccaaaagtaaaaatccgggtaatccttaaaatcagcgtaatcctgagaaagacaacatccgcgttaaacgcgttcgaacaccattgccgcgccctgtcctactcccacgcacatggtggccaaaccatatttggcgccgcttctccgtttcatttcatgcagcagggtggctgtgatacgtgcaccactgcatcccagcgggtggccaatggcaatggcgccgccatttacatttacgatgtcgggattcaatgccaggtcacgcatgcaggcgagcgactgggcagcaaaggcttcgttcagttctgccaggtgaagctgggcagctgtgataccggcacgctgtaaagcctttctggaggccggcaccgggcctatccccataatggaaggatccacgccggctaccgccatactttttatttgggccagcggctgaagattaaattgcttcaacgctttctcagatacaattaatactgctgcggctccatcattgatgccggaagaattaccggcggtaaccgagccgccttttgcaaatgcagggcgtaatcctgaaagtttttccagcgtagtatcgcggggatgttcatcttttgaaaaaataacctgctcttctttattaggcgtgatgggcactgcgataatttcatcctgccatttgccggcatccagggcttgcctgtaaagggtttgactccgtaaggcaaaaagatcctgctcctcccggccaatattccattggttcgccacattttccgcggtttctcccatagaaaaaggatagtacatatcagccagttttttattggtaaaacgccagccgatggtggagtcatacatctctgttttgcggctgaaagcaccatccgatttactcattacaaaaggcgcgcgcgtcatgctttccacgccgccggccaggtatacatctccttcaccacacatcactgcgcgggcggcatccatgatggcctgcataccggaagcgcataaacgattcaccgtattgccggcaaccgttaccggcaaaccagccagcaacgcagccatacgcgccacattccggttatcttccccggcctggttggcagcgccggcaattacatcttctattacagcaggatcgagagaaggatttctttccatcagcgccttcaacagatgagccagcaggtcatccgggcggacagtactcaatgcgcccccgtaacggcctatcggcgtacgcaccgcatctacaatgtatgcaacttgcatgtggttgttttggtttatatgcaaataaaacacatcccgccaactcaaccaataaaacatcatcccccttttgtacagaaattcacaaaaaccgccagatataaccctattcccgccttccagtaattgtcgcttgactcatcaccctgccgggcctagttttgccgctgtcattaattctatcaaaaaataaccccaaaaatgaaacaccttagtagcgtggtgtggctggcagcctgtatgctcagcactacacctgtaattgtgaaagcccaacaacccgcgggcgaaaatgagacaaacctctccgaacttttgtacagaccgattaaacccactgccaaaatcatggaaggcacagaaccttcccggcaggtagcaactccccgtggcgccgtaaacgtgagaaatctacgcgccgcccctaagtggaacctggttaccaataacacggcacaacaaatcaatatcgataacctccagttgctgccggaaaaagtgattactgttaagaaagtgaatgcacctctgtattgcacgcctccaacagtaaccatcggctgctgcagctattccatcaaagatgaagtagccaataaaaacctgatgtatgcctctcctgcagcagtgttcagcaacgaaaccgatgcccgcacttttgccggcagcctgtcgccaaaagttccgttcttcctgccgtataccaacagcaaagtatacccggccggcgcatggaaatatgataacggcagcggtcacggctctgtagacttccttaaaaccagcgacgcctacggcgccggcatcgatcctacttttggcgtatatgcttccgcctccggaaaagtggtgaccgccatgtgggatccgttcttcggcaacgtggtgatcattgaacacaaagcggcagacggaacatcctaccgcaccggttactttcacctccgtggcggctttgatcatgatgtggctaatgcgaaagttattaaagtgaatgaccccaatgataaagatgcccgcgataccaagtataaaaaatttgccaacctgcccaacccatcgcagttactgtggggtaccaacgctcaaaagctgaaggtaaaagcaggagataatgtatacgccggccagcaaattgcctgggcgggtaatacgggctttggtggcgccggctggggacttaaccaggatggcacccctaccaatcctaataccggcaacaaccaccttcattttatgctgtgggtgaaaagcccgggtaccggcgccgactggatggaagtagatccttatggcgtgtatgctacctcagaaagcagcaacagctcctgctatgaaataggcgccaacggcggattcaaccgcttctttgcacctttctatccttcttttcataatgtaccagtgcagtatattacccaatactggggctattataccggcatgggcatggcgctgcaaaccctgagcgtacataaatccggtaaccagtacctggcatccggctctttccagcagggacttcccggcgcctggtattgccgcattaacatgaacagcacccagtaccagcaatacttcgacgagtattacggaaaaggatatattccccgccagatctccgttaccaacgacaatgccggtaatccgctgtttaccgccatctggcagaaaagaggcaatgaaaacttcgccgccgtacacaatgctacagacgaagtatatgccgccaaatggaaaacatatgtagaacagcagaaaatgcgcgtaaccgaacacgtagtatactacgcaggcggtaaacgctaccatgccggggtatttggcagcagcaaccccggagggttttacatgtattatggcatgaataccaccgacttcaccaagaagttcgaggaattaaataaagcaggtctgatgaccgtaaacgtaaacatcgaggaaaacgggagccagaataacgtaggtgggctctggtggccgaaaagcaaggcgtactattcttacatgaatatgaccccatccgattaccaggctaaattcaccgacctctctgcacagggataccgcctgttcagggtacagggatatgacaattcctcccattttgccgctatctggatgaaataagccgaatacatcatatataactgaatgccacagctggaaacggctgtggcattcagttttaagggacattctgtcagtacgccaatattacgtatctttgccgttactttccgactgccgtaaggcagccaactgctcaattaatgataatgaagtctgacaataaaaatatccggcatttaagtttaccggctttacaggaatatttcgggtcaataggcgaaaagcctttccgtgcaaaacaggtatacgagtggctttggctgcggcatgccgatagttttgaagcgatgaccaacctctccaaagaattacgacaaaaattaacggagcatttttcccttcctgctgtaaaggtagacgccgtacagcaaagcaatgatggtaccataaagagccgtttccgcctacatgataatcacctggtagaaggcgtgctgattccgacagacagccgccaaaccgcttgtgtgtcctcacaggtaggttgcagcctgagctgtaagttttgtgctaccggttatatggagcgcaaacgtaacctcgactacgatgaaatttatgatgaagtggcgctgcttaataaacaggccctggaatcatccggcaaaaagctgagcaacattgtattcatgggcatgggcgaacccctgctcaactacaagaacgtattacaggccatcgaacgcattacttcccccgacggcctgggcatgtcgccaaaacgtattactgtttcaaccgccggcgtggctaaaatgatccgccagctgggcgacgataaagtacgttttaacctggcattgtctttacacgccgccaacgataagaaacgcagcgaaattatgcctatcaacgattccaacaacctgaaggaactgatagacgcgctgaattacttctacaaggctactgagaacgaaatttctttcgaatatatcctcttcaaagattttaacgactcaaaagaagatgctgatgagctgattaaaatatacaggcaggtccctgctgatctggtaaacatcatcgaatacaacccgattgatatggcccggttccagaaaccggacgccaaaaaagcagaagagttcatggaatatcttgccaaaaaccgggtgaacgcaaggttgcgtcgcagccgtggtaaagatattgatgctgcatgcggacaactcgccaataaaggctgattctataataatatatctactggtcatgtacgcatgatcatcaatcaataataatttatgaagaaaaaacaacctgctaaaaaagggtttggtccatcaagggataacaaatttggtaaaagcgacaaaccagcaggcaaccgcaatcgctcctccgctgatggcgaaaggccaggaagagcatctgcaaaagataaccgcagcgctgacgacagttcctcatcccgcaagccccgttttggtggcgaaagcgccggcgatgaaaaacctgctttccgcaaacgtactttcgacagcaacggcagacctgcccgtaaaaaaggcccggctaccgatagctttggaaatgataaacctcaacgcggcaaacgcagcaccggcagcagcgaagagaaacctccgttcaaacgcagcttcggcgaaaaaggcgaagaaaaacgctccttcggcagaagtgatgataaacgttcctttggtaaaagcgacgacaaacgttcctttggtaaaagcgacgataaacgttcgtttggaaaaagtgacgacaagcgttctttcggtaaaagcgacgacaaacgttcctttggccgcgatgagaaaccaggcgcacgcaaacgtttcgacaaagacgaaaagcctttccacaaacgcagcaacgacaacgactttaaagaccggaaagataaaccagatggcgatcgcgctttcagcgctttcagaagagacggagaacgcccggaacgcgtacgcagcttcgataaagaagaaggcagtgaaagagctccccgcaaacgtacttacggtgcaggagcagctaagaaaactgacgacagcagcgcttttcatttccacggagaaaagaaaaaaggtggaaaagaaactcccagtggcttcaaccgcaagaaattctttgataaaaccaacgaacgcttcgccgataaacaagataaaaaaaaaggcacaaaagtaagaggcgctaacgaccacgaacatacgaacgaaggcaaagaaagcatatttggccccggcgaaatgccgctgaacaaatttgtggcccattgtggtctttgctcccgcagaaaagcagtagacctgatcaaggaaggcaaggtaacggtgaatggcaaagtggttacagaacccgctaccaaagtaaccagcagcgatgtggtaactatgcaggataaaaaaattaccccgactaaaaacctggtgtacattctcctgaataaacccaaaggctacattaccactaccgatgatccggaaggccgcaaaactgtaatggacctgatccaggacgctacagaaaatgaaagggtatatcccgtaggacgcctcgaccgcaatacctccggtttattgctgctcaccaatgatggtgaactggcgcaacgcctggcgcatcctaaacacaatatcaaaaagatttaccaggtagaactggataaaccattgactaaaaccgacttcgagcaaatcattgcaggcgtaaccctggaagatggcgtagcactggtagatgcactgggttatgtagatccgaaagataaaaagcaagtaggcatcgaaattcacagtggtaaaaaccgtattgtccgccgtatctttgaacacctggagtatacagtggaaaagctggaccgtgtaatgtatgccggtcttaccaaaaaaacactgaaccgtggccagtggcgctttctcaatgagaaagaagtaatcctgctgaaacactttaaaaaataactgccgaattacggaatgcgattatctgaacatattatactagaaacgcctgattttgttgtagtaaacaagccttcaggaatgcttacgctgcccgaccgtcatgataatgagctgacctccctgatagcgatcatgaaaaaggcttacggcgaaatattcacggtacaccggctcgaccgcgaaaccagtggcattatcctgtttgcccgcaacgaagcagcgcataaatatttctcgcagctttttgaaagccgggatgtaaaaaagttttacctcggcctggtaagcggccagccaatgcctaagcagggaaatgtgagcgaaggaatcatggagcatccggtacagaagggaaagatggttactaaccgtaaagggaaaccatcttctacagattatgaagtgctggaggaatttggtctttacagcctggtgaggatgcagatccataccggccgtacccaccagatcagggtgcacatgaagtacctggggcatcccattgcggtagatgaattttatggcagcgcacaaccggtgctgttatcttctatcaagaaaaaattcaaattaggcaagcacacggaagaagagcggccattactcagcaggcttgccctgcatgcgtccatgctgatcttcaaagatccttccggtaaagaatatacaatagaggcgccgctgcccaaagatatgagcgccctgctcacgcagctgcggaaacaccgtggtaagcagccggcaggcgaagaataaaaaagaaagggccgtgtaatgtacacggccctttctttttatattttattttaccagctctccggctttacccagattagctgctattgtattcccgttttcaagatagatcttaccatccctgtaaacagccgggcatgttttcccatccctgaaataatttcccggaacgggaatatctccttcccttcccagcttgactggtgctttaaacctgtcaataatccattcaccggttgaagggcggaatacagccatttctgccctgccatcgccatcataatcaccgggaacggggatatcgcccggcacatgttttacctgcaacgggatattccccaaacttgtttgccacaacgaattgtcggtacgaaatatgcctacatccagcataccatccccatcataatctgccggaacgggaatcccgtttttatgcccgaaccggatgctgtccatgccatcaaaataccaggtaagcgtagatggacgatacactgccacctctgcaaaaccatcgccgtcataatctccgcacaccgggatatcgcccggctgaccaagcgccactacttccccgccctgcatataaaacttaccttctgaaggccggaataccgcgagctccgttttgccgtccccgttataatcagccggtgctggaatatccccggccttgccaaactcaatttccttttgtcctgctatcttccataagccaccggaaaagaaggcgatatccgtaagctggtcattgtcataatcgtggtagcgggctaccgtggtatgatgcaaccagggaagtgtaaactcactatccgcatccttttcttcttcgccggtataaggcgaaaatgtgcggacactgatcaggtcttttgatttcgaaaacttcatcaaacgcattaatccatgaccaccttccggccggctttggtagtcagataaaaatgaccggataacattccctgcgtaaccatcctggcgatacccttcgccgttatcccccacatgccccgataaggttaacatcacgttgggataactttttaaccggtcgaacatacgttgggcttgttttgaaaacttcgggaatcccttcctgttggtacctggcgtcttattaaaatgaaggatagaatgactcaccaatatcgccttcctgtcgctgtatttttcgagtacctggctggcccacctgttcattccttcaatatcttccccataagaatcgtactctataaagatgctgataaatggaatgtcgccggcttcaaaaagatcatagtgactatcgttgttatcgccatagtgaccaccataccattttttatctttaaaatgtccgatgccgaaatacttattgtactgatctgttttaccgcttagcggatactgacttttcgtttgatcatgatttcctacggccatgccatacggaatgccttgcggataaccgggttgcggtttttccagcacatacatggatgcagctgcatttacccattgttgcggaaacttttcaccatcgtcagatatatctcccaggtgaatcacatatttgatgttttcctttgctgcattttttacgatccattctgtttgtgcagtaaacatttctttcttcccaccgttcttctccgcggtgtaatactgggtatcagggagtatggcaattgaaaactcgtcttcctctttttgttgtgtattgctaaagctactggtagttaacagtagcaatatacaaaagcctcttttcatcatcatgatgtgttggtttgaaaactattaaaaatacccggggttctggatgatctttggattgagcccgacctcgttttgtggtatggggaacaacaggtgatgctgatcgatcacgtatgcatctgatgaaagatagggtagttgttccctgatttttacgccaaaggtgttgatcacagatattgccttaccacttctgagcaggtctgtccagcgatggttttcaaatgccagctccaccctgcgttcgtgaaaaatagcggcacgcagctgcgcagcatctgtattcgtgtagtcggccagtcccgctcttctccgtactctgttcagtggcgccagtgcgtcggacgatttaccctgttcatttaaggcctctgccagtaacaataatgcgtcggaaaaacgataaattgggaagtcgtcaccagatccggtaggtgattccaacggagcatgcaaatacttttttatgtagggaacaccaattttccccgttgcagacacgtaattgatgatgcttttggcagctgaataattgaaatacctgctggcgtcgtaagtaccttcagcaataccgatagatgcatccaggcgtttgtcgccggattcaaaatcattgatcagatcatcgctgggcgtattccatccacctgtgcccgtattgtcaatagagatacctgttaacagtttggtatccttacttcttggtaaaaaattaaaaggcagcacattaggcgtagctcctgttagtgtaccgccgagaaactggatctcaaaaacagattccttaccattcttattggctggcataaatgcatctgcatagttggcgttaaggtcataacccatagccagcatactgtttaacagcttctccgcgtccgaccattttttctgtaaggcatacacttccgcaagcaacagggtagccgaaccttttgtagcctctcctgtttgcggaaactttgaaggcggcgccaactcggcgatagcgtcctgtgcatcagcaatgatctgggcatatacttctgcttcagttgagcgggccttaaatgcgtcttccgccgtggttacttcttttataaacagtggaaccccaccgtataaccgtacgagtttaaaataattcagggcccttaaaaatttggcctgtccgtccagggttgcttttacctcatctttaagatcactgccttttagtctttcaataatgatattacaacgggagattccggtgtaactatgctgccaggtggcggcaacataagcattagtagaagtattggtaaaatcggagatgttttcacgttccacgatggaagtacccctgttaccaggtatagcctggtaaatggtgttatccgagtgcatctctgaagtaaagtaatcattcacaagcacatctctgagcggcgcataagcagccactacggccgatctgaactgttgttctgttttatagaatacgccgtcggtatacgtatcttccggcgcccgttcaataaagtccttggtgcaggatgttgttgctgcacacaaaagggcaatcactgcatatagctttttcatattttgtcagcgttaaatgattatttaaatgtggtggtgaatccaagagaaaaggttcttggtatagggtaggcattttcatctacaccaacacctgaggtaggatcggctccgcccacatttatttccggattcatccctgaatatcctgttaatacaaacgcctgctgcacagaagcaaacacccgcaggttctttatcattgcatttcttaaaggcacggtgtatccgagtgttatatttttagcggtcaggtaagatccgtcttcaatccactggctgtttacctgccgtcccatggccgtggtacctgatttggtacgcggataaataccggaacctggattctcttctgagcgccagcggtcggccgctgcggctaacagaagacgtgaaccgtccatgttggtttgatacgcccatttagcggcgttcaggatctttccgccaacagaaaaggtcatgtcaatattcaggtcaaagtttttataccggaagttgttgacgataccaccggtaaatgcaggtgtgggatcgccaataaaagtgcggtcgttcacgtcgtcaattacgccgtcgccgttgatgtcctttacttttatggtgccgatatccgagttaccattgggcttggcggtggtacttaaatacttgggggagttggccaggtcggcagcatctttatacaatccttcaaaaacaaatccataaaattcacccagatggtgccctacctgctgacggtaataatcagaactcaccgttacatttctcctgatataaccgggatccacgaggttggtgatcaggtttctgtcgaaagacagcaccaggttagtgttccatttcaggttgcctgtgaggtttttagaacttacagagaattcatgtccccacattttgagttcgcccacattaaaaatgatctggctaaacccggacgatgtaggtatggaacgttgctgaatgaggccgtcggttaatttgcggtagtaatcgtaagtaaaggtgaggcggttatctaatacgcccaattccaggccaatgtcaaactgtttgttacgctcccatctcaggtctttattgggaagccggttgatggtttgcccctgggtaaccacgttattaaagttgtagtaataagtacctatagtggcctgcggatcatagttgccggcaaagaagttattacctgtgatgccgtaactcgcgcggagcttgaggaagttaacgccttttacatttttcataaatgattcatcgctaacaacccaacctgcggctacagacgggaagctgccccactgagtattcattccgaactttgacgatccatcgcgccggagtgctgccgacaaaagatatttccctttataattataattcacccggcctattgttgacagcaatgaataagatcccgcaccactgctgccggtaacactggtagcagcgctcaggtattcaatatcatcgctggtaaaacccaaacctgtaagggtattgctatagctgctgaattcctgcgcagaatagcctaccaatgcttctatattatgatccttaaagaaggttttattatatacgaggtttccttctgcggtccatgaaccgttatcaaccgccgagctggttccggtagtttgcccctgtgtacctgtcaccaaccctgactggaaatacttacgggtttcagctcctttatctgccgccagattagccttgacacttagtcccggcaagaattcatagttcaggtaaacgttgcccagtatgcgcgttgttttataatcgtcgttggttaattcataggtagccagtgggttgatataggccaccataccgggagaagaaacgttgcgagtgtaggtgccatctgcattgtacggacttgccagcgggctggcctcgaagaacctttcaaagtatcctcccaccccatcactgttcagccggttattatgatccagcctgtagctgggcgccaggttaaaacctaatttgagtttattattttcagtagtaaaatcctggttaaaacgcatggaatataacttggtgccggtattgatcaacacgccctgttgctcctggtagccggctattacggtggaggaagagtgttcgcgggccgaccgtaccgtgaggtcataactttgaatgggggctgttctggttaacaatttaaaccagttagttccttctccatactgctcagggttgtcgtaagccgcatgatagtccgcagatactgaatagccaggttcatacttcaatccatcttctgcacgttctttcatgaatgttgcaaactctcttgccgtcatcatcttcggcaacttacctgttggaattttctgtaacccatagtagcttgaaaattcaattttcgcatcgcctggttttgcatgtttggtagtaatgagtaccacaccgtttgcggctcttgatccatacaatgcggtagcggaggcgtctttaagaaaactatagctttctatttccgcagggttgatgttgttgatacttcctgtgatggggttgccatcaattacaaaaagcggctggttgcttgagtaaaaagaggccgcgccacggataataaagcccataccacgtccgggctggccgctggtttgtgacacctgcacacctgctacttttccctgcaactgctgggcaaactgtgttaccggcatatcctgcagggaggctgcttctactgttgcaatggaacctgtgatctcgcggcttttctgtttaccgtaactaaccaccacttctgtgagcttgttatcagccagctgcatggaaaaatcaagcgaggtggtttttccttcttttataacaatgctgttcgatttctgagatctgaacgaaacataagatacttccagtgtatagttgccgggtttaagattgaacgtataatcgccgttagcattgctttgaacaacctggccggtttccagcgccctgatggttgcaccaggcaatggtgctcctttttcatccaccactcttcctgataatttacccggctcctgcggaacaggtttggtatcaatcacaacatagccttctaccaatttataatcgaggctggtagattccaatactttttcgatcaggtattttacggtggaatgatccgaatcaatactgattttttgcttgagacctgccatcagtttttccggcagtacaaaccggatcccgctctttgcctggatagccaacaggctttccttcacgctggcacgatccagcttaacagcaattactttgtccagttgctgggcacgggcatttccagccagcagcacgccaataaatgtgagctgtgcgattaaaagtatacatgaacatctcatcataaacttaattgtgggatgtaatcctttttgcattaatttttgtattagtagttggcccggcgtcagccggaatcgttgttaattcctttcgctttattcttgtgttgccctgggcaggcatactgttttcacaacagcgcatacgatgtccgcatccaattatggacagttttttttaatacatatcgtttgtatattttaaagtttagcgaataacgacttccccgtttttcatttcatagctgaaatggcctgctacggccagcacgttcaatattttatctattggtactttggcatccagtgtcagcgtcattctttccgctgattttgtgtgttgcttaaatgtgatcttcacattgtaccaccgctgtaatacttctgaaatatcattgagtgaagtgttgttaaatgttaacctggcttccttcagatcctgtacttcttccggatcaactgtttccctttttatctcaccgtgatcaaacaacactttttgtccgggtgttaaaactgccagtgatcttgaaaagtcatggtgtatctggtctacctttactttaccagtggccacttccaccagtagtggtttgtttttaaatgcttctattttaaaagaggtgcccaatactttggtttgcacatcgccggtatgaacggtgaatggtttatgtttctctttcgttacttcaaaaaaagcttctccatacaaatagatatccctggtatccccggaaaaattctccggatacttcaggcgactgcccgcaccgaggtataccacgctgctatcagcaagcattatttttgaccgctgtccattcggattatagctttctgcgaaagccacctgacgcccttctttattacttaaataactgatggtataaatacccatacaagccaggatcagtccaatccagatggcagcattcctcagagatagtaagcttgtacgcctggtattcacatatcctattctttcctgcattgatttttttaaatcctcttgccggggatgaacagatttgttattttcaaataccgcccaatctttagcggcatttgccgacaggatctcgtccagcagtttttctgatgcgggatctttcagcaacaggtttaccagccgctcctcttcagcggaacattcacccgctaaaaatttctcaattaattcccggtttatttgtctcgacattctggtttaacagcgtacaaaaggtccctgttaatcatatagggacaaaaaaaatgacaaggggctattcgatgtggaagaaaaaacagaaacataatttaccggggatattattatatagataaaaaatatcatggacggagacataatctgtaacccaaatccaggattatttacctggctgtatagctatttcaggacggaacagtgtattggaagtgtattggaagtgtattggaagtgtattggaagtgcatggggagtgcatcaggagtgcatggagagtgcatagatgctccatggtatacgcaggtttcaggcatgggagaagtaaccgtgaaatattggctgcattatcccgggggctaacctaacctggcattatggttactaagctgctttctgaaatgattcagggaaaacttaatatggttcttcacggtattaacagagatcttgaggtcattggctatttcagcgtgggttaaatctccttcccggctcatttgaaatacaattttgcgctgggggctcagtgagtcgagatggaaatgatatttctcttccagttccctggagtccagttcgtgatcggcaggggtagccacaaaggaaagattattttcaataaacgctatcggcgctattgaaactgcttttttacggatggctttaatcgtagcgtttttggcggctctgaatatgtatggcttaaattcgcccgctatttgtaacgtatgtctcttgtcccatacccacatcatcaggtccattattgcttcttctgcaaagtattcatccttcacataaccaagcgcgtaattgtacagtcgtccgaaataacgatcaaataaagtattaaatgctttgagattgtcgttggtacattcttccagtagctgcttatctgatagtaaacgatattccataaaaatggattgaatgtatttttcagcaaaactagcgtccggcggttgtttttatactacgtgggatgttaactgtgcattaataaactgttacctccatataaactttgatgggagaagtgcaggggtgttccggaactgaaagcaccggcgggtacagggcataaaaaaaacggggagaaatccccgtttcgtaaaaatcaaaaaccaaccattaaaaaatctttatagaagcagccttccggctctttaagtattatttgttgggctgtggtgttgttctcaggtaaggcttaataattttatggcctttcggaaaacgtgcaggaatgtctgctgttggcaccgctgccgtaacgattacgtcttcaccatctttccagtcggccggtgtagccacgctgtatttagcggtcagctgcagggagtccaatacgcggagcacttcgatgaagtttctgccggtagaggccggataggtgatgataagttttatcttcttgtcgggtcctatgataaacaaggatcttaccgtaaatgtttcagaggcatttggatgaatcatatcatacaggtttgccactgttttgttttcatctgcaataataggaaaagttacgtcacactgttgtgtttcattaatatcatttatccagctcaggtgtttatccaatggatctacgctgacagccagtactttagtattacgttttgcaaactcgtcctttaacaaagctgttttacccagttcggttgtacatactggtgtaaaatctgcagggtgggaaaacaagataccccaaccttcacccaggtaatcgtaaaaatctatttcccctaaagtggtattggctttgaaattaggagcagcgtctcccagtcttaaactcatagcttacgattttaattgaccaaaaatagcattttcctacaaaatttatagactttaagggatttttttcagaattttgcggtttttttttccggggcaaaggatttgggggctaacaaacaatggaaatcaggggttaattcaaacgggataccagggctaacaccaatggatatcaggggttaacataaatggatgcaaggcatggcggttaacgtaaatggataccggggttaacataaacagatgtccgggaattaacatacatggacaccggggctaacataaagggatgctttttcatcaatgtgcgtctttcagggttaacgtaaacggattatcagggttttcaacagataaaaaatatggctaataactatttaagtatttgaggtatacagctgccaggcataatatgccatactgaacttattatcatcttccagtgcggccattacccgggcagcgttttcccccaattctaattcgataaaaccgagatacaggttatatgcgtcatgaagcatctggatacaatactccattttctcattggcatcgtttgaattgtaccgggctgcaggcggtaaggtaggcagggtgggtaccggcatctggatcacacgttctatataatagcactcttcatcggcataggcctcccagttatcatcctgctgcaaacagggcctcctcatgtgaaatacgaggtggtcgaataccacggctccacccagctctgcttccaggtcaatgatgtccggtgtgcggcgcatgtcttccagtttctttacaatcgtcatctgcaccgcatcgtgcttgtcctggctgaaacgcagcatggtgttcattacttcgtaagtagttacaaaatcgcagggataccacacctcatccagtagcgcctggccccagagcgtcaggtaattggaatcatccataatgatctgcccaattgaaatggcctgtacctgcgtaattgctgtagttgtatttaccttattcataaccatcaggttttaataacactacaaatttaccgacgccgcacgcaagggatttgcgtagtgatcttttaatgatattttttttaatcctcgtcgcaaaagcgggaattgtttatttttattatctaaattttatcttttgccaaagaacaaagacgcggtgtcgcgctaccgctggatcgacgagcggttgcgcagcaagcagaagcccaaacctaccctggataacctgattgaatatgtatcggacaagatgggcactgcaatttctacccgcactatccagaaagatatccaggatatgcgccaggaccctgaactgaactatatggcgcctatcgtttacgaacgtagcagcggcacctaccgctactcagacgatagcttttctatcagtaattcccctattgaagaagcagatctccaggggctggaaattgccattggtatactggaacaattccggagcctcccggtggtacagcagtttgaagatgccatcctgaaaattgccgccagcctcaaaatgaaccgggaagccctccagcataaaggactcatcaaatttacccgggcatcccactacaaaggcgcagaacatatccccgaaatagtagacgccatcaaaaacctggaaataatccgcatcgcttatcagagcttcgaccgcgatgaacccaaggagcactgggtggaaccatatcacctccgcgaataccagcaccgcttttacctcatcgggaaaagccagcaaacccgcggtggcgcagtggttacctttgcgctcgacagggtggtgaaactctggcccaccaataagcattttgatgaaaagaattttgatgaagccagctacttccagcatgcagtaggcattaccgtacacgacggagatcccgaacatgtactgctgagctttacaccacggcagggaaaatacatcaagtcgcagcccatccatacttcccaggaaatagtggaagacaacagtgatgaatgccgtatatcccttaacgttgttattaacccggaacttaccatgacgctgctcagctatggcgcccaggtaaaagtgctgaaacccgcacacctggctaagaaaatggctgaagaagccaaagccatggcggcgttgtataaataatactgtagcccgctattgcgcccgcgggcgcaatagcgaaacaacctcttaaggatttggtttggtaaacaaactatctgctaccggctgattcgtttcaattttcaggatattgattttaaccccgccaggatcctgctctgtaacacccggataagtaagcccctccggcgttttcttgtaatcagacaacaacgttaccagctccatatcctgtccctgtacattcatatgattggtagcctttaccagcagataagttttcgcatccaggtaggcaatacccgatgttccatccgctgccgtgatcttcagcttatatgccggcgacccgttcaccgaatccttccccaataactctatctttttacctttgttcttgtaatcatacagctctcctctcacatccagctgggttttcatcagcttcagcatttcaggattcatctcctgcggcgttgtttgctgcatcaccggcatcaggctccagcccgcattacgggttactacctgcacattgctggtgccattcaccgtaaactccagccgcatggcttcatcctgcttcacccaccgctttataggaacggattgcccctgtacttccatatttccctctacatactgcgacttaattccttttaacttcgcctcacctcccatcgccacaatattctttgcgatcaattcatctgcagattgcgcgctggtgcaataaccagcgatcagtaaagctgctaacaatgtataaaacctggttcctgtcatcataaaaaatttgtttttccctgataaataaaaatatcctaagcacatccggcatctctttccaaaaaatacgccagcattgaaaatacgacctattccttagctttgcaacatgaatacattccagatctcaggcaacctggtagatatactgcaacaggaaatatatccggctactatacatattacggatggttatatcagcagcattgaacgcaacaataaccaatacaccacttacctgctccccggatttaccgatgcgcatgtacacgtggaaagctctatgctgatcccttccgaattcgccaggctggccgttgtgcacggcactgtggccaccgtaagcgacccccatgaaatagccaatgtgatgggcgtaaaaggtgtggaatacatgctcgaaaatggcaggaaagttcccttccggttcaacttcggcgccccttcctgcgtaccggccaccatttttgaaaccgccggagcggtagtcaccgtggccgatatcgaagctttacttcagagagatgatatcaggtacctgacggaaatgatgaacttccccggagtactgcataaagacccggaagtactcgctaaaatagccgccgccaaaaaagccggtaaacccgtggatggccacgctcccggcctccggggtgaaaccgcggcagcatatattgccgctggtatcagcaccgatcacgaatgctttaccatcgaagaagcgaaagacaaactgcaatacggcatgcatatcctcatccgcgaaggaagcgctgccaaaaactttgaagcattgtacccgctgctgcacgaccacgcctcacatattatgttttgcagcgatgataagcaccccgacaaccttgtagaaggccatattaacctgctggtaaagcgtgcattagcttatggcgttgatcttttcaaagtattaagagccgcctgtattaacccggtactgcattacaaattagacaatggtttgctccgcgtgaacgaccctgcagattttattgtaacagatgacctccaaaactttaacattctcgccacttatatcaatggcgtgaaagtcgcggaaaacggacaaacgctgataccttccatcccttcatctcccgtaaataattttatagcagacccggtaaccgctgccgattttcgtatgcccgttaacgatagcaatgcaaaagaagtaacggtgaaagtaatcggcgctatggatgggcagctgatcaccaatgcccttacagcggtattgccggttaccaacggcgcaatagcaagtaatacccaacaggatatcctgaaacttgtagtagtaaaccgctataaaaaagcgccgccggccatggcatttatccatggcttcggcctgcaagagggcgccatcgcctcttctgtggcacacgacagtcacaacattattgcggtaggtaccgatgatgaaagtctcgctgcggctatcaataccgttattgcagcacagggcggcatcagcgcggtggggaataatgcgacacatggacttcccctacccgtagcaggactgatgagtaacctcgacggatatacggtggcagcccaatacagtgcgctcgacaaagccgcaaaagacctgggatccacgctggcatcaccttttatgaccttatcatttatggcgttactggtaataccgcatttaaaactgagtgacctcggactcttcgatggagatagttttcaatttacagcaacgcactagcgcataaaaaaagcagcggttacttccgctgctttttttatagcaataatatgaggttaatgggtggtccacagcgcgccgttaatagagtcgcgggaagccccggtaaccccgctcagcacattatcctcctgcctccagcgtaatgttccgataagcgccatgatcaacgcctctttgaaactaacggtttgctcatccggcacttccacggtaattcccaatggctccagctgttcccggatcgtattcaccaggaaagtattaaacgcaccgccaccggtcaccagcatcttgcctggcccctccggcatttgtgccttcagcgcttttaccgccccggtgatctgtaccgcgatatgctctacataagtgcgcagcttaccctgcacagaaatgcgcaaaggcgctatcagcggcaatatggtatgggtaccaaaatcgttcgccagtgattttggccacggtctggtgtaataatcaagttgattcaactgttccaacagactgttgtcggccacaccaccggcagccagtgcgccgccatcatcgtagggtttattcagcgctgccgccaatgcattcaataccctgttggcggggcaaatatcaaacgccacaaactgttcgggcagctgcgccgaaatattggcaataccgcccaggttaagccagtactgatatcccggtaacaggtacttttcgccaatgggaacaatgggagctccctggccacccagggctacgtctaccgcacggaggtcgttgataacaggtaaccccgttactgctgcaatggccgcaccatctcccagctgggcagtcatttgctgcgcaggcatatgaaaagtagtatgaccatgcgatgcgataaaatgaattttatgatccagctggttcttttcaatgaaatccaggatacgccggccggtataatggccgtatgcagtatgtaacagcaggtaatcctttgccggcagggaagtggcctgtgccagctgctccacccattccggctcatacggcaggctttcggaggccttgataacataggtccattgtccgcgtatctcggtcagttctgcaaaaactatatctaatccgtctaatgagctaccagacatggtgccaatcacgttatataccatcgacaaaaaatttcagcaaaggtagttttaaaatatttttttaacgatttatggaatcaggatctcccggcacatcctacaggtagaaaaactactttgttatgaaaaaatatctctctttactattgctcagctgcctgatggcatttactgcctccgcccaacaggtgcgggttatcacgggtattgtaacagacagtttgcttaaaagccccctcgccaatgtagtggtacgggtaaaaggcacagatgtattgacggccacagataaaaaagggcaattcagcctgaaaactgccacgggtgcgctaatactcgaaataaacgctactggctatccatcggtggacgtagccgtgaatgccatgcaaaataaattaaccgtacaattgaccaggccgcagttgtccgatagtcaacacttaacggaagacagggtaatcggggcattgcagggcaaagttgccggagttaccaactcggccatgtcggaagtagtagtgataggctatggtgcgcagcgccggaagtccgtaaccggttctgttaccaggatcaggggaaacaaaatgaactacgcccctgctccggtttacaacacagaggactacagccccattaacgaaaacatcttccactccgccacagagcagccgctcagtactttcagtattgatgtggacagggcctcctacagcaatgtgcgccgcttccttaaccagggcatgatgcccgagccggatgcagtgagagtggaagaaatgatcaattattttgactatcaataccaggcgccggaaggaaaagacccggtagctatttataccgacatggctatttgtccctggaacgccgcgcatcagctgatacgggtagccctcaaaagcaaacaggtggatacccgcgagcttcccccttccaacctggttttcctgatagatgtttcaggttccatgtcgggtgaaaaccggttgccgcttgttaagcgcgcctttgcggttttaacggagcagcttcgcccggaagacaaggtagcgatagtggtatacgccggcgccgcaggagtagtgctcccggctaccagtggcagcgataagaaaaggatcctggccgcgctggatcagttagaggcaggcggctccactgccggcggtgcaggcatacaactggcctacgacattgccggtgaactgtattccaaaaacagcaatacccgcgtaatactggccaccgacggcgacttcaatgtaggggtttccagcgacggagaacttacccgcatgatcgaagagaaaagagaaaatggtatctctctttctgtgctgggttttggtatgggtaactataaagataataaactggaactgctggcagataaaggcaatggtaactatgcttatattgataactttgaagaagcccgcagaacctttgtgaccgaatttggcggcacgctttttaccgttgcaaaagatgtaaaactgcagatagaatttaacccgcaattcgtgcagtcgtaccggttagttggctacgaaaaccgcgtgctggccaatgaagatttcaacaacgacaaaaaagacgccggagatatgggcgtaggccatactgtaaccgccctgtacgaaattatccccaccggcacaaagggaacggccgttaactgggtagatccgctcaaataccaggaaggcaaagtgattggtaataaatccgaagtgcttactgtaaagctgcgctacaaacaaccagatgcccaaaagagcatattgatggagaaggtgttgccttacagcaaccaggagattactgacgcgccggaagatttccggatggccgcttccgtagccgctttcgggcaattattacgcaactccgcgttcaaaggcaccgccacctacaaccaggtattatcctgggcaggcaattccaaaggaacagataccgaaggctatcgcgctgaattcatccagctggtaaaaaaagcgatgctgctggacaaacagtagttccactatttttcggtaatttgcggcctcaaagggatagctcatgattatcaatttaagtgaaaccaattcattggtgggagaatggttaagcgagatcaggaatatagatgttcagcaggaccgcatgcgcttccggcgtaatatggaacggctgggagaagtagctgcatatgagatcagtaaaacactgagctacgaagaaaaggaagtaactacccccatgggcattgctacctgccgggtgctgaaatcacaaccggtactggctactatcttacgcgcagggctggcattacaccagggattgctgcactacttcgataaggcagaccatgcgtttgtttctgcttaccgcaagcataatcacgacggcacttttgatatcagcctggaatatgtgagtactccttctatcgatggacaggtactcatcctttccgacccgatgctggccaccggctcttcattggtaaaaacgatagaacacctcgaggaaataggtaaacccagtcatattcacctggtggtcgctattgcctgtaccgtaggaatcgaatatgtattacgcaataccaaagcaagtttaaccatctgggctggtgatattgatgacgaattaaccgctaaaggctatatagtaccggggctgggagatgccggcgatctggctttcggaaataaattacaacaataacctcgaataatcgttttacgaatagcagttttgtatctttaaaagtacaaagctgctatttgttttttgcaggaccggatcgcttatacatgaatttaatttgagatatgatttaattagtgtaccttcacccgtattgcataataccctatgctttaagcttaatgatatgaaaagagctttactattcctggccatattactttattttaatcctttgcgggggcaggacccgcacttttcgcagttttttgcgtcgccgctaacccttaacccagcgtttacaggtttattttcaggagattatcgtttatccggtaactaccggtcacaatggaggagcatttccactccctttgtaacaggtactgccgctattgatttcggtattttgaaaaacgttatttcttataccgatatctggggcgtgggcctgatggcgatgtacgacagaagcggcggtggtgcgctcacctccagctacctttccttcagcacagcctatcacaaaggcctggatccggaaggcaatcataccctggccatcggcttacagggtacactggtgcagaaaagaatagacaataccaaactgcagtttgaaaaccagatcgacaacaacgggtataaccctatgattcccagcaatgaaacactggtaaatccaaaaatttcctacttcgatcccaacatcgggatcctctacaatggcttaatcggtgaagcatccaatatttacatgggggcttcctattatcatattacccaacctaccgaatcattcatgaaccttacccagaacaggctcagctaccgctggaccttacacgggggcggttctgttccggtaaacgggcaagacaggtttcatgccagtatcctgtacatgaaacaaagtactgcgtctgaattcacctttggtggcgcctatggcttcatgctcaacgacatggacgataatcccaccactttttacctgggtagctggtatcgactgaaagatgccgttatcccctatgtgggcctcgaaataaaaggcttccagataggccttacctacgacaccaacgtatccagcctgaaaccagcctccaattaccgcggtggcctcgaaatttcactgatctatatccacacccggaacgaaaataataaatacaaaacgctctgtccacgtttctaggacaatggctttcctgataaaataattatcctgatttgggagatcatagcaacaaaattgacatgctataatctcccaaatcaggataatcatttaaaatcatgataatcattgttaattttgcgttagtttcgttactctttcataaaaaccaggaaaaaccaattcagttacaataaaatatcaggcgttgttttcattcagagaagtactgtcggcgatccagtcttacgggaaagcccatcaattcatattacagcataaattgtggaaatggatcctgattccgggggtgatctattgcctgttattttttgcaggcttttactttgtgtggggctactcgggcgactttgtagaatatctcacccgcctgctgcatatcacagaatgggtacaggacctggaaagcagctgggtaagttttctttttatacttgtcgcgttttctgtccgcattgtattcgtattctggtacttctcctactttaaatacctgttcctgatagtagcttctcccgtgttttcttatttatctgagaagacagaagccatactggatcataaagacttccctttcagctggtcgcagctgggccaggatatcctgcgcgggatcaaaatgtcgtgccgcaatattgtttatcaaacagccgctatactcatcctgctgctgatctcctttatacccgtgatcggctggctcaccccgatgctggggttctttatcgaatcctatttttatggcttctccatgatggattacagctgtgaaaggcatcgtttgaatatgtcgcaaagcatcaactttatccgccagcaccgtggcatggccatcggtaatggaatggtattttacctgtttatgctcatccccgtattgggctggatgctggcgccctcctatgctgtaattgcagctactattgacttacaaacaaaaagactgaaataatgaataccaccggcaaagtgtacctggttcctactgttttgagcgccgacgccctattcagcattcccgcttatgtaaccgctatcgtgcagcaattatctgttttttatgtagagaatgaaagaacagcccgcaggtatctgaagtcgctggacagaaacatcgtgatagataacctgcaactcctgctgatgaatgaaaaccaggcgcccgacctggtactggcaaaaaaattactgctcgaaggaaaagatattggcatcctcagcgaagccggatgccctgctatcgctgatcccggccacctcatcgtaaaactggcacaaagcatcgatgccagggtaatcccgatgattggccccaactccatgctgctggccctcatggcctccggtatgaacggacaaaacttccagtttgtaggataccttcccatcaaaccacccgaaagaacaaagatgatccgggaactggaacaggaatcggaaaagaaaaaacaaacacaattgtttattgaaacaccttaccgcaacaaccagttgctgaaagatatactggataactgtaaggactatacgcagatttgtatcgcggcagatatcaccgcaccaacggagtatattaaaaccaaaacggtaaaggagtggaagaaacaattacctgatcttcataaacgaccggctattttcctgctgtatgcgggcaacgaataaaaaaaggggaattacgaaaccgtaattcccctttatatttttaaggcagttccgacttcaccggctccttgatagaaataatactgtctacaataaatgcgctgtatcccctccacggaatggctcccaggtactctttgtagtgcagttccaccattttcccgctggccgtcatcagctgctgcgcaatccgttcgctgctcacggaaaactcaaattcgttcgactggatagtaccggctaccttgccccggtagcccgactggatcactttgccttcataggttttaaagatgtatcccttctgcacaaaataattcagctccccggctttaacgccctgtccgaaaacaaaatagtatttatagaagaaaatacctcccagtaccagtataataacagatacaatgataaagacaaaccgacccatagttagtttttagtgatggatgatcagaaattctgatctacaagataaatgaaacccgccataccaaacgcacccaattccagttctcttttattcaccgcttcaaacacatcgttcgccgcatgatggatatcaaaataacgctgcgaatcaggagaaagttcagccattggcgtaccaattgcttcatgcagctggcctacatccaccccgcctcccggttcttcaaaatcataaataccatacggctcaaaaagtggcttccagctattcatttttgccttcaggggcgcgtccatagtggtagtgaagccgcgtggcgtaaagccgccggcatcgctttccagggcgaaaacgtgtttctcctggcgggctttggctagttcagcatatttcttacctccacgggtaccattttcttcattggcaaacagtactacgcgcagcgtatgttccggtttcatgcccagtgctttaaaggcgcgcagcacttcgatggattgtacacaaccggtaccgtcatcgtgcgcaccttctgctacatcccatgaatcgaggtggccgccaaccgtgatgtactgatccagatatttactgcctttcagttccccgatcacattatgcccgatggtatccttcttcatttcgcaattggtacgcagaaacacgctggcactgttatcatctttcaggcgctggctcaaacggtctgcatcttccaacccgatagccaccgccggaattttaggataggcgctgtcgtactgcatcgccccggtatgcgggaaattattggcgccatgcgtcatagatcttacaatcactgccaccgcaccgtatttagctgcccggctggcgccctgtccacgatactttacggcatcgccataagaatgaaatgtttttatgaaggtagggttgaaatgatagttatagaaaacgatcttcccctttacctggtctttctttgtttccaggtcgtcgaaagaagccacttccagtacaggcgcggttacgccatccggtccgctgcccactgagttacccagggccagtacttccagtggtggtataaaatcccggcgtttggagatgatgcgggcttcttcctttgcaccccggatccaatgcggtaccatacactcctggagatacacggtgtctgcaccggccgcttttagcgcctttacgccccagtcttcggctttcaccatttgtggagacccggccaaacggccgcctatctgcttcgtgagaatccgcaggttttcgtaggcagtgctgtgggttaatacttcatccgctaatttcctcaacgtcactgaatccttctcctgcgccactgccagggccggcagggtacaggctaacaaaattggcattatagattttctcattgcagcaggttaatttatggttaaaactactaaaaaagctgaaggagcaaagcataaaggtatctagttgtcaactcttttgtttaactcccctccggctaccgctcatcccacttccctatgcattatgtgatatcgttctgctttttagtacctttgcagaatgcaaaaaattaactcatgcgcataggaatagtatgttaccctacttacggtggtagtggggtgctggccacagagctggggaaagccctggcagacaaaggccatatggtccactttattacatatcaacagccggtaaggcttaatgcatttcacgctaatatatattatcacgaggttcaggttcctacatatccactttttgatttccctccttatgaatctgccctcagcagtacgatggtggacgttatcattaatcagaaactggacctgttgcacgttcactatgccattcctcacgcttctactgcctatatggccaaacagatcgtgaagaaacatggcagaaccgtgccttttatcactacgcttcacggtacagatatcaccctggtgggtaaggataaaacctacgaaccggtggttaccttctccatcaacgagtcggacgctattacggcggtttctgagaacctgcgggaagaaacctataaatcgttcccgatagaaaaggatatcacggtaatctacaactttgtggatacccagcgcttcagccgccgggaactgcctcatttcaggcaggccatagctcccaacggcgaaaagatcctgctgcacgtatccaacttccgtaaggtaaagagagtacctgatgtggtaaagatcttcgcccaggtacgtaaagaactgccggccaaacttttgctggtaggcgacggccccgacaggccgtctatcgaatgtctttgccgggaattggggatttgtgatgatgtaagatttgtaggtaaacaggagcaactggaagatgtaatgtcaatcagtgacctgttcctgctgccgtcagaatatgaaagttttggattggcggcactggaagcaatggctgcccgggtgcctgtgatctcctccaacgcgggcggtttaccggaaatcaatattcccgggcaaaccggttacatgagccatgtaggcgatgtggacggaatggctgcccatgcgatcaaactgctgaaagatgaaaaattactggagcaggtaagacagggagcatgggaacaggcgcaacgcttccatatcgataatatcattccacaatacgaagctttatacgaagaagtactgcaaaaacaggtgcagctgctttaacgggcacgtatccatttttccggattctgtttcaccatgttgcgatatatctgtaattctatttccccggtattgctacctgcacccggtgcggccacacccaatgtttgaccacgttttacagatgctcctttgctgacacggatatccagtaatctcacatagttggtaaaatattttccatggcgcagggttaccatataccctgcgcctggtaccataaataccataattacttccccgtcaaaaatggctttcactgcggcgcccctagccgttgcgatgatagtgccgttgtgatccacatcaattttaccaaccctgccggcgccgaaatgacctgtaacacggccagcatctactggccagggcaggcggccacggtttgcctcgaaatcgcgcgacaagttgagtgcttccggagtggctaccagcgcatcttcactggaagttttagctaccggcgcatcgtcttcttcctcttcttctttctctacttttaccggtgctttcttacccgctttctttgccgcagcaatagcggctcttctgcgggcggcagcctgttcgcgccgccgggcatcagccgcctttttacgggccagcgcctgggccgccgcttttttctgcgcagcagctatttcccgccggatggcatcctggatagccctgtctacctgccgggcttcagctttatttttattgatgcgctgctgtagttcctgttcctggtctttcagctgggcaatggttttatctgcttcctttttatcctccagcaaatctatccgctgccgttgttctgttttcaacgcacctgttttctgtgcccgttgctgctgtaatgcagtcagcttttctcccagcaacgctttggtggatagcaggctttccgcttcccggcgcctgttttcacggtattgctgcaggtattgatacctgcggatggcatcattaaaactggtggcagaaaaaaagaaattcagcacatcatacgaatcacgggttttgtaggcgtacaccaccagctgcgcataccttgccctgagagaatccacttccctctccagcgtttgtacgttactgttagtattgctgatgtctccttctattgaactgatttccttgttaatattaactatctgcgcattgcgggtggagattttttgcagcagctcgcgctgcagggctacattttgccgggtggatttctttgtttgctgcagggatttatttgcttcttctatttctttcaatagctcctgtttacggctttcaagtgccgcgcgcgattgcctgctgccccgctgagcatacaacagcgcaggcaatagccacagagccatcaaaagagggatcaactttctcaaaaaaaatgcatttggttagtaagcgcaaagctgaaagcacccttaaatgctttcagctttatctcgtatagtttcagctatgtttaaattatcttctcctgatccattgctcaggattctgcttggtaatgcctttccagatctgcagctccacttcaccggtattttcaatatcgttggtgctggcagtaccaattacctgccccgttttcacattatcgcctttcttcacacgggtagtttgcaaacgtacatacgtagtaaagtattgtccgtgacgaataataattacatatccagatcccggcattactactactgatttcacttccccgtcgaaaatagatttcacggcgccgcccttattagtggcaatcacaattccatcggatggcacctggatatgttccattaccgcatgctggtgtataccaaaatgctcgatgatattaccggcatcaacgggccacggtaatttacccctgttggcttcaaaactttctgacaatgccagtgcttcgggagtggcttccagcacattttctgtacgggtggtcgctgttttttcaggttccggtgcaggctccggcgctttcaccggaggaggcggtggcggcggtggcgtattggcagcattgctattgttattattggcagccgcagcttttgctctctcggcagcagccagtgcggcagccttgcgggcttcttcttcacgcttacgtctttcttctgcggccttgcggcgggccgtttcttcctctatcgctttacggcgcgcctcttctatttcccggcggattaccgctctaatcgccagctgtactttctgggcatctttcttacgctggttaatatcggttaccagctccttctcacggcccttcagcttattcagcacttcatctttctctttcttatctatttccagcgtgctgcgttgttcctgctccgttttaagtgcatcagaacgcctcacgcgctgcgactccaggttctggatcttctgattcagctgatcctgtgtagacacaatattatctgcctgccggcggcggtattcacgatactgctttaaatactgaaaacgctttactgcatcgttaaaattctccgcggaaaacacgaagttcagcatatcgtaagaggaccggtttttatatgcgtagatcaccagctgggcatactgggccttcagggtatcgaggtctttctgcagggtttttacatcccgtgcagcagtattgatatctccattgataaagttaatctcttcgttgatgttattgatcaaacggctgcgcagcgtgatcttgtcgcgcaatgcacgcagttgaccaagactctctttcgtagacttcttggtttccttcagttgttcgtttgcctcatctatttctctttgcagctctttctttcttcgctccagttcttcccgcgattgttgctgctgcccagtattctgagcaaccaacatggctggcattaaccatagcaccaacataaacgggataatcttcttcaaatacaacatgacttaatttagtaactgcaaattaaataaatatacaacgtttattagtttaatgaagacgacatttacgcaattaacattttacatacgtttatagctggcaggcgtgctgaatgggaaggtgagcggcacatcaaaatcataacgtgtaaagtccagtgcaactttagtcacgttcttttcttcgatgtaaatacggcgcgtagtggggaatttacggccggccacttttgtgtagtctccgtaggtcagctcacaggaacgtttcactgtgccggtactgtctttatccatcactttgctttgctgcaatccgtagtcatccgcaaatacattaaagagactgataaactttgcatgatcgcagctgaaagaaataatagccggcgttttcactacctggtatacggaatccgtaagatataccgggttgccgatcaacatatcctggagggtattaaaatcaaacgggatattcagcaattgctccgcgtccgacatcttccgtaaaaataattgtttatccaggcggttatacatcttcagactgtctggtgtgatgactgccctgatcacttcgtctacaatcggcgcggaaacagatatccatatgatgctgtctttctttatacggaaagtagcattcaggttattatggctcttcttgtctgtttcaaatgccagcttcattttagcggaaaaagtattaaactcaatatgattggcatgaatacctttcagcatttcgctggtaaaacgggtgagttcttcattcgttgaactatcttttcccagggttacccgattggtatcggcggcggggaatgtagtacgggccagctttttaggatggcggcaggccatcattcccaaaccgatcgttataattaaaagtgtgacttctatttttctcttcattgagcgatgacttatagcaaatgcttattgaatatatcttttttcagcgatcttacgggcaaggtctacagaggatgcacccttatctttagccatttgccagtattccactgctttggtaacttctttcagattaaacaggatatcaccgtaatgctccagcacgttcgggtttttctgtgcttcggggtattgcaaagctttctcgatccactcttttgcttctgcaaatttttcctggcggaaaaggatccaggcgtaggtgtccatgtaggttggactttccggttccagttccagtgattgtttcgacatttctgctgccctttcgaggttctctcctcttaacgaaagatagtagctataattgttcatgatcagcgcatctttcggacggagcagtaaggcgcgttcgtagctgctgtccgactgccggtgctgcccggtagcatggtaggaatcgccgagcagggagtaaatatctcccaggaatttcttctccccgttacctatatccaatgcggtattcaacgaattgatcgcagcgggatactgttgcagcaggaagctggctactcctttaaagtagtagcccataaattctttcgggaacttaccggttacactgttgctgagtgccagcaaggcggtgggatcatccttgcgggaatagatccacatcagctgataccacactgaaaaacggctgtcatccaggctcagggcttttttatagcttgcctccgcactgtccagcatgtcggcctgtgaaaacatatcaccccggagcgcatatgctttggcatccgccgggtgcgctttaatgatgagggaagtgaggtgcaatccttcttccagcttggtggtatccgtgttcatcatttgcaggtacggatatacgtaagctactttttcatcgatgctgtaacccggattggcaaatgctttggtaagattgttccaataagtaacggtgtcgttatttttcttcgcgtaagaagccagtgctatcagggctcttggattatcaggatctttagagagaatggtatgatacacttccgcggcttccggcacacggtcgttagcatcgtatatttctgccagcaggtaataatacctgatttcctctggctcctggttaatcagcttctttatttctgtggctgcatcatccaccatgctcattttcagcagcagcttctgtttctggtaaatgagttcttccactatgcctaccttcttttccagctcattaaatgcagccagtgcagaggcgggcttattggcttttgccagtaaaattcctttgttataaagataatcttcgttatcagggtatctgctggtaaggccctcaaaaacataggccgcgctgtcaaatttttcattcaccgcgtaagcgtccgcgagagttacctggaaccaatggttctgcgggtccagcgccgcagcgcgacgggcaaagatgagcgcattaccggcgttttgtacttctataaaaagacgggctaattcataattaacggtgggattatttttattcagccgcagatagtcggcatactgggtaatagccgtacggtagtcacccagcattttagagcgctgggcggcaaaaaagaggctatcagcccgctgtgacagcacagcggcgttattaacggtagtgtctttacgtgatgctgatgatttggcaccactacaggctcccattaataaaataccagccagccctataacggtgaagtatatccgcatttatcaggatttaccggtatgtccaaatcctcccacacctctaacggtttctgtcagcacggttaccggttcaatgaccgcctgaacaaagggagcaatgatcatctgagcaatacggtcgccgggttgtatggtttgcggttcgttggataagttgatcattataattttaatctctccccggtaatctgcatctatcgtgccaggcgtattcaggagcgtaagtccctgtttaatggccaaaccgctacgggggcggatttgcgcttcatatccagccggcagttccatgaataaaccagtagggatcagcatcctttccagcgactgcaaggtaactgctgtttccaaatgtgcgcggaggtccattcctgccgcatctgccgttgcataagctggtaattcattacccgacttattgattattttcacaatgatatccgccattgaacaaagatattttaaaataattatgaatgaagaattactgggtgatatgctccagcagtactaccgcatgcgctgtgaccccttcttcacgaccaacaaagcccagtttttctgtagtagttgcctttacagacacgtcctctgtactcacatgcaggattttggcaatcacggtctgcatttccggcacgtatgcctttattttaggcgcctgcaaacacagggtactgtctacgttaaccacctggtatcccttttccccgatcagctgcgcgcagcgtgctaataatattttactgtcgatattcttgtaagtgttatcggtatccgggaaatgcaccccgatatctcccagggaaagcgctcccagcatggcatcacaaatagcatgtaacaatacatcggcatcgctgtgccccagcgctcctttatgatgtggtaccagtacgcctccaagccagaattcacgtccttctgtcagctgatggaaatctactcccaatcctatacgtatcctactcatatttgtaataatttaatcattttgccaatccgcaaggtaagtcaataaatataaaaatccccccgttttgcggagggattaaagcggataattattttatatcattaaacgactaaatatgtgttaccatcctgtccggctttcctcatctcttggccccaggtcgaatgtgagcgtgaagcgcagtgtgttggaaagcgggttacgttgtattcctgatcctgaaggaaccaggtaagaaaaattaaggccgaagatatcgtacttaacaccaatacctgcggtaaaatatttgcggtttcctttgttcttgttttcgttgaaatagcctgcccttactgcaaactgctggttgtaccagtactccataccaatagaatacatcagttcctgcatttcttccttgatgggggcatcgccaaaggaactgaatattccttcgagtgtacctttctctttatatagtccggcagaatccggggtaggcaccagtaatttattgatatccaaggcaaaggtcagctgattcgcttcatccagtgccaccgtataggcggtaccgatacccaggttggtgggcaggaagtctttattggcggcagaactggtgtaggaaatcttggtacctatattcgtaatggccataccaatgttcaacctgttcaccaggccgtcatctttctcaaaatctttggtataaaatcctgataaatcggctgcaaaggctttacccggcttaatgctaacgctaccgttgctttgtccgccggccaggttggagtaaatataacgggcggttaagccaataccaaaatgatccgacagcttacgggcataacctgcatccagtgcaaattcacgcgggcggaaatcaccggtaggcgtacctgtaacatccgtaaaattgattgttccaagagaaaaatatcttaaggaaccggaaatggcctgttgttcgtccagcttggtatagccggatacggtagccaggaaaacgtcgtttaccagttcttttaaccagggggtataagttactgccaaaccgccatttttttccgcaaatggaagtttggagagattgttataaatagaagatgcatccggcgatattgccactcccacgtcgcccatggctccactgcgtgcatccggtgtaattctcagaaaaggaaccgcggtattgatggtgttggtacgaccatctgtttgtcccggggtaatttgtgctgaagtttgtaaacttatgaaagtaccgtaaatgaacacaaggctcattgttacctttcggatcatgcagattttgtatttgataaggatgtaaaaataatcttatttattaatataacatagaaaggggtttatttgggataatggtaaaaattattttcctgcataggctataataacaccagcttaccaccctttatcttcattcccgtggaagtcttgattgttatcctgtacacgtacaatcctgaggacagttttgctcccgaatcatttcgaccatcccagggcatgccctcaaaacggcctgctgtggaaattattgtgctacgcatagtttttaccagttttcctcctaacgtaaacacctgtaacgtgagttcaagctcttctccctgccggttgtgtaaaaaagaaaaccgtgttacatcatgaaaaggattcggaaagttccttacttcatctacagtcagtactccctggtctgctactttgaaataaatggtggtagcagcaccattgttccgggaatcccatgctttgattgtaatccggtgttctcctgttgacaatccctttaacgggaaaagtacgttaccctttttatagctatccaaagatgccccaaaataatcatttaacacaatatattctgtactatccagaattgcggttagcaggtaaagttcgttattacctgaaatgttaatgccgctgctgtctgccaggtccactatcaacaaaggatcagggcctgtaatatctccactccggaaactgcggctatcgagccaggcatttatcgttgggccgctgacatcagctactggcggaaccacctggccaccggtggtgaaattatcaaaataaccattgccatcctgctggtcgttgctggtataataactgattttccctctgccgtcgccttccctgatatctccgggggccacaaatgtaaaagaaaatctgccaccatttactgtttgtgtaccctggaacaatagattgcgctgcaatttataacccgccacctggctgccggcatcgttgccacgggttttcaacagggccggctggtcatacaccgttgtatacataatgccattataagccggtaccgggttgccctgcgcatcttctatatggccttttaccgtatacaggccgagtcctttcaccgtgtcgggttgtcccgcagcagccctgccgttaatggaatcagtgatcacccggtaagttgggaatgccagggaaagcgccggatcgcccagtaactggaacttccggttattcaccgcatcgccggaactgctgtaggtaaggttcttggccagcatggcagcggcgcccaacgaaggcatacgcccatctgccagtgatgtgaaggccacttttaaataattagcgttcatcaactggttggaagcagaaaaaaccgcgcgggtggtggtcatcagggcaatggcgccgccggtatgctgcagtaatatcttatgtcccaatgaagtgatacccggatcatcatacggcgcaaaatcgcaggtagcggtaataaacaacggcagtttattttcattatgccagtcggctatactacctgcatccatgatgttttctgcggccaggcgggagttactgccatgaccggtatagttcaacaccagcgttcctttattgatctttaaggcaatagccttgtttacctccgggtacaccgggccggaactgcctgtttcctgcggataagcgtcttcatagatcttatctgtattcagcagtttcgcgtcgccggaaaggatggtccccattttttccgcatcatcgaaatgaaggttatcgtcttcatcatcggccagtaaagttacctggttacgccaggcgccaaacgctgccggctgccggtagcgcaggatcttatccaccgccaggcgggcttccgtttcgttgcgcgcaggaatacggccaatgccgatatccagcagatccggtttagccgttcccgtgacatccccttcatctttcagtatcccaaagtaatcgtcggatacatacgaccggatggcatcgagcgaggcttcgctttgccaggaagggatatcgttcgtattattttttacacgttgccggtaatcataggaggcggcgccgaacaacaacaggtaacggggtgcgggtccgcggtcgtaaaacatttttacatagtccctcaccgcggtgggatcgggtgttccggaggcaaactcctggtatacctggtcgatgatggctacctgcaccgacagctgatcggcggccctgtgcatggctgccagccgctccgcctgcggcaggagcgcgcgtgtggtgataatgagcatatctgccggcccttggccatgcagatcctggttgggcaccgttcctgcgaaatcaggcttcccggcggcagcggtgcggaaagcaatgtattcatgcaaccggtcgtttttacccgtaaacagcagggaatccccctgcagggttgttttcatcacaaccgggttcaacgggtccgtaacatcccagatatacgtttgcgtgttggcgttatgtaccgcgaaccggctgggttgcccgctgccggcataacgggtactgcgaaaatccagcataccggtagctggtatcaccggcttacagcgggcctgcacttccaggtaatccagccagcctttatcgttgatatttcccggcaaaaattccacgcctatttccagttccggctgaccggcatctgccccgcctgttgcggcggcggcagtagctaccccttcaaaaatattacctgttaccggcagcaggtacatattggttacagccggcaatttatttatggtggcattgaagttgctcccaacgctgcttcgtgcagatgcccgcatgcttacccatacttttccttctccgggggaaggcaggttaaaccggtagctgcgcgttaagcccactaccttactgaactcctgcccccaccactgtttgccgctattgaggaaatttaggctgtctctttcataaaagtcgtgataatcaaaggtatattcaggcgtggctcccgccggctcatcccctgcggccacccggagccctgttccgccagtggtgatataataccaggcggtatccgcatacaggttccgctgatgggtaaaggttttagtgctgctgttatacagccagcgatgtggtccgggggcgtaaaaaagggcatagtcgctgccattgagcacgccgtccccgccgtcttccacgtgcagggccacttccggcagatcgtcgtaccgcggcgccggatttggttccgccagcatctgccctccggttccaaaaagccgcaacccggcagatgacaacccggtgatccccatactctggagaaaggttacatctattttatagataccgggagcgctgatacctatcttataccagttgcctgaggccagtacagaattttttttatactgccgaaggctgctttgggcatatatttcccgtttccctaaaaaagaaagcaggaaaagacctataaaaatataattgagtttcattaccttaatcgcagtttttcggccggttgatgtagaaagacccttatcagcgggaacgattggcagcaaattacaaattaatttttttcgccataaaataaaaaagagtacatttgcgtttactgtaaatatactagactaaagctgtatcgcatgcgtagattaacctctttatcattgctcgtaggtaccagcgtaatgctatccatgagtgcctgtcataaagacggcgggggacttttcggtaagaagaaggaatcttcttccgctacgggctggaactataacgaccagaaaatgggcggtttcagcgtagcaaaaaacgtgaaccagcaaactggtccgggccttgtttttgtacagggtggtactttcgccatgggagctacggaacaggatgtaatgggcgactggaataatattccgcgccgtattactgtttcctccttctatatcgatgaatctgaagtagccaacgtacattaccgcgaatatctctattggctgaaccgcgtatacggggaatcattcccggacgtataccgcaacgcaatgccggacaccctggtatggcgtagtgagctggcctacaatgagccgctggtagaatactatttccgtcacccggcttacaacgactatcccgtagtaggtgttacctggaaacaggcaaccgactattgtaaatggcgttccaaccgtgtaaacgagaaactgctgatggacaaaggtctcctctccaaagcggatgtaggcaaccagtcagacgacaacacctttgacaccaagtcttacaccgccggtttatacgaaggtacacctggtaaaatgtcgaagggtacgaaagaccagttcaaaaattccgatggtacgcctcgcaatgctgcctttgaagatggtatcatgttacccaactaccgtctcccgacagaagcagaatgggaatacgccgcactgggttatataggtcagaaccccggtccttccaaaaaagaaggcaaacacggggaagagctgatcatgaacaaacaggtttactcctggggaaccaataccagcggcttacgtgatatccgccgcggtaccatgcaggggcagttccttgccaacttcaagcgtggttccggtgataacatgggtgtggccggcggcttgaacgaccgtgcttccatccctggtcctatccgctccttctaccctaacacattcgggatctataacatgtccggtaacgtagcagaatgggtactggacgtatacagaccactgaacccgatcgatggggaagacttcaactacttccgtggtaataaattccagactgtttaccagaacgaaaataaagagttcgaaaaagacagtcttggtcacctgaaaatgcgtgatgtaactgatgaagaaagtgccaaccgtcttaactaccagaagggtgatgtaatcaactacctcgatggtgactccctttcacaggtggaatatggttatggtatcactaccctgatcaatgataaatcacacgtgattaaaggtggtagctggaacgaccgtgcttactggctttcaccaggtacacgccgttacatgcaggaagatatggccactaacaccgtcggcttccgttgcgcaatggaccgtgtaggtagccctgaaggcaacaagttcaaaacaggtaacctgttcaagaaacaacgccagaaacgatagcgaattttgtctttctcaggattacgctgattttactgattacccggatttttactttttgatttataaatgattaagggagatataagcggatattcgcttttatctcccttaatttttattcataaaatcttaaaaaatccaaaaaaacaaaatcaaattaatcagtaaaatcagtgtaatcctgagaaagacaaccttcgcttacttccataactccaggatctcctctgtatggttctttgtgtcaggctttttgataatatgcgcaatcacaccattttcatcgatgaggaaagtagtacggtgaataccgtcgtatgttttgcccatcatttgtttttcgccgtacacaccatactggtgtacgatctttttatcttcatctgccagtaaagtaaatggcagttcatatttctctataaatttctggtgactctgctcgctgtcggtgcttacacctacaacagcgtatccctttttcagcagggtactatagttgtcgcgcaggttacaggcctgggccgtacatccaggagtcatatctttcggataaaaatacagcaccacccgtttgcctttaaagtcggtgagggatacggttttgccatgctgatcttttcctttgaaaacgggcgctttatcgccttcttgtaagtttcccatatttacggttttagctgtttgaaatgatatcttaacgtttgaatgataatctgtagctaccttcatttccggctacatcggttaccttcagtaccaggatatgcgatcccggctcacaatgttcatcaaacgtataggtaagtacgttacctctccgcgacaacaacaaccatttgccatccagttctgcacggtagcttttaataccgctggcatcattcatagcaaaagatattttagcggcttttgaaagaacagcgcccggcttcacgcccagcggggttacctttggcgccacggtatctacttccaggtggaagttgccgaagtcgcggaaagtgcctttataccagccgttttccagggtggtggcggaagtgctgctaccctgtccttctctcaccatcactattttcgattgcagattttccggaacattacgggtggcgcgaagacgtacatcaaagaagtcgtgcacaggcaccagcgcattgtgcaggtggtatacattggaatatgctttggtgcttacagacgctgtttccaggtaattgaaacatacctggtcgtagagcgctgtttcatccaggtaaaattccacctggttattttcaaagatattacgtgaatcggggtacatggtgttggcgcatgctttctgtgcatcgtctgtacctgactgctgcagggccagtttcaccgtagaagtattgccgtaggcatcctttaccagcagctttacattatgtacagcgccgtccgacaggtgaatggtaccatcacctttcaggtcgtggtaaatatccagtttatttccgggcagggaaaacaccagctggtagtagggtccgccgcctttctttgttttataatcgatgtgggcgttcaggtaacgggtttcctcatacccgatgttatccagctggaaatcgatatccggttcattattctggaacagggtcacttcataaatgccatagatattaccggtattcatccggtcgatggcgcttaggcctatgcccgcctgcgctgcattaattttaacaaccggctgggtggttacatattcgccgcccactttcttcactggtattatgagtggcttttgctcgtaaatacttttctcccggtcgtatatcgccaggcggtatacatccggggctttggtatctgcaatatcgaaaccaaagagcaaggggttcagtggtttttctgttgttgtattcctgatttcaaagtgcaggtgcgggcctgcagatccgcctgtattaccgctccaggccacaaagtcgcccttttttacggggaacatgccggcaggaatggcaaggtcgctggcccagctttccgcctggtattgctgctttttcacatattgctgcagggcaggaaaaaaggcgttgagatgcgcatatactgtcgtatagccattagggtgagtaatataaagcacgttgccgaaaccggtatgtgataccccgatgcggcttacatagccatctgcagctgcgtgtaccggcagattttccttttgctgggttttaatatccatccccgaatggaagtggttgggccgcagctccccaaagttaccggccagtatgatcggaatatttaatggattcctgaaatagccttgcggatagtcctttaccgggatggattgcgcctgtaatagttgcggaagcaaacaaagtagaccgatgactctcttcataatatgcaaatgtagggaaaagcggatttatgcggattttgtctttactcaggattacgctgattatactgattaccttgattttgtttttaatttttaacttttaattatatccgttatccatctacaaaaaaaataaaatcaaggtaatcagtataatcagcgtaatcctgagtaaagacaaaatccgctttttttaagtactttagttcccgcaaaacgtgcaagcatacatgtctatccaggtatcagaactcagtaaagtatacggcgaacaacgggcggtggatgctatttccttcgagctaaaaaagggagagatcactggtttcctggggccaaacggcgcggggaaatccactaccatgaagatgatcaccggtttcttaccgcctaccagcggtaaggccagtgtatgcgggtttgatattgtgtcgcaatcgctggaggtacggaaaagggtaggatatctgcccgagtccaatcccctgtattatgatatgtatatccgggagttcctggaatttgtggcgggcatccatcaattgggaaaggcaggcgcacagcggattacatccgtaattgagctaacggggcttcaaccggagcggcacaaaaagatcggcgcattgtctaacggttataaacaacgggttggactggcacaggccctgctgcatgatccggaagtactgatcctggacgagcccactaccgggctggaccccaatcagctggcggatatccggcggttgatcagggaactgggggccaataaaacggtgatcctttccacgcatattatgcaggaagtagaggcgctttgcgaccgggtaatcatcattaacaaaggaaaaatcatcgccgacgataaattatcgttaatccagcaaaacaacaccgggaatggttatttacaggttacctttgcggagccggtaagcgaagccgaattactggcaatcaccggcataagccgtgtggtggcccgggaagaccatagctggcagttatttaccagccaggtagatgaagtgcgaaaaaacctcttacaatttgctttgattaataacaggaacatactttctttgcagagcaattcacagagcctggaaacaattttccgggaactgacaaaagcctccggcaactaactgtagcctttagcaacccgggagtggtgaagggactaacagccgcagctaacgccagatgctaaataaatagctaacaataataacttttcgaattatgagtatcatttcagaaatccatgccaggcagatcctcgacagccgtggtaatcctacaattgaggttgatgtaaccacagaagacggacattttggccgcgcagcagttccatccggtgcttctaccggtaaacacgaagcagtagaactgcgtgataatgataaggctgtttacatgggcaaaggcgtactgcaggccgtaagtaatgtaaacgatatcatcgctgaagaactgattggctgggaagtaacggaccaggccggtattgataagatgctgattcaattagatggtactcctaataaagctaaactgggcgctaacgctaccctggcagtgagcatggccgtagccaaagctgctgctgaagaaagcaaccagccactgtaccgctacctcggcggtgtaaacgctttcactctcccaattcctttaatgaacatcatcaatggtggtgcgcatgcggataataaaatcgacttccaggaattcatgatcgtaccagtaggtgctccttctttctctgaaggcctgcgctggggcgtggaaattttccaccacctgaaatccgtactgaaaaagaaaggatacagcaccaatgtaggtgacgaaggcggctttgctcctgaaatccagagcaatgaagaagctatcgaaactgtactggaagccatcaaagcagccggctacgaaccaggtacccaggtagctattgccctggatgccgccagcagcgaaatgtatgacgacgctaccaagagctacaaattctacaaaagctcccagaaagtaatcagcagggacgaaatggtagcttactggacggaatgggtaaataaatatccgatcgtttccatcgaagatgggatggcagaagatgactgggatggctggaaaaagctgaccgaatcagtaggcaaccgcgtacagctggtaggcgacgacttgttcgtaaccaacgtactccgcctgaaagaaggtatcgataaaggtatcgccaacagcatcctcgtaaaagtaaaccagatcggtaccgtaacagaaaccatcgatgccgtgaacatggcgcacaaagccggttacacttccatcatgagccaccgttccggcgaaacagaagatactaccatcgctgatctcgctgtagcactgaactgcggtcagatcaaaaccggttccgcttcccgtaccgaccgtatggcgaaatacaaccagttactccgtattgaagaagcactgggcgaagtagcgatctatcctaccaactctatcagtgtgaaaaaataatccttcgggaaaaacttttggatctcgggtatccggcaacatcaccgccggatatctgaaatccaaaaatgatttgtaaattgctgtatgtccggattaaaatttataaaagtgccaaaggtcctgaagaataaattcttcatagcttttgctgcctttgtaatatggatcgccttcctggacaaaaccaacctcatgtaccaataccagttccaggcagaggtaaacaaactcgaaaaccagaaggaattctttatccagcaaatcaaacaaacccgcgaagaacaacaggaactgctttccagccccgaaaaactggaaaaatttgcccgcgaaaaatactatatgaaaaaagataatgaagacctgttcattatcacccctgcacccgcccaataactccgcctcctttccccttgtgcatcttaaaaatttatcttaaattaacaatagattccgagcaaaatccgttataaaagagaacctattattagtattaaaataataatgcatgagtaattttacactttctgtactttcaaccctgtgtcttgttaccaaaagcgatataaaacatcaccaggaggatctttctttaacccgggaagagcaagccagctttgacaacaccaaagcagccctgaacaccgtacgttatgcgccaagagtagccaccctccagttgattttcgactacgccgccaataaacaaaaagcggaagaacagtaacagcgaccatacttttttcatttttcctatctttatggcatgactcaaaaagagcgttatgcatttgttctcaaatactttgaggaacatgctcccaatgccgaaacggaactcatctacgacaatccataccaactgctggtagccgttatcctgtctgcacaatgcaccgataaaagggtgaacatgaccacccctgctatctttgcgcagtacccggacgtatatgccctcagcacagccaccttcgacgacctgtttcccctcatccggagcatcagctatcccaataataaaaccaaacaccttatcgggatggcacaaatggtggtggaagactttaacggcgaaatacccgctaccgtaccggaactgataaaactgcccggcgtaggccgtaaaacagccaatgtaatcacctccgtagtacaccagcaacccaacatggccgtagatacccacgtattcagggtgtctgccaggataggactcaccaccaacgccaaaacaccgctgcaaactgaactgcagctgctgaaaaatattccgaaagaaaaagtacacatcgcccatcactggctcattttgcatggccgctatatctgcgtagcccggagcccgaagtgcggcgaatgcggactaaggcccgcctgtaaatattatgcaaaacttgtaaaggccagctgatatgcgtccattcctcaccgccgactggagaaacctgctgatgatcaactttgaagcagatcccgccgtactcaaggcgtatgtaccggctcatacagaactggacacctggaataataccacctacataagcctcattggctttctcttccaggatacgcgggtgaaaggattttcttttcccggtcaccgcacttttgaagaggtaaacctccgcttttacgtacgatacaaacaggccggtgaatggaaacgtggagttgtgtttataaaggaactggtacccaaagcactcatcacctttgtggccaacaccctgtacggggagaagtatgccacccatatcatgacccactcctgggaaaatcccgatgaggccaccctgaaagtagcttaccgctggaaagtgaaaaacgaatggaatcatttgtcggctaccgccatgcaagcgcgtcagccgatcattgccggcagtgaagaacaatttattacagaccattactggggctatacccgccttgatcaccaaatcaccggtgaataccaggtaacgcatccgcaatgggacattcacccggtcaccggatttgattatcattgcagtacccggctattatacggcgccgcgtttgaaaacatgctgcaacaaacacccacaagtgctttactcgccgccggctccggcattacggtaatgcccggtaaaaagatcaggaacagtactttgtgaaccgcagaagtttctgttatccatcaataatttcaagccgcaattatgaaattttattatcttaagcggttcatcaagattcaattaataaagcattagtcgctatgagatcagctgttagggtacaactatcatttatgatgttcctggaattttttatctggggcgcatggtttgtgacattgggcacattcgtattaaaaaatctgcagggcgccaccgatacccaggtaggctatgcctttcttacgcagtccatcggtgcagtaatagcgccttttattgtgggtattattgccgaccggtttatttctgcacaagtcatccttggggtgatacacctcgccggcgcggcgctgttatggacatgctcgggcatgaccagctacgacagcttctacccggtgttgctcatttatatgatcctttacatgcccaccctggcgttggttaattccatctccttccggcagatgagtgatcccagtaaagagttttcttttattcgtgtattcggcaccgtgggctggatcatcgcgggcttactcatcgggtggctgcagtgggaaaaaaccaattcgctcgaccttacctttaaaatggccgcaggcgcctccctcctgttgggattgttcagcttcacgctgcctaaaaccccgccggcaaaaaaaggcacacagatctctgtaaaagaaatcctcggcctggatgccatccggatgctgaaaaaccgctcttacctgctgttcttcctcgcctctattgccatctgtattccgctggcattttattataatttcaccaatccattcctgaacgaaataggcatgaacgctgccgccggcaagcaatccatgggtcagatgtcggaattcctgttcatgctggtaatgccgctgttcttcgccaggttaggcgtaaagaaaatgctggcattaggtatgctcgcctgggtggtacgctacgcattgttctccttcggcgacattgacgccaactactggatgctgatcgtaggtatcatcttacacggtatctgttacgatttcttctttgtaaccgggcagatctatactgataaaattgcaggtgaggaattcaaaagctccgcacagggctttgtaacactggctacctatggcgtaggaatgttaattggttttatcatctccggccctattgtagacgcatataaaacaggcaccaacagccacaactggcataccatctggctgatccccgcgggtattgccgcagtagtattagtattgtttatgttgtttttcagagatagtaataagaatacggttgttaaacattaatcatcggcaaaacgattattatggcaaaaatagcaatgcttggttcaggttttattgcgcggttctatgccgactccctgcagggacagcgtagccgtgataaaattgtaagtgtgtattcccgccgggaagaaagcgcgcaaaagttcgccacagattacgatgttgcttttcagaccacggaaatggaagctgccattgcccgtccggaagtagacgtagtttgtgtatctcttcccaataacctgcatgaaacggcagtcaacctttgttgcaagcacaaaaaagcagtgatctgcaccaaaccgctgggacgtaatgcagcggaagcgaagcgcatgctggaagcggtagaaaaagcgggcatcttccatggttacctggaagacctggtgtacactcccaaattcctgaaagcgctgcaaagcgtgaaagagggtgcgctgggaaggatcctctgggccaagtccagggaaacgcatcctggtccccacagcgaatggttctgggataaagaacaggccggcggcggctgcatcctggacctgggctgccactgcgtggaaattggccgcaactttatcgggaaggatattaagccggtagaagtgatgtgctgggcagatacgcaggtaaaaccgattgatgcggaagaccatgctattggcctcgttaaatatgagaacggcgctatcggccagtttgaagtaagctggactttccgcggcggcctcgatctgcgcgatgaagtaatgggcacggaaggaaccatctggctcaacagcttcctgcgtaccggctttgatatgtttaccaccggcaaaggcgccgattacgtagcagagaaagccgaaagcaattccggctggctgtttcccgtaggcgatgaactgaatgaactgggctataatcacatgttcaccaatatgtttgatgccatggaagccggtaaggaagccaatgaaacgttttacgacggctatgtggtaaatgctatccttgatgcggcctataaaagcgctgccaccaaacagtgggaaccggtgcaactggaaatctggcgcggacaggaaggagttaccaaagcaaaaaccttaacagaatataatgatcagtattacctcgtaaaagaagaaatgacacatttcggggctaaaaaactgatcctgaaagataaagtgagcgggcagatcattgaacaggtattgtgatctttatgatagatgtgattgtcctggtaggctatcaggataatcacatccccgctgttagcttatttttacaaacaaggctttgcccagtgcatgatttacctctacctgttttaagatcccgttttcatatttgaatatgttctttttcccttccggtagtatcagctcatacacacctccacccaggggtttcacgggcaggaagcggcccagcgtttcagaaaatacacggttcaactgccggggttcaataaaataaagatcagcaacacactcctctatttccgtatctatgacggatttttctccgttcactatgatcgtatattctttaccgttacgacggataatcgtttgtttatcttctcctgatttaccggatacacgtgaaacctttgcattggtgagtacattgttattgtattcatttgcgatgtcgctgttgatcttcgacagcatgatctggatccgtgtttttataatgatgcttttagcgcttccggtgagcttgcggttagcctcaatagtccctactgcgtgattggcaatacgcacttcgaaagtattggtttgcgcatttacctgcaaaaacaatacagctactgtgaaggtgataaacaaaatcctaaaaagactattcataatagttgacttaaactaacaatatattccggggggagtagtagctgtaagtgttccccccatcaaggaaaatacaaaaaatcctgtcacgacggacaggattttttattgtgtactttaaaattatatgtagccgtagtttatgccagcatttccctgattttggtaatcagttcacctttggtaataggtacgcccataattttatgatagccttgtgcgtcaataaggaattgatcacggataattttgatcagctggccgttattgatttcaggaatcagcactttatcatagctgtgcagtatttcgcccaggtttttagggaaaggacggatatagcggatatgtgcatgcgctacttcgtgtccttctgccagcaggtccagcacggcacttttaatggcgccataggtggagccccagcccaatacgaggaccttgcctttctccggaccaagttctatttgctgtaatggaatatgatctgcgatcttatctactttttcctggcggatcttcaccattagctggtgattttccggatcgtagcttacgttaccggtgatgttctgtttttccaggccaccaatccggtgttccaggccaggcgtgccgggtactgcccaggggcgtaccaggttttcatcacggtggtatggcaggaattgttcctctccttcttccaggcctttcttgaattttacttcaatggcgggcaggtcagcggctttagggaagcgccagggttcagaaccattggcgatgtagccatcactgaggaaaataaccggcgtcatatgttttacagagatacggaacgcttcaaataccgcgtcaaaacaatctgccggagtggatgcagaaactattggcatcgggcactctccgttacggccataataggcctgtaacaggtcggactgttccgttttggtaggcagcccggtagaggggccaccgcgttgaatatcaacgattatcaaaggtatttccagcattactgccagtcccatggcttcacctttcagtgccataccggggccggaagtagtggttacgcccatatgaccgccataggacgcaccgatggcggaggtgataccggcaatttcgtcttccgcctggaaagtacggataccaaaattcttgaagcggctcagttcatgcaggatatcggaagctggtgtgatcgggtaggtaccgaggaacaggggcaggtttgccttctgtgaggctgccaccaggccgtaagccagggctgtgttaccggtgatgctgcggtaggtacctggttccatccgggccttttccacgcgatagcgggtggtaaaggcttctacggtatcggcaaagttgtagccggcatgcagtactttcaggttactgtccaggatttccggttttttgccgaatttctctttcaggaacacttctgtattttccatattacggtcgtacagccagtacaggaatcccagtacaaacatattttttgcgcggtctttctctttcatacccagggtagtatccttcagcgcttcgcgcgtcattttggttacatccatggtatgcagctggtatggcgccagggagccatcttccagcgggtttacgccttccgggtagttggccaggcgaaggttcttagcatcaaaaccatctgtattggcgaggataatgccgccttttttaagtcctttcaggttggccttcaatgctgccgcgttcatcactaccagcacatcgcaggcatcgcctggggtgaatattctgttagaagaaaagtgtagctggaaaccgctcacgccgggtaacgtacctattggggcacggatttcagccggaaaatccgggaatgtgctcaggtcattaccgaataatgcggtgttgtttgaaaactgggtacctgttaactgcatcccgtctccactgtcgcccgcaaattttatcactacatcctccagctgttgaatcgaagtattaggcatctatttattcttttaagatattctttttaaagatgtaaatttaggtaatcgggaggtaggaacccactgccctgcaatattattcccgatccgatcacaaaagtacacaactttagtagactattcttacctgaataaagcattcccattacttatagttatggctgataacgggaagttatggttatagaaatgctaattttgcgcgttttcagcagtataactacggctgatatcaaatcaaatcgtatttttaacccataaaattaaactatactttatggcactctttgaatcgaacaaccctgtactgaagcaaagtatatttgataaagcgcctcacatcgcaggggagaccatgaccatccgtggcaccgttaacaaaatgtcttttatgctcctgatgttaatggcggcagcgattttttcatggggagaattttacaggaatagcggcatggtaatgccgttggcctttggtggcgccatcggtggatttatactggcactggtaattatcttcaaaaaagaatggtcggcttacctcgcccccgcatatgctatagcagaaggtttatttctcggagctatttccgctatgtttgaggccaaatggccgggcattgtaatgcaatcagtaggtttaacctttggtactttcattgccatgttgatcctctatcgcacaggggtgatccgggcaactgagcgttttaaatccatcgtgatgactgctacgctgggtatcggtatcttttacctgattgccattgtactgcgcatgtttaacattgaaatgccgctgattcacagcagtggtactttcggtatcatattttccctggtggtggtagctattgcagccctgaacctgatcatggattttgatatgattgaacaaggcgcgctgcagggtgcacccaaatattttgagtggtatgcttcgtttggtttgatggtaaccctggtatggttatacctggaaatactgcgcctcatgagcaaattaaacagaagataagttacagatataagcaccttaaaaaggccgccacagcgaatgtggcggccttttctttttaaatataccggccattgtttttgttaatgtcttccaaaagatatgttaaatggtatcacttcaaaatattatggcatcgtaattgcaaaatcgggctataacaacaagttcttttacatcttaaaacagtagtaaaaaatgctaacacctttacttaccatgtaacctttattgttaaaccgtttaaaattgtaagctatgaagaagataaaagtaagcatgttagcacttgcagctgtagcgtttggagccttcgcatttaggggcgttgatggtggaaccatagcaggcaaagtaacaccggctgaaggagctaccgaagcctgggccattcagggaacagatacgttgacatcgcctgttacggatggcgcatttaattttcagaatgcgaaagctggtgcatataccgttataataggagcgaaagcgccatataagcctgcaactgttacagatgttaaagtggatgatggaaaatccactgatttaggagaaattaaattagcacattaaacaagagcaatagtttgttttcataggggttaatcaaaaagccggttccgtacgtctgtacggccggcttctttcatttataccctctcctggaaaatattatcttttctcccctcataggggtaagcctttctctaaacgtcatttcttaaagtaccccttttttaaaatgatgtttatgaaaaagcagtttattataacgtatacaagtttgagtattggatggttgctgctgatgattgccatctttagtattatcttatccggctgtaccaaagaaaacatttccggctctggcaacgtagtaacggaagtccgtaccacaggtcatttcacggatgtggaaatatcaggaccatttgaggtacacctgttacaggaaaacaacgcgaaggtggaaataaaagcagaagataatattatgggtgtgatagaaacgggaatgcgcagcaataccttatttatccgggtaaaaaaccaggttaacatccggcatcatcagcctatgaaaatatatgtacacaatcctctctttcaacgaataaagttcgatggttcgggatccttagataatcaggataccatacatacttccttatttaagtatgaactcaatggcagcgccaatgccgcgcttatactggatgccgctacgcttaacacaactatcaacggctcgggcaatattaacatgcgtggatttgcgggctcactaaacagcgatattaacggcagcggcaatatcgccgccatgaacctggaagtgcagcatgccagtattaccatccgtggttccggtgagcatcgcgtgtatgtaaggaagaacctggatgccaggatctatggcagcggaaacattttttataccggtgaagcgaaggtagtggcggaggtaaagggttccggtaagatagtgaagcagtaatgatatgaacttcgtttaacctacactgttatactgtctgtgtttaaaatgaaaaggcccctgcaggtgcgggggccttttattattttaaagatggtgcatttatcaggcgccacctaatttgcatttctgcagcacttcccatgatttaccgttgtgacggaggaagtagaggttgtttactttaaaagtagcctcgtagtccttgttttcatattcaggccatgctttgttgaactgatcatcttccaggtctttaaaagccacggtaacgtgaggcgtaaatcctgtacgtgccagcatagtgctgaatccaaattccttacgcaggaagttgatcagctgacggtgcatagcagacatggtttcacttttttccacgttgatgaacagtacacggttctgtttattcgggaaagtaccgaagcctttcagggaaacttcgaaaggagcctgagttttggcaaattccgtcagttcatcacagaaagctttttccaatgccggatcagcagtgaaaggtacctgcagggtaatatgcggcagcactttcagtgcgtacataggaccgtattgttctgcaaattcctgtttgatctttataatttctttacctacttctgcagttggcagcagtgcgataaagtatattttgttatctggttttggttcgaagcgctgaggtcttccaccttgtcttggagcgccgccgccacggtatccaccaccgccgccaccgccgcgattgtatccaccgccaccgccgccgcgatcgtatccaccgccgccaccgccgcgattgtaaccaccgccgccaccgccacgatcgtaaccaccgccgccaccgccgcgattgtaaccaccaccgccgccgccacgatcgtatccaccaccgccgcttccgccgcgatcgtatccaccgccgccaccgccgcgattataaccaccgccgccactgccgccacggtcgtatccaccaccgccgcttccgccgcgatcgtatccaccaccgccactgccgccgccgtagccaccaccaccacggttgtagcctccgccaccgccgccgcgatcgtatccaccgccgccactgccgccgctgtaaccaccaccaccgcggttgtagccaccaccgccgcttccgccgcgatcgtatccaccaccaccgttgtagccgccacctgcgccatcacggttgtaattgccgccaccaccatctcggttgtagccaccactaccgccatcacggttgtaaccaccactaccgccttcacggttgtagccgccacctgtgccgccatcacgattgtagtctgtgcgcggacgatatccgccttctcgattgtaaccagtgcgcccttctgagccaccactgttgtagtcgggtttgccgccttcccgctcgttatttaaattgggtttgtcatcgcctttctccttattgggatcattctctttgttggtatcagaagaataaggcctgcgggggcgttcgtttctctcaaaagtcatcttacttaattaagcgtttgaagcaatattagctatgatttcataaaaatgaaatacgtcctgataggagttatataagggtgccggtgataccctgataactccgggctctctccagtcaacgattataccggcatcggtcatccgttgatgtatctctttacctttgtctaggaacaacaaagataactgagcgccacgttcattacaatttttcggtgttataatctggaaatttatgccttttaactgttgcaaaagaaattcaagataattggtcattccttcacttttgctacgtaaagcgccgataccggccgcttcaaataattccagggatgctttcaggctaaccatgttaaacacctgagcggtgctctgttgccatccttcagcttcttttttaggcacaaaccctttttccattttaaaacgtgcactctcttcattgccccaccagccgcccagtctaagaaaattacggtcgctggcgtgtttctcatgtacaaatgcgcctcctactgcgccgggtccaccattcaggtacttatatgagcaccaaacggcaaaatctacttcccaattgtgcaattctaccggtatatttcctgctacgtgtgccaggtcgaaacctgcataagcgccggccttatgcgcagctgccgttatagcgggtatatcaaaaaactgtccggtataataatttatacctccaaacaaaaccaatgctaagctatcactttctgtgttaataatctctaaaatatcttctaatcttatcaaatgttctccgggtcgcggggaaacttctatgattgcactttccggatcgtaaccatggaactttacctgggtttcaactgcgtactggtcgctcggaaaagcccctgcttccattaacactttaaaccgctgtttgtttggccggtaaaaactaagcatcattaaatgcagattcaccgtcagcgtattcatcaccgtcaactcctgctgactcgcacccaatatcgctgttaaaggcttactgcaatactgctgataatataaccatggattcttagccgcccaatacccctctactgcacattgttgccaatccgccaactcctgctctatcgccgctttcacattctttggctgtaatcccagtgagttgccacataaataaatagcatccttcccgttacgttgtggaaaataaaactgtgctctgaatttatttaaggtatcctgttggtccttctctttagcaaatgctaatgatgctacatactccatggtcttccaatcttgtctgcgccttagttatcttttaatggcggtgctgctattgtcaagaaagctgtgctgattatcttatttctctacttactgattattacaggctaatggcctaactgaactgttcaaaacaggcgtctttatttatattatctcttattttatcatatggcatataaggctaaggctgtatatggctagtaacgtgtcaacaactgtctgaggggtcaaaagtaataaaggcttttcaaatgccactcattccaaatgttaaaatttgttaatgaaagaaaaaaagtcgttccggctgtaatatacaaaaaaaatccgtcccgaagaatcgggacggagactgttaacctacaactgttacactgtattgaaaaaaaacttaattaacggagataccatccactttcttcttccccagcaccggctcttcagtagcttccggctccgggaaaaagtcatatggcttgggcgacaggtactttggatcatgcagcttcctcacttcatcccgcttcatgaacaccgctttgataatcagcaccaggaaaggcacgtacttcagccaccgtggcatattgaaccggtccagcacatcaatggaacgcttgttcatggcgtacatcaccggcaccagtacgagggtcaggaaagtcgcgaaaatcaacccgtataccattgtccaggccagcggcccccagaaggccacgttatccccaccaaagaatatatgcggtttgaactcactgaacagcgcggcaaagtcgatgttaaagcccactgccagcggaatcagacccaaaatagcagcaattgcggttaatattaccggcgtcatacgggtacgacccgcttccaccaccgcttcatataccggcatcttctgctggatcaacaggtcagtaaactctaccagtacgataccattacgcaccacaatacctgccagggccataatacccacacccgtcattacaatggaaatatccattttaaagatggagaagcccaggaacacaccaatgatactaaacaggatctccataaagatgatcatcgggcggccgatagagttgaactgggtcaccataatcatcaggatcaacccaaatgctcccagcatcgccatcatcaggaagttcatggtttcctgctggtcttcctgctcaccggtcattttaatagtcacggagttcggatgggtaaagtccttcagcgatgattcaatatgctgtaccacttcattcgcattcgcacctgttaagatgttggaatacagcgtaattacacgtttctggtctatacgcttaatacctgcaaaagtgttggaataatgaatatccgctaccgccgataacggcacctggcgtattgctccgcccatattcatgtcgcggtataccaggttgaggttcatcaggttattaatattgttccgctgatcctcatttaatcttaccataatcttatactcatcttttgcatcacggatcttggaggcttcagctccgaatagcgctgtacgaagagctccaccgatctggccggtagaaataccttccgcattcgcccgctcccggtctatatctactactatctccggcttattgtcctcgaaatcgctcttcagttcctctacacccgcaatctgcagggaatcgagataacgtttaagtctgaacgaactgctggtcagctcatcaaaattatcgccgctgatttcaatattgataggcttaccggttggcggaccaccctgctcctgctctaccgtgatattggttcccgggatacctttaacggcattacggattttatcgagatattgtacggtcgactgcccatccctcgcaccaaattccacaaaggcgaccgttaccttacccttctgcggctgcgtgctgagatccatctgcgaaggatcgccggcgcctttggccacattggaaataatagattccactatcgggttcttttcacccactactttagtgatacgcttttccaccaggttagtgatagaatcggtatacttctggtcggtaccattgggtaattctatgtaagtatagatgaagttgggatctgcctgcgggaagaacaccactttcggatttcgtatagccgttagcataatactgaagatcagtaacccaaacgtagccaccacgatccataccgggcgccatcccagcaaacaccactgcaatatgcgtttgtaacggtcctgtactttcggccagaatccatgctggaagcggcgagccacgccacctaaccagaaacgttccaatacgatcaacaggtaaaggaataccacaaaattgcccacccctatgctgccattggcataacctacaagcgccagcaaggcaaacacacctgagaggatcgtaaatttcttatcaaacttaggcttcggatggttttcaccttcgtgcctgtccatgaaatccaccgcaaacaccgggttaatgatataggccaccaccagcgatgcgccgagtgttgtgatcagcgtaaccggcagatagaacatgaacttgccgatcacaccaggccagaacagcagcggcacaaacggcgctaacaccgtaagggtaccggaaaacaccggcaggaacacttctcccgcagctattttagctgctttcacaatacccaggtcctttcgctggttataaatacggtgtacgttttctatcaccacaatggcatcatccactacaatacccaatgccagcaggaaggagaacagcaccatcatgtttaacgtaaacccgtacatcggcatcagtaaaaacgcgatgaacatggaaataggtaccgataatgccacgaagatcgcgttaaccgctcccatgaaaaacatgaggataacagttaccagcaggaagccgataataatggtgttgatcaggtcgtgcagggttacgcgggtagatttcgactggtctgccgtgatagttacttccaggtttttagggaagtagttttccttcatgtcctttgtaatcgcctggatcttatcggatgcatcgatcaggtttttaccactttgcttaataacgttgagcgtgattacgttctttccgccaagccgcgcatagctttcctgttccaggaaaccatctaccacgttggcaatatctttcaggtatactgttgcaccagactggccgcgtacaatgatgttacctatttttcccggatccttatattctccctttatgctcaggctacgtttctgaccatccatcgcaacaagaccaccggagatggtcttgttttccccctggatggcgccgataatatcttcaaagctgatcctggccgcatccattttgtatttgtccaaattgatctggatttcgcgttccagttcacctaccaggtctacgcgggtaatttcattcagcgcctcaatccggtctttcatatcatccgcatactttttcagtgtttgcaggtcaaagtcgccggaaaggtttacgttcatgataggaatctgcgacacatctatcttcacaatctgcggttcctgggtcaggtccttcggcagatctttctttgcatcgtctactttttcccgcacctgctgacgcgcagcttcaatatcttcattggcattgaactcaatggtgatcgcagagaaatcctgcatggaagtactcttgatcttctttacaccagagatgccgttcagttgtttttctatcggtttggtcaccgttgtttccatatcttccggggaagtaccggcattgacggtgttgatatagaactgcgggaacactacctcgggaaactgttcctttggcaggttaatataggaaagtatacctgccaatgcaatgataatggtagccacgtatacgcttaccttattatcaatggaccagctggtaggcttaaattctttatggagattgtcttgcatacacttggttttagctgtttgaatcagctttataatttaatcaggtcgttatcgttcaacccctgaaaaccggtggtgataactttatcacctgttgtcaaaccactctttatttcagccttgtcattgtatgtgcggcccatatctattgttttgcgctgcgccaccattttaccgttggcattcttcgctaccattacataaggttttccggaggtatactggatcacgcttaccggaactaccactgcgtttttagcgacataatccacgatcctgatgcgggcgatcatgttaggacgcagaccggcatccggtttcagcggcacttcaattttgatggtacggctcagcggatcaatggtcctggaagcaaacccgatagtgctgcgtatttcgcggttaatatcagggaaagataagatcactgcatctcctgatttcagcaaaccggcgtaagcttccgctacgttggcagttaccttcaggttgttggcgtttaccacgcggaaggctggtgcgcccggggctgcattgtctcccaccttggcgattactgcatctacggtaccgctgataggtgcaatgatgcgggtttgcgactgctgatcctgcagggtggccatcttcctttccaggctttccttctggtttttggcgttgagatattgtacttcagaacctattttctgtgaccacaggtttttctgtttttcaaacagggtattagccaggtccatctgggtacggagttcggccatgttggctctcagcacctggtcatctacctgggccagtgtttgtccctgttttactgcctgtccttctcttacaaaaatgttggtaattactcccggtacgcgggcggaaacgtttacgttttcgcgggcgtccacacttccctgcacatctatataatgttcaaatatggtatcagtaatagcagttacggtaacatctttcattttctgctgcgtcgtatctttcacacctgcttccttttccagcgctgctatttttttgtcgatgtcttcgttatattttactttctcctgtttcagcttctccagctgttcagctttatttccaccaccaccgcaggatgcgagcatcagggtgacaaaagggatcaggaaagaatattttttgatcatatagttagtagtaaatagtgattgaaataatggagcttatagtttgccatacgatttcagcaggtcaactttagcaacaatagcgttaaacaatgcagtgaaataattattctgtgcagtgagcaaatcgttttcagcagtggtcatttccaggctggaacctacgccctccctgtatttgatctgggtggtgttatatacgtcctgtgccagttccatgtttttctcctgtgcttccagcgtgagtacgttgttgcggaaagtagaataggattgctctctttccaggtcgatgcccagcttcgcattttcgatggccacttcacttttctttactgccagccacgcctggtctacctgccgtttgcgctgcataccactaaagatgggaacagagaggttcagtcctgtgtttacataaccgtaccacatctggttctggaggtaatcaaatttatcacttccccttaatgcgccggtagaaccgaatagttgcagggagggtagacctttcagcttatatcttttcagatcatattcatttgctttcttttgcgtttgcagcaactggtattcaatccgctgtgagtagtcgaatttatccatatccagcacatctgctgcaatcctttctgtagaaagtgtatccgttaacgttatagcctgtttcagtggcatgcccatctggtatttcagtgaagcagtacccagttcaatcaggttacggagtttggtttgctccgtttgcaggttggtatattgcactaccaggcggtctacgtccagtttttccgcaagaccgtttttgtagatctctttggtttcgttgaggatcttttccagggaacggatgttttcggaaaggatggtcaatgctttgttggcagacagtacattgtaataggctttgtacacggtggatttcacgtctatttccgccttttccacgccctgtgataccaggtcttccagtgttttacgtgcctgtaaagctacgagtacgctgggatcgaagagtacctgtgtaagtttcacttccccaaccaggttatgcggtagctggaaggaaactgctgtaaaggaatcttttggcaatccaaagttcctcatgttaaacatctgtttctgggtgatcgggttgtactggtaagagccggtaccagcgacattgggcagtgccaggccgctaacctccttgttcttggccagctggatgagttcgtccagtttggcggttttaacggtgctctgattagccagtgcgtagtctaccgcttctttggcagacaaacggatgggttcaggcgtaacctgctgctgggcgccggcgatggtcgccagggacagcagccacaccataaaagccatactggtgagccttttgattgatagcatagtgttatttattttgcgatagttgtttatattcttcaataagccggtatccttttacagaagccaccccatataaaaaattctccagcaacactttctgcactttgttcatatcattggcgccagggaacacttccggttgaaaacagatcatacaggcgtatatcctgtattgggtcagtattttaatgtcgatatctggccggtatactttttcactgatgcctctttccatattttcacggatcatggtggccagggtgttgttccggtaatcgaggaacagctggtaggctttcgagtgaaatttctgcaggtccaggataatgacagggttcatattgcgcaggcggcggtccagcatgtccattacgaggaataactcgtcaatggcgtctttcgattttttccggtcttcgatacagtcttcggtaacgatatttatgaaccggccgatggtttggcaaaccatatcgtccttatcggtgaaatgggcgtaaagcgttttcttcgaaatccccattctcacagcgatgtcatccatcgtgatggagcgggtaccaaattgacgaaaaaggccaaaagccgtgtccataatgcgttcctgtacttccatagattttatcgcattaaccctgttgttatgctggacaaaactatggaaactttccaaacttccaaagtttccagtactatttttttacatgtggcaacattcaattaaccgtccctgcttcctgctttgcgctttattgtctaatttgcagccctaatcacaaaccatgtcgccaaagcttagattaaaagtatttgcatcacgattgctgcgttacttctttcagggattgctcattctggcgcccattggtattactgcgcttaccttgtactgggcctttattactattgataatcttattccgaaagagctgattccggaaggcgcttcttttggttttctgaggtacaaaggagtagggtttgcattggtgctgctgctgatcatcggggtaggttacctcagctcctcctttattatcgggcggatctttgatttgtttgaccacctgctggagcgcacgccttttatcaaatatatttacacctctattaaggatgtttttgatgcgtttgtaggtgaaaagaaaaaattcgatcacccggtgctggtgcaggtatacggggtggatgtgtgggagatgggatttattacacagacggatgtcagcaacctgggcctcgaaggatacatggcagtatacgttccccatgcgtatgccattaccggtaaggtgtttatggtaccaaaagagcgggttaaaccgctgaccaacgtttctgccggcgaagccatgaagtttgccgtaagcggtggcgtaacccatatctgatccggggatgcttcgtagatgaagcgtagatacctcgtggttaaagcgtgcttacattttctgttgctataacaatgctgatattttattatccctggagataaaatatcagcatactttttttcgctatattcgtcttcccaaaaatatagtgacatgttaacccacacctggctacggattcccgtactatttactgtaatcatattttcctgtacagatgtttgtgcatggggattttttgcgcatcagcggattaaccggctggcggtattttgcctgccgccggaaatgatggtcctctataagccgcaactggagtacatcacggcacatgcgacagatccggacaagcggcgctacgctgttgctgcagaaggtgccaggcattacattgatatcgacctgttcgacaagccgccctacgcgcagattccccgtaactgggcagatgcagtcgccagatacacggcagattccctgaaccgcaacggcattctgccctggcatcttgaaaagatgctggccatgctcaccgccgcattccgggaaaaggaccagcagcgcatcctccggctgtctgccgagctgggacattatatggcagatgcacacgtgcccctgcatgcctgttccaatcataacggccagtttaccggccagcagggtattcatggcttgtgggaatcccgcatccctgaattactggcagataaaacgttcgattactgggccgggaaagccgtgtatatatctgatccccgtaaatatatatgggacattatcaggataagcggaatggccgcagatacagtactggcctacgaaaagcggcttagtgaaaaatttccgcccggcaggcgttacggttatgaaaaccggaatggggtattaattcgtacttacgcagaagactatacgaaagcatacgcactttcgatgggcgacatggtggaacgaaggatgaaaaatgcgatagcagccgtggcagcagcctggtacaccgcctgggtaaatgcaggacagccctctttacaggagctcacccatacaacccttaccccggaggagatacaggagatggaacagctacaacgtcaatggctggaaggtaagctaccggtgagggaggaatgagccggttaaaatatttatggtaatacttaataattagaaaagaaattttatctttgcccataccatcttttagcctgtcctacaccacgcgccttactggttttaaaacacccgtgccgttttttttccgtttccttagaaaaaccaaaacaaagtggaaagatcaaaaaatgaatttaatctgaatcgcaacatgaaggtgcataattttaacgcaggtccttctgtattacccaacgaggtattgtacaaggccagtaaagctctgattgactttgaagggtcagggatgtctatactggaaattggccacagaacgcaaccgtttatagcggtgatggacgaggcgcgcaacctggtgagggaactgatgcagcttgatgatgactttgaagtactctttttacatggcggagccaccacgcagtttatgcaggtgccaatgaacctgctggaaagcagcgaatctgccgcatatgtggataccggagtatggtccaacaaggccatcaaagaagcaaaattgtttggcttcgccgacgttgtggcgagctccaaagaaagcaactacaatcacattcccaaacagttcaccatcccccaaaaggcaagttatctgcacattaccaccaacaataccatctatggtacacagtggcaaatgacacctgttaccgatgtacccctggtagcagatatgagcagtgacatcatgagccgcagcatggactttaacaagtactcgctgatatatgccggcgtacaaaaaaatatgggcgccgcaggcgctaccatggtagctgtacgcaaaagcatgttgggcaaggtaacgcgcaaaataccagccatactggattacaggaaccacatagaaaatggttctatgctaaacacccctcccgtattcgctgtgtacatttccatgctcacactccgctggctcaaagaacagggcggcattcctgccattgaaaagatcaatgataaaaaagcagcactcctttacgatgaaatcgaccacaacccgctgttccgcggtactgttgtgaaagaagaccgcagtaaaatgaacgcctgcttcatcatggataaaccggaaatggaagaagaattcctcaaattctgtaagaaagaagatatcgttggtatcaaaggacaccgtctctccggcggattccgcgtatctatgtataacgcattgccatatgaaagcgtagaagtaatggtggaagccatgaaatacttctccctgaaaaaggcataagaaaatatccttattgtattacggagttgcaggtagatcagctatctgcaactccgtaattcgttagcggtaatccgtattttttttattattacatttaccactcacacatatctacatcatggctattatcagaccctttaacggattaaggcctacagcagatctcgcagcaaaagtagctgcaaggccgtacgacgtactcagctcggaagaagccaaagcagcggcatccggtaacccttactcatattatcatgtttcaaaatctgaaatagatctgcccgacggaacagacacccacagtcagcccgtatatgataaggcagcggaaaacctgcaccgcatggtacaggaaggtaccctcttcctggaaccacaggccgcctattatatctacaaactggtgatgaacggccgcgctcaaaccggactggtatgcgtttccgccatatcagactataacaacggcatcattaaaaaacacgaatttacccggcccgataaagaactggaccgcattaatcatattaaaaccaccaaagcgcaaaccggcaacgtattcctcgcttacaacgacgtaccggaagtaaacgccctggtagaccactggcaggaacacaaccaacccgtgtatgatttcaccgccgaagatggtatccggcacaccgtatgggtaatcaacacccccgctgccatccaggacatcactaccctgttcgctgaaaaggtgccctgcacctacatcgccgacggccatcaccgcgccgcctccgccagcctcgtacaggccgcatttgagaaagaaggaaagatcacctcggtagacaatcccgtcaactatttcctcaccaccattttcccggccagccaattggccatcctggattataaccgcgtggtgaaagaccttaacggcctgagtaaggaagcgctcctctcccgtctggactacgacttcaccgtggaagaaatcgggcacctgccccagcaaccctccatgctgcatgaattcagcatgtacctcgatggccggtggtaccgcctggtggcaaaagaaggcacctataccaccgatcccataggcatcctcgatgtaaccattctttccaataacatactggataaactgctgggcatcaaagaccagcgcaccgataaacgcatcgactttgttggcggcatccgcgggttgaacgaactggtaaaacgggtagacagcggcgaaatgaaagtagcatttgccctttaccccgtcaccatccaacagctgtttgacattgccgacagcggaaacgtaatgcccccgaagagtacctggtttgagccgaagctgcgcgacggactgatcacgcatattatttaaacatactatacgctttcccggcgatatccatctgccgggaaagcccgttatttcattgtctccctttatacccgcatccatgaaaacaactgatgatacccgctctatttttgatgatgatcccttactggcagaaaagaaaaagttttatcccacactcggccacgcctggctgatacccgtgtatagcctggtaatttggtatttaccctgcaggatcaatttgatacatctgtaccgcaggtgctaaattcgcctgtttgggtgggtgcgagtggtgttattgccatcatctgcttaattatactacaaaccagttttccatcaacaaataaagtaataaaataatataacaaagatatcccttctatcttccttcccatagattgatctgtgggacattaccccattttccttacttttacagcaaacgacagacagggatgaacatacggtcttctttattgaaagcactttttgttgcgggagttttattttcacaggttgcaattgcgcaagacgccaaagagctgtataatacagccacaggctttatccgcggaggagattattccaatgccatactggtattaaaccaggcattgcagctggaaccggataattttgaattaaagaaacagctgggatttacctattatctgaagggagaccttgtaaaggcaaaaagcattattgaacctttacttggcagcagggaagcagacgtacagttatttcagattgcaggcaatatttatgtgggaagggaagagtggaaaacggcacaacgcatgtttgagcgggccatcaaaaagttccccaacagcggcgagttatacaatgataacggtaccctgctgatgaacttcaaaatgtatgacggcgccctccggagctggatcaaaggcattgaacaggaccccggttttcccggcaactattacaacgccaccaaaacatacgacttcagcaataatccgctgtggtgcatcctctacggcgaaaccttcatgaatatggaaagtttcaccacacgcacggctgaaatcaggaatattgtactggaatcttataaaaaattattcaatgacccttcgctgtttgaaagcgccataccagaggataagaagggcaggaaaagcagcaacgaattcgtagaagcatataaggcctgtatgggcaagcaaatcagtgtagtaaccggaggaatagatccggatgtgttaattatggtgcgtacccgctttttactggattggtacaacttttacggtatgaaatatccgtacgcccttttcgattatcagcgcaggctgctacgggaaggaatgtttgaatcgtataaccaatggctgtttggcccgtcggccaaccaggccagctacaaagcgtgggtgggattacataaaaccgattatgatgctttcctgaaatttcagcgcagcaatccattaaagccgaaacctgatgaatattacaatgatggaaggtttacgctgatcaattccgggtattagtatttagataatttttgatttacgggtttagtcaattagttgctgtagcaactgaatgactaaatccgtaaattgtaaatctcaaaatctgaatatgctcgttaacaaacaccaaaacattatcgacaatgctgtaaaggcgaaccacgaacgaactttctattcgcaatacccggagcatcccaaagcttacggggaagaagcccatgccaaaggcgtacagagttatcagcaattactgggaaaacctttcaaacagttactgcaaaccggcgaaaccagctgggccggagaggaagtatcaccctacacccgcgaggtactgggagttacctatcccgtttttcctgttggcgacctgataaagaaagccacagaagccggcaaaagctgggcgaaagtaccggtatccgaaagagcaggtatgctcaccgaaaccctggaaagaataaaagactacttttttgatatcgccaacgctaccatgcatactaccggccagagctttttgatgagcttccaggcttccggcccgcatgccaacgaccgcgccctcgaagcagtagccaccggctatcacgaactacagcggtacccgccatcattaacctgggagaagccaatgggtaaagccagtatcaaactgtacaaaacttttaaaccggtacccaaaggtcccggtgttgtgattggctgctccaccttcccggtatggaacacactccccggcgtttatgccgacctcatcaccggcaaccccgtgattgtgaaaccgcatccgaaagcagtgctgccgatcgccattgccgtaagcgccatccagcaatcacttcaggacaacggctatgatcccaacctctgccagctggctgccgacagctcagaccacctcattgcaaaagaactttgcggacaccccgacgtaaaactgatcgattataccggcggcagtgcatttggaaactatgtggaatcactcccgggcaaaacggtatttacggaaaaagcaggcgttaattcggtaatcctcgacagcgtaaccgacctcgatgcggtgattcagaacctcgccttttctgttagcttatattccgggcagatgtgtactgcgccacagaactttttcattcccgaacagggcgtcaaaacagccaatggccaggtatctttcaatgaggtagtgcaaaagttcaaggaagcggtagtaggcctcgtaaatcatccgaaaatgggcgcaggtacgctcggcgctatacaaaacgacagcaccctctcccgcgcacaggaagcccgtcacctcggagggaaagtgatcctcgaaggcaccccggtagtgaatgaagaattctccaatgccagggtatgcgctcccaccatcctggaagtaaccagcgcggatacagccatctatgaaaaagaacttttcggaccggtgatcctgatcatcaaaaccagggacacggcacatagtatacaactggccaaacaaatggcatcgaaatacggcgccattacctgcggggcttataccacagatccatctgccaaagaaaaaatagcagaagaaatgaacagcgttttcacacctgtatcttttaaccttacaggatttatctgggtaaaccagcatgctgcgttttccgatttccatgttacgggcggtaatccggcaggtaatgccagctttaccaaccaggaatttattgtgaaaaggtttgtgtgggtaggcaaccgggaactggcggaatagcgaaattttctgacaagcgcccgcttaaacagggcgcttgttttaaagcataccagtaattatgaagaaactcttatgtatagtattcgttattacctgcggcatcgtggcatgcgaacaggcgcccaaagctgataaagcccggatcaccgatgcgcagaccgtgcaaaccggcaccggtaacgcttatcttccggataccgccttaagtgtggtgcgatggatcggtacaaaacctaccggtaaacattacggcgcattgaaactggccggtggcgcactgtatgtaaaagacagccttatcaccggcggccagttcattattgatatgaaatccctccaggatgtagacctcgcagccgattccgccatgaaacgcaagctggaaaacgaattgaaaggagagatgttcttcgacgtaaaaaaatatcccgccgccacctttgaaataaccgaggtaacggcattccatcccactgatggcgatgaactcacccttagaaacgctacccatattgtcaaaggaaacctgacgctgaaagctgttaccaaaaatatatccttccctgccaggataacgcttaaagacaacaccatcatcgcaatagccaattttaacatcgaccgtaccgaatggggtatcagctatcgcgccgacaaatcattacaggacaaactcatcaattcacaggtaaatatctccttcgatataaaggctacccgttaagcccgcttttttcgtttttttctgcgtgaagccaataaaatattttaaatttagtacaacctctggtacctaaaactgacttccatggaaacaaatcaagaaagagataaccgactttggcgcatcgcaaaagccagggcaggatttaagtcccacctgatcatctatctcgtgattaacctgggattatgggcagtatggtttctgacagacagtgacaaaacaagcggtactccctggccggtatggcccgcattaggatggggcattgcattggctttccagtatttcaacgcataccacaaagatcctttcggtgatgcgttaggggaatatgaaaaactgaaagaacaacagcacacacgtatctgatatttgagccaaaacaaaattacagcagcatggaccaaccgcaacgactattcgatgtgatttcttaccaattagccaactttcccaaagaggatatgctggccgggaaagaaaacgggcaatggaaaaagtacagcacaaaagaaatagcggacctcactctcagattcagctccggcctgctcaaactgggtatcagaccgggaatcaagcaaaatgaggagaaagataaaatagccatcatttcacccaacagaccggaatggatcattaccgacctggcatgtcagcaactgggcgccgcgctcacccccatttaccccactatcagcgaaacggagctcgcctatgtactgaatgatgcggaagcacgcatcctctttgtgagcgacaaagacctgctggataaagtaaccgccatgagggataaatttccctccatccgcgaaatattcaccttcaataaagtagaaggcgcccgtcactggacggaagttcccgcactggccgacaccgccgattttgaacagatagaggaagtaaaaaagaatatttccccggaagaactggtcaccatcatttacacttccggaaccaccggcacaccaaaaggcgtaatgctcagtcatcacaacattatgagcaacgtactggcctgccagccttatctccccgttaacaaagaggcaaaagcccttagctttctgccattgaaccatatatttgaaagaatggtgacctacctgtatctccgcgccggcgtaccggtttactacgcagagaccatggaaaccatcggtgataacctgaaagaggtgaagccaaccatctttaccaccgttccccgcctgctggaaaaagtgtacgaaaagatcatgactaccggcctggaactcaaaggcattaaaagggccttgttcttttgggcagtagacatcggtaaacggtatgaaatcaataaagaccagggcgcctggtataacctgcagctcaaactggctaataagctggtcttcagtaaatggcgcgcagccctgggtggcaatatcgaatgcattgtaaatggtgcagcagcctgccaggtccgtttgttgaagatattcaccgccggcggcattcccatcatggaaggctacggccttacggaaacctccccggtaatcagcgtaaaccgcatcaacgtggaagaccgcatgtttggcaccgtaggtcccgttatcagcggtgtggaggtaaaacttgcggaagatggcgaaatcctctgtaaaggccccaatgtaaccattggttactataaacgccccgatctcactgccgatgccatcaaagatggttggttccataccggcgatatcggcgtaatgatcgacaacaagttcctgaagataaccgaccggaaaaaagaactctttaaaacctccggcggcaaattcgtggcgccacagcccatcgaaaacaagtttaaggagtcgccctacattgaacagatcatgatcgtcggggaagaccgtaaattcacggcagcactgatcataccttccttcagtaacctccgcaactgggcgcagaaacgcggtatcaccgctacctccaacgaagaactcgtgaaaaacccggatgtacaggacctctacaaacaggcggtagaaaaatacaaccagtttttcagccatattgaacaggtgaaaaaatatatccttctcccccgtgaatggacggttgatggcggtgaactcacccccaccctcaaggcaaaacggaaggtaatcctggagaaattcaaaaaagaaatcgatagtatctatgcccccgccggtggaaaagtagatatagaaagtctttaaatattaatttaaaacccttacttttgccacccgatcccaggattggggtaaaaaatgatggcctcatagttcaatggatagaatagaagtttcctaaactttagatacaggttcgatccctgttgaggctacaaggaggtacatttcagggctgtaccctaatggtgtaccggacaaaaacaatgagaccagccattacagccagtctcatgtctaatctaagatctgtagtaggtatacacctggttgccttcatggccggcaatcacttcataaacgccgggcgaagtctctaccacatcatttatgttgtaaactttaccacaaagggtattgccaaatttacatccggataaacggggatcttcacctgttccggcatatgttacggggttaccattcgcatcaacataaaacttgtagtaatccactaagggccgggtatttgctttagtaacaaatacacaaataacagaaattccaatagccaacaggcctaaacggtactttttcatgaggatatattttttttgaataataaaaacgcctggtaaaatcgcgctgtgaaataagccccccttcttctttttgaggcccagatgcccgttatggccaaaagcatgaatatgatatttaaccacaaatgccatatccatgacataaagtttatcacaccactacaggcacagggaataacataatctccggttagcatcattacgatataaacacttatagacaggagtagtagaaaagcagtatataaggctatcaggcgggaccttggccagagcaggaaataagacagcaccagttccaatacaggcagctgccaggccataccggcagcataaccacttattaatggaaagctgctgagctgattcctgaatacctgataatccaataattttatcaatcctgcgtaaacaaataaaataatcaacaatgcagcaataatgttagcagcgtattctcttttcatgagtatagtcattttgtttgcagacggaattccagtgtatccaccacatctccctcttcatttcctgtaatatggaagggaataaatgcaggcgatgcggtcatccccagggtaagtaattgtgcatgttctatccgggctatatagtttccgggagcaagtccgctaaagctgaagaaaccatcgctttctgacagcaggcgggcggccaggctgccatcttcactgtaaatacatactacgatgcgccccaggcctttcccattcaggtatacctcacccgacacttctccgaccaccactacaggcacctccacgggttttacacgattgggatctattatcacgctgaccgtaggatgttttaaccgccatgctatattatcaaaactgctgcggcgcatatcaattaaataattcgagtacggttccagttccagtatacggatagtagtatcccgtttgttatgtatgatacggccgccgttcaccattatctgcagtcctgcaactttaggttctcctttgtcacggtggccattgccgttcagatccagaaaaggctggataacaatgccgccggtaccaacactggtccggctggttagatccataaagtcacccagtatcaaacttcctcttgcggattgcacaaacgtactggtcgcattactgcgcgaagcggaaaagcctacctgagagaaagaaaaatcatagcggataccaatactcacattactgaagttgcttctatagttccgctcatacgacatattcaggtagccatttctgaaaaaatacttccccagttcacagcgagtgccaataatctttttctgcatatactcatactgcacctgcggcgtgatcatcaattgctttggtaaccggaaagacagggcaaggttactgtacagatatggatctgattggccggctaacactgcataggtggtaaaattagctcctacacccagtattgcaccagacatcagccattcggcagcagtgtatttggctccgggtaatatgaactggttgagggtaagcctggaaaatacggcaagtttgcgaccaacaaaagtgcgggacactgccagcttgcgttcttccaggtaattgaaaataatagccttctgcccttttttataccgtgtgtagtttgcttctataaggagattggcaggcaggcgccaggtcatcatcccctgtgcccttacaccataagtataatctcccgagaatagcaggttggaagccaggcgcatggaagcattcacaaaaggcatggtttccccggtggtaacagaagaaagatattcaacaccgccgccaatggtaataaggcgtgtagcgccatagttaaaacttacacggcccaaccggctgttcacactatcttccaccacacctgcgctggcggtatattcaaattcacgatgcggcagaaaattgaaaggcacactgatattctcctcacggaaccgctcctcgccccatggaccgtaaaaacgaagttttacaactgttgttccatataccaatggtacctggaaagtaaaaaacccggacgcatctgctttcgcataatctaccagttcattgttcacatataattcaacagtccagttgggttctgtaaaattactcagggtatagaaaccaaaagtacgcctgtttgtagtaggtgtattggtaacctgtacacctaccaccggatcgtaaacagaagcagtggattgcgcaaatattttcccggctatcacctgccgcaggcctttgtgatcattatttacaaaacgccagcggtagtattgctgccttctctcaaaaggcctgaacctgtaatcgctgctatcatgcataacggattgttgtgcgccatagttgttgtaattgagggctacattcgtttcgcctcccgcaagcgtacctcccagggacaggcttgcccttgtgtcatttccaccctttcctctctgcgtggtaacaacagaccagtctgccatacccaattgaaagagcggataatccctgccaatcacagtatccgcttttacctggcctttcagacgattgatattctgatgcatctgctgctgccgcatttcccggataaccggcaactcatgttttgtatccatactaacggacaggttgcggaagttgaacttacaattcaatccaaatacacgtccgaaaagttctgtactcaaataaagaccaacaggtgtgctgatcagttcattttcttgcagtacaaatgtttttccctcatactggatacagttatgggttttatcaatgagataaatagcctgttctgtaataaaggtgccggatacagtatctgcgctcccggataacgtgttcctgatctgtaagaaactgaatacatcagaaacagacagataggcaatatcatcaactatcagggccggcagttctattccacctatgccttgcaccataaagaaaatagatgtttcataatacggagatacctcctgcctggcaaaagcaggggaggtcataccaatagtttgtagcaaaatgaaaatagtgatacgggatagcactcctgttattcctgtataaaggtgatcgaaaataaaccactatatgcgccaggtggattagccaggggactcccaattgtaagcgtacctcctatccttacctgtgtacggccgggtgatatagctgtggcaatgaaaggtgatcctgtactcgcggtaccgatgtgtaacatcatagatcccccgttacttccggtgagcataacgtctggtccgttcataatagtgataagcgtaccggcgttagcatccacttcaataatgccaggcgaaaaaggaaaacccaggccagcctgtacaacactgcctgtaacagaccgggaaccatccggatatataatcaccgtaccacctgaaataccctgataaaaagcaccaaaaacaagtccctgtaaagggttcacataaatagcgattgggcgtggaggcggttgctgcgcctgcattacctgccaggtgaaaaacagcaggatcattacactcacggttaatttattacacaggatcatagatctcttaattaattgctgatcaatattttttttgaaaacttctgttgctggacaaaaaaggtaacaatgtacacgccattcctaaacgctgaacccaggtcatgatagccattaccataaagctgcttccgtaatattacctgacccagcatattcgtgatcatcacatcacatacttctccccgcatctctccaatatgcgcaagcaatttgccgccagccgtataagcattgaaaatagccgtgggcgcttctggtaaaatatccgggtctttcacacggaacaccaggaaaaaccggttctcatatccgccggcattcaggtaaagacggtaaccgggatgttcttccagatcctgtcttataccggtttttgagtcatagaggtatatgtgctgtccgtagggaatacgttccaggtcagatacattaaaggtgatccacccggcccgttcggttttaagacccagctgtattacatctgcactgtctttcataccaggccaggaacaaatagaaagccgcgcggcatccggactaatcacatataaacttggcacttccccatctgtattcatcagcttgagggcatccatttctgtatcaaaagccttcgtggcattatcatcaaaataaacaaccataggatctgctgctgttacatcatccttgaatcctgctgttaacctcagcaatggagatgttagcgggataagccggtgaaaatcaggcagcagattattaaggcgtgcgttattattaactgacaacgttgcagcaacaggaaatgtccctatggaaacatgcacaaaaaatccctgcatggcagcaataacatgaccggcaattccatcactggaaacgccattgatataagaactgtaggttcccgtatattgattaccagcgcccgtattaaagtagtataacgcgttgtcaatattagtgcggctccatcctgatgccgtattccagtctataggtgacggatacggattacctgccaggttaaagcccagggtgtagggttgattatgattgtataacgtagccgaggtaattgtatggttattcaccactcctgtaatatccgccgttttagctgtggaagatgcgcccatgttagcggcgtatccctgcataggtgtgagcgtattggaagtattggtataacgcacccagccggaagaaggcaggttttcatcatagcggtaaaatgcagggaaggtcgcgttaagatttacatcatccgaaaactcattgacggtagctgcctgaaatggtgagctgaaatatctgtatccgaaaccagatggcaggtatcgttgcatgtcgatgtttcccagcacctctccggttccactgccatcgatcaaggctgtttgtgcagcagtagataataaggtcagatttccatttgcctgaagggtgccgttgcttaaaagaatggccttcagggaatgcccggttgagctgatagtagttgtactacccgttgcgatagttatattattaaaggtagtcgccgatgttcctgcaatgacctgcgttgttcctgcgaaaactattactccattgttatgaacaaacgtgccattgtttgcccaattagctcttagcacgatgctgccatcaccggcaataacataggtattcgacgcaattataattccctggctgtaggccattacaggtaggaacaggaataaaatatagtaaagctccagtcgcatagatcttattgtataagcgttatatcaaagattacagtacccaggaattggattccgctaatacctgcgcccgagttagtaaagttgatcagcatggtgtttgttgcacttatcctcgaccacgaaatagcaacaccatccggcaatgaggtgcgcggatttacaataacagtactatttagtactgcgcccgtaacggttacggttttagttacactggcggagtaagtgatgggagaggtaatatctgtaatggttacggattttctggatatgttattcagcacactacctgctgcacccagcttaaaatttcctgctacatccaatttggccgttggcgcaatggtagcaatacctaccaattctccggccattatccgcatcgcttcattagctggcgccgttcctcctaccaggaaaataatatcttttgttgcattattattaaccatgtatagatcattccctgaagaaataatgtaaccatcattagccttaccggtttctatgggattaccggtttgatacaggtatcctgaaccattaatacccaggtcgatgaagttggtagtttccgttccattatccgcagtagccacatagtcagaactgctttgggttcccggagaaagattctggatgttcatctgcatgtaactattgatactgcctttggcgtaaaaggcattaacagaagtagtaacgcccatatctaccaggagtttttccggattgacaagatcaaatgtacttgtccctataccaacgccacctgtttcgctgatacgcatcctttccgtattactggtaaaaagccgtaaatccgataggtcgttgatgccggaacccatgtaaaaggcgtttatccccgaaccggtattaagagaaaaagctgaatttatacgggccgaaaaacgcaacgagcccattagatctcccttcagaagattgagtggtgcagccaggataccccttgccttccgcatatgtaatccggcggtggtggtgttgccataatcatcaaacaggtaatcatttccggactctgaattatctgttactttatgaatgcctccaagcggaatagctattcccaatcctaaagatccgttggcagtgatccgcattttttctgtgttattcgttataaacggcagatcaatattatcgatggtacccaggctctttgcagttgttaccgtattgccgttcaatgaccagccggtaccggcaccaccggaggagagatttatccaggcacttacagaatagtagtaaaaccctttggtattatctgtctggtaaaccagcaggccttctgcaggtgtggtaatagccaatctttgcacctgcgtcattcttggagccagtaaaccttttgtagttgatttaatatccagcactgcggttgcctgtcctgttgtataggcagcatcatctgttacgatcactgtttgggtatatcccttcacaccggttaacatgaatacaaacaggatgtatagcggtcttatcatcataggaatggttttagatcctgactatttcaattgcaattctgcctttgccagttgcgtggatacagtgcctttctttgtagtgtaaaccacccggagcattcccttgtgataatccacaccctgcttgtcatccagatttatattaaactgacgggagagattaggtgtataaactgccaggccgttaaccacgccaacctcacttactttccctttctctgaaatatgtattactgttatgccaccgtatatagaagcattacccgtacggttaaatgtcatgctaaggcggttttcaggggtaagcgtcagcccggaaatatttgccgcagccctggtatcacccacacgaataataaccgggatgctaatcccaaaaaccgggattaattttacggacagaccaaatgaatcttttaaagcactcctgtccgccaatggtttctccatcgattccgccctgaagtatatatgagagcggtattctccgggggcaagctgactggtttttacaagttgtatcttaattgtttgggcctcattgggggcaagtattacacttcgtggaaaataacgcaggttaccactggcaaattgctgtccggaatccggttggctgatctgcttaaacgtgccgtcttcgttcattttgatctcgatgaaagagatcaggtacctcgccgtatcctttccggtattagccagattcaattcctgcattctgctctgaccttcgaataccactctggcaggtgctattaacagattgccctgcgctgtagtatttatagaaaaaaaaatcatgcatagcatgatcaggtactgtttcattggatatgtttagtgaaaatctgctaaaaaacggatacgatgcacgcgcatcgcatccggaaagaataactaattataatttacggtcacatcaaaaggtgtggcagatacgtatacaccagagggttgagccgctgctatatttaatgtggcgcctacgttaagggtttgttctcctgctgtaagcacgccgccggctccggacggtgtacttgtaaatgtagttaccgtcatggtattagcaccactcgcaatagtgacggcagaaacaggtaacgtgatcgtgtaatgataactgcctgtgccagtcactgtaaatgaagcggcacttatagttccactggttgagggcagtgttaccccaccggttgctgtacgcgatcctgccggggataatacaaccgtaccgccagcggtagattgaacggcgacgttgccgaaattcatatcaacatctttggtgatgctgataggtgttacaatagtagcagtggcggtggcggaagccgtttcctgtgcagatgcacgagtggtaaggcctgtgagcgtaaccactgccacgcataaaaaaagtgttcttttcatgaatgaaattttaagtagatgttcttgatcaataggaaataagcattctagtctcgcatggttacctcctgtgttttacgtggttcttcggttttttggttttttggttttcttataggatacgacaaaataaataaggtatacaagtataaggataggactggtataggttattcttattcctcctttctttcacatcaaaagtaggtgtatgcaaaaccctgcgcaatgatcatgatccattttaaaatgatcctgatcatcggttaacaccgaagacaacataaatagcctatattacatctataccgtagatcatgacttacgcttaaagtgcaggaataagtggtatataataacgttaaccctcataagacattatctgcatatatgtaccatagccacaatattgatttcgatgtgctctttaattatgccactatgggtatcattatagcagacggcagtggttgtatcctgatggctaatcctttcatcctaaaggaatttggatatcttaatgcagagattgttggccagaaagtagagaagctgatacctcaccgtttcaggtcgcatcatgaacagcacagggaagtatacagtgtaaatccacgcagccggccaatgggtgccggacgagatctttttgctgtcaggaaagatggaagtgaggttcctgtagaagtgagcctgggtacttacaaaacggaagatggacaatttgctattgcttttgtcagttttatttccgacagaaaggatgcagaaaacgcattgaaacaattaaatactgatctggagaagaaggtggaagagcgaacagaatccttaacggaaacagtccggcaactaggagaacagataaaagaagcaaaagcaaaggacatagaattacaacgggtgaataattttctgaatgtagcgcttgaaaaagaaatagagctgaacgagttgaagtcccgttttgtttccctcgcttctcatgaattcagaacaccgctcagcacaatcctgtcttccgcctacctgaccggtaagtatgaagagctggctgaacagcccaaacgggaaaaacatatccagcggatcatctcctccgcaaatctgctgacaggcattctcaacgacttcctttccgtagggaagatcgaggaagggaaaacaagcgggaagaaaatcaggttcaacatagaaaagcacatcgataccattataagtgaaatggacggcctcaggaaaaagaatcaaaagatcgtataccgtcacacgggtaatgtttttgtactaacggacccttccctgttaaaacacattatgctgaacctggtatccaatgctattaaattctctcctgcggatggagaggtcgttatacaaacaactatctcaaaaaaactgctggtgatatctgtcagcgacaatggcatgggcatccccacatcagatatgcaacatttgtttgagcggttcttcaggggaagtaatgtatctaatatacagggtaccggtttgggtttgcatattgtaaggaaatatgctgagatcatgaatggcactatcagctgcagaagtgaaataaataaaggaactgaatttacgatcactatccatctttaaattggtttctacgtgaaaaagatattaattatagaagataatattgaaatccgtgaaaatatcgcggagatacttgaactggccagttattccacccttaccgcagagaacggaaaggaaggcatggaaatggccattgcgcaattaccagacctgatcatctgcgatattatgatgccggtactggacggatatggggtattgcacatgcttcataaaaataaacgcttaaggaatacacctttcattttcctttccgcgaagtcagaaaaaccagaaatccggaaagggatggaaatgggaggagatgattacatcactaaaccctttaatactacagagcttctaaaagccgtagcctgccggttgaaaaaagcggaacagatcagcaaggaattacctcctacccccaaaggcctgaatacgcttattcaaacagcggccaataaagacagccaggaatccataaaagaggatagtaatgtgcagaagtataaaaagaaacaggaggtgtacctggaaggtcatcgtccctcttccctttattatatcatgaaggggaaaatccgcacctacaaacgaaatgacgaaggaaaagaactggtgatcggtttatataatgaaggtgatttcctgggatatactgccttactggaacagcgggtttataatgaaaacgcagaagtgctggaagatgcggagctggtgatcattccccgggaagactttgaatccctcctttttaataatttaggcatcctgcacaagttcatacaattgctttcccgaaacgttacagaaaaggaagaacaattactggggatcgcatataactctcttagaaaaaaagtttctacagctttattatccttatataagaaatataattcttctgaaaatgccaattacagtattgatatgagcagggatagtctcgcagccctgacgggtgtagctaaggaatcattgatccgtacactgggtgatttcagggatgaaaaactcatttctattaaagaagggctcatttttgtccttaacaggaagaaactggagttaattttaaactgacgacttttcatttattttgctctcaatagcaaactccaatgcttgcccaaccaatcctgcacctattttgttattaagttatgccacgtcgccataaccctgatcaactgaccttatttccgctgaatgccgttcctaccacgatggtatcctacgcagttattatttcgccaccccgtaacataatggatcatgtcaaattcctggagaataaagtttatgatctgctcccgcaggtaaaacacggacaatattcaaaagcacatatctccctgctgaaattaacatcagaagagaatgacacctcgatcatcaacctcgtcaaaaatgccgtatcagctttatcttcctttgaagttcagttgaatggatgcaacatttttccacatggatacacttccgactcactggttttacagatcggtaatccccagccaataattgatgtccataaatccttgtttaaagcgcttaagcggaaaacaccaaagatgacaccacacatgactatagtaaaagaagtaccgcataataagctccgcaaaacagatctctccgcattcgattatcacaattcctttctatgcacaaaaattactattctaaagaaaatggctggtgataaacagtatgataaactctttgaagtatgtctatccgattaataattcgcttgcccaatatccagccggttaattctcccgtccttatcgatatgaaacttaaaataagttttaaaatctccccattgatcgctgtgaaacaggccatacacatccattccgttattctctactttatcgatacttgtaaagcgttcatgtccaatggctttctgccagaaggatttaaaatccattttatttccatcgtcaaacagttctgctttatcagcaaataaggcaaaccatgttttactgtcgtttgtttgcagggcgttgatcgcctgtttcaccgtggcatgcgtgagtttatctgtattcatggtaggacttttttgctgcgcaaagagtactggtgacagaaagccgataatggccaataacaacatcttcattttgcgagcggatgctgcaaataaatgataacaagattcaggaggaagaaaggcacctcgatagcagcacctttcacatcacggccatacaaagaaaagcagataatcatcaggatcgttgcggccatgaggaagttacccaacaaaaatgttctgggaaacaggatcattaaagcactcaacaccgttaccactccattgatgatgatggctgttttactaaagtgccaccggctgaacattgtaatcatttccggcttctggccaatcattgccaggccttgtttcaggcccatgaatacagtaaaaatgatcaggacggcattgagtactttaagtaccataataatagattttagttggtggcgcctccgttcaccaacaggtgctgaccggaaacaaaagaggataaatcgctggcaaaaaactcagccaggttagctacgtcttccacttctgcgagtcttcccattggacaactatccagtaattgttttcttagtgcaggataagccgccgggtcggcaaaaatgccggaatgatctaccgcaaaagggataatcgaatttacggtaattcctttatgtcctatttctttcgacaaaatatctaccaggtatctcggggtggttttacttccgccgtaaaccgccataccgggtaccgggaaggaggtagtactggatgcgatataaatgatacggccattattttcaacatgttttgctgcctgctgcatggtaaagtaagttccttttgtgttgatggaaaatactttatcaaactgctcttctgtaaactctgttaccggcacttccaccatttcaatacccgcattggccaccacgatatctatcttaccaaaagcctcttttgctgttgcaaacagtttttccagatcagctactttgctcacatctgcctgtacagcaattacgcgggcgcccatagcggtaatgttgcttaccacttcatctgcagacgctttgtcttttgagtagttaaccactacatccgcacctaaagcggcataccgttctgcaatggctttacctaatcccctggctgatcctgtaatcagcgctactttattttttaagctgttcatgatattatatttaatacttttttagaaagaaggacactttatcctcaggccataccgccatttacaccaatattctgggcgttgatccatttggcgtcgtcacctgcgaggaatactactacctgtgcaatatcatccggttcgccaatacggttaaaggctgaaagggaagccagtcgcgcgatcacttcttctgatttaccattcgtaaataattcggtattggtagggccgggagaaacggagtttacattgatacccctggcgcctacttctttggagaacacgcgggtgagctgttccactgctgctttggtggccacataggtgccatatgcaggcagcataatacggtttacagaagtggagaagttaatgatactgcctttgtcggccaggcgggtagcggcctccctcatggtattgaaggtgcctcttacattaatgtcaaactgacgggtaaaatcttcatcggtggtatctttaatcagtttggtgatcatgatgccggcgttattcaccagtacatcgatacggccataatgcgcgatagcggcgtcaaacagggcttttacctcgtcgcttttgcttacatctgcctgcagtgcgatggcatcgccaccctgttgcctgatgtgttccaccacctgctgcgcggcatctttaccaccggcatagttaacgattacttttgcgcctgcggccgccagttggccggccattgtagcgccaatacctcttgaagaaccggtaaccaggatgatcttatcttttagcgtgctcatatttttgtgttttattttgataacacaaagatgagccaaccgttgccctgaaaagtataagaattacactaatagttacaaatatctaagatgcatgttgctttctgtatgaaacgggagaaataccggtttgcttcttaaaataattgctgaaatgagtggattctgtaaagcccagttgagcggcgatttgtttgatagacgcaggggaatgttgcagcaatgtacgggcttcggtgatcgttttctctgtaatccaggtacttatgggctttccggttttacttttaatcacattgctcaggtaattgggatgcaggtgttgtgcatcggcataatcctgtaccctgaataccttatctgccttcccgcttaccaggtcgcggtagtgctgctccagggttctcttaaactgttttacaatctgtgagctgcggttgccttcatatatagggttataatcttcccagaaatattctttgatcttcagcagcagcaccacaaacaggttccctatcatccgcgttctgtacgtagacgaggaaaaatactccttttctatctgcagatacaattgttcaaactccgcaaacacttccggctgcaatgtcctgggcggtacggtttccgccaggagaaaaggaaattcctcaaaaatcttctggtgtacattttccttcagaaaagattcactgagtgtaatcaggtgtacatcgttaatttcctgccattcaaaagatttaaaatgacccggattagtaaaataaatagttccgggagaagtgttaaaagtttgctcatcggtggtatacctgccaatagcatctttcacaaaaacaaaagaaaagaaattagtccggtatacgatggaagtataaggcagctcaaaatggatgtccttcaggttatgaatggtaaaggcggttttggcgtcgatgctgtccaccggtaaaccctggtaaatatactgatccagcagggtattgaatataatcctttcctcctggcgtgctttcttttctggcattcgatgttaggttgctttatgtgaagttaaataaaaagattctcctcatctttatgtgaattttcccttatttcgtcatcatactttcaaagctcccatgaaactactatacctgtttctgatttttaccttgctaacagtaccgcttagcgcgcagcttcccggcaacccggtctattttaagagcggcgcccagaagctgggtgtgagttcgtgcgaacaactaattatcacctcaagagccggagaaattgtaatggctgattctattcagggctattggaggtccgtactggtgaacacaaacccgaaaaaacccattacacgattaaatattgaacgtgccaccttcttcaaccgcgatacagggtttatttccggcttcatcgccggcagttccggtaaatatgatattatttaccgcaccactgattttggaaaaagctggacagtcgtggatgtcgggaaaagtggttggatggatggtgcgtcatggctcgataacggtgaagcatggttaaccgtttccggcaacggcattgttcataccgccgatttcggcgctacatgggatggcatgaacctccccggatggggaaatagtcaacgctacgaccagttgttctttactaccgggcatgagggaattaccggctctgtatggaacatactcgcgctattccatccggaaactgcctcctgggaaaaaatccctactccactggaccaaaaagcatatgccaaaaccaacatcgcgagcaggccatctatagctggcgtagccatttataaagattatctgttagctaaccaggaaggtttggtcttctacagccggaaagattcggtcaactggataccattgcccgactatgacaatttttatacagatgccgccaatacagcgctttattttcatggaagcaatggccagtttgttaaagcagatgatcaattgcagccggtattcaattacaataccgctgaaacctactacgatgcagtttgcaaaaatacgagcctgtttattttataccgaggcagaatgatgcagttaaaagctgaccggcaagttattacggccaatatgtatactatggataccactgttgccgaaccggaaatgattggctcttcgggcaaggaaaattttggcatactgggaaatgaaatcctggttcaaaaaggtaaagacgattcatggaaacattacctgaccttgcctatatctgccggaaatattgccggcatcagtatgagtaattccgttataaaatgtaatagcaaaaatgattcgctctatacttacaacatcagcacccgaagcgaagcaatgaaatccaataccgatatcatccgcgacttctgtatggcaggaatcaaaactattacttttacaagtggcagccagggctgcgatcaacaaacttacggcaaactcatgttccggaaaaccaagggaggatttgaagcggtagaagctccttcttccagtacctattcctcacaaatgattactgacgtgtcttttatagatgaagcaccggtacttaatttcattaacaatatcccgtcattaccaggcaaacaaaccaccattcagcaattgaatttttcagaagaggattacgcacaatgcaaaagtgatatccttacttttaagcgggatatcaacaacaataaactaaacatctatgcgaacaatctcaactttgaaaaattgctgtcaatagtggacagcgtaaaaaatatcgatccggcgctgcttaacaatatgttgcttaatatggaagacatagtcagcactaccagcttcacaaaaggtctgatactggtaaatcagaaagatgaggtgatgagcctttaccatggctattatgaaacttacaatccctggctgttcccctggaggtttcatataaatggtgttcatggaatgagtaatgctattgaaatttctgaatttatccgcaaagtatatccctcctttctatcgcggcctgataaaataacggctttgcgcacgatcgtaaaaaacctttatatgatagcaaagtaatactgcaacaaaatagacgggcatgaagcccgtttattttgttgcagtattgctactccctgatcgtattcttgtccgccagtgccatcttagcaatatcatctttccttttaaacgttacgccggcatgctttttcatataggcaaacaactcgctggtagcttttaccatttgcggggtaccgcctatcctgtcgtgaaaactgatagacatcatgcgttttcgccgggcagattcttcgtacaactgatcgaattccatctttatctgttgcaggaactgatcagtagaaaaccactggcctgctaccagctggatatcattacaacgtaaggtatatggtactactacaaagtcgctgccgttcacttcagtgataaaaggttcatcacggctcaggtcatcgatatgatacaggaagcccagttcctgcaggatattgagggtattatcgccccggcgcagccagttggcgttgtagcctaccggcgttacgccggtggcctttcttactgcttccacgccatcgctgataaactgtttttcttcttcataggacagcatgtattgcgacgaccagtcgcggccatgtgcggctgcctcatgcccgcgctgcacaatctctttcgcaagggccggatgcttttccaccgcgctgccaaccatatgggaggttacttttatgccgtgtttgtcccagttatccagcatgcggggaatgccttccttgaagccatactcgtaccatgtagtggcaggaaggtctttatagcctttgagcatattctgaggaaaagggctttcgggcctgtctggctggccgccggcttcaaactgcatagatactgatactacgaggcgcgagccatctgcccatccggcgccggatttggctgttggagtggctttcgcctgtgccaataccgttccgggcagtaccataccggctaaacctgcgaggccggctgttttcaggaattcttttcttgtagccattattttttaataagatgatcaactgcaattgtgttgtattggataaaagccagcagtacggcgaagaagacggcatggatcagttgggagggcaatgcttcccagttttctatcatggcagtgccaaatatcaggagcaccattactacacccccgccaataagggaagcacgggtaaataaccccagcaggagcagcagcccgattataaattcggcgataggcaaagcatagctgaaaggcactaccagcaagtcgggcaacatggatttttcaaagctttttaccatccaggcgctgaagccatttaatttagggagccttaccaggccgtgaccgaacatgctggcagctaccgccagccggagcaacagaaatacgatagggttgttttccatttgtttgattttttgtgacacaaagatcagccggaacccgggaaataatttgtacttttttaggatcattctgtacttttgcaggtatgctacaagagaatttatatcagccttttgagatagaataccgggaatgtacagaatgcccgatagatccgcataaacataacttttttgaactggtgtatattgtggaaggcagtgggatgcagtgtgtgaataagaaccagctgccgtacagcccggggaaactgttcctggtaatgccgcaggactgccactcatttgacgtgcaggaatctactaaattcttctttatccgctttaataacatctaccttcaaaatcagcataaagactggatacagcaactggaatttatttttcagaatcacaaccatatgccgggatgtatcttaaaaaataaaaatgataaaccgctggtaaaagcattggtagaggcgctgatccgcgagctggtaaaccagcagccctatcaccgggaaatggcccagcaaattgtaaataccatgatcatggtgattgcacggaatatactgctgcaaatgccggaacagcccaaacatcctgcgaaacaggatgcttccatgaatatattgcactatatacacgaaaatatttacacgcctgaaaagctgcgggcagagcagattgcagcccactttaatatctcgcccacttatctgagtgaatattttaaacgtaacaatggcgacagcctccagcaatacattacccagtacaaactgaagctggtggaaacacggctgcagtacagcagtatgcgggtaggggaaattgcggatgaactgggctttacagatgaaagtcacctgaacaggatgtttaaaaagtataaaggtgtaaacccttctgcttaccggaaagaactgcagctgcacgctaactgacgggcataaaaaagcgcccgcagtatgcggacgcctttttacaataccttttcctgttactattcttcgtcctcttcttcttctccatcatcttccagccactccatgtaagagtagtaccagtcttccagctgttccagcagttcctgtttcttttccggagcgcttttatagaattcctctacattatcgatttcatgaatgatatcgatgtaggcagtttcttcatcttcttctacccgtttggcaaagaagcggggtttctcggtatgaaaaatatattcattttccggatctgttacaggatcgtctgcaatcagaaatttaggtagctgtgccataaaggagttatttacttttaatgatgttgtactcttttcaagagctacaaaattattgataattagcttataaaaaacatgcagtgggaatgaataaatttattgattaaatttcacatctttatagtcgttaaaacccataccatatgcagcaatattggctaagatgggagaactggatgcagcagcacgcccccagactgcttaacatcctccatcccggcgttacttttgaggcggtggaatctcttgaaaaactaataggaacggccatgccggcctcttttaaagcattttatgctattcacaacggacagcagaaagccagggccgggctcgtagatgcggatcagctgttaagcgtggaagacatcaccacccaatggcatcactggaaagacctgctggatgccggaactttcaattatcacgaagaacccgtgctctccacacctgataccggcataaaaaacgattggtggaatcctttatggatcccttttaccggcgacggctttggtaaccacctgtgtatcgacctggaccccgcaccggaaggcaagcacggacaagtgatcacgttctggcatgacgacagtcaccgcgccattgtagccggttcttttgaagaatggctgcaggattatctcactgccctcgaaaagggagaatatatttttgtgaagaaatggggaatcgtgcacaaagacaccttcctgaactacaacgattgattatactgtaccggcgaactgcccgtccaccgcttaaaagcccttgtaaaagcacttaactcattataaccaagcatccaggaaacatctttcaaagggtaattaccggacgaaatataatacaccgccagtgaatgccgcaccgcatctgcaatatcctggtattttacaccctcctctttcagcttacgctgcaaactccggggactcatattgaaattggccgccatgtcgttcagcgacgacacgccgaggtatgaattcgccagcaggtaattatagatcctgttttgtaaagttttgtgctgacctgctgtttggggtaaactgcttaccttctgcaacaacaggttctgaagctcataattagccgttaacagtggctcatcccaatacctgctgtcaaataccaatgcatactctcctgcccgtttcgacggcttacaacgaaaaacacgctcatattcagcagggtccggaaccgtgtaggccagccgcgctgcctgcgggactattttttccagcagcaggccatccagttcatgaatcaccatcatcaataaaagatctatcaattgccggaaagcatagggtggcgctgcgccataatcaaccgccggcagcagccgcaccgtaaagtttttagcggtacgcgttacttccatccggcactcgtccgttaccaggtgcgttagcgctgcagcgtgagttaaggcctccccaacggtagcgctgctccggattatttctcccaccacccccagggcagcaggttgcagggactcgccaaagtgcaacccaaacaacggatcgttggttaaccggcccgcattcagccacaaatcctgcagctgttgtacagttaccggcactgcatgactccttttcaatgccgccaggtcaatacccgccagcttacaaagctgtgcagcatctacatcccgctgtacagcatacgcgataatactcaataccagctgtttcatatagcaaaggtatttcgtccggtgtttacaaaaatcatcctgtcgctaaatggtaagtaattgtcgtgtaaaggtaaatgataaaggggtggcagatggtagctttgcattatcaattcatcaacaactaaaaaagtatacaatggaacaacaaacactgcaggtagtaacagattttgtaaatgccgtacaacaggtaaaccttgaaaaactaggcgcactgctacatcccgaaataaactgggaacaaccgggcaacaaccgcttctccggcactaaaaaatccagcggggaagtattccagatggtaggcggtatgtttgaggtatcacagaataccatgtcactcgctgccatcaaaaccattgcagtacacggcgaccaggcatctgtagtacttacctggaaagcatcccggccgggagcggaactgcatacagataacgtagacgtatatacggtgaaagatggtaaaattgtggcagcgaaaatatatgcggaagatatccagcacgaaaatactttctggggcaattaaattacaattcaacacgggcaacaccttccggaccacgggcagtctggagggtgtttttttgtgcaaataattctcccgctgttacggataacagtcattttttagcatcaactaataaggagaaatcaactatcgtttagataatagctacgcgttactttaattctccccgtgaggtgtaggaacagatagatacagaccttcgactacttcacaggcagagggtttaccgtaaatgaatatacgaaatttaaatgatcccgccacgggaaattccccggtatgtaccagcaatgcggtaaaaaacacatttataaaaaactgtattacaataacaaaccaagtggcactattgttgaataataaccagcgtcaggcaatcatttttaaaaataaaaaagtaataacatgaaaactccaaaacttctgatagctgcggccatcggcgtagcagtaacactggccggtcagcatgcatttgcacagggaatcgacagcactgcaaaaaaagtgggaaataaaacagcctctatcgctgttaaaggagcctccaccattacagataaaacctttaaaggcaaggaaggccccaacggggaaaccgtttatattgacagaaaagacaggaaatacattgtagatggaaaaggtaagaaagtgtatctgaagaaatcacagatacatgataagaaaaaagactaaatctacactgccataaagtaagccggccagggaaacctgccggcttttttattgccacaaaaaacagtaatggaagataattccatgacaacaagcccgatatttgttacgtatattcatattgccattaaatacccacttatgcaactgaaaccaggcacctgttacaaggtaaataccaggaccattgcagcgctgcagcaatttggtgaatacgagtttgtagtagccgttattcacgccaacgatacctccgacagcgtggtttttgaacttaaaaaactgctgggacactacagcaccgaacaggaaatagccacccgccaggccattgaaactcatgccgatggtttctcactggaagatatcaccgggcatcaacttaacctgctacaatttgaaagggaaagcgcttttataaaatggatcgcagaaggcattgcggtgccgtacgactgtaacgcgtaaataattactcgtaacgcaacgcttcaataggatccagccgggaggccgcctgcgccggatagtaaccaaaaaacaccccggtaaaggcgcataccacaaaggaaagtataatagaagactccgacaccagcgtaggccagccaagcgtgagcgtaattaccttggcagaagtaatccccaacaccacccctattaaaccacccgttacgctgataataattgcctctaccaggaattgcaataaaatatcaatgccccgcgcgccgatagacatgcgcagccctatttcccgggtgcgttccgttactgatacatacatgatgttcatgataccaatgcccccaatcaccagtgaaataccggcaatagcggtcaacaggatagtaagcaggctggtagtggaactcagcgtttttatcagttcctccatggtcctcacctggaaattattttcatcggcaggacgcaaacggtgtgttgttctgagtatatctataatttcattggtagcctgctctgaagcgccttcgcttaccgcggaagcataaatactctggaaataaatggtcgccaggatacgtttttgcacagtggtgtaaggcgtcaggatgatatcatcctggtcctgcccgaaagagctctgtcctttcggcgccagcgtgcctattacctgcaatggaatggaacccaggcggattacttttcctacaggactctctccactgggaaacaggttgttgatcaccgtttgccccaatacacacactttcgcagcagtagccacatctgcatcggaaaaactgatgccatcattcaccgtaagcttgcggatatcaaaataagaaggggccacgccctgcagggatgtaggccagttcagcgcgccgtaaatagcctgccctttggtagacgctaccggcgacaccgcgcttacatattccgcattcttttgtatcgctaatacatctgtgatagtaagcgactgaaagctttctcctcctatcctcaccccaccggctacgttgctgcttggcaaaatggtgatcatgttagagcccatgctgctcaactgcgactggatactttctttcgagccctgcccgatggccaccatcgcaataacagcggccacaccgatgatgattcccagcatcgtgaggaatgcccgcagcttattgcgctgcaatgcctttaacgctatcattatgagattgactgcactcatgctttcgctgaattaataatcttcggccggaggcaatgatgccagtgcttccttcgccgagcgtatgttttcattcttgctgtctttcaccacttttccatcccgcaacatcaccgttctgctgctgaaggccgctatatccggttcatgtgtaacaaatacaatcgttttgccttcctggttaaggtcctgcatcagggccataatttcgtaagaagtacgggtatccaggttgccggtggcctcatctgccaggatcatgaccggctgattgaccaacgccctggcaatagctaccctttgttgctgcccgccggaaagctggctgggcgtatgatcttccctgtcggccagtttcaccgcctggagcgcccccagcgccctgttacgccgctcctgcacagataactcggggttgtaaaacaacggcagctccacattttccaatgcagaggtacgcggtaacaggttgtatgcctggaacacaaatccaattttatgattccgtaaccgggccagttcattgcgcgacaggttactcacattcacgccatccagcaggtaactccccgacgtaggtttatcgaggcagccgagaatattcagcaacgtggttttccccgaaccgctgcttcccataatcgtcacaaattcgcctgcaaacacatcaaaagacacgcctttcaatgcgcggaccgtttcagtccccatcacaaactcacgcttgacctgctgtagctccaatattttgctgctgctcatcgtcttcgccctcccatttttggtaaaaacggactggtatttcctcccgcggccgccacggctcccccggcgctgacgcccgttaccaccacatcattttcgtttagccctgagagtacttcaatatgcgtattgtcgtttagtcctgttcttacatgtttttgcaccagcgtatcaccgcgtaatatccatacataattggaggaacctatacgcgtggtgcttttaaacttaccacccgtagtatcctttgtttgagcggggttacgggttctcctcacggcgctttgtatcacataatcctttagctgtactgagtcgggaataaatttaagtgcctttacgggcagcagcagcgcggagtctttttccgcggtataaatcgtaacgttggccgtcatacccggtttcagcttcctgttatcattcggtgcgttaataatcgtattgtaggtaaccacgttggaagacaccgatggctgcagcctgatttcctggacacttccggcaaaaatatcttccaggtaagcatctacggtgaaggttacacgaagtgagtcttttacattgccgatatctgcttcgtctacgctggcttctacctgcatcttggtgatatccttggcgattacaaacaaggtaggcgtattgaaactggcggccacggtttgtcctacgcttacattccggttcagtaccaccccgtcgatcggtgaatggatttctgtaaaagagaaattctttaatgccgaattcagctgggcggttacgctggccacatttgctttggcctgccctatctggttggcagcaatatcgtggtcggctttgctgatggcgccggttttatacaacaattcctgccgctggaaattattcctctggtattccaggttggtttgcgctacctgtacattggcccgcagctgatctacctgtgcctggaaaagatctttatccagttccgccagcagttgtccttttttcacctgggtgttaaagtccacgtataaatatttgagcgtgccggacacctgggtacccaccgctaccgtatctaccggctgtatagtaccggtagcggttacggtagtggctatgtgcccgtattccggtttggcggtatcaaacctgaccggttcttttttcttcctgataaagaaaaaccagatcgccaccagcagcagtacgatcaccaccgttatgataacacctttatattttctcatacctcaatttacatttatagttttaccggtatgcccctgtaaaaatcatatatcctgatgttcagagcagcattgtatttcgcctgtatataagattgtaatgcctgtatatataaattcttctgctgaagaaaaaccacgatattggcagcgcccacttttaattgttcgctggcaatccggtaaccttcctgtgaatattttaactgctccacggcagcatcgtactgcgactgcgcattgagcacatctatatatgactgttctatcgtttgggtaagatttgttttggtatcctgcaacaccagcttcgactgatccacctctatttttgctttttccacattggttttcacgacccgccgggtgaagatgggaacagataaagtgagccctatctgctgataaaaattattatccatttgcttgaaataagcgctgttggctcctccgctaacataagaagatcctaatgcgcctccggctgtaagcgtaggcaaatacccggcccgcgcctttgccaggtccaggtccgatacctggatgccgagttcactgcttttaatttccggcctgttggccagtgcagagtcctgtacttcctgtaaggcatacagccgcgtgttggtgatcagtgtatccggctcctggatttcaaaatcatagctgctgggcagttgcaacagttgtttcagcaccagcttgttctgcctgtgctggttttcggcggttaccagcaggtaacggtcgttcgacagctgcgcctttaactgcaccagtcctatcagggcaatgctgcccacatcatattgttgttgtccctgcttcacctgcgcttcagaggtggctaccacgtcctgcacatatacaatgttttcctttgccagcaggatattcagataggcttgtgtaatcagtaccgtgatatcatttacctgctgggcaatattcagtcctgccatctgcgtgagcaggttcttctgcttaatatcattattaagatatccgccctggaaaagggtaacgttggaattaacgccataattaccggtggtatttacccggtaagaagaattgccggtagcggtaacagatttgccgccattaagatcctgggaaacggaccccgtaagattaggcagcttggccgcacgcgacagcagcagatcctggtcactgctcattttgctcaggcgcaggctgtttaactggatattgtttttcagcgcataatcgaaacactgttgtaaagtccactgtgcggggagctgctgcacggtgctatcctgtgcgttcagcctgggtgtcactgacaacaaaaaaataaaaatgaatagaaatcttccgggctgtctgaaaaacatcatcgtataatcattgatgttagtaaaggctacaactggaataaggggccaaatagtaatacaagataacgaattatgatggtattaataaacgaaaaacggacccatagaaagataataacggataactcgtccgtttgttctctccatagatccgtaaattaccatctccgtcctatcggtttctttgcctggtttgccggcctgttatacagcgttcttaaaagttgcgtttgaccggcccgttccctgcggagggccctggtgccagttttcatcgtagtatacaaaaaaggccatccagatggtacgggaccatcgcatcagcaggggttgcaggattagcagcaacagggcgtttaccccaagccaccagaaaatccggttatcgtaaatggagaagccgatgaacagccaccaggcaatgaggctggccacgcacaccgcaatggacagtgcatagctcacatagccggtaccgtagtaaaagcctacttccacttccaccggctgaccgcataccgggcaaacatcgggcatctttaagcagtttttcaggtcgtagggatttggggtagtatagatagatccccttctgcaacgggcgcacttgttccccaacaggcttttcagcaggctgggttttacattatttttatctgcacacatataatgaagatttatcaggaaatatgtttccggaactcttccggtgttgttcctgcgtattttttaaaaaacttcgtgaagtaagaattgtccgcaaaactgagctggtaggcaatagtggcaatactcatatcggcattgatcaataaccgttttgcttccagcagtacgcggtcgcggataatttccccggccgattttcccagcatatgccggcaaaaggcattgagataattaggtgttacatacagcagggcggcatattctttcggcaaccgcagctgcatataatgctgttccaccagcttgcggaaattgcgcagcagcacataattatgcggcaattcctgacgggtttccccctgcctgctggcgcggcttacggcaataaacattcccaggacctgtaaccgcagcatatcctggctgtaagcctggtcacctttcatttctttcagcatgccttcaaactgcgcggttacaacggggatagcggctttaggcaactgtactactccttctgcgcttaccccgctgaaaaaaggaaaccgttccacgtaatcagcatcctgcaggaaggcattaaaaaaaccggcagatacattcattacgtaaccttctatcccgccggaaaaaaaccagctgtgtacctggccgggtaccataaaatataattgtccgggctttaccgggaatttttcaaagtcgatcgtatgacttccacccccggcagtaaaaaatgccagatgataaaatgaatgccggtgaggaaaatgaatatcccggtgtgctgccaggtaatcggaaaacctggccaccagtatatcttccgatgccggctttcccatagccagggaacagatatcgtatgttggaatgagcgcctttgacatgatgcaacaaaggtacaaaggaagtaagaacgggggttgtggtattaggggctttaatggtactttttacttatcgtaataatttctgtgatgatccgggcggatcatcacagaaattacggggtaatatttattgttttacatatttcatcagccattcgtccatttcccacagcatatgcaggatactttccttagcggcatagccgtggctttcctgcggcaggaataccaggcgcgccgtgccgccattgcctttaatggcgttatacagtcgctcgctttggatagggaatgtgccggagttattatcggcttccccgtgaatcaggagaatgggcgttttcagcttatctgcataagagaaaggcgacattttataatacacttccggcgcctgccagtaagtgcgttgttcgttctggaatccgaatggcgttaatgtacggttataagcgccgctgcgggaaatacctgctctaaacaggttcgtatgtgcgagcaggttagatgtcataaaggcgccgtaagaatggccaccaactgctatacggtccttatcacccacgcctatttccgtgatcttgttcacggcggcttccgcattcatcaccagctgatcgataaaagtatcatttggttctttatctccttcacccacaataggcatttcggtagcatccattaccgcaaaaccgcgggttacccaaaaaataggcgagccatagtttacgcgggtaaacctgtaggcagaaccacgtacctgggcggcatcgctggcagatttgtattcacgtggataagcccacatcagcaccggcaggcggccatctttggcagggtcgtaaccttccggcaggtataacatagcggtgaggtccaccccatctttgcgtttgtatttcagcagttgtttctgcacgcctttcagttgtggctgtggatgcggaaatgcagtaagcgccacggatgatttctttttcaggttttgcaggtagtagtttacgggagatgaaaccgattcgcgtgctatcactaccacgagtttggcaggatcaatcacatcggccacctgttcgtaataaggtgcagcggagcgccacaggatattttgtttgccgttatttaaattaaaggaagacaggaacgggcggtctccttcaggagaagcgcctggcgccgtcatcagcaattcatgtgaaggcgacacgtataaaacagccctgttgtattggttctttattgttacaggtgtgcccggatcgttataccggtcgttttcagaacgatcgatcagcgtaaccggcgcctgcgaagggtttgcagggtttatgcggcttacctttattttctgttgcgtgctgttggcgtcatacaccagtgccagctggtcatttgcccagctgatacccgcgaagcggttcacggttttcaccaattcctgcggtgctgcgctgaatggagcggccagggtatttactacatcgcggaaaggcacttcctttttaggatcgccgccatcgagggcctgtacccaccagatagtggctggtgcgtcgttacgccaggagaagaaacgggggtaattgctggtagcatcaaaacctttgggccgtacctcatccagcgggttgctggcgagtttctttaccagttcgccattcattttccatatttccacttccgtggggaaacggtgggcgcctaccaggtaagaatatgggcggtgcaggctttccatcagcaggtattgattatccggcgatggagcggcggtgatgtaaatagcgggtttaccgattacctgttcgccgctggcgcctataatcaccggttcggattgaaagtaataatcgaacagctgttcgtcgtatggatttttcagcatgtcctggtaagtggctgccggcgctgctttaccggaagtttgttgtacggtggggcctgcgggcgcaaggggtttttccggtgctttgccaatagcggcgggtactgccagtgccaggatgcggttatcatcgatccaggtaaatgccgggcctgcaatgtcgttgagggcacgtgtactttgctgtttggcggcgccggtagcaacatccgctttccataaggtaatgcggttgttgtctgtaatggtgaaggcaatacttttctgcgatggcgaccagctgatattgccaatacgcgcattggcaggcaggccggtgacggcgtattcgctgttgcccttaatatttttaatacggatagctgtaatgtaacctgcgcggcttggcccgaagttagcagggttaatacgtgttcctgccagcctgtattccggttgcgataattcttcaatagttgggtaactggttcgctccatgatcagcatcacatctcctttgctgctaaagtctgttgatggcgaaggagctgccatcgccagttccaggatactctttgggggagtctggtacttcagcgcatcctgcgcataggcatggaaggtgatgaataaggataatgacagtattaattttctcatatagcagataatgtttataagcaatccgggcaaaataaacttattgccacagtttgcaaagcagaaaatgatgaatgaaagtagggtaaactttaaccaggattaacgggcaggcgtgtaaacctttttcaggacttagccggggtggaagtgtatggggagtgtatggggagtgtatggggagtgtatgaggagtgtatcatgagtgtatgagaagtgtatgggaagtgtatagggactataaggagagtatatggggactatagggggagtatatggggactatagggggactatatggggagtacgacacatacgctactcctaagtaactgagaagtatccgagaagtatcccagaagtatcccagaagtaatagctgcataattcatcacgccatctatcccctcctctctaaaataaatgaaaaagtaaaaagttctgttatctttgcaaacatcagatgatatgatgactacaaatacttctcctttaaaacgactcagcctggctgaagaggtagcggaccgcctgcaggaactgatcgcttccggtaaatacgccgtggggcaacagttgcctacagaacctgagctgatgttacagttttccgtggggcgttccagcatccgggaagcagtaaaaatactggcgcaccgggggctggtgcgggtacaacaggggttgggtacctttgtgttatcacaatcaggcacgggagaagcgctatcgcagcggctgcagcgggccgatttcaaagacctgaatgaagtgcgcttcctgctggaagttaagattgcggaaaaagccgccatgcaccgcaacaacaaggatattgaaaagatgaaaggcttcctgaaaaaacgttttgaatatgcatccggcaaccagctggagctttgtatccaggcggatatcaactttcacaacgccatagcggaagcaggtaaaaatgaaattatgcgggacctgtacaaaacagtggcagagcacctgaaaaagtcgttcctgctgcggtatgccaatacagatacctttgttgacacacagcattatcacgacgcactgctgcaaagcattatagataaagatcccaaaaaggcgctggtttgggcaacgaaaatcagtgaccagaacaaataatttttttacccttaaacatcagatgatctgatcttaaaagaacagaaatggaaacaacattaccagaacagcacaaagccgccacgcaacaggcagcacaacaaacggtgctgtcgatcctattggcgttaagttttacccacttcctgaatgacaccctgcaatcgctcattccggcgatgtacccggtactcaaaaattcattgaaattaaattttacacaggtagggcttattaccctcaccttccagatgtcggcatcactgctgcaaccgctggtgggcctgtacaccgataaaaagccacagccttattcactggccattggcatgagtttctccctgcttggactggtatgtttatccttgtcgcacagcttcccgatggtgctggtatcagtaggactggtaggcgttggctctgcggtgtttcacccggaagcctcccggctggcgcatatggcctccggcggaaaacacggcatggcgcaatcactattccaggtaggcggtaacgccggcagttcacttggaccgctactcgcggcgatggtgattgttcctttcggacagtttcatgtgatctggttttccatagccgccttgctcgcgattgtggtaatgctgaacatcagcaaatggtatctttccaatacacaccgcatcaaacccaaaaaagctgcattggacctgaacaagccgaaactatccaattccactgtgatattttcattgggtatcctgctggtgctgatcttctccaaatacttttacatggccagtatgaccagctactatactttttacctgatggaccgcttccatatttccacgcaggcttcgcaggtgtacctgttcatcttcctgtttgccgtagcggcaggtacctttatcggcggccctgtcggcgaccggatcgggcgtaaatatgtgatctggatctctatcctgggtgtggcgccgttttcgttattgctgccacatgccaccctgttctggacggcggtactcagtgtattcattggcgttatactctcttccgctttctctgccatccttgtttacgcacaggaactggtaccgggtaaggtaggcatgattgcgggattattttttgggcttgcctttggtatggccggcgtaggctccgccctgctgggccgcctggcagatgccaccagcatttcctacgtataccaggtttgcgcctatcttcctttaatagggctccttaccggtttgttaccgaatcttgaaaaaaagaaatagcctcgtttagcggaggcgatggcctccgctaaattcacatacattcgcagcactaaaacaattcttatgtggaaaggcatactgcttgtgctgcttggcgcatgcagctttgggatattatcaacgatcgttaaatcaggctatcagcaagggtatacattaggcgaattatgcagtgtgcaggcgggcttcggcatgcttgctttatggattatccaggcattttccggcaggaaaacagtgggcctggctaacagggatgcccgtacctgctttatcctgggcagttccacaggattggtaagcattacttattatcagagtgtacaatatattccggcaagcattgccatcatattactgatgcagtttacctggatgagcatgctggccgaatggattatttataaaaagcggccttcccccatacaatggctggcagtatttttcattcttggcggcaccctgctggcgggaggcgtatttaaccacacagaaaccgcgctgaactggaaaggtatcggcttcggtttgctggcagccctgtgttatacggtatttatagtagtaagcggccgggtagcggcatcgctgggaccggtgctgaaaagcgcctggatcgttaccggcgcatttgtactcatcagcctcatcttccctccgctgtacctgtttaatggccggtttaccggcaccagcctgtggatctggggaattccgctttcactttttggtaccgtgctgccacctttccttttttcaaaggggatgccgcaaacgggggtatcgctgggcgccatcctcagtgccgccgagctgcccgtggccatgctggccgctaccattttccttcatgaatccgtatcgcccctgcagatactcggagtggccatcatattaagcgccatcgccatggcgaatctgaaacgccggaaatgaaaacccatgaggtgttttttttatttatctttgcaccctctattagtgatttacgaactgttttttcatgaaagcatttaatttttttattctatatcgcctcccgatcggtattattttactggcaggcggtattgcgctgggccttactgttggctggtgggaagccaccattgtgctggtgctggcactggtatgtttggtaacacatgtgatgtttggtcccatgagaatggtacaggaagccgtggaagccggcgacattgaaagggccaccgccctgatgaaccaggtaaagttcccgaaactgttgtacaaacccatccgctctgtgtattattttatgcaaagcaacatggccatgtattccaatgatcttgataaagctgaatccaccatccgccagagcattaactccggcagcccgatgaaagaatacgaggggatgcagtattttcagctgggcactatcgcctatcagaaaaatgacctgaaaacagccgatcagaacctgaaaattgcgatgcggaaaggcttgccggataaggaaaacacggcagcagccctgttaacactggcttctattgccatgagccgccgcgacttcaaatctgccaaggaatatttccgcagggccaaagctcaaaagcctaccactgcgcagatcgtaagccagatcaaagaaatggataaatatatttcccggatgccgggataagtaaattgcctggggcaatttacctttgaaaatgcagcggagataaagtaacctaacctttgtcccagctgcatttttattttgataaaccttcaactaatatttcgcggatgcaattaaaactttacacttccttatttttatctaccgcgctgtatactgctgctgccgcacaggataccagccgtatcagccagctgaatgaaattaccgttaccgccgctaaaggtccgcaaaaggccggggaaaccggcaaggtggttaccatcctttcacacgaatacctggagcgcaacagcggcagaagcattgccggcatcctcaaccagcaaaccggcctgatcatcaacggcgctgaaaacaacccgggtacagtacccaatgtgtatatgcgtggggcctccaacggtaataccctgatccttgtggacgggctgccggtaagcgacgcctcccagatcaataatacctttgatctcaacttcatttcccccgaccaggtagaacggatagaaatactccggggcagccagtccaccctgtacggctccaatgcagtagcaggcgtgatcaacatcattacccgcaaaaccggcagtaaaaagtttggtgtgggcgccagtgccagctatggcagctatcacgatttccagggcaatgtaaatgtgcatggcaatgttaaccgcttctcttacctggtaagctataaacatgaaaaaaccaggggcttctccgatgcttatgactctacctataaagccggatttgataaagacggcttccggcaaaacagcgtttttgccaaactgggtctggcagcaggaaaacgctggaacttcggctacctgctgaattacagcaattaccgccacgacctggatgaaggcggctataaagatgaaacggattataacggcaaatcaaagtacctgctcaacggatttaacagtgaataccgctttaaaaacggctcctggcatgtattatacagctaccagcataccaaacgggatattttaaacgattccggctatgtaggcgtgggtgcttatgcccggtacgacagctccctgtttaccgccaacacccaccaggtggaaagttatgtgaacctggacctgagcagccggatcaggctgatcggaggcgctgcctataaccgttccgccaccgatcaaaaagacttcctggaaagcaccttcatgccggggatcgttaacaccacgttatcgccggatagctcgcacactagccagatcagcgtatacgcctcgttcctgctgcgtaacatgggtggctttaatctcgaagtgggcggccggtttaatcatcacaacctgtatggtaataacgaaaccttctccattaatccatcttacctgattaatccgaatcataaggtatttatcaatatatcttctgcctacagcgttccaactttataccagctgtatgcaaatggctatggcaaccgggatctgaagccggaaaccactaccaattacgaagccggttaccaggccaatgtggctgatggcaaaatagatttccgggtaaccggttttgcccgtaatacccgcgacctggtgatcttttattttgatcctgtcacctttttcagccagtaccgtaatgccaataaacaaaaggcatatggcgctgaagtggaagctacctggagaattaccaggaccctgcagctaaccgccaattacgcctatgtggatggccgtgttacggtgaaccagaacggcaaggattcttcctactacaacctgtaccggatacctaaacacgcggtgaacgccactttaggttaccaggcaacccggtcgctgtacgtggcggccaccggtaaatacatagataagcggtttgaaggcgccaaaccgatgggggattattataccctggatttatatggtgaatataaatttggtaacttgcttaaaattttcgccggtttcagaaatattacagattatcagtattttgatatctcgggttataattcacgccggttcaattttaataccggtattgtatttaatttgtaaacattaaaaccaacataatgtctttaaagaatcttaatccacggtttggcgtactgctgctgtttatactggcagctggtgtaatacgtatcgtgttgggatcagatgccaccatgcaaccaatcgccatgtttacgccggtaggcgcaatggctttatttggcggcgcttctttttcgcagaagtggaaatcatacgcctttcctttattgacgctgtttgtgagcgacattatcctgatgcaggttttccataagcaatatgcagaaggcttgctgtacaggggctgggtatggaactacgccagctttgtgctgatcgtattactgggtcagcttttaatcaagaaagcaagcgtggccaacatcctgatgggttctgcaggcgcagcgctgctgcacttcctggtgtccaacttcggcgtgtgggtaagcggttctaccaacctgctcaccggattaccgtacaccaaagatgccgccggattagcaagctgctatatccaggcgatcccttacatgtggtatgtgctggtaggcaatatcgtttacagcagcattttctttggcagcttcgaactggttaaacgcagattgcgttttgctcaataatatttttacatttgttttttagagatttgggctcaggcagatgaacacatttgtctgactctaaatctctaaattattatagggattcactatttctctcttctgcatagcatttctgtattagcaccctggctacagtttaactgtaatacccatacgaaaacaagacatacgaaaataaatcacaacacatgcgcagcatttcacgcaaatttcaggtttcctttattgcagcagtattcgctattgcaggactagcctcctgttccaaagataatgaggcagaagtaattgtaccacagattgtagctccgggcttaaaagacggcaaagacaccatctatattggcgacacccgggtgttaagcccgcaactggcagaggtgaagaaccctacttttctctggctggtaaatggcgtacaggtaagcaccgattctacctatactttcaccgcagcagaaaggggtgattataccatctcttataaaataatttccggtaacgcactggccacctactattaccgcatcaaggtgctgggcaaatttgaaaatggttttttcctggtaaatgaaggccagtatggtaaggaaagcggcgatgtgaatttttaccgcaacggggaagattccgtttaccagtacgtatttaagcgtaataaccccggcaagcaactcggtggcaccaccgactacggcgccatttacaacaataaaatgtacctcgtatccaaagagggcgccttcgtggtagcagatcccggcaccatgaaagaaaccggccgcattgatcagctgccggcttttgccaatgccttctgcggcgtgaacagcaataccggtttaataagcactgcggatggtgtataccccgtaaatctgcaaacactggccctgggcagtaaactggccggcgtaaccggacaggtaggtggtatggtagcagcagaaggctacatcatcgttatgtcggaatcacagggtatggtggcattaaataaaaccgatttaagcgtgtcaaaagtattaggccctgcggatgtaggtttcacccgcacaccggatggtaccgtttgggccgcccgcaataacatgctgtttgctattaatgccaacaacctgaaaatagataccgttaccgttccattcccggtatatggcgcatggggcgcatggaatgcaggtatgctcagcgcatcaactattgaaaacgccgtattcattggcaaaaccaatgcctggggcgccggtggcagggaagtatacaaatatgcagtagggaaccctaactccctgaatacgccgtttgtaaccattccggccggccgtgaaatgtatggcgcaggtgtaagatataatcccggtaacaataccatcatagtaactgacgtaaaatccggttacggcgataactataaagataatacgctgtacatctatgatgccagcagcggcagcctgaagaaaagcgtgaacttcatgggcttcttcttcccggcaatgccgttatttaactaataacttccggtggttggctcttataaaaagccaaccaccgggaaaggctaaaagcttttctatgcttcacttaattacaggcggcgcccgttcgggtaaaagcaggtacgcacaggagctggccttatcacaaagcgctcacccggtatatgtggctaccgccaaagtatgggacgatgactttgcacaacgcatacaacggcataaagcagaaagaggatccgcatgggtgaactatgaagaagagctgtatgtaagccggctcccgctggacggccataccgtagtgatcgactgtattaccctgtggctcgccaacttctttactgaacatcattaccataccgataataccctccaggccatccaggcagaaatacacgcacttcaccagaaagcaggtacttttattattgtgaccaatgaaattggaatgggcgtgcatgccgaaacggaagcggggcgcaagtttacagacttacagggttgggtgaaccagtacattgcccgtatagccggcaccgttaccctgatggtttccggcattccggttgtaattaaaaaagacgcgtaaaaaaattcctcatgatgaatgatatccggataacacctgtatcacccgagctgagaactgccttacaggacaagatagatcagaagaccaagccacccggatcgctgggcagactggaacaaattgcgttacaggccggcctggtgcaaaatacactgacgccttccgtgaagaaccccgctatcattgtatttgcaggcgatcatggcatcgccgccgacggacaggtaaatccttttccacaagccgttaccgcgcagatggtgtataattttctgaatggcggcgcagccatcaacgtgttttgcaggcagcatcagctggacctgacagtagtagatgccggggtaaatcatgagtttgcgccgcatccgcaattgaaagaccgtaaaatgggtatgggtacgcaaaactttttgcatatgccggccatgtcgctggaccagtgtaaattggccatgcaggcgggcgccgccgaggtaaagctgctccacgaaaaaggttgcaatgtggttggttttggagaaatgggcatcggtaatacctccgcagcatcgttgctgatgagccactttaccggcatagcggtggccgaatgcaccggcgccggcactggcagcaacacgcagcaactggcgcaaaaaagggccattctgcaacaggtaatggctaaacatgcctcgccggcatcgccggagcaggccctcgctacattcggcggctttgaaattgccatgatctgcggcgccatccagcaggctgcggccttgaaaatgctgatagtaatagatggctttattgtaaccgccgctttgctggccgccgtgaaaatgcaacctgcggtgaaagactattgcatcttcgcccattgctctgaagaaaaagggcataaagccatgctgcagcatcttgaagtaacgccgcttttacagatggacatgcgtttgggagaaggcaccggcgcggccctggccatcccgctgattcgcagcgcggtagcttttttggaagaaatggccagttttaacagtgctcaggtatcaaaccgtactatatgaaaaaacagtggcagctattgctaaccgctatcatgttctatacgcgtatacacgttcccgttaatatcccctactccccggagatgctcagcaaagctacccgctatctcccgttgataggatggataaccggtgcaattatgataggcgtattgtacatcctggggggcattgcgccgccaatggtgagcattctgctggctatcattgtgggcgtatgggtaaccggcgcttttcatgaagacggatttgccgacatgtgtgatggttttggcggcggttggaccaaagagaagatcctggagatcatgaaagacagccgcattggcacttacgggatgctggggctgttgctgatcatgactcttaaatacctgtcgctccgcgaactgtcgctttacaaagtaatgctcacgattgcaagtgcgcagccattgagccgctttgtagcggtaacggtggtatatacccacaaatatgtccgggaaaacgaagacagcaaagcgaagcccattgcccagggcatttctttaccggacctgggaatagccgccatatggggctttattccttttatcgcagccatgatttacctgcataactataccctgctgcttaccctccccaccctgatactggcccgctggtatatggtgcggctcatgcagaagtggataggcggctataccggcgattgcctgggcgccgtacagcaggtatcggaaactgttatttacttatgcttttgtattcttacatggaaatatatctgatccggcataccacgccggcaatagaaagtggtatttgttatggcgcttcggacgtggatgtagcaggcagttttgataccgaagcagcccgtataaagccgctcctgccggccggccctgtagatgtatataccagccctttgcagcgttgtgagaagctggctgtcgccttgtatggcagccattacattaaagacgaccggctaaaggaaatgaattttggcaactgggaaatgttgccttgggataacatcagcaaaaatgcgttaagcaaatgggccgataacgtagtatttgaacacattccgggcggggaaagctatgaagaattatataaccgtagtatacaggttctggaagaaataaccgccgccggcagggataccgtgttaattacacacggcggggtgatccgctgtatagtggcgcatgtgactgatacgccgctcgtggatgcgttcgatatttcggtggattatgggcatatttcgcatttgcaagtagagaacggagaggcaaaagtgatattttctaatctgtaaacaactggctttaagccaattatattaatatttttaaatatctccctaaaaaacaaaaaaactggtaattcgtgctaactttatgtttgcatataccgtatataaaagcacataataaaatctgttataatgacaacatcttttctgaacatcccgcttttgtttttgcaggaaataggtatcaaagaattactgctgatagcattagtagtattgttattgtttggtggtaagaagatacctgagctgatgcgtggtttgggtagcggcatacgtgaatttaaagatgccaaagatgaaccaggcaaaaaaggaactaaagctgacgcgacagacgctaaagcgaattaaattcctgttataaaaacgaacggcaaattgcgcattcagcatgcacgatttgccgtttttttatgcattccccgccattggtcaggctgcaatctgtacttctcgcccgaggtttgaagtacttttattgttcactgattcatatctttttttaaaataccaggcagaagctatcatcattactatgccggtaacggatacgcccagtactgcatccataaaaaactggctccacgacaaagccatgccactgaagtttttaaacagcatcaccagcacacttcccaggtaaccaaaagaatcggccacataaatgataaagcccacattgctgacgtatttaaacactgcaatcaggcgttcaaagaaaatacagttaaacgggatatatcccatatacaagcccaagccggttaaagtcatccaccataccgggtcaagccggtgctgcttgtataacagggtactgatcaatgccaccaggaatccggtgatcacaataaagtgattcagcataaaggcatgaaaattattcttcacaaataccagcaaccccataatcacaatgatagccactgacacaggaatttcggtttgagtgaagatgcctgcctgggcgccatagccaagatctttccagatatctgccgcaaaattatcccgcatatcccttaatacggtgagcaacacatagctggcaatcaatagcaccagccccggtaaaaaagcctggagaaacgcctttctctccggtttattcataggcgcgcggcgtgttctcaattgctcatctgctgctgtaggaggcggtatctgttccagcaacaatatgcaaatcataataggcactataaaaataaggcccgtgataaaaggcatccaatactctgttacatgccagttcaccaccgtcattttacccaccgactttacaaatcccgaagaaaaaataaagctgacagacaacaccgcacccataaattcggtgctgcgccggccttccaggtaactgaataccagcccccagatcatgcccagcggaaacccgttgagaaaaagaaatgcgatattatacggcgccggtaccaccgcaaaacaaaacagcgctatccacgctatccctatcaacaccataatactctgcgcccgcttgttccccttcatttccgcaataaaacggataccataaaatttactacaggcataaccaattgtttgggtaattaccagccagatcttgtaatcaatacccaggaaagtaacgccctcgaaaatccccgccgtaaaaggcttacggaaagcatacatgcaggaataagtaccaaaggccaccagggcagcatacaatgaaaatgtaagatgatgcgcctgctgcaaccgcttctgtatccaggtaatattcaacatcgtaaacaaatggtttgggacaaaggtgagagtccaatgtaaaccaattgttaacaaatgctgaacttaatgttaagtattattaaacacagaggcggattttgtcttggctcaggattacgctgattatactgattaactggatttttactttttgatttttttggatttttagattaataattaagggagatgaaaacgaatatatccgcttctatctcccttaatcctttaaaaaatcaaaaagtaaaaatccagttaatcagtataatcagcgtaatcctgagccaagacaaaattcgcgccttcctatttcagcagccacatatccgcgttgatgtcgtctgtggtgccgccaaactggtttttcagggaggcggtccagttgatggtattggaagagcggtcggaatcaggatacttgaaacgtttggggataatgccgctgttgcccgtaccggagcctacgctgaaagtggggatgccggttcttctccagttgatataagcttcccagcccgagttttcaaaaaaggcgaggtatttctgggtcaggatttgcgcaagtccctgtgcattgttgcctttatattgcacgttcgcttgtttataatagttgttttcaaaatcgaacggtacttcataacgttgaccaccatacgttttaataatggagccggcagcttcggccggaatgctataaaagctgagagaggctttgatcccctttttataccaggcttctgcatctgcctgtatccagccacggttggccgcttcggccaggttaaagcataactccgggaaaccaagcaatacgcccggctcagcggcataactgctgtaatagcggctgcggctgcgaacggaatatactgcattatttacatcagacatttttgaagacatattatccaggctttcaccggaagcggcgcccacataagcagtgatatcagctggtgacttacccagcttattcacctgttcagtggctggttctgcggttatatatgcccgcggatcattgagcgctaccagagtattcagataggtggcagacatattataccgcgtagcatcgaagcccaggttatccgggttggatggatatttattgatgttgttgtagataaattgcaggttctgatcggccgattccatcagcggatatttagcaggattgctaacaatatctttaaactgctgggctactttcagatcagcatcggctgctttcttacttaaagtaatgagcacccgcaaacggaaagtgtttacagcgcgctgccatttgccgaggtcattgccataataaaaatcacctttcaacaactgtccttctgcggtattgcttttatccgggttggcaatctgctgtcccagctgtgtgttggcttcatcgagccactgcaggatctgaacaaatactttcttctgttcatcatatgccggcgtcaggttatcttttccctgtagggcatctttcattggtaaatcccctaccaggttggtcatacgataaaagaaccaggcccggaaaaacttacccaatgcagaatatggattcacggcctgtccgcctaaacgggtggcttccacttccattttctgcacgttggtcatgctgtaataactgttgagatctgcaccgccccagtcgtaacgctgatcgccgtaatagttatagttacagcagtcgaactggttccagcgcatcacattgctccatggtttatctgtattcatatctgccagtacaccgcctaataccaggctgggaggcgtttgcgcaggcttgttggtgttgatagcatagtcatcgtacttcttgttacaactactgagtacagcacctgttaaagcaaggaaggttaatattttgaaagatttcatacaatacattgttttaaagtgacagatcagaagctgagattgatattaaagccatatctctttgtagtaggtgtttgcagggtagaagcgccctggtccgcacccggatactggtcgagatccacatctttattctttgcaaaatagagcaggttcctgcctacaaaagatatattagctgatctgataaaagtgcctctcagtatggtttgcggcagtgcgtaaccaatggttacctcacgcagttttgcaaatgttttactgatcaggttagcttcgtttgttctgtagtatacgctgatataatcctgcaggaatgttttggtagtgtttccttcatactgcagtttatcgtagttggtaacattaccgttgttgtcatactggataggtacgttgttgctcactaccacgccctggcccaggtaagattttacgcctttataatcctggtagcgggcctctcccattgcgccttctgtggtaaggatattacgtccgccacggaaagtttgctgctggatataatcgatcatgttgccacctacgcggccatcgaactggaagctgaggctgatgcctttataactgaaactgttgttgataccccaaacccagtcggcgctggcgttaccgagaaactgctgcgttggattcaccaccgggcggccatccgaaccgttaatgatttgtccgtcggctgctctcacgaaggtggtaccatagattttatctacccggtcgcccacgcctacaaaggcgttcagcttatcttccccgtcgtagatcttagtatacttttcctgaaaggtagaccagttggcggttacgttccagttaagaccattcgggtttctgagcggactgccattcagtgatacttcgtagcctgttttacgggtgtttacgccattgatacggttctttgcatagccggttgcacttggaataattacatcgtaaatctgcgggccattctcactggtgaaataggtaccgtctatgcctatacgatttttcaggaaacggatatccacgcctgtttccaccaccttgctggcaaatggtttcaggtcgggattagcgatcgtttgtgaaatataggcgcctgcctggttctggtaaaccggggccacattatagaaagaagtattgtagataggaccgtcataagacgactggtattcagaaccatatccgagcgggtaggtagccagcggtgtagcgccgatggtagcctgcgtaaagccgccttttacgttagcataggagccgcgcagcttcaggaaggaaaccacttccggcagctggatataatccgacaatacggtgctgactgcaacggatggataagagtatacgttgttttgtattggcaggttggaggctttatcgatacggtctgtgagggagatggtagcatatttccccaggtcgatatctatataaccatacgcgctcaataccagcataggtgcatagtagttggtggcaaacaatggatcgcggctgttggcaaatccgtaccatcccggcgcattgaggtaaccggtagacacgtagctggagttatacctgtaagaacgtgcattaccgcctacagaagcgtggatgcctattttatggggaaaggtattggtgtaagacaacagtacatcggtgttgttttcaaacatgctgcgtttgtcttcccggtaatcgccttttccttcttcacgaccataagggtgtgcggagaaaggcactttttcattcctcatcaggtcgtaggtagtgatttgtgtgcgggcgagcagttccagcttatcgctgaacttatagttcagttttgcatacccgtttacgtctgttttatagtggccgcgtaaccattcgtaggtcatgaaccaggggttatgataacgttgatattccgcgtaaatagattggataccttctttgcctggctgccagtagttgcgcatatcatccatgctccagtcggcgcccgcccatatcagggtgttatagatgatactgttggggccataggttacatccgggaaattgttggaatactggcggttatagttcatgtaggcatccagtcgtaaccgggggttgaagttataacctgcggagatattgaagttggtaatgttcaatgaggtgttgggaacaattcctttctgataggaatgcgacagggagaagcgcagatcggctttttctgtgtgggaagataccgcgatgttgttggtgctcagcatacctgtttgcaggaagcgttgcaggttgtttttaccgcgggcaatccatggtgtgccggtacgtttacctgttgccgggtctaccgggctatcgtactgagggatgagctgcccttcgaatttagggccccatacgtcgtagtcgccatcgttggttcccccacctttaccatctacaaaagcatatttaccatgatcgccgggaccgtattcatcctgtacttttgggatggcattgaatcctttttcgaacatggtactggagttaaaatcaatagaaaggccgcgcttatcttttgttccttttttggtggtgatcatgatggcgccattgaggccacgggagccatataatgcggaagcagttacccctttcagtacggtatagctttcaatatcatcgggagaaatattccaggtatcagaattaatgggtacgccatctactacatacaaacctatattattaccgcggagcaataccagcggggccgacagcagttcggcagaggcgcctacggtgagaccggctaccttaccagccaaaccatttaccgggttgggttccctggctttgatcaggtccgctccttttacttcctgtacagaataacctacccgttttacttcttttcgtatacccagggccgttaccaccacttcgtcgagggcctttttatccggctgaaggatgatcgttacatctgaagcgcctttcagtgcgtactgttcagggaggaagccaataaagctgacctggagtacatcggtgccggcggcggagatagtgaagctgccggcggcatcggtaacagcgccgcggttggcgccttttactttaacggtagctcctattaccggctggcggtcgtcgcctgcgataacttttcctgtaactgcctgctgggcatgtacagatagggtgatgaacagcagcaataacatggcgcatagctgccttttgagcgcccgatgtagatttgattgcatgtaaatgtaggtttggataatttattttacatgcaaagctcaaaatcctatgtgaccggaatgttaacctatactaaatttaatgttaagtatttgtaatccttatttgtcgctgtcgaggaagaaatatacgaccaggatctgtgcattgtccgggcctatgttgcggggtttgtgtccgaggcggccgtcgaagaagagggagtcgccttcttccagcacatatttttcattatcgatgaggtattcaacggtgcctttgataatatatttatactcataggcatcggtttttactgtctgtgagcggtgggcgccttttttcagctccagcagcacgatatctaccgggaaattctttacatttttggtgagcacccttttataaacaaatcctttggcgggttctttttcaaactcctggtaggcggctttttgtttgatgatgacttttgcgctctgggtttgctgatcgatttcgttgaagaactcgttcatgtccagccggagggccttgataatattgataagtaccagcagggagggtactgttctgttattctctatctgggatatcagccctttactcacctcggccctgtcggccagctcctggatggtaattccttttgcctttctcttttctttgatcttattactgatctgaatgatgatatcctctgtcatactaaacgtaattaaaacaaatataagcagaaagcggccaggataaaaacgttcatcaatctccctatatttacacaaaatagcattcatgttcagcatcgaccaaattctggccattacctttacgttatttgcagtgattgatattgttggctctatcccggtactggtgtccctgaaggaaaagctcggacacatagatgccggcaaagccacgctggcatcgggtttcctgatgattttattcctgctggtaggggaacctttccttaaacttttgagcgtagacgtacactcctttgctgtagcgggttctatcgtaatatttgtaatcgggctggaaatgatcctggggctggagttttttaaaacagaccctgatgccaaagccggcagcgtggtacctattgcttttccgctgatcgccggatccggtaccctgaccacgattatgtcgctcaaggccaacttcgggcaatataatatcctggcaggcatctgcctcaacctggtaatcatatacctggtgctccgtagcctgaactatatagaacgcttgctgggcaaggccgggctgatggtactccgtaaatttttcggggtgatcctgctggctattgccgtaaaaatctttaaaagtaatatcaatctttaatgcaatttgggattctacattagaaaatgtagatttgcgcgagttttatggcctcgtagtacaatggatagtataagagtttccgaagctccagattcaagttcgattcttgacgaggctactacatcaacgcccaattgcagtataactggaattgggcgtttttcatttgatcccagcagccttttgaagtttgcaatatctgaatcatttattaacttcggacgacaccagtcacctgaaaattaaagtaccggatttaacgattaacccatccctgatttaatctatgaaaaaaacattatcatcgctgttattgctaacaggtaccgtatcggtaggtcacgcgcaaacctatattaacaatcagactacgctgcagccttcgtcaaatttctacatttccggaacagcgcaatctaacaccttgaaaacgacggcaggcacaagtgccacaggaacgtcccacttctacatgtacaccggcgacggtaatacgcctgctaatctcagatggacccagggctttattggggctgagggggcttccaatgcgggcgctgatttcagactattccggtattcaaacactggcgctttcctgggaaccggactagccatagaaagggcaaccggtaatgttattgttaataatcttactgctgccaacgggtctaaaatacagggtactggtaccaccgctaacgcatcctatctgcaatttatgcaaagcgacaataccaccagggatggattcgtaggtttggggagtacaactaataaggatgtttatcttgcaagtgacaatggcaatgttaatctggtaccaaaagccggtggcggtatactccaggtagccagtgcacaggtacagaatacaactggtaccttcctgatgtcgaatgctacttccaataatataagcttcaatgcagtgggcttagccgggccttcctttaccacgcggagtattggcagtaaagttattttgtggaattccccattgaatgctactacttccggctgggacatcgggatggaaaatagtcatatgtggtttggcatccctgcagctttaaacacccagggctttaaattttatggaggtactacgcagattggcagaattgacggcatgggagcaaccgactgggaaggacaaggcaggtttaaaggttggtataccgccaacggaaccggccctgctgcagaaatagggatgtctggcggacgggcatcattcattggctttgaccggacaccgggagccacaaaatatctacctgtgctgcttgttggaggtaccacagcaaataatcaaaaaacgctcattattaccgatgttggcgttggcatcggaacatataccccacagtcggagctttccgttaaaggcaccattaccgcccagcgggtaagagtaacccaggctggttgggcagattatgtattccatcaaagttatcagcttccttctttagcggaagtagaacgctatgtgcgctccaaccagcacctggaaggcattccttctgcagccgaagtagaaaaagaaggtatagatgtaggagagatgaataagaagttgctggccaaagtagaggaattaacgctgtacctgatagaacagaataagaagatcgcggcattggaagaatggaagcagcagcaggaaaaactccctgttcatccataattaccaggacatactattaatctgtaagctaccggcaacttccaggattgccggtagcttatttttatagcccttccataacggaaagttttatctctctatgcccggtgctgaaaatcgagacttgccactgcattcgtgaagcattgcatataataaaaaacatattcaacaaagcgatttttacagcaggaaagcgtttatttgtatgttaatgtttagctttgcaagcgattttcaggggctttttagaagtaaatgtatatcctgaatttcattaagccacgggaatccataaagtgctaattggtcgctgaatacccgttaaaatcattcatcctgataataattatccatgaataattataaaatacctgtttaccggccttctttaggagaactggaaaagaaaaatgtgctcgagtgtttggactctacctggatttcatccaaaggaaaattcatcaccgaatttgaaaaggggtttgctgactatttaggtatggatcatgcagcagctgtttgtaacggcaccgttgcgctgcacctggcattggtagcattgggtattggcagcggagatgaagtgatagtacctactttaacctacatcgcatctgtaaacgccatcgcctataccggcgccacacccgttttcgttgattcagtagcagaaacctggcagatcagcccggcagacgtgaagaaaaagatcaccagcaaaaccaaagcagtgattgcggttcatttgtacggacatccctgtgaaatggatacactggctgctatatgtaaagcgcatgacctttttctcatagaagactgcgcagaagccattggcagcaaatacaaaaacaagtacgccggcacctttggcgatatttctaccttcagtttcttcggtaataaaacaatcacgacaggcgaaggcggcatggtagtaacaaacgaccagaccctttacgaccgcatggtgcatttcaaaggccaggggctggctaagcaccgggagtactggcatgatgtgattggctataattaccgcatgacaaacatctgtgcggccatcggagtggcacagctatcaagggtggaagaaatcatcacccgaaaaagagaaattgcaaaagcataccaacatgcctttaacggcagcagtgttacttttcatgccgaagctgaaaatgcttttcattcctattggatgtgctccatcctggtaaaaaatgccgatgaacgggacgaattgcgggacgtccttaaaaaggccggcgttgaaacaagaccactcttttatcccgcccacaccatgccgatgtactccggtaaatatgaaagacatatcgtagccgaagacttaggctggagaggtatcaatcttccaagcttccctgaactgacttctgaagagatcacctacatctctaatctcattcttgactattataaaaacagggaaaccgtttgaggttatgcagaaaaggaaaataggcatacatgctgcaggctttatcggatggggaggtggaattgattttctcaggatgatcattcgaagtattcttgatacaaagaaatatgaggtagtcatattactacctgatcatttaagcttcagggatagggtaagaagaagtttgtcacgtttcagcttaaccgcaaataaaaaaaataatgcccccaggcaattcagcgatcaccggaatttatttaaggagtttagccaggaagcgaaaagtgttacctataagaaaagtttaaagaaagccgtaaagcaacaccgtattgacctgctcattccctgcatagaggctgtaaacccggatattgatattccctgggtgggctacatctacgatttccagcatgaatatcttacacagtttttcacccctgaagaaattaaacaccggcaagtacaatttggcaacactgtacacaccgccaaaaatgtaattgtaaactcatacgcagtaaaaaaagatattgaaaagttttatccggacagtactgccaaagtcaccaatcttccttttacgcctttattcaacaggcaattacttagcagtaattttacggagataaaacaccggtataccttacctgataagtatttcatcatctccaaccagttctggatacacaaatcacatatcacggctttccgtgccctgcacattttacattccatatcgaatgaacggattgctatcgtctgcacaggtgataccggtgattccaggcgcgctgattattttgactcgctgaaaaaagaaatccgggatttaggaattgaagacaacgtatttttcctggggtacatttcaaagcccgatcagatccagctgttattgcattcagtagcgctgatacagcccactcttttcgaaggtggacccggtggcggagctacctatgacgctattgccttttcaaagccagccatcatctctgatatagatattaataaagaaatcaatgatccgctggtaacttttttccaggtaaatgatcatgctgacctcgcagataaaatgaaaacggtgcttgaacaacataaaagcagccattggaaattagacgttaataaactggaagaagaaacagcacaaaggataagcatattgggagatgttctttcagcacttattgattcgatctgatgacctttattttatctatagaggaagatatcagtcctcctctatagataatggcgctattatccatttatttcactcagctccagccaacgcattcccttctcatccagtaattgaataatttcaccaatccggtgggtcaggggttccatcttatcaaagggcaattctccacttgacaaagaggcttcaattcttttcttttctgtttccagttgctccatctctttctccagcagctccagttcccgtttctccttaaaagacatcttgcggcctttgttctctacaacaggagtcactgttaccatgggttctggtaccgcttcttttttaggtacaatggtctttttcttgtcttcttccttctgccattcacggtactgagtatagttgccaggataatcgcggatttcgccatctccttcaaaaacaaacaagtgttccaccagtttatccataaaataccggtcgtggctcacaatgattacacaaccctgaaattcctgtaagaaactttccaggatgctaagggttggtaaatcgagatcattggtaggttcatccaataccaggaagtttggattgcggaataagatcgataacaggtgcaaccttcttttctcaccaccgctcagttttgagatgtaggtgtattgcttttccgccgggaacagaaatagctccaggaattgtgcggcgcttactttagtgccatctgctaatgggaagttctcggcaatattctttacgaactctatcacccgcatatcttcttttaccaccagacccgtttgtgaataattaccaaacacaatggtttccccgatattgatcttcccggaatcgggctgttctgtacccaacaacatattcagaaaggtagatttaccaaccccgtttttaccaacaatgcctacccgttctccttttttgaaggtataatccatccctttcaggatcttcagatctccaaaagatttatagactttctttagctccaggatttttccgcccaggcgggtcatcttcacatttagttccagttgctggtcagctactttggtgctggctttttcctttacctcataaaaagcatcctggcgggatttggatttggtggtacgggctttaggctgtttacgcatccattccagttccttacggtaaaggttacgggctttgtccacacttgatttttcgctttcttccctggcagccttcttttcgagataattttcataatctcctttgtagataaaaagctgttcctggtccagttccatgacttcgttacaaacgctatccaggaagtaccggtcgtgcgtaacaagcagcagcgttaccttttcctgatccaggtaattctccagccactcaatcatagatacgtccaggtggttggtgggctcatccatgataagcaatacgtgtttatgctcgaagccaatttcgatcaacaccttagccagtgctacccttttttgctggccgcctgaaagggagccgactggttgatccaggttatggatattaagttttcctaatatctgtttcactttggtatcgaaatgccaggcattcaactcgtccattttagcaatggagtcggtcaacttatccagatcaggctcgtgtccttcctctgtgagcagttcatactctttgatagcgtttagtaccgggttattatgattgaagatattttcgattacggttttggagagatcaaagtctgattgttgctccaacattacaacggttacgtctttatgaatccagactttcccactgtcgggcacatcctttccgcataaaatgcggagcaaggtggattttcctgttccgttaagcgccaccagcgctattttatctccttcttcgatatgaaaagaaatatccctgaataatggtttggttccaaaagatttggtaagcccttctactgtaacgtaatgcatggtgcgaagttataaattatcggcaacactggaagggaacagggattatgtatttgatattatgatttttttcgtatattcattacaggataatcagggtttcctgtacctgacatttttttcgacaaatagttatttcggcctttgtccattattatcctcccctctttgcgatgaaaaataaaaaaagcccttgcgctggtgcggaagggcttgtgtctgtatataatttcatcagaagtcgtaataaagttgtctgaagctactgcgtaggccaaattgaaatatcagctctttgttgtcgtacaggctatttttttctcttcgacctgttacagacagttccaaacgcaagttatattttggattgagcaaaaaggctactgagccctgaacatacgttaaattagttttcaagccctgaccaatatggtttccgtaatcttcgttacgtgtattataagacttaaaaatatctttcccataatttatacccgcagtatccaggccatattttgccaccattaattcgcctttaaagaaccatctacggtattgatagtctgcgatattaacccactcgatgaaattagcccccattgggtgtgccagtggttgattataatgtccgtagttgtttaacgtagaccgctgtgagtaagtatatggtcgtgctgcatttacttcggtcagaacattcagcctgggcaccttaaagatattgtttgaacggaaccctatttgtcctccaaatttatttgcccaccagccttttccactggtcatttcactgaatttaaattcatcaagcaaaaactgcccatatatggtagaattaaccgaaggtgcatattttacattcagccccatgagtgcattatccggagagcctactgagaattccaccgggcgcagaaaaacaataggattgagataactcatatcaaaccctctttttcctgttgaatcggagtcctgccaaataacagcctcgaaaaagccaatcgtaactttctttgatacattccagtcgaggtagttaaacaccccccactttttccgatagccattgtcgtatgaggccctcggatatttcatatcaataaactgtgcccacattgtggtatactgtactcttcctacattagctattaccttaaggaagggatagttaaacgaattatcagaaaggagcatggacctgtatccatcgcctatgaaatttttgtcatatcccaattggaaatcgagaaatttccccgccttataactgagtaaggcagatgaatacgcaaagtcaaaagctttcccattgctatagtctttccattgcccctgtcccggaacaatcatcgtttgacgaccgtagcgatcaatgtactctggaaacttgccctggttctcgtaaaactctgtacgaaatgtaaagtttttccccaaacgtcctccggcaatcacacctcgtgtattcaaccacgtagtgccattatcagaactattcccaataagcagatcaggtaaaaaactggcataaaaatcatagtctgccgtactatactggagcaggtgttcgttgaagagcttacggtgaaaccagcttctcttcttggtggaatcttcctgggggagttgaaactctggttgtatcatgtagtcccgttgggaagaatgatagctgaaactattggtatcagcggtggctttataaaagcctaaggaaaactgtctgccggcactctgcgcaaatgatccaaaactaatagcgagacaacttaaaatgaaaagggctttaacaatctttgtatgtaacatgtattaatgtgtgcttgcaagacgcaaatatatgcttttaagcacattagtatcactactataaatgagaattaagttagcagccacctttctgaaaagcaaagacagccggaagcgctaatggacccggctgtctttgttcataaatccgatactggaaaactaccttgaaaacatgttttggtcttttagtaacccatttatggcattggtagtgatttgcggtatccgtggcagtgtaaaggaatacatggtacaccagtcggtggtcggtatattgataaccgttccggatgcgggcgtttttttaaacacaatagccgtaggcaccgtttttattgttctgaaagcaaaatcatatcccaataattctactttttcaaatttgagcagtttagtattaagaatcggtgtgccatccgcctcgaaaccagtcaaaggggcgccatcatactctctgctgggacatctgataatatccccctttttaagacccaaaccggcaaaaagaggggaattgggactggttaccttaaatccttcccaaccatcattcttagcaatagtgccatagccacctccgtcaaaatcgcatccaatacttgcgataataggatattttaattttgattctttccagtaaattgtcttcagactatcggcaatagggggttcacccaatcctttataacaaacaagctgatgttgcaggctgtccactctaacctgccaccacattacattaccggaaagtaccaacgcatgcttcccttcggctacaaacctgtcaaagttccgtctggctggccttgaccagtattcactgtgcccaataatgatcaggattttgccttttatgttatcgaagttttccagatcctggtcgcagataaccgtgtatttatagttttgcgttaacatccatttaaggaagccggggccaccatattcggaaaaacggataggtcgaagaaaggaaactttctttgctacaggaagcgtgtaaagacttctcctgccggattccgagtaggcgttctcggtgttggatgggtatactactgtaaagtccgcagcatcttttgatttaattacaaagggaattttcttaccaaccaggtagacgcccgtcttcgcgttggctggaatcctgaagcgaatgggatgttcatattggaaaccatcctctgatgggagttctcccttaggactttggtgatatgactgctcaacttttacaacaaaactcacgtcaccagccatgtcatatacgttaactgatttctttttatgtacactatctgtggatataaagagcgcagcgctatctcctgggaaataagacatcttatcgggataaccatttagtatagcaccgtcactaataactgaatccgcgccgggttgtattggtggcgctactgattcgttgttggaagactttttacaggaataaataacagcagtaacagtaagtagagccagcacggctacctgcttaattttcagatgatacatgaagcaacaattgcttgggttaggaaatttgattactaatagctaaacttaaaatcagacatcaaaggatatcaattatacagatttacttttctgaatacagcctgttcactatccaggggaggcaacgcgactggtaacttatgggctgcagtggtatctgttaatttcttcagaaaagagattatactttgtttttcttcctctgtaagatttaacttttccggagggagcgtctgatttactaacgcaataccctgtccaatccctccaccatcattataaaaatccagtacttctttcaaagtataatagattccgttatgcatgtatggtgcagtaagcgcaatatttctaagtgttggtgtacggaaggcatataggtatggggccgccgggtaaaggttgtagcgtccccggtcttcgtcaacctctcttgatcccggaaaccggggaacacctatgacttccacctctgccttggcaaaatcaggaggaagcgagccattaaataaaggtgcaaaatggcatgtgccacatttagctttccccataaagagattaaaaccatgtatttcctcagggtttaactgcgaatgatcaccgcgcatatacttgtcaaatggcgaattaaagctggtcagggatctaatataagtggcaattacattttgcagatgatatggcgtaagtgcctctgccgaccggggaaaagctttcttaaaaagtgcggtatatgccttacttccacgtattacatccattgtttttgcaatagaaccgtgcatttcgttggggttggacaacacgtcggagatctggtcctccaggtaagttacccgtgcatcatagaatagtgccggttgtatacctgcattcaacaaggtaatggtgtttctgtttatgaaaacctggccactgatagccgggctttttgcaaagccatctgtaaatgctttccccggctgatggcaggtggcgcatgaacgtttgccatttccggaaagagccgggtcaaaaaacagatagcgcccaagcgcctctttttcttcaccgggatattcttcttcatcactgatataaaaatcaaaagagaaagcattcttatcaaagagactccctgctgaggtactcacaagttcttttgaaccgcttatcactatccctgcctgctttaacaaacctacaagcattgtccccagagggtttgcatacgtcgtaaaaaaatgcagccgatcgaatgaatcaaaatcctggttatgctgtaaataagcaatgccactgtctacaagattattcatcttcttacacgccgcaggatcagatttacctaactcgtcgttgtaaatagcaataatatcatggaatgacgaccaaaccgaagcaacttcctgtatagcatttccgctcaacggagtgtcatatccagcaagtccaagtacagaagaccggaataattcctttctaagtgccttaaaaactatagtgtctgtgagttgctttttttcagaaatataaatagcttgtcgtaagcttataataagttcttttgtcagccccgacaattcagtgctatccttactgttatattcagggtacaataatgcttctatcacctgaaaaccctcagggggctgaatggtattggcattatcttcttcttccacttcaggaactggagcgccattaattactttggccaattcaggatttatgtacgctgttagaaactccacctttttatagtgcagcctggcttgtctgaatagttcccggatctgaggaagggaagccttatttctgactgctctatccaattcctttacttttgcatctgtacccttaaggtgttcgaggtaataatattgtacctcttcagtttttacaatggtgccggtaccgcagttacacgcctgcaaaaaagaaaacagcaacaggcagcttacttttagggataaattcataaatattggattcctgaaataacaatacaaccctcaggataaaggatatattaaaccagaccccgcttttttcacggcatagcgtctcagctaaaatttaaaacgccctgggaaaggaaaagttacaggtataggtagcatattttagcgggaaggaagatggtggtcataaactgttgtcaaaatttaacagggaatactttttaagcaaaaaaaaatcccgttaaagccgccggtcaagaccagccgttttctaataattgtctgtaaacattctttatacctgtttccagctctatatttgccttccagccataagaatgaagtttacttacatccatcaatttacgtggagtgccgtcaggtttggtatggtcaaatttcagttgaccttcgtagccaacaatcccgcaaatcagctttgccagatctacaatactgatatcttctccaacaccaatattaaccaatcctttttcatcatagttctccataaggtagaaacaagcatccgccatatcatccgcgtgaagaaactcccgtctcggtgttccggttccccatataactacttccggtacgctcttaacgtgtgcttcatgaatttttcgaagcagcgcaggtaaaacatgtgaattattcaaatcgtaattatcattggggccgtataggttggtcggcattaccgagataaaattgcatccatattgcgccctgtatgcgtcacacatctcaatgcctgcaatcttggctatggcataaggctcgttggttggttccaacggaccggttagcaaatattcttcctttaatggctgcggtgccatttttgggtaaatacaggaagatcccaggaacatcagcttctttacccctgccttaaaagaatgatggatcacgttgttctggatcatcagattttcataaataaaatctccccggtaggtgttattagctacgataccaccgacctttgctgctgcaagaaatacgtattcgggcttctcgttttcaaaaaatgtggctacagcctgctgattacgaagatccaattcagaagacgttcgtgtaataaaatggtgaaatccggcagctgccaatcttctcatgattgctgagcctaccataccacgatgtcctgcaacatatattttactatccttttgcatcttcttactcaaactggtttaatactttataacccgaatcttttaataatttctcacgtttgaacagctcaacatccgcttccaccatttcttttaccagtgcagccaggttatatttgggctcccaattaagctgtcttttcgcttttgccggatctcctattaacagctccacttctgtgggtctgaaatagcgctcgtcaatagcaataacttcctggccaggtttaagcagtgaaccggatgagttaacatgtttcactattcccttctcatcaacacctgcacctttaaattccacttctatccctacttctaaaaaggccattttaataaaatcacgcactgtattagtaactcctgtagctatcacaaaatcttccggtctgtcttgctgaaggattaagtacatcgcttccacataatccttagcgtgtccccaatctcttttagcatccagatttcccatatacaacttctcctgcataccgagagatattttggcaacgcctctggttattttcctggtcacaaaagtttcccctctcaaagggctttcatgattaaacaatataccgttacaggcaaacatatcataagcctcgcggtaattgacagtaatccaatatgcatacattttagctacggcgtagggagaacggggatagaagggtgttctctcagattgcggtacttcctgaaccagcccgtataattctgaggtggatgcctggtatacccttgtctttttagtaaggccgagcaaacgaacagcctcaagtacccgcagtgtaccaatcccatctgcatctgccgtatattcgggtgattcaaaactaacctgtacatggctcatggcgccgaggttgtaaatttcatcaggttgtacctcctggatgatacggataagattggtggaatcggtaagatccccataatgcagtttaagcctgacccctctgtcatgtgggtcctgatagatatggtcgatcctgtctgtattaaaaagggaactccttcttttaataccatgaacctcatatcccttgtccaaaagtaactgtgccaggtaggctccatcctggccagtaattccagttataatagcttttttcattattgatattaattctccgcaaaaatactcacaagatatggttattgttattgaataaccttcatatttttacttttattaatttgtgagcttggtttacttttggtctcctctttcatggccctgatgagtgaagttttgtcatcgtcggtgtcaccatttatctcccatatcataatcccacccacatttctcatggcaagatcaactttcttcttgatggtgtttatgccattataatagactccattaaaagaatctgcgttgggatcagcacctttacttatcaggtctttgtaatacggcggcactaccttagggttacggccgtaagtaggtaaacctagattcgccttctcccggggaagcttgcggtcaataatccaatagttcaggcaatttacagcgaaatcatagcttgagtgcgaagcttgttccatatcatcgtaagccataatattaaaatagtctaccaccggatatagttcatctggcgctaaagcgccccacttaggcttacctgatacagccatggttaataatttccctttctggtgaagcctcacagaaaactttttagctaactgtaccaacttctgaggctcatctgaattaaattttggatattcccagtctaaatcgataccatccagttgatatttgtccacgatagccattacattatcaacaaacttatccatcagcgcgtcactttcggcaatctttgagaatgtcttatctgtgtattgtccgccaagcgccgcaattactttcacttttttaggccttgcattggctacaatatcatatagcttgtcataggtcttatcattggcaattgtaccatctggcattggctttaggaaagcaaaatttacgcaggtaatgttatcatacttaatttttgttaccggtccccaatttgagaaatacccaatgattctaaacggggcagtagccgcagacttagtagtttgggttattttctttttcttttttgttctttggcctgaaacaggaatggcgactatcgcactcatcaaaagcaggagcagctgaaaagatctaattttcatatgattcatttttctaacttttacgccgggaaaaagtttttctatttcccgctattacatcagcaaaaacttcttcatgaagcttaataacacgtttccaattataatagttgttaatcttgctattattacccgacagaaaaccatctttattttttgcagcgagcatatctacttctgaaatacatactgcaagctcacggctattagtaaaataaagcgcgtttgcgcccaatacccctctgttaaagttattaccatgcgcaaaaataaaagcatttgaagccattgcttctaataatgaaggattggttcctcccacggtatgcccatgcagataggccttacaataacacctgagcgaatccagcttttgtttatcatatacccctccgagaaatcttatattcttatttttatatttttctttcagataatttccatatttgttctgatggtttccgataacaataaatggagaagaatgccctgattcaaggtatccatccaatatcatagcaatactgttttcaggctcgagcctggcaaccagaaggaagtattcattagctttgagatcatactctgtcaacagtttctcctcaaaatcataaactgcatctgcaccgtatggcaaataaatcgtatccgtattatgaaactccttataatattgctgaattcccagattatcggaaatcaggtaatgagatttttttatagccaacgtctcaaaataccgcatcagccggcgggtaataaaattccatttagaacgcttccattccagtccatccatattggttaacaccggaattttactgttcttcagtagaaagtaagatggagatgccgtaccatatcctgcctcataaatgagatcaaagtcttttgtcagcgcatgcttaagggatctgtaatcataaataaagttcccaacagctccgatactctgctcggggcttttcactttctcaatctttacccctttaaaagtatcttcctgataaccatgaaaatgcggattatatacagttacatcgtgtcctaactcaacaaggcccacagaaatatactcggcaaactgttcaaatcctccgtaattattgggaatcccccttgtgcctaatatggctattttcatcttactctactatttatcatttcttaattttaaaatcattaatcgcggctaataaatacaccactggcagtgcactcacaatattgttaatccctaccttaaagacagggtaatgcgacaacgtaaaaatgaaataaacaaaaatgattaaacccagaaaatattttttattcctattaaaaagcaacacaattaaaggtgacaaatataaaagaagtcccgccaatccgatgaagtacatagtagtgatcagatatacttctgaatagattttttcaacaagtcccgggtttccccccagaaaaaaaaccagcgtatagtcattaaacaaacggatagggttgtgataaatatgctccaccaaaatatccatatcatgcgtgaagatcattacaaccatatttactatcatttcattaaaaaacaacatgaccgcaatactgagcacaatcaatgccagaaaaaaattaatagcggctttaacattggttctcatcaatataataagccacatcagcagcatgataagataggcagtttttactcccgacagtaagatagacacaacgatcagggcaatcttccatcccttcattttaacggggaatttctctatctgcaggataataagtgtggcaagagggatataaaactggctgtgcgtatccagaaaataccctgcatgcctcaaaaaaccattagttccttccatatccaggtaatcagcgagattctggttcagtatttccaggtatgattttacagccgcataattacccaatatcgtattgaagaaaaagtgaataatatttactgctgctataaaaagtcctgcactgataatccacctgagcaaaacttccattctaccggttctgtaaaacgtgaaatagcaggcataaccgagataccagtaaaaataaaaattagaaattgttctcaggccttccagtgcaccatcggcaactcctaaagctgcaatatgaccgagcactgtaaccgcctgcaataacaaaaagccaatgaagtgagtataaattgcgggactcgccgctcttgaaatgcaaataaatgtaaatacaagaacggataccgaaataagaaaatatgccccgaacgggtttaaaaatttgcccagataaataaatactaaaagacagatgaccggcagtaataattgaaaagtcaataaagagagcaggatcttttcccggagcttttgcttcgaccacactattccgccagagagctccttattgatctgtattgtattcatttaccgattactttttttacccgcaactttgcaagatccttaactgctctaaaaaacaccctcatcaatatccagttggtatacttgaaatcaactaccagtctggatacgacataattggctttcagaattgaaataaattcatttttatgtatcagcgagttggctgttaccctgtatttgactaatggctccgtaatgatcctgactttatatcctttaaaaaacaaagttagccagagataataatcttctacactgataagccttttctcttcttcaaatacaacatccggcgtttttcgtaccattaccgatgaggtacagattttattatgcagcaacatctcctcaagtgtaggtaatgccggcaactttggagaccaggtttttacacgatctccgaaaaagaaaatgttagtagacaccaggtccacattctctgtagtaattacctgatactggcgttccagtttatcgctaagccaaatgtcgtctgcatctaaaaaagccagataactgccggctgacgctctgattcccatgttacgcggtccggcggggcctccaaagttctgtgcaggtttaaagtacttaatcctgttatccttttccacgtatgccctgataattgatgcgctattatcagtagaacaatcatccactaataacaattcccagttagtatatgtttgttgcaatactgaatcaatagtatcagcaatatatgcctccgcgttataaacaggtacgatgactgaaattagatgctgcatacttttaacttacttgttactggcgttttattctagccactaatttagccggattaaggctaattgccaggaaaagataccacatccgtttcaaaagatttttctgaaagagaaacctgcgataaaatttcagatgataatatgtaagctttgatctcaacggcccatagctggtgtgaaacaattcattacaaatagcataaggttcgcggattgctttgtatttaaggtcgttagaaacgcttcctgcgtgtatgcgaacaaatgtaagtggcgctgtcaggttttgcataacagcaccatccgcaatcatcctggcaaagatagcataatcctcggcagggacatattcctgttgataaccatatttttggaaaagcgccgttttacccattacggttccatgcaatactccatgcatagcagtatggtagcgtttttttatttcttcgtaagtagctggaaagttggttttgaaaataattttacctgtatcactatcaaaataagcagcattgctacccaccacatccagttcccggttacgctccaacaactcatattgtaacctgatgcgatcttcgtgtacgaaatcatccggatcaagccttaagatataatcaccagaggctatttttaatcctgcattaagtgcattggcaaaaccctggtttttgttcaggaataccggttttagtatcttagtttcttctgcaatttctgtcaggatccttacagaatcatctttagatccatcgtcaactactatgatctccctcggtagcaacgaggagttcatcaatgagtcaataaactgacggagatattttccattattgtaattagccgatactactgatatattcgcctgctgacggttcataaaaatatttggattaaccaattataaaaggccggaaagccctgtgcccctggcacaaactgctgatatccaatcgataatggcaaaaggccttgaaaaccgttctgtacctcagcttttcttagctgcatcttccagcgattttattactttggcaggaattcccccggcaaccactctatcgggtacagatctggttacaactgatccggccccaatcacgctgttttccccgacagttaccccgggaagaataattgcattagctcctatccaacatccttttttcagcactacaggcctggacggataatgtccctggtaataaattggtatttcaggattgtcaaaattatgatttgttacataaatatgaacaccactccctatcagcacatcatcttcaatagtgatactaacgtcaagattggcagacgccccatgtaagtgtgaacatggccggataaccacccgcttccctatcgatatctgtgaacaacccacagcatatgctccggcccggaactgggcggttttatcaaaatgataaaactttttctggcaaagtttcaacatggtcgactgaaaatgtagcttccaatgtgtagaaggtatgtcaggccctatcctgtcggctagcctccaaaatttcagtttatcgctcaattctttgatgaacatgataaatatctaagcgtgcttgttttgatgattttaaagcttgacgtccttcccataccttgtgcaactagtccggcaactatactgagaattccggattccgttccttaaaaggaaacaagtcagggtgaaattgtttacaattaataaaacgctctcagcagagacaaaataccttgctagcgcaagtttacagcaaaaaacagggataaacaagaagagatcattttttttcaatatctttaaatcttatgaaaacgatatctctgtatattatatcgttgaggttcccgtcgaaaggatgagcaacgtctgccaaagataattagatgcccggaaatcgagatgtgctgacaaatataggccattgcatttatacaactattttaataagcatatagtacataaaaccggtttaaagccaatttatgtttcattatttcagcatataatatttgtttacgactatgataaagaaaatctatcgaaaaattatcaaccgtcttgattcttcaccgaagtttccagcagattttgaagctgagcaccaacgtatctgcgccaaggttgccccatttacaatgaccagccaggaaagggtttttagccttattgaagcagtaaagtatatacataaatataaaattcagggggatattgtggagtgtggtgtctggaaaggtggcagtatgttggctattgctgagacactgaaggccgtaaatgataccgacagggaattgtttctgtacgatacgtttgaaggaatgtctgccccctcagccgaagacgaaacctttaatggagaagatgcctctgaccttttgcaacaggatcaggcgaaaaaaggacttatatgggcttactctgcattggacaccgtaaagcaaactatgggcctgagccaatacaaccctgaaaaaataaactatatagccggaaaggtagaagacactattcctgccaggatgcctcaaaaaattgccttactccggttggatacagattggtatgaatcaaccaagcatgaattaattcaccttttccctcttcttcaaagagggggaattcttattattgacgactacggcttttggaagggcgccagaaaagctgtagacgagtatttcgatgaatatcaatttcctgttttcctgagtcgtattgatgataccggaagaatcgccattaagcaataataacttcgctatattatgtctgctgataaagtaccgtataattttaatccggatatccgttaccctatttatcttgtccgtaatggcatcctaaaggctgtaaagaaatactgcccgcaattgaaaggcaccttaatggattttggttgcggatccaaaccatatcgaagcttattcgatgtaaaagaatatgttggtgttgacctgtacaaccccgcacacttgcatgatgacgagccggtagacgtattctatgacgggaaaaccattccttttcctgatgagcattttgatgcagtgttcagtagtgaggtttttgaacatgttttcaacctggatgatatacttaaagagattaaccgggtgatgaaaaaaggtggaaaaatgctgatcacctgtccttttgccttccccgaacacgaagagccttatgactatgcccgttacactgttttcgcactaaaggagctgctgggtaaacatggttttaatgtgttatctattgagaaaaccggtgacagtattcaggccatcatgcaacttcagattatccatatggtttcctacaaatccaggataagaatcatcaatggtatctactggagggtggtggttatctggatgaatctttctgccctgctgctcagtaagatcctgcctaagcggaaaaccctatatctgaacaacattgttttatgcgaaaaaaacggctaaccgccggtaaagtttaaattgatcgaaaaacttccagataacgtttcattatcagacgattgctgaatttttcgaaatatcgctcccgactgctacgccccatggttgctattttttctttgtccaacatcttttgaatagcatttaccaattcgtccggagcatcgggagcaacaacatagccagtcaccccgttatcaatttgctccgggataccggctacccttgagccaactactggtttacccatcatcattgcttctatgatgacatatgggaagtcctcattggcaattgaaggcgttatgaatatatccatatccctcacatactccattacatttggcctgaagcccggcaaaataacgacatcatccagattataatcctttatgagcttctcgagtgctgacctttcctctccttcaccaaatattaccagcttatacctggccaatggttgtttttgtcttaacatggccactgctgtaattaagacgtgatagccttttctacgggtcaacagccccacggcccccattacgatactatcatcatcaacaccaaactcacgccttaaaatccctgatccggctatactcgtttcttctgtctgggttaataaagtattgggaatattgaagcacttttgctgatcaaaattcctggcctcagccagccggtcactcgcagcttttgaagccgttataaagtaactgacatacttgttaatatatctgtccttccatttatcccaaatattcttttgcggatatgccatattattgactacaaaaagcacacttctgatccctgccatcctggcggcaattgcagctatcctgcatgtttcagctgcgggataccccccattattgatcaataatatatcaggccgttcccttttgaaaagcctgaataacactaggccgttatacaactgaagaagccctatcttattaaaaaccagtcctaatgtatataacaccctcgtataaacgcgctttgcctttccttttatttctccggattgcaatggatgtccccattgcggatacggattgataagtttttttactgactttacattttcggctccgccaaactttcttttgatccccttctcgtattccttattataggcataatagaaattcaacaagaactcctcctggatttcttctgagcgcaaaatgttttcaatgacattttcacttccactataaacaaaacaatcactgtaaatcagaacttttctcattggaatacttcttctgtgttaaatagtcaggtgaacagattagttattttcctttctgttcttactcaaaaatctgttgataaactgaagatttctgtcaaggttttttccatcaagcttaccaatatatttctcaagaactgatttcttaagaaaaacatcataaatcgggtcttttttatagaacgcaatgatcttctctttaagggacgttttatcaaacgccgttacaagttctgatttaccatcaaatggtttgttgatgatatgctggtctttcttatagtacaatgctggtattccgagaatagatgcctcaaacaatgtttgtgaataaaaagaaagataaaagtcagcttctgctattacctctttaaatggtttttgctgttcaatccgcactttcatatgtgggaagtactcatccaaaaaacgactatactgtgaagcatagccattctccctgactttcaacacaatactatgtttgtagccctccccttcaagatccgataaaacttccagtaaatcatataggaagtcaaattcgtaggctaaataggagttcatatcaataagattataacctcccgcaccaataataataacaggattctccctgtcaataaccttaggctgctgattgctataatggtccattctcgggtcgccaagacagattgcattatccattcctccaaagtaatcttccttaatcgcctcactataactatttacccaatcgactcttctcgcatcataggaaaagttattcaccaacaagccattgatgatcatataaaccgggatacctttcaacttacaataattgataatcaggttattctcaagccacagctctgttacaggtaccattagccgcacatcttgcggaccaaaataattctcaatatcctcaatccgcgaaaaagcactttgcagaagtttgggcaatttgggaacaatcaattccagcaaattggcgcctatatcaaagccatcaattttccagtcgtaaaatgacctgtttttgaaagcggtcaggctggattctattatatcagcgggtattgttctgttacggtaaaataccctccgttcttttaacgcgttaaccgggctcgaataatttgccatgatgactttgacatcacgattcttttttaattcatcaatgataggaaaagttggataataattttgcaggtaaatggcgggagcgtcgtttctcattaaggtttctcttaccctgcctatatactcgaataggcctaccccccaacgctttattttttttacaaatgtgtccgttttcattttctcctccatccaggcagatatcgggaaataataagcgggcacttcgctgccatccacttcttctataaatcttgccgcggggaaaagtatcttcacccactttttgattacttcatccgttaccgcacaaatgatttccctgcatgatacaaccttgactgcactcaaataaataaagaagtgaaagttataggtcacatcattaagtatgtttaaaagataagcgcttccaaccggcactcctttataaacaataatgtcatttccatctttgtcgagataccacttattcagaaaatgatgcaattcatagtttctctcttcaaggtaatttctgtcaagtatattatctaaataaaaaacttctattttttccttttccagcattttcatcaagcccagatctattaccaacacgagatctgtttcttcattaaacaatggtttacaagaattccagtggttcctgtcttccacaataaagaccctgttaaaatccctttcaggaataccaacaaatgcacgttccatttagtcctatttaaaaaaaagttttggttttagctggcttatcatttctaatacatactttctgaaaatacgggaacagatgtaatataaaaataatcccatcagacaaatagtaccaatgataagtaaataccagaacaggtttaacctgttatgtcctatcggtatgtacgatttaacaaatatacatgatattattaccgccagagctggtaaaactgccggtaataatacggttcttattgtatccttcacattgaattgtaataatttacaactcataaaaaaatacgccagcgccgacaaaacaaacgacaacaacttgaatatcgcaaaggaagtaagtccccagaatgaataggtaacggcgataccaacccagaaaataactggcaacatagcacttgtaacatatatcatcttcaccttttcatacgccataatgaggatacccgccggagacgagataaaacttaaactataacaaagtatcagcaattgtgtgataaatacagaggaagcatagccatgtcctacccagttaataactaacgcctcagaagtgatggaaaggcaaataacgggaaaaagcgttaatggtagggttattaccaggacattcacaaaaacccgcttcagcccctcaatatcgttggctccgagatagtgattaaatcttgctgtaaatggcgaaaacaagatcccatacaacgacctgatataggtcagcatagtaagaccaattgcatacaccgccaccgcatccgcgcctatcattttcccaattacaaaaggatcaagctgataataaagtatccagcagactgtgagaaaaacagagctaaaggctagcttctttgttttatcaaataactccctggaatatttaaacgagcgaagtaaaaaaaacagatcataattcagtcgctttttcacctgccacaatccggctatcattgctaccgcattacatatttgggtaaatagaaaataccccaccagcgaatattctcctcttccaaagaaataaaaagtagacaatattttgcacaaattggatactatcagcaggcgctgaaaatgataatcctccattcttaccgaaaaaatgacctgcaacatacgctgcaggataaaggttggagaaaacaaagccaataaaaccagtaaggtactggcagtttttgtttcatcaggtttcagaccattaacaattaaatcaggacgaaaagaaatgcccagcataataaccaggaataatcccacaaatacggtgaagataaatgcaacaaatcccacaatctttatttctcctttcctgtcgtttctggcgtatgattcacttgcatattttaacccggcggaaatgaagccaaaatccgcgtaagacaggaaaatgttcaatgaaactataatggtatagataccaaataacgatttatttgaagacaaaaaaggtgttactacgaataaagttccgaaattcagcaggatagaaataaactgccacaaatatattttgatgtacttacccaacattacgcggatcgtttgaattacgtttttagtattaggtcattaaatgacagtccacccgccatcaacaaccagattatgccccgtgatatatacggcatcatcacttagcaaaaatccaacagaaggcgaaatatctgcaggtgtgccaagtcttcttagaggaactttatgttcatattgttcaatgaatttctctggctgatgattaaatatgccgcccggggaaatacagtttaccctaacattatgaggaccataaaaggctgcaagatatctggtaaaattaatgactccaccttttatagctgcatatgcagaagggtttattattggtgttccttcatatatggtaaaatccggtccggtaataccataaatagatgcaacatttaccagggagccctttttttgcttcatcatctgattcagtacaatctggcagcattttacgtagcctactaaatgccagttaacattcttctcaaacgattccattgattcctcgttaaaaggaagtctaccccaatcgtcggttcttggataagcattattcacccatccatcaatagcgccaaacctgtccagaattatctgcaaagcctgtttgatggaatgctcatctgtcacgtcagcgcacaggttaaagtcatcttcagtggtaattaccttatcaatagcaattacctttgcaccatggccacgcagatatgtaacaaaattgctgcccaattgcccgtttcctcctgtaacagcaatcaccttatcttttaacttgctcatcattcaaacaaatttttaaaacattaaaagcagattggatatcattcattatataaccgttatcctcttttatagctgaaatgaaatacttcatctgttctttatatgtatatagtggatctatgtctgatgaaaatatcaattcctcattacaccagaccttttgctttatcaaatctatagaaacagtattgtcttcaaataatatttcacaggtcctttttgtatctcttctataataattcagtacaatattaacggtgaattgctcatactgaaggagataattagcgtaatcaacggcatcgatattcaatgaagaagtgcttctaagggtagcggctgatgaattaggtgttccccaaagccaggtcacatagtcgagttcatggatcaggtcaagatgtactccgcctcccattttttcatttgcgctgtaaacctgtctgtaatcaattcccggcctccagtctggtaaatacgaaccagcatagatgttcacttcgtttatccgttgactcttttggcggagcagatctttaataaatacaatacatggatggaatcgcagattgcaggctatataagtttttactttactactaatgatctggtcaaccaactgctgcccaccgtcaagtgtatgaaaaagtggtttttcaataaaaagcggaatgttgtaatccagtaatttgcggagcgtatcgtaatgagaaaaagtagggttggaaactataacaaaatcgaaagagactcccgcctccccgatagaagaaatattggtaatgttaggaacttgattgggtaacgcgctactacgaagggcatataacgaaatttcaccgctactgatgtttgttaatgcctgaatatgcttttgagcaattgatccgaggccaatgatcagtactttcataatatgaaatccagtttattattgaccaacaagtattccataaagtcaaagtcaacctcatcatcaagatcaaagcacatatgaggaatttcatatacaagcgatctattcgtaacagccgtatgaaacccgccatcaaaaaatcttctcttatagatatagaatgaagcgttcatgtcgtaaaccttgggtgctgactgcctcgttacaaattctcccttttttgccagttcaaaatacccgtttttattcgcttctaccatgttgaaatacggattccgtttagctggactaacagaaaaaatattcactgcttcctcatcagccgtcagcatccgcagcgctatgtcgagatcgttggctgttctgaaaggagaagttatatcaagatcaatcagatagtcaaatgttactccccttttcttctcctcaaaatgcatcaaatcgataatcaccggcattttaccaatagtatctgttgcaagttcagcgctccttttataatcggtagccagtccgaaacccgccgcggtgctaataatctcctccgagtccgtagaaagagctattacacagttctttgttgatgcaaaattcttcgccatctcaatggtataaccgatcaagggtttacctgccatggaacgtatattctttcctggtattcctttggaccctcccctggcacatatggtaattaatatactcattttagaatttgatatgtttaatgtcattctgggccttctcaaaatcctcatgtcttcctatatccaaccaatagccaagaattggataatgaaccactttccgtttttttgaaatcagcatttccataaaatcggtagcattatagaaagaacctactggcaggaactcaagcaggcttcttttaaatagatagattcccccattcgagtaatagctgtaggtaggcttttcatcaaatgaaattacctggccattatctatttctaatacggcataaggaactttcacctggtatggaatgctcgccaccattaaatctgcgtcggcatcaataaacgatttgtaaaaatcagcaaaatcaatgttggtcagaatgtcagagttcattaataaaatattctctgtattgaacgactcgaccaggcttagcgccccaaaggtgcctaaaggaacatcttcctcaacatattgaatattcacatctttggaagagccatcattgaaatactcttttatctgatcacccagatacctgatacttatgatgatacggtttattccgtaactggctaatctgtctatattgtgttcaataataggtttattcccaactttcaacaacggcttgggacatttgtctgtcagcgggatcaaacgttctcctcttccccctgccatcaatacagtatccagcggcaacaacgatgacttaatacgcaggttcagaatgtcaataatcctacggctgttatctattatcgggattatttttaaattcttttttgcgaatatttccagttgatcaatagaatagttatccttataaatgaatataggatctggttggatatactccattatgggagtatcaaatgtaaggcccttgataaatcctctcctgatgtcaccatcagtaagtgatccgatcagtctattgctatcatctacgacaaacagtacagcatcaatcgccaataaattcagtttattaagcgcatctttaatactggcattccctgatataagatgtttagtaaattccattagaccttatcaataaatttgatcaattgaaaagcttccgcgtatcttacacccacactcgcaccccggaaatgcgctagtgctctgatattttccagacttctgggaaacggatgttctcctaattctgattcatatatttccattatggagagtttatcttctataaatgcagaaatatccacataataattaggcataaatactttctctggcaaggcaggtgcaaactctgtttccgagagacactcatacattagcactcttttgattccgggataccggaatgatttagtacatgccacaaccgcgtcaaaaacaaccctgtgatcactatgtgcatccgaccgattcataacatatacatattccgggtccacctgtttaaaaatatctgagatcttcggaaccatttctattagcgaggcgccatgtaaatgcattgtaggatagtcgagttgaaaggtctcttttatccccaataagctggcaactttttcaatctcctgttgacggctatgaattctttcctgactaaatccatactcttcaaacagtttggtaacaatcagccaaaaaatgttatcgccattcttcgtatgcttcagtaatgtacctccagcacctattacctcgtcatcaggatgtgcagatataataataatatttgccataatactatagatattaaaatataaccaattggctatatcagataaaatcactaaaccttataagtgatatttttatatatcaacttatcatttatagaaatacttctcagcacatcacttattttctttgcactattgccatctccgtaaggattcactatgccttttacggcagcacggtaaacagggttataaatcgattcccggatggctgttgcaatttccactctgttatagtcaacataaattacatttccggcactaaaccgttcgcgttgacggctaccaatatttacaaccggcaggccaatggaaggcgcttccaatataccggaacttgaatttccaatcagcacagcggcatttctgagtaagttaatataattgacccggtccagatttttaaacaggtgaaaaatttcaggatactcaccggcatatttacctatcatctctatgatggcgaagttccctgcatcagaattgggataattaataaaacactttatgcccagatcaacgactgcctccaatgtttccactatctgcttacccgcatcagtggcttcggttataattgggtgctgtattaaaaccaaatatggctcgtcgcctgttttcaatacctttagcggcgcaatttcattttttggaatcaccgggcaatgaacaaatttatccaatgcaggattccctgtattaaaaatcctgaagtcatcttctcccagcaatcttaatacctgggcatgctgttcaagaaaagtaaaatggatgtgcgcaaacttggaagttgcatatcggacagcgttatcgatattgccatcattagcaatatcgccaccagccaggtgagctaccggaatacttaaatacgcagctgtcatagacacggtaatagcctcctcacggtcaccaaccaccacaataatgtccggttgctcccgtgcaaaagcatgagccaggcccgtaatctgggtacctattcctaccactcttcctactttatcttcactactaactagattatagatcctgtcagcaatttcatatccatcgttttctatattcttaactgttttgccaaatgtctcggaaagatgagctcccgttactattaacttcagttcaatatcattacagttatttaactgttcaagtaccggctgcataatatcatactccgatcttgcgcctgtgacaaataatattttacgtttttgaatcatttgcagtgggggttattaataaacatctgaatctccaagctggaaccaccaattatctgcggattccaccgtctgggaagcaaagctccggattccgaaataagttaccggcagaccgttgctaaatcctagcttctcaaaagataaatgcctgccatctttcagcggtatccaaatattaaatttttcatactcttccgcaggaaataatgctgcaagatgctgaagtactactttcgtaattctctcattatctgcgaagcaccattcgacaatatctaattgctttttcttaccggaaagctggaattcttttagcactacaaatccttcatccccggaagtgttttccagaatcacatatttattggagggattattaatatatctccagttcaaatattccgtgcttctcttcacttttacactgtagttattaaatattcctgtgtgcaaatcttcatgctgagttgtaaacttagtaacgatactaagcgatgccgactttttagctgttataacggctacatcgcaagacatcattggtatggttgttatatctttccagtccagatttttaataaatcctctatgggaattattgttaggaaatccccatactgccgtcatcccgtgaatctgcatcatatccttgtatagtgcctcagataattgctggaatattcctaatcctgtgtactccggatgtgtcatggtggtcatggaaagacctgttagctgttgttttcctgcgacatccaataacacgggggaaacagcataatgaccaatcagtttctgttcattccacatcaattttattgcgtacttattacatggattatctttaaaccgccagcgccagtatgctataggcattggtttcccaaaaaccagttcgaacagttttattatctcattctcatctccacctgtataatcacggatttccatagttatcttatttaaagtgtgatcagttcatctgcttcaaaatccttcacggctattttgccaataacatgatcccattccatggggctgataccattccccggtcgtttaacagtgaggtttttttcggaaaacagttcccctttctttatatcagcagcggccacaatactttttcttgccaccaatttgttcttctcttcgatagcagtaggagccttatttcctgtaccaagtgctttttcaatattccggatggcagctaccatctgcttcaactcagtaggatcgagcgaggctgcatgatctggtccctccatagtcttatccaacgtgaagtgtttttccacaagagtggcacctaatgcaacagcagcaacaggtacttctattcccagggtatgatcagaatatccaacagcaatatcaaatttctctttcatttgaagcatagctttaagattgatatcttcaaccggtgccggatattcgctggtacaatgcagtacagtaacttctttcgcggttttaccttcggcaaatataacatccaatgccgctgctacttcctctatcgtggccatacccgtagagagaataagctccttaaaactttgcgccatttttctcagatatggcaaattggtaatttctcctgatgggatctttcctaacttaattcccattgacttgagtaaatcaatgctttcgagatcaaatggggtagaaaggaaactgatattcttttcgttgcagtataaaataagctcgtcatgggcttcgggtgtcagttcaagcttctttaacatactcacctgatcttcggcctgtattccggtatttctcagttggtaatccgctttacgtgcatgcttactggctatattttccgctttaaatgtttgaaacttcacgtaatcaactcctgcatcggaagccgcatcgatgagcgcctttgccagttcaatgctgccattgtgattaacacctgcttctgcaattataatcgtactattcatgctcatgcaattcttgtaaatggaacacctatgtaagtgcccggttctttaatatttttatggactaatgagccggaacctatcctgacatcattgacaatacttacaccatggttaattgttgcaccacttcccacaaatacttcttcgccgattttacaattcccattcaccaatacaccggtagaaatatgacaatgatcaccgatggtggagtcatgctcaatcacagcccttgtattgatgatagcattgcatccgattactgctcccgcattgatataagctccatgcatgatgatactgcctttgtttacaatagcatattttgaaacatgcgacaatggagaaatcacagtggctatatttgcattatttgatgacaataattgccacgtctttgttcgtggcagtgctgatttaatctggccaatggttatgagaaaccagtagccctgctttatcagtccggcaatatcattgtcattcccaataaccctgtaacccaatacctgcgaatccaatttatccggaacatcaataattccttcaattgtaaagttccctgattcctcaattacatcgatacatgattttgcatgtcctcctcctcctattaaaatcagtggtttccccatatcattattttttccgacaaaggactatttaagctgttaatactgtataattcctgcgccccaggaatatcccacaccgaaaccagccaccaataccttcatacctgatttaatcttcttctgctcctccgcctgtttaagggctatgggaatggtagatgagaccgtatttccacaattggccatgctaacaaaaaacttctcttccgggattccaagtttaagtcgtaaatgatcaagcatatacttgttggcctggtgaaaaacaaacagatcaatatcctcttgttccagactattcttttgtaatatctgtttcaccatcaccggcacagatctgagggtaaacgaaaatatctcggcgccattcatgaataaggtggtaccagataagccattaggactgggaatggtaccttcagaatctgaaacacggggatggcgcatacctcctcctttcactatgaggttttccgcaccgctaccgtcagtaccaaaagtaatagcccgtatgtctgccccgtgaccgtttcttttaatgaaagttgcactggcagcatctccaaaaatagttcttacgcttttatcgtgatcatgaatatgcttactgtatgtttctgaagttatcaataaaacgttctccacgtctccggaacaaattaatcctttagcgaggctcaagccatatacgtagccggaacaaccaagattaaaatcgagggcacctgccgtggttggaatacctaaagcgtgctgcacaatacaagccgttgtaggtaaaaaataatccgggctctgcgtgcacagtaaaataaattgtatctccgaaggagttattttatgttcctcaaacaacttgcttgctgccttgatagccatcgacgaagcaaactcatcttttgctgcaatccggcgctctatcacaccggttttggcagctattttatttactgaccaatcaggaaataattcatgaaggtcatcattggtcaatgtttcctccggtaaataatatgaaattgcatcaagtgttatcatctttaacctcatataattgttaaacctccatccacaaccaaagttgttccggtaatccatttactggcagctgaaagcagaaagatagctgcattcgcaacatcttccggctcaccataatcgcctaaaggatacttcaatttatcttctttcacgctctcgtcagacacttgttttatcatctcatgatacatctctgtttttatcatgccaggagcgatggtattaaacctgatcttccgggaggcgtattccagcgccattactttacttatgctgttaagtgcactttttgaaccggcataggctccaaaacctttaactgcagtatagactccattcacagaagtcagaaaaaccaccgaggcggctgattgaatcttttttttattcaacaaaaggcgtgtaagattaacaggagccaggtaattggtttcagtaatctgctttaactgattgaagtccagtatttttattggagcaagcttcaatataccagctgcatgaacaattccatctagaggaggtatcttatcaacagccgcagcaattgcaatttcatctgtaatatctaatgataacacaatatggccggccccatcaagcagctccttaacgttcgttagtttctcagcgtttcttgccactaaaataactttcgcgcccatcgacgcaatcgagatcgcaatttgcttaccgataccggacgatgctccggtaataagtattgttttctcttgaagattaaacggggattctggcatcaatcaaactattattatgcaattactatatagttgaaaactatcttctatttcgcaatgatattatacaactcctcaacagtagcagcattcataatatcatttcccgagatctgtttattatattccctgtcgaccatagcaattataacgagactggtcattgaatcccactcctctaattcacgatagttagtggcggctgtgattgtgcctggctcaacatcttcaagctgctgctcaaattttgtaataaactcttgtattcccatttattagtatttaatataattatctaacactgcttggcagattaacgactctttcctccagccataaagcatttgtgagatctgtagattggcatgcagcatacatctgcaatttattcatcaatctccagattggccttgtcattaccttctgctcgttcgtttctttaagaaacaaatgctgggccgtatgatccggcaaaatgattgcatttaaccagtaattagcctttgtgttctcaatttcccttacaaactttatgtccgttcccgtaaagaattcagcatataaatcagcgagttcccgtttgttctgcaacatcatttccagttgttccagctgtgcacaagccaaagctgcattaagattcgacattcggtagttatagcctacctcatcgtgtacaaactcccaggcatggggctgctttgctgttgtggataaatgcttcgcatgcaatgctatggattcatcatcagtaacaattgctcctcccgcaccacaggttacggttttattgccattaaaactgaaggtgcctatttttccgattgtacctgtatgcttgccattgtaatagctaccgagtgactccgcagcatcttcaaccaaagcaatattgtatttcctgcaaatatttgaaatatcctggatcctcaatggaaacccaaaagtgtgcatcggcacgcacgctgcgatccgcttcccggatactttattgatgcaatttccgctactatcaatataagtgtgatcgtgtaaaaactgttccaggcttattggcgacatccccattgtatccctgtccacatctacaaatacaggtattccacctgcgtgaacaatggcattggccgtagctacaaatgtaagcggctgcgtaatcacctcatctccatttttcacaccagccagcaaaagtgccagatgcagggctgttgtgccatttacggtagcaacagcatattttgcgcctgtaatctcagtcatcatcttctcaaactgcgtaacataagcacctacagaggaaacaaaagtggaatctattgtatctaaaacatactttttctcgttacctgtaaaacggggagcatgtaatggtataaaagtatcttgctggttaaaaactgtcctgatgaaatttataatgggctcaaaatccataaccattctttaaatgttgtatatgtttgccttatagctactgaggttaccagggatagaaaaccattcgatcgtttcttttagcccttcttccagtgtatacttttgcttccaggctgtatgctgactaatcttctctctggatccatacaagcgaaacacttcacttttttcaggtctcaatctgttttcatcctgaacgattcttgcagctggattcaggagtttcaccagattggcagcaagatcaccgatgctcacttcagattgagttgcaatattacaatcctgtccgatcagggaatccgctttagcaatctcaataaatccatttgcggtatctttcacgtataaaagatccctggtaggcgtaaggtctcccagacttatttcagttttaccattcagtaattgtgaaataatagtcggtattactgctctcgccgattgccgcggcccaaaagtattgaagggtcttacaattgttaccggtaaattaaagctcctgtaaaacgattctgcaatacagtcagcaccaatctttgaggcggaatacggtgattgcggctgcctcggatgcttttcatcaataggaatatattgggcagtaccatatacctccgaggtagaggtgacaagtaccctctctatattgagatctttagccgcctgtataatatttaatgttcctttgatgttcgtgtcaatataagagtcaggagaatgataactaaagggaattgcaattaatgccgccaggtgaaacaccacatcaatgtctttcatggcggttcttacaccgttaggatcccggatatctcctgaaaatatttcgagttgggacagctgatcctgcgataatgtatcgagccaaccccaactattaaaagagttataatatacaaaagccttcactttacaaccctcttctagtaaacgttctgtcaaatgacttcctataaagccatctgcacctgttattaaaacccttttattctttagttccatgattattctaaattatttcctgatttcaatccactctgaatagtataattatgccagtatatctttgagtaccttcctcagcgtaagaaaaataacaatgaagaaaccacccatcaaacctccaataatcacacccttcgtttttcccagtttttcttttttcaacggcagaatgggcgtatcaataacctggatgatcggagtttcctgcgccatagcaattttacctaactcaagatttttgacaacttcaccatacattgtttcaagtaccattttatctctactcgccagttgtgtatttatactcgctacctgacgggccggattcatattaatatcctgggcaagtgctacggaatacgttttccgattcaacattttttccaacgaatccgcttctgcctgtaaacggtcaacattcgttttggaccgctgtgtcctggtgtcaatataaaaattggttgcctcagtcattaaacgctccgtgaatgctttcgcgaaaagctcatctctggttgtactcctgactacaataaagttaagtttcttgtcaaccttttctactttcaataccgactttccaattgactcctgcaatgtttgcagaatactgtcctgaagcagggaaaatcgtcttctatcgccacccggtgggaaagaaatgcctttcaacgaaggtttggcggcccaccctaaacgaagctcattaaaatctatatatctctcagcgagcgtttgctttttaccatttatcatcacagtagaaagcaaagccttttcaatcattaaccttgacttaagaaaagtcatgatattatcaccctgaaaaacaccattactccccgaaccaccaaggtcaattccaaactggctggcaagtccggcataagcccctaacggactgccgctattgtcctccacaacgaaggtaagttcagcgacgtatttggtttttaaaataaacgataatattaatcccgtagctccacctaaaataccaaacagcaaaataatataccagttcttaaggaagtatttccaccaaatgcccaattttataacaagttctctgacagaaatttcatcattatttttatcactaacattcgtatttatattagaaatctccatttggttatatttaattgcaattcctgttttttatacggtgtttatttaactcttgtcaggattgtaacaattattaatgcaatggacgcaataccactacttagtccaactacttcctgtcctgataaacctttcctctctctcttgctcggaacatatacttctgcacctggctttactttgggatacttattaaagaagaatatcttcctggtactttttacttccccatttgcgtatacaacgtaacttcttcttttcaaagccgccgatgtatacccacctgctcctcttatataatccctaaatgcataagctttatcgaaacgaattttcttcggaaaataaatctctccaaataattgaacagtttgtaattttttaggaatttttaatacatccccctcttctaacagaatatcatatttcgatcccggcttctttatgatatctgccagattaatccctaatagttgatacttccgctccatcatactcttaacgctattaatacttgagctgtcttccagcttattgtagaataaagcgagcttgttcgtaagcagagccgaatctgaaccatttatgtaggttttacgcaacaataccgctccttcaggaaaagcttccggcttaaggcctccagatctctcaataagattagaaatatgttctcctttattaacaatggaatattgtcctggataaactacttctccatcaattaaaatattagcctgctcactgtaaaccggagatttacgaatactaacctcgtcaaacggctccagtaatacttgttcacccgcaatagcattcaaatctgcgttgatatcaaattgtttaatgatagcctttgcactgtccttgccattgtaatcgcccttcctgattctccttgatatttctacacgtttcaatgatgctgcatccctgagccccccggataacaaaatcagatcttccaaccgcatactatcagcataaggaaacgcccctggtttgttaacctcacctcctattgatacaaaatattgctgtctcagatctagcttagagaatacaattacactgtcttctttcttaataggaatgctggatttaccactgacaatatcctgtacattaaagctaatgatagctggcgtaaagtcatcctgcaaacgccgtataatgcctctgttcaaagaagcctcttctcttatgccatctgcttttttaatcaaatcggccaccgtcattcctggctccaaaccataatttcccggatgaaaaacagcaccgctgatagtcacgcggttactaaaccggttcaaaatagaatctacaaaaaactgatctcccgacttgagcttaaacgtggcaatctgatcagcggggacattgatgacctctctttccttattattaatgcgataccctgttatgttctccttaaacgaaccatccgtatatccgcctgcataatccagtatattctgcaatgtctcattttcctttgcctcaaaaattgcgggccgcttaacttccccgactaattcaacacgggtcttatacggattcactttcacaatatcctgatcctgtaacacaatgttattggtgagatcaccctgcgtaagaaaatcatacaaatcaaatgttgcagctacatgaccattacggatcacctgaatacttcgaaaagaaccattatcatcgggccctccggatacatacaatgcattcgctacagtagccaatgatggcaacgtatatgttcccggccgttgaatctctccaataagcaatacccttatactacgaatgttacccagtgatacctgtacaaaggttttaccactggaaatagtagagtatattgtagacaactgctttgttattctgttcttagcctcatccattgtcaggccattcacatataccggtcccagattaggaacacggatatacccctccgaagtgactgtcaatttatactgcacctcagagtagccatacacatctatcattacctgatcatctgcagctagtctgtaattagagggagttggtattctcaggttaggttcaaaagtcagattcttatttgtaaacaattcagcgccaaatatcttctttcgtttaatttccgacggactcgcattttgcctgaataaatcaacctgagtggtatccgaatcattgaatgaccttcctgaatattgcgtgtcctgctgaaaaatctcaccgcttttctttttttccagtgatttatccagtcccattgcctgtatcctcgttttcaatttcgccgcctcggccggaggcacccctttctgctccgcgtacgagtcaatatcatccatagacatattattctgtttcatctcagcaacgatacgcctgatctgatcatctgataaattatctacgtttacttgttttatctgagctggggacggtacctgtgccattacacaaaaccctacaaacaggaacagttggaccaacagtatttttcttaacatgtataataggatctaaaactttctcgaataccttttttggaaacaatcttatccggcgccggccaaataaggtgcaaatctattaaaaataacatataaatgttagttcctaacacttttaacctgaaaaccttatgtgctgtctgatatacgtttaaacatcttcccgggtgttgggcacaccccgctgcaaatatgcatccaaatatcacctatccattaattttaagttatttataatatgtgaatattattaatacaataactcaaatccttttctcactcttttacgttaatgcatatagagagtcacctgtatttacctgtttgagaaaatttggatcactacttaaactaccacctgttttaccgatctaaatattaggcataagacaaattacttgataatcaataaaatataacggaaaaatcatgtattaaccgccccgcggtatcctttgaaaactatttaccctgttttcttgtttaaattagttaaggcaaaacttaaacattatgtcgtctgttgaatttaacaccttgcttgtcggaaacgctgatttcctgaaaccctttgcttttaccctcaccaaagatgccgaacaggcaaaagatctttaccaggaaacgcttttcagagccctgtccaaccgggaaaaatacctggaaggcacaaacatccgcgcctggctatttaccatcatgcggaatatctttataaatcattaccggaaaaaattaaaacatcgcaccgtcgcagaaccaagtgccagtgaattctttataaaccatcatgagaacatcgtcagcaataaagcggcctctaacttacaaatgaaagatatccatgtggcagtttaccatctgccgggcatcttcaaaaaaccctttatgctttactacgagggttacaaatatttcgagattgcaaatatgctgcaagaaccattgggcaccattaaaagcagaatacatttcgcccgcaaaattctcaaatcacaggttccaagacaataatcccttacccttaccgaaaatcccacacgcatccgtccggccaaaacgccggataagcattgctatgaacggggataaccgtacaccaggcgcaggtaatgctccttgaggtgcgactggaaataaaaagcagtaatcataataatagcagctgcacagagaaatgcaggatgaggccagcaataataacctgccaggcacaataccaggtaacgcgcatactccaggtaaaacacccatttcttctgctccataatagcgccgcagttaatcagcgtaagcaggatgagcagcgctacacatacctgtataaataccggcacatagtgctccagcaacagaaaggaaaacaatacaaccaatgtggccacaatttgccacaaaacataattaaacagtttaggcgcctccgtgatatggggattacgcagcaggaacttttcctccaggatcttccgcgcccccggatctacattgtccggtttaccaaaaatcacgcgcagcttattccgccagccttttgcctgccgggcagaatacaacatctccaggataaaatggaaatgctgccacaaaaaactattgctttccagtggcttggttaaaccatacaccggctcctcttcttcttttacaaaagtgccaaataacttatcccatattataaatacatcaccataatttttatcaagatactgggggttacttgcgtgatgcacccggtgatgcgaaggcgttaccaatatatattccagtatccccaacttcccaatggtacgcgtgtgaataaaaaatggatacagtccatgcaccaggagcatactggtaatcatagccggaggaaaaccgattacaggaagtatagcccagaaacccgtacgtatgaaagcctggaacaccgtaatccgcgcagataccgtataattaaactcttcactctggtgatgcaccacatgcgcgcaccagaacacggtaacttcatgcgccaaccggtgataccagtaccagataaaatctgtacagatcaacaacgccacccataacaacacactggatttgatatcaaaaatggcaaaatgacgatacaagtagtcgtatacaaaataaaaaagccctactgtaaaagtatccagtaagcgctccgcaatacccacactcaggttggtaatagaatcattaaacttgaaataagtctttccgttttttcgcgccaccaggtattctaacccaataaaagtcaggaaaaaaggaactgccaatgccaggtagtttaaatgcacttgatataattttaaatccggaaatccaaatagtaagacataggctaatacacggtgccagcccatgcataggtttaactggtaaaactggtggtggtaaattaccacaatgataaggaataaaatttaattatcctactattttaatagactaataaaaacgaaaggcggaaacaactttcgccgttatccgccttcgcttcattgcatatttttatcagtcctccggaggtccgccatcagccattcttaccaccttcggtacaaaccggccaattacttccaccagcgctgtttgcgccgccatcaccgtatcaatattcttatacgcacccggcgcctcatccaaaccacctccaatcagtgttacaccatgttcctgcaattgttgccttaacacctgttcagtgatagatgactttgcccgtgtacgcgacatgagtcttccggcgccatgcgacgcagattgtaaactttcctcttcaccctttccacgcacaataaatccgggcgctgtcatggatcccgggattacacccagtactcctttacctgccggcgtagcccctttccggtgcacaatcacctcttttccccggtatatttctttccaggcaaaattatgatgattctccaccctcgccagcaaagtggcgcccgtagcggcaatcaaccgcttatgaatcaggtggtgacaggcagacgcatagtcacccgccaggttcatcgccagccaatactcctgcccttccgctgtatccaggttcaggtaagccaggtgctttgcatgttcgggcaacgggcaaatctctttcgcaagctgtgtatagtgccccgctatctgcgcacccattccacgtgaaccggagtgcgacagcaatgccacatactcaccaggcgccagctgccattcattctccggatccgtaattgtggcaattccccattccacgaaatggttaccggatccggaggttccaagctgccctgccgctttatcaaacaggtttcttacaaactttatctccttaaattcacttctctccagcaccgggtccgcctcccgctttttccactctgcaccggctccgaattttgtgaaagtcatcagctgcttagcatacgatgtttcattcattaacaacgtttgcaccggcaaatccaatacactcaaacacatacggcaaccaatatccacgcccactccatacggtatcactgcattatccgccgccaacacaccacctatcggtaacccgtatccctggtgggcatcaggcatcaacgaaccggcaacggcaacgggcaaacgaaccgcgttatttaattgcttcaccgcgccctcctctatataggactccccataaacggaataaggtaccggcgtttcacgcaaggcaatcactgccggcgctgctggcgtcaacagttcacgggctatttcacccagtatcgcatcatctgcatagacagcaggatccgccagtactttggtcaataattcaattgctgcttcttccgttaagtgtccataatgttgttctataacattcatggctatacggaaaacaggactttggggataacctatctccagtaattttctaccgttgatttttaaacttgacataaagggttaatttattcgtaccattcttcctgcaacagttgctgcagggtaaattgcttaaattgatatttcttcttatactccggtaaccattttctccggctggattgctggctcctcgtaaggctccatatcctgtgttccaattgatgctgcttcagaaagtcatccaaccggtccatctctgattgcagttcgggcgctgctacccgctgtttggtgatcatattggggcgtacctgcaacacaaatcgccagggttcttttacaacaaaatactttatctgatcaataccgttcttacaataacggacccgttcttcaaaacagttgatctcttttggggagagtttcatcttcttaaaatgataatccaccggttgcagtaaatgctgctccctcagcacatgtatcttccttcctctctgtcgcttctttactttaaaatctttccggtggctataatcatacgtattgatctttttcaacagctcctggaaaaactcaccatcgcggctcctcatcacatcttcccgtaaaacaaagtaccgtttgtaacctttcattaccggcggatccagctccgtataaccacgttgattccatgcctgccgcaattccttccgccttctgctgtattgcaataactgtttgtcgtattgtttaagcgcatcgcgctttctgcgcctgcacgttcttatccgtgaggctgccatataattttcgatttcctgattgtccatcatcagtcattaaatgttcaatattgtttactccgctgatatatatggacaattgattttttttcatttttattaatttttcaagatgaataaatactatttacgcgatctcttccagcatttcccgcctgaacccgatcacatgttgttttgtttcaaaagagggttcatgctgattggcaatttctgcaatagtcatcgccttattgatcaccgtatcaaaacccatgtgctttgataatgcctgtgccttagccaccggcagccgtttgaactcgtactttgcaatcagcctgcctttacgcagcaacgcattgtcgatagcggataagtcgctgttgaaagaacaaaccagctgtatattcaaacaatctgccaataatccatccgacaggttcaacaaatttgaaacagatgagttaccggaaaacttacgatccataattacattttcagcatcttcaatgatcactacacaattaggattatcgatcagcagttccatgaactcaggattcataatgttgtttgccaggtccggcgaaacaaaaagcacccgcttctttatccggccaatcaggtaacgcagataagtagttttacctgttcccggcaagccatgcagcaatacgatccccttgtctttatccttcttcagccgctgctggattaccttgtctatctctttaaaatcatcttcataaaacatacctatatccagcttggtacgttttatttccaggcttttcagttccagtcctttacgtccgctggtgatcaggttaatttcatgcggttccctgcgttgcttttctttatatcgtgtaaccgtttccgttacttctgatacaaaggcaggaatagtaccattatgcaatatctcgcaccacgattgccagaacgctaccacgctgttattacttaacacaaacagcgtttgattatgcttatactttttcttcttgttgtcataatcggtatagcggtgcgtatgaacaataatactttcatatttcttggcaaaggctgcggcggctttatcaccatctacttcgtaaatgttattgatatcggggatagcactaaaatgaacggtatacactcctttcggatcaaaatgttcaccatctgtgatatctatgttattattaactatctgcttcatagctgcttgttctctttaatgtgatgttgtcctgatgataaagatttcccgggaccaggccgggcccgggtaaatcgtatttatcatggggtaaattacaggttatccttctgataacctgatgataaggggttaaaaatgcaaacagagacgaaaaaaaatatcttaaaaaggagatgaaagcggagcaggattactccgcctgcctgttttttatgtacctcctcaaataatctttatactgccgcataaaaaaacccggtctgtttaaaacggaccgggtcatataacgttaacgtatacactacgtcaagacatacctcgtccgtttagcattaattgaattaatgctatctctaaaccatttactgcggcggatttgaatccgttctgtcattcccggtaaattcatcattccaataaatcgataacaaaaaagcccggatccaaggacccgggctgctgttatacttacaaatattttttatctacctgtaatcataaaacgcccggaatccgctgccatcttgctctgagcaaggtgttgcgttgtccatatatagattaatgcgtttcatgtttatcaatttgtttattatcaattttaacgatgcaaagataacaggatatattttgaatttgcaaatttttaacaaaatattttcaactattttatttatgttttttttgattttcgaaatctgaagcagtgtcaatgatctgcagcaggtcacaaaatataagcgcaataaaaagccggaagtgataaacttccggctgtagttatgatcaggattaacaaaaacagatggtggtggtcgacctaagttatattaacaccgcgctttcttcgaattccttctgaaggcgctgcatctgacggatatgccgttcgatatgcttggtgaggaaatagatatactgatagatgtccagcttgcccagctgatttacagacatgttagtgaacaccagcactccttcaccgtttttcagtaaagacaggttgtacatgcactgtgcatactgttgcttcaggagggcttttacttcctgcatatttttaagtccggtaggttccatatgttcgggtcttacccaaccaaaggatttgctgccgatgacatctatttgttctaatttattggcataatctgccgggagtatcacggagtggccggttttcttacgttccagcgcccggcgggtactcttattgatgatcagcagcaaaaagtaattggtgagcgtaatatgctccagtacttcccgtatgctccattgatcacggtctggtttgaaatccagtaatgccggttctttttcaaaccactgatccaactccctgaaattggtgagtaaggcctctcttacaacttgaataacgtttctcatcatctaacgtttttgggattatgcactttacttctttgctaatcaaacgggttagcgcataacatctttgaataaatattttgtttgccatttttatgccggatttggccacaaaaaaacccggccgtatttacggaccgggataaataatgtagaggggttatctcacattatcgcataccttgtccgtatggcttttttaaggcaaagccattccgtttacgccatgaggcgcatttttcttgcattacagttatcgcttgaaattctttcaatgtcgtcatttcattactgcttcaaaagcaaaaagtcccacacttttctctagtgcgggactcttgtttatatcgtttgataacttttcgttcgttaacaatcggtgcaacatgcccgcattctggccttgacctgcttgtgttggcaggccatcgctgaaatctcgtatgttgatataagttgcacagttatttttgttcttgaagcaaaggtaatttttattttttttattacacaaaaaaacaccctacttttttcccagacttaacaattagtttaaagtgcaactacatatcattgataatcagaacaggcttaattgcgaattcggccggcggaaggctgctgtattgaattcgaagcgttcctggttcaagccattcttctttgtatgaattttaaactgctgctttatgaggtccgcaatgttgccttctcccctcattctccgcccaaagtcgctgtcattcacctttcccccgtgcatactttctatatggtgccatactttatctgcccggtcggggaagtttttatagagccagtcgttgaaaatgatcttcaccgcatcgttgagccgcactaccgtataccctgcatatttagcgccattggctgctgcagcttccagcaggcggggaatttcatggtcattgagtcccggaatgagcggggccgtcataacgccaacgggtatcccaagatcactcagctccttcaccacctttagccgttgcgccgccgtagcggtacggggctccattttttgccgcaggtcttcctgcaacgtggtgatagacaggtacacgcataccaggttatcctgtgccagctgctgtaacaggtaacgatcccgcaataccagcgagtttttagtaatgatccctatgggctgtttgtattccagcgccacctccagcaactgccgggtaagccacatcttgcgttctaccggctgatagcagtccgtattccccgaaagggaaatcggcttggggtcccactttttattatccaggaacctgcgcagcagttccggggcgttatgttttacaataatctttctttcaaaatccaaacccgcgctcaaaccccaatactggtgggtgttacgggcataacagtaaatgcagccatgctcacagccctggtaggggttcatggaataccacatccccacatccggactgtccaccttattcacgagatttttcgcatgttcctcgaacacctgggtaggtacatctgcctgccaccattcatcaatgccttcggcatgctcctgcgcatattcatctgccaggtatttattcttgggattaatctgtgctccgcgccctttatagtatggattttccggtgcgccctcctggaatggcaaagtcatagactaaatattttagtaaaaatactaaaatatttaggatttaaataatttccatttgcttcatcaggaaagtggcgtttttatttctcgcaataccctcccggatgcggtagtcgaaaaacaaatggttgtcctgtatagtgctttcaaaacaataattcctgatctggtgcggataagccgattccagctgccccagttccaggtcgtgcgtagcaatcatgcccaggcagttatattgcaggaaatgctcaatcaggctgcgcgagcccgataatttatcttcagaattggtgcctttgagaatttcatctaacaaaataaaaacccgcgcaccggttttcaggtgatggataatatgctgtaaccgcagcaactctgcctggaaataggaagtatgactggcaatcgaatccttgattcgcatggaagtcatgatacgcatagggctgaatacaaaacggtccgcacacaccggagcgccgcacatagccagcaacaggttggagcctacgctccgcaggaaggtacttttaccggacatattcgatccggtaatgatcaggaaatgatctttacggccagtggcgccgtcattctttacgcattcattggccgggatcaacggatgccccagtgccgtagcctccaggacacgcccttccgcttgcggcgccggccacgaaaattccggatgattaaaggcgtaggtagccaggctgttccacacttccagctgggtaatcacatcaaaccacccggtaatgtgctgtttatgctgtttcttccaccgttccaaacgcaggatgcaatggaggtcgtacagcatcagggagttaagccccagtccaatcaaaaggtttagccgctgatcaaaggcattacatattttagacagctgccgcaatgctacatcggcttctttggccttatcctgctgttgctgcagcaacgcggattttttgaaactgccgttttttataagatgtaataagatagaaaacttatccagtatcctttccttatgcgaaatcaatacatattgcgccatgatctttttctgactagcgcccagcagcaaccagtttaacatgatcagtatcaacaacgggtagtatttaccagtgatggcataatatacaatggagccggttaccagcaaaggactcagccagataaccacatttataaatttgttgtgcagaaagtggaaaggcatttccagccatgcgctgatttcccggcgatcgctttcttcttctttcgccagcatggcattggcagtaagcagctgccggaactccagttcgggtgtaagtacctgcaaagcctcctgtgtggccagaatagccggggcatcttcaagcgggtcacgcagcgcagccgccagctggcgtctgccggacaatgtacccgtgcggttaatatgctgaaaaacagaagatggcccaaaaacatcgaggtcgctgctgaaatcatggctgtcgtccacgaactcattcccgtcgtcaaaagccgattgcccggtagtgaccaactgccactccttctcattcaactccagcagggatttaaaaagctgcagcttctgctgcgctttggaataccatatcaacaacactataaacgcaagcataccggcagctgttaccagcagccatggcgcttcccagccgctccggataaaaaacacgatgccggctaccatcaccaggaaactggccagccgggcccatgaaaggctggcggttaaccgcttctctttttttatcgcttcccggaactggtgaatcctttgctggtaaatatctgctggcgtcatttatctggtattaataactaaaaaaatcagggatttcatgatgtatgttcgcaatatattgaacataaaccacaaaatccctggtagaaataactggattatttatgcgtattgtctcttcagcagatcaggatactcctggcttaccttcaggatcagttcaccaaagagtgtattcacccaggcaaaccacggacgggtaaatttagagggatcatctttgtgataagattcatgaataaagccggtttcaccgtcggtattgcgcaaggttttaatacaggaagctatttcctccttatcatgactggtcaacgcccgcatgataatactcattggccagatatagtcgttgccggtatgcgggctacctaccccatcgccatatttacccctgtaaaaccagggctggaaattactccatacaaagtgccgggatgcctggtacaacggatcgtcaatgccggtatatcccaggtaaggaatagacaggaggctgggcacattggtatcatcgaggaataaacggtttccgaaaccatctacctcaaaaccatacatcatacctaacttaggatgctccacaatggcatgcgacttaatagcacggtctacctcatcagccagcgccgtacattcgtgcgcaaaggccgcatctttatatattgtttcactgatttccgccagctgacgcagggataccacggcaaacatgttggacggaatcagaaaaggaaatactgtagcatcgtctgaaggacggaatatagaaacgatcagtcccaccggagaaatagggttcccccagcctccgttggcaacagtatctgattgtacaggtgaattacgctgaaatttgtaaggaccgtggccgtctttacgctgctgctccttaaatgttttcacgatgagctgcgccgcctgtttgtatttatcatcgaagggggtattatccccgctgattttccagtaattataagacaaccggaccgggtaacacagggaatcaatctcccatttgcgttcatgcagctccggcttcatggtggtcagatctttatcccattcgctgccggtagggccttcattaaaggcgttggcatacggatcaatgaggatacatttcgtttgacggttgataacgcccaccaccatttctttcagtttcgcatcatcctttaccagtggcaggtaaggccatacctgggcagaagagtcgcgcagccacatggcgttgatatcaccggtgatcacgaaagtatcgggccggccgttttctttcttaaagttaaccgttgtatcgagcgtgttagggaaacagttttcgaacagccatcccaatttggtatccgcaatctgggactttaccttgataattgtcttttccaccgcttcgctggtgaatttccgctttgccaggggcggacgttgggaggtatacccattccagccaaatactgttttgggcaatccaagcccaacaacgcctgctaccagggcgccgttcttaagaaaatctctccttgcaaccataacgtttttgaatttaggaaaccctaaaatagaaaagttttgcggatttgcttaatcgatttatcaatcgtcctcatcttcggcagcccgtaacttcacaaaagcgcttctcctgggcgccggcatcactgcctgttcaccatgaatagccttccacaccacctcattcagctccaggtcaggcacccggtcttcatgcgccaggtcgaagctggccgaccggcgggcgctttcattccaggcagtatttctttcgttaatatccacatttgcaggcaatacggtgtacggccgcagatcaggcgtagcggaaaataattcccacatgggagtagccgcagcatcatactggctcatcgccggcaaacccaggatcaactccatcgtacgcagcatacccgatgtggaatacatgttatgatttacggcattccgctttacgtaagggctgatcacgtaagccggtgaacggtgggcatccacgtgatcagggccattctgcgcatcatcttccagtataaaaatggcgctctccttccatatcttactgtgggagatgtaatctaccagccggcctaccgccagatcgttatcggccacggaagcatacggcgaataggcgcccttccgcatgccgctggtatgatcattccccaaacggatgctgttaaaatgcggtactgcatctatcgccagcaatgaatcgaaatcatgctgccagatttcctgccgcgcaatatcctgtatggaaaggtcgaaagaaggataatcgctgcagaaatgattgtccagcgatttcagcgcggcctttcccttgccggcaaactcaccgtaggtgcggtagctcacaccagcgcgctgacagtaatcccaaataaatcctttttccggataagccactttacggctgccttcatagtcgtagctaccaccgcgaccaccataactggtaggccatgtcttctccacgtaatcagtagcataagctgccatgctccagttatgcccgtcggcgcttacttccgcatctacataaaaattatccagtaatacaaactcgttggataaacgatgctggttaggagtaatgcgctcagggaaaatacataagctgctgtcgccattaccctgcggcatgtcacctaacacctggtcgtaggtgcggttttccttgataatataaaatacatacttaataggcgatgattgtccggcggcacggggaataggattccccgcttccccagcggcatgctgctctttctcttttgtgtaaggtgtattttcatacacctgtttggaccagcggcccagcagcgcttcgcccggttcattgaataccgacagtgtacctttaaataaaccggctatatactgtacgggcctatctttacgggtattagccaggtgcgatccgctttcatctttcctgctcaccggattaggcccttccggattagccatcgacgtaaatcccttgccattggctacaaatatttttttgccgatccttcttacacaagtgggataccatcctaccgggataaacccttccgacctgctcttacctggtgtttccacatcaaaaacagccagacagttattatcggcattggcaatataaagtgtgttgttattggcagacagcgccaggccattagtggtggagccggccggagcatccgggtacagcgctgtttgcagcgattcaatcacccgttgaccggtagtactgatcaccgataccgaattatcattggcattagccacgtacaaatatttcccgttggcagacaatatcatttcgttaggatgacttcccgttttgatagtgtttataatcttattagtggcaatatcaaataccgccaccgcatcgcctccccagagagagatgtataacaggttcctgtttttagatgagacaacagtatatgcttccgcacccaatgccactttgcccaccaccttattggtaagcaagtcgatactatataagctgttgtcttccttggtagctacgtataaccggttacgtgagtaatcaatggtcattccggtaggacaaattttctctttgggccacgacaatcccagtcggatactatctgttacctgtaatttattattgttgatagcatactgccatatcacgttatcgttggcgccggaagcatacagtttcttttcgtccctgctgaatgcaagacccagccaggctttggggatactcacttcatcaagtatcatctccttcctggcgtctatcagctgtatggtttgtttgctctgcccgttgttggtaaccgctatcatttttttcgacggcgatactaccatattcagcggtagatctccgagcggcaacgaatgccccaccggcgttaaggcccagccattgggcagtaacacccgcttcgccatggtatctgctgtttgggcatttgcctgcaaagcgctcaataaaaccaaacccaagagtattttcttcatagtagttccgataagtgaagctgtaaaaataggatagacatgcccggctgataatggccatcaaaaaggtaatactaatataatacaaagcggcataaaaaaagcccgtatcaatatctgatacaggctttttataacagtattaagattacatatttcttctgtactgccctcctacttcatacagtgcatgcgtgatttgccccaatgagcaatgcttcactgtttccatcagctctgcaaagaggttgccattgctgaccgctacctgctgcaattgcttaagtgcagcagcgctcttatgctggtgcctttgctggaaagcttcgagggtatggatctggaattccttttcttctgtagtagagcggatcacttctgccggaataatggtaggggagccgtttttattcaggaaggtatttacgcctacgatcgggaattcgccggtatgcttcagcgattcatagtacaggctttcttcctgtattttgttgcgctggtacattctttccatggcgcctaatacgccgccacgttcggtgatgcggttgaattccgttagcacggcttcttccaccaggtcggtgagttcctcaataaagaacgctccctgtacggggttttcgtttttagcagtacctagttcacggttaatgatgagctgtatagccattgcccttctcacactttcttctgtaggtgtggtgatggcttcatcataggcgttggtatgcagggaattacagttatcgtaaatcgcgtacagcgcctgcaaggtggtacggatatcgttaaaatcaatttcctgtgcgtgtaaactgcgaccggaagtttgaatgtgatacttcagtttctgggagcggtcgtttcctttgtatttatacttgatagccttagcccagatacggcgggccacgcgaccaatcaccgcatactcggggtccatcccattgctgaagaagaacgacagattaggcgcgaagtcatcgatgttcatgccgcggctcaggtaatactccacgtaggtaaaaccgttggccagggtaaaggccagctgggtgataggattggcgccggcttctgcaatgtggtagccggaaatgctgacggaatagaagttgcgtaccttttgggtaataaaatattcctgtacatcgcccatcagttttaatgcaaattctgtagagaagatacaggtgttttgtgcctggtcttccttcaggatatctgcctgcacggtaccacgaacagtgctgagggcatgcgctttgatcttttcatacacatctttatcgagtacctcttctcccgaaattcccaacagctgcaaacccaaaccatcgttaccggcgggcaggtcgccgctgtaatgcggcagcggatgatctttgaatttagttttgatgagggcctttactttttctgtaagcccctgctccttgatatatttttcacattgctgatcaatggcggcattcatgaaaaatgccagcagtatgggcgccgggccgttaatggtcatagacaccgacgttttcggatcgcagagatcgaaaccgctgtataattttttagcgtcgtctactgtggcaatgctcacaccggagttacccactttaccataaatatcggggcgtattgccggatcttcaccgtaaagggtaacgctgtcgaatgcagtagacagccgctttgccggctggtcgagtgatacgtagtggaaacgtttattcgtcctttcgggaccgccttcgccggcaaacatgcgcgtaggatcttctccttcgcgtttcagcgggaacacgcccgctgcgtatggaaattcaccaggcaggttttctgtgagctgccagcggagaatatcgccccagtctttgtatttaggcagtgatacctttggaatacggctgtggctcaggctttcgctgtacagcggcagtttgatcactttgtcccttacctggaactcataaaaatcggcggcatatttctctaccagtgcaggccattcctccacgagttttttacattcgggatgtaatgatttctccaggtgggctttcacgtcggccaatgtggcggctgatgccggctgcagcgccatcacgccttgtacctggtatagttgtgtagcgagtgtacattgttcatccacccatttgctgtaatcgccgatggcttctgaaatctctgccaggtagcgtaccctggccggggggatgatctgtgatttggtagaagtagatttaatgctttcatgcgccatagggccgaagctggccccggttttctcttccactttttccattactttttcaaacagcaggttgatgcctgcgtcgttgaactgggaagcaatagagcccactaccggcaattcttcttccttggcgttccagaggttatggttacgcttatattgtttacgcacatcgtgcagggcatccagtgcgccggccttatcaaatttgttgatggcaatcacgtcggcatagtccagcatgttgatcttctccagctgggaagcggcgccgtactctggtgtcatcacatacagcgatacatcgcagtaatcggtgatagccgtatcgctctgcccaataccggatgtttccaggataataaaatcgtaggcggccagtttgcagacatcgatggcttcctggatatgttcactgatggctttatcgctttcacgggttgccagcgaacgcatataggcacgtggatggtggatggcattcatccggatcctgtcgcccagcaatgcgccgccggtcttcttcttggaagggtctacagaaattacagccaccgttttatcggtagtatgattgagatagcggcgcaccagttcatctgttacgctgcttttaccggcgccgcctgttccggtgataccgagtactggagacttttccggctctgtggcagtatgggtaatgtgtgcgccggcggtttcatctacggtgacagcggttcttgttttctgcccgctgagcagggctaccggcatatcgttttctgccaggctgatagccctggcaatgatcttaggatttttgtctgcctgcagctgcgggatatcttccacaccggcgccggcagttaatggcttgatggccgtatcgcattgactgatcagatcctcaatcataccttccagtcccatttgccggccatcgtccggtgaataaaggcgtgcaatgccataggcatgcagttccgctatttctacaggaagaatggtaccaccgccgccgccaaagatcttgatatgaccgcaacctttttcctggagcaggtcgtacatgtatttaaaaaattccacgtggcctccctggtaggaggtgacggcgattccctgtgcatcttcctggatggcgcagtctacgatttcagctgcagaacggttatgccccaggtgaatgacctcggctccctttgcctgcataatgcgccgcataatattaatggccgcatcatgcccgtcgaataaagctgccgctgttacaatgcgaaccttatgttgtggtgtataagacatatcaattaccggatttttgaccaggggttcatgcttcctgcatgaaatccacgaagaatgcaagttacggaaaaagcagctgaactgccggtatagcgcgggtttacccagaattagaattgattgaacagctaccggatcttattgcaaaatatttaactgatccccgatcgggttagtatttccctaaaacaactttcccctgtacattacctgtacaagggaaagcataaagtaagacacaaggcattaatgcttagcggtcttctgtttcataacgtggaactataaaatcaaactaatgataaatgatttatagcttttcaaacttattaaatggaatttctacatacggaaataaacaaacgaaaaattgcttttggcgaacaagttaaattttggttttataacgattattgtttgcttctaagatgtgtatatcttacacaatcttacttaaagttttgttaaaaaccaacttttttttctatttagatagaaaattaacctggctgttttttgacagacacaggccatcgcaaatccttcgtgacaaaggatttcaatctcattcaaattaacaggaatacaagagaatgcaaaagtgatggagaaaaaaatatcagatcgtcatctttagaagcctattccgagataacgcttctttctttggtcatatttatcgaaattgaatttatagagctttgccggacgatgaggtacatcttcctcttcttcattcaaatccatcaacaaatccatcgacaaaaacttctttctgaaattacggcgatccagttccatatccaggatagcctcgtacaggttctgcaattcgcggagggaaaacttgcggggcaacaggttaaaaccgataggctgcaccagcacctgctgcttcagccgctcatggcaggtatccaggatctgcttatgatcaaaggccatttcacgcagttcctttacactgtgccaatgcaattcgttattactcatcttcaattccacatgctcaatattcaccagtgaatagtaggccacggtaatcaccctgcctgcgggatgacgctccaccgccccaaaggtttgcacctgctccatgtatacgttatccagcccggtgcgcgccttcagcacccggtaagctgcttcatccagctcttcctccggccgtacaatatcgcccagcaacgaccacttacccttaaactctttgagatcagattctatcaacagtaccttcaactcgtcgttgttgaacccgaaaatgacgcagtcgacagaaatagctaccttgaaataatcctttatttcaacaaggtgcgtgttgatgttcttggtgtacatagacatcataaagacgtggaattacagtaaaactcagtttatcaataacacgcggaactatatccaaatgaaagaaaaaaatatcacatttaaaacaaaagtgcccggatttttttcaacagatatctctaacctgaaagataagtttaaatttacggctcagttatatcaattatgtacacaaaggagatagaaataaccctgacgcagctggccaaacaactgctcagccatttaaagcaggaacaactgctgcaatccattgatgaaaccctggatgcccttcgccgtgtaatcagctataacgactggcgttactacgtggaaagtgaacccgtgatcagcgactatgaatacgaccagttgtatgcctggctgaaaaaactcgaactggaaaatcctgacctcgttacatccgactcccccacccagcgggtagcacaaggcctcaccaaagaattcattacggtacctcacctggtacccatgctcagcctcgaaaactcctacaatgcagacgacctgctggactgggaccgtaaagctcgtgaaagcgcccgccttaccgaaattgaatattgcgttgaacccaagttcgatggcgccagtatttcactcatttatgaagacgaccggctgacacgtggcgccacccgcggcgatggcgtagcaggagaagacatcaccaccaatatcaaacagatccgctccatcccgttgtctgcctccttctcaaaatatggcattcaccagatagaaatacgcggggaagtactcattaataaaaacactttcaaagcctttaacgataaacgtattgctgacaacctccccccgctggccaacccgcgcaatgcggcctccggctcactgcggatggtagatcccaatgaagtggccaaacgcggactggaagccttcctgtatcacatgagctatcataacatgaataccgggaaaacagaaccggatgcgctcaaaacacatagcggcacactggaactgttatctacactcggtttccgcagtcctgccaaagaaaagaaagtgataaaaggcatacaaggtgttatcgactacgtattaaaatttgaaaccgaacgggataacctgccttatgaaatagatggcatggtgatcaaagtaaatgactatgacctgcaggacaggctgggcatgaccacccatcacccgcgttgggccatcgcctataaatttaaagcacggcaggccaccagtaagctccgcagcgtggagttccaggtaggccgtaccggctctgttactcccgtggcaaaaattgaccccgtacccattggtggggtaaccgttggatctatttcccttttcaatgaggaagtaattaaagagaaagatctcaaactcggggataccgtgctggtagaaagagccggagacgtaattccttacatcgtgaagtccgtagccgacctgcgcgacggcagcgaacaggaaatcattttccctacccgctgccccgtatgtcatgataaactcgtaaagccggaaggggaagccgtttggcgctgcaccaatatcaactgcgaagcacaggtggtagaaagaatgatccactttgtgagcaaagacgccatggatattaaaagcttcggcgaaagtaatgtgcgcaaattctttttattaggactcctgaaagatatacccggtatttatgaattggattttgagaagataggcgcgctggaaggctttggtaaaaaatcactgaccaacctccaatccgctattgagcaatccaaaacacagccgctgcaccgcctgatattcgggctcggcatccggtacgttggagaaacaaccgctaaaacactggccaatgcagtgaaccatatcatggacctccaaaactggacagaagaacagatcctggcgctggaagatataggacctaaagtagcaggctccatccggttgttcttcgccaacaatgataacatcgaaatgctgaacaggctggcagcgttgggtatcagcatgaccaatactaaaaaggaagcgcatgcgccgggtcacctcaacggacaaacgtttttgtttaccggcacccttcataagctgaaacgcaccgaggcagaggaaatggtagaacaggaaggcggtaaaatagtgagcggcgtgagcagcaaactcaactacctggtagtaggcgatgatgccggcagtaaactggaaaaggccaagaaaattaatactattaagatcctgtcggaagatgagttcctggcaatgatcaacaaataattatcagcctttggttgctttgcaattaaaggctgaataccaacagcggttatgacagacgaacattttatgcggcaggcgatgcaggaagcacgcaaagcctttgaagacggagaagtgcctattggcgccgtagtggtattaaacaaccgcattattggccgtggctataatcatgtagaaagattgaacgactgtaccgcgcacgcagaaatgattgcgttaacagctgcgttcaatacgctcggcagtaagtacctgatggaagctactttatatgtaaccgtagaaccttgcctgatgtgtgcgggagcactgtattggagtaagataggcaggattgtttatgcagcggcagatgacaagaacagctaccggagagccaccggtgaccggtccccgtttcatcccaaaacaaaactggaggccggcccgtgcagcgaagaaagtttacagctgatgaaaaccttctttgaacaaaggagataattattttttggtggaatccatcagcttattcatacccatcatttgtttcatggtatgatccatcccttcggaagaaccatccaggaagatgacgtttccttttgagttttcagcaaagtgcttaatggcttcggtccacatggagaagaggatcacagaggtatccaggttggcctgctgcatttctttggcggccatactcatacccttggctacttcttcacggaacagggccacacccataccacgcagctgggcagcctggcgctcagcttctgctgcaattttaatagcattaccatctgcttccgctgctttggttttagtgatcagtaatgcctgaccttcattttcagcagccgctttcaggttattggaagccactacctgcgccatcgacttcatgatcacttcatcaaaagtgatatcattcatctgcagatccaacaggtggaaaccccattcttccagggttttgtcgatctgttcttttacgtgttccgtaatatctttacgcagacctaatacctccgcctgtcttttagtagccacaaatccacggatagagccttcaatggtgcgtaccagcgcctgcatgaagcttctttcatccataaatttgaacgccacgttcttcagcgtttcttcttcctggttccatacggcatacagcagcatggctttaaagtacacattcgcctggtcaatggtgatagcctggaattccagttccacagacctgttctggatggatacccttttaaataccttttcaatgatgggtattttccagttcagcccgggaaaaagtacccggttgtatttcccgaatatagtggtaacagcaatgtttccctgctgcaccgttacaaacgatgatagtatgacgactaaagccagtactatcaaaacgatcaagataacattcatagaatgattgtttaggtagggtttaggctggtaaatataatgaattaaagccaacggcagatgtggacgaaaactgcgattagtcgcagtctctatattctttgttttcttctgaaatatataaatacgtcgtccagctctatttgtttcaactggtacgccaaccgcgttctcaggtcctcggtttcatcttttatccttctgtattgatctttaaggatttcgtagcgggcaacaatttcttctgcagtggcagagtcctccagttgtaagatgtcaaatgctctttcctcggttatcatagtagttataggggtgtttcagatagtaatcatcccggatgtttaaaaacatacgtaatatttaatccactaaattagtcgagtttgaaaaacgagcaaatacccaatgttgggtatttttattcaaatcctatcttacgggcaatggccaccaattctgaggtgttacgtactttcagtttcagccggatatttttccggtgggtttccactgtataacggctaaggttcaacgattgggctatttccttgttgttcagtccttttacggccatccccaacacatctttctcccgtggggtcagtttgttgaaaagggtttcattttgccggcgcataatagcagccagcgcttcagacagttgggcattggtatcaacagcattggtaagatccaggaaggcacagatgatttccaccacccttccgtttttatcgtgcgtaaacggcacttccagcccaagcaaccaccggtaatcaatttctccttttttgcggatgcgggccagtcccccaaattgtgccttgttattaataaacgattgctgcgctaccgcagccagcttaaagtcgtcaggatgcatgatgtgccggaaaaattcaatgcccatacccgtcatctcatcagcagaaaaaccaacggtttctgcgagacggtcgttgcaccacgtcacagatttattattgttatcgtaactgtaaatcatggcgggtacatgatgtaaaacgctctccaaccaatggatacgattttttaaatgctcattttccttctgtaaggcattgagggaaaaatgtagccccgagtccgagcctgtctgcatactataagttttaaacaaacaataggtaaacaactgccaggcgcatctgaaaaaatatgcctgacgttacgttctgttaaaccgagtatccgtaaatataaaataattttccatatgatcaagccctggcgttgattgatttcgcctaattaacaaggttgcccgttgatcactaaaccggttatctcattaacttaataattaaatgtctaaattttaacggattggcagtaaatttggcgactatcaagaaatcatattttaaaacccataaaactttgagttatggcatttacacttccgagcttaccctacgcaccagacgcgttagagccgaatttcgataaactgacaatggaaattcatcatggtaagcaccaccaggcttatgtagacaatctgaacaaagcagtagcaggcacagaaaacgagaacaaatcgctggaagaactggtagctaatgccggtaaaatcagcccggctgtaagaaacaatggcggtggtcactggaatcacagtttcttctggaccagcctggcgccaaatgccggcggcgctccaaccggtaaactggcagatgctatcaacagcacttttggttcttttgaagccttccaggaaaaattcaacaccgccggcgctacccgcttcggctccggttgggcatggttaaccgtaaaagatggtaaactggaagtttcttccacccctaaccaggacaatccactgatggatgttgctgaagtaaaaggcacacctatcctcggtgtagacgtatgggaacatgcttactacctgaaataccagaaccgccgtccggaatacctgaaagcattctggaatgtggtagactggaacgccatcagcaaacgctacgaagcagctgtataagctatcaccagttcatggaactgcataaaaaaatcccgtcaggtaaaccttgacgggattttttatatgcttgaccaattgtttatagttccctgatctttaaatttttgaaccatatttcgctgccgtggtcctgcaatgcgatatggccttttttagacatcccgtagcctttggcatccttccatttgccgtcctccttgtgcttcttccattcaggcgtccacagttcgtaatcggccgttttctttccattcagccaatgctctacatgacccttgtttacaatgatcttggtaatgttccattcgccgatgggattcgcagcatctgccaaaggaggattcatggcataattggcgcctgttttctgccagggctccagcttctccgggaaatttttatcatcaatgatctggtattccggcccactcaactgaggcgtttcaaattcttccgataccatatacatgatgccgctgttgccttgcggcgacagcttccagtcggccgtcagctcaaaattctcaaactgcttatctgtgatcaggttcccccgtttatcagacttgtctgttttattacccaggcaatgcaggatccctttctccgctacccaggagtcggccggtttatttttgtaagtccgccagccctccattgtatggccgttaaataacagttgccagcctgctgccttttctgcttcacttaacacagctcccgtagaatctgcaagcgcagtgcttacaagagaatccgccaccgcaatggcattcttgttctcgttatttaccgtattacctccgcaagacgccaccacaatagttatcacggacaacgcaggaaccaaaaggtgcttcatatgtacgcgtgtttaattacttgttcactactttcagattcttaggatcccagtggatgatcttattatcgaaatagctttcgttgcacaacagcgccggcgccgctgcacggaaaccgaatgtaggatcttccgctactttaccgttggtacgcatggcgttaaacaggttgtagaagtgatcgaagtgcgctcctttgtatcctttctctgcctcatagatcatcttttcaggatccagcatgttcgcacggtgataggcatacgattttccgttattggatgcagcagcattggcagcagccagcggatcgttttcatctacctgtacattattgcggaacagcgttaccttatcccattctacggtcatagagccctcactgcccaccatgcgcaggtagttggtgccaccggtaccatccacgaagttcacgcggagcgacaggttaaacgcagggtgtatttctgtttcaggataatcaaacatgcccagcataatatcgggtacttccctgccatctttccagtaacgtaatccgccggtggccattactttattgggaccgagtgaaccggttaccaggtgaagactggaaaacaggtgaacgaacaggtcgccggaaacgccggtgccataatctttataattacgccagcggaagaaacgcaatgggtcaaaatcgcgcttaggcgcgtttttgaggtaagtggtccaatcaactgttttagtggaggcatccgcaggaatagggtattgccatgcgccggtgggcgacatacgtgcccagaagccttcggcataattaagtttaccgatagcgccatctttcaggagctgcctggctttttcattacccagggaactcataccctggctacctacctggtatactacttttccgttgcgttgctgggcttccactactgcgggtccttcgctgatatcatgtaccattggtttttcgcaatacacggatttgcctttattcatggctgccacggaaatatctttatgccagaaatccggcacagcgatgatcacggcatcaatgtcttttctctccaggatttcctggtaactgcgggtagtgtaaatatcattcccccatttcttttttgcatctgccaaacggccatcatacaaatcacaggcggctatcagctttacaccgggcacggtgattgccgtattggcatctgctgttcccataccacccgcgcctatcagcgctatctgtatctggtcgtttgcactgtatttttctttcaggcgggaaagtgactgaatgtttctttgcttatcagctgcggtcaggatacttggcagcagcgatgctcctactactcctttggcaaatttactgatgaaactccggcgagagtcttcattggaatttactggcatgataacccttttagattgagaaatgatataagtttattattcactggactctcaaaatataattattctaccggaattcataatttatatgagaattggaaaaggaggaataatgaagcctgcaaacaaactccggtgacaaccggggcttatttgcaggcttcattattaccagggctaaaagcggttacttcgctgcggtaagcagctgcttatattttgatgggctatgtaataaatcgatggcggcatttacatcattatcccactcgagcgacctgataatacggcctctctgcaaataataacggttcacgatttcttcttccagtaaccgttttatttctgttttatttttcagcagatcctgctttttatcgtgcttcattttcgtttcaagcgtttccagttctttagcgatcgcatcatagtacttttcttttcttgcggtgcttttgaaagaatccagggcttcttcactgcgtgttttgtagctgtaatctttgttatcgagatagcgctcaaaatcttcgaagtcgctttcagacagtgcaaaagagcctgcagcggctattttaggatggctgtagtaataattggtagcgtagtcgaaaataaattgtttacggataagggtaatggccacctggctgatataggtgggatcgacctttgcatcgggttcaataccgccgccatcttttacggcacggccgcctgtggtggtaaatgatttacgcagggaatccggtacataatccacgctgccgtcgtcgttacggtgggagtagtcgatggcctggatacagcggccacttggcgtataatatttagcggtggttactttcagtttggtgttgtaaggcagctggcgggtggtttgcaccaggcctttgccgtaggagcgttgtcctatcaccaggccgcggtcgaggtcctgtatgctgccggccactatttcggcagcagaagcggaggagtggttggtgagcacggttaacgggagatgcaggtctaccggctgttcggatgtttcgtagttgcggtcccagttctttacttttcctttggtgctgacgatgagtttatttttatctacaaaaatgttggcaactacaacggcttcatccaataatccgccggggttgccgcgcaggtcgaggatcaatcctttcagcgcggggttggtttgtttcagttgttgtactgccgtgcgtaccatggcgccgctgttctctgtgaactgggtcattttgatatagccgatatcatttttcaggatgccggcatagctcaccgcttttacattaatttcttcgcggatgatttttttcggggtttccacgccggttaccgggttgcggaacaccatatccaacggggtaccggcagcgcctttaagctgtctgctgatttcttcctgggctacatttttactggacttgccatccatgctcacgatgatatcgcctggtttcacgccggccctgtccatcgggctgccttcatatacatcggtgatggcggtccattcgccgctggtattgatggaggcgcctaccccgccgtatttgccggtagccatgaatttaagatcgtccaggttttcttcggaaacgaaatcagtaaaaggatcggtttcctccagcatggcttcaatgccttttcgcatcaccttttcaggaggaaggtcatctacgtaatacgtattcagttcccggtagaaagcggcgaatatgtccaggtttttggcaatctggaaatatttatcgttttcattgaaagcgaagatccctgctgtagtaataaccaggagcagggctgctgtcagtttccttcttttattaaaaaacgcacgcatgcaacgagtgtataagatgaaagatattagttggcaaccggtggtgactatttatggcaccggatcatatccgtgtccaccccaggggtgacacgacaagatacgctttatggtgagatagccacctttgaaagggccatattttttaaatgcttccagcccgtattgtgagcaggtaggggtataacggcatttactgcccaggaggggcgagataaaccattgataaatttttatcaggaagataaaaggaaaactaagccagcgcacaacacgattcataagcagcttttagcagtaaaaaataagcagagcatttaacagcatgttgaatgccgggtttgctgcaatcagctaaaagctaaccactgagtgctaaatactggtttgcagcttctttaaaattaccgaaattttgtctttcagggtagaaaaaccggcgatttttttgtcggtgtagatgaggaaaacggcgatctgccttgattcggaccggagatggtcgtagagttcctgcttttgcaggcgccaggcctcccggcccaggcgtttgatgcggttacggtccaccgcatggggaaaccggcgggtagcggcgctaaagcctacctgcacggggtatttacccggttctttcaacggcatgtaaacaacccggtagggaaaaacagaaaacgcttttccttcacgaaaaagcgtttcaataagttttctgctttttaacctttcttcctttgtaaaagaataagtttttatggcaaatagtatttagctactataattatttcagcttacgctcgtcagaaacagtcagcttcttacgaccttttgctctacgggaagccaataccttacggccattagcagtttccattctctttctgaagccgtgaacgctctttctgcgtctgttatgcggttgaaaagtacgtttcatttcttttttttgtttttacctgtactatactaaaactcccgtgttaaaggattgtggtttttaaaacggaaggcaaaggtagcagaaaatatttgaaaagtaaaattaaaatacgaattcttaaatgtaaaggtggaatgcagttttcaccacattccacctttaagtattaaatttattaactatttaactcccagtttagtctttacagcagtcaggatatcgtctgcagcaggagaaaccagcagcataccggcagagctgtcgattacgtagttgtaacctttttcctttgctacatcttcaattgccttacgggctttatcgtagatgggtttcagcagctcctgttgtttagcctgtactttctgttcagcgccttcacggtagtcctggatacgtttctgtgcgtcctggatttcacggcctttgatttctttcatgttgtcggtcatagtggccgctttatcatcgaattccttcattttcttcgtatactcatctaccagtgctttaccatcaccttccagtccttgtgcaaaagtttgcagatcagtttctgcctttttagcttctggcatgcttgctaccagtgcctgtgcattgatatgcgctactttggattgtgccattgcattcacgctgaacaaaccggtaaccgccacaaaagcaataattacgtacttcttcatgatgttgtctgtgtttaaaaaaatttaaatacttatagttaaaaaataggtacgggtttatttcttgactcccaaagatttcaggatttcttcgcttttatccagctttggatcagagaatataacggtggcgcctgcagccttatccagtacaaaatcatacatcctgccggcagaaagcttctgcactgcattatagatcttatcctgaatgggctttaccagttcttccctttttttgaaaagatcaccttcgtaaccgaaacgcttcttctgcaaatcctttgcctctttttcccgggctacgatttcatcttcccgcttacgtttcaattcttctgtgagcattacctgttctgcctggtaagacttatacatcttatccacttcctggaacttagcgtcaatttccttctgccattgctctgcaactgcatccagctttttctgtgactccttgtattccggaatgctttccaggatatattttgtatctatcacgcaatagcgctgtgcacttgctgcaccgcccatagccagcacaatggcggctgtaataaataatttcttcatgctacaataatttttcgcaaaaccaaatgacggttaaacttgcaatatataattattttccacattattctggttcgaagccgagcataaatgtaaacttagcagcgtctttcaaaccaccccctggctggagacggtcaaacccgataccatagtcaaatccaagcaatccaaacatcggcaggtagaaacgcataccgatacctgcagaacggcgtaatctgaacgggttgtattcattcaggtctttataaccgttagctgcttccaggaacgccaaaccaaagatggtggagctgggattcaaactgaacggataccgcagttccatcacgtacttattaaatacggtgaagccggaatagttggcaggctgaccgttttcaggattgatgctcggatcggaagtataatacaccgggtaacctctctgggagatgatatcacggtcgtagatcgcgaagttactcaaaccatcaccccccatttcaaacctgccgaaaggcgacagggttgtacggttgttgtaacggccgatataaccaaatttcgcggctaccttcaatacaaatgttttgttatcgctacccatcggacggctcaaaggcacgtaccattctgcgttaaagcggtatttctggtactcgataaatttaaactgctcagaagccggctctttggagtaatccttgtcgggattaaacagggagtatggcggcgtatactgcgcagataccatgaagttggaaccactgcgcgggaagatctgctgatccacagaagaacgcgacaacgtcagcttgatgttaacgttattggacgtaccgctttcaaatccgggaataccaaagtagttatagttcttcagcttatactgctgatagttcacggaatagatcagggtgaaatagtcatccggccatttcagctgtttacccagtgatacagaggcgcccaatactttaaagtgaccatttgtagaagtagtggtatcacccggcagcttataataatcgttgtatgcgtatgggttctggtaactgctgtaaagacttacagaaaactggttcctttttttacctcccagccacggctccgtgaaggagaagttataggaacggtaagctttaccattggaagatacacgtacagacaatttctgtccgtcgccacttggcaatggatcccaggtttcttttttgaagatattacgcagggagaagttgttgaaggtaacgccgagggtaccggttaaaccgatataaccaccccaacctgccgacagttccagctggtcattggctttttcttccacggtataatcaatatccacggtaccatcctgtacgttcggcaccgggttcatgccgatcttttccgggttgaagaagccgaggttggcgatttcacggttagaacggatcagatcctggcggctgaatttttcacccgggatcgtgcgcagttcacggcggataacgtgttcattggttttttcgttaccggctatacgtacttccttgatggttgcctgcggtccttcacgtaaacggatttcgtaatcgatagtatcgccgcggataccaacttccaccgggtcaatctggaagaagaggtagccatagtccatgtagtagccgctgatatcgcccccttcctgtgacatttgtttaccgattcttttttccagcagttccaggttatagatatctccttttttgataccgagaatacgggtcagtacggagtcggaataacgggtatttcctttccaggtaatatccccgaaataatattttttaccctcagagatctgcatatccacattcagattctgtgagtgggttttataggtggtatctcttacaatcaccgcatcacgataacctttggagttatagagcccgatcactttacctttatcctcgaagtatttgttttcgttgaatttagcagagctgaacagtttaaagcggaaataagggtccagtttctcaaatgcgcgggtgggttgcaggaagccataggtttgccagaaatcatccggttgggccagggaatccacgtacacctgttccagatccggatgaagcgtgaagcgggaacgctctttggttcctttcatcttcttcttgatcttggagtcggctatactttcattacctacgatgttgatatcctggatacgtaccttactacctttggtaacattaaagatcaggtgtttggagtttacctggccggtatcccctctttcctcgattttaacggtagcatttccgaatcctttatctgcataaaatttatgtactaccccgattacgttttgtttcagggcctgtgtgatcacatttcctttacgtaaaccggctttggtggtaatatcgtctgcttctgtttttttgattcccctgaaaacgaaggaggacatgcggggcatttccgttaatcctatttccagccagattttattatcttctatcttggttacataaatggttacgtcggcaaacagtctttgtgaccagagactctggattgcctttgtaaactggtcaccgccgggataagtaaccttatcgcccacagtgaggccggaaagcgacagcagcagtgatttatccaggtattgggtaccggcaacggtgatatcggcaatttcatactgttgcggaatacctgtgttgataggagaaacggccggcggattagcagggggctgcgtaggaggcacggtatctttttgctgagcggatacacgaatgcctgcactgcaacataatgctatagccagaaggcccttaggaaataatttcttcattctgctgaatttgttcgcttgttttgccaaagcgccgttctctggtttggtaatttaagatggcttggtaaagatgttcattgcggaagtccggccagcgggtatctgtaaaatacagttccgcataggccagttgatatagtaggaagttactgatcctgcattctccactggtacgaatcattaattcagggtccggcaggccggcggtacagagatatttttcccatacctctggcgtcacagctaccgggtccagggctccacttttcacatccagggctattttcctggctgcattcacgatttcccaccttgcactgtagctaagagccataatgagattgaggccggtattttggctggtaagggcaatggcctcctccatttcccgctggcattggggaggtaacattcccatgtcacctattacgctcagccggatattatttttcgataacgtattcacttccatacggatagtgtttacgagtagttccataatgccattaacttcataaaccgggcggtcccagttttcagtagaaaacgcgtatagggtcagataacctattcccagttctgcacaggtcgtcactatattacgcacactttctaccccttcgtggtgcccgtacagcctgtcttgtccccgctcctttgcccaacggccgttcccgtccataataatggctatatggcgcggcaaccgttgtaagtccaatttttccttcaagctcatttgtgtcaggcgtattataacagattataacagatttactaaaagggtgcaaagatacaaaaatagagtaatgacttttttggcaaagcctaagaaggtgttttaacgtagttttaacagcgaattcaataccagtggggattttagcaaattgggaggcttatcagggcggttggcaggtacggaaagcccacccgcagaaagtattttttattgtaaattaaaatttacaattgtaagaagtgaaaagaatactaatggttaattcgattgttacgaactgatccttatccctgctgtttcctctttgcctccctatcaccccgataggactgcctttcacagccgacctgtcctgcaactgggccgccaccgtaggctgaccgtcaggaagcgccgggaatgcggcagggccggcatatgtagtgcttacatcatccaggtaatccgtttgagtgaaccggtatagcgcttccaggcccacatttacttttttggaaatattatatttaaaacctcccccgatcaaccaggcataagaaaccaggctatagggcttgcgctccggataaagggcggtaccctgcccttccgtacccaggggctgtaaaaaatatttgacgccgttaaggtaagcatatggattgtaataaaaaatactggcgccaccagtcagatagggggaaaaacgctcatataagctgcccggttcaaaccggaaaaaattaaagtccccctggagggacaactcccataaattagtattaaagctgaggttccggcggttctggaattcatttttattgtaggtatccgaatagccgagttgcataaaccggccatgggcgcggaggcccacgtagtcgttcatatatttacggtagtaaatgccaacagcaggcttcagggtatttaatgctccccgggtgttcagatccccgaaatactgtgcgcctcccacagaaaaacccaactctcccacatattccagctcattttgcgccgaagcacgttccgcgaacaaacaaccggccgataccagccatataaaaacgatgtatttggaatatagaaaaggtttcagcataaatcagttctacttaaacgctaaaatgccggatttatttaatgtatggctgatgattatgcttacttatttggcgtttgctttcctcacggggcataatttctattacaatcagcatggaatgtatttgtaaatataacaatatattttacatttctatattttaatcgtattccgggcgtcaattccccagagcaatttattccggagcgtatgcaggaaattgctgtcgtccagccggagcaggctcagtttgaactcctctttcttaatagccagctgcacccggttatcgatggtttccatacggctgtcgagggtacaaaggaactggtcgctgcggccttccacttcaaaggaaatgatattattgttgggcacaatgatgggccgtacgttcaggttatgcggcgccacaggcgtaatcacgaagttgccggcgtccgggaacacaatgggaccgccgcagctcagggaataaccggtggagccggtgggggtggctacaattaatccatcggcccagtaagtgttcaggaattcgccgttcaggtaagtatgtattttcaccatcgcggaagtatccttcttatggatggtgaattcgttgagtgcgtatggaacatcaccaaataaggggatgttggcatccaggtgaagcagcgaccgctggtctaccacgtaggtgcggttcagcagcgcctccaccagtgcatggatctcgtttttaccgatgctggccaggaacccgaggcggccaaaattgatccctattaccgggatgttggtatcacgcacataacaaacggtatccagcagggtaccgtctccaccaagacttaccaggaagtcgatttttcccgggaggtcttccgcacaggaaaacagcgttggtacgttatcgaaaggaatgtgttgctgcagcgtatgaaaaaaaggttcatagatgatggcctctatctctgcccgctttaattcctccagcaataagcggatgtttgaaatatcttctgtaataaatcccctgctataaagtgctacctgcataatttttaagcttttaacgatcggctctgaagtgctacatatccacgctcgtgtgtaaaaatagtcctttttgccctaactggttaaagctgtattcaatcctgaggcaggtatcatagaaggaaacgatgtccagtcctatgccgccggtatacaggaaacggttattcaggaagctgttgccggggaatttattgtaggcgtaaccggcgtcgccaaaggctttggcgaagatgcgcaccggaacggtattaaatttctttggaacaataggcaactttactttaaaggaaaggagttcctgccggagggttgatttcaggatggcgaagctggtgccatctatcacgtaatattccagtccgcgcaggtaatcatcccggtaacccagcgcctgctgattgatatatggctgttcattggagagcttggccgcgctgcggatacctaatgcagcataggttttgggccgtagctgccagtatttggccatgttaagccgaaagtgaacgtcatccacatcattgagaggacctattccctttttgccaacttctgccagtaaccggaatcctttgagaggatatacccagctatctgccttaatataagtgagacggtaggtgatatctatgtaacgtacattggtgcggcctttcccaaggtagttggggttgatgatagccaccgaatccgccactttttcataattataatttacaaatacctggtgccgggtgttaatggccttacggtagctgtagttaagcccgatcatatatacctggcgcagaaaatcatctttccggaaaaactgctgtttattattgctggtgctgtcgttcacctcacggttacggttataggaggcgatgatacccaggccgtgacggaaacgtttatcgatatacggtatattatactgtaatgcgaatcgctgggtatagccgaactgcagcgcggcgttcagcgcatcattgcggccggtgaggttttcctgggtaccgcttacaccgaggttgatacggctaaggctatggttcttttccacccaccactggttaaagttacggtctgccagcttgaaaatgggataagcgaaggtgtaccagcgttcccatacttcaaataccacgtcggcttcgttaccggtccagtttttcacattggcggtaacgttgagaaagagggaggtattgagtaattgttttcgtctttcttccagggtattggagagatcgcggagatagatggtatctccgggtacagtgcttatttcccggagaatgatggaggtccgggttttcttgttaccggaaaccaggatgttgcgcactaccaggtagttggtatccgttgcaggcgccgactgtccttccgcattttccggtatcaccattccaaacaggcagactaaggccagcaggtagtaacagcatctcagcatgtaggtccctaaaacattttaaaagttgacaatagcgcggattttgtctttactcaggattacgctgattataatattgatttaaaggatttgaacctttttgatttttttgattttaaaagataaaagcaattcaccttttgtttttttgattttgagtgataaaatcagaaaaatcaaaaaggttcaaatcctttaaatcaatattataatcagcgtaatcctgagtaaagacaaaatccgcttacatgccgatataattcatcagcaggtcgtagtttttcttcagcagctcttcttccggttcttccgcaaagatgtatttgattacataattaaagcgttcgaaagtagctaccagaccttgcagttcctgccggtttgttttgagtaccacctcgagtttaccggtaacggggttggtgatggtgtttacgctcaggagcgtaacatcatttgattcagcgatacgggcaatttcgctgagagcgtaatcgcgcgggtctacttcaaacgcgatgataccgccgggttcctttaccccgttatatcttgctaaagctgccagcaggttatctttggtaatgataccgaggtattcattttcctttgttactaccgggagggcagacaatttaaagtcgtaaaaaagtttgagtgcttcgaatagatgagcgtattccatgacagccgggcgggtactgctgtactccatagattccaggggtacatccggatcttcgagatccatgatatcgtcttcttccaccagggccaggtatttgctatctactaccatcgggagctgcgtgagatgatattcgttcatcaggcgcagtgcctttgttcctgaatccgagggatgcagaacaggtactgaagatatgagttctctggcgatcatgttagcgtattctgatacaataatagtaaagaatatgccaacagaaaaagaaattacatgtacgcgaaatcgctgcaccggttggtacagtcgtcgggctgccggtaaagtgccggtttaagtggcaggttgaaacttcagtttctccaggaaagcgtgcagaattttgttgaattcttccggcacctccatcattggagcgtgtccgcatttatcaataaactgcagttcagaattaggtatcagctttttaaattcttcgcccaccataggaggagtaacggtatcgttctggccccagatcagtaaggttggttgctggatatctttcagttcatctcccaggttgtggcggatggctgattttgccagcgtaatgatcttgatcactttcaggcggttgttcactatctcaaacatttcatctaccagttctttggtagctattttcggatcatagaaagtaagttctgcttttttgcggatgtattcatagtcgccgcgtttaggataggtttcgcccattccattctcaaacaagccggagctgccggttaggatcagggattttacgggtgcttcagggtgttttaacaggtatacgatggctacgtgacctccgagtgaattgcccagcaggtgtacatttttgtaccccctggcttcaataaacttgtgcacatatttggccaaaccgcctaccgatgtttccaggatgtttaaatcgtacaggggtaacatcgggatcacaaccttgttatactgccggaaatattcgatcatgtgcgagaaattgctcaaagcaccaaaaagtccatgcaataataccagtggttctccttctccttcttctataaaattaaacttaccctgtgttttgatttcgtaatccattgccaaatcttgaaagtcaattttacgctaaaataattctttttattaatctaaataatctttggaacgagttatccaggttgaatatgccgggctgcctgctcaaaaaaagactgtaactcggtgaacatattcttaaaaaccgggatcacacttcccatatgatccaatacccacgggccaatattctctatataaggatataccacagattgcagctttgtttcaggactcagccagtatacctggttagccatccacagcactacactgtaaattattataaatataacgctatacaacagtattccgcccagtttattcagccagcccaacattaccagctccaccaacttctgcaaagctcctgctcccaacctcacgagcaatattactcccaggaaaaggcacacgaaacagattacaggcacccagcgggaatgcatatcccagtgttcctgtacatataatgcagtaatggctgttaatttcagggctgccgctaatcccaatatggcggctaccaaagaaaataaggctactatcagaccccgggtgtatccccggtagatggcaaaaaccatgatgatagcaaaaataatgtctataggcatggttgaaatatagggaatccggtatttaactcgctgatttttttgtttccgggagatgttatctgcccggtttccgcttatcagccggttaaataccagacagcactatttagtaagcaattctttcaccagggcggaaattgccttcccatcagctttaccggccagttgtttggtggcaacgcccattactttacccatatcagcgggtgagctggcgccggtggaagcgatgatatcagtaatggctgtacgtaattctgcttcatccatttgtttaggcaggaagcgttcaatcaccaccagttcctcttcttctttcacggcaaggtcttcacggttctgggcgcggaaaatttcaagagaatcctttctttgcttggcgagcttctgcaacaatttggactcatccgcttctgtgagctctccgctggcgccttctgctgttttggccaccaggatagccgctttgatagcacgcagcgcacgcaggtcagcttcctttttacccagcatcgcagctttgatttctgcgttgatatttagttctaatgacatatggttaggtttaatggattattttcctgcttcttcggcagcctgcctgtcctggaatttcttaaagaaatcctttgcaaaagcgcgcatgtcgtctgcctggtctttataaggagtggctcttccgtaagtgtcagccatggtcatcatggtctggaaaaagaagtccgccatttcatccaccatcatgtcctttgtccacaggtcgatgcgcagcgccaccttttcagccggatcccagaaagatacgatcatgcccttggccttaatcattctttcttccttgttatctgtagcgctccactctatcgactcgggcaccttttgatcatccagtccaacctggatctttatggtagatactttactcatgattttcaattaaagcgcaaaaatagccatcatttgctgattttggaaaaacccgtcccggtgagatgactccacagctgctccgcagcatgctcccagctgctgaaaggctttgccgcagggatcttggccagcaaacgggatcttaattgttcatctttatataaaagactcattttttctgataaatcgtccaaactcgccggatcagcatataataccgcgtctccacctgcctccctggcggcagcgccgtccagcgcaatcaccggcacctcacaccgctgcgccgcgtataccggcaatgcaagcccttccaacctcgacggatatacgagggcataagcgcccccggtgagccgggcaagggtatcttcatcggcatcttctatgcacaccacatcctgccggaacttgtagctctgcagggccgtggcaatatccgctcccgccggggttacactccccgccagcaccagcttgatattgctccgctgccgcttcttcaatgctgaaaaagctttcagcaccggtataatattgttccggggatgcatactgcctgttaccaggaaatactccgccccaccggaaaaagcccgcttcaccgtttcgcgctgctcccactccaggggtttgtactgctcactgataccggtttccaggcggatcagcttatcttttacgcccggtgcataacgcagcagttcttcctgtgcggcatcagacagcacggctatacgccgcgcccggtcgaggtatttcgtaatgttatttttaagcgaccgctgttgcacacctggctgcaggccggcattgcgcaaaaacgaaaggtctctcagcaacagtcccgcaggaattttgctacgcaggggcagcgtgccatccagccccaggaacaggtccgggcggaaaggcttcatggcccgtacctgctgccactcctgccaccagtacaaatgccagggtttattgcctttcaggggcaacaccacgttggtcacattggccggtactttcaggccggcgggtacctttccgtcaaaaaaaaatgtgaactgatggcctggctgctgccggcacatcgccagtattatctccgttgccacattcccggtatcggcaggcatgtcctgtcgtaaacaagcggcattaacagcaatttgcataaacgattcctttgtctgcgagcttgcaaacctacacaattttagattcgggactgccggattttaatgacccggctattctccggacttattggtaaggaaaaatacctgcggaggagttacattgccggtattacccagggacgccagcctgacagttacctcgtatgttttcaacggcttcaggtgacggagcgtaatggtaaagggggttgctttaatatctgctatatcgtcctggggcagcggaataagccccgtttctgtggctacgttcagcgtaactttcacgcctttatcaggcaacttgctggtgatgttcaccttcagggcataggtgctgtcctgcgccatattatattttcccacctgtacttcaggcagcgcgaaagccagtgtttcttcctgcgtactgggtgcaggattatctttcttcttctttttacaggaagaaaaagtaagcaatgcaatagctaagaaggcagggagaaaggttttcaataacatatttccagttatataggagcatgaaattagctttttttaatatgcaaatcaaattttacttcttacatccagcgcatcccgtaatccgttacctaacaggttgaaagccagtaccagtagcatgatggccactccgggcgccaacgccagtaaaggattatgggtgatgatgaagttgtagttttctttgatcatcagtccccacgacggctgcggcggttgtacccccacgcccaggaagctgagtcccgcctccaccacaatagcggtggcaaaattgccggcggctactaccatcaccggtcccatgatattgggcaaaatatgttttactataatccgcacatgcccgtagcccagcgccctcgcggcttccacatattccagctcccggatacccagtacctgcccacggataatgcgggcaacgcccacccacatcgtgagccccacggcaataaacacctgccagaatcccttgcccagcgccagggtaagcgcaaacaccagcagcagcgtaggcatggaccataccacgtttaccagccacatcaccaaatcatccgtccggcccttgaagtaacccgctatggcgcccagcaatacgccgatgctcagcgaaataactacggcaatacaacctacacctaagctcacgcgggtgccaatcagcagccggctcaggatatctctgccaaatttgtcggtgcccagccagtaagtgcgggagaaaatccgttctgccaatatcttttcatgtaacgatttcgatgacatcgggcggtccggcggatggccgtaccacacctgctccagggagtaggtttcctccctgctggtagattcatccacgtaccgttgtaccaccagcacgctgtccctgaattgccacgaccggacggggatccagtttacatcagactcctggccgtataacaaccggtgaaaaacagacaccttttggatgggctgttctttccgcatggccagcatattgatgcggaagccggggtgctgcccctctatttccagcaccatcctgttggcgttgggtgtatgatccggcgcaataaaataagcggttatgctgataaacaccgccacggcaatcaccagtaaaccggctaccgcacctttattccggtataactttttccaataaggctgcatatctgacaaaagaaccaggatttaatttacctgccggcctttccactgataactgccaaacttcccaagccacccggcaacaacaatataaggaatatgaaatatctgtcccggaataaaccatagcaagagttctgttttattaaaaaacctggctacaggaagcaggaaataaagttccagggttattttaaacagtaaaatgatgaggaaccagggccaccataccggcaggaacagggccattaccgccagcgccagtaagccggcattgaacaggtaaaccagcagtaatacccaggtcagtcgtttatcttcatacttatctgctttcgatgaccaccggatccgctggttcataaagtccctgagcgtatctaccgcgagtgtacgcactacagcttcttcacacttcaggtagctgaccttatcggggtatgcgctgtaaattttgtacatcagcagcatatcgtcgccggaggcaatattatcgatgccattaaaaccgcccacttccaggaaggcctttttttcataggccaggttagcaccgttacacatggtaccggaggccagttgggctgcagcgccggtaatgccctgcatggtcatgaaatcgagcgactgtaaccgcttaaaaaaattatgttctttatagaagctgactggtgcggctataaatttaggttgatgatgttcgtaaaactgcaccagtgtttcaatccagcgcggccccattacgcaatcagcgtctgtggttacaataaggtcgcccgcagcttttgaaatagcaatttctattgctttcttcttgaaagaattcagccgctcctcttcattgagatactgctttaactccagcaggtgaatatttgctgctgcgaaattgcgcaccactgcggctgtttcatctgtagaaaaatcatctattacaatcacttccagtaaggccgggttgtacgtttgcttcttcaatgcctccagcaaggcgggcaaattggcggcttcattcctggcaggaatgatcacggtaaccgcagtatgaccaaccgatggcgctgccggtgaaaaactcttcaggcgcttccagcccaggctataccataacatcagtataccatatcctaaagccagcaccaataatataattacaaaaagatacatccgggttaaaggtttgttttgatgataagccccagctgggcggaaatcaactggtggcctttttccattaccagtattttgcagggaaaagacccatctgcaaagcgggtacccagcacaggtggaattacacggtcgtatttcccgaatatcaggagtgttaaaacgttatatctgcctaataattgtttacaccgctttttatccggcatcatccggcgtaaattggtccatacgttgtataccagttcccttttctccgtttcattcatacggtgcagcgcaaatttgtatacgctctggttcagcagtcctagtcttctccaggtatgcaataacgtaaaaaacagccttgggtggtaagtattatatttaaacagcctgtttccggcagtggtttgggttacaaacatatgccaggggttatttctcaggccatccccggcggcgatgaccaggtggttgatccggctggccatcttttccacgaggcaaagcgacaggcgtccgcccatgctgtagcccagcagggaaaaacgctccttcccgtgctgctgtagtatcagttccaccaacgctaccaggtcgtctttctccagcacccggttttcctcccattgggtgcttccgtgcaggggcatgtccagcgccactaaagtgaaagtatcgcccaatgtggcggttaacggctgaaaatgagccgcactttcgccaaacccgtgtaaacagatcaatagttcctccccggcaccttctacggtgccatgaaaccggcttttcaaatatgacagataaaaatcaggcataaagggcaacaatgatacagaataaatgcctaatgacgatggatatgattatcgagggggcggtgacctgtggataagggagcatatcttcaaccaggaccaggtaatctaccccgggcaggtctatttattttttgttaaaaatagcggcctctcaacaggagtgccgcatttaacttacattcagtaagttaatatggcaggtagcagggaaatcagtttagccccccggtgaccggttttgcctaatgcttttttcagtaaattacagaactaccaaaaatacagtaacatggacgcaacagttgaaaataagactgcgttaaaaggcgcagagttcctggttaaggagagtgctcctgaggaagtgtttactcccgaagatttttcggaagagcagctgatgattaaagacatggcagatcagttcatcagtaaggaaataacaccgatagtagagcggatagataagctggaagaaggattgatgccctcattgctggaaaaagcgggcgagcagggactgctgggcgcttccttcccggaggagtatggtggtttaggtaaagattttgtgacagcaacgatcatcaacgagggactgggtgcaggtcactctttctccgttgccatggccgcccatacgggtattggctctttaccgatcctttattttggtaccgcagaacaaaaacaaaaatatatacccaagctggctaccggtgaaatgaaaggcgcttatgcccttacagagcctgattccggctccgatgcactgggcgctaaaaccaccgccaaattaaccgacgatggtaagtactatatcttaaacgggcaaaaaagctggatcaccaactccggtttcgctgacgtgtttactgtatttgcaaaaattgacggggataaattcaccgcttttattgtggacaaaggcacacccggatttacactgggtgcggaagaacacaaaatggggatcaaaggatcctctacccgccagatctatttccaggacgccaaagtaccggcagaaaatgtactgggcgtaattggcaagggccacctcattgccttcaacatcctgaacataggtcgcttgaaactttgtgcggccgcactgggcgcctccaaaaaatgtatcaatacctccgtacaatacgccaatacccgcacacagtttaaacaaccaatcgccaactttggcgccatcaaacataaactggcggaaatggctatccgcacctggacatcggaatcagccctgttccgtacagcgcagctgatcgatgacaaggaaagagaactgctggcagaaggcaagcctttcaacgaagccttactgggcgccgcggaagaatatgccgtggaatgcgccatcctgaaagtaaatggctccgaagtactggactatgtagtggatgaaggtgtacaaattcacggtggcaacggcttcagcgatgaatacatcatttcaaaagcttaccgcgattcccgcatcaaccgcatctttgaaggtaccaatgaaatcaaccggttgctgacactggacatgacactgaaacgtgccctgaaaggtaaactggacctgatgacaccggccatgaatgtaatgaaggagctgatgagcattcctgatttcggcaacgatgatgaaagtgccttcagcaaggaaaggaaaatgatcgttaacttcaaaaaagcaatcctgatggctgccggcgctgccgcgcagaagctgatggtgaagctggaaaacgaacaggaaatcctgatggatatcgccgatatggccattgaaacctttgtggctgaaagcgcgctgctgcgcttaattaaactcaccaacaacaaaggtgaaagcgccgcttccctgcaggcagatattgtacgcaccttcatttatgatgcggccgaccgtatcaataaatccggaaaagacgccatcaatgcctttgcagaaggcgacgaacaacgtatgatgctgttaggcctcaaacgctttaccaaggcagaaccatttaatgctaaagatgcccgcagaagaattgcggacaaactgattgcagataataaatacagctggtaacaaccagcgcctggcatttagaaaaaatacagcaggtacactatcccgctgcattttttctaaatgctttttttcctattcccctcacctgcttatctttaccatctttcaaagatattgatgacagggtatgacgctaacagcaaagtttttttctacgtttcttattactatttgtgtccccttttttgcaatcagtcaggcaacactgcgtatcagtcagccttcaagggatcagaataacgtgaacacctcccggcaatttatcgccggccgcacctgtaccggctgtacggtaaggatcaataacgatactgtacacgtttataacaccggcacctttgctgcaaaatatgaactgaccaccggcaggaattccttttccgttaccgctaccacacctaacggcgaaacatatacgaagaacatcacctattactataaccaaccgccagcaccggctgctactaccgttttccggatagattatatggagatatccccctccgggaatgttcaactctcggaaggcgacacgctgcggataaagatgaaaggttatcccggtcaaagcgccagctggttcaatgatgtaccactgaaggaaatgcctgtttcgcaaacaggtggcgtacctggcttttacagcggcagctatattatacaaccacgcgactccctgctgaatggaaaaattatggtacgcctccgcaaacaaagcggcgaaaccgctatcctcggcagcacctaccgctacagcgtgatgcacaatgaaataccattcaccggccgcacgatcgataatatgacctacctcactgccagtccgcatggcgaccggctggggcccgataaaatcggttacctcgataaagatgtgcttttacatattgtaggcagacagggcgactattacaaagtaaagctgtcgtcccgtaccaccgcctttattccggagccgctggtagacaccgacattccacaggaagagcttcccgtaagcattgcagacgatgccaaaatatggggagatgaaaaatatgattacgtgtcagtggccttgtcggataaaatgccatacacttccacgcaactggtttcttctaaaaagatcatcatcgatatacatggcgcctatgcagagaaaggattgaactccctgctgcaaaacaccaaagaaatcacgtctgtagcctgggggcagccatcgcccgatgtatgccgcatggtaatttccctgcaacatgcgccatggggctaccaggtgtactacgacaataaccgtataacggtgaaggttaaacgtgtaccacaaagcttatcgctgaaaaatatggtgatcggcctggacccaggccatggcggcagcaaccctggcgctaccggtcttaccggcgccgtggaaaaaaacatgaccctggtactttcgctgcaactgaaagctttgctggaaagagaaggcgctacagtgatcatgtcgcgcacaaccgagaaatttgttgccaacgaagaccgtttgtcttttttccgcagggccgatcccgatctgctgctgagtatccacctcaatgcttccggcaatcctgtagatgtatatggcaccgccacctattacaaacagcctttctgcgaaccactcaatgcagccatccatgagcgtttgctgcaaaccggcctttacgatttcggcaataactccggcttcaacttcatcctcaacaaccccaccgaattcccggacgccctggtagaaacacttttcctcagcaatcccggcgacgaagaaaaaatactgaaccctgcgtttcagcgggaactggtaactggcatcgtggaaggcgtgaaggactaccttcgcgaggcggtgaaaacgcggtgagcggtgagcggaggagcgccttcggcggtggaaattgtcttggctcaggattacgctgattaaccgtgattacactgatttgattatgttttgattttacttttctgattttacttttttgattttaatagattaagggagatataagcgaatatatccgcttatatctcccttaatctattaaaatcaaaagtgatcaaatcaagctaatcagtaaaatcagcgtaatcctgagccaagacaatttccgccgccgaaggcggcccatactaatgaatgttccctaagtaagccgacagccggttgatggctgctgccgccaccgttatttgttcctgggcttccttccagcggcgttgctcgatggcttctcttacgccgggaatggttttaacgccatagccggtataaaatccgggagcatacagggtatgtttataccagttgcgggcgggcaggccggcatcgttcagcagttgttgctcgccctggtacagcgctttgttggctgtggaggagagtttcctggtggcgagcgatgcggtaacggtgtctaaaccggtgagggcgttctgcaatggagaaaagtcgagatacggcacttctgttttgggaagtggaggcgacaaatgtttggcggtatctgtggtgagctggtatttacgatcgcggatcagttgattgtcgatggcagtagactcgcgcaggctgctggtgagttccgttaactcattcacatagccgttaactgtttcatagagtttgcggtaatcgaatggcagggtaacggtgttggctacacgcaaagcggtatgaccggcagtttgagaaagtgctacgccgtaattaaaaccggggtctttaaaccgggtataatcgtcgtaggaatcgtagatggagtggtattcaccgcctgcatcttctcccccaaaaccaaaatcaagagagggcacgcccaggtgctggaggaaggaagagtaatcggaaccggaacccatggccccgatagcgatgccttgtttggccagcttttcctttttcagcttgggagtagttgccttcaatacctctgccgcctgtttacgggcaaggatgctgacctgcgtttgcgggtcggtaatatcacgggctacttcattcacgagggtttccagggcatgggaaccgctggcattgagaaatccgcggccattgttatctgagttgatatacaccactgctttttctttcaattcggcagcgtgatcttccacccattcggtagacccgagtaagccgggttcttccccatcccaggcgcagtacaccagtgtgcgttttggctggtagccttgcttatgcagcgcgccgatggctttggcttcttccaggagggctgccagtccgctgatgggatcggcggcgccgttcacccacgcatcgtggtgattgccgcggatcacccattggtcgggttgctcactgcctttcagtttggcgatcacgttatagcaggggcgtatctgccagtcgaacgacagcttcaggtgtaccctggctttgccgccaccgatatgataagtaaacggcagtgcgcctttccattcgtccggtgctacgggaccttccagggcctgcagcagtggcgtggcatcgtggtagctgatgggcaataccggtattttcaggagattgggcgcctgcaggcgatcgagccgttgggcattggcggtagcgccggtgttaggggtaagcgggtcgccgggatagatgacgatatccatcacggagccgcgctgtacgccatactcatttttgaacgctcctttagggtatacatcgccgctgtagtagccatcatctttcggatcggagtagatgatgcagccggcggcgccgtgttcctgtgctactttcggcttgctgccgcgccaggagcggccgtatttggcgattacaattttaccttttacgctgatgcctgcccggtcgaggtactcgtaatcttccggtagaccgtaattcacgtataccagttccccttccacgtcgccatcggcgctccaggcgttataagtaggcaactggccttcctggccggaggtagcgtcttccttcagggcaggttctttcagcagtgctttataggtggtaggacctgtaagttccacgaggcgttctttgggagtgggaaaaagtacctggtaggtcactatttccgcgtcccagccgtaacttttgaagcgttgcaggatgtcttccgctactgctttgccgcgggcggagccaatgtgatgtggttgggaagagagtgctttgatagtttcaccaatgtgactgctgcttaactgcttatcgaagcggctttccagttccagctgctgggcggcggcgttcccggcatacccggtgagctttttatcctgcgcccgtgctgccccgcctgtgcacaatagcagtgctatgagcagggagaagttggttgttgtcataatttcgatccagatcttgttgaaaaagagggtttatctgctcaatatacaaatagtctattatatcaatagactaatttaacggatgtttttgatgcaataacttttggttatgatccataaatataggttataggccaaatagtctacttaaccggtagattaatctatatttgtaaatcctttcatagctttattgggtgaaacgataaacaaaacacataaacagcagttatatggccaatgcgattcaggagtttaacgactaccgggctaagatgaacgaggtaatacttggaaagcagaacaaagtgattaacaggcttttcaacctggacaccaatacctatgcagagggggcgctgagcaccaaaacgaaggaaatgcttggactggtggcttcaatggtactccgttgcgacgattgtatcaaatatcacctggagaaatcgtttcagcagggtgttaccaccgaagaaatgtatgaaatttttgcggtagccaatatagtaggtggcacgattgtgatcccgcatacccgccgggcggcagaattttgggaagaattacaggcacagtgagctgagaattacagctatctatcgtaactttacggactctataatatattattttaactcatactaatgtcaacagcaactatagccccgcaggcgccacttacgtcaaaagactttacaacggaccaggaagtccgctggtgtcctggctgcggcgactactctatacttaagcaggtacaaactattatgcctacgctgggcgtgccccgcgaaaatattgtgatcgtttccggtatcggttgttcttcgcgctttccatactatatgaatacctatggtatgcactctatccacggccgtgctacggcgattgcgtccggtttgaaagcagcccgcccggagctgagcgtgtggatcgtaacaggcgacggcgatggcttatccattggcggtaaccatactattcacctgctgcgccgtaactttgatgtgaacatcatgttgttcaacaaccagatctacggtttaacaaaaggacagtactctcctacttcagaagaaaataaagtgaccaaatctaccccaatgggtagtattgaccatccgtttaacccaatggcccttgccctgggcgctgatgctacttttattgcccgcagtatggaccgcgacccaaaacacctgcaggaaatgctgaaacgcagccatgcacataaaggcgcttccttcctggaaatataccagaactgtaacatcttcaatgatggcgcctttgaagcctttaccgaaaaaagcagcaaagccgatgaaaccatttttgtggagcacggtaaaccgctggtatttggcgccaccaaaaacaaaggaatccgcctcgatggtttaagaccggtagtagtggaactgggcagtgagtatacagaaagcgacctgtggatccatgatgaaaatgatttctacaaagcacagctgctcacccgtatgtttgatgatgtacgtattgaagggcatttaccccgtccgttcggcctcttctacgaggctttccgccctacttatgaagatatcatgggcttccagttaacagaagcgctggctaaaaaaggccccggcgacctggataaattgctggcaggcagcgaaacctggactatcaaaggataataaacacctccaataaaagaaaaagccttccgtgtatgacggaaggcttttttatatccaactatttttaatgtcccatggcacctacgtcgaacaatactttataaagcaacaccacgccaaaaatgatcatgctggcgccggcaatacggttcagccactctacattggctagcgttaatttgtgacggatcttatcagatacaaataccttcaggatatccgccgataacaccaggcttaggcaaaccgtatacataataatccggtgaccagctgtggtggcgctgttcgccacacaaacccctaaccagaagataataacaccgggattgagggtattcatcaaaaaacccgcaagccatattttaagatagtcatgggtgcggaacatttccggcttttcttctcccgtactgatctttacttttttaaacaacagtccgtatactcccatgcatatcagtaacgctcctcctacaatacctatcgaccttttatattcttccaggccactgataaaagaggtggtcaggttacctgtcaacacaaaaataatatcgctgaaagacacgcccagtgcgaaactgatccctgccttaaagccgttattgatgctgtattttataattgcgaatattaccgggcctactgataaagaaagaaataatcccagtcccagtcccgctacaattgatgctatcatgcgtataatttccgtgtcacaggtgcaacttaactcttaacggtttttcccgcaagaaatttctcccagtctttcagtttctctcctttcattacacggggaaatttattcatggcgccttccttgcctttgcaacggaggtaatctataaacgcatcattcggtaatatctctacaaatacttccttcagtgctgcagagcgttctacggcataatcatcatttacctccgcgagggtttgatcgatgatttcgcgcactttttccgcatccacaccaggtgtatccgtgcccacataccagcggtgtgcaaacaggttctgataagggaaccccgctaccgtaaactcacggacgttaatacccagtttcttctgcacattatctatcgccttgttcatgttgtcgatactcatgtgctccccgcagaggctgaggaactgtttggtacggccaacaatcactatttcatgttcttttactgaagtaaatttcaccacatcgccgatcaggtaacgccaggctcctgcacaggtcgacaacatcaccgcatattccacatcttccactacctcgtggatcatgtaagatttaggattcggttttacttctccttctgcatcaaagttttcttcattaaaaggaatgaattcatagaagatccctgcattcaggaccagcttaatgccctttgtacccggacgggcctggaagccaaaagaaccttcagaagccatataggtttcaatgaacgcaatgggctttccgagcagcttctggaagctatcgcggtacggctcaaaagataccccgccgtgaatatataccgccaggttgggccatatttcatgaatatttttaacgccgtgatatttgatgatttcttccagtacgatctgtacccaggcaggtacaccgcaaacagtacctacatcccactccttcgctttgcgcacgattaacttaatacgctgttcccagttgggtttgcgggatattttgcctcccggcttatagaaacggcggaaccatttcgggatatttttggcttgaatgccgctcatatcaccttcataatagtcgcctttttcatacaacgaggtagtgccgcccagcatcaggatgcctttttcaaaagagcgtggcgggatgttaaagttagccatggaatacagctgcttcacccccactttcttcaccgttctcagcatggctttggtaacaggtatatgtttgctcgcagattccgaagtacctgaactcaacgcaaagtatttgatcttctcgggccagctcacgtttgcttcaccttccaggcagcggtaccaccactccgcatgcattttagtgtagttatgcacggggactttatcgcggtaatgactaataaaattagcgctatccaatacttcctgaaattggtagtggcggccaaactctgtatccttggccttttccagcaaacgatgcagcacctgcagctggtattggcgcggtgttcctaatttaaatgtgaacttcttcctgatgcgtagtgacctggaaataagattacctatgatggccattaactttccctctctttaattgaactacaaaaataagtggaatattgaatataagttgactgataattcggaattacagattatgtagtatcattaagtcatctatacatataaaatatccaaaacatgtaggttataattcgcaattcataattcgtaattcgtaattacctttgcggcatgttaaaaacaactttactcaaagctactgaagacagcggaaaaatactgcaacaatatttcaacggtcctttcgaggtgagcagtaaaagtacggttaacgacctggtaacagaagtggataaaaagtctgaaaccgctatcatcaatattatcagggaaacttatcctgatcattttatcctgagtgaagaagtgggcgagatgaagacggattcttccgtgaaatggatcattgacccgatcgacggaaccgttaactacgccaatggcattcccatctgttgtgtatccataggcgtggaaaaagacggggaaatgatactgggagcggtatacaacccttttatgaacgagtttttcctggcagaaaaagggcagggagctacgctgaatggtaaaccgatccaggtttctaccaaagccaatgtgtcaacctcctgcctggtaacaggttttgcctatcaatggcaggatagtgccaacaatcccttacaggtacttgagcgcgttattaaggagggcattcctgttcgcaggctggggtctgcagccatagatctctgctgggtggcctgcggccgctttgatggattttatgaacaccatctccaggcatgggattctgccgccggctatctcattgtagaagaagcgggtggaaaggtaacagacttttcaggcaaccgttactccccctatcagaaagaaatactggccaccaacggtcatatccatagcgcattacaagatcttgttaacggtaaataagtattgggaagatggaacaggaaagaactgaaatacaggacctgggagaattcggattgatcgaatatctcaccaggaacatagaaatacaaaacgccagcaccgtattaggtgtgggcgatgatgcagccgtgatcgatcacttcggtaaacaaacggtaatcagcaccgatatgctggtggaaggcattcacttcgacctgatgtacacaccactgaaacatctcgggtataaatcggtagtggtgaacctgtcagacatctacgcgatgaacgccacgcctacgcagatcacggtgagcattgctttctccaaccgtttctccctggaagcgctcaatgaattctacgaaggcgtgtatgctgcctgcgagaaatacggcgtagacctggttggcggcgataccagcaactcacaaaaaggttttattatcagcgttaccgccatcggcgaagtaacccccgaccagttcgtaaaacggtcgaccgcagaaaagggcgacctgctctgcgttaccggcgaccttggcgcggcctacctcggtcttacactcctggaaagagagaagaagatatacctggaaagcccggaagtaaagcccgacctggaagaccagacctacatcattggccgccagctgaagccggaagcccgtaaggatattatcgaattcctgcagcaggaagacattaagccttcttccatgatggatgtaagcgatggtctcagctctgaaatactgcatatcgccaaacagagtaacctgggcgttatcgtgtatgaagaaaagatccctatcgcccaggaaagcaaggaaatagccatgaaatttggcctggaccccactgcctgcgcgctaagtggcggtgaagactacgaactgctctttaccatgaagcaagcagactacgacaaaattgtactcaatgagcagatcagtgtgatcggctacatgaccgatatcaccgaaggagcacacatcctcaccaaaggaggcaacaagtacaaactggtggcacagggctggaacgcgttccagcagtaagcggagggaccgccttcggcggttgtaaattgtcttggagcaggattacgctgattttactgattagcttgatttttattctttggattttattagattttagaaatattaagggagatacgagcgaatatatccgcttatatctcccttaatctattaaaatcaaaagtgatcaaatcaagctaatcagtaaaatcagcgtaatcctgctccaagacaatttacaaccgccgaaggcggtcagctgcattacttctcaacaatcacgggtatcaccgggctgttgtgtgtgggcggcatgtcgccggcaaacacggagaacttcagctggtatttgcccggtttatcgggcatcaccacttccaggttgatgaggcgtcgcagcacggcccgttccagggtcatggaggatttcaccggtggcagggattcgtctttggccatgaacccgtagcccagtaccggttcgttggtcctgtcgagccggatgggctggtggtagccattggtaggttgcaggatcacatttacatgttcaccacgttttgcccggatacttttcagtgcgggtttcaactgtatcagtgagtaagaataataatcagattgaatgtagtagtcccaggtgccatgaatagttttaaggctatctgtgattggaattcctgtgccgggatcagataccaccattacgggcttaccccatagttgtgtttcagtgtcccagaaattatactggctcctgcgggcatagcggctgttaaggctgtaggaaagctgcccggtataaaacatgtacttcgacggacgttggtagctgttcacaaaaaccactggtctaccttgtgcgcgggcggctacctgtgccgtccattccttgttatgatggatttcaggtcttatctccactcccggcataaaatcccagaccatgtatacccgcaccaggagtaccagcagcaacgtaaccggcaaagtatacaacaaccatttctgcgaccagcctttccgtacaatggcctgatgcgccagtattactaccggggtaaagagcatcaccgtccagttggcttccaccctgcctttgaaggtgctgagcaggaaaaaggacaatacgccgatcacgcaaaatttcagggcgcgttcgaaggagttggtgatggggctgcggaaggcataatacagtatgagccagcccagtaaaggaccgaataataagagttgcccgccgagataatcgagcgagtaactaatatcataggaagatgcgttcctgtctaccaggtgatattgcagcgaagggaaaccgtgggtatattgccagtaaatatgcggcaggaacaacaccgtggtgagcacgcaggccacataaaacttaaatacttttaacaggtttacgttggataaaacagtgaagaacaccagcaggatgccgtggtatttactgtaaaacatcagtgtcatggaaatacccagcagcagggtgtttctccaggtttgctcatttacaaaattgcggtagacccagaaaaatactgcggcaaaaaagatcaggggaacatccggcactgccagtatgccgccgatctgcatggcgcccatagatccgatgagcaggtaaaagagtttattgtcttttgaagcaatcagtttggcggtaatccagagggtgagtgtgtttaccacaacaatgagcagcctcactcccagttcattatgaaagatcccgtacccgattttgatcagcagcgcaatcataggcggatgatcaaagtagccccagtccatgtggcgtgaatacacccagtaataggcttcatcatcccacagctcagaaaagcaggcctgtaacaggcccagtaccagccaggagagcaggaacaaatttttataccggtcttttttcagaaagcgagttagtgcgctcatgcggatatacagtattattaatcctgcgaagatagggctattaacagtatactgtagtttcccagttagagtcgatggctaccaatgctgcgtcatagcctaccgcaatacggcccaatgcctgttcacggccaattgcgcgggccggatacagtgatgccatacgtaaagcttcctccagcggaatgcccacctgttccacacaattgcggacagctttggtcatggtgagccgtgagccggacaaaacacccgaggcgcttacatagcgatccgtctctttaatatacacatacccgccttctttattctcctccactgcatctgtaatcaggaacaggcgttctttcatgatctttttgctgatcctgatggaggcaaagtccacatgtacaccatctgcgacgatgctggcggatacccgggggtgatcataaatggcgcccaccaggccgggagcacggctttccagcggcgacatggcattaaaaagatgcgtagcatgatgaataccgctgtcaaacgacgtataggcctgcgcgtaagtagcgttgctatgtccggcaaatatcacgataccggctgcctccagctgccttaccagttcgggatcacagcattccggcgccagggtcatgatcttcaccacatcacggccgttttccaggatccagttaatatcttcctgggtaggggaatgaatatattgttcgaggtgtgcgccttttttcttcgggttgataaaaggcccttccaggtgcagtcccagcacgccttgcccgccctgctcccaatacgccttcactgcattcatggcctccagcataatttcggggctgatggttgccacggtgggcatgatccaggcggcgccgccacctttgctgtaagccacagtggccgccagggaggtaaccgaaggatacatggaaaacacgtggctgttgcctccgtagatctgcagatctataaaagccggggccagcaggcctcctttcaggtctgtttcgctgccggttgttttccattctgaagaaggaacaatgctggtaattttccctccttgtgtaatcactgcatgatcatccaatatctcttccccggtaaagatccgggcattgatgtaggcaacagacatagcaataaaattttacgggtgttaaatgacttcgtataactctaaaggcaaaccgtcggggtctgcaaaaaaggtgaatcgttgttgggtatgcggatcaatgcgtagtggttcggtagtcacgcctttctgctgcagttgtgcaacggcggcttcgatgtcggccactgcgaaagcgaggtggcgaagcccgcatgcctccgggtggcttggccgtggcggcgggtccgggaaagaaaacagctcaataatgtactggttgcccagtgccaggtccagcttccaggaatcccgttcttcccggtatacttcgcgtattacctgcaggcccagcacatcggtataaaatgttttactccgggagtaatctgcacaaataaccgcgatgtgatggactgcctgtaacaacatataaaaatatctttagttagaacgttgctattatccttttgggagaatagtaaatgcgtcggcatctttcaggaaaggaatgttcttcctcacttcttccagccgctcacgtttaagagtatacgtaaatatgtcttcatcgtgcgatttgcggtaaatgatttctcccatcggatcaatcaaactggtttccccgctgtgataaatattgttgccgtcgttgcctacccggtttacaccgatggcaaaagcctggttttcaatagcgcgggcctgcaacagggtagtccaggcagttttacgcctctccggccagttggctacatacaccagcagatcgtaagctggttcgttagtatccggctggatggtattgcgcgaccataccgggaaacgcatatcaaaacagatgttcagattgattttccagcccttcacctgcgcaataaggcgcttatctccgggcgtgtagtgttcgtgttcacctgcataaccaaacaggtggcgcttatcataagtgccgtaagtgccattgggcagcatccagaccaggcggttcaggtattctccgttttcctcgataatcaggctgccggtgatgatgatattcttctccgccgccttcttcttcatccactgtactgcggttccatccattgtttcagccagctgcgctgactgcatactgaagccggtgctgaacatttcgggtaaaaataccacttcggtcctctcctttatgctgttgattttctcatcaaacatacgcaggttggcttccttgtcttcccaatgcaattgggcttgtatgagtgttactatcagatctgacattatcggttattgtgatcacaaaattacggcctgacgggttagaaacttttcaaattattgcccgcttaagcctcgttctttgcgatttgttcaagtgcttcgttgatgaggtctggttcaaaacctctttgaaggagatattgcatggccttatacctgcgcttcatggctgtttctcctttgagcgactggtattttttctctgccagcttgtgaagtactgcgatgtaatcatcgtcatcaatttcctccattccttttttgatgcagtaggcagatacctgtttctgcttcagctccatcataatttttttgcgcccccattgcttgatccggaatttgccgccggcgtaggctttggcaaacctttcctcgttgagaaaattttcagcgatgagctcagcaatggcttcgtctacttcctctcccctcaggcccagctccaggcatttgtattttgtttcctggtggctccgttcctggtaggcacaaaactgccggagttttaacatcgcggttttcatgtcacttatcttactattctcagcttggcgtagttcagcataattttcttttcaccgccgcctttagggaagttgatggtagcaatcctgttgttaggtgctccttccaatgctgcgatgataccaaatccaaatttctgatgctctacctgcataccgggctccatgccggccggatcgtccggggcaaaatcagcggaaggtacgtgggtagtggcgggagaaaaggtgggtttggcagcgggcttctgtgccaccggctgcgacggttgcgacggcgcctttttccggtcgaacatattattgctgttgctccatccggaggtgctgccaccgccgaaagcgttgcgtacgctgcctccgccggcatagctgcggtcaatgaatttctccggcatttcttcaaggaaacggctcggttcattctgcaccaggttaccaaagcggtaacggctattggcgtatgtgagccataagcgtgcctttgcgcgggtaatggctacataaaacagtcttctttcctcttccagttcttcccgggtgttgatagacatgccactggggaacaatgtttcttccagccctacggtgaataccaccgggaattccagtccttttgcggcgtggatggtcatcagtttcaccacatcgctgttttcatcgctgccctggtcggcatctgtgaggagggtgatttgctgaagataagaacccatgcttttatcaagcagctctccttcttcatcgggggtttctgtaaactctttgatggagtttaagagttcctgcacgttttcataacgggcaagcccctccgtagttttatcgttaaacagttcttttacaatgttggtagatttacccaccgcaacggccacatcataggcgttgtgcgaggtgagcattgcctggaagcttttgatcatgattacaaatgcttctatggcttctacggtaccgcctttaaagccgaactccctggccctttccagtacttcccacatggtgatattgtgttcattgctgagcacaatggttttttcgatggtggttttaccaataccgcgaacggggtagttgatgatccttttcaggctttcttcatcgcgggtattcatagtaatgcgcaggtaagccacgtagtctttgatttccttacgctggtagaaagacaggcccccaaagatgcggtatggaatggctttacggcgcaggctttcttcaaaggagcggctctgggcgttggtgcggtacaggataacaaagtcgcggttatcataatgattccgcagtttctgttccgaaatagtatccgcaacaaatttaccttcttcgttgtcggtcatggtgcgtaccagtttgatggtatcgccttcggtgttatctgtccagaggtttttttctatctgtcctttgttatgtgcaattacttcattggctacattgagtatggacttggtgctgcggtagttttgttccagttttaccactttcacatcatcataatccttttcaaactggaggatattttcgatggtagcgccgcggaaggagtagatactctgggcatcatctcccactacgcaaatattttcattaacagcgccgagtaatttgatgatttcgtactgggcagggttggtatcctggtactcatcgatcatgatgtatttgaacttgtgctggtatttatgcagtacttccgggaatgttttgaggaggatatacattttaaacaacaggtcgtcgaagtccattgcgccgtttttaaacgtgcgtttggcgtacatgtcgtaaattttgccgatcagcggcctgttggcgcgcatatcttcctgttgtaccaggttatccaactggtattcgtccggtcccatgaggctgtttttggcagctgagatgcggttataaacgaagttgggtttatagtgtttatcatcgagattcagctcgttgataatggttttgataacgcttttggcgtcgtcggtatcgtagatggtaaagtcgttgggatagccgagccggtgtgcttctgcacgcaggaggcgggcaaatacggagtggaaggtaccgatgtaaaggttacgggcttcgctgccaccgaggatcttttccacacgttccttcatttcccgggcagccttattggtaaaggtgagggataaaatattaaacgcatccacgccattccgcatcaggtgtgcgatacgggtggtgagcaccttcgtttttcccgaaccggcgcccgctacaatcatcaaagggccgttgatatgtattactgcttcccgctgttgttcgttaagctcgtctaaataatttgccttcatcacgactgctgtttatattttatatgtagaaaagatatagtatttctgaagggtgtaaaagtacgaaaaaggcggagaatagaatcgcctccggtgatgcgtattttgtcttggctcaggattacgctgattttactgattagctggatttttacttttggatttataaaggattaagggagatagaagcggatatccgctcttatctcccttaattattaattattattaaatcaaaaaatctaaaaaaatctaaaagtaaaaatccagctaatcagtaaaatcagcgtaatcctgagccaagacaacctccgctacggtttcgcgccgagcgctttcatgaagcggaagtgcgatactactgctccctgcatggtagggatggaattgtaagtaaggttatgttctgcgcatttggcggccacaattttgctgagggccgggtaatgcacatggctgatccttgggaacaggtgatgttctacctggtaattcagaccacctacaaaccaggaaatgactttatgccccggtgcgaagttggcagtggttttgatctggtgaatagcccattcgttttcgatcagtttggcatcttcgcccactgcttcaaattcggtttcttccaccacgtgagccagttggaatacgatggcgagggtgaagcccattaccacgtgcattactgcgaagccgatggcccaggcctgccagcctaccaatacgatgggtaaagcgatataaaacgccaggtataataccttgctgccccagaacaccatgtggtcggttaatttcatgggttgcagcggggtagtatatactttccggctcaggtatttcacaaaatccatgataaatacccatgcgaaagaagatatagcgtataccagtactacgtaaatgtgctggatccggtgcatgggcacccatttctgggagctgcactgtctcatgagcgggcttttggcgatatcatcatccaggccgtctacgttggtgtaagtatggtgaatgatattgtgtttctgtttccagatgaaagcgttgccgcccaatgcgttaagggtaagaccgagggtgtcgtttactttgctgttggtagagtaactgccgtgacatgcgtcatgcattacattaaacccgatacttgccagtacaaaccccagcaaagcgcataaagttaccgagagcatggccggcatcgatataaataataccgaaaggtacagccctactgctaccggaataaggacagcggtttttatatatagtttccagttacctgttttctgaatgttgtttgatttgaaatagtcctctacagcggatttgagtgctggaaagaataaggcattcttgttgttgaaagttactttaggcataaaaaaataagcattgttgttgccgggcgtacagtttagttgtagagaaaccggaaaaaaattgaaaagtctacgctaataaacggcttttaaaccggtttttatatatttcccccgataataaatggttatttaacaaagatttgtgcttatagaggggattggaagcagggggatgacaatcggaggaaaaatggggataacagaagttcacaaacaggctacagcaataaccggttatctgccgggggcagacaataaaacacacaaacaacaacacctgctacggggtattagcagcgtcttcaatggtcacactgagggtttgcagacttctgttatccaagtctgatgatactattgtaagattaacgagcggctaatgccttgtgatacgcgtcttcagcattttccgggcaaagtggatacggctttttaccgtacccaatggttcattgagtatagctgcaatttcataatacttatagccttcaaaatacaacaggaatggttgcttaaaaataaccggcagattatacactgccatctgcacgtctttcacccgcaggtctgattccgcgaagtttccgatggcagaaggctggtggctcaacaggtaatctcctactgcattatccagtaaccggtattggcggttaccgcgacgataattattaatgaagatatttctcatgatcgtatatagccaggcgcggatgttagtgccggcgagatacttatcacgattagacagtgctctgaataaggtttcctggtaaagatcttttgcggattcagagtctttagtcaatgttacagcatatggccgcaggaaatcggcatttccgagtaataagttattaaattcggtggatgacataacggttaactttaaagtattcacaattagctagaacaacagcctgtaaatgggccgggagaaatagcatctggggtaccgcgggtctccttccggcggatactaccggcacctgccacgctaatttaaaagggaggtatcaacaccctgataaacggcagcaacaggtgccctagtcaggtgttgtgacaatcataaagaacggttttagttaaagaataagcttgcataaatggggtgctttaaaaaatagtaaatcagggtattatattcttcaattatatagctatcgtttaatgcttcgcagtctgaatgatagtaaaatgagcatgattcctgtgaaaattgcgtatatcccaaagatccaggtaagtgtaacggcggcagccacggggtttgcgacgaggagaatcccaaagataatggtcagcaaaccgcccgcaatataccagccctcacctgttatcaccttccttaacctgatggcaatgatcagctcaaacaggcctgccagcgcagcccagaaagcaaccaggtaaatgagtgcagcgccggtagcaaaaggattgtaaaaagtgaggatacctaatataacgcccagcaggcccgaaagcaggaaaataccccagttctcgttcgttttcctggctgctattgcacctgccacagcaaaaaggccggcaataaaaagatatgcgcctaagaaaacgatcaatgtggtaaaagtagcaccaggccaacctacggccagtactcccaaaacgagggcgaaagttcctcttaataaaaagagccaccagtaagcgttataaaaatcaggcatgcattctcagttttaggtttccactacgagtgctgtattatggcagggtgtaccattgcgcgctatgagcatttccgtttctcaacattctgaacaaccaggattattagctacaaatacttcaatgcattaactaggtgtttccgtcgtaaaacaatcaggacacaagggtgctcgccttgtgggatagtattttataaaaacagaaaggtggcaggtgtttccatactgtaagttatatggttaataatcgcctcaactacttgtaacttgattcacctgttcatttaaaaaaagagtctatacacaatttaaaaaaatttgttaaaaaaaacaaaaaggatttagccggtacatccataccggaatcagggattttttggaagatttaagcttattggtttatttttcgtgccggtcgaccaccagtttctgctcgcggttggcaatttcccaggcggtgtaaaaaaccaggcgggccctttttgccagcaggtcgtagctgatcttctccacagtatctgttggggcatgataatcagcatgtgtgccattaaaataaaaaatgatgggaatgccatgctgcgcaaacatatagtgatcggagcggtagtagaatccttccggatcgttggggtcgttatatttataatccagtttaagatgggtatatgtatcattggctttttcattaaccggccgcaattcagagctgagtttgttatcgccgattatatacacatagtttgtatctttttcatgtgcaggatcaatgcgtcctatcatgtcaatgttcagatcggttacggtgttggtcaacgggtaaacgggatgctcggtataatactgggagcctagcaatcctttttcctcgccggatacggtcatgaataccatacttctccgcggaccgttgccggcttttttggcgcgtgcaaaagcggcggcaatttctatcacagcgctggtacctgatccgtcgtcgtctgcgccataaaaaatttcgtcgtcttttttaccaagatgatcatagtgggcagtcacaaaaacaacttcctcttttttatcggtgccttccaggtaagccagtacattggagggttgcaaaacggtagctgctttatcaaaaacaagatgaaccggtatttgcgtaaccggcgatggcttccagcccctgtttatttcttcgaggagattatcgcctttatcggtacggagtatatcggcggccagagccggggtgatgtaataaatatttggattccaggaggtatctttttgccagtaaagtccggtggtatggagttttttctgctccagggagcggtatctgccggcagcggggctgatgatcagtaaggcagccacgcctttatttttcgcggtgctgatcctctcgtcgaggctgcggcggtcccgttgcaatcctttcctgacatcatccctgatcatcactacctggccttttacgtccatgttttcataatcattgtgatctgccgtaactacacctgcatctgcataaaatacgcgggatacgcgtagatcctgtttgttgccggagcggagatccgcgagaaagtcctgtgcaaataaatatgttttattacctacggtgatagtgcttttgagcaaactatctgaatagatgggataatattgttcccatttcccatgggcgccgggctgaagtcctgcggccgagaactggctgatgatataggctgcagccctctcctgtcctcttgtggcggtttcccttccttccatttccgggcctgcaataatgtgcagttgccggctaagaccggcggcggtaatggtttcaccatattctgcagccaccccgttattggtttgtgcctgcgcaatattcatcagcaacagtaaggcgacagcaaacagaactctcatggagtaattttttatagtcagattcacatgaatattaaataaaaagagccggttggaagccggctctttaatattactacaatttcgtgtattcgttacagtaaaaaatgatatatggctttaaaccgttacaggcaaaccattttacgtacgcggtcctggtggcggccaccttcaaacggcgtacccataaacacttctaccatttgattggctgcaggaatatccacaaaacgggcagggatacacaacacatttgcgttgttgtgtgaacgtgccagccgcgccagttcttctccccagcagatggcagcacggataccctggtgtttgttggcggtaatagccaccccgttggcgctgccgcaaataagaataccgaaggccgcttgttccctttctactgctgtagacaccgggtgcgcataatcaggataatccacagaatctttcgagtgggtgccgtaatcctttacctgcaggcctttcgactccaggaaagaaattacttcttctttatattcatatcctgcatgatcagaaccgatagccacgggcaatgtcaggttaaatatattttccattttcaatatcttattaactgttagagataattaagaccactcttccacatctgttttagccatcttgtcttcacgatctttcagcgcctttttcgatataaagatactgatttcatacagacagtataagggtacaaatacgatcagctgatctatcagatccggcggcgtaattactgcagccaggatcaggatcaccacgatggcatgacgcctgtaagctttgaggaaatccggtgtgaggatgcccagtttggtgaggaaaaatacgaggatgggcaattcaaacaggatccccatacccagtacgatctgtgtcatcagatcaaagtaatcatctataaaaaactggtttacagcttttgccgtaacagtataggaagcgaggaagttgatggtgaagggcgccatcaggaaataggcgaatccgataccgaggaaaaactgaaaagatacccagaagatcacgcctcttgctcctttcagttctctttctttcagcgctggttttacgaagcgccagaactcccagaaaatgtacggaaaggcgcaaataaagccgatcatgaacgccagtttaaattgcagcataatctgccccaccatcttataattcaaaaactggacctttacaggcgtaatacagagccggtcgcccatgcctatccaatggctgattttacatagtatcacgtaagaagggaagtcggcgttggtaggtccaaaaattacgttgtccaggatttcctctgtatataaaaagccgaatacgctgaatgcaacaagtgccagggccgatctgacaaggtgccaccggagatcttcgaggtggtcgaaaaaagacatctctgccttatcctcattgcttgcgaataatttctttaacatactttatacggtcgaacgatgttgaatacagtttcttattaaggatcacaaatatagcggttgcatactacaaattacagtgtgcagccataaagtaccctattttaatattgctttaatcgaaggtggtgactatgccaatggcatgtacgtaaaaagaaaaaatcaggaagaagaaaaagaagaaaagcgtaggagcagttgggagaaaaaaaagagccagcccgagaagaatcaagagccggcctttcatccattgtttgttaaccccaaaaaagttgaattcgagaatgtctttagcttccagttatgctacttacctaattgatggcaagcgttcagaataagtaagaatccctggttgcgttttatattgtaatacaaaaataacaagaattattttattatcaatgttggaacactttttttacaaccttttaacaaaaatcaaatcattgtgttacatcatctggagcaaatgtatacaatccgtgttaaattcctactactttttttaaaaacgttttagcaaaattgttattgtatcgttaaccattacattacggaaataattatatcatattaatatcagataagtcaaccgatttaacggtaacccttatactaacatcttcatcttcaccatttcgatcctggtatccgtaacattcagaatatcaaactcataatcatcgattataatgcgttccttgatctttggaatggtttcgtgatggttgataatgtatccggacaatgtttcactttcatcttccggaaagtccagtccatatcgctcattcaagtaatcaagctctaatcttccggaaaaaatatattctttttcagcgatctgcttttctacaaattcttcttcatcgtgttcatccttgatttctccgaaaatttcttccagtacatcttcaatggttacgatacctgccgttcctccgaactcatctactacccaggcaatgctcttacgttctttgttaaacttgctgagcaggtcaatagcgctcattgtttccggtaccgccaatatgggatgaatgatgcttttaatatcaggcgggctcttaaacatatccaactggtggatgtagcccaggatgttatcaatggaaccttcgtaaataatgatcttagatagcttggtgtccataaatttactccgggcatcactgagtggccggtgtatttcgagcgcttctatttccttgcggggaatcaggcaaccacggatttttacatgtgcaagtgacaaagcattttcaaacagctctgtattcagctcctggttattttccccgaagtgctgttgcgactgccggataaaatgttctacatccacgcgggtgaaggattcaccattttccacgatacggacgttgaacaaatatttcagcatccattcggagatcgaagcgagtacattaccgatcacatacaatggcttggccactaaggaaacgggcagtgcaaagaaactgagcagtgcttcgggtcttgaccggaaaattgcccttggaataaaaaagccaaggaataataccagcagggtggccagtattatttcaacgaaaataataaagggttgaatgctggcggaatcaggcgtccgcataatagtgtccagcgccggctgaaatacgcctgccacgaggatcccataaacaactatggtgatcgtgaatcctaccaggctggtagccaggaagcgactggggttttcattcagactggccagtattttgccagtagccctgccttgcttttttttgagctcaatgctaagtttgttaacattggcaaaggcagcttcgatacctgaaaagaagcctgccagcaataccaggaaaaccaaaataattattgtgtatccatccatcctaacaaaaataacgaattaggaaaaccaacgatcacgtcgctattttatatttaaaaaatctgtcaccagtttttttacttcttcataggcgtgctccagttcgtcgttcaccacaatctggtcaaattcatgggaaaacgacagctcatagcgtgctttggcgagccgttcgtccagtgaggactgtgattccgttcctctttcactgagccggacgcgcaaggcatctaacgaggggggctgtatgaaaatagtgagtgcgttgtcgtgatatttttctttgatagataatgcgccctttacatcgatgtccaccatcgggatctggttgttgttccagatacgctccagttcacttttcagggttccgtaatatttaccggcatacaccatttcatattctgcgaaggcgttttcttcaatccgctgatgaaattcatcggaggacaggaagtagtagtcttttccgtgtacttcgctggcacgcggggtgcgggtgctggcggaaatcgaaaaggacagtaccggcatgttagccagcagttttttcacgatggtggttttaccggcgcctgaaggagcggtaacgatgatgatctttctttccattattaattacaatcaaggtagcggttacttcaaatgcaaaacccaaaaaccagtaaaatgttttgctggtatttgggtttgatgaagtatgaacaactgtttatactctctttatgtctgctcccagctttctcaacctttcgtcgatgtactggtagccacggtctatctggtcaatgttctgaatggtgctctttccttctgcgctgagtgcagcgatcagcagggataccccggcgcggatatcgggagatgacatggtgattccgcgcaggttgtgctggcggcccaaaccgattaccactgcacggtgcggatcgcataatacgatctgtgcgcccatgtctatcagtttatccacgaaaaacaggcggctttcaaacatcttctgatggatcatcacgctgccttttgcctgtgtggctactaccagcacaatactgagcaggtccggtgtaaacccgggccagggatgatcagaaatggtaagaatggagccatcgaggaatgtctggatttcgtaggagtcctgcgaaggaatataaatatcgtttcccctgatttccagttggatacctagctgacggaatttttccgggatgatacccaggttatctacacctgcattcttaatagtgatttcgctttgcgtcatggcggccaggccaatgaaggagcctatttcgatcatatccgggagcatgctgtgttcgcagccgccaagatatttcacgccttcaatggtgaggaggttggagcctactccgctgatgcgggcgcccatgcggttcagcattttacacagctgctggagatatggttcgcaggcagcgttgtaaatagtggtggttccttcggccattaccgctgccattacaatattggcagtaccggtaacgcttggctcatccagcagcatataagtgcctttgagccctccggaagattccaggcggaagtagttatcatccgcatcatatacaaacctggctcccagtttctcgaacccgatgatatgggtatccagtctgcggcggcctattttatcgccaccgggttttgggatgaaggcgcgtccgaaccttgccagcagcggacctgcaatcatcaccgagccacggagacggccggatttctttttaaactcagggctttccaggtatttcaggtctactgcatctgcctgaaattcgcaggtatccctgctgatacgattcaattttacgccagcatctcctaacagctctatcagcagatttacatctactatatccggaatattggtgatagtaaccttttcgggggttagcatcacagcactgatgatttgtaaagcttcgtttttggcaccctggggtataatttctccctttaagcggttgccgcctcttacttcaaaagcactactcacttgttcctgtttttgttgtatttgttattgtgcttattgttattatcccggcttttgctgccgccactgccgctattgctgcttttgaacttgttttgctggaagtttttgcgcttactggagcggaactggtcggctgcgcctgctacgttaccgcttggtacaaagcttacaggggctggaatatgggcagcatggcccgggtggaattccagctggttgtctgtaatagccagtaattctgccttgatggcatcatcgtgtacactttccttatgccagttactgtaggccagtttcatatagttaccgatgcattgggtaaatccttcctttttttcgggattatcttcgtgtacggctttgtcaatgatcatttccaggtttttaccgaagtgacggttcctgggatatttctttggataaggaagtctgtcgggtttggccctgagcttttcaatagtggggattggatagggtgattccaccttcaggttaaagccggagatattaaaaatatgatcccataatttatgcctgaagtcttccacattgcgtaaatgcgggttcagcgtacccatcagctctattacagccatagcattacgctggcgctcttcgtcgtcttctatggttaccaggtactccaccattttctggatattcctgccatattccttcattatcaggtaattgcgcgtggtattgtattccattactagtatttaaaaaaacatgatttgatgatgggacatcttaagtgaagaaaattaatcggcaacatctatgcaaacataataaaaaaatatgaggaacatttcattgggctgtattgtttattagagcaaaaacattgttatggaccaattgaaaaacaaggtagcgctggttactggcgcgggttccggcattggtaaatgtgtagcggagctgtatgccgccaatggcgcggctgtggtgatcagtgatattgatgaaaagggtggaaaagccgtggcagacgggatcaacagcaaaggaggcagggccatctttgtaaaatcggatagcagtagcccggccgactgtgagcaactggtgtccaaaaccctggcggagttcaaacagctggatattgcctgtaataatgccggtattggcggagcagcagcgcccacgggtgagtataagctggaggagtggcaaaaagttattaacataaatctcaatggcgttttttatggcatgcgctaccagttgccggtgatggaaaaagccggtagcggtgtaattgtgaacatggcctccatacttggagcggtaggtttcgcagggtcctgtgcttatgtggcggccaaacatggcgtggtagggcttacccaggcggcggcagtggaatattccgccaaaggcgtccgggtaaatgcggtaggaccgggatttattgaaaccccattattaaccaaacatctgagccagcaggagatgcaggcacttgtgggtttgcatcccataggccggctgggcaagccggaagaggttgcagaactggtattatggctcagttctccgcaatcctctttcgtaaccggcagctactatcccatcgatggagcatacctggccagatgatttggttatgttgttttttgggtatttcagggagataaaaaatagctatctccctgaaaaattcaaataatcaaacaggcaaatccaaaatgtttgctagttttagtcaatgcaaacacataaactccccatactttttttacatggcgcactgggcgcctcttcccaatttgaaccgctggctaaggaaatgtctgaccattacgatgtgcacctgattaatttcagcgggcacggcgatgtgcctttttcggagcaggggttcagtatccaggtatttgcggcggaagtattatcctatcttgaaacccatcaactcgactttgtacacattttcggatacagcatgggtggttatgtagccatgtacctggcgcggcattacccggaaaagaccgggcgcgtgattacgctggccaccaagtttaactggaacgaggctactgcaggaaaagagatacggcagctgaatccggatttaattgaagagaaggtgccggcttttgccagggtgctggaagcccggcatactgccagcgactggaaaaccgtggtgacgcgcacggcacagctgatagaggaactggggcatcagtcgctgctgaagccagccgattatgcccgggtagtaaccccttgtatgctgatgatgggcgaccgggacaacatggtgtctttccatgaaaccattgaggtgtacagtggccttccgctggcgcagttaacggtgatgccggatacggcacatccactggaaaaagcggatgtaccgttactggcttattatttaagaagatttaccacgcaggatatctgacggcgttttactcgcccatagcaattttaccccagttgttgagttcttcttccgtccatagttcggggaagaaaacgatgcgtttattttttggaggcaggaattgctgccagttggtgcctccggtggcggcaatgtcttccggccttttatgcaggtatcttaccgcggatttgtagtgcatcagcggccagcgtacgtttacattgagatcgtactcctttaacagggggattaattccgtttgttccgcgggggagagctttttatagctggccagcaggttactgtctttgtactcagtggccagtttcaggaaggtatccatatatttcagttcaaactggcggagggtaagcgtttttttacctgtagccagttcggtggcgccgcttctccagtagattttgtccagcacgtctttcagttcctggccttccacttccgggcgctggggttcgtataccaggttgtttagccgggtagagcagatctcgatcatgcggaattgtccgctctggaagccactggcaggtaacagcgccatgcggaattgcaggaactgttccttgtccatcccatctaccattatttcaaatgagctgataagactgtggaaatagttgttgatccttttaagctgggttttaaatatctcagctgacagtacaggtgcaaggctgatttgttcgattgcctgcaacgataatttcaaatacaattccgtgatctggtgatagatgatgaatattctttcatcaggaattggtgtgcgtggatgttgcagattaagcaatacatcaagctgaatataatcccaataagtgaggtagtccgcgtacagaaggccatccaggtaggatgacaggttctggcccatggcggcatacttttcttccagccgttgaattttttcggcgatttctgttgtaaccatggcgaaaattaataattaagaatgaaatagcaacagggtaagcctttcatccttaaaaactaattattctaccacgttaattgttctgtaaaagctttcttccagggaaatcagggtttcagttctctcaatgcctttaattttctgcagttcatcgtggaggatacggcggagctgggtgatatctttacagataatttctgcaaacatgctgtaactgcccgttgtatagttaaggcgtaccatttcgggtattttccttaattccttggctaccgtgtcgtacatggagcttttttccagataaatgccgataaaagcgatcacatcatagccgatcatttttaaatctacatgtaatttagtacctttaactacacccagttcttgtaatttcttcattctcacgtggatagtcccgccggaaacgaacaatttcttccccaggtcggcgtaggagatctcagcattagacatcatctcgctgataatctgcaaatctagtttgtcaatattcaaattgtggctcatttttacaatttgtttttgattgttttaaagttatatgcaaatatttaaaaaatatcgaaaattccaaaattcttcttaaaaaatttgcaagaaagtcaccttctctttagatttgcatcataatcattacgaaaacggctcacggaaagcaacagctggtaacgattcaaacacattgtgggatgatgaaattggcagacatgccctcttgtctcgagggtggggatcacaggataaacgtagtataattgggttgaccactaatcttacttgtgctacagctaactgccccgtggaggttcgactcctcctcctacagcttaattggtttaaagagctcgtaagttatcatgcttacgggctttttttattggggaatgcgcatttaggttctattaacacattagttgttatcccatagtacattagaggccattgtttttttaaatgaagtatgatacttatcagctgttacaggcatcagcagacctgcgcatctttacttttaccagtattggcccgaatggaaacattataaagcagttggagttccaggaaacgataataccgggcatatacaatctttgcctaagcgatatcagtgaaacaggcgattccgacgatgaaaatgtgaccaataacaacgacagaaaccttgttcttgctactgtagccggtcttgtggacatctatctggaaagaaatcccaatcactggatacttatcgagggaagtacattatcaagaataagattatatagaatggccataggagttaactttgacgaattatctgccaggtttgatatctatacacagcgggatggaaaattaattccctttaaaaagaatatgcctgctgaaaactttattattcgtttaaaaaacacctaactttaaaatatgaacaagaagaaaatgaaacttcacagtgcgctactcaataaagagataacagtcgttatcagcagctcattgcgcagccttcaatccaatgaactgaatatcaacaaattagccaaggcaaataaacgcctcagcgaattgaaagagttccccggaaagtaaacttcttccgctcccctcctgatccatttatattttcttctttcggcttacttttgcggcaaatgggacaaaaaaaattacaacgatttgctgaaatcgaaaccttccccaatgtattgatatacccggaaggtatgcagggaaagtggaatgaattcttcaaaaacagccaccctgttacattagagttggcctgtggcaaaggagattataccctgggcatggcccggctgtttcctgatcagaattttctgggtgtggacctcaagggcaaccgcatctggagaggcgccaaaaccgcgctggaagaaccgctgccaaacgcggccttcttacgtacacaaatagataagctccctaattattttgcgccgggagaaataaaggacatctggattacctttccggaccccttcctgcgcaattccaagtcgaagaaaaggttaacgcatcctaaattcctgcagctattccagccgttgctggcgccgggagccaccatcaacctgaaaacggactccccgcagctgtatgctttcacgcaggaagtaattgccgcggccggatgcaccctgatagaagatattcctgatgtatatgcattaccggaagtaccgccgttgctgaagatccagaccttttatgaaggcatgcacctcgccgatggcagaacgatccgttatctcaaatttcaattgcctgctgcaccgttgaactggcaaagcattaaactgccttccgatgaagcaaccgttggtggagaagattgatttttactataatgcccagggctatatggtatttaccgaaaaattccacctcgaccggggcttctgttgtggcaatggctgtaagcactgtccttttaattatgaaaaagtacccgaacccgaaagatcagcactccttgcccgtcgcagggacgaaggaaaagaaagccgctgagccggtttctttttttgaaacggtttttaaaattgcacgtaccataccgcgcggcagggtaacctcctatggcgccattgccgacgcttccggtttaaaactcaccggccgtatggtaggctgggcaatgaatgcagccggcagcgccaaaccggctgttcccgcgcatcgtgtggtaaacagcaaaggagaactcagcggccggagtcattttgccacccctaccctgatgcaggaactactggaacaggaaggtgtaattgtaaaagaagataaaatagaaaattttaaagccgtattttgggacccgggacaacctttaaaaaggggcagtaaaaagaaaggataaatttttattcaacatccggaccgggtgcagcgctacttttctatatgacaatactcaagcttaaactggacaacgaccaattggtagaggacttctttgaaagtacctacgtaataggcattgcttccaccacgcgggattatcagttgtgctggcatattaaccggcagttgcataccaatttcagggtaaataacaacctggaaatcgccctgtctaaaaaaacaagatcctttcattttcccgtatttgagtttcacgaacctaccaactcggtagcgcactatttttacaacaatcgctgccaggcagaattcctgctgccggaacttaaacagatcaattttctgtggatgataaagggtgattactatcaacccggcgatgtaaaaaaattattagaagaattacgccttgttccgcttgtacaattagtatctttacttgatatcagagatatcaaaaataagatgaaccttattttttagaagaggcacaacgcatcagcggtagtattttgaccagattccatgacagacccgatgtttttttactttttaaattcctgattttttatgtgggaagaaagaaataaacagctttaccgggcttttgaattcaaagattttcgggatgcatttgcatttatgaccaaggttgcactgattgcagagaaaatggaccaccatcctaactggagcaacgtttataataaagtggaaatattcctgagcacacatgatgccggtgatatcatcaccgctaaggatgaagcaatggcaaaagctattgacaaattgctataaccaaacttatattacactttgtgaagcgcattattctaatgctgctgttgtattgttacactgcagaatcctttgccactgtagatcgtaccccagtagacaccctgatcactgatactgctttcgcccccgcgaatctggacctgcggccttatatgtacgtgctgacagccggcgagcagcacctgagcccggagcaggctgccaacatgccttttacccggcaggaaagtatctttcatagtaatacccagaataacggacgggttaataactgctggctgcgacttaccgtaaaaaataaaagcaataaaccactctcttatcagctgttttcaggctggcacgactatatgtactggtatgtgcaaacgccgggtgataagccccggctattgatggaaaccggtttaatgctggataagggaggggtggaaagatggaaccactacgcgtttgtcgtacaggtaccggcaggagcgcttcgcacgttttaccttcacatcatcaataagtcgtacaacgaaggcgccctgatgccggcactcttcaacgctgaagcctatggcgttttccgggataaacaactggatggcttccgtaaggaggccgtggtaatccaggtattgctgggtatgctgctggtatttttcagcatttccattattaattatatccagttacccgacaaatcgtatatctattttgcgacctatatacttgggttgatcctcttttttgccttacggctggacgataagccttaccaattgtcttttttccaccgctggcccatgctgaaatactattgggacattccgggcctgctgttttgcttttacctgatgtacctgctatttggcaatgcctttcttaacctgaccgagcggtatccttttatggaacgggcatttacatgggtagcggcaatagtagggggactgatcatcctatgcgtgtatttcatcaggataggccaataccatatgcccaccatcatatacagttatgtatattttgtaacgctggtacccttgctggcagtatttgtggcactggcgcggcgctctcgccatcatccactggtgcgattctttttgtatggatccgtatgtttatacctggcctgcctaggctccttcctgatgcatgtgcggccactggggctgctcggcgccctgggagaactggcggcgcccactatcctgctgataggcggcgtattgttacaggccatgtttttccttgcggggctgagttaccgcaataaactggtacacctcgaaagaacccgtacacaggaacttctgattaagcaactgaataaaaataaagagctgcagcggaagctgaatgagcagctggaagagctggtaaaagaacaaaccacagaaatcctgcgcaaaaagcaggaactggaggagcagcggaaaaagcaactggaaacagaatacgataagaaacttacagaaattgagctcaaagccatccgggcccagatcaatccgcacttcattttcaactgcctgaattccatacaattgtttgtaatgcagcgggattatgagtatgcgcagaaatatctctccgatttttcttacctgatccgtaaaaccctggacttctcccggcgtaattttatatcgctggcagatgaaattacctatttgaatacttatcttgggttagaaaagatgcggtttgaaaaccggatggagtatgaaatagtagtagaccccgtgattgccaccgccgaactggaaatccccgcaatgctgttgcaaccttatgtagaaaatgccgtaaagcatggtatgactaatcccaaacagccaacaggaaagctttccatttactttaaccaggtggcgtcggatatgctggaatgtgtgatcgcggataacggaattggcattgcacgttccaaatcattgcgcatgctgccaaagcatcatcagtcgtccggcatggaaataagccagaaccgtgcagagttgctgaacaaaatgtataatactgaaatccatatagaaattattgacagatcatctgaagatgaatcggacagcggcacgatcgttaaaatactgatcccccagttataatttagtgtatccgttaatgttacttttttatgataaaggctattataattgatgacgagagaaacagccgggacatcattgcgttaatgctcggtaaatactgccccgaaattacgattgccgacatggcctccgactgtgcggatggtatcgaaaagattaaagcgcaccgccccgaactggtatttcttgacctggaaatgcctgatggcaccggcttcgacgtactggccggcaccctacccgacattccttttgaagcagtatttgtaaccgcatttgaaaaaaagttcctgcatgtgatccgcttcagcgatgtggaactgatattgaagcctattgacaaagaaagcctgttgcaggcagtggcgctcataacagaacggattaacaccggcagcagcaaagaccgctaccgtgtattactggaaaatttcaataacagcaaaccggtagcctggcagctgttgatccctgctactaacggggaggcctatactattaatattcccgctatcgaatacctggaggtaaaaggcgataactgtatattccgtttaaactccggtaagctgattacggcagtacagtcgttccgctactatgctgatctttttacgtccctccacttctaccagatcaataacaaccagatgatccagatatccaacatcagtcacctggatggcccctcagggaaggtagtgctgaaaggcggtaccacattggatatcactgaaaaaaggcaacgcgatctgctacacaaaatggcacatcattagtcgttccgtttcgtatatcccttcccggtaattatacaatttcaatttttccggggtcatactttcgatttagttaacgatttgccaacgtttttgtgaacgtgtaagtatttcgatgggttttctttcgttttaatgtgttgcgcgaagggtacgtaacaatttcttaacaaaaaaatttggtggttttagttttggtcgtacatttgacccgcaaaacgaaatagtcaaacagtcagttttggtttgcatcatactatggcggaacaggacctgaaacgaacgatgattctggaagcggcgttaaagcgcttcaagcggtttgggttgtcgaaaactaccatggaggagatagccagggatctggaaatttcaaaaggctctttgtattattatttttcagataaagaatccatttatgtggcggtggtagagcgtatgatagccgattgttttattgacatgtcggcatatgtggaagaagcacgatgcaccgcggatatcatggatcgctacctcgcattgaaggaaaaaatgttgctggagtatcattttctgtttggtgtaaacgaatggatcaaggatgttccttccagccggatgcggcaaacgattgagttgctgcagcaggtggaaatatcttttctttcagctaccatttcaaaaggggtgagcagcggggaactcaacaaagacacggatacggaactcacggcgcagctgctggtaaatgtattattcggtttatgggtaatatggtgcaagtggcaggcagcaggttttgatccgcacgaccgggaagcgctgaaatgctttatggctcgtgaaaaacaagtactgaccattttttttaatggcttaagatatcgaccaaacatcaaccagggttgctagaacgtatgtagaagaaccaataacacaggaatagttttaatgaatatttaaatttaacgacagatgaaaaagttgattgtattggccgcagtagcactgttcggcacacaagtagcaaaggctcagttttcgaaaggcgatgtaattttaggaggtaatctgaatgttacgaccagctcacagaaagtaaaagacacagacaacaaaaccaccagcacttccttcggtatcagcccgaaagttggtgtggcactgactcctaactgggttatcggtgtatttgcaagatcagaattcagcaacgacaaaaatgttgcaggtgttaaaaccaaatcatccgatatcactccgggcgtttttgttcgtaactaccacatgatcggtgaaagcaaatttgcattcttcgctgaagccaatgccggctaccactttggtacagacaaaactgatgatacaaaaacagctacttacaacggtttctccgtgagagtattgcctggtatcacttacttcgtaagcaaacatttcatgctggaaggtgcattcggtggtctgagctacgcttacgatcagaagaaagcagaaccaacaggtgttaaaaccaacaccagcacttttaacttcgatttccctaaagaatttcaggttggtgtaaactggatattctaagcatcatatgatgttttatgtaagatagttataaggttagatagattggataatcccgccgcagtaatactgtggcgggatttttgcatttgtatggatattctcttaaaacaacctgtcatgcgaaacctaaaacttgtactgtcgctttttgcagctgccatcatttacagtggctgtgtaactactcatcccggaggtaatccacatggactaccacccggtcagcaaaaaaagatctatggcactaaatccgccaaaccatttgcacccggccagcagaaaaaacaatagccagtatcttataaaagcaaaacccgttacggacaaccgtaacgggtttttacttttataagataacctgtttctagctgttcatagagatcaggaattcttcgttgtttttggttccgcgcatatgttgcagcatgaagtgcatagattcatctgtgttcatatcaccaaggtggttgcgcaggatgtggatacgtttcagggaatctttatccagcaacaggtcatcacgacgggtagaagatgcagaaacatcgatcgccgggaagatacgtttgttagccagtttacgatccagcaacagttccatgttaccggtacctttaaattcttcaaagatcacctcgtccattttagaaccggtgtcgatcaatgcggtagccaggatggtcagtgaaccaccatgttctattttacgtgccgcaccgaagaactgctttggtttctgcatggcgttagcttccacaccaccgctcagtactttaccggaagcaggtgccacggtattgtgcgctctggcgagacgggtaatggaatccaggaggatcaccacatcatgaccgcattctaccaggcgttttgctttctgcagcgcgatggcagataccttcacgtgtttttcagctggttcatcgaaggtagaggcaatcacttctgcctttacgctgcgctccatatctgttacctcttccggacgctcatcgatcagtaccaccatcaggtaaatttccgggtgattggtagcgatggcgttggctacctccttcagtaacatggttttacctactttaggctgcgctacaatcagtccgcgttgtcctttaccaataggcgtaaacatatccatgatacgcgtggagtagttattggaggtagtggttaatctcagtttttcgaaaggaaacagtggtgtcaggtaatcgaaaggtacacggtcgcgtacttcttccggtgacttgttgttaattgtttccactttcagcaaagcaaagtacttctctccttctttaggcggacgtacagagcctttcacggtatcgccggttttgaggccgaagagtttaatctgcgacggagatacgtaaatatcatccggggaactgaggtagttataatcggaagagcggaggaaaccgtagccatcgggcatcatttccaggacaccttcacttacaataacaccatcaaattctatattgaaaactggttctttcttgttagggaagcggttcttctgtgctgcaggcgctaccgggatttctccgggtactacaaaatcgtcgtcttcatccagctcatcttctgccggaggaatcactaccacttcttcttcctcttccggatcttcgtcttctgtaaaagaagggataatgatatcatcatcatcatcgaaagtgagagaaggaatgctgtccaggtctatttcaaaatcttttattttaggtttggcagaagataccggtttctcgtcttcttcattatcttttgatttcgttccggtagctttttttgctgctggtttcttagcagccggtttttcttcagcgtgagcaggttcttcagcagcgttgtttgcttcgtctttctttacaggtttgcgtttgcgtgctttcttttcgtctccgttggattggttatcttctgaggctaatactgcttgtttatcaagaattttgtagatgaggtcctgtttgttcagtttttttgcgttgggaacgtccagtttctctgcaatatcaagcagctcaggaacgagcatgtcgttcagttgtaagatgtcgtacatcatctgtgttgtcaaattttagaagtgttgtgaggcgggtaccactgcataccaacatacaccaattacaaataattgtttttgagtcaataaatttaattagcttattaaatttgatagggaatgattgagtttaggaactgccgatgaagatggaaaaatgaacttaatcaggcagaatataccgcaagattaaaacaagttttactattatccaaaaatatttaagtgcaaattgccccaaagtggcccctaaaaccgctcttccccgggctgtatcgtactgttagccgggcgcccaaacccttgtttatactggggtagcgcctgtttaacccctcttttttaacatttcctttgcagtggcatcccggaaaaaggccggaacccgtactacctactatgaagttttccacttatttttgcagtcctaaaattatatatattatgagccaaagggtgaaagtcaagcaaatcttgtcagacgacaaggcgcattacgaagttacagttaagggttgggtgcgttcattccgcaacaaccagtttatagctttgaacgatggctccaccaataataatttacaaattgtaattaatactgaggatacggatgccgcgctgctgaagcgtatcactaccggcgcggctatcagcgccaccggcgaaattataccatccctgggtaaagggcagaaagtagaattaaaagctaccaccctggaaatactgggcgactgtgatccggaaaaatacccgctgcagctgaagaacaagcccagcctggaatacctgcgtgaaatagcgcatctgcgtttccgtactaataccttcggcgccatcttccgggtacgtcatgcactggcatttgcagtacaccgcttctttaacgatcgcggattcgtatacctgcacacgcctattatcaccgcttccgacgcagaaggcgccggtgaaatgttccgtgtaaccacgctggacatgaaaaacccgcccctgaccgaaaacggcgatattgattacaaagaagactttttcggtaaatccaccaacctcacggtttccgggcaactggaaggcgaactgggtgctatggcatttggtgatatctatacctttggcccaactttccgtgctgaaaattccaacacagcccgccacctggcggagttctggatgattgaaccggaaatggccttctatgagctggaagataatatggacctggcggaagcatttatcaagtctgttatcggatatgtacttgataacaatcgtgatgacctcgacttcctggctaaccgcctcaccgaagaagataaacaaaaaccacagcaggaacgcagtgagatgggcctgattgaaaagctcgaatttgtactgcataacgagtttgtacgtattacctacacagaagccatcgacatcctgaaaaacagcaagcataacaggaacaagaagttccagtacctgatcgaggactggggcgccgacctgcagagcgagcacgaacgctacctggtagaaaaacactttaagaaaccggtgatcttaaccgattatcctaaagagatcaagtctttctacatgaagctcaacgacgacaataaaaccgtacgggcaatggatatcctgttccccggcatcggtgaaatggtaggcggttcacagcgtgaagagagctacgataaactggtaaaacgtatggaagaaatgcacgtaccagtagaagaactaagctggtacctggatacccgccgttttggtaccgcaccacacgcagggtttggcttaggcttcgaacgcctgatgctgtttgttaccggcatgacgaacatccgcgatgtaatcgcctttccgcggaccccgaagagtgcggagttctagcgcggattttgtcttggctcaggattacgctgattatactgattacctggatttttacttttggattttataaaggattaagggagatagaagcgaattgctttttatctcccttcttcatttttatcatcttattgatcatcttaaaaaatctaaaaaataaaaatccaggtaatcagtataatcagcgtaatcctgaaccaagacaatttaaaagcgccgaaggcgccccgtatttatggaaacccgccgccgccgcatctataacaatgaaagcgctttcaaccaatttcgtttaacctaaaccgttatatatggctgaaatgaacactgctccgcaacagggtaaaaggggaacccgcagcaataaaaaatccacacgtgtagatatgacacctatggtagatctgggcttcctgctgatcaccttttttatgctcaccaccaccatggccaaacccaaaacaatggatttgattatgccaaaagacgatggggatccgatgtcgttgccggcaaaaaaagcgctgacagtaatccttggtccggacaaccgtattgcctggtatgaaggtattggcgacgatcccgttatgccgccacaggtacactatagcagctatgccaaccgcaatggtatccgggatgtgatcatggcaaagaaggctgccgtgtatgaagctttccaaaagaatgaactgatggtactgatcaaagcacaccaggcgtcgaactataaaaatgtggtggatatgatggatgaaatgctcatcaataaagtagaccgctacgccgtggtggatattaacgataaagaggccggctacttcaaatgagctatttttccctacctttatcgctccaaaacaacaattcaaaatatggcaactacccactctatcccctcagtggaccttgcagacttcacatccggagatgcagggcgaaaagcagcctttgtgcagcagttaggtaaggcttatgaagaagttggttttgtagcggtaaagaatcatgggattcctgacgatctgattgcagacctctacaaatacgtacaacaattcttccagctccccgctgacaccaaacaccagtatgaaattccggagctcgccggtcaacgcggttatacctcctttggtaaggaacacgccaaaggttatgacgcgccggacctgaaggaattttttcagtttgggcaaacggtagaggacaacgatcctatcagctctgaataccctgccaacgtacaggtggcggaagtgccggagtttacgcctaccttctttaaagcataccggggatttgagaaatccggcaggtacctgttacaggccatcgccctgttcctgggactggaggaaaactattttgatgataaaatccataacggtaattctatactaagggccatccattatccgcctattacgcaggagccaaaatcggctatccgtgcggagcagcatgaggacatcaacctcatcactttgctggtaggcgcttctgccgatggcttgcagatcctggataaacaagataactgggtaccggttacctccctgccggaacagattgtggtaaatgtgggggatatgctgcagcggttaacgaataaccgtttgaaatcaaccacacaccgggtggtaaatcctccccgcgaaatgtggaatacttcccgctattcgattcccttcttcctgcatcctaaatccaatatgaaactggatagcctggaaagctgcgttactgcagagaacccgctggcatatgagcctatcaccgccggtgagtacctggatgaacgcttacgcgaaataggcttgaaaaaataaagctattacatagcaaagtcccggtaaaattgtttaccgggactttataaatatcctgcgtataagcaagtctcttctttaacggttcttcctgatatggttattctttagatccgaacatttttcatgccggtgggtgattaacctgtctgacaaactgatacaacggacaaaaggccatattcgttataatagtcaccgatattacaagtattgtgcctttattgttttggggatttccgatattagcagcaccgttgtattttgtccggatatttgattaccttataacctgtccaatcggcatacactaaaataactgtgcttctacgtcatataccttttcttaaagctgtgctattacatagcatcactgcctacggaggcccgcagggtcatctggccatgatgatgaaaacatttgtacagcaacggaaggatgtaacggaacaggagctaatggaatacaatgctttctgccagctgcttcccggtgcttcttcttcccaaacccttaccttaatcggctataagcgcggtggcgcgatactggctattattaccctgctgatatggatttctccggcctgtttgatcatgggctccctgagtttcctgttacaatacttcggcaagaacgccctgcatacagatatctttaagtacgtacagccgatggcggtaggcttccttgcttatggcggcatccgtgctttccggatcagtattaatagtatggcaacatttgccatcatggtggtatccatgttcaccgctttcttcctgaaatcgccatggacctttcctgcgctgattatactgggtggtattgtttccaatttcagtaacaagcgtattcccggggtggcggaaaaaccacgtaaaatacagtggggcaatatctggttatttgtgtcgctgtttatcctggccggtgtcctgtctgagctggcgcgtacccatgaatggataacgcggcgtccttttaacctctttgaaaacttttaccgtttcggcagcctggtatttggcggtggcgatatcctgattgccatgatgctggaacagtatgtaacgcgcgctaaatcgcaatacctttctgcggaggaactgcttaccggcgccggtattatgcgggcgctccctggtcctaccttttccatatccgcctatgttggcggtatggccatgcggaacctgggtatgggataccagttcctgggatgtattatagcgcctatcgctatcttcctgcccagcctgttgctggtattgtttttcttcccgatctggaacaacctgaaaagatacgtggtgatataccgtgccctggaggggattaatgcggtggtggtaggcattatgtgggcagccacttttattctcttctttgtgatcccggtcaactggtacaacctgctgatcatggccagtacgctggcactgctgtgcctcacaaaggtgccctcgccctttatcgtactggcgtgcctgttattaggctggctgttatgatgcgctgatattgtattccttaattttgttgtaaagggtggttaagccgatgcccatcagttctgctgccctggttttattgcctttggcgtgggccagcacgcggataatatgtgctttctccatatctgccagtttaagggaagatgcgtcctccgcgttcccttgctggaaatcgaacggcagcacgggggtatccaggatatccgtatccgttaggatggccgctctttcaattacattacgcagttcgcggatatttcccttccagctgtgttgttgcagcgcgtgcaggaaggcgggcgtcatcccggtgatacgtttattcattttgggcgctatctgctgaagaaaccaggtagccagcaggggaatatctttccgccgttcgttcagcgagggcagggaaatctggaaggcagacagccggtagtagagatcggaacggaaatgccccgccgcaatttcctgttccagttgccggttggtagcggcgatgatccgcacatccgttttagtgggtttcgtttcccctactttataaaactcctgtgtttccagtacgcggagcattttagcctgcagctctatggccatctccccaatttcatccaggaaaatggtacccccgcgggcttcttcaaaaaaaccttttttgtcttttactgcgccggtaaaggcgccggctacatgtccgaataattcgctttcgaggatttctttaccaaaggcgctgcagttaacggcaacaaagggttgttgcttcctttgacttccctggtgtatggcctgtgcaaatacttccttaccagcgccggtttcgcccagcaggagcacggtcatatccgatggcgctactttttccgctaaagcaatagcggcgtgtatttcaggggattctcccaggatgctgccgaaattatacttgccgccgattttcttttcgaggtcgcggatgcggaattgcagatgggctttatccattgccttgctcaccagcgggaggatccggttgttatcatctcctttggtgatatagtcgaaagcgccgtttttaatggcctgtacgccatcggcgatgttaccataagcagtgagtacaatggtttcaatttcggggtacctggtgcgtatctgctgtaccagttccaccccgttgccatccggcagctttacatcagacaggatcacctgtacttcttctttctccaggatctttaaggcggaccttatattgcccgcctcatgaagtgtatatccttccagggccagcaggcggcttaaaagcttgcggagctggtcctcatcatcgattattaaaatatggcctttagacatagccatgcaaagataatagttcctatggcttccgtgatttatctgttttttggttagccttaaataccagcccgccgagtatggcggctaccacacccacaaaaagatttacaaacaatacattccccaggaaatagatccagaaatttcctttcaccgtatcctcttccaccagcgtgtgcgaaggattaccacccactaccaggtgaaatatgagcaaaaaaacagcatatatgatggtggcaataagcgtagtacgccaccccatcgtaaaggccgacgtggcagatgttttatccttatgcaccctgttgtaatggataatggaaatcagcacaccgaggaacatgataaggttaccaaaatatcccatccataaattaccgtataactttgttacataaaaaatcagggtaaaaacgatgcatattgctccaagaatgaaaccatatgccggtaatgattttgaagataaaggcttttccatgacatcagttttaaatgaacaaaatgatcaggcgtgcgcattgctttctatttcacggatcactttacgcaggtcatttttaacacttttaatatcgtgccacaagtcgccaacttcgtttatacgttccagtgagttgtggatgttaaaatcgctgatacggagcttttcgtttacctcttcccacagcagcggcatagacacggtagcaccgggtttgggacgggccgaataaggagacgccacagtctgtcccttgctgttctgcaaaaagtcgatatacacttttttattccgggcagatttggcgcgaaccacactggtgcttttcggcaactcctcattaacatgccgtgcaatatattccgcaaacagccgggtagcttcataaggatgctttgccgaagtgggcacataaatatgcaaaccggtagagccggaggttttacaaaaagaagtgatattgaaactgtccagcatgtttttgatatgcaaggccgtttccactacatacttaaagtcaatatcttccggatcaaggtccagtatcataaagtccggcttgtcgaggctgcttagcctcgacagccagggatttatttctatacacccgaggttaaccatataggccagcgtggcttcgttgttacacaccaggtaatctacatcctttccggtagaatctgcccgcagcggcacactctttatccatgccggggcctgctccaggtcgagatctttctggtaaaaagacgggcccttgatgccgttgggaaaacgatgcagcgacaggggcctgtctttcagatggggcagaatatattttgccaccgacaggtagtaatcgatcagttgtccctttgagatctgctcatccggccagtataattttgtttgattggtgagggatactttcttgctgttgagcgtgagggtgcgttctttttcaatagtagtagccatatttatcttttttgctgtttcaggatgtacttcttttgccggcttgtcttcccgcaggccgaggaaaaccggttgccgcagatgtccgtcgccggtccattcctggaatttcacttcacacaccagttccggctttacccaggtaaccggcatattggtacccaccttttcggagaagggtgacgttttagtgattaacggctgcagctgcgtgtatagctgcgcgatagtggcttcatttaatccacctccacagtgcccgatatattttagttttttgttttcatacattcccagcaccagggcgcctatttgtttccggctgcctcggggcgcggtataaccgcagatcaaggcttcctgctcgttcacaatttttattttcagccatgccattcctcttctgccctcttcatacacactgtctgcttttttcgcgatgatgccctcccactctcgtgtacgggctttctcaaaaaagtttattccttttttaagcacgtgcggggaaaaacggatggttttatcatttaactccgttatcacatctttcagcaggcttttccgttccagcaggctcaggtgctgcaattcattcccatccagatgaagcaggtcgaataccacatataccagttttcccttacctgtagtcctgtagttttgcagcgtttgaaaatgggatttgcccttattatccagtacaataatttctccgtccagcaccacattatgcgaaattttctccacggcagccactaccgcgggatagtcttcattaaaagacttctcattgcgggaatacaaatttgcctgatggttttccacgctggcaatggcccggtagccatcccacttggtttcaaagagccagtctttgccatcaaacggttcactgacaagggttgtcagcattggtttatatactttttttattttccgggcggcgcggggtgttttatttttcacttcaacgccggctactgctgattttttttttgccaccttcgtggcagctttgtttttttcaccctgtgcttttattctttccggcgtatagtcttcgctgttatattcatcaacggcgtatttatctttgtgtttgatcagcagccaggcattttcttcgcggcctttcatctttaccagtgcaaattctccttttagcttctttcccttcattacaattttcagatcgccggatttcagctcccggagggcttctttatcaaaacttttcccatcgggattcatcagctcaaaggtgcctttgtcccagatgtacacggtacctgcaccgtaattccctgcgggaatggtgccttcaaaatccttgtaatcgtagggatgatcttccacttccattgccagccgtttatctgccggattcatggatggtccttttggtattgcccagctttttagcacgccatccacttccagcctgaaatcatagtgcagccgggaagcatgatgccgctgtaccacgaaaatgtgtttccctgccaccggcttacctgtagcaggttcagtagtttccgtgaagtttcgtttctttttatattccgacaaactcatgatgcgcgttttttggtggccggtttacctccgaggctggctttcagctgatcgaacaggttatcgctcttggtgtgcaccacgcgcattttcttcaccaccggctttttaccaccggctttggcctttataattttcaggagttctgccttgtattcatctttatactgactgatatcaaattcggtggtgtattgttttaccagttctatggccatatccagctctttcttagccagttttacatgcgttggcagggtaaggtcctcagcggaacggatttcttccgcaaagcggagttgttgcaacagcaggtaattttcccgtggccggatcacggccaggtgttcctggctgcgcagtacaaaccggctgatgcctgctttacccgttttctcgagggtttgctgcagcagggcgtatgctttttcgcctcctttggcgggttcaatgaaataaggattttcaaaatagatatcgtcgatctctgtttcttccacaaaagactctatttcgatgattttacttttcttaggactggctgcttcaaaatcttcatcttccaggataacatactcatctttatacagatagccctttacgatctgctcccagggcacttctttacctgtattttcattgatgcgctggtatttgatgtgcgccccgtttttgctgtccagcatgtccaggtccaggcggctgtcctgggtagcgctgaatagttttaccgggatgtttaccaacccgaatcctatggatcctgaccatatagctcgcataaaatgatagttttggtattaaataaaagttaacacaaatggtaccatgatcttaaaacatcgcggcataacttttggttttttaggtttaactaaaacctttatttatggaaaagccaggcgaaatgacaactttatcaagggtattggaaaagctgcatgaaaaaggatttgatcacgagttaaagatgagtgatcatggcaggttgcagaatacggatgagcagaaaatctataacccggaagacctgactatcattaaaacctatcgttttgagggagagtcagatccttcagattcctcgattttatatgtaatggaagaccaggaaggcaataagggctatatactggatgcgtatggcgcttacagttcacacgaagaggcaggttttgacgaatttatccagaagatcaaagtagaagacagagaagatcagctgatatttgggtagcccgctatgcaggcgcctttacctgctaccggcttccttcagaaattgcatgagtaacttttcatccgcatgtaacccgccactggcgggtttattgcgtttagcccgtagctgttgcagccagggttccagttccccgttttcgtagctgttgaggatttgcggatgaatgtaatattttttgcacacggcgcgggtattccccaatttgcccgccacaccgtctattatcgctacaatgttccggcggcattccgtaatggattcaaagggtgtaaggtctgccagcaaatttaatgcgtttacggtacctgcccaggtacggaagtctttacaggtaaattcattgtcggcgcagcactgttttatatactcatttacttccccggagtcgaggcctctatgttcgccgttttcatcgtaatattgaaacaatacctgcccgggaatatcctgcactttttttagcagctttgcgagtgcagcgtcatgaagttctattttatgctccactcctttttttccgcggaaccggaaaaaagcggtgttgccattgatcttcacatgcttatcccgcagggtggtaaggccatgcgagccgtacagcctttcataggaggcgttgcctacccggatcagcgtttcctccatcaccgatagggcaatagcaataactttatctttatccagcgagggccgtttcagatcttcgtttatacgtttccgtattcccggtaacgcctctccaaattgcaggaggcggtagtatttggtttcgttgcgggctttgccccagtcgagatgataccggtactgtttacgtccttttacatcggtgccggtggcctgcaggtggccattggcccaggtacagatccacacgttttcccaggcgggaggcagcaccagtttccggatgcgatccagcacttcggggtctttcactgttttgccgtctcggtcgaggtagatgaagtctttccctttgcggacgcgtgaataccctggtgcatctgcttttacgtaccgaagcttcactgatttggctacggctacggggtctgttatcaggtctatgctaaccatttacaatctcccctccattgggatgcaggatctgaccggtgagataactggcgtcatcgctggccaggaatacgtagcagggggctacttccacgggttggccggcgcgtttcagcggtacatctgttccaaactttgctacttcctccggggtaaaagtggcggggatgagcggggtccagataggacccggggccacgccatttacccggattcctttttcagacaaggaggcggataaagaccttacaaaagaaacgatggctcctttggtggaactataatcgataagatgactgctgccgcggtaagccgttacggaagtggtacaaatgatacttccgcctttgggaatatacggcagcgctgctttggtgagataaaagtgagggtaaatattagtttcgaaagttttatgcagctgggcagcactgatatcttcgatacttttctgcgggtattgtacagccgcattgtttaccaggatatctatcttcttaaacttctttattactttcttaataatatcattgcaatgcttttcattgctgatatcgccggcaatgagcatacattcgcggcctgcgagggtaatgtgttcgcaggtggtttcagcgtctgtatgttcgttaaaataggcaatggctacatctgcgccttctttggcaaaagctacggctactgcccggccaatgccgctgtcgccgccggtaataagggctaccttattgtacagtttgcctttttttgcgttgtctttttcaaacaccggggcaggactcatgacctcttccagtccgggttgtacggattgtttcctggcgggccttactggttttttgggattggatttttgcatagtatcaggttaaaaaaagtccctgtgtatgcagggacttttgcagtttccattaacaattatacaaatgatcgttaacctattcagctgcagcttcctcgtttacagtagtttcagctacttctgtgagcaggctgtcagcgttcttttcttcttttaaagtttgctccagtaatttaactacctgtgagtgtcccattacattggccagcgtacgtaagctgccgtaggcagaaatttcgtagtgctcaattttctgggaggcaatgatgataccggcatctctcacggcagtatcggcatcggtatctgctaccacttcctgtccttcagctatcagaccttccatggcctcacattttttagcctgtggttttttaccaagtatttcaaatacctgttccaggcgggctacatgttctttggtttcttccaaatggttgccgatacattcgctcaattcttccgaggtagcagctttctgcattttgggcaatgcttttaccaggtttttttctgcccagtagatgtctttcagttcgtccataaacagttcatggaatttggactccggcattttttcactgcctgcttttcttgcggtgccgttgccggcggatttagtggtaggcattgtaacagattttttttagatgaaagaatggttaatgtttatcaggtgattgtcttttaaaagcttcttcttttccctctatagcctgcggattagcgggggtatgaggtgtatccctgtccggtatttcctgcgggatgggttcaatttccggcttgtttggcggcggttgaaccggtgttgggttttcttttcccggctcttgtttatctggagttggatcaggaatcggctgtttatttctatccggattattcataactcacaattttattggttaagaactattgttagttatccaaagttcattccactaactgaacaggttatttttgcccgggaaacaactttctaaaacccgctacagaacagcgtttaaaggcacccgtatctctgcggtaatagtgagacaggtgtgcttacattgcttgtagaatttaccggcattctgtggaatatgttgctcagaaagaccttcacggaaaaaggatattttttagtagcgaaattcaggcagaaatagtaacttgaaatgctttctcaagatctcatacatacagatgcatttttcagtacacaagaaaatccgactcgggtttttcattgcatttaccgttatcgtggcggcctcggtattttcgtacctggtggcaaagaacctgctggacaatgccggcaggcttaatcacgccattgaagtttccaaacggctggaggtaattacccggcaactcaaggaggcggaagccgccatcaggggatatgcccttacaaaagacagcgccttcctggatcccagtatgcaggaacgcagcaacaggattgagcgggaatacctcctgctccggcaaataaccaacgataacccggttcagcaaagacacctggataccctccgtaggctgctggccatcaaataccagcaactgcaactgggcggagaaaattccacccagctgaaacagctctccgatgttaaggaaggcgaaaagtccatggatctcatcgacaataaggtgcgtgacatgatccggattgaagaaagcctggtacaggagaaatcggaactgtttcatttcttctcggtgatgtgggtgcccatgatctttatatcctcgctggtagccatcctgataggtatctactcttatatcaccctcaccagggaattcaaactgcagctgcatattgaaagccggatgaaatcctatcagcgtgatctgcaacaaaatatctccctcctgaataaaaccaaccaggagctggagcagtttgcctatgtggcctcgcatgacctgcaggagccgttacgcaagatatcgaccttcagtgaccggctgcagatgaaatataaagaccagctgccgccggatgccacgcagctgatagaccgtatggtgtcggccgtttcccggatgcgggtactgatcaatgacctgctcatcttttccagggccggccgcattaccccggaaagcatcacccccgtggacatgaccaaactcctgcaggaagtgatcagcgacctggaagtgacccttgaagagaagaacgtgcagatcaaatacgaccagctgccggtaatagaaggcagcgacacttcttttcaccagctgttccagaacctgctggccaattctattaagtttgccagcccggacaggcgcctcgaaatcaatatccatcacgaggtagtaaccgggaaggaattgggcattgtaaaagaaagccggtggaacgattcttactgccgtatcagcctggacgacaatggtattggatttgagcaggcttatgccgaccggatttttctcattttccaacggctacatggcatcagcgagtattccggcacagggatcggactggccatctgcaaaaaaattgtagacagccacaatggcttcatacaagcccacggagacccggggaaaggcgcgtcttttgttattatcctgcccctgcgacagagaaaccggaatgatgaatctgcggagcaataaaggttagcacctttattgctgtgaattttgtcacaaattgcaaaactcctaatctattgcgatgagcgagcgcccgatacacattttaatgatagacgatgatgaagacgatttctttctcgtaacagaattactgcatgatatttcacccggccaatatgtgcttgaatgggcttctacctatcagaagggactggctgccatagaagacaatacgcacgacgtattcctggtagattaccggctggggcctaatacgggtattgatatccttcgcagactgcatcagatgcatcatcagccgccggtaattatgcttaccggtaaaggcgattataatatcgaccgggaagcgatgcaggcaggcgcctacgattatttggtgaagggagaaatgaccgccgacctgctggaaagatccatccggtacgcgctcgatgaatttaaccatcgccggtctattgaggaaagtgagaagaaatactatggcattttcgaaaaagcacatgacctgattgtgctggccgattgtgaccggaatattattgatgccaatcccgccgcattaagaacccttcaatacagccgggaagagattctaaaactgcatctgcgggacctcttcatctccaaagaccagagtgagaatttcctgaataatatctgcaacagcggcattgctaatttacaggaatatgattttaaaactgccgacaacaaaaaaatggtggtgctgatcaatgctgtaatgctggacgaagcagcacagatattcctctgtgtaatccaggatatcactgataaaaagagggaagaacaggagaaacaacaccaggaaaaatttgtgatcaccggacgtattgccagggtgatagcgcatgaagtaagaaacccgctcaccaatatactgctggcggtaagtcagtttaaggaagaagaggaagtggtggccaacgatgatacactgatgtatacagacatcattgaacggaattgcacacgtattaaccaattgattacggaactgctgcacagcacccgtatgattgaactccacatggaacctgtggggattaataacctgatagagaaagcgctgcagctatccgcggaccgtttgaaactgagtgaaatccgtgtagaaaaaaacctcgtatcgccggatgtgatcattaatgcagatgaagaaaaagtggtgattgccttactgaatattgttatcaacgctattgaggcgatggtgccggggaaaggcatactcaccattaccactatgcgtaaccaggataaggcaaaactgatgatccgcgacaatggcactggcataccggaagaaaaactggcgcgtttgtttgatcctttctataccagtaagtcgaaaggcaccggtcttgggttgaccagcacgcagaacattttactaaatcacaaaggaactatacatgtagatagtgagcccggaaagggagcggtatttacgattgcaatacccgctatcgtataaatttattccctgggagatggctctcccagggaataaacatttgtttgatcaataatttatattcagcaaccgtaatttattatacagggttttacggtcgatattcaatacctgtgctgcttttgttttattatacttcacttctttcagcacatttataatcttattgtattctgcctggagggccactgtttttaggtcattgtcgttggaaagaagcgccagttcaccggaaacgtgtacttcttccgggatctggttaaatgattctttcatttccagcggtaaggcaatcatggtaatatcttccatttccggcgtaagcaaacaggctctccggatcacatttttcagttcacggatattaccaggccagttgtattgctggaagcaatcccatacttcagaagaaattttaccgcatgatttatccagttccctttccacctggtctacaaaggcggtagtgaacagtggcaggtcttcgcggcgttccctcaaaggcggaatataaatggtgaactcattgaggcgatggaacaggtcttccctgaacttaccgcgctgtactgattcagagagcttttcgttggaggctacaatgatacgtacgtcgatcggtatttccttcaggcttcctacccggcgaattaccttttcctgtagcacgcgtaacagggccacctgtatgtcatatgataaattggagatttcatccaggaacagggtaccaccctgggcctgttcaaaagcgcctattttggtattgatagcgccggtaaaagagcctttttcatgaccgaataattcacttgccgccaattctttggagaggctgccgcaatccagcgcaacaaaaggctggtgatttcttttactgtgatggtgaataagatgggccacggattccttaccagtaccggtttctccgaaaatgataacgctgtagtctgtgggcgccaccagtttgatttgtcttattaattctttcgcaccttcgctttcaccgtatacatatttattgttcttatcgtcctggttacgggacagtaatgtttcccggacttcttcgggttcactgcccgactccactggcctggatgcgcgtctttcctgttccgcctctttatgggcgaaggctttatgtaccaggttgagaatttcatccgggtacagtggtttggaaagataatcgtatgcgccatttttcaccatttccacagctactcttacatctgtgtaacctgtaataatgataacaatggttgaaggattgatttgatggatatcctgcagcagttgtgcaccatctgtatctttcagccggtaatcacagagtacgaggtcataggttttttctttcatcattttaagtgcagcaccacctgtcatggtggtatctacatcaaaaccatgtttcccgagaaatttactcaggagtgtacagatattaatttcgtcgtctattattagaatatttttcatacttctttaatatagtggtgattggcaacagaatagctggttaaaattactgattataaccaatcgggcgttatcagctttttattttgatactatcgatcagttcatcaacatttttgagactgaaaggtttagccaggaaaaaagcggctccggctttcagtgctgtttgcttttccatcgcattgtcataggcgctgatagtgattacaggtaacgtaggacaacgttccttgatcaccggcaaagcctcgagtcccgatccgtcgggcaggtggatgtccagaaaaaggagatcaggctgatgtttgaaaatggacttcatgcccgcctccagttcatgtacgtattttacattatagccatgacgtacaagcgtaagttgcaataatctgcatatatccggttcatcatctataatcaatatgctgggatatttcatgttattctcagttgtagccaagtctgactggtgccaggctgttttgtttcggtgtaacatacttatgtttattccattgttccattaatagtctggcaatcaggtaacatacagttgactcggcgccctgattctggtttatgttatttttttccagtccgtcgtagcaaccgtaagttaatggattataaacaagttgtttcaggtgattattccctaaataccaactgaatgccaaacgcatcttttccagatatgatttattttttgtggtgttataaaacgtattcaaagccagcatggtataggctacttctatagattgttcgccaccgtcttcctgttgctgggtgttattcctgtggtaccacgttttattgctgatcaccttcatatggctgtctgtaaaggttttgctgcagaggaaagccaggctgttttccgcggttctgcggtaagcgtctatcccgcttacctggtaggccatcatcattgcctcaggcaatacggcattaccgtaggtgaggtaggattcgtaccaatgccaggtttcatctgcttcctgtttgtaatggtcgtacaattttgcagccagatgttgcaaaatttccactgctttgccaccgggtttataagaaaggtaataatacagccctttgatggtgaatgccatcgccctgggtgattgcagtgattccatccagttgaagcatttgctgaatatggcggatacgtcttgcacggcgtcaaagggcaggtgatgctgcgaagcgagggcataccccagcgcccagaccgcgcgtccattggcgtcttccaggtttacttcctcattcattttattgaactggcggtcgatatccacataattaaggaatttcccggaaggctgctgacagtaagcgataaagtcgatgtacttacgggtcagcgagttaacgaagctgctggaatttaattcgctgctgtacatgcaggtagcaataagcgcccgtgcgttgtcgtccagcgtatatccgaatgcaggatcggggatgtcatgtttggaaaactgcagcataccgatttcatcggtcatacgatcgatgtgatcgaggtatggtggcggcaggttgggcaggatcttgtcttctgccagtgcttcgctgattacgctcatatgtgcgatggctacgttttcccagatggagctgcgtgttttttcgatggccgactggctcatctgtgcgcgcagttccggattgccgagcagcggtattgcgcaggcagcaatttgttccgggttattgaaatctaccaggcaaccggcgccgtcttccagcatttcgcgtgcctgtacaaatgaggtggagatcaccgcgcaaccggcgctcatggcgtaaacgaaagttccgcttactgcctggtgcgggtcttttgacgtaaaaaggtaaatatctgtaagagataaataatcgagtaatgttttcagggagagataattatttacgaatcgtacattgttttccaggccgagttcctgtaccagttgttccagtgactcgcggtatttttctccttcacgggagcatactacgggatgggttttcccgagcaccaggtaaatagcgttgggatactgttttacaatatccttcatggccctgatgcctgtttcgatgcctttgttttcactgagcaaaccaaatgtgctcagcaccatcctgccttccacgttgtattgttttttcagtgcatccacatcttccacgatatgcgcgtgtgtaccgtgtggtatatgcacaatcttttcggcgggcacatgatatacctgctgcagtaaggtggcagaggagcgtgtcattacaatcacttttgcggcgagtgcactgatcaggcttactaccttggtgcatttatgatcaggataaggcagtacggtatggaaacgtaccacgaaaggtttatccagtaaggaaagcatggccaggaggttatgaccgtattctccgccatacaggccaaattcgtgttcaaaacaaaccaggtctattttgtcgttctcatttattttctgtgcaaaatcaatacatgcatcaatatcgaacgggttcaccgaataagtaacgggtgtttctttcatattggcaggtttgcctgcttcttccagtgctgccacctcaatattcagattaccggcaaaattcttattcattgcgtttaccaggtcctgtgcgaaagttgcaattccacattcccggggcgggtaagaagtaacaaaaagcaaggttctaatcttcatggtaaaaattttatactacgcagttaacaagtaaccaggtcctcaattttccagatcgggacataggatgtttcaaatatcaatccaatgcctgctgtattaggtttcaggggattcagctatccggaagtgtagaaataactctacacatattgtcccgtatccacaggtaggaggtgtggataaaataaaggcggaccatttacatttgattaacagtcattataatcataattgtttataattgtattacaatttgcccgaaatagtggtaattagggatacaaatagcaacattattatcgtaattggtaatcaataatgtttctttgtccatttcagcttattttagctgaagtaagcacccaagctaccatgtgaagcgcaaattttaaccattccattttctcatttaaacccaatcgccgttatgcgaaacattgcatgtacatttaatgtagatggtgttccaaccaaaatcagtttgaggaaactcccacggcaaaggcgctttcaagccattattgaccgtaatatcacggaatatatcatctcggacgagaccaatgagattgagtattacgagggaccggtgttaagcgagtatcttttcacccggattgccagtcttattaagcagtatttcccgaatgtgcgggcaattatgaagatcggggaagataattatgaggactacgatgatttttaggcgactggcaaacggctgttagcctgggaagactaacagccggccattttatataaatcctttttcaagggacaggaacgcctctgaaggatgcacctgctgccataagatagcatatacggcctgggcaaccggcatatacgcccctatattcctgttcatttcatgcatacatttactggcgtaataaccttctgcgatcatattcagttccagctgggccgcttttacactgtaccctttcccgatcatattaccaaaagtacggttacggctatgcagtgaatagcaggtaaccaacagatcgcccaggtaagcgctggcgctgtaattatgcactaccggctccgttccggccaccgccgctttctgttcttcatatttttcgaggaaactttgcatttcccggaaacagttggtaataaatacgctgaggaagttatctccatactcctgcccgtgtgcaataccggcgcccatggcgtaaatatttttaagtaccgccgccaactgtacgccaatcacatcggtgtttacaattgtttgcaggtaactgccggtaaatttatcggcaatggactgggtagtgtccaggtgagcgccggagaaggtaaggtaagacagcttttcgctggctacttcttctgcatggcaagggcctgtaatcgtgaaataccggcttgccggtaaattgaattgtttgagaagatattctcctatcaggtcgttggtacttggtaccagccctttaatagcagaaatgacctttttattgatcaatgcatcggcgggtaataagcccaacacatcttccaaaaaggcacttggaacagccagcaccagctcatcgcaggccgccactactgcttttacatcactactgaggctcagcaggctggtatcgaaatatacggaggtgagataatgtttattatgatgacgcagctgcatatgacgtatggtgtcttcattccttatccaccaatgtatatgatgcccgttatctgtcaggatcttagccagtgcagtagcccagctgccactgcctataattccaatgctcttgctcacaatgcaaatttttatgcaatgtaattaaaaagcaataaagccgttttgcgggcgcggaggttgtcttactcaggattacgctgattttgctgattaccacgatttttattctttttctcttggagatgggataattaaagaagtgagggaaaatgatgtacgtgatgctttgcagttgcttttaacatgctttggagatactatggagatactttgaacatgtctttaatgtggagataacatggagctgatgtggaggtgacgtggacttgatcggtaagatggtggtagtcagtttgttgcacagggttttggtgtgctgcttagacgcgcttcgaggaaattcgtattatatatcaatgttttatacatttttcaaagataaaactgatcagcgaaaacaccaaaaaaagaggtcgtttttctatgttgaaaaacgacctctttttttatatgaagttgtgtaactgcgttattttgcctgcccttcaaacagttcggccttcggtactacttttacttttttgccattttcgagggtacgtgagatggcggtataaggagcgctgatcacctggtcgccggctttcaggccggaagtgatctggatccaggcgtcgtcctgtacgccggttttaacgggtaccattttaacggtaccatctttctgcagtataaataccacctcgttcagcacgggtttggtatcggcagaagaaccgggggtagtattatcctgtaccggcgccgctttctttttgtcgtcctttcctttggtagaatcggcgtcgcgggtagttacggagttaattgggatggccagtacattatttacatgcctggtttgaatatccacactggcactcataccagggcggaagggatacgttttcttgtttttatcaagaagatcctggtagctttcctgcaggatgcggatatgtacaatgtagctggttacctgctctgcggaggatgcagtgcttaccgtagcggtggcggcgcctttgctggagctggcaatttgtgttacaatacctttaaactcccggctgttatacgcatccacttcaataatggcggtatcgccgtattttacttttggaatatcgttttcgcctacgtctacctgtacttccatggtgttcatatcagcgatacgcagcatttcggtaccggtcatttgtgcagtacccaccacgcgttctcctttctttacagacagcagggaaacgataccgcccatgggagcggaaatggtggtacgacccaggtttttattggcttcattcaggttggcctgcgcactggcaacggcaaacttgtttccgttgatctgttgcacagccgcgttataatctgccagggaggcgagataagttgcttcggctgtttcaaactctgatttggagattactttctgggcaaggagttctttgttcctgttgtaggcagccttgttttgatcaagacgggccttaaaggagttcagcgccgcagcggagttggccagctgcgcctgcgactggctcatggaggccgccgctttatctaccatcgatccgtagatatctgcgtatatacgtgccagtacctgtcctttttttacggagtcgccttccaggatgggaaggtctgtgatttcgccggaaacgtcggagcttacttttacttctatttcaggataaattttaccgctggcggtaactacttctataatatttctattagaagcattgtctacagcaactttaagtccttcttccttaccaattaccccggccgctttaagcaccaggaacaaaataacgagtgaacaaagtatgcctatgaaccagtaaagttgtttcttcttcataaagcaatttaatttcccggaacggctacagtgatattttctgatcccggtagaattccagcaatttcattttaaatatgtaatcgtattgagcaagcaccttgtttacctgcgcattgtacaatttactttgcgttgtgatataatcaatggtgttcattaatccgaggttgaagcgtttggtggcaaaatcatacgctttctgggctgccattacgcctgtggcagatgcattatatttctgtaaggccgctattgcattggcatgggcggtataaatatcctgccggagtttctggtgatccaggtcgcggatcagttcctggctgtatacatttattttagccctggctacagtggtacgttgctgccagccattaaaaataggtatgttaagcgttaatccaatatttttccggtaggtgttgctgatctgatcatgaaacggcagcacctttgtttgcgcaatatcctcgtaatagttattggcgtagtaggtactgaggccgccgcttatgctcaggttgggatacaactgcgctttggccgcctggtatgctttggcggcgctctggatcttcagttcatccgattttaccagcgggtagttggttaaagcggcgctgtacaccatttccggcgccatttcctgcaaggcagataatggcagggaagaaatattttcaggtacatccggtttaaaggggatctcaaatccgaggttgagataagccttcatctggagaatggccagggtcacgttgttctgggcggttacgaggttactgctgtccagtgccagttgcgcttccaggtcggcctggttgctttccggtacggaacctgcgataaccagtttcttggtattatccaggttggaattggtcagccggacgttttcttcgtttactttctctgtttgaatattgagcagtatctgcaggaaagcagtggccacgttaaacgcgaggtcattcctggctttttccagcaggaagctattggcctgtgcatccagtttgttggcggcaattgttttttgctgataaaaccagctaaaaaggttcgcctgcatattcaggttaccactggagttaaacacggtttggttaacatactggttatctcccaggctggcgcttctaccatccgtataccctcctgttactgacccgctgaaaccggggatcatttgcaggcggctttgctgtaaagtgagatctgccaggcgtttttgaacttcctgttgtttaactgtcaggttattttgcaaggcataatccacacaacgttgtaaactccacgtatcctgcgcatcagcggatgttatgttagcaaacaataaaatcaggattactcctgctattcgggatattctcataacattccaaaaatataataattgtgatgatacttttccacccttcttgatagaaggcaaaaatttagtaggtatggcagtatacctcactaattgagtgtacaacataatcttttttttacaaattcttaaaactgatccgcctttcttatggctgaatatgtccatcgcggatctggataacgcggttgccataggtggcattcacgtctgagtgggttacctgcacgattgtaattttatcttgttcattcaggtgtttaaacagctgcatgatcactttcgcctgatcggagtgcaggttaccggtgggttcatcggccaggatcacccggggttcggccacaatagcgcgggcaatacctaccagttgctgctgtccgccggatagctggttgggaaacaggtcttttttagctaccatattaaagcggtccagtacatctgccacccggctctttctttctgaagctggaatgttcttgtacagtaacggcgtttcaatattttcgtacacggttaattcgtcaatcaggtgataggcctggaacacaaatccaatggaaccccggtgcaactgggtcctttttttctcgttcatcctgtccacacgctctccttcaaacaggtattgtccttcggatggttcttccagtaaacccataatatgcagcaaggtagatttcccggaaccggagggccccataatagatacaaactcgccttcattgatagtgaggtcgatatctttcaggatataattttttccgaatccaaccgggtaatgcctggaaattttctgcaattgtatcatgatcggtaatttgtttttaatttatgttgatattttctgcatatcggctcagcaatataattaaaagtagctgctccggttatccagattagtttattctgatctcaggcttttaaccgggttcattaatgccgccttcactgactgcaaactcacggtgagcaaagcgattacaatggcgatagtgcctgccaggagaaaggtgcctgcatgtaaacgggtgtgataggcaaagccttccagccattgatgcatagcataccaggcaaacggggaagcaatacaaagcgatatcagcaccagcttaataaaatctttcgacagcaacgccactacactggtggccgaagcgcccaacaccttgcggatacccacttcgcgggtacgctgttctgcagtaaacgcagccagccccagtaaaccaagacaggaaacaaggataataacaatagaaaaggttgataaaatggtaccggttctgaattccgatttatataatccgttaaagtcttcgtccataaaatgatatccgaaaggcacagcgggcaggtattccttccagatcctttctatccctgctatcacctgctgctggttatctcctgaagttttgataagcacttccccgaaccattcatattccgggaaaacaacaataggttcaattttggttttcatagaagcgaagtgaaagtccttcatcacccctttgatggttcctgcgcggccattcatcaccatgcgttttccaactgccgtttcagccgtccagcccagctgctttatggcggtttcgttgagcaggaaatgatatacccggtctttatcttcctttaaaatatcctgtacatcggcgtcggttaagtttgcaccggccagcaatgaaattcccattgtttgcaggtaatctttctccacggggatcgcggtaatattcatactgtaatccgccggtttcccttccaggttaccaatagtgtagccaccgcccaccgataccggtgagtcgtacgaggcgctgacatatttgatacctgactgctgcaacagcctgcccttgaaggcttccagcatctgccggttaaaattttctcctgataataccaacacctgcgacctgtccagtcctaatttcttttgctgaatatattttagctggttgctcaccaccaatgtgcagatgataaagaacacggaagcggcaaactggaatacgacgaggcttttacggatgctgccacctgaagtgtgcatgacccgtccctttaatacctgtaccggccggaagcccgacaggaacaaggccggataggtacctgcaaaaaaggtggtacaaagaaaaacacccgccagccacaggtagatgtgatagctgtccagtccgagcttcagggtaacgccggccatattgttaaataccggcagtaataccaacgcaatcattattcccagcaccacagcgcagaagctgatcagcgtagactcggcaatgaactgccagaacagctgcccgcgcacggcgcccagggctttccgcacaccgatttcacggcctctttccgcggaacgggccgtggcgaggttcataaagttgatacatgcaatcagcagcaatagcgcggctatgatggtaagaatataattatagcggatatccccgccagcttctgttgaattaagggcaatagaatggagatgaattcccggtacggactccggcacaaaatcaagcgtaacgccactcctggtaacactccccatctgttcttttatcaggttctgtaacctcccgtgcagcgcgccggtagtggctttgccggccatctgtacgtaggtgtaatcattggctgaattccaggtgtcttgcctacccagcgaggcataactggctacaaaatcaaacttcaggtgggtgttcgcaggagcatctatggctacaccggttacctggtattcatttttgttattaatcttcagtgttttgcctactatatccgtggtgccaaaatacttcctggccattgtttcagatagtaccaccatattgggcccgctcaaaacagtggctgcatttcctgctatcagcgggaaagaaaacatgttgaaaaaagcaggatctgcataaagaaaccccttctcgttcattaccttgtcgccataagccaccgtagtagctgaaggataggccctggagatgtatttcacctccggaaaatccttcatcaccggcgccagtccgctcggggtgagggcggtatgggttacttcctggtctttctcgccatagtcgaagcggatacgatataattccgtggcatgtgcatggaagttatcgtaggtccattcattccttaaatacagcgccagcagtatgaaacaggcaatgcccgcagacagaccggtgatattgatcgccgaatacagtttacgtttcttcagatttcttaaagctgttttcagataattacgccacatcataggtgatattttaatattaatcccttgttaaactgtttaccgggtttgccagcgcggctttcacggattgcaggctcacggttaagaatgcgatacataccgccatcagccctgctgccccgaatacccaccagtgaatggtggtatggtattcaaagccttccagccattgatgcatgaaataccaggctgccggggcggctattaatacggctacgagtaccaggcgaagaaaatctttcgataacagcatcacaattccactcactgatgcgcccagtactttacggatcccgatttcttttttgcggtgtgccatcaccagtactgcaatagcaaataatcccatgcaggaaatgataacggcgagtaccgccccgctcataaatatctttgaaaagcgttgttcctgtgtatatagccgttgtgcattttcatcgaggaaagaaggatcactttctgacagctcattaattcccttccagagtgcagtgatctttttcagtgatgccaccgggttggatgtttctactttaacgaagatataattcaggggagcgttcatgatcatcaccagcggactgattttcttatgtaatgattcaaagtgataatctttcaccatgccgatgacgtgcaacggcggctcgtcctcgctcatgcggaagcttacgcctataggatcagttacgcctaattgtttcgccatcagttcattgatcaccacagcgttactgtctgttccatactcccgggagaaatcgcggccggataatattttcaggtccagtgttttggcgtagtcgtaatctactgcgaggcattgcgtggaaacatggcgatctttatacataaagcccctggtccagttgccggaagacccgtcctttcccaggccgaggtttaacatgctgccactcacgcttcttacttcgctcagctctgtgagcctgtttttcatggaagtgatatcagacggcgtagcattatcaagcgggatgctgatcacctgggatgagttgtatcctaacggggccgactgtatgaaattaagctgttgccagatgatggaggtacagctgatcagcaccactgctaccataaactgtactataataagcccgttgcgcaccccgctgcttttacccatacccagcttgcctttcagcacctccaggatattgagtcgcgctactttccaggcgggataaccacctgccagtaatgtgatcacgaagaaaccggcaatggcgccggctaacacccaaatattacggaagatgcccaatgcaatatgatgcccaaacacctggttgtaataaggcagcagcaggatcatcaggcccaggctcagtaccagtgcaaagcagcacaggagaaaagcttctgcccagaactgcagcagcagctggccattttgtgcacccagcgatttccgcaatcctatctcaccgctgcgggcaaaggatctggcaatggaaaggtttataaaattgatagcggctatactgatgatcagcgtagcaaggatgatcatcagccagggataaaatttattcaggccactgtaaaaagtactctctgcattgaggtgaaaatctttcagcggcaatcctttcaggtaaaacacatttttaacgccacccgcattcttctgaaggtcttctatcttccctttataatatttgttcaccaccacactcatatttttctcgaaagaagttttactgacgccaggttccaactgaacaaacagtggaaaattagaggcgctccaatcgtttttggtgatgttatactccggttcattctcaaatcgtgtgagtaattcgaagcccattccagaattatcggggatatctgctgctattgcgcttacaatgaaaggctgccatttaccacccaggttcagttccaccgtttggcctaccggatcggtatctttaaacagtatgccggaagcgcgttttgtgagcaccacctggttcaactgctgcagtgcgctattcttatctccctttagcagtggaaaggtgaacatcttcagaaaatccttgtctaccatttgcgcacccaggtaatagtggttggtaccatatcttacaggcacgttatacccggctataaaagtggtatactttacgcccggtacttctttctgcaaagctactgccagtggcttcgacatactggcgcctgtttttacctggcctccggtatcttccacgccaatcagctggtatatatcttccccatttttatgaaaattatcgtaagtccattcccggtatgcggtaagagacaaaagcaatgcagcacataatgcggtactcattcccacgatgttaaccgcagcgaacactttctgtttccgcaaattcctccaggcaatttttaaatagctctttaacatacggttatatttaaagtgataaaaataaaagcagggcgtgtagacacacactctgatttgctgttcacttgttattcaatttttaatgcgtttaccgggttcccgacggcggcttttacggtttgcaggccgatggccagtaacgctgttgttacggcgataatggcagccaatataaacatccagggttgcagatcgatgcggaaagcaaattgctgtaaccattgctgcatcaggtaccacgccaccggtgaggcaatcactaatgcgatcactactaaccggataaattctttcgacagtaaggtggtaatctgcgccacactggcgcccaatactttacgcacgccaatttcgcgtgtacgctgctcagccgaaaaggctgccagtcccagtaatcccagtgccgatatcagcacggtgagtaccgtaaaccagccaaagatcccggccaaccggtcttccgcagtatacaacctgccaaatgcttcatccaggaaggtatattcaaaaggttcctgcatatcatacgcagcatatatcttttgtattttcgccatcagggcaggcatattctgttttggcgccacttttacaaacatgcatcctgggctgttagcgccccataaagcggtattatccttctccacatttatgcccagcggggtgatggctgaatgcaatgatttatagtgaaagttttttactacgccaatcacctctaccttcttatctcccaaatttatatacttccccaacggatatcccgaaaaaccaaagctttccacggcagattcattcagcactattttatccggcatgcccagctgtgtggaatctgccggcggaaatttccattgcagtcctgttaacccaaacagggaatgatccatgctgagcatagacaacgccattggcggacggttaccttctcccatcacaaaccacatatcgtaaccgccatacaacggataacgggctgtagccgtttgctgcacaccattcaaagcagccacctgctgccggtaagcctggtagtgattccccatagagccctgaaatggcagcattaccacgttctctttattgatgccggttgcagcatgacggaagaaatacagctgccggttaataacaatgctgcaaatgatgagcactgctgcggttccaaactgcaataccgttaatactttccttacggaggcgccgccgcttacgcggctcatcttccccgacaaaatgtaaacaggattataacgggaaagaacaaacgaaggataactgcctgccagtaaaatagtgatcagcaataacagcatataaatcatgagtactaccgggtggtaaagaaagcttacatccaccttcagctgcagcaggttgaagaaccaggggcgtaataactggcacaacaagagcgccaggcaaaatgccaggaaagcatagagggccgattctacataaaattgtttggcaatgcttttatgatcagcgcccagcgatttccgcacccctatttcacgggcgcgcatcgttgcccgggcggtggagagactcatatagttaatcaatgccatcagcaggatcagcgctgctaccaggggaaacaacttcagatatcgaagattaaaccccgggctgaaattagcatcagtatgcatccgggtgatgggtaccatcaccgctctcccctgatccaactgagcagctatcagccggtcgatattttgtactacggcggctgcgtgagcgggatcatccagcttcaggaacactttaaaaaagacgccggcaaatccacgttcaccggaaataatttccctcattgattcgatgccggccatactggaatacgacaacagtatattagcctggatactggaattggaaggtgcatcggccattactcctgatacctggaaaatgtacttgccattatatcgcagctgttttcctattacatctgtacttccaaaatatttcctggcagtggaagccgaaattaccgctgtaaaaggctgcttcaatacctcattcttatcaccggacagcaaggggaaagagaaaaagctgaagtagttggcgtctgtaaaccaggtgtcacgctcctcgcttttaatattgggattggccacactctgcatgataatggattcgctggcgaggttgcccatgcggatataactctccacggccgcgttctgttgctggatagaggctgccgttgttgcgttaaaacgctccagctgcatcgtatctttctctagtttaatcttctcaaacagtgaataaatcctggaactatctttatgaaaacgatcatagctcagctcatgcactacatacaacataatcagcatgcaggcgcacaaacccgctgccagcccaccgatattgatgaagctgtatagctttctttttgcaagattgcgccaggcaagttttatgtagttgaatagtagcatagtcaatcgtttctcaggttatctgccggattcacttcaatagctctccaggtttgtgaaaaaatggtaatcagtgccaggaataccaggaacaggaaacttcccagcattgccaaaatgcccgtgcttacccggtaagcaaatatctgcaggaaaagcaggctacctatatatcccagtggcagggcaatacagcctgctatgacgattaattttatatagcttttagacaacagcattaatagccccgctgcactggcgcccagtactttgcggatagcaatttcctttctgcgggtaaaagaggtgtaggctacaatgcccagcaaccctaatgcagctatcaaggtggtaatgaataccaggaaacccagcatggaaattacttctctcccattccggctacggagctgttcatccatccattccgacgtgaatacttctccgggatgcatggctgtccatatttttttcacgtccgctacctgctgctctttatctcctttcagcatcgctaattgcagctgacggaattcgttgggagcaaaacggatcgccatcgggcggatatttacttctatcggctgatagttgaaatctttcactacaccaacaatgcttacgggaagggaatccgacaggaacagtgttcttccgatagcatctgccggtgattttatacccattacactgaccgccttttcgttgacgataatatattgttctttttcagcagaagcggattcagggaaagtagtgcccgccactagtttcaggtgcattactttgaggaagtccgcatccccggcataatagccaaactccatcctgtctttgctgtcgccggtgcggataacgcagaagttacaatgtcttggcatgcctaatgttccggagctggctgttgccgtcgtcacttccttcaattgcatcatgcgttccttcatccgttgaaagtccacatccgccagcggaacattgaggatatcttcacggtagaagcccatgtccttaatggctttgtaatggaactgacgataaacggtgaccaggaagatgatcgcggttaacgataaggaaaactggatgacgataagtgttttccgcaatcccaatccgccaaaaagtttaatgtcgataaggttctttaacaccttagccggttgaaaggcggataaagcccatgccggtatagccccggctactatgccaataacgatgctaaataacaggaacaacaggagcagcctgggttcgaggaggttgttatccggaacaggtaatccgctgaaatgagtggactgcatcagcatcagcaataaaaccgccatgatcagcgacaatatgcacatgatcacagattcggtaataaactgtaagaatatctgccagcgttgcgcgccgtttacctttcgcacgcctacttctttagcccgctgcagggaacgtacaatagataaattggtatagttaaagcaggcgcagataatcagtcccagcgctacgcctatttccgcgagtaatttgccccagggcggcgtaccgccgatatcgtccatcagctcctgcgacggcgtgattttgccgagtgcctgtggttcgaaagccatgctgccctgccctttctgcaccaacccgtcgtagcgatgggcctggtccttcagcgccgactccagggcggataccttttcgccgcggcgcagcaccacataggtgtagctgctctgtacctggtcccagttattcagcttatccggcaatactttgctttgttccagtaaaggcacggacgacattgccgcaaaggcttcgtaatcgatatgggatttggagggagcaggttccattacgccactaacgataaagctgccaaagcgatcgaacaggattacctttcccattggatcagtggtcccaaaaaaccgttgggcagtttctgcggtaagcacaatgctgttgggcgtaagcagggcggtgcggggattgcccgcagccagtttaaagccaaacacctcaaagaaggaaggcgtggcaaatgccccatagatatggatcttcttcttatctattttcccgtctccatttaaaacaccatataaggtggcctcattttcaacggcagcataattattttttaatgccgctcccattggtaatggcacactggccatatgatattttctgccatccggcgtttgcgcatgggtagtgattctccaggtacgcgaagcagcaggatgaaaattatcataactgaaattttccctgacagatatcaatacgatcaagcatactgtcatgctcacagccagcccggcgatgttgataaaggtaaacaacctttgccgctgcagatttctgaatgttatgacgatataacgcttaaacatatacgttaaattattcggcttttaaagattttacagggttggccatggcggctttcaccgactggaaactcacagttgccagggctatcaccactgccagtaagccagcaataataaagatccagacagataaatttgtatgatatgcaaatccggataaccagttattcatcatgtaccagctgataggcgtggccagtaagataccaatgatcaccagggtcaggaattcttttgaaagcaaacgggtaacgttcattacggaagcacctaatactttccggataccaatttctttcctgcgctgttctgcagtaaaaacagatagtccgaacagccccaggcaggaaatcattaccgctaccaccgcaaatacctgcgccagtttacgcaacatcgtttccgacctgtacatgttatcaaaagtttcatcgaggaagtgataatctaccgggtagccggcgttcagcgtagtgaatactttttccactgcggccacctgattggaaacctctccttttgccaggcggatcatcatgtaattattatcgttcggttccagcatcattaccatcggcgaaatattttccctcatagaggcaaaatgataatcttttaccacgccgatgatggtgcctttccccttccagaaactgatttgttttcctacagggtccttcattcccattacacgggcggcggtttcattgatgatataggcagcggagtccgaagcaaagtcccgggagaaatcacggccttccttcatcgtcattcccatggtggaaacatagtcgtatcctacctgctgcggcgcggtatttacaatcagcttatccggctttccttcccagctcaggtcggcacttgagccgccaatagacaatggcaggaaactgttgtaggtaaatgacttcacctgcggcagctgcgacattgattgctcaatcgcctgctggtttgcggcaaagccttcgcccaattccacatacattacattttccttgtcaacccccaggttacggtggtagatgtactgcatctggttgtagatcactacgctgctcacaataaaaatgaaagagagcacaaactgcaataccaccaggtttttccggaacagggaggctccgctcccgctgctcaaatcacctttcaataccttcaccgggaggaaacgcgataacacaaaagcaggatagctgcctgccagcaagccagtgatcaatattactcctaacagccccaccaggtacttaacagtaacagacagcgtaaacgtaatatgcttgccggtaaaattattgaataccggcatcagtaagtacaccactactgctgcggcaacagccgctatagcgcacatcaggattgcttcgccggtaaactgcaacatcagcgaaagcctggaagcgcccatcgatttacgcacacctacttcacgggctcttttagatgcctgtgcagtggaaaggttcatgaaattgatacaggcaatggccagtacaataagcgccgtgatgaaaaacaaacgtacatattcaattcttccaccggctacttttccattttcatatttttcatgcagataggtatcttcaaaaggttgcagccatacttcattcttattaccagggttgagtttagcgtaatgttgctgcatctttgcggtgaggcggggaatatctgttccggctttcaccaccatgtaattagaaatactatagctgcccggcctcaacagccagggatcctgcttcagggaaagcgcaaagggcagtataaagtcgaactgaatggacgatgcagcgggcacgtctttcacgatagctgttacctgcagcgctttgttcttttccacgttaatgatctttcctacaagatcggtggtgccgtaatatttttttgcaaatgattccgtcagtacaatagattccggctgcatcaatgcggtatgcttatctcctgctactaccgggaagtccatctcttccagcaggttagaggtagcgaatatgtaatttttttccagggcggatcgctgcgctgttttaaacagcatgttgctgttggtcacccggactttcacattcgccatgatctccgggaagttacttttcaggtcatccgccagcacagttggagtgacggtcatggtgcgtataccgccccagtccacattcgcctgcagccggtaaatattcttgccatttgaatggaacttatcaatactatattcgtctaaaacccagcagaggataaacatgcacaccgccatgccaaaggccaatcctgcaatattcacagcagcgaaaaactggcttcttttcagattcctccaggcaatttggaaatagtttttaatcatgtttattcggatctaagtgatttaaccgggttcattaacgccgcttttatggattgcaaactaacggtacacaatgcaatcagcaccaccattccagcggtgagtaaaaacacccaccattccacgtgcaccctgaaagcaaagttttgcagccatttttccattccgtaccaggctatgggagaagcgatacagatccctatcaaaaccagtttgagaaagtctttagataacaacagtgaaatattggcaatagaagcacccagcactttgcggataccgatttcttttgtacgctgccgggaaatgagcatagacaatcccaggaggcccatacaggctataaagatggcgaggccggagaagataccgaataatttgcccagtgtacgttcagatgcatactgtgcctgtatatcatcttccacaaaagtgaaattaaatggcacatcgggaatcatactgttccatgcggcttccacacgttttaatatagccttttgatcgcctgctgcaagccgcagggtaatgatcgctacttcatcctgccttaccaggtagacgataggctctaccggcatttgcagggagcggaggttgaaatcttctaccactcctataatggtaccatgtctttccatatacccgggtcgccactcaatccgtttgcctactgcatcatccttaaagcctaactgtcgtgcagcggcctggttaacgatataggcatcggaagaatcagtagccagcgcagggtcaaaatcacgtccggccaccagtttgatgccggttgttttgagcaggtcgaaatccgattgaatgattcctgcaacaaagccgtctttatcatctcccccttcacgtactatcgggttgttattaaacacaccactgcccattaaaaaattatgcatggaagcctgctgcacacccgattggtttaagaaggcggatttcagcaaagcaactttggcgccatccacgccggagaggtatatatttacgaggtgttctttatcgaatccgaggttttttgtttgccagtagcggagctgggaaaataccaccaccgtggaaatgatcaatgccacggctaccgcaaattgtgccaccactaatccacggcgtaccagcacacgggagccggaggtaacaaaatttcctttcaatacgcgtacgggtatcagcccggacaggtagagcgcaggatagctaccggccaccaggcccaccaataataccagcaataataagccggcatataaaaaactatctgcggaagaaagcaacagcaattgtttgccggtaatagtattaaacaatggcatcgccaatcctaccagcaaaatagccagcacaaaagagataaggctgatcaccagtgattctgtaagaaattgcaggataaggctttttctttcagcgcccagtactttacgcagccccacttcttttgctctttcatgtgcccgcgcagtggtgaggttcatgaagttgatacaggcaatcaggatcaggaaaaccgcgatagcaatgtataaccagatcaacggggaattatctattcctttatcgccctgcgggtgcagatgtacatgctgaatgggttgcaattccagcgcaaactgtatgttatgctttttcagtattcgaccaatatgagtagatacaaaagtggccagttctttggtaagtttagcaggatctgcgtggtctgccagctgcacataagtaacattattgccaaacatgaaccactgtttttccatatcggtgcccgcttttaatgcttctttcagcatggtggggtacgatatgatcatggtcatgcggagatctgtattggatggaaagtccttagccacaccggttaccgtgcagctgtaaccattgcctacctttatcagttttccaatgggcgattcatttccaaagtatttttttgcagcagatgcagttaatacgatggagtatggttcttttaaaacggtagccggatttccttccagcagcggataattgaaaacccggaagaaaggttcatcggcaaagcctgtattttcttcccatattcttttatctcctgcagtatagagggtatttcccggtgcgtaaatacgtactgcttctttgatgctgctgatatcttttttcagattggggccaacaggaaactgggtagccgcgtcatgttcggtattacctgtgggacgggtagtttgagttgtaacgcggtagagacggtccgcattatggtggaacctgtcaaaacccagctcatcgcgcacatacagcgtaatcagtatgcagcaggccatgcctacagccagcccggagatattgatcaccgtaatgaacttatgacgctgtaaatgacgaacagcaattttgaaatagttccgaaacatcatgatgtggttttagaatggcggaaaaaaaatcacacatgaaactgctccttgatattctctgtcaccacgcgtccatcaaacaggttgataatacggtgtgcaaaccctgcatcatatggggagtgtgttaccatgatcagggtggtgccggagttattcaactcctgtaataacttcatcacttcttccccgttggtggagtccaggttacctgtaggctcatccgccaatatcaggttaggtttggctaccacggcgcgggcaatagctactctttgttgctgaccaccggacagctgctgcgggaagtggttgcggcggtgcataatattcatgcgttccagcacctcttctaccttcacctttctttcggcggcaggaactttcagataaagtaagggtaactccacgttctcgaaaacggtgagctcatcgatcaggttaaagctctggaacacgaaaccaatagagcctttgcggagctgtgccctttgtctttcactcatacgcgctacttccttatcccagaagtgatactcgccatcactggggttatccagcaaacccaatatgttcagcaaagtggatttgccgcaaccggagggtcccatgatcgccacaaattctccatcctgcacttccatgttaataccattgagagcagtggtttctacctcttctgttgtaaacagcttctgtaagttaacagtgcgtatcatatgtgtttttaattttaaatgctagtttatataaaaaaatggatgaactaaaaggataaaacatctttgtttccgaaattctcataggaagaagtaattacctggtcgcctggctgcaggccctccagtacttcaaaatatagcggatttttacggcccagcgaaatattacgttttactgcgcggttgccgcttttatctactacgtatacccagttaccaccggtgtcggagaaaaatccgccgagcggtaaaaggatagcttctgcggacttacccaatacaaggcggataggagaggattgtccacggcggataccttccggcgtatctttttgaaaggtcatatcggcctggaaacggccgctttttacttcaggatatacctttgtaaccagcatttcgtaagatttcccatcgaattcgaaggtggctttcaacccggcaaatacctgggaaacataatgttcgtctatatcggcgcgtagtttaaaaccattcaggtcatcgatctggccaatattctggccggcggtgatgctggaaccaacttccacatcgatggaagagagctgcccggataccggggcgcggacaatcaggctgttcaggttttcccgcatcaggtccaggttgcgctgggttctggccagggtgccttccagctgggtaatctgcattttggcattgtcctgctggtatttctgggattgcagctggatatctttctgacgcaggagtccttccagttcaaacttgtttttgttgaattcctggcgggccacgatcttttcttccaccagttgcttgttccggtcgtacaggtcctgtgcagcggctatcttggcgtcaatgtctgaaatggtttgctgcatggtaaattcctgctggcggatgctcaggcgggtattctgcagttcgttgcgtaaacggtagatctctgtttcatggtttacgaagtccatcatcatgtgctggttgtccagccgcaggatagagtcgccttcctttaccatactaccgccatccaggtacttgcggcttacatatccgccttcaatggcatccaggcggatggttttcaggggcattaccactgcggtaacggcaatatatacgtcaaaggttcctttctttactgtagagatagtgatcttgtctttttctacattcagggtggccctgtgatccgcaaaaagcaacgtgtacaacagcagcattactactactgctccgccacctatcatcaggatgcgctttttattccaaaacttcttttctaattttctatccatgttctttagcgaaaagtttgctgaccggagaaagtcaatccacatgccaaagctgaaaaccttttaccagcaacgttttcaaggaaaaatggtttaaaaaaacgtcctttgccggacaagcggtgtccataatcggacacttttaaaagttcctgaaattagctgtgggtttgaaagaatctttgtttaatattgtcacctattcaccattcgcatatgactaccatgcaaccaggaaagattttaattgttgatgatgatgtagatgttttacgtgcggcccgcctgttactcaaaagacatttcgaacaggttgattttgagaagaatccgcaaaaaatcccttatctcgtatccaacttcgattacgatgtaatcctgctggatatgaactttacccgcgacctgagcagcggaaaagaaggctttgaatggctggaccggatcctggatataaaaccgcaaacggccgttgtattgttcactgcttatggcgacgtggaaatggcggtaagggccatcaaggccggtgcggttgactttgtgctcaaaccctgggaaaacgaaaagctcctggccactattcaaactgcctataacaaacgtgcagcccaacaggataaacctcccgctgccgtacatcatccgggcaaccaggtaatcggcaaaagccccggcatgctcgccgtatttgataccgtatccagggtagctgccacggatgccaatatcctcatcctcggcgaaaacggtaccggtaaggatatgctggcccgccagatacatacacagtcgaaccggagcagcaaacccttcgtaagcgtagacctcggcgccatcagcgaaaccctgtttgaaagtgaactgtttggccacgtaaaaggcgccttcactgatgcccgcgaagaccgcgccggccgctttgaagaagccaacggcggcaccatcttcctggatgaaataggaaacatctccatccccttccaggcaaaactgcttaccgtgttgcaaaacaggtcagttacaaaagtaggctctaataaaagtatacccatcgacgttagactgatctgcgccaccaatcgcaacatttcgcacatggcttcgcaacacctgttcagacaggatctgctctatcgtatcaataccattgaagtacacctgccgccactgcgcgaacgtgtggaagatatcatcccgctggcagaacacttcctgcagctgtaccgcgataaatataaacgcccggtaaacagcatgcacgaatcactcatcacgcaactgcagcgctacgactggcccggcaacatccgcgaactgcaacatgcgctggaaagagctgttatcctatcacagggaaaaaccctccagccaaaggatgtatttgtaaaaaacaataacaacgcagatcaggcgatggacaccggctataacctggaagaaatggaacgcaacatcatttcccaggccatgaaaaaatgcaacggcaacatcaccgaagccgccaaagagctgggacttagcagggccgcactttacagaagactggaaaaatataacatatagccgttggctttcagcggttaataatcactgaaagccaaacagctaaaagcgctccaatgaatcgtttcagcattaatatcagcttccgggtcatcctgctggccgccacgctcacagccgctatctggctgttcatgcacggtatgcagccactcacattcctgttgatcccgctggtatttatacagctgtacggcatctatcattatctcaaccggattaaccggaaacttaccctgttcctcgagtcaatccgctatgaagatttttctatccgcttcagcgccgataataagctaggcaaaagcttcagtatgctcaaccaccagttcaacgaagtactggaggcgttccggcaaacccgcgcagaaaaagaagctaacctgaagtatatcgacaccatcgtgcagcatatcagcatcggggtattgtcgtttgatgcagaagggaaaatagaactcattaatcccgccgctttccgcctgatgggcatctaccggctgcgtaatattcacgaactgaaaacggttcatccaggcctgtccgaattactgatggaattgtcgtcgggaaataaaacactgtatgcaacaaggcaggaacaacaactgtctattcacgctgctactgtgcggttacagggccggctcatcaaacttatttccatccagaatatccactcggaattacagaaaaaagaactggaagcatggcaaaacctcaccaaaatattgcgccatgaaattatgaattccgtaacgcccattgtgtcgctgattggtaccatgcaggaaattgtggacctggatattgcccctggcgcgcagcaccaggaaggcatttccgacctgcgcgaggcgctgcaaaccgtggaaagccgcagcaaaggcatcatgaattttgtaaatgcataccgcgattatactacccttccgcaaccacagtttaccacggtgaatgtaaggaccctggtaaactccgtgagcagcctgttccaggccgatatgaagcaggcaggcatccggttttccgtagaaacggacgccgaaaatatggagatccatgcggatatatcgcagttgcaaatggtgttgatcaacctcgttaaaaatgcgatggatgccctggaacatacacctgaggcgaccatcagcatgaagctgtatctcaacaacatccagcagatatgtattgaaattaccgacaatggccctggcattgataaagacgccatgaacaaaatctttatccctttctttaccaccaaaaagaaagggtccggcattggcctgagcttgtcccaacagatcatacaaatgcatggcgggcagctaaaagtgatgagtccgggtattaacggtaacggtactacgttttatatcctgttgaatacttaacagaatatttgtaaattactggtacaatccctttccatgttccgcccaaaacacctgattatttattttcttgtactattggctgatatcctgttgattgcctttggcagcgaggaataccggtatgccaccaagccgctgctgatgattttactggccgtgtatgtgttgtatgccaatgtaaaaatgccccgctccttccgtatttttttgttgctggcattatttttttcttccctgggagatgacctgttgttgtttgaaaatcttttcctgccgggcctcggcagctttttcattgcacaggtgatgtattgtatcttcttcctgaaaataagatacagcaacctgccggtaccgttgtgccggtatccgtatatattcctgaacgctgcggtgataatcctgttcatcctcttcctgctaccctatctgggcggtttagccatacccgttatcgcgtattcaattacccttttcttcctggtgcaatgcgtactgcatgcctttcatttccggcggcaacctacgggctggtatgcgctggtgggcgcaatgctattcgtcatttcagatgccatgatagcagtgggcaaattctatcatccgtttcccggcggcgatatcctggtgatgctcacctatggttttgcacaatgggggctggtgtatggcagtacggagtacttccgggtaaaaattagccggtaattcttacttttgtctaactatgcagcaaacagactttcttgtcatcggttcaggaattgcagggctcacttatgcgctcaaggtatcacaacaatgtccggataaaaagattaccatcatcacaaaaagccgggaagatgaaaccaataccaaatacgcccagggtggcgtagcggtagtaaatgacctggagaatgacagtttcgaaaaacatatagacgatacgctcatcgcgggcgacggactctgtaacgaacagatagtaaagatcgtggtgaccgaagggccggaaagagtgaatgagattattgaatggggcgccaacttcgacaaaaacgccgacggcgacttttctcttggccgcgaaggcggacactccgttttcagggtaatccaccacaaggatattaccggtaaagaaattgaacgcgcgctgctggacgccatccaccgccgcccgaatatagaactgatcacacactgctttgtggtagacctcatcacccagcaccacctgggctacctggttaccaaatccacacctgatatagaatgctatggggtatatgtattaaacctcgctaccaataaaattgaaaagatcctttccaaagtaaccctgctggctaccggcggcaatggccaggtataccgcagcaccaccaaccccaacatcgctaccggcgatggcgtggcaatggtgtaccgcgcaaagggccgtatcgaaaacatggagttcatccagtttcaccctacagccctctaccagccgggtgtaagcccttccttcctcattaccgaggcagtaagaggcgacggcggtattctccggaatatccacggagaggattttatgcaaaaatacgatccgcgcctgtcgctggctccgcgcgatattgttgcccgcgccatcgacagcgaaatgaagatcaccggtacagaacatgtatacctcgattgccggcacatggacctggagaaatttatccatcatttccccaatatctatgaaacctgtaaagccgcaggaattgatgtggcccatcagatgatcccggtatcgcccgccgcacattacagctgtggcggtattaaaaccaatgaatggggactcacctctatccgtaatttatatgcatgcggcgaatgcgccagcaccggccttcatggcgccaaccgccttgcctccaactcgctgctggaagcaatggtatttgcccaccgctgttttatggatgctaccagcaaaatagacctgctggagtttaaggaaaatgtgcccgactgggacgcaaccggcaccagcgcccccaaagaaatgatcctgatcacgcaaagcctgaaagagctgaagcagatcatgagcgattacgtagggattgtacggaccgatgtacgtttacaacgcgccctccgcaggatggatatcctgcacgaagaaacggaagacctctacgaaaaaacaatggtatcgccgcaattatgtgaactgcgcaaccttattactgcaggttacctgatcgtaaaaggcgccgccttccgcaaagaaagcaggggacttcatttcaataccgattatccgtttaagagcgatctcgtacaaaacattgtgctgtaagctaaacggctgtctttcattacctttgcgttggatttacaaccatcaggaatatgtattatctgctgcttgctttttgttatagcctttccatattgccatttccggtgctttacttcatcagcgacgtattatacgtgctggtgtaccatgtgatcggatatcgcaggaaagtagtgatggagaacctgacccaggcctttccggataagtcaaaggaagaactcacccttcttgcaaaaaaatattatcacaaccttaccgatatgatggtggaaaccatcaaactgctcaccatgagtaaagcgcagctgcaaaaacgcttccgctgcgatcttacggtattgcatgaattatacgcacagggtaaaagctgccagctgcacctcgggcataactttaactgggaatgggctaacctgttttgcatgcagggcgtggcatttcctttcctggtagtatatatgccgcttacgagcaggccggccgaccggatgttccgtcatttcagggaaaaattcggcactattctcattcctgccaatgatatgggcaacagcatgcgggcatggaccaacaaacaatacctgattgctttggtggcagatcagaatcccggtaatccgcgcagctgctactggtacccgttcctcaataaaatgacgccgttctacaaaggcccggaaatgggcgccaggagaagtaatatcccggtggtgtttgtggatatccgtaaagtaaaaagaggttattaccatgcttcactgaagctggcctttgaaaatccgcaacaggagtccgagggcgctatcacagaagcctttgtaaaatatctcgagaaaaatattcatgaacaacctgaagtgtgggtatggagccaccggcgctggaaacatgaatataaagggaattaaaaaatagtttttttacaggagatggatacctgattatctcctgtgctgcttcaggctttcacccggctttcttacttgacctgtacgttattcgttacttttttcgtggagtacttttgtgcgatttgcagcatattatgaacgtttttccttttaacggctccgctgaggatgacttccccgtctgaaacagtaacggtaacgttagtaaacctgcgggcagcgtaaacggagtcgagagagcgtttgaggataacatcgggatcaggtcctgcaggcgatggcgttgttgttgtgggtgatggcggtggcggtgcaaccacggctgttttcacggtgatattatcctgtaccgacttcactcccttcactcctttcagcgcgtcttcagcggccgatttggccacttcgtcgcccacttcaccacccaggatcacgacgccgtttttcacgtctgcagtgatgccgggaatatgactcagcttttcatttacttcttcctttagttcttcatctgaaggtttacagccaaacatcaatatgtttataaacatcagcgaggctattgccagggtttttatcgtcatgcccaaacaattttatagcaagaagataacaaatacgcagggaatagccaaaagaaaacgggaccgataagaagaagccagtgcttctttttatcgatcccatttaaaaatatgaaggtaattagttcaataccgttttttcctgcacaacctgtaatcctttctggtccttcattttagcgaagcctccttctatgttacgcaaattgtggatgccttctcttttcatgatagagcaggcaatgatgctgcggtaaccaccctgacaatgtacatacaggttgtggttatcttccaggtcagctaattttccggggtccatcatatcaccgagggtaatattgagtgcacctttgatatggccatccgcaaattcaataggcttacgaacgtcgatgatcaccaggttgggatcatgcggaatatccattgccagttcatctgcttctacggtgatgatcaggtcttttgcttcaccggcggcttcccatgcaggatagccaccatcgaggtagcctaccacattatcaaaacctacgcgggccattctcaccacggtttcctcttctttaccgatgggggtaaccaggataatgtcctggtcaaacggcaggaggctgcccgcccattcagcgaaacgtccttccaggccaatgctgatggagccgggtacatatccgtcgccaaattcagtggcgggacgggtgtcgagaatcagtgcgccggctttaccttttgctttgaatgctgcaggggtaagcggctgcattgccttttccattacggctttcagggcatcgtatccttccttgtttatttttgcgttgataggaaagtaagatggcggcgtagctaagccactggtcacttcttcgataaatttatctttatctgtagccagcaatgcgtagttagtggctttttcctcaccaatggtgctgtaggtgtttggtcccaggtttttgccgcaggcagagccggggccgtgtgccgggtatacgattacggtgtccggcagtgttttaattcggttgttgagcgaatcgaacaggtatccggctaactcttctttggtgaggttgccgctgaaaagatccgggcggccaacgtctccgacaaataaggtatctcctgtaaataaggcatacggctgttgctgttcgtccgatagcaggtaacaggaagattccatcgtatggccgggtgtatgcagcactttaaagcttactgcgccgatgtcgaatacttcattatcttttgctatataagcatcgaagcttgtttctgcatccgggccatatacgattttggcgccggtagcttctgccagttccaggtgtcctgaaacaaaatcagcgtgaaaatgagtttcaaagatgtatttaatggtggcgttgcgttcttttgccagatcgaggtatacttcaatatcacgcaacgggtcaatcactaccgcgatcccgttggattctatgaagtatgccgcttccgacaaacagctggtgtacaattgttttacgtacatggtttttgatttttacaaatttacaacttctgaggctgtacacttatggataaaatctataccaaaataaaaaagtagccctggggctacttttttatataatacttttccgtagtacacggatcaatgcttttaaccaacaagttcttccacaaacttcgccacttcagcaatacgttgcttgttgatggtgtagtgaataaacttaccatctctttctgtaattacaatgccagcacgccttaatatggcgagatgttgcgatgctaccgattgttccagacgcaatttcacgtaaatctccgtcacggtcattttcttgtgatcttccagcagcttaatcatctgctggcgcagcttatggttgatagcacgtaaaaccatagcagccttctttacggcaatgtaatccaatttgatctggtctttttcattggtacctctagaaataataagagtattagaagaggtagttaataatgttttttccatcgcataatagttttaaaaaaatgatgaaatgaaagggatcaacggacagtactcgcaaacagttagacaacaactgcggtaatcgatttatacaaaaatataatatctatcacaataaaaaaaatttccataccttaaattatcatatatatgccccggatacttgcaaattagatgtaatttgactctcccatgacaaaactaagatatatgtcagggcttttgaggagaataaaaaggcttgaggtaaaacggactgaaataagccaggtcaacgaatagctttttttcataagcctgggccgacagcggcgccatatgcgcggcacttatcacatattctgcgaaaatagcgtttttgtgtgaagataccattacttgccacttagggctgccgtcaccgaaaaagtagacctggtgcgccgccagggggccatcaagagagtttggctccaggatcattgcctgtggcggcatgatctcctgtaaacgggcatcatacaagcccataaacacttcctgcctgcgggcgtccagcataggacaatataatgcctgctcattttttacttcggagattaaaccctgcgccatcatctgaagcgtggaaatggccagcagtggcttattccaggcataacataatcctttggcagtggccacgcctacacgtagtcccgtgtaagaacccggtccggcacttaccgctaccgcatccagctgcgcaggagtaattccctgctccttcaatatctgctgaacaaacacgatcatagtagcggcgtggtcctgctgcttttcatttaccagtgtttgtatcacctgcccatcgcgggaaaggctcacagagcctattgttgttgcagtatctatattcagtataagtgccatgtaagaaaaattaaatcgcttcgtaggctgtttgcagtgaggcggccacctggtaccggtcgtctccggtagcatcatgtatagcttttaatacttcatacacctgcttgatgcctatccgttcactccattcaaacggtccgtaaggataattggtgcccaaacgcatggatgtatcaatatcctctggtgttgcagtgccctcctgcgctgtgagataagcctcgttaataatcatgcagatcacccgcggtgttaccagtcccaccgcatccgctaccagcaagtactgccagccgagcttatacatgagggtatccaatgtttccttttgcccttcatccagcaccgatacttccagtaccggcatattcaccatccctgtcaaaaaattacagcccatgatattgaatccctgctcaaacgcatactgaccaatgatttccgtcagggaggttttcactattcctgccagcaccgggatacccggatttttcgcatacacctgcgcgtgatccggccggtcatcgaaaataagatccagtaccaggtcaaaaggcttaagagataatacctcctccaggcttgttttccattgtacatcatgatgcttggccattcccttctcctgcaattcatcaaagcgctgcgcatctgctattaccaggatattcatgcgttaaatttcggcaaacctaataaagaatcattaattatagtacatctgctttccatacattggtgcgttctcaattattatttactttcgttttcatggaaaagcaaatcattaataccaacaatgcgcccgctccaatagggccttataaccaatctgtgaaggcaggcaacaccttgtatgtatccggtcagatagccctggaccccgcttccggcgaactgatcaaatcaggtatcgtggatgaaacccaccaggtaatgaagaatttacaggccgttctcactgcagccgggctgggattccagcacattgtaaaaaccaccatctttataacggatatgaaaaatttcccgcaggtgaacgaagtatatggcagttattttaccagcgactttccggccagggaaaccgtagaggtgtctggattaccaaaaggcgtaaacgtggagatctctgtaatcgcagtaggggcttaactttacagcaatgcagcagaggaaacagttgttccctctgctgcatttcctattatttaccaaataaagaggcggccagtttcttatcgtggccatacacatcatccctgaaattcagccgcccatcgctatctacaaaggcggtgaagtatacaatgaacacgggcactttctcttttatcgtcacatacttctctttgtttgcattcagggcctcatcaattttcttttctgtccaggaagaatctccccgcagcagccattccgcgaggtgcttaggctccgcaaccctgatgcagccatggctgaaggaacgcttgttttctccgaagaggtaacgtgcaggcgtatcatgaagataaatgttgtactcattagggaaaaggaacttcactttgccaagtgagtttttaccgccaggcttttgccggacgatgtaagggaaattcgcgcctgaatacctcgcgaaattaatggagcctggtgaaataactttaccgctggcgcccactatttccatattctgacgggcaagataagcgctgccactacgtttgaggccaggcagcacttctccgcccaggatacccggaggtacattccagtaaggactgaacactacataacgcaggtcttttgtgaagataaccgtgctggcgcccggtttgcccactaccacgttgcagctccacgataattttcccttatcatatacatgcattctaaactgggggatattgaccaggatgtaatctgtagtgggttctaatggcacccagcgtaaacgttccatattaagcaggatcttttgaatacggtcctgtatgggcgtattcaatgcatccagtacccctttgttaatgaggccatcttctttcaatcccattctcagctgaaaattacgcactgcagagtccagggcaacagtgaaccgccgggtggtatcggcttctttcaggtcgccataagctttcaacctttctttcacggcggcgataacttcggaggagtctccttttttaaagctcttctgcgtggtgcgaatagaatcccatttggtggaagattcaatctgcgccagctttttcagctgctgacgcagcatgatatagtgcctgttcaccggctcgtcgtcttcaaaagcattattctttttattcaccatagagtccagcagactctccatatctatttttttgcgggggataaaccattccaggtccttggcggaatcggcggtgagtcctccccatactttatttccgtaggcaaagaattgcgcggtaagcagcatttcaatgcggggaatagcagtatcgccgggtttcagccccacatcactcaccagcagggtatctgtgagcctttgcaggtcagggttcatcaggctgctatcttttataccataggcggcatcgttcttcatcatgttgatgaagttgcctgcctgttcggtaagaccatctttattaatccaggcaaaatggtaatcgcgtttgcggtaaaagttgcgaatatattcgtcgtaggcgtcatacgatgaatgtgactgcaggaaattatttacataattgctgtcgagagcctgatcaatatactcttctttggtatagtgagtagtatctcttgcttttgttcttttccgggagccgctctgctgctgacaggcagcaaaaataatcaatgtcagtaaggccaatgaggaatagagacgtatagtcataagcgtaatggatgttgaatatttacttaaaaacaaacatgacaatcaaactgttgggatcagaagggtattatgtggtaaatgtatgaaatatatgtacttatcgcttcagaccgttgttaaaatctgctgtatcagttatatttaatctctaaaagatataaaaatgaacaaacctgctcctctggatacgattcctgtaaaaaatacgattgccgggcattacggccggtttgtgcatggcagtaagagtacattggctttctgggagataaaggcgggatttgaatcgccggtacatcagcatccgcatgagcagatcacttatatagccgaaggtacttttgagatgagccttgacgggcggaagtatacactgaaacagcatgacacgctggtgattccgcctgatacgccgcatggcgggcgggcgttggaagattgtaagatcatcgacagtttcagtcctgcccgggatgattacagatattaaaaagaaaaggtcctgatggtatcaggaccttttcttttataatttgatttcttcgtcgttagcgtcaaagaagcgatattcagtaagatggtaattggagtcagctttgagtttgatccattttttatattggaagtaccatttccattgtttggatgccaggaatcctttggtaaggaaggcatgcagtatggggtgaacgcggatggtgaggcctttgtgttggtgattaagcaggtattgcaggttcttttcaatgtcttcgaggatcagcatggatgcaccgattttaccggttcctctgcaggtagggcaatcttctgccacggagatggtgatctcaggttttacccgttggcgggtaatttgcatgagtccaaacttcgagataggcaggatggtgtgtttagctctgtcctgggccatgaatttctccatagcttcaaagatagctttcttgttttccggcagtttcatatcaatgaagtcaatgataatgataccgcccagatcgcgcagtcttaattgccgggctatttcagcagctgcctccaggttggatgcgagggcattttgttcctggttgttgctggagcttttgtatccgctgtttacgtctacaacgtgtagtgcttctgtggcttcaatgatgagatatacgccgctgtcgaggttcacggttttaccgaaggaggctttcacctgccgggtaatcccgaagttgtcgaagatgggggaaccgttgttgtaatagttaacgatatcagacttttccggcgcaatcttttggatatacgttttggtgtcagtgtagatatttttatcgtttacaacgatgcggttaaagctctcattgagcagatcacggaggatgctggcggttttggtttgctcgctcaggatcttttgcggggctacgcctccactgagatttgcctggatatttttccaggtttgaacgagggtggtcagatcttcgtgtaattctgcagttttctttccttcagcggcggtgcgtacaataacgccaaagttgggcgttttgatggcttccacgattttctgcaatctttttctttcttcggaggagtggatttttttagaaaccgcaacaatatcattaaagggtgttaacactataaatcttccgggtaaagaaatttcgcagctaaggcgtgggcctttagaagaaatgggttctttcagaatttgtacgaggatattgggtttaccgcccagtacatccgtaattttaccggtcttgactatttccggttcatttttaaatttggtaaaatcaaatccatcgggcgttttatcgctgatggccattgaagtaaatttaagaatggagcggatataggggctgagatccgtgtaatgtaaaaaggcatctttttcaaagcctacgtcgacaaatgcagcatttaagccgggtatcagctttttcaccttgcccaggtacaaatcgcctactgagaagttaggattgccactttcgtgatgtaactccactagcttcttatcttccagtaacgcaatttccacccctgtgggagccgcatttataataagttccttattcaagcgtccaaaattttaacctttaaaacttcacctttatgctatgcacacggctatttaagaacagcttactgcataccaaaacaatagctcacctataaagttagcgtatttcttcacgttcgtgatgaatggattgcttaagggttcagcgatcactgcaggtaatgtccggagaattcaattgcgggatctatggaaacaacctgcatgactatagcaatttaagaagtaaatgctagaatcatgcaggatatatgaaaatttttatccgaccaccgcgccgggagcataccttgttagtataaatggcgggaaactggagtaattatttcttcttacttttatgccggttctttctcagtctttttttacgcttgtgagtggcaattttatgtctttttcttttcttaccgcaaggcatacgctgatacttttttaaatgattgaaaaataatattattgaatacttttaatataactatctacttccttcttcagttctggatcggtcatgagttgtttgcttttttcaaacagttcaatcgctttcttcttatctcccttgcttctgtacgattctgccagcacaaataacacttttgcgttatccgggtggttcttcgcaacgccttccagtctttcgatagctttatcgtactgacctgatgtaatagcaaggttagctaaagtaacctgtgcatcaatattatcagggtgtgctgcaacgacttctctcagctttgctacgccggtcataggttcgccggtgttcatgtacaccatggcctgtgatattttcagcgtatcgtttgccggattcaattgtatcgcctggtcaaacaaagtgattgcctgctgggcttcccattttgctacgcgcggatcttctgcatgttgcaagtgggccaaaaataaattggctgcaaaggtgaggcttttttcggaattttccaacttagcggcttcgccaagataatatgcggctacgggcagctggttgaggctgtcccaggtgttgtacaattgatggtacgcggctatctgttgggttttcacatccccgcggacaacatttgtttcaatagtatttacctgtaaaagtttttcagcaggaattttccctttagctgtttccagcagttcggagaaggcaataggtgctacatcctgtccaccctgcataggggcggcagatgacataggtttcttttctgaccggggcacagtacggccaaaggcgaataatatcaccaatagtgctaccgcagcacccaccagaagaacttgtgatttttgcatcgcctaaattattaggctgcaaaactaagaacttttgagcttctttacttcagcaacaaattctttcgaaggtttaaatgccggaataaagtgctcggggatctccacagctacgttcttcttgatgttacgcccaatcttggcggcccgtttttttgtgataaaacttccaaacccacggatataaatatgttctccgttagcaagagcttctttcacctctttaaacatggcctcaagtgtgactaatacatcaactttggggatgccggttttttcagcaatgttgttaattaaatcagcttttctcatatgaaagcgagaggattactttactctcaaagttaatttaaaaattctaattgctgaattttaagcaaataaattttatcattttttcttataactggtattggcgataaattatatttatttgcaggcccggaaataggtatccggtatacctcatagggtttttgtacagcatttgccatatcaatatactaaataattttattaaaataatatataaatgatatcaccccgacaattttttaccgaaaaattactggaatggaaccgggaaacgaatacccgcaacatgccctggaagggtgaaaaaaatccctaccggatctggttatctgaaatcattctccagcaaacccgcgtggaacaaggctggccatactatgagcggtttattcaacactaccccaccgttgaaaaactggctgccgcaccggatgaagaagtgttccgtttatggcagggactgggatattatgcccgctgtaaaaatatgctggcagccgccagggaaatttcggctacctatcaaggtaagttccccgaccagtatgaacggattaaagcgcttaaaggaataggtccctatacggccgcagccatcgcctctttcgccttcaatcttccttacgccgtgctggatggcaacgttttcagggtcctctcccgctatttcgggattgaaacaccgatcgacagcaccgcgggaaagaagcagttcgatgtgcttgcccaggaactgctgccgcaaggccactctgctgaatataaccagagtatcatggactttggcgcagtggtatgcaagccccagcagcccttttgcggggaatgtgtgctccgcaaaaaatgcgtggccctgcatgaacatcttgttccacttctcccggtaaaaacaaaaaaactcctgatcaaaaaaagatatttcaattatctcctagttcattataaggaaggtatatatatccgcaaaagaacagatagcgatatctggcaaaacctgcatgagtttgttctcattgaaacagctggtccgtcggacatcaccgcgctgcaatcgtccggagcctttgaaccgctgctgggaaaaatgcctttcgaaatagaccgggtgtctgctccatttaagcagcaactcacccatcaaaccattcacagccagttcattagcatcaccgtgaagaaggtgccggccatccccgggtataccctggtaccccgcaacagcctgaatagatatgcctttcccaagaccatcaccacttttctggaaagtaatcacctgcaattattctagtgaacacgcatagagaataaaaatatacattaagtgttaaggcactttaggaatagtgcctggtaacaaaatccggcttaacctgctgccagtaagaaatttttccctatcgattggaaaaaaatattaactttaagaaggttgtttatttattaaaagaagaactttttaacaatagactaaaaaaacctacaactatgagaggtgttaataaagtaatcctgataggcaatttgggcagagatccggatgtacagtttctggaagggaatattgcagtagccaaattttcactggctaccactgaaacattcaaggacagagccggcaagctcatttcacaaacagagtggcatacggtggtgctatggcggggactggccgaactggcgcagaaatacctgcacaaaggcagtcttgtttatattgaaggccgcttgcgcacccgcagctgggaagacaaagaaggcaataagaaatttgccaccgaagttgtaggagataacctggttatgctggataaacgcatggacctcaacaaccaagatcaccccatacctcaccatagcagtacagggtcaggcagtggagaaagctttccgggactggaaataccaccttcactgaacgaacccgcagacgatctgcctttttagttgcaaaaaaatattaagttttgaatgtacgtaatcccatatagggacattacttatatttgcgtgcagggaaagcaattccatgaattactttcccctattttttgattaattacatcaaagttgaacatcttgggcatcctttcggcaagctacgtatcctattttttacaagccagcgcaccaattggcgcccctaacgtggtggtatttctgcttgttatttttattctgctgctgctaacctttattgtttccggtgcggaagtagctttcttttcccttaatcacaaggatctgaatgtgcttaaaacacgccagaacgcatccggcaaactaattacccggttgctggaaaaacctaaatcactgctcgcttccttacaaattgcaggtatattgctcatgatcgcctttattatgatcaccaattacctcgttacccagatggaagacctgcaaacactgccggtagtatccctcctggtaaggatttccgcgatctgtctcatcttattgttcttcggccagatactccccagggtatgggcagctcaaaacaatatccgttttgccacctatttcgcctggttcgtaagcggtgtacatgccaccatggaaccggtcagcgatttttttgtgggcctcagcaccagcattgaagatcgtttctttcaccgtggcagcggtccggttaattaccacgaaattgatgaggccatcgaaatgagcgtggacgccaccgcctcccaggaggaaaaaaatatcctgaaaggcattctgaaatttggcaatattaccgtaaaacagatcatgcgcggccgtttggacgtaaatggcgtggaatatgacagcactttcggcgatatcgtgaaaagcgtagccgacctgcattattcccgcctgcctgtttataaggataacctggataacatcgtaggcgttatccataccaaggacctgctgcctcacctcgacaaaggcaacaccttcgactggcacgaagtaatgcgccagcctttctttgtacatggccataaactgatcgaagacctcctttctgaattccagagccggcgaatgcactttgcagtagtagtggatgaatttggcggtacctccggtattgtaaccctggaagatatcatggaagaggtaatcggcgatattaaagacgaatttgatgaagaagaatttaactacaacaaagtagataacttcacttacgtattcgaaggcaaaaccatgctgaacgacgtttgccgcatcatgaacatctcccctgaaacatttgaaaccgtaaaaggcgaaagtgactctctcggtggtcttatacttgaactggccggaaaatttcctgaagaaaacagcgttattaactacaataacttcgatttcactgtactggaagtcaataaaatgaggatccagaaagtacaggtaaccatcaggccggatgcagctgataaagtgtaactgcctgctaaataagcgtaaaatgccagcgattaaaggaaaggccctcaccctgttcgtggggctgatgtgtatatttgccgcctgtgaaaacgtacccacaccaaagcccagaggctatttccaggtgaaatttccggagagaaaataccgcaccttcgatatgcccggatacccctatacgtttgagtacccggcatacgccaatatcatcaaagacacctccttttttggcgcagcaccggaaaacccgtactggatcaatattgacttcccctccctgaacgggaaaatttatatgagctacaagatcatcggccccggtaacaacagtttccgcaagctggtagacgatgcttttaaaatgacctacaagcatacctataaggccgaatacatcgacgaaaacaagatccatacagctaataacgtaagcggcaccttctatgaagtaggtggtaatgccgcctcttcaaagcaattctttgctaccgattccgtaaaacacttcctgcgcggcgccctttattttgatgttacgcccaatgcagattccctcgcacccgtttaccggttcctggaacaggatatgtggcatatggtagaaaccctgcgctggagataagccctgaatgctgtaactttgtggtcttaaataagattgtctgtctgttatttcaggcaaaagagcattccagatgattatcattgacgataaatacataagtgacgaagtaattgaggagcaattcgtatgcaatctgtccgcttgtaaaggcgcatgttgcgtagcgggcgattgtggggctccgctggataaaacggaagttaaaaccctgaagaaaatttatccgaagattaaatcttacctgcgggaagatggtatcaaagaaattgaacacactggtaccaatactaccgacgatgagtatggatatgttaccccgattgtaaataaaggtatttgtgcatacgcaaccatagacgatcacggtgtagtaggttgtggcatcgagaaagcatacaatgatggtgtggttgattttaaaaaaccgatttcctgtcacctgtaccctatccgtattaaaaagtacgaaacatttgaagcagtaaattatgaccgctgggaggtttgcaaacccgcgtgtaagaacggtaaaacccttcaagtgccagtgtatcgtttccttaaagatgctttggtcagaaaatacggcacggaattttatgaagtgctggataacatcgcaagaaaagaacacgggtaaatcattttcggatttaactatctttaattaggaatattgcttgcttatgcatcaaacagcatctacttttctggaagaaagtgaaaagaaagcgtctgatctcggccaccgccagacgatcaacttcaatataggcaaatacaatacagctgtaaaggccggtaaacaacagtttacggatttacctggcgcaagggaaagggccaagaatatcaagtggagagctattgagcacctggataatcacctggaagaatttgagcaaaactttacccgtcgcggcggcaaggtcatctgggctgaaactgccgaacaggtacaacaggaaatactggccatatgccaggcgaaacaatgcaaaagcattgtaaaaagcaagtcaatggccaccgaagaagtacacctgaatgcctttatggaaagtaatggcatcgaatgtgtagaaactgacctcggcgaatacatacagcaactcgacggagagccgccctaccacatcgttaccccggccatgcacaaaagcaaggaagatgtggcccgcttgtttgcggaaaaacttggcactgatcccggtctcactccggagcaattaacccttgttgcccgcgaaaaacttcgccacaaataccttcaggccgaaataggtatcaccggcgccaacttcattatagcagataccggctccattgctgttacggaaaatgagggcaatgcacgtttaaccactgctttccccaaaacgcatatcgtactggtaggtattgaaaaagtacttccttctattacagacctcagcctgttctggcctttactggcgacctatggcaccggtcagcagatcaccgcttacaacagtattttcagcggtccccggcaggaaggtgaaatagacggtccggaagaaatgtatgtcatcctgatggacaatggccgtaccaacatccttcaggatactactgcacgtgaaagcttatactgcatccgttgcggctcctgcctcaacgcctgccctgtttataaaaatattggtgggcactcttatgctgccacttacagcggccctatcggcgctgtcattactcctcatctcaaagggatggattcctacatgcacctgagttttgcctcatcgttgtgtggtaattgtaccgaagtatgcccggtgcgcattaacctgcatgaactgctgctacataaccgtcagaaagccgtagaggaaaactatacttccggtggagaaaaatttgcgtggtttatgtggaaacaagggagtaccagccgtaaaatgatgaacatggccagcggcagaatgaaaaatttcctgctgcgaagattctttgccaaaagctggggagataacagggaactgcctgtattcgcgtctaaatcctttaaccagcagtggaaggagcggaaataactacttatctttttgcacggtaaactttaccctcacctttactttagcgggctttccgtctgaagcgggtgtccatgcggggccttctttgattacccgtatagcttccgcatcacaggcctcattcagatgacggatgactttaaagttttgcaggctaccatccggcataacgatgaaggatactcgcactgtaccactgtatttattttccgggttaactgttttggttttcagatagttttcaaaggctgtttcccctgttatcggagcgggttcccggtaatcggtgttatcagcatcatcggacgagacttctaccccggccacttttccggctaatgcagtctctgtactggagtcgaaaacagagtcgcgtctgagcacactcaccgaccctgtgacatttttcctcttctgcacaccgtaacccactactactacgtcgtttaatgcgttatgctggctgtctggtatattcagcatcttacttcgtcccctgatcattatctgtttctctttttcggcagaaggaggaggaataaagttccgctgctggtccgtgcgttcggcctgagcggccggtacagcagcaaacatatctgctgtgtcagacactcttttgttctcaagagaaattgttttgtctgctgcttcgcttttgaagtcgggctttgttttataggcgcctgctgcctgttcttcctttgcttgcttctcaactgttagcggcttaacgggtgttgcaggcataatttttttagcgggatgatcagcacttaccgccgatggggcggtgtctccatgttcggagtataccggtgccgtctccggtgatggttttggcgtgcttacgttggcaataggtgctgttcgctgttggttccaaaggaaccagcctgcagaaaacatcaacaataaaatagctgctgccgctgcggcccggtaaatcatgggacggatgcggcctctgggcgcgaccctttccgacagcctggaggcaagatcttcctggtggaccgtttgttccggagcgtgcagtgcatagccttccagcgcgtcggccaggaacggatcgtccagggcctggcgttccagggcatgcatggctttatcgtccagctctcccgctaggtattggcggatgagcccggcgagttcttccggttttatatgtggccgcttgtcagtcatcttgttgttccatacatattttcaggttacgctttccgttctggatgtagctttttaccttattcatttcatatcctgtaataacgctcacttcccggtagctcttctctttcaggtaaaacaagtctacactgcgtttttgttcttccggtaaagtttccaggcatttttccatactctgcaggttatcttccagtgatacgccgttttcatgatgcccgttttcaccgttttccacaacgaggtgatcatcaatagatacctgccgggattccttatttttcattgcccgcagcttcattaagcaatgattacgggcaagtacatgcaaccagcttttaaaattctgaacttcgtgttgctttaccttgataattagttcctcaaagatctgcattacggcatctttgctggcttcttcatcaaaatatctcaggcataccccatataccaggttcatgtaacgctggtaaagggcggcaagaaaatccagtttaccggtggttttaaactccccgatcaaccaggcatcatctgcatcctgcatgatattttgttgaataaaagacatttgtagcagctattcgcttatggccttggcttttaggatgatattgatttacaagtcgacaatactattattttttttgaatattatgagatgaaaataagaaagcaccgggaattccggtgctttctcttaaaaattccaataattacgattagtgtctgaagtggcgcatgccggtcattaccattaccatatcatgctctttacagaattcaatggagtcgttatccctcatagagccaccaggctggattactgctgtaatgccatgttcgtgggcaatgcttacacaatcattgaaggggaagaaagcatcggaagccattgctgcacctttcagatcgaaactaaactggccggccttttcaatggcgtggcgcagtgcgtcgatgcgagaggtttggccacatcctttaccaatcagctgctgatcttttaccaatgcgatcgcattggatttcaggtgtttacaaacgatgttggcaaactccaggtcagatttttcagcgggtgtagcaggacgggcgcctacttcgttccattctttgtagttaccattatcgctgtcctgcagtaaaacgccgttcaatacatttttaaacatgtatttgctctttaccggttgtttctgttccaggaggatgcggttctttttggcctgcagcacggtcagtgcatcggcatcaaaaccaggagcgatgaggatttcgaagaaaatttcactgatggattcggcagtggttttgtcgattaccctgttggttaccagtacgccgccaaaagcgctttccttgtcgcctgccagtgctgcatcccaggcttctttcagtgtgccacgggaagcaatgccgcaaacgttcgtatgcttgatcacagcgaaggtagtcgcttcaaattcctggatcagctggcacgcagcgtctacatccaccaggttgttgaaggataattccttaccatgtaatttgttaaagatttcatccaggttaccatagaaaacaccacgctgatgtgggttttcgccatagcggttcacttgtccttccggaatagagagctggaaatttacgccgggctcattattcaggaaatactgggagatcgccacatcatagtgagcgcatacttcaaacgctttggcagcaaagcttctgcgatcttcaatggtggtagcgccgttgttatcggtcagtaccttttcgaggtcggcgtattgatctttcgaagcaacaatcaccacatctttgtagttcttgccggctgcgcggatcagtgacaccccgcctatatcaattttttcgatgatggtttgttctaccgtcgtgctttttacggtttcctcaaacggatacaggtcaacgattaccaggtctatttccggaatctggtattccttcagttgttccagatcctgtggattatcacggcgggccagaataccaccaaataccttaggatgcagggttttaacacgtccacccaaaatagacgggtaagcagtcaggtcttctactgctacacatttcacacccaggtcctcaataaatttttgggtaccgccggtggaatagatggtaacaccttgttcacctaattttttaacaatgttctccaggttatctttatagaaaacggagatcagcgctgatttaatttgcttttgcatgaatggaaaacattagaaattaataacataggctccctggtccggaaccgaaaagaagcgcaaagttaacacgtaacaatcacttttccatttctcaatccttcgcgcactatttgaagccgcaaaaatgagcgtatcaaatgtataaaaatcacacaggtacctgatattcactggtgtattacgtgttaataaaatataattggtcttaaatttttcagatggcgcccgatccggcaatgcgctgtctataatcagtatccgttttccctcgaagctcaggaagcggccatattgctgaaaagaagcgggtgtaccggcatgcgcgcgcaggtttgcgcgcgtgttcaggagttgctgtgctacgggtaattgccatacactatcattgccggcaaattgtaccaggttacctttaatacaatcaatggccgtataggcgggcacgttatagataataatactgcattgtctcttgcaggcggtcacccaactgacacgggcgatcagaaacccccagatacaaagaagtcccatccacaatccgggtcggaaccttaccagtagccacagcgccagtgccgcgatcagcagataaagcagtacggtttgcgccagcgaacagtgaatatccctgatcactgcaccaggcaactctccaatccacctgatgcagctattcattccgaggatcatatatttcaatgcactgcccagccaaaccgccggctttcccaaaggcgacaggagcaacaatattacttctccgtaaatgattagggttgacagcggcaccgcgatcaggttagccggtaaaaaataattgggaaactggtgaaagtaaaataggctcaccggtgtggtgatcagttgtgccgccaacgacaccgccgtcatttgccaaagccagtctgcccaccggcgtttccactcgaacagatggtaaataggttggtaaaaaagcagaatgctgagtacggcgaggtacgacaactgaaaccctgcatccactaccaggtagggattaaaacatagtaacatggctgcggaagccgccaaagtattgtaaatgctgctataccggtgcaatacaaaatgtccgacagtaatacctgtaaacatcaccgcagaacggagtacagaggcagatgcaccggtgagtaaggcaaatccccacagcacaacgaggatgatcactgcttttgttacatgcatccagcgatgggctggtagccattgtagcaaccatagcagtgtactgtacaacagcgcaagatgcattcccgaaatagcaatcacgtgcacaataccagtattactgtagctctgcaccacatcctggtcaaggtcctggcggtaaccaataagcaatgcttctgccataccggcttccggtccgttaccaatatactttttcagattatacaggcaataatcccttgcctgcagcaataacctgcttaccggatgcccacgattatacggtaacaggtaaaagtctgccgggccgagatacacctgctggtaaacctgttgtgttaccatatattgctgatagttaaacgccccggggttaccgttaaatttgatgaattcgggccgtttccgggcaattaattcgtctccgtagtgaagagcaggcgaaagactgtccttgcccgtataaagcaataaacagcctttaacaggcacccattcaccctctttgcaaacggctattacctgtgcggtggttttaaaggaacggggcttttcctgtggaggttcatttatgcgcaacaggtaaaatggtgtatcgaccaggtacctatcgtaaaaacctttgctatggcggatatcggcattatataacagcaaaccgccacaacaacagatcaacagggagcataatattcctggtagccaggccgaggcaaaacgccattgcagcggtaaaaaacgaaacgctgatacacctgccatgcaacaacaggctactgtaatgtaccaaacaggattcaccggtatatacagctgaagggtaattccagctactaatggtgcgatgatacgcagaaaaggtgcacgcttccaccatttcacaacaaacaatgcagattcaaattccatgcagggttaactttatcgggtaaacaaacctcgcatttatgagtagtaaaagcgttttggaaatgttaaaaggggatgtttctgactgctaatatttatatatgatatcttgaaaactttcactttacctaaataaatcccggcaaactaataaagctcatcttctttttaagttattaataatcatatagtatcatattatacactaccgcatctgttattgattagttaacatctcttttaaatataatattatttgtaaactgcattaccggtcacgctatatgaattgtatcaagattcaatagtcgtgtctttaatggttattttgagggaaaagaaggagcctgatttttatcaggctctgttcattttcagataaaacgatttatacataaaaaagcccttccgatgtaacggaagggcttttaatatttggtttcttaacaggaaactacttgctcagatacatactcttttctttgaaaagctgtctgaaatacgggtcacgcagatccttgataaagcggatcgcttctcctgtagatttcatttcaggtccgagttccttgtttacacccgggaacttattgaaagaaaataccggctccttaatagcaaaacctgtaagattctttacaatggtaaagtccttcagcttattggcgcctatcatcactttagtggcaatgttcaggtaaggtacctggtaagctttcgcaataaacggtgtagtacgcgatgcacgcggattagcttcgatcacaaacacattaccatctttaatggcaaactggatgttgatcaaaccacggatatcaagtgcacgtgcaatcttttctgcatagtactccatagtggttacctcaattggcgacaggttgaaggccggcagcaacgcatggctgtcgccactgtgaatacccgctggttcaatatgttccatcacacccattacatggaaatcagtaccatcaaaaataccatctatttccgcctcctgacaacgatccaggaagtgatcaatcagaattttattacctggcagatgtctgagcaggctcagtacagattcttccagttcttcttcattgataacaatcctcatgcgctgcccacccaatacgtaggatggacgcaccagcaccgggtaacccacttctttcgccacatcaatagcgtcatccgtgttgtaagcagtaccgtactttggataaggaataccaagttctttcagcatgtcggagaaacggccgcggtcttccgcaatatccatgttgtcaaaggatgtacctatgatcttcacgccatttgcttccaggcgcttcgccagtttcaacgcagtttgaccacccaactgaacaatcacaccttccggtttctccagttctattatttcccagaggttttcccagaacaccggttcgaaatacagcttatccgccatatcgaaatcggttgataccgtttcagggttacagttcaccatgatggcctcatatccgcaatcctggatggcttgcaaaccatgcgtacagcagtagtcgaactcaataccctgtccaatcctgttgggaccggaaccgagtacaatgatctttttcttatcggtaggaacactttcgttttctgtatcaaaagtagaatagaagtaaggcgtttttgcttcaaactctgcgctgcaggtatctaccattttaaatgtgcggcggatacccagctctttacgtttagcgtatacttcatcttcatcacaatcgccaaacaggatagccagttgcgcgtcagagaagcccattttcttggcgtctctcagcatatcaacggaaacagtctgcaggtcgagttccagcaattgtttttccaggttcacgatatcctgtatctggtgcaggaaccaacgatcaataaaggtaagctggtgaatatgttttaccgatacgcccgccatcaaagcatcttttatacggaagatacgatcccaggttggacgctttaatttttcaatcagttgctcgctcttcatgagtgatttaccatagtaacccaatcccagcgcatcgttctcgaggctctggcaggctttctgcagggcttcggggaaagtacgtccgatagacattacctctcctaccgacttcatctgcaatcctaaagtatcatcagctcctttgaatttatcaaagttccagcgcggcattttaacgattacatagtccagtgccggctcgaaaaatgcggaagtagttttggtgatctggttttccagttcatccagtgtataaccaatcgccagtttcgcagcgatttttgcaatcggataaccggttgctttggaagccagtgcagaagagcggcttacacgcggattgatttcaatggcaatcagctcttcattttcagggttgagagagaactgcacattacaaccaccggcaaagttgccgaggtcgcgcatcataaccatcgctttgttacgcatgtcctggaaagcggtatcgctcagggtcattgcaggagctactgtaatggaatcaccggtatggatccccatgggatcaagattttccacggtacaaatgataacaacgttatcattcttatcacgcagcaattccagttcaaattctttccatccgagtacggctttttccaccagaacctcatggatcggagaagcttttaaaccacggtccagtgcttcatccaggtcgtctttgctatgcacaaaaccaccaccggtaccacccagtgtgaaagaaggacggattaccagcggaaatcctatttcctgggcaaactctttaccttccaggtaggagttcgctgttctggcaggcgctacgggtattcccagccggatcatccactgacggaactgttcgcgatcttccgccttatcaatggctttgatgtctactccaatcaggcgaacgttatttttttcccatattcccagttcgtctacttccttacaaaggttcagcgcagtttggccgcccatcgtgggtaatacggcatctatctggttttcttccagaatctgctcaatgctttccacggtcagcggcagcaaataaaccttatcggccatcataggatccgtcatgatggtagccggattggaattaatcaaaatcactttaattccttcttcccgcagcgaacgtgctgcctgggaaccggaataatcaaattcgcaagcctgaccaataataatgggtccagaaccgataatgagtacagatttgatagatgagtcttttggcatttgtgtaatctattgaaaatgaaaaaccaaattgatttttctgccgtgtgagggaacaaaaaaatcgtgcaaagttacgggatttgaaatttataaacagaaataaattttgttttgggagaagattttttgtggagatggatgaatgtagctgaatttatatagaataaatccgttatttggtagaaataaatccgacatgcaagaaatccccgaagcctggaaagctgttcaaaataaatatggaagcaaggcaatctttattaaaggtgattatatccagccgaattacagcttcaattttgactttaattatcaccttgcagaaggacatttgtctttttcctggagacacaccaagaatacctacgaacaacagcaaaaattcaaatggcacgcaatcgatgaccccaggcgacaaatcggaaacatctatgatactcagacagtgctgttaatggagctaccagtgcaaaaaaacaggttgaaaatttttactactggtccgctcatgaacctgttaaactggctatatccgggcaaaattagcacaggtcacgctaactttgatgaaaccttcatcaccattgcgaaaccagcgtccatagtaccaagtctaatgccatatctgggctttttattgcatccctcacttggccgttcattgtcgcttaatatcagttggcaagatgcagaaacagcactattctacctaagactaaaaatcaaccaattgataacagatgaacaagacctcgaattcatcctggcgaatacctttaagctgacgaatcaattaagccgatgctgataaagatcccctgatcatgatcttccgggaattaccccgttcctcattttcccgtataaatacttatcatgatttcatcttattctcctaactttatcatccgcagttaaaaatatactgcgctgcaaccccaaaaaagactggcactaaattctacgacagccctgcccgcagggaatccttcttttattttttatttaaacaccccaaaaattaaacgtcatgcgcacagctgaaattcattacggcgacaatggtcacgtagatgttgccgttcccaaaggcaccaaaatggaagacatcgccaaactgcaatccatggtgatcaaacaaatcaatccccgcggatgccaggcctgcttatccggtgttcactttaacatccgggaaaagctggaagaagtgattaaagttgacctggataaaatggcggtcatcaaagacattgctatcaaacaacaacattaatgcggataccgtcccggccttgccgggacggttcttaaacctcctcaccatgtcacaagtattatcaacaaccagggtgggccgtctttatcagcaaactattccacaattgggcgtaggcctcctctacaatcctgcgctggaactatacctggacgcatgccccggcatttgcgattacgtggagattatcccggatatgttctggacggatcgcggaaacaatactccacaacggtttgaagaaattgaatcctggatgaaagtgctggataaaatagcggcccaatatcctctaacttctcacaatatctcctactccctcggcagtgcaggtatcttcgataaagcctatctgcaaaaaatgaaagaatggcatgaacgctatcgctttaaatggcatagcgatcacctttcttttgtaaaagtgcataacgaagaacaggaagaacacaatgcaggacttgctgtaccggtaccatacgattatgaagtgctggatatgatcggtggccgcatcaatgccatcaaacgctccatcagcacacctttcctggtggaaaataatgtatactttatcgaccttcccgaacaggaactcagcgaaaccgccttccttaatgagttatcgcgcgatacttcctgtggtttgctgctggacatccacaatgtatatacgaatgcggtaaatcatcacttcgatgcaaaagcttttattgcacaactggaactggataaagtcattgaaatacatattgcaggcggaaacgaaatggccggcatgtacactgactcccacgcagggccgtgtccgccggaagtatgggaattactcgattatacgttaccgttagtacccaacttatgcggcatcaccttcgagtttcatgaatcttattttcacctgctgcaattcgacggtgttacccgcgagctgaacagggcgaaagcagcctggaacctttatcatacctgaatactatgtcacttctatcttttcagaaagcactgacggacctgattgcctccccgcaattatgcctgcagctgcggaatgatgccgctgcagtattatcacggtacgatcttaccggccgtgagcagcgacggctgcaaacagtagtgtaccagcagggcatgtcggtaagttgtaccctgtaccgggtaaacaggatcacgcccatttacacgatgcttccttatacctgttttttactgggcgggcaactgatgccggtaatagaagcgttttgggccatcgacaaccggtcggatctgcagtttaaaagggaaatcaacatctttggggaattcctgttgcagaaattattgagcggggaaatggtgaatccttacctgcgggaaattgtagtaatggagctcgccatgaatgaattgaaatttttaccgcgggaatcactgatggaaaccggtgacgatgaaacaagcctacatccgctggtcaggctggtgccatttgatcatccgccggaacccttgctcacagcgcttgcaggcatgaagctaccagaacgggaagaagataccggtgaatactggctaatgctcgaccaccgggaagaagaactttctttccgcgcgctgccccacaaaaatggagcagcggcggttgcaggattataatttgatcctggaagacatcacggctatagcagcgcccataacagcaatcatcgtaaaagccacgccaagattcgtagcctgcgctacaaacccaattagcggaggaccaaacaggaatccaaaataaccaatggtagataccgtggccagcgccattcccggcggcagctttgtggatctgcccgcagcactgtataccagcggcactactgccgatacgcccgcgcccaccagcataaagcccagcatggccggaacaaagtaaggaaagataaccgctaccagcaaaccactggcagtaagtccgccgcttatcagcagcatctttttaacaccgagccgtgtagtcaggtaatctgctatgaagcgtccggatgccatggtgctcataaaggctgcataacccgcgccggaccatccctccctgacctgtatcaccctgcggaaataaaccccgctccagtcaaacatagtgccctcgcagatcatagagcacatggcgataattcccagcgtaaacaggaaagcatccggcctgccaaataaagaaggtgcattattttcattggttacacgaaccaccagccggttcattgtgatgacgatgaggatccaggaaaccgcggtaacaattaaaaagtgatataccggcgccaggtgcaaacctgtcatccaggtaccaaaagccgccccggtaaaacccgctacactccacaatccgtgaaacgaagccataatagaacggccatacatggcctccacgcctactgcctgtgtgttcaccgcaatattggcaaggttaccgaaaaagccaaagaataccaggaatgcactcagctccagggaagtatgcgccagtccgagcaccggcagcactgcggcgtatgctaccgccgcaatcagcaatacctggcggctgccatatttcgatactagtatgccggccaccggaagggaaataatggaacccaccggcagcgccagcagcacgcttcccagcccggcatcatttaattttaatgccagctgaatatccggaatgcgggaagcccagctggaaaagcatagtccggttaaaaaaaacaaggcgctcaccgcaatacgcgtggctcttttattaatcattaccatcgatagatcgtgtaacatcttcggtcagataaaagttgaattgatcagatcacctgtattcccaggttaatataaggttttagtgatggcaggtccggattatctgtaataatcgtatccaggccagtgatatcgcatactttaaacggttccgctgtacccattttatcgctggtagccagtgcaatggttttattggcagatcccaccattacacttttcacatctgcttccccaagatccaggcctgttacgcccgcatccggatgcaaactgcagatgcccaggaagcagatatccgcccgcattttttccagcatacggatcgtatccatgccaccggccgtttgggaatctttaccaatcagcccacccgtgaaaatcacctctatgacggggtgctctattagttgcgccactatcggtacactgttcgtaataacggtgatatgaagattagcaggaaacagttttgccagcattaaagtagaagtccccccgtcaagaataatagtttgaccattatgcagatacgccagggctttggtagcaatatgtttcttatcatcttcatgatatacaatacgctccttaaaagaataaggatttggtgaatgcgggatcgctcctccccttactttgatcagctgcccgttttgcgccagcgattcaaggtccctgcgcacggtgtcttccgatacctgcaaatcgctgctaagctctgtttgcagcactttatgatctgtttgcagctttttgaggatataatccaatctttcctctctcaacatgggtcgtgctattttatgcaatattatgaaagattatgcaataatttgcagaatatcgcataactttgcacaaaatagcaaaatatggcaagaatagcaatcgacatggacaatgtaatggcagaccttacccaacatctgctggatgtatacgcaaaagaatatggcgaaataatagatccggagcgtttgaacaacatccccgaaggcagcgcattccctgaaggtgtagccacgaaaatactgagtgccccgggatttttcagggggataccggtaatggcgggcagccaggaagtagtaaaggcactggcagaccaacacgaagtttttgtagtatccgcagccatggaatttccattgtcactggcggaaaaacacgcatggctgaatgaacatttcccttttatcagctggaaaaacatagtattctgcgggtctaaaaccattgtggaagcggattacatgattgacgaccacgataaaaacctgtctgcttttaaaggaacgccactcctgtttacagcaccgcacaatttaccccttaccgattacagacgggtaaacaactgggaagaagtagctgaatattttgaattgagtgctgtaaaaaatgaaaaccatttgctggctgtgagctaacaccggattgatcccggcttacctggattccagggtactgatccttttttcgagggtgcttaccttgcggacgtactgttgtacctccatacatttgtccaggtaggcttccacccagttaacctcctgctttatagcaggtggaccggtaaagtaaccgggtgataattgcagatgttcctgtaacagctccaactgcttgtcgctaaataccgcagtatccagccattcatgcatattatttaacgatatgtgcaattgagccgccagttgctcatctgttattttttgcttcgcaagatataattgcagcagttcaccctgatggcaggtatttccttccagtgagttccagtggtaaaaatcctccagcgtaacgggaacagcttccagcaatatatccagcttttcctttttaatagctgcctgcgaaaaataacgatacaggccttgcggggttaatttaactttcttagcataatgcaggatcacaatttccttttgcctcagtatacgccgcaacctggcgcctgcatgaacataatatggaactgacatttatacgattcctgttttggtgaagaatggggtgtgtatacaaatataatacttttatattctcaaaacagcggttgttctcttgaattttaaagcacactggctaaaactatcaacaaatatcattataacaaactggatgctattttaactattttgtttgcggaaagccgccagttctttctttatctgcagcaactcatctttcagtgcagcatgacttttcagcaactgcgtatattcttccagctgcttataatacttttccctaagcaacatcatttcttcgctatccgtattacgggcttcctgcacggtaccggggttaagaaaggcatccacgctcatatccaatcctttcgccaccctgtccagttcgtccggcgaaaagctttctttctcaaataagttatacatggtacggcggctcatatccaaacggccggccagtttgcttttattcaaccctttctctgcaatgatatgctgtaagcgttctccgtgatgtatacttttaccattcgttagctgcatcgcaccattccatctcataaattcttccggggtaataccaataagcgcgcaaaagcgctccatcgtagcgcgtttcatgtcacttttccgcaagtgataatgagcgatctggtttgtaaaaccggccatagtggcgaaatcaacaatctttatttttttttgcttcaagatctgtttcaaccggtgtcccatgtgtatcaggctcgactgcatcccttttcattttaaattataatgctacatacaggatgacctgtcgtattatcgtataatttaacaattaatatttcattctgtaaataaaaatatcaatttaacgaaaaaaatataagtccgtaaccagccctggcaacaaatatccgtactaactataaagggtatacgcaaaaaaataacaagaaatatttatcgatttaataacgatgaaatcagaatgataacaaacaggattattgtgtaaacgatacacatcatttatagattaacgaatcataaacaaaagcataataattctctcaaacgcgctactgcaaacggttacatcattacatattttttttaaagaaagtaaagttttataattataaattgcatgattataaatatatttgcttacaccttaaagtaactttaaaacatgttctactattccgacaattcatttgttaaccatatccaatcattctgaaaataatacccactatgagcaaagaaccaataaatgtgctacttgacattcataccaaactttccagtcttcctgtgctgttcagggagaaagtatgtgaagaatgtaactggagcacacccacattttatcgcaaaatgcgcggaagagataagccgaatccaaatgagaaaggaaaaatcattcctgcactcagtaatgcggaaaagcaacgaatcattgaaattatggaagaagtatttgcatccggtgaagatgacctggccaaataccggaaaccttccaaatgaccactgttgcctttcatccgccgtttgtaaaaacatcttacgtaaaagtaatcatgctccgtaaagccttgttccccaccccgggcaaacgaggctttacttttactagcatcgccttcggcgatggaaattgtcttggagcaggattacgctgattatactgatttcactgagatatcttttaggattttaacttccggattacgatcaactaagtttttctttttaaaactaaattattagttttaaggataaatacaatgtctatgaaccggattatatatcggataacccagtggtttatcagcctgctgctacttataaatatcgctaccatggccctggcacaggaatctatcgaccgcacgcagctgatggaatacctccagaaccagcaatatgaagccgccatcaactacctgcagccgcgcgtacaggaaaataatatcgggcagctttccctcctggcatatacgtactacctctcgggaaaaacaaaagatgccatgacccattatgaaaaggtactggcactggacagcaacaatgtaccggcacatcaatacctggccagcatcagcatgcagctggaaagcccgctccccgccatttttcactaccggcaaattgtccgcctacaacccgccaatgccactgcatacaaacaactcagcttcgcctgcttcgcagcacaacagccggatacggcatttttctacctccaaaaagcatatgcgctcaatccggcagatccaaaagtaaccgcacgtttcggggaagaactgatcgaaaagcagcaatatccgctggcagacagcatcctgcgaacctttctgaaaacagactcgcttcagcccaccgttatcatgaccgccatcaggtccgcctggtttctgaaaaattatacccgctgtaccgatctcggcacgcaactgatgcgcatgaatatcctgtcacccaacaccttcagcatcgtttctgctgcctggtacacgctcaaacaatacccgcaatgcatcaacgtatatgaatacgtgcaggccaataaagggcagtctgaaaccattacgtattacgcagcccttgcctataccgcattaaaaaactatacggccagcaatgaactgctgcaaacctgcatcgacatggctacctcgaaaagcctgaacagctactacagcgggaagtcggtgaactacgaaggcctccgccaatacaaatcagccgtcgccaacctggataccgcctactacctttttcaccaacccctgcaccaatacagtattggccgcatctacgaggtacatctccgcaacaaaccactggctacccgctactataaacgctacctgcaactaggcaaccctgctaatccccaggaagcagatatttacaaatacctccgctcatatgttgaaaaataatctgcttttaatatgattttttagattatctctaccaaaccatctggtttttcttaaatttaaagcccgttaggaaaatgcttgtacttaaccaataaacaattacggtgctatgtcgtacccataccagatcaagagtatcgaagattatcagcaggcttatcaacagagtgtgattgacccggaaggcttctgggccaatgtagcagaccatttttactggcgtcgcaaatgggacaaggtattggactggaacttcaaagacccggaaatcaaatggtttaccggcgctaaactgaacattacagaaaactgcctggatcgccacctgggcacactgggcaatactcccgccatcatctgggaacccaatgacccggaagaacaccaccgcattatcacgtaccgcgacttatacaacaaggtttgccagtttgcgaatgtgctcaagaacaatggcgttaaaaaaggcgaccgtgtatgtatttacatgggcatgatcccggaactggctatcgccatcctggcctgcgcccgtatcggcgctgttcactccgtagtattcgggggtttcagcgcacagtctattgccgacaggatacaggatgcccagtgcagcctggtaatcacctgcgacggcgcatatcgcggcgcaaaggatatcccgctgaaatccgttatggacgacgcattgatggcatgtccatctgtaaaaaaagtaattgtatgtacacgtacccgcaccccggtaagcatgctgaaaggcagagacctgtggtgggaagatgaaataaaacaggtagaaacaatgggcaatccgccctgcccggcggaagaaatggatgcggaggatctcctgttcatcctttatacttccggctctaccggcaaacccaaaggcgtggttcacacctgcgccggctacatggtatacgccaactataccttcgtaaataccttccagtaccaacccggtgaagtatatttctgtacagcagatatcggctggattaccggtcacagctacattgcctatggtccgctcagcgcaggcgccaccacgctcatgtttgaaggggtgcctacttatccggacgcaggccggctgtgggaaattgtagataaattccgtgtcaacatcctgtataccgcaccaacagccattcgcagcctaatgagctatggcctcggccctgtaaatcataaagacctcagctccctcaaaaaactgggcagcgtaggagaaccgattaacgaagaagcctggcattggtttaaagataatatcggcaaaggcaaatgccctatcgtagatacctggtggcaaacagaaaccggtggtatcatgatcacccctattgcaggcatcaccaaagaaaaaccaggatacgccaccctgccactgccgggtgtacaaccgatcctggtagatgaaaatggtaaagaactcaaaggcaacggcgtaagcggaaacctctgcatcaagttcccctggcccggtatgctgcgcagcacctacggcgatcacgaacgtttccgtaaaacatatttctctacctacgaaaatctctacttcaccggcgacggctgcctgagagatgaagatggctactatagaattaccggccgcgtggacgacgtactcaatgtaagcggtcaccgtatcggtacagcggaagtggaaaacgccatcaatatgcacgccggcgttgtggaaagcgccgtggttgggtatcctcacgatattaaaggccagggcatctatgcttacgtgatcaccgaacgcctcacgcatgatcctgaactgactaaaaaagatatcgcgcaaacagtggcccgcatcatcggtcccattgccaagccggataagatacagatcgtaagcggtttgcctaaaacccgttccggtaaaatcatgcgccgcatcctgcgcaaaattgccgaaaacgatatggacaacttaggcgatacctctactctgctggatcctggcgtggtagacgaaatcaaaagaggaaaactgtaacagcttcaaagcttttaaaaaacaaagggatgcagattattttgcatccctttgttgtacctgattatactatgaagcgttttttcaaaaagctggcctggacctgcatcatccttttcgtattactcaatatcatcggggcctttcacgcgtggaagtttacccacttttatgacgatggcggccgcaggaacaaactcccggaacaaatgagtacgggtgaaaagataaaaaccattttgtttggtgtacgcattgccaaatccgctaccaccagtttcccatcagtaccttacgaaaccgtattgctgcacactgccggcggcctccggctggaaggctggtggatcccagccaaagcggctaccggcacagttatcctgttccacggttacaatggcaataaaggctcactgttgccggaggcaaatcgtttccgcgcgctgggctacaatacttttttactggattttcgcgcccatggcaacagcgaaagatatacctgcagcgtaggctacaaagaagcagaagatgtaaagctggcgtgggagtatgtaaaacagaaaaacaagcaaccggtgatcctgtggggagtaagcatgggcgctgccgctattttaaaggctgttcctgaatacgggctcacaccaaagcaactcatcctccagtgcccgtttgctacccttacagacgctgtaaaaagcaggatgcgcgcggtgcatctgccggcattccctttttcacagatccttaccttctggggaggaatagaacaaggtttctggggcgccggttttaagccggaaagctatgccagccaaatagatatgccggtattatatttttacgggaaacaggatatccgggttacggaacaggaaacacgggaggtatttgctcatttaggtacccggaaaaaaaaactgtatatcttccccaacgccagacaccagtcgttttgcggcaaagattccacaacctggatgaaggaagtcactgcttttctgcaaccataaaaaagcgcgcaccatacgagtggagcgcgctcttcacaggatctgacccgccgtttatatttgagtcatggtgcagtagtactgccccactagatgccgtaccggtttgtggtggatgctaaattacaacatgcaactgccaccgggagtcactgcgaaataatcagcaaaaaccttaccggcgaataaccaccggggttcccactttgattacctcgtataattcgttaacatctgagttcttcatactgatacaacccagtgtccagttaatacgtccttccacataactatcccagataccggaattatattccactccgtggatgccgatagccccgccaatactggcactggaggagaccatgccctgtgactgacggacacggaacttctgccaggacacctcattgggatagtccagcagcatgaacctgctccagcttttatccactcttttggttaaaatatggaaagttccttccggtgttctgcgatcaccttcaacttgtttatcggtttggtcgcggttaccaaataccaccttgtagatttttctcaacgtcacgtcttcgtatacatacaaccggtaatcgcttttatctatcagcaggaaaattttatcaggatcaatgttggcagcatttaaccttacactatacaaatcagattcgttgataaatccacttagcggcagcagcaacagaacagctaccaaccagtaatgacagcacttcttcataggagtaataaatatgcagataacgtagcagaataatcatttattgtttgggagatggttgaaaatacaaaggcacaaagcgtaaaactttgtgcctttgtattttatcagattttttcttacggtaatcagtagccgaagatctcttccagcgtgagcttcttcacatcgccatattttttcagatcgtctgtgctgatcttcttttcagaagcaacaatacaataagtatatggtttgtgcgccaggttctcatcatggaacttcttcacttcgtcaaagttcattttgtcgatcgactcgtacacctgtttgcggatatccgtatttaatcccagcttctgtgcggcgaggaaactgaaaacaattccatcgttggtgatacgttctgtttcaatatcctgcttcatgctttccttagcagtttgcaacagtttatcggcacggggaatatcattcagcaattcgttcatacctgaaatggcgtcattcattttatctgcctggctaccaacgtaggccaatacagaataacggtcgtcttttttatcgggagatgcgtagtaggcataggtggaataagccagtgctttggactcgcggatggtttggaatacaacagatcccattccgccaccgaagtagctgttaaacagcgtcaccacgcctgtgttggcaggactgtatgccgctgaattccttacccagtttacttctgtctgcaccatatcataatctgcaaacagcacctggcttttatcctggttatctttcgcaaattttatagcttccggtgcctgcttaaaggttgccggcagcgggtgcagtttctttacttcagccgcggcagcagccagtggctgaggcccccagtaaataatggtatgcttgtaagcaggtagttcatgcaaaatagtaacgagttctgatgcggtaacaccatccagctcagcctgacttaactggttattaaacggattttttgcgccatacattgcatagtttactactcctttcataattgcgcccttattcagtttgctgtcggagcggcctttctggatgcggcctttcagtgctgccagcgcgtcttcattaggtttgcagttggcaatcacatgttcaaataaggtaacggccttatcaaaattttcctgcaaaccgctgatcaccaccgtggtgttttcagcagaagcggatacgctgaagttacaggcaatgttataaaactctttgctgatctgctcagaggtatatttgtcggtgctcagatattgcaggtattgcgctgccagggccagtttcttattgttccaggtacccatatcgaaacggtagtacaggtggaaaagaccattgtctttgttctgtacatacatcatatcagtattacctatcgcggttttctggatatctttttcataatccagccactgtggctttaccggtgtggcgggcatagcagctacctgttgcaggaaaggcgactgtgcttccctgtttacttccaccggggtgatggcaggtttttcaaccttttcgatgttcttatcttcgcccttgcgtttgtaaacaattacatagttatcattgaggaatttattggcgtaatcaacgatttgttttttgttaaccgtgcccatatcatccacataggctacatcatataaccagttttgacccctgctcttaatgaatccgtccatcagggcggtagcgcggttgttattgctttccaggccctgcagttcgctcagcttggcgttattaatgatggctttcaccagggtttcatcaaaatttcctttcttcaggatatccagctgacccagtaaaagcgcttttacttcttccagggtttggccttgtttggctttaccgctaagtgagaagatggagtagtctttcaggccaagtacacttacgctggcgttcagtactttttgctgcttgttgatattgagatccatcaaaccggctttaccattctggagaatggaagagagcacacccagtaccaggttggatttggtatcgagggcgccgggcattctgaaggcgatatctacgctttctgcatccggacccagtacttctttcattaccggcgatttgatcggcgcttccggggcaggcttgtattcctttaccggtttggctttcatatagctgaatttctgatcgatagatttaatcacataatccggatcaaaatcacccgccattacgatggccatattattaggcacatagtactcattgtagaattcgcggattactttcaggtttggatttttgagatgttcaacggtaccgatggtagattgctggccatagttatgggtaggaaacagggctgcgagcatggtttcgtacactttccggccatcattatccagtccgcggttcttttcttcgtatacggcttccagttcggtgtggaacaggcggaaaaccgggtcacggaaacgctccgcctgtacggtcaggtatttgtcgatggcattggaaggaatatcttcctcataaatggtttcttctacccaggtatgggcgttggtgccctgtgcgcccatgcccgacatcattttgtcgtattcattggcaatggcatatttggcggctactccggaaacgctgtctatttcatgataaacagctttacgggcagcagggtccactgttttattgtatttatcatacaaattggagatctcatcgatcagtggtttttcctttgcccagttgagcgaaccaaatttttcagtgcctttaaacaggaggtgttcgaggtagtgcgccaggccggtgtggtcttttggatcgttatcgctgccggcgcgggtaccgatcaatgtctggatgcggggatcttttttattgacactcaggataactgtcaggccgtttttcagcgtataaaagcgtgccttcatgggatcatcggaaacgtacttataggtataaccgccaccagtagcctccttccattgatattttccctgggctcccgctactttgagcgagcaggcaaacaggaatagtaatacgactcttttaagactcatacaaatagttggttttttgaaattagtctgtcaaatataccggaagtcaaaattataaagcgggaaaaaaagggagaattgtatgagcggtagatgcataggaattgcaaccggttgcctggccggtgatcaaattaacaagaagaggattgatatcaggggttctggttattataaatggtatactttccgcgcacaaaaacctggttaagcagcagcgagtcaatggccatgctattaccggcctgttttttcgctttcgcccggcgcctgttatggctaacgggagcggttatggtattggtggcaggaattacctgggaaatgtacctggcagcgggaatgctggctggtgcaactgctacgggcaactgctctggctgatcaataagtaagttatttttttcgagtctaacgcctaacaaacgtttctcacaggagtgaatccatgcaatgcaaccaatacatgtcatcaaagcaacaaaagaacgcataaacacaatttaggactggctaataaatcttagaatccgtttaaccggatacctattgaaaatggatactgttgtaacccatagtcatgtaatgccgtaagggcaaaatttgcatacaactttacaggtccatagcccagttcactggtaaggccgaaacgccacttgttaagattaaagtcgtccgtttttctaaccttgcctctttcttcacttacctgcttggttctggatttgaggagataaccaccagagacaccgaaactcgcctggaacgcacggctcgggcgggcagggttagaattaaaattaagcattaccgggatcgatatatattcggcaaacagcttattttttgaaaattctacggaatctctgattatttgtgtaggataacccggtaaatacgtaatgctccgggcatacctatagttattcatctctaatcctaaagcatataacaagttaagtttgtgttttgttatattaagtcgctgttgaaataaccagatattaaaattgattgattttccggtgattagcttaaattctgaaggcgtcaacggcgcactggcatcccttggggcaaaagtggcgaggcctacggcagaataatcatatgatttagacaccggggcaggtgctccattgtaataagcgctgttattggggtagtaattaataaagctggctccgttatagtcgctgtgatcaatataattgttgaatcccaggtcaaaaacgaaccatttggtttgcaggttctttttgagcttctggcgggcataggcagtatcgttatagaacttataactggttcggcccttatcattctttcctttgataatgatcaatcctttgatctgtatggtgtccggtggtgccggtgtagttttatctgccttttgcgcatgagcccacccgccacataataccagtaacaaaatgagtaaaaatttatgcttcatatgctatgaccatgatttattatttattccttcttcgggaaaaaagctttgcaacattggttaccttatctaaaatccggctgtcgctgccacttacagacatgatcaactcaccgggagcgcctggctgttcggttgcaggaactattttattatttaaatgatcgtttgtattggtattggctgccagtaccgcttccttattaacttccggccgaaccgccacaacatgggcgttaccagcctgttgcaggtgctcttccactacttcactcatagagttgcgctgcggcggcaactgggaaataaccggcaaatctgctttgggtacgtctgcggcagccagtgcaggctcatttgcaggagcggcaactggtttgttttcacgtggcgttacggctttatggttttgggccggtacgggttggttgctccgcggcgcagcaacaggcgcattttgtgttgcagctgcggattggtcaggagcaaccggcgtagttacttcaggagttacggctggtgcaggtacagtaaccgcaggtggtgtgtttaccgcaatggcaggtttttgtgctggttgttgatcgctggctggcaataaccagataagcaggcccgctactaccgcggcggcagcagttgcccacatcatgcggcggtataccggggtaacccggcgtttgctgcttctgtaaagagatgctttatcagcaaataccaaagtggtatcaggtaccagcctggtggcctccaataatgccagttcacgctgcgctgccggatgttgctgcaggtattcctgcaaagtggcttcctcagcagcggtcagctccccgtcgatatggctcagcattaatacttcgtaatcaacggcagctgttttatacaaagcagctttattatcaaaaacaacgtgtttatccggcgtcagtttcgctccttccagcagttccagttcctgacggaaaggaggatgcttttccaggaaacgttccagtgcagccagctctgtctcattcagctcaccatcaatgtagctgaggagataggactcgtagtttgatatgttaatttctatcgacaaaaatctaatttattataaaaatattatataacattctccatttttaccaggtagttcttcagatgtatcctggccctgtgcaggtaaacctttacctgcgaaggattcagctccatcatttctcctatttcctcgtaggaatatccttcataatccttgagcataattaaggagcgctgtacttcactgagcttggataatgctttttctatgacttccttcgcgttatgtatcttatgatccgatactttatcctcgtctttgaactggtctacaagtgtgatccgctttaccttacgtacatgatctatcatattgtggtagccgactgtaaacaggtatgactttgccttttcaaaaggcacatcctggcagtgcttccacaatatctcgaatgaattctgtactacgtctctggcatcttccgcatgctccagattctttactataaagcggaataaattgtccgaatacagatccacgcatttattgtactccttttccgtcattccggtggtgcgggattttagtgctaagttccgacaaatactttaatacccatcattgaccaaatccatatttgttacccacacctactctaaagctggtacattcttccccacagttgtagtaacagttcctttcaaactgagcatcaacctcttatcaagtatgctcttttagcatcttttaccaaaggggtgaattatcagttttccacttcatggcatcaataatcatgatagtactatgacggagggcggcgggcaaatgttacacctgggtcaaactttttgcttatccggtcgttactgatttacgcgataaataatcgtaatacatttattgccataactttggtagatccactttaaatattgcaatttttatgaatgagaagtttataacccgtttacgggaggaactcggcgatatcaataaagccggcctgtacaagagagagcgcattattacatctgagcagggagctgaaatacaggtgggtggcaaaaccgtgcttaacttttgcgcaaacaattacctgggtctgtcgtcacaccccgctgtggtgaaagctgccaaagatgcaattgatactcatggctatggcatgagcagcgttcgttttatttgcggcacacaggatattcaccgggaactggaagaaaagatctccaaattcctgggtacagaagatactattttatatgtagcggcattcgacgccaatggtggcgtatttgagcccctgttcaatgaacaggatgccattatttctgatgccctgaaccacgcctccattatcgacggcgttcgtctctgcaaggcacagcgcttccgctacgagcataacaatatggccgacctggaggcaaaactgcaggaagccaaagactgccgcagccggatcatcgttacagacggctcattcagcatggatggtaccattgcccagctggacaagatctgcgacctggctgataaatacaacgccatcgtaatgtccgatgaaagccactcttccggattcctgggtaaaaccggtcgcggtacccatgagtaccgtggtgtaatgggccgggtagatatcattaccggcaccctcggtaaagccctgggcggcgcctccggcggattcaccagcggaccaaaggaagtgatcgacatcctgcgccagcgcagccggccctacctcttttccaactcagtggctcccagcattgtcggcgcttccatcgcggtactggacatgctgagcgaaaccaccaccctgcgcgataaactggaatacaataccaaatacttccgcagcaaaatgacggaagccggatttgatatcaaaccaggcgaccaccccattgttccggtaatgctttatgatgctgtactgagcgcccagtttgccgacaaactgctccaggaaggcatatatgtaatcgggttcttcttcccggtggtaccaaaaggccaggcccgcatccgcgtacagctcagcgccggccacgaacaggaacacctcgacagggccatcgccgcctttaccaaagtaggtaaggaactgggcgtgattaaataaaacttgctgccgtacccggtgcataaagattgagtatgattaaataagactgcgggttagtggggagatagacgccggaataatcccggttgccatctccctgctaacccgtaatcgtttttcttacgccgtaattcttacttttgcacctcataactactcaatcattatgcagatgaaacgatttggttggatgttgctggcggttggcctgttcctcgctgcctgcgcaccgaataatgtaaaagaagaacaagactgggaaaaatattttgccgaatacaaagtagaaggcactttcatgttattcaacaacagccagggcacctttaaagtatataacctcgacagggctaaaaagcgctttcagcctgcatctacctttaaaatattcaattccctcgtgggcctgcataccggcgttatcaaagataccagcatggtaatccgctgggacagcgtaacccgccagtttcctgcatggaaccaggacctcaccatggcccaggcatttaaacaatcggccgtaccctactttcaggaagtagcccggcgcatcggccagccaacgatgcaactgtggctcgactccattaagtacggcaatatgaaaatcagccgcctggatactttctggctggataactccctgctcatttcaccggatgaagaactgggctttgtaaaaaaactctatttcgaccagctgccttttgcaaaaacaaccatgaaaactgtacgggaagtaatgctcatggaaaaaacgccgaaatatgaactgtcttacaaaacaggatgggattataacgacgtaaaaaaattaggatgggtagtaggatggattgaagaaaacaggcaccctaccttttttgtgctgaatatagaaacagaagatcctaaagtggatattcctaaagtacggatggccatcctgagaaacatcctcacagatgccggttactttaagggcgaaatgtagcaattcgggcttaacctgcccggcctggggaccgggatcgttaaaaaaacgataaaaccccactcctacagcttgcaatacgtgacaaaaaaattatttttgataccttacctggtgtactcccggtaacggttatcttaaaatcgaatatgttacgatttcagcatagtgaatatttatgggcactggtgctcctgttggttttacaggtggccttcctgggcgtgtcgtggtggaaacgccgctctatacgccgcatcggggatcaggcactggtagaaaaactctttaccggctactcccgcaaactgtttatattaaagttcctgcttattttcctggctttcttcttcggcgtagttggattggccaacctgcagaaaggcagccgcatggaaaaaatcacccgcaaaggcgtggatgtgatgatagcgctggatgtaagtaaaagtatgctggctacggatgtgcagccggaccgccttacccgcgcccgccagctcatcagtaagctgatggataaactggataatgaccgcgtaggcctcgtggtatttgccggtaacgcttatctgcaaatgcccctcaccgttgattattctgctgccaaaatgtacctcagcaccgtatccccggacatgatccctacacagggtaccgccattggtcaggcaatacaggtatccgacgacgcttttaacaaaaaagaacgtaagcataaagccctcatcattatctctgatggggaagatcatgatgaaactgctatccagcgtaccaaagccgcttttgagaacggcgccgttaccaataccatcggcatcggttctgtagcgggttctcctctgccggacccggaaaccgggagctataaaaaggacagggaaggcaataccgttatttccaaactgaatgaagcggagctcagaggcattgctgccgccggcaaaggcatttatcagcacctggataataataccgacgacgtagtaaatacccttgtcaataagatagacggcatggagcagaaagaatttggagagaacgtattcaccgactacaacagttattttcagtatttcctgggtgtatgcctggcattgctgctgattgaattttttattcctgaagttcgcttcaagcgcactcctgaatcaccggcagtttaattcattactcatgaaaatcatttttataaaatatagtttccttattgcagtaatgctcgccagccttaccggcttcgcgcagaacggctccaataagtatatccgcaaaggcaacgaactgtataaaaaacaacaatacaccgatgcggaagccaattacaaaaaagcgctggaacaaaacgcccaatccgccgaaggcagttataacctaggtaactccctctatcagcaaaaacgttacgatgatgcacgcgcgcaatatgccaacagcctgaaactgggtggcaaaccagccatcaaatccgacgctgattataatatcggcaataccttcatggaaggcaaaaaatgggaagaaagcatcaaatcctacaaacaggcattgaaggtcaatccctccgatgaggatgcccgttataatctcgcctatgcccaggccatgctgaaaaaacaacagcaaggcggcggcggcaacgataaaaaagataacaaagacaaggacaagaataaagacaagaacaaaaacgatcagaacaaagacaaaaataaagatcagaacaaagaccaacaggataaagacaaggatcaaaacaaagaccagaacaaggaccagcagaataaagacctggacaaaggcgataaagacaaagaggatcagcagaagccggagccacaacccagcaagatgagcaagcaggaagcagaacgcctgttgcaggctttatcacaggaagaaaagaaattgcaggacaaagcgaagaaagtaaaaggtcagattgtaccaaaagacaaagactggtaacattttcatcctctccatatcaaacatcccaaagctggtagtcccgctttgggatgttttatttaggcgcagaaggtacactgccggtgtatttcttatatgccttaatgaaatgattctgatcgtagtagccattatccagggctataccggttaatggctgcgccgctttatgcacatcgctccacgcatgcaaaaaacggatattactgatataatgtttgggagtaacgccggtggacatacgaaaattccgctccagccatttgtagtttactttcagggcttcacagatatccgctacggctatttttcctccacattgccggatcatcatcgccgccgtttgaagcaggtaattacccatgacgttgcggggtatccatcgctccaggaatgcgttcagcaccccggattgccgctgcggggatccggccgctcttatctcctgtaacaatggccgccatgttgccggtaacggcgccaatggcgcgtccgtttgcggcagcagtggctttaaccaggcccacccatctgctgtaaattttactaccagcagtcgggcgccgggggtaatatcttcgaggtaagtattttccaggattccgctgcagaaaaaaccctcactaatagtaaagttatgccgcccggtaaactggacgctacgccggttcagcaaaaataccaacgccggttgcccgtctaacgcagccaatattttcctgttgtgtagctgtgtataccagcaatagcattccaccacccgcaacagtgcagatgatggcggcaaggatctcaccgccgctgatggctgatgacaaataagatgtgcaagaatatctaccggcataaccatccaaaattaggaataaaccagcaacccattttacaagtgtctaaaatttactattaccgctgtttccttctgaatttctttgcagaaaagaaagaatatgatcctgccgatcatcgcctatggcgccgctatattaagacaacgatgtgaaataattatgcccgcaacagccggcacaggggaactgatccgtgatatgtggaccacactggaacgggctaacggagcgggtttggccgcaccgcaggtgaacaggccggtacgccttttcattgtttccacagacgattttaaaaatgtatttattaaccccgaaatattgtggtacagcgaagacaccacctatgatgcagaaggttgtctcagcattccggatatctgggaagatgtgccacgcggagctgccattacaatacaataccaggacgaacactttataaagcacaccgccactttcagcggaaacatcgcgagggttatacaacatgaatatgatcacatcaacggaaaactccatctcgattatctatctcccttaaaaaaaaagctgctgaaaaataaactacgggccatcacaaaaggcaaggtaaaaacagcttatcccatgaaattcctttaaaaaactcaaagcaatccatctaatcctcctaatcctgagtaagacaacatacgcgcataaaaaaaccggaataggaatattccggccgttttacctaaacctacaattgttacgcggcgtaacaattctcttcgtgttttaaagcaacagcgccccttgcggaagcgctgtattgcctgattcatcagggaagtatgtttgcctgctatccgtcactctttaccttgccgaatacagtctgttaaatgattcttttgtccgttgattcctgtttttttctgacgattcatttacctgttgatccatttttcctgcaaacaacttcccccctttaaacacacattattttgcaactgccgttaacggcgttccttcttttatttcatcactgccattctgtaccagctggtcgttgtcggacaaatcaccaaaaacctccacctggccgttggattcatttccacatttcaccgggatccacacggctttgttattcaccgacttaatcacaaataccctttctgaattactgatgatggcagatttaggcacgatgtacacatctttcttgcccggcattggcatcagcacttctgcatacatacccggaagcaggcgggcttctttgttggccacatccatttccagtatttcagaacgcagctttacgtccaggctaccggctatacgggttaccttcgccgtaaaagtgtctcccggcaaggacttcacggtaaaacgcacgtcaccggcgtggtgggcatcatctgtatagatctcaggcacggccacggacaaacgcagtttttgctgttcttccaaacggaacaacggtttatctgaacccttgcctgcaggacctacgtaagtgcctgggtgcacattacgctggctgatcactccgctgaacggagcgcggatcaccaggtagcccagcatttgctgtacttcatggtaagaagagcgggaggataacaattccgcgctatcggcgctcattttctcaaacgccatatccaggtcgttgggggaaatggtacccggcactttactggttttgagcaaacggtcgtacgtggcacgactggcgcgaaacatcgcttcctttgtatgaagcctggattgcgcctccagcaattgtgtattcatttccggcgcatccagcgttgccagcacctggccggcagttacctggctgcccaggtctacatttacattttttacatagctgttcacctttgcatagagatcggcaaattgaaacggctttatttctccgggtaatttcagggatgcatccagctggcttttttgcaggtgaataattttcacctgaacacctccgtcttctttttcattttcatcgtctgcccgggaactgtgacaggaggtgaaatacaaaccggcagataataatgcagcagctgtcatgacccgatacgacaggctgtatttatttatattcatgatattgatatgtcgtttagtcattatagttatacctgtgttaaacgcgtgccgctcccggaacataatacgggctgttttcatcttcagggtccagtgataccgatttcacggttgacttctgctgtacccatgcgaagatcagcggtaaaataaacagggaagcaaaagtgctggctatcaacccgccaattaccgcgcggccaagcggcgctgtttgatcgcccgcttcacccagtcccgatgccatcgggatcatacctgctaccatggcgatgctcgtcatgaggataggacgcagccggatagaagtaccttccagtgcagatctgcgggcatcatgattttccagccgcagcttctctgcgttggtgatcagcaggatcgcattggctaccgacacgcccaccgacataataatccccatatatgattgcaggttgagcgtagaacccgtgatcagcaacatgatcagtgaccctgccagtaccgcggggatcgtagacaccaccaccaacgctactttgaacgattggaaattagccgccagcaataacaggatcacaataatggctaccagtaatcccgactgtaaactatccagtgtttcattcagcaggttcatcaaaccgcgcttctctacggtaataccacgcggtggctcgccggcacgtttgatggccgctgctacagcagcagaggcattgcccaggtcttttttgtgaatattggcgccaatagaaacaattctcacagcgccgatacggtcatattctcccaccacggtatccggctgtaacgtagccacatcccccagtgaaggccgggtgttgtttttgctgataggaatagcggccatatcattaatactcgacatctcattttccggtacggagatctgaacaaaataagacgttgcatttttctcatccagccagttatttttttccgtaaaacggctggaggaggtggaagctgtgagtgatttagcgatgtctgtaacgcttacacccagctgtccggccctctcccggtcaatgtttatccggatagccgggtaatccatcgcctggttgatctgcacgtcccgcaggtagggaatcttcttcatttctgccaatacctttttcgcatagggtacgctttctttgagatttttacccatgatggcaatttcaatcggcgtagaggcgccctggctcattaccttatcggtaagatctattggctcaaagctcatcttcacttccggcatctgttcatggatccgcttgcgcagcttttctttgaactcatccatgttgatcttaaaatcctctttcatgttcacctgcaacacggcttcattaggcgtagccataaacaggtaaatggggttggtagaataggacgatggatgagtaccgatgaaggaagaagtaatgtcgatgtttttggcgccgaccacctccttcagaatttccgtggatttaataagcatggtttccgtccgttcgaggcgcgttccggtaggttctttcagccttaactggaactgcccgttattcagtttaggtaaaatatcacggcctataatactcatacatagcgctactataccaaaaaccccaataaagtaggcgccaatcaccagcttccgtcttttcagcagcgtttccagccagccgataaagcgcagcttaaagcgatcgaagccggaaatagttttggcgtgttgcttttcatctgcaatttctgtttcaatatacccggctgttttatgcacgtcgttgctaggcacatgtgggtggccatgatgcttgaatttattggcatccagcatccagttggcgagaatgggcaccagcgtttgcgacaacaggtaagaagcgatcatggaaaagccgatggccagcgacagtggcataaacatcgcacggggcacgcctttcatggtaaacgaaggcgcaaacaccgcaaggatacacaacaggatcaggagttttggaaaggcgatttcctggcacgcatgccagattgcctgggctttgggcttccccatttccaggtgctggtgaatgttttcaatggttaccgtcgactcatctaccaggataccgatggccagcgccagcccgctcagggtcatgatgttgatcgtttgcccgaagagcttgagcaacattacgccaatgatgatggataccgggatggtgatgatcacgatataggcgctgcgccggtcgcccaggaacagcaataccatcagcgccgtgagtacagcgcctattacgccttcactgataaggcttttcacggcattgatcacatacacgctctggtcaaatacaaaggaaatctttacatcttccggtaataatttctgaatattgggtaatgctgtcttcaggttatttactaccgtccacgtggaggcatctgcagtttttatgataggtagatatacagagcgctttccgttgatcacggcgtagctactggtgatgtctgcggcatcttctacctttgccacatcccgtacaaatacggtagggccatctcccattaccagcggaatattctcaaattcctttaccgtgcgtatcacggtgttggcgggtgtgagataagtgatatcgccgatacgcacgttgccggccggtgatatctggttattatcttttatagcggctactacctggtcggccgaaagatggtgactgcgcatcagttgcggatccacatggatcacgatagtgcgggagttaccgccaaaaggcgcaggtgaagtaagcccggcaatccggctgaacgatggacgtacgacggtcatagccagatcctgtagttcattattggtgcgtgtgggactgctcagtgccagctgaccgattggcaaggtggatgcatcaaaacggataataaagggtggttgcgtacccgaaggcatcgatgcaaaggcgcgattggccatcgctgttacttccgccgcggcctgggccatgtttgtcccttcgtaaaaagagatcttgatcatggtaaggccctggatatttttggcctcaatatcttttacgccggttacatacaggaagaggttctggtagttggtggcaataaagccttccatctgttgtggcgacatccctccatatggctgtgatacgtatatagccggcaggttaagatccggaaagatatctattttaatatcccgcgttgcttgaataccaaaaaacaatagtcccatcactaccacgatgatggctatcggcttttgtaatgcggttttaatcaggttcatacagttatattcaggaaatgatgctttccggttaattacagttgattcaaaaacaattgcagatcccctacggtagcggatttatacaatatcgcctgccacacgccattgtatgcaatatcccggtctgtttccgcgcggttaatattgtacagtgcctgggccaggtcggcaatattggtcaggccgttctcatacagggtacttttctgcaggaaggcgtcgctggcggctttcaggccaatgggcgcttcccggtatttcttcaccgcattatctatctgttgttccgacagctgcagctgatgttgcaaacggctgtaggtttgattgtattcattttttaatccttctgtggtgtagtgctgacgggcaacctgcgaatgtgtgcgccacagatccgtcaccgtccacgaaagattgaggcccacgaggtaattggatacctgcggcttcacgcccgaccagtatgcctggctgtagtggctgagattagcagcgccatagtcgtagtcaaacccggaaccgcgcgtttgcatcacacccataaaggacagtcgcggcatggcatttttgctgatcagcttttgatttgcgtcactcaatgttacgcgcgaactgaacagtttcagcaagggctgattcttcagtgatacagaatcctgtgcagacaccgtttccagcagctggttaggtatcttggtaataaacgtggtatccagtgtaaagtcctgcgcaggcacgtccatcatttccgcgagcttgttgctttgtgcattttcgtaattcacagcgtctaccagtgtcagtttcgctttggatacttctgcgttggcgatggagctgtctaccccggcactgagcccgttcaatgcgcgggaaacaatgatatgctgcagatcctgcgctcgtttcaggttcgattccatggagccccgcaaccgctgtgctgccagcaggttaagatatgccccggcgatgcgtacctgctgttcaaatttctcctgttccaggtcggcctggttggtatacaattgttctttcgcggcctgcacttttgcgtgctgacggccaaaggtgactacatcccagctgatattggccaggtataatccaccgaaggcggcattccagttctgtgatggcagggccggcccggaagcgccggtagtccagcctttatatccccacataggaccattttcaccattcacggtaccataactattctgggcggcaaggttcagatcaggtaagtattctctttttactgcactgatattttctatagctgctttagcatagttttcttttgctttgatggactgataatttttcaatcctgtttgtagtgcttcctgtaaggtgagcgggcggggctgacccatcacggccaccgaacagcagcctgcaatcaccagcaggcaaagcggtttccagatgttcatatattaatctatagcgtcttaaaagccgactgatgcgggctcacaaataagaatgcaaatatagaacggggtaagtggcgggtgttaggacaaatcagctattgacttggactatttgaacatcatatcccggaaatcctggggagagataccggtattgttcttaaaaaagcggctaaagtaagcagggtcctcgaatccaagctcataacagatctccttgacacttttgtgactgaaggccaggtttcgttttgattcgagcacaatccggtcgtgtaataattcggtgacggtacgaccggtggtttctttggtaatttcgttcagccttttgggggtgagggcaaaggcgcctgcataaaaggccacctggtgttctgtgcggtaatgttgttccagcaggcggcgcagctgcacaacacgtgcgtcgtgcgccagcggcatcatggtttccgcggcattgcgtttcttttcccgttctatcagcaacaggaaggcattcaggtaatgtttcacaatgccctggctgccggcaggcgcgcaggatttttccctgctcatcagttgtatcagccccaggagagactccgaggtatggccgctggtactgatgggcccgtatccgtgccagttatcgaaaagcgaagtaaaatcgtaaagggtttctttatcgtgcttattggtaaagtaaaattgttccgtgaaatacaggaaatacccttcccgctcacaatccagctgatgcacctgtcccgggcgaagcaggaagatcatatcatcttccacttcataccacacgaaatccaccatgtgccgtcctttccctttggtgatccatataatctgaaaatgatcatggcggtgaggctggtccgttaattcattgcggaacatgcccagggaagctacgttgaactgcccggaaaagggcaattgctggtaaggtatatctatgcttttattcagtaacatacagtggctcaaaaatacacttttatcccctatttgtgccctttggcgcccgccgttcgtggaatttaatgtagctttaagctgcggctttattataccacaggtttactaactttgcttccgcaggaaaacaaaaacaacgtatgcagctttattgcaactctctgacagaatacaaacgactggccacactggaagtaaaggtgggagatcttatcatcggaaattttaacccggtccgcattcaaaccatgactaccaccgataccatggataccgctgctaccgtggcgcaaaccatccgttgtatcgaagccggtgcagaactggtacgcatcaccgcccccagtaaaaaggaggccgataacctgctggtcatcaaaaacgaactacgcaaacaagggtatacgactcccctggtagccgatatccattttacgcccaatgcagccgaaatagccgcccggattgtagaaaaagtgcgggtgaacccgggaaattatgtagataaaaagaaatttgaacaaatcgattataccgacagcgaatacctcgaggaaatagaccgcatccgcgaacgcttctctcccctggtaaaaatctgtaaagaatatggtaccgctatgcggataggcaccaaccacggctccctgagcgatcggatcatgagccgctacggcgataccccgatgggtatggtggaaagtgccatggaatttttacgtattgcggaagacctgcaataccgcaatatagtgttgagcatgaaggcaagtaacccgcaggtaatggtacaggcctaccgcctgctggtacaaacgatggaacaggaactgggccactgctatccgctgcacctcggtgtaacagaagccggcgacggggaagatggccgcattaaatctgctatcggcataggcacactcctcgaagatggcgtaggtgataccatccgtgtttccctcacagaagatcctgaatttgaactcccggtttgtaaggatattgtgaaaagatatactaaccgcaacgactatacggctattccgcccgtaacagatatcccctattcccctttcgaatacaaacgccgcgaaagcacgcctgtagagaataccggcgaaaagcaggtaccggtggtagtggcagatttcagcgataacaacggcttacagcccgccgatctgaatgccatcgggtatacgtacgatgagcccagcgataaatggaatatcggggatgccgccgcagattacatttacaccggcaaacagttacctgccttcggcctgcccggcaccctgcgggtagtgatagatgcggagtattggctgagcatcgccaataaacaggaactggtgccttactttgatgcccgtcattatgtaaccgcctgcgaacaacaggaaatcggccgtatcaactttgtacaattcgactgcaatcacctggataccgaacatcatgaacaactgctgctgcaactgggtaaccccgccgtagctgccggcaccgtacttgtggccaccgcttccggcagcaatgcgatggcggctatcaggcgcctgtttatcttattgctcaataaaaatatcagggtacctgtcatcatccatagtatcagtaatcagccttcggcagatgaacacctgatccaccatgctaccgaagccggcgcactgctgctcgatggcttcggcgatggattatggctgagtaatcaaccctcacaacccggccagcatgccacgttgaacaatatttcattcggcatcctgcaggctacgcgtacccgcatttccaaaacggaatatatctcctgcccgtcgtgcggccgcacgctattcgaccttcaggaaactaccgcccgcatccgcgccgtgacccatcacctgaaaggcgtaaaaatcgccatcatgggctgcatcgtaaacggtccgggtgaaatggccgacgccgactttggttatgttggcagcggcgtaggcaaaattactctttaccgcggtaaggaaattgtgaaacgtggcctcaacagcgatgtagccgtcaacgaactgataaacctgatccgggaaaacggcatgtgggtggaaaaaaactgattattaaatctggcttaaaaacagcagcagcggatacagcaatgctgggaaaagcttaattttcataaaacatatttaatatgaaaaagttcctcaccggattattggccatgttcatgggtttaaccgtagcaatggctcaaacacccgccaccgccaaaaaagaagcaaaaccaaaaacagaaaagaaagcagagaaagcaacacctgctactcccgctccagccgctactactaaaacaaagaaagacggcacaccggataaacgatataaagaaaacaaaacagccgcagctcctgcaggaccaacaaagaaagacggaacgcctgatatgcgctacaaatcaaacaataaaagcgcaggtaagaaaaaagcataaccattacctgttactgaatcataaatctttaagccctgcacagtcaatactgtgcagggctttctttttgagttatatttttcaacatgcagccttttaccttttatgcggatcgccaataaggattggagccctgccggccagggtatttataaacacttcggctttacgccgcctgagttgtaaggtatttttgtatttttagtgcatgttcgatttcagactcagggtatttcacaccgtcgccaagcgtctcagcttcaccaaagctgcagaggaattatatatttcacaaccggctgttaccaaacatattcatgaactggagcagcaactgggcatggcgttgttcgaaaggatcgggaataaaataaaacttacccgcaccggcgtgctggtaatgcatcacgcagaaattatttttaccgattaccgcaacctggagtatgatgtaaaccagctgaaacacatgcagggtggcctgctgcccataggcgccagcactaccattgcgcaatacctgatcccgccgttgttggccaaattcaaccagcggtacccggatgttaaaacatcgctcaccagcggaaatacagaacagattgaacaggcgttatttgaaaaaagtattcagctgggtatcattgaaggcagctctaaaaatcctttactgaaatatgtggagtttgcgaaagatgaaattatattggtcggcaatatgaagcatcagtatggcaatggcgaaccgcttggcccggccgatcttaaaactattcccctgctgatgagggaacatggttccggcacgctggaagtgatcaccgaggaactgaaacgcctgaaattaaagatcaccgatctgaacgtagccatgtatatgggtagtactgaaagcattaaatcctacctgcatcattcgccctgtgcagcctttatttcctcacaggccgtgcagcgcgaactggaactgggcgaattcaggatattaccggtaaagaatttcaaactggtgagaaaacttcacttcacctatctccagggcttacaggataagctctgccagctcttcatccgttttgcaaaacagaacatggtggagtaacggtcatgtacctacgttatttattcaatagttgccagtgcagcatttccccgggcgatttcacttcttccatccccaggtgttgcagcaccttcatggatgccgtgttggtaacgtcgcattcagcaatgagctttttcacatgaggttgccggaaagcccattccaccaatgcggtggcggcttcgcgcatataaccttttttgcgccaggaaggcagcagcgtatagccgatttccaccacgccgtttttatcgggccggcctttaaacccgatgtccccgatcacggttccttcttctttatttacgatgatccagagcatccagggaaacgacctggggtcgtgctggagcaattcaataaaatgaggtaattgttctttcaggtcgggttgtggccagttttccgggatatttgcctgcaacgtttcccgggcatgcggatgccccaggaatatctccgtaagcagtggtaaacggcagggatgtatgaacagtcggttggtattgaggggtaacatatatcaggatttaaggcataattgttcactaatgattgccggccttcaccatggcggtatccagtatttcgcctggtttcagttcatggatctgtaagcggtccaggtcttttgtcagcgcccgcagttgctcaggcgtaccggtgagggtgggcattgttccgtaatgacaggggatcaaatgctttattttcagcaaacgcgctgcgtatgcagcttccagtgggcccatcgtaaaacggtcgccgataggcaaaatggcgatatccggttgatatatctccccaatcaattccatatcgccaaacacagacgtgtctccggaataatatacagagatatcgtcgctcatccagacaataaatccattgctggcatgtgggtagccgatcttaccatcgggcaggttgatgtgcgcaaaatgaaaggcattggtcatggtcacttttacattcattacagataaggtacccccggcattcagtggttcaaacgcatgatcgggcacgccctgttcctgcaaataaaacctcactataggattggcaatcactttcggcgacctggtgcggataatgtccaccattttgctgtcgaggtgatcacggtgcccatgtgtgataaggatgagatctatcttatccggaattgttaaaccgggaggcagggcaggattatttgtataccagggatctatcaatatcacatgaccttcgggggtggtaatcctgaagcttgcatgcgccaggaactgaatctgtgactgttgcgtgctcatagtactgctggttaatgatctaaatatacatcttttgaaaaaaagacagcggagatcatagaacatgatctccgctgcattaatgagctgacacgatgcgtgacagtggttatttacgttgcagggtatatataattgctgcacttttattttcgaagctgatatttgctctccaggtcatcacgctacccgcgccggtaatttccatgcggtaaccttcggttacattctttgctttatcgccgctgtacagtttcttgaagccgaacatgcttacgccgccacttttggtcagcgaccaggcaattttctgggtaactgcgctgcaaccattatctgttgaggtgagcgtgtaggaacccatggcatagttgtccggcaggatccactggctaccgataaagcacttcgcgttggcttcatcaaatacagttactttggcgttttcggggattccttcgtatttaatatcagttaaaacccagttaccttttacggcgcctttattaatgtcttgggtaacaccttgtttgggagagcaggaagatgcaaaaacggcaactatcgccattaataacgctgcaaatgaaaattttctcatgggaagttagtttgtgtgtttaaatgccaatgtattcaacacgcagctatcggataaggttttataacagccggaatacaggggcaatttcagcatttgcaataaacgtaccaaatgaaagtatccccgcttaacgggttacaggagcgggataggctgcaggagggactttaagcttaaacaggatttcttccagcctctgggcgcggtggtagaagtgccaggtactggctgccagcgccatggcggttaccgcgagggcaataaaggcgcaccgccaccatacgctcaccgtgatccggcggttccagaaagagtcgaggggaatgtaggtatgatggaaattcgtatgctcataagggttataactgctccgggaacggtctgtccagtccttatccggcttaatccgctgcaaaacggcagcttttatttttaccgggggtaaggcgccttcttccatcagtttatcttctatacgcagttctgcggcggtgaattccaggtccagcaacgggtatatacggcgcaggtgcagcaactcatcctcctgttcaggagaagcaagtcccagcagataacgctcaataatgccgctttctatatagttactgatgttcaaacccttcgctttaaccaacggatacgaaatataaataataaatactatatctatagatacgttaaacccacttcaggtggattctcaaaattgtaaaatctttaaaataacgataatccggatagaaaattataacaagtggctttgcgtttgctcctgccggatcatctggtgcaggttgtcgctgcgctgctgctcctgcgacatacgatacttgaggtaataaaaaatggccaggaaaagaaataccttggacatgataaagaagataataaagaagatcttccaccagcggtgaacagtgatatgactgccgtcttttggctgaatgttaataaaagtatagttggaagaaggatctgaataggcatgtccctcctcccacctgatcttctgtagcacccgttcgcgtatttccacgggcggcatggcgggctcatcaaacgcggctctttccaggcggcgttcaacgtattcgacttctgtatccagttccggatacagccttctcatgtgctgcagctcttctacttcctcttcagaagccaggcctaacacgaaggactcgataataccgctttctatgtaaaattttagttccaagtcttttttaagaattgtctgaaagactttatcgcctctttcaggatttcatttatctgcccctccggcaaagccagcaaacgagctatcgttgtgattgataatcctttaaaataactaagccggaacacctgttgttgatcggccggcagcatcaggtagaattgctgcagtaagccatcttcctgcttcatcagctccgtgccggctaacgcggtttccggcagggcctccttgatggcgaattctctcgttttgcgcaataaccaggcaaataaagtatggtggcccgaggtccggaatgttccaatgtgctggaacgaccagagaaatacctttacaattacttcatttgctcgctcttttactggtaccagctgtaatacaatgttataaagggccccggcataacggtcatatagctgctctttcgccgcaggatcccctatcattaaccgctcaatgagcatatgctcacttatatttgccaaatctcgccgcaaagaaattgtgtaccaggtttagaatgctaatatatagaaataaaataggtgtacgtcataacacctatatgaatttatcaacatggttagctaaaatggataactactgccccaaatccagctggtatggccccggcagaggcgcctcagatacggcaattccccttgggcttgacacttatcagcgcaacaaggtttaaattacaacatgacaacgctcatttttattctttttcccgcacgataattttgaagaaaataatcaccgtatgtcctacacttcgatcacagcagccgcacaactgatccagtccggccaaaccgtatttattcacaccgcggcagctacgcctcgggagctggtgaacgccatgaccgtccgcagccatgaactgaaaaaggtacggctggttagcatacataccgaatgggaggcgccgctgatgttactaaccgcgccaccatcagctatacacagaaaacccggacggcatggatgatcggtaccgggaaccattctgtaggcaatataactctcctcattcctatctcccctacaactattcccggccattaatgttattatcaaaactatatcccatgcatgttaaattaatggtacttgctgtttgtacaatggcggctgtttcctgcgccagcagcggtacaaaaacggggagcgacagcactgccgccggcggtgattcctccataaatgtacaggcaaaccccaacagccagctcgaagtaaaacctatctccggctatttcctgaaaaacaccattatagtaaacgacagccttaccttctggctcattgataaccaggcctctttcgacagcctgtttggcgcggctaaaaccatgaacaacaccatcgatcaacccgactttggcacccatatcgtagtggcagccactatgccgcctacattctatggcacacaaattcaactggaatctgctacctcagacaacgtaaacaataatgccgcactgcatttcgtggctacttccaatcccagcaggggaagtgccagtacagttcccctgtggctgggcgccgttcccaaaaccggcaaaagcaccttccagttttacagtggtgagcatttaacaaaaacgattactactcagcagtaggcagaccaaatattttttcaacggcctgaaaccggtatcggaacaagtcctccagctgttttcttacaaacagcctgtgggccagctttcccagccagccaaaaggcagccggtaatgaaccaggtccgtcattttcacaccaccgggcactttctggaaatgatgttcatggtgccagatgctgtagggacccacccgttgctcatctacaaaataatccaggtaggccacatgggtgatttcggtcatccactccagcgggatacccgctaccggcgatacaaaataggtgatgatctgtcccgggtatacctgcccggtataaggcggagaagttactgtgaaccgcatagcgggaggcgtaatatgcgccaggttattggggttggaaaaatagtcccaaacctcctccggctgggccgggatcacctgggtatgctgcatcaaataaatacttgccatatataagattaaggaaaaaatatggttctggtcataagcagctgccaaattcgtgattctttgaaatgagttcgtaagtttgtgcctgattaatccgatcaggtacatgaatcaatatatcaggggctggattttctggctgatgttcatactcgtttccatttcatttacgcgatgtgccaacattgtgcctcccagcggcggaccgagggacagcttgcctcctgtattgctgcaggcaactcccggcgactctacgcttcactttaaaagcaaaaaagtgacgtttatctttgatgaatatgtggaactggataatgtgaacgataagctgattgtgtcgccaacactgaaacgcacgccgattgtaacagccaaactgcacacagtaaccctggaaatcaaggatacgctgaagcccaatactacctacacgttcaattttgcagatgccatccgggatatcaacgaacgtaatattgccgctgatttccagtatgtggtgtctacaggcgattatctcgacagcctccaggtgtccggtcacctgatagatgcggaaaacggccgggtagacagtaacgtggctgttatgctgtaccgcgatctgaccgactccgttgtgacgaaggaaaagccggtatattacgccaaaaccaaaggggatggctccttccgttttaaaaacattgcacccggttcttataaaatttttgcactgaaagaagaagaccgcgacctgcagtataatcagcctacagaaatgattgccttcgtggaagcgccggttgtattaacagaaagcaacctggccgatgtgaacctgctgttgtttatggaagctgatagtaccatcaagccaccaccggagcccgtggattcgtcgatgcttgaacaggaagaagaagaaaagaaaaagaagaagctgcctaaactaacggccacccctacgctcgacggagggatgcaggaattgccggcgccgttgaggatcacgttttcgctgccattgaggaacctggacagtgcaaggaccattcttgcggaagacagcgcctataccccggttacctttaccagcacaatggattccacgcgcaccaagttaaccatcggttatacctggaaagaaggtacgccgtaccggttcattattcctaaagatgcgcctacagatactgcggggcagcaactggccaggccggatacgcttaatttcaggaccaaaaaggtggccgattatgccattttcacggttacagaactcaatatcagcgatagtaccaaaaaagccatcaacgataccgctatgaattatgtggtacaactggtgcaggataaaaccattaaatattccggcaccattgtaaacggtaaatggagccagcggtttattacacccggtgaatacgaaatccgcctgttgctcgataccaatggcaatggcaaatgggaccggggtaattattataccaagcctaagaagcagccggaacgggtcatcaatgttgaaaaagtaaatctgaaggcgtactggacggtacccaagaagatcagcatctaaataatcgcagcggaaggaacagtgctgctccctccgctccaatattcctaactttgcactatgatattttcctctgcgctgatagaaaacgcggtaaatgaatttgccaaactgccgggcatcggtaaaaaaaccgccctgcggctggtgctgcacctgctgaagcaggagacggcccaggtggaacagtttggcgatgtgatagcacggatgcggcaacagatacagttttgcaaggtttgccataacgtatctgatgcggaagtatgcagcatctgcagcagtcattccaggcaaaagcaggtagtatgcgtagtggagagcatccgtgatgtgatggcaattgaaaacacacagcagttcaatggtttatatcatgtactgggtggtatcatttctcctattgacggtattggcccggaccagttgaatattcattcactggtggaaagagttcagtaccagggtgtagaagaagtgatcatggcggtgagccctactattgaaggggatactaccatttactatctctctaaaaaattaaaagaattcccggtaaaaattaccactattgcccgtggtattgcatttgggggtgagctggagtatgcagatgaaatgacgctggccaggtctatcagtaaccggttaccgctggaaaactatgtacagaacaaataaacaacttctcggggttatataaaaaaatacgggtgctcaatagcacccgtcttcgtttaacctgtaattccacgttatgaaaagttgtcagacagcatcctttgaaggatggtctgtaaatattgtatgattggtttctgattcctgttgttgttgcagctctttccaccgctgcatttcatatttatttaagaagcataccttaaacacttcagactggtttccgttgccggactgtggtaccggttgcaatcccaggctcgccaggtgctgatgaagggtatgaatatgttctgatatagtcatgactgacgttagttttgttgtaataaatatttgagaagaactaatgatgaatctgttaattgcggcaacggcaactacaaagagtgcgggcggagggctggtgggtggccataaccgggtaaatcactatatttctatcactttgttgcattgtatctttctattaccctacaaatatagtagactttgtagactacttccaaattaaatttataagtataaacaaaatctatacatatccataaagatatataggcttaaaaaggatggatcaaagccggtcaggtccgggaatccatgcaaatcacaaaacaataaaatagctgggaaaaggttatatttgtgaactcgttcagggtggatttgtttattgttcgaccctgttcatttcttaactgtaactaataaacgccttgataaatatgaaatctttacaagactgcgccaatgagcgcatacttatcatcgatggtgcaatgggcaccatgatccagcgatatcaactccaggaatccgactacaggggcacccgctttgctgactatcccagtgatcttaaaggcaataacgacctccttaatcttacacagcctcaaattattgaagccattcacaaggagtacctggaagcaggcgctgatattattgaaaccaatactttcagcagcacctctattgccatggccgactatgacatgcaatcgctggcctatgagctgaatgtagccgccgcacagatagccaaaagagctactgctgagtataccgctaaaaaccctgataagccccgctttgtggctggcgccatcggccctatgaacaaaacgctgtcgctgtcgccggatgtaaataatcccgggttccgctccgtatacttcgatgaagtggccgccgcttacgaagaacaggtaagaggcctgtctgaaggcggtgtggatatcctcctgatagaaaccatttttgatacgctgaactgcaaagcagcgatttatgccatcaagaaatactaccgcgaaacagggaaacctgagatcccggtaatgatttcgggtaccatcacagatgcctccggcagaaccctcagcgggcaaaccctggaagcattctatatttccgtgatgcacgccaacccgttctccatcggtttaaactgtgccttaggcggtcagcagatgcgcccttatgtagaggagctttccaacatagccagctgctatgtgagctgctaccccaacgccggcctgccgaatgcattcggggaatatgatgaggaaccggaagatactgcctgcatcattgaagactttgccgcctccggctttgttaacatagtaggtggctgctgcggtactacacccgatcatatacgccacattgcagaacatgtgaaacatatcaaaccacgcctcaaacccgtattggccgaaacactcgcctgatcaaccgtggcaggttttctatttaaacattacttacagcagaaatgagcgaaacaactataaataatacagatatcatcaacgaacctattgtcagcgaagaacgcaggatcatcaaaccctttatgcgcctgagcggactggaacctttggtggtaagacctgaaaccaacttcattaacgtaggggaacgtaccaacgtaaccggctccaagaaatttgcccgcctcgtaagggaaggactgttcgaagaagccctgtctgttgcccgccaacaggtggaaagcggtgcgcagatcctcgacgtaaacatggacgacgccctgctcgacggggaaacggccatgtctaccttccttaatctcctggcaggcgaaccggatatttcccgtatcccggtaatgatcgactccagtaagttttccgtgattgaagccgggctaaaatgcgtacagggtaaatgtattgtgaactccatcagcttaaaggaaggagaagccaaattcattgaacaggcgcatatctgcaaaagctatggcgccgccgtggttgtaatggccttcgatgaacacggccaggccgacaccgaagataaaagggtcagcttcagtcaccgtgcctataaaatactcacggaagtagtaggatacgatccccaggatatcatcttcgatcccaacatcttcgccatcgccaccggtatcgaagaacataataactacgcggtagaattcattaacgctacccgccgcatcaaacagctgatgcccctggcaaaaataagcggcggtgtaagtaacgtatccttctctttccgcggtaacgaaaccgtgagagaggccatgcattccgtattcctgttccatgccatcaaagcaggaatggatatgggtattgtgaatgccgggatgctgcagatctatgacgatatagaaccaacgctccgtgaactttgtgaggatgccatactaaacagaagggacgatgctaccgaacggctcatacaatttgcagaaaccgttaaggccaaaggaaaagtagtagagaaagatgaaacctggcgcctgggctctgtggaagaccgcttaagccacgccctggtaaatggtatcaccgactatatagatggagatacagaagaagcccgccagaaatacccgcgcccgctggatgtaattgaaggtccgctgatggcaggtatgaatatcgtaggcgacttgtttggcagtggtaaaatgtttctcccgcaggtagtaaaaagcgcccgcgtgatgaaaaaatccgtagccatcctcacgccatatattgaagaagagaaattacgcatacaggccgaacacggcggagaaataaaagcagccggaaaaatcctgctggccaccgtaaaaggcgacgtacacgatatcggtaaaaacattgtaggcgtggtactggcctgcaacggctatgaaatcattgacctcggtgtaatggtaccggctgaaaaaatcctccagaccgcccgccaggaaaaagtggatatcattggcctgagtggcctcatcacgcccagcctcgatgaaatggtacacgtggcccgcgaactgaaacggcaggatttcaatatcccgctgatcatcgggggcgccaccaccagccgcacacatacggccgttaaaatagcccaggaatatgcgcatggggtagtacacgtactggacgcatcccgcagcgtaaccgttaccggcagcctgctcaataaagcactgaaacccggcttcctcgcgggtatacaaacagaatatcaaaagctcaacgaggctttcaagaataaaaaacaaactaaacaattcctcccgatcgctgctgcgcaagccaataaaaccgtcattaactgggatacctttaccccggtaaaacctaaaatgaccggcgtaatgaagtttgagaattacgatctcggggaaattgcaaagtatatcgactggcagcctttcttcattgcctgggaactgcatggtaaattcccgcagatccttactgatgatgtagtaggcgtggaagccacccgcctgtttaatgatgcaaaggaattattaaacaaggtgatagaagaaaaatggctgggcgccaacgctgttattggcctcttccctgccagcagggtggctgctgactctgtgttggtaacaccagaacaaccggagatcaaaccggcacaactggaattcctccgtcagcaggtaaagaaagcaccgggtcagccgaacctttcccttgcagatttcattgctcccgcggaatccggcaaaaccgactatatcggcggctttgcggtaactaccggtgttggcattgaaaagtggctggataaattcaaagcggaacacgacgactataacagcatcatgctgaaagcactggccgacaggctcgcagaagccttcgcagaactgatgcacgaacgtgtacgtaaagagttctggggatatgctaccgaagaacacctgagcaacgaagacctcatcaaggaagcctatgcaggtatccgtccggcgccgggatatcccgcctgccccgaccataccgaaaaatggaagttgtttgatctgctgaatgctaccgagaacactggtattacccttaccgaatcactggcgatgtaccccgcctccagtgtaagcggttggtattttgccaacccggaaggcaaatatttcggcctcggaaaaattgaaaaagaccaggtgatagactacgctgcccgcaaaaactggacagtggaagaagctgaacaatggctccgtccaaacctcgaatacgatatctaaaagcattacagccaacatgagaatcatatcttacaatgtgaatggcctgaggtcagccatgactaaaggcttcacagaatggttacaaacagatcccgctgatattatctgcctgcaggagataaaggcccaccaggaaaatatcgactttcagcaattcgacaaccttggctatgcgcattactggtatcccgcgcaaaagaaaggatacagcggagtagcagtgctcacccgtattaaacccgactttgtgcagtatggcagtggccacggacaaagcgatctggaaggccgctttataaggcttgatttcggcaatattaccctgatcaatacttacttcccatccggtaccagcggcgagctgcgtcagacctataagtaccaatggctggaagagttttttcaataccttgaagagttaaagaaaacccgcccgaacctggttgtatgcggcgattacaatatctgccacaagccaatagatatccatgatcccgtgagtaacaagaactccaccggctttttgccggaagaacgcgcgtggatggaccgcttctttgaaagcggctttgtagacagcttccgtcattttaatacggatccccatcagtacagctggtggagcttccgggctaatgcaaggaacaataacaaaggctggcgtattgattatatcaacgtttccgctccactgaaagaacagctcaaacatgccactatttaccaacaggtaaagcactcggatcattgtccggtatttgtggagctggccgtataaataaagaggcgtatgattatatataatgtaaccaccaaagtagccacagatacatatttacagtggatgcaatggttgcgggaagaacatattccggcaatgctggccaccggattattccgtgattaccgcatcagccgcctgcttgaacaggatgatgaagagggtcctacctatgttgtgcaatattttgcagacagcctggacgactatcaatcctttgcagaccagcaccaacaggccctgcggcaaagaggatatgaccttttcggcgatcgttttattgcctttaacaccgtaatggaggtgctgtaagtaagggatctttactaaacttatccacaggaaatccactattttcggggtgtcaggagtctggtacaatagttggttcgatcctgcgttaatagtaaaaaagcatgcaaacatgccacggtacagggttctatgcgattctgctaaaggggagtcctttagcagataaaagaccaatcagctgtaaccgttaccagtagcgtttttcagccgataaaattttctataaaaaagctgtaaaaaatttggtaatctgataaaacgcgctatatttgctcacatcaaacattttttcactagttaaatcttactaactatgaacaaagccgaattaatcgacaagcttgctaaagatgcagctattaccaaaacccaggctaacgaagcgctggactctttcaccaaagctgttgctgataccctgaaaaaaggtggtaaagtaactttggttggtttcggtactttctccgtttctaaacgtgcagcacgtaacggtagaaacccacaaaccggtcagatcatcaagatcaaggctaagaaagttgctaagttcaaggctggtaaagctttatccgacaagctctaatcagttaacacaacttattcaagcaaggaacagttatgtttcttgctttttttttatatcaaacggccagtactacgctatttcatcgaattgcagtattttgcagcctgataacatcatatttaacaacaacaaacttcaaattattcgttatgggtagaggagatattaaaaccaaaaaaggtaagatcttcagtaaatctttcggtaaggttagatctgcaaagaccaggaaaaatactgccgcaaaagctgctgcaccaaaagcttaattttacgctttagtaaaatgccgctaagattattcacataatcttagcggcatttttattttaacacctggaatatcatggagccagccgctcaattttccagccgccttccggcagtaatgtatacaggatcctgtcgtgcaaccggctgcttctcccctgccagaattccatcacctgtggcttcaccacataacctccccagtaatcaggtctctggggggcctcctgccggtattttgccgctacctggtctacctgttcctccaggaaagtacggtccggaatgaccttgctttgcggcgaggcgatggcgccaatccggctgccttccggccggctgttgtaatactcattactcaccgataccggcgccttactaacggtaccctctatacgaacctgccgttccagctcccgccagaaaaacaataaactaacatgcggattctctgccagttcctgtcccttacggctttcgtaattggtaaaaaacaaaaagccatcctcatcaaagcttttcaataatacaatccttgcagatgggcggccatccgccgtactggtggccagtgtcatggcattggcttcatcaatttcactggtgatcgcatcctgccaccatttcccgaactgggacaaagggtacggcgccacctcgctttcatccagggaagccagtttataatcttttcgtaaatcagctattttctggttcaacatggtctgttatttttatgattcaaacgggtactcaaaggtatggaaggataatagtaattttgaggtacctgatataaatcatactatgaaaagagtttctctactggtactgctgatagctgttgtactcctctcctgtaacacacggaataacaacaacagcaaggcaccggctaatacagccaacctggttgtaccactggcttctactcccctgttctatacccagctcaaaggaaaactgggcgataaagaaattaccatgcaattgctgaaaaccgcgccccacctgttccgcgggtactattgcgatgatagcaccggtcagcccattcctttatggggcaccctggattcaaccctggcgaacatctatgaagaaaccaataacagttcggaagaccgcctcttcagcggctatctttctgacgacggaaaattcaaaggtgtatggcatggcaacggcacttcctatcattttgaactgcacaccgatctgaaaaacgccgtacccctgaaagtattctaccagattgattctgcaaagctggcgccttccatggcccaatcaccggcaggcaccgtgtccaacagtatcatatggcccgactccctggtggatagcaccaccgcccggtttattattggtcaggtaacagggaacagccgggctgccgacccgcagaaattcctgagaaaaggaatcgactcctttatcctgatctaccgttattcggccaaagatgccgacagcacaacgtttaatgataacaccactgccgcgtcgtggaactggaccacagataacgacatgaaagtagtgtataacacctggcctctgctggtgatagaaaagtatgcttacaactttaccggcggggcccatggcaactggggcgccacctattacacactggacctgtcgaaacgtaaagtgcttactcccgacgatatttttaaatcaggctataaagaaacgctgagcggcttgctggataaagctttcaggaaacggttcaatatgggtgaagaagatgccctggatcagcacctgctggtaaaaaacatccctccgaataataatatgattgttaccggcaagggagtagcgtttagttatgtgccatacgagatcgggccatatgcactgggccaggtaactttatacatcccgcttgcggagatgaagagtatattaaaatagcagccgtttgacgacataaaaaagcagcgaagaacaaatgctcttcgctgctttttttatgcgtttacttatccctttactaaggtacccacatttttacccatgatcacgttcaggaggttaccctgacggttcatatcaaacacgataataggcagcttattttcctggcaaagggtaaaggctgtcatatccatcacgttgagggatttctggtatacttctgagaaagtaatggtttcgtagcgggtggctgttttatctttttcaggatccgcggtatagattccatctacacgggttcctttgaggattacatcggcctgaatttctatagcgcgtaaggaagcggcggtatcagtggtaaagtacgggttaccggtacctcctccgaaaattactacacggcctttttccacgtggcggatagcgcggcggcggatatagggttctgcgatctgttccattttgatggcagattggagacgggtataaagtcccactctttccaggccgctttggagcgccataccattaataacggtagcgagcattcccatgtaatctccctgggctctttcaataccggtatcggcttcgttcattccgcggtagatattacctccgcctataacgatggctacctgaactcccagatcggtaactgccttaatatcgtaggcatactgagatatcaccttcggatcaataccataatttgcatcccccatgagggcctcaccgctcaatttgagcaaaatacgcttatactttggcaacatgacgctataaaatattgtaagattgtgattttcctaatactgattacggtattctaatatacaacttaaatgcagaaaggaggaaaggaagaaaaaaatgccttttctgatacctgtttactgtccttttatgtgtatgattagttatgcgcaaaaaaaaggagagaaacgaattctctccttttttttgatatgtttttcttaacctaaagcaattcgcttaaagccagttactttcaggtcagcatctactgatttcaggtaatccgctactgacttgttattgtccttaacgaaagcctgttgcagcagggtgctttctttgaagaatttatttactttaccggcagcgatcttttccgccatttcagcaggtttgccttctgctttcacctgttcaacagcgatttctttttcgcgggcgatcagttcagcaggaacgctgtcagcatctactgcgataggactcattgctgcgatctgcatagcgatatctttacctacttcttcagaaacaggcttagagaaagcaaccagtacacccatacggtagttaccgtgaatgtaagaggttacgccaccagcttcaacgaattcaaatttattgagggtgattttttcaccgatttttgcaacctggtcgtttactttatcagcaacgctcgcgccatccagttgagcggcattcaggtcttcaacggttttgataccgttagacagtgccagatcaacgattgactgtgcaaattttacgaagtcttcgtttttggcaacgaagtcagtttcacaacccagacccacgataacaccggatttaccatctgctgatgttttagcgatgataacgccttctttggtttcacgatcggaacgtaaagcggccactttctgacctttcttacgcagatagtctactgctttttcaaaatcgccatcactttctaccagtgcctttctgcaatccatcataccagcaccagtttgctgacgcagtttatttacatcagctgctgtaattgttgccatgagctataattagtttaattgttgtaaaaattattgcaagtacttaatctgctttcagctattagcctttagctgttagagaccataatggttgaactaactgctaaaggctaatagctaaaagcttaaaatattatcttccgccgcctggttttctaggaccgctgctgccggcaccagatggacgacgttgtccgcctgctgcaccgccaccacggttaggaccgccaccgccacggttagcgccgccaccctggccaccaggaccacggccgccgccaccacggttagcgccaccgggaccgcctggaccacgaccaccacctggtgctcctggtttgcgacctctttcacggtcttcaccaccttcaacttcaaatttgcgtgctttatcgtctgcttcttcttcttcctctacttcttcagatttctctgtagctctttcagaaagaccttcagcgatagctgcacagatgtagctggtgatgatagcgatagatttagtagcatcgtcattcgcagggatagcgaaatctactttagtaggatcggagttggtatccaccataccgaaagtagaaatacccagacgcttagcttctgccagtgcaatgtgttcgtggctgatatcaaccataaacagcgctgccggtacacgtgccagttgggcaataccacccagcactttctccattttctctttatcgcggcttaaagtaagacgttctttcttggtaatgttatcgaatgtaccgtcctgcagcattttttcaatgctctgcattttctttacactcttacggatcgtagagaagttagtgagcataccacctaaccatctttcagttacgaaaggcatgttgatgttacgcgcagcatctgccacgatttctttcgcctgctttttagtagcaacgaacatgatcttcttaccgctcttagcgatagatttcagggcagctgctgcttcctgtaatccttctacggttttgttcagatcaatgatatgaatacctttcttttctgcgaaaatataaggcagcatcttgggattccactttttcttcaggtgaccgaagtgaacacctgcctccagtaactgctgctgcaatgaggtattattttccatgtttatattgctcaattaaaaggatcaaataatgtttagcttttagcatccggcgaattagcccggagctaacggccaatagctcaaaaatattagcgtttagagaactggaagcttcttcttgctttcgctttacctggtttcttacgttcaactccacgtggatcgcgtttcagcaaacctgcagctttcaatgcaggacggaactcaatgttcacttcgcataaagcacgggcaatacccagcttaatagcttctgcctgacctttgataccaccaccctgtgcattcactttcacatcaaatttatcgagcgcctcgatagttttgaaaggcagttccacctggttctgcaggtagatcaaagaaaagtagtttttataatctttgtcgttaactgtaatgttaccggtacccttgttgatataaacacgggcaacagcttccttacgacgacctattgtatttttttgcttttccatgtatcagagaaaaattagaaagttaatggttgtggtttctgcgcagcatgaggatgttcagcaccagcatatacaaataattttttgtacatcgcacggcccagacggtttttaggcaacatacctttaacagccttttcgatcaacacttcaggacggcgacggatcaggtcctttgctaattcgattctctgaccacctgggaaaccagtgtagtgcatgtattctttttcctgcattttattgccggtcagggcaatcttctctgcattgattacgatgatataatcaccacaatcagtatgaggcgtatagtatggcttgtttttacctctcaggatagcagccatcttagcagcaactcttcccagtgtcaggtttgttgcatctactatatgccagtcacgctttacgtaagcgtcgttagccgatttagttctgaaacttaatgtattcattgttgtatacgataaaaattacgtcttgtaaacaattccccgattatggggagtgcaaaggtacattgcccattcttaataaccatacattttagggacttttttacggagcacctttgcaattgattgattttcaataaaaaatttgtataaaagttattaacagcaagtaccggcacggttaataactgctttttttctcatataaatgaataaaaaaagggcgcctgagcgcccttactgttttatattatacaatactttttaatacccggggttctgctgtccggtcaatttaccctgactggcatctatttcccgctggggaacaggtaacaccaacttattatcatcgtagctcttgttgccgatattcctctttaatcttttaaatgtccataacttatccccctcaaacaacaactcgcgtacacgctcatccgccacctggtctgccgtaacggccgccagctgcgaagcattggacctcgctcttatttcattgacatcctccaaaggaggcgcaccaacagctgttcccgctcgaagattagcctccgcacgggtgagcaggatctccgcatagcgtaccaccgggatcactttgtactgacgctgccatttggtagtataggtaccgctgcctacattgataccgcggtcaagatacgtaaaggttctgcgtgcatcaccactctcaaaaccaggcacaacggtcaggtcaacggtaatatcacccctgcctgaaaatcccctgcccgcatagaaagtttgcagaccgttattggaagtacccgcattgctctgagcagtttgctgaatagcaaaaatatcttcagaagtattaataacactgttgaacgccttatcataagcattattcagtgtataggcaccgctctgaattatagaatcagccatcgctactgcctcggtatattttgcttcagccaggtataccctcgacaggaaagcatatgcagcatatttgtttgcacggccttcgctgccattgtcttccggcaaattagtggcggcatcctgcaaatccgccaccacctgtttgtatacagcatctacagtagccctgccctgatagcctttgggaagatcagcaatatccgtgatggcatctgttaccagcggcaccgccaggttagtagtaatattaccggcagaatatggcttgccatataaattaaccaggtagaagtaaatcatccccctgataaatttggcctcggccagtattgccggacgctcgtcttccggcaccaggttgatcttgtttatggcaagattaatattattaatagtaaagtaactacgtctccagatctcttctgcgatatcactggtagcgtcctgggttttggaatcatattgcccgtagttaaaaaaggttccgcgaaaactcaactctccattaccagccagcagatcaggaatcaatatcaatctttcccccagggaacttgaattttgcaggttggtatatgcgcccattaaaacgccccgcacatcatctgccgttttaatctggtcaggaacaatgtccttaccaggcgtcacgtccagttttttattacatgctgagaacgtagccactgctaccaccaacattattgcgctgatatatttgttatagattttcatcttttctcttttaaagcttaaaatttaacattcagtcccactgtgatctgcctggcctgtgccggtgtgtaataatcaataccaccaccaatattatcaggttcaccggctgtgctatatgaagcaccggagttcacttccggatcgccatcgaaattggtgattgtccagagattgtatccggctacatatacacgcaggctggatattttaagcgtgttcaccacactctttggcagtgtatagcccagtgttaatgctttcagacgcacataagaaccatcagaaatccagcggctggataagcccgcggcagaacttccatcagcaaacgcttgtgttaaccgtggcacatcggtgatgtcgcctggcttttgccatcttttcagaatagtgctgcgttggttgtcgtaaccggcaaaactattgtcctggtattgacctgcacggttaaagatgtcattaccctgcacaaaagagaagaacgcactgaggtcaaagccgtaaccggtaaaggtattggtaagaccacctgtccaatcaggattggattttccaactactacacgtggcgcattcgaataatcggtggtgcccttaccggtagaatcctggtataaagcgtctccggtagccggatccacacccacaaatttgggcataaagaatacaccgataggttggccttccaccgcgcgttgttctttagccggactttctatgatctgtccgttcaggtttttaaccctgttcttattataggcaaggttcagggtggtggtccatttaaaattacgggtgtctatattcacactgttcaggagaatttcaactcctttattttccatctttccaacgttcaggtactggaactcataacccgtggaatatggcagattggctctcaacagcaggtcggaagtttgcttgttataataatccacttcaccacttaacctgttgtcaaataatccgaactcaaggccaacatcaaactgcgctgttttttcccatttcagattagagttacccatctggcttggtctgtaaccaggcaggaaaggataagccgttgtttccagcaaagtgaggtacctgttttcgccgatttcagcattaccggtattaccatagctcgcgcggagtttcaggtaattaagggttttattttctttaagaaaatcttcttcagagataatccagcccagggatcctgcagggaatacaccataacggttattaggtccgaaacgggaagatccgtctgagcgtatgctgaaggaagcaatatacttgttattgaaagcatagttggctctcaggaagtaggaaagaaaggtataacgttgtacttcagaagaaccaaaaacaatagatcctgctgcagatactgttttcacaagatcagaaggaaggtattcaccttgtacctgggtgcgggacaaatcattctgcagataactcataccaatggtggtactcagcgaatgctttgtgccgagatttggtgtgaatgtaaaatagttgttggtattaaggcccacattctgcgtaaagtaggattgtgcaaaaccttttccaatggcatctgatgccagcctgctgataaactgatcttccgtgaggttggtgatatctgttccaagctctgaacggaagcttaatgaaggcaggatcctgtagttcaggaacacattgccgagggttctgaaagtaacctgtttatccctgttatactgcgcatcatacaaaccgtttgaataaagcacattgtcgttgttaatagtaccatcctcataatagagtggcgacaatggcgattgtgctaccagctgacctggtgtggagaatatgttatcattcgctaccctgtccagctgtgtacggcttacattcaggttcataccaaatgaaagcttgtctgtagcgctatgttcaaggttaaggcggccgccataacgctggaacttgttgtttatcacaatagcttcctggttgttataaaatccggaaacgaagaactttgttttttcggttcctcctgtggcagaaaggtcaatctggttagtgtgggccacatctcggtacgacaagtcttcccagttagtacctgcacccgggttgtgccagtcctttccaacagtcagataagggaataagccatagtcggggttttcaagtccgtctttaaacgcagcaattgcctcttctactgtagcatattcgggattatcggggtcttgtgtagcaaaagcggttctgccatcattggtagctgcttcttccagcaggtctacatattgctgtgcgtttaagaatcctcttttacgggttggtttaccccagctgctggctgcattcagctccagccttgttttctcacctgttttaccttttttggtagtgatcaggataacaccgttagaaccgcgtgcaccatagatggcggatgcggcagcatctttcagtacttcaacggactcaatatcgttggggtttatgtcggccaggggattggtggggtcattatttatgtcagagctgcttacagacaatacgggcattccatccaccacatacagcggctggctgttggcagaaacggaagaagtaccgcgcacgcgtattttcattgcctggcctactttaccactaccggattcaatgaccacgccgggcgatttaccctggatggccgattcaaagctcactaccggctgattctcgatttccttcgccgcaattttacttactgcgccggttacctcccgcttgctttgcgtaccataacctactaccactacttcagaaagctctttgttaccggttcccagctcggcattcaccacctgctggtcgcctacaaccacttctttatcaccatagccaacaaaggagaagaccaatgtggttccttttgcgggaacgttcagtttatatgttccgtcggaggcagtgacggttcctatagtgccgtttttaattttgacagtaacgccaggcagggcgctgccgtctttctggtcggtaactttaccggtaactggtttggactgggcaaacgaaagcatgcaaaatagcaataggatgcccataaacgagaaggatcgtatcatggttcttagtttagatttggtttaatgtcagcaggctgaactatttgattgaatgatctggttgaatgctacatcgggctcaactctcatataagcaaaaacaccggaaactggttaatcgtcatccgtatggtaaaactaaaaaatattttctgtttttcttaacaaaatgttaaatcgcttatttacaggttattaaacgataaaaggcgacctttggtcgccttttatcaatataacaatattatttaattagtccctgcttcttgccccggtgtatatcaaaatataatataccagcgtggctatggaggcaagtgccgctaccacgtaggtcatggcagcccaccagagggcgtttttcgccttgtcgtgttcctccctgcgcataatagtggtattatccagccaggccagcgccctgcgggaagcgtcgaactccacaggcagcgttaccaccgaaaatagcgtggtgagggcaaaaaggataataccccccaataacagctgcgggaaggtatttatgaggaggataccggccagcaatacccatgaaacgatattggagctgaactgaacaattggtaccagcgtggaccggaggcccagccagggataggctgccgcatgctgcaccgcatgtccgcactcgtgggcggccactgccgcagcggctacattggcgccattgtacacatcggggctcagattcaccgttttatcggccggattgtagtgatccgacagaaatcctgctgtttcacgtacctgaacgccgtatatctgattgtctttcagcatcttctctgcaatttgcttaccggttaaaccggaagaggtgggtatttcgctgtaagcccggaacttacttttgagtacgaagcttaccagcaggctgatccccacaaaaatcaacgataaaaacatgattccaggtgtcataatgataaatgttaggtggtcttatggcacaaatatctcaccagatcatcccttttaaggtttatttagcacttgactgccaaccttgctttttgtctgtaaattataaatttaacactgtcattatggcgttaaaataatttttctgtgtgaaaaagcgcctgtttgtcatttacaaaaatgtgttttattaaattttatttatatacaaaaatcatcaacatcaaccctatttatcaacattttacgagcccccaatgaaagtaatattagataaaaacaacccctgaaacaagcgatggcagccactttcttagatcaggcaaataccccaaaagttattcacatcaattaaataaacttttttattctgaagccattttgtaatttagacctgaatttaatgggttagtaagtagaaagagtcagcggaatcttccgtttggctcttttctctttttatacctcttcctctccttttttaacacttctcttcttatcatttcggttcaataaacgtaaaaacgttactttgtaacgcatcttttttatgaaaattatgagtaaaattaaaaccgcttttttctgtcagaattgtggatatgaatcagcgaaatggaatggaaaatgtccgagttgcggagaatggaatacgtttgtggaagaaagagtgcaaaaagacattccacttaaacaagctgaatggaaaaacaatgatacctcctctccccggacacacaaaataattaacctctcggaagtagttgcgaaagatgaagaaagaatattaacaccagataatgaattgaaccgtgtgctgggaggcggcatagtagcgggttcgctggtattggttggcggagagcccggcatcgggaagtcaacactcttccttcagaacgcgttacagctgaagcatatcaaaacactttatatcagcggtgaagaaagtgaacaacagataaaaatgcgggccgaccgcatccagaattccaatgaacaattctatctgctcacagaaacttctacgcagacaatcttccaggaaattaaaaaattacaaccacaactggtcattgtcgattctattcaaacactgcattcaccatttatagaatctgcaccgggaagcgtatcacaaatcagggaaactactgccgaattacaacgcttcgccaaagaaagtaataccccggtttttctcatcggacacattaccaaagatggctccattgcagggccgaaagtgctggaacacatggtggatacggttttacagttcgaaggcgaccaacattacgcctatcgcattctccgtaccatcaaaaacaggttcggttctaccgccgaactgggtatttatgaaatgaccggcaccgggctccggcaagttaccaacccttcagaaatcctcatttcacaaagggaagatctcctgagcggtgtagccatttctgccaccatggaaggaatgcgcccgctcctggtagaagtacaggcactcgttacacaatccgtttacggtaccccgcaacgtaccgccacagggttcgacctgcgcaggctgcaactgctgctggccgtactcgaaaaacgcggcggattccacttcggggtaaaagatgtgttcctcaatatcgccggcggcatccgcgtggaggaccccgccattgacctcgccgtgttatgcgccttgctttcatcttatgaagacaatgccatttcacccaaaatctgtttttcgggagaagtaggcctcagcggtgaaataagagccgtaaaccgcattgaacaacgcattgcagaagcagaaaaacttggcttcgagaaaatatttatctcccgttacaacaaaaaaggaattgatttcagtaaattccatatcgaagtaattgctgtagggagagtagaagaagtataccagcggttattctgattaccacatatctttaaaaaaccattcgatgctcaccagtttgttttccccactggttcatctgttctatccgcattgctgtgagctgtgcggcactgatctgcatcaaacagatgaactgttatgcctgcgctgcgtgcaggccctacccctcacccatttccagcgttacgccaataatcccgtagcgcagatcttcaacggaagggtacctgtacaacaggccactgccacttattattacaaccagtcatccggtttgcaacacctgatccaccggtttaaatacggacaacgtccggatattgctacctggcttggtaaacaaaccggttaccagttgcaggaaagcgcctggatcagcaccgtcgattttgtggcgccggttccactcaatccccgcaaggaaaaaaaacgtggctataaccaggccaccctgctggccaatggcattgcgcaggtaatacagctgccggtacatccggccactctccgcagggaacagttcaccgccacccaaacaaaaaagggacgaacagaccggtgggagaacgtagccaccgccttcagtgccaatggcaacctttcagccggatcgcacgtactactggtcgatgatgttattaccaccggcgccaccaccgaagcctgctccagggcccttcaacaggcgggcgcccgggtaagcatctgctgccttgcctatgcctggaaatgagacggctaaattcttctctttttttattccgggaatgctaactttacaaatacagccccgcgctgtattttaatctgtctttaaaaaaaatctatatgttcagattagctatactatcagttgttatgctttttgcctcatcccatctttatgatttcaaagtagatgctgttgacggaggaaaaatcgatttctccaaatacaaaggaaagaaagtattgatcgtgaataccgcctccctgtgtggtaacacgccgcaatatgaaggcctggaaaaactctacaagaaataccacgacaaactcgttatcgttggtttccctgctaataactttggttcacaggaacccggcagcaacaaggaaatacaacaattctgcacaaaacagtatgcagtaaccttccccatggcagccaaaatttctgtaaagggaacagacattcatccgctgtacaaatggctgctggatgaaagtaaagccaaacacatggagccggcagaagttacctggaacttccagaaatacctgctggatgaaaaaggtaacctggtagcagtattttctcccaaaactcaacctgagtcagcggaagtgattgcggccattgaaaaatagtttttataactgttaccaacttttgcgtagacaaaaaattttgcagatacttgcgtaaacgtatatccgtttacgtaagtatcctgttattaatatacaacgcgcaaccgtattcatgaaacactactttgttcctaccaataacgccttgccgctaatggcattgctgtgctttttactgatactttccgcgtgccagcacgatgtagatcccccttcactctcgtgccccgaaatgcaaatggttaccaacataggaaccagcagcaacaatatgaccttcagccgcagcctcctgttccgtgaacggacggataccggcggactcaaattcctcagtgtggaaactgtatcggattcctgcagggtggtatttaatctcacggatggtatgtacgacgaagcggggttgaagaatgacagcctgcacctgaaaacttatacctacacccggcagggagtgcaaaccggcggactggtggccgtagccgttaaaaacaacaatggggaattcacctatctcaccaccgactcttccagtgtaaccatccgtaaaatgaatctccggacacaaaccatatccggcagcttttattttacagataatgagaagaacatcagcggcaccggcacctttgaaaatgcctgttatgtatctcttcaataaatgattagcccccttttcattatcttgcgcccatgcttttttctgatattataggacaaggggatgtaaagcaacagctcgttcaatccgtacagcataaccggctaagtcatgccatgatactgcttgccccggaaggtgcaggtggtcttccgctcggactggcctttacccaatacctggtttgtgaaaacaaacaagcgcacgatgcctgcggacaatgccccgcctgcaccaaggcttcacaatttgtacatccggatatccattactcctacccggttattccgcgcaaaaccggcgataaaccagtaagcacagactatattaccgaatggcgggagttcgtaacaacgcatgcctatggcaatgcgtacgactggctgcagttcataggcgccgaaaacaaacagggtaacatcactgccaccgaatgccaggacattatccataaactgaacctgaaaagttttgagagcggttataaaatactggtgatgtggatgcccgaatacctgggcaatgaaggaaaccgcctgttgaaactgatcgaagaaccccctcagaatacactgtttatcctgatcgctgaaaaccaggaacagatactggccaccatcttatcaagaacacatcttatcaaaataaacccgctggcaaaagaagacctggtgactgcgttggtgcagaaaagtaatgttccccctgcaaaggcccagcaaatggccaccattacagcaggcaattaccgggaagccttgtacctgttgcagcattcagacgacgactaccacgagttgctccgcagctggctgaaccacctttttaccggcaaccgggtagccctgcaggaatggatagaagggatttccagtgcaaaaaccggcagggaaaaccaaaagcagttcctccgttatttcattaacctgctggaacatacgctccgtttgcaatacctggataagagccagctggctttttccacggaggagatggacttcgccgccaagctggctaaactggccaacctggaccaaatgcaggaaatcacggaggcgctgaacaacgccagctactatatagaacgcaatgccaacggaaagatgctatttcatgccctgtccatcaagctgcaatatatatttaaaaagaaacctataccggttatgtaataaccaccggcttcctgcggagctatcagctccttttccctatctttgttgcttccggccttttgtttttctgaaaggaaaaacgtattttgaagaactggaataacctgaaatgcttatttataaaatttaaactaattaataatatggcttgtgccggatgtggtacgggtgtggaagggaagccgtcaggatgcaagagtaatggaggatgcagcacaggaggttgtaacagactgaacgtgtttgactggctgtccaatattccccttggtgatagcttagcaccatttgacattatagaagtgagttttaacaatggcagccgcaaggactttttccgtaacgtaaccaaacaattctttgataaaggagaaatggttaccgtggaaggggtcagcggttttgacgttggaacagtaagcctgacgggcgagctggtaaaactacagatgaagaagcgacgcgctgaagacacacccgaagtaaaaaaagtgctgcgccgttcaacgaacgacgacctgcagcgaatgaatgacaacaagtcccgcgagaaagaggcgctcataaaatccagagcccttgcccgcaacctcggacttgaaatgaaactggcagaagtggaaatacaggccgatggccgtaaagccaccttcttctataccgcagatgatcgcgtggatttcagggagttgattaaagtatatgcctctgaattcagggccaaggtggaaatgcgccagataggcgcccgccaggaagccggaaaagtaggtggcatcggcagttgcggcagggagttatgctgctctacgtggctgtctgacttcaaaagcgtgaataccaccgctgcccggtaccagaacctgtctatcaaccaggccaaactatctggacaatgcggccgtttaaaatgctgccttaactatgagctcgatacctacctcgatgccctgaaagatttccccgacgatgccgataacattgaaactgccggcggcgttgcccacctgcagaaacgggatatcttcaaaagcctcatgtggtactcttatgaaggcagtaacaaacagtatccactcaccatctccagggctaaggaaatacgcctcctgaacaagcagggcgttaaaccagacgacctgaaaccggtagaagtagtaaccgccaaaccaaaagaagcggatctcggatacgcagatgtggtgggattaatcagtctgaaatctctcgaaaaaacagctcagaagcgtaaacagaaggatagagacaaacaaaaacaacaacgcggaggagaacgcggcgaacgtggtgaacgcccggatcgtggtgaacgcggcgaacgtagcgaacgtccggatcgtggcgaacgcggagaacctaaacaagcccagggtcagggtcagccaagaactgattcccctaaggcaggtcaaaggcccgacaaccgccagccttcagagcgtaaacccaaaccggataaccgccagcggcaacaaggcggaggccagcccaaacagggacgtgaacaacaaccccgtaacgagcagccatcaaaccggcaggaacagggacaaagacaacctgcgccaaagcaacccggtcagcaaccagcccaaccaggcatgcctggaggacagggacctaccaatcccaaacaggacaggcgtccaccacggcataaacaccggccgcccaaccctaacaagaacaacaatcctgaaaaaggacaataaataaaaacaaaaaagacaaccggactggttgtcttttttgttgcatactgcaagcatttcttatatgttcaagccggcacacggagctgactgaccttcattacccttacttcacggatgcctcttccatgccgcatacctgcgtatcccatggagtatccatgcactcttcatggactcatgatgcactatcaatgcactccccatgcactatgaatacactatgccccttccgggacctattattttttgaatatcagatggtgaggaaaaattgttagagaaaaccaagtaaaaggccgcccagacgaggcagcctttgttaacaattggtttttgcttatgagaaaacttaaaaaatgctattttatatctcttcacaaaatcaatcacacaggcgcctctactgcttatcacacactcttacgcttcattctcaaacagtagtttataatagttcatgttggtggcttcatcaaatccgcgctcaatcatctcacggttgccatgaatatatacatgaaagttacgatccaatttcagaatgctcttaaatactttctgctgtttctttacagcaggtgcagatatttcaaactcgtcagggatatcttgttgaaaatgattcgcatattcgtttcggtactccttaaaagaagcaatagcgtcgggatgacctagtacctctttcgcaaaatcgtccagttggaattgttctttttctttgaaataagcggctgatttatttaacagatctacctgatctactctgtccatctcatactccgttggcaatttgttgtgtataaactgtttacacatgtccaccgcggtttctgtctgatgataactgtcctcccggcgttgtacctgtaaaaaggcatccttccaatacaccgcctcggtttgtttgctgttactgtctactatacttactttaaagccttctgtttcttctgtattaaataccagacaacctttatccagcttattaatatttataccgtcctcgtaatttacctgataattctcgtctgccagaaatacttttaaataggtatcgcggttctccgacttaaaaatgcctatggcttccacctcttcaccatccacctggcacttgctaaagtaggctatatatagctctcccccttttattttaggatgggtggaatgtttatatagatgtttggcaatattgaccgactgctcctggaattcattttggtcagtaaatatacgtcgacaatattgaaatatttcattcaattgcagatctgcgtcatgacggaatctgaaatactctgctgcattggcaaacggctgaataaaataagtcaccaataactggctgatcgtttcatcctccagctgcaaaggcgctttggaacagagcagggcctcatcgttagtgggattccctaccttgtgtatcgttaattgcgccaaatctttaaactccgaaacatggatcatgggcgcaaaattaataaattagttgacaggcaacagatccgtttctcccggtaattatttcttgataatttcattacataccctccctcccatccatatacgctgaaaaatatggaatagttccttaatttaaagtttcaaaacaaaacgaacatgagaaaatatatctgcctgctggcaatgacggccggatacggtctcccgctgatggcgcagcaaaaaaataccaacaggcccgtattcgaaacccgcgacctcacggcagaaaatatgttttccgtaaatattgaaggacccaactttgacaaagcaggcaatttttacgtggtaaattttcaacaggatggcaccatcggtaaaataaataccaaaaccggcgccggtgaaatattcgttaccctccccgatagcagcgtggccaacggcattcatttcaacagtaaaggaaccatgtttctcccggatttcatccggcataatgtgctcaccattgatatgaaaaccaaaaaagtaggcgtatacgttcactccgatcagttcaaccagcccaatgatctctgtatcaacagcaaggaccagatcttcgtcaccgacccgaaatgggccagcaacaccggccagatctggcggatagacccgggccaccacacccccatcctgcttgaaggcaatatgggcaccaccaacggcattgaactcagtcccgacgaaaaaatattatatgtgaacgaaagcgtgcaacgcaagatctggaaatacaaggtggataaagcaggtaacatctcccgtaaaaccttattcgccagcttccccgactttggcttcgacggaatgaaatgcgacaaggtaggcaacctctacgtagcccggtggggaaaaggcgtgatcgctgtactctcgccaacaggaaaactgatccaggaagtacccctcaaaggaaaacaatgcagcaacctggtattcggggataaagacggcaaaaccgtatacgtaaccctgcaagaccgtaaatgcgtggaaacattccgggtaaacgtaccgggtaaacgcttttaacgcggagtttgtcttggctcaggattacgctgattttactgattagtttgatttttactttttggatttttttgattttcttaagatataattaagggagataagcgaatatatccgcttctatctcccttaatcctttataaaatccagaagtaaaaatcaaactaatcagtaaaatcagcgtaatcctgagaaagacaaaatccgctggcgatcaaactactttataatcagcagccagcccttgttcttttctacggggatactggcatctttaccaaatacctgcccttgctggaagttgcgtatgtccggcgccgttatcgttgcctttgtagggtctatgcccagtgctttccagtcgatggtgagtttaatggtggtgttttccggcgcccagctggcgagggataccagtactgcgccatccttacggtaaatggtggccggtaccaacgggttgttggttttaaccgggttattttctacccagtaaccaatcatctttgttccctgcataccaaaatcatcccacactttccagataggacgcggatcggaagtagcagtccacggcatgcggttggtcataccatacaccataccccgccactggttaccaccatcctggagcatttcgcccatcaggccaaaaggaataccgcttacttctgtgaggaagaaatcaggattgtttttttcataatcaaagtactccccaaaccaaagcctgttcaggtaagggaagtgctccatataaagcaccgcactgttaataaatccatcggatttgttatactggttggccgaatgcagatcaataatgcccggatgattatcctttgtcagcacgcgtttcacacgtttcatggttacccggtcaaaagctacgtcgtccaggtaaataccatcgatccctacgttttgcaccagccagttcatcccttccacatagtagttatgccagcgattcatgccactgttgatgatggcggcatccttaaactccggtacaaaccatgccgcgatgtagtcttttcctacatgctcctgcagccaggagaagccgccacccttacccggactgtatacttcatgccctaaactgcgcagcgggaaggtttcccaggcatggttcgataactcccttacggtattatagatcttaactttcagccctttctgatgcgcttccgcaatgtagtccttcatcgccttccattcaatgaacggatagttgatccaggggttaatctcgttgccatggtgaatgtttaccaccgtggcgccggtagtcttgatgctgtcgaggttattataccggtgatagaaacgggtagaccactggaaatcggtgttaaccgggtggaatggcgtgatgatcaggtggaagttgtaatacagtacctctcccttatgcagcgttctttcaccgctatagttatttaccagtatagcctttcctttttcgcccacggtgataccgcctttatcgccattaccccatgaagtgggcagcagcagcggcttctggaggtagaagtttgtattcagcgggcgtacataattttcatcccgcaggttaaactggatgcccgcgttcacatcgccaatccaggcgccatcctggtttttgtttttcacgtcccacttccagtcgatcttctccgggcgtacgccacctttctggttcagccccatcatgtactttgcagcgcctttatcaaacggcaggtgcatcgtgatatctttcagggatacgtcttccagcgctgttactttcacggtatagtcgaggaaaccatcaaattccagggtgccgcttacttccatctccaggccggcagtagtgttcaccgctttccagctgattttccccggcgtttgactggtaactttccagccattgctttgccagcgaagatcctttcctgtagcggcttcaatgaaatggaaatgtaccggttcggtgaaaatatttttaggttgtgcagacagcgacgtcatttcaggcgtgaaaaaagtctggatctgcgcagggaagccatctttatggatacctactttacggcccagtaaactgatcacgctgtctttcatttccagtggcgtgtaaggtgcaatcacggcatcgtcctgtgccagcgtggagtttagccatttcaggcgggtttgtttccagggctcattaaagccactgttcacggccagtttattcgttaccgttagtgtgattcttattggcatggcaggcatgccggctgcctttatggtggcaatacctttatagatgcctgctgcagcgttttccggcacatctatcccgcaccacagggcctgtacttttccttcggggatattcaccgttgccgaaaaaggtttggcatcgtaagtggtaccggtggtattgatacagttgagttgcgttgccgggatggtttgtccgccagtggttttcaggtcggcaaaagaaatctgcacatccttcatttcatggcgggcataaacgcccagctgaaaggcatagtattcgcctttatcggcttcgccggagaaggattgggaaggccctttctttatccagcgctgtggcaggtcgtccgtcattttaatagggaactgccggtcttcgggaaacagcatatagccgccacccggatgtttcagcagcagctgctttctttctgcttccgtggcgattacttccatcgggtagaaggtattgaagctgtcaatagcttccagttgcttcacagtggtattgggctttatgcccgctggtatggattgcagccagttgttatcggcggtttgttccggcgccaggtacacgcctttcgggtagttgtcgcggccttcgtttttggaaggcaggtaataaatatagtagtcgcctttaccggaagttggttcaaagcagatatcgccttgctcacggttaagtgtcaacgtttttacattggtaactttttgttttgtttttgcatcttcaacaatgatccgtttcagctccggatgctcgtctctacggcgccaggggattataacccgggctacgccggcggcgccattaaaggaaactaccgcacggtggttaccgagcgagtctgcgttccagttattgttgccattggtatacttcaattcctgggcgagtgctgtggtaaggaagctgaaagtaagtcctgccagcagcaatcctctcctgaaattgcgggaagggtggtttgtctgatacatgaagaataagcaattttttaaatgttcaccggttataaatttactactgttgcggtttcttttcccgattattttataaaagcaaaagccccgcagaacggggctttcaccgggtaatactattgaatcgggttttgcaccaggttaggatcaagcaatatttcctgttcaggaataaagtgtaccacccttgcatctgtataagaaactgtttgcggattattttgtacgccgggataattgcggtatacattccggttattgcggaacaggtcaaatacacgatgtgtttcaaaggcaagttccaggcggcgttcgtccagtactacatccagcacggaaggatagccatgcaggtcagatacggtaaacagcgccgcgccgcttaacccggcccttttacggatggtattcacatcatcgatggcggcagcgttgttgttcagcttcgcattcgcttccgcacggatcaggtacatttcagccaggcgcaataccaccggtgaactgagggtaggcacgttatcctggttggaatatttcagcacgtaccattttggaacgccattgcgggaagccattactttctggccgccggcattcacggaatcccggccatcagcgcctttcaggtacaccgcttgcacaaaggagttacgggcatctgccgggtatttgtgcagcaggtcgaggtacgactgggaagcatacatttcgccatagcccataccaccgggcgacatataatacatagagccgatagagctccaggtacggtcgtcctgcaaggtatgatgaatagcgaagatggtttccttgttgttttcattggttttggtgtaataaccgggaagatcagaagtattcaccagggaatactgacccgaagtgataacagaatctgcataaatacgggcagaatcatttttccccatgtagagatacaccctcgccagtaaagccatagcgccatatttggtggcgtagctgttggtgttggagttgtccatcaggtcttttcctttcttcagatctgctaccacctgcgcgtatacatcctgtacagtgctacgtttaggcatggcagttatatcgaatttagtaacaaccggtacccccaggttggttgccgggctttgtgtataagggcggccgaaagatcttaccaggctgaaatgtacaaaggcgcggatgaacaggttttccccgatcatcttattcacggcgtccgacttaccttctgtcattacctccagcagcttattacagccgttgatcgccttgtatcctgcccgccagatctgcaatgcgttggcctggttggtcaggtgcccgtaagtgtatgaataaaaaagcgcatcagtagtagcgccactcagtgctacatcatcactggggaactctcccatctggaaatagttgcgcgtaaagttttcttctttcagtaacgcataattacctacagtggccgccggccatttagtttcatctttcagaatattatcatccggaacagcactgtacgggtctttcttcaatgagcaggaagtagccactgataacagcaacagccctgcaaagtattttgacatgtgtttcatgatcatctctttttagctcctgttaaaaattaatttcaaggcctgcaaaccacttggtgctggacggatacttgatgtagttgataccgcgatcatctacttccggatccagaccggagaatttggttaaggtccacaggttatcaccgccaatagaaattctggcgtttccaatatgcgcgcggtccagccaggccttcggcaacgcatagctcaggtttacgtttctcagacgcaggtagcttccgtcttccaggaaacgggaagatggtttgtgtgagtttttatttcctttgatagtatactttggatgggtagccacatcacctggcttttcccagcggctccagtctttatccagcgacatcatattataggtataatatgcgccgtcattgtccatcagttcacgggtgctgttatacacatcattaccggaaacaaacgccaggaaggcacttagctggaaatttttataggagaacgtattacgcataccaccaaagaatttcggcgtggcagaacccacaatctgcagggacgcatcgttatagttattggtagtggttttaccggttacgttgccattggcatctgtcactagtttttcccacagcggatcaccattggcaggatctacaccggcccatttacgcatgtagaaactgcgcatatcctgaccctgttgcaggatgaaatagccgctgatcggatctacgatctggttcttcccggtatacagttcggttaccctgtttttattgaagccgatgttgaagtcggtgctccatttgaaggcgcctacgaggttatctgtactcaggttgatttcaagtcctttgttacgcacagatcctacgttctgtgaaatgtagctgtaaccggcagtagcaggcagcggcacattgaacaggaggtctttgttatctttctggtataattccacggtcaggttaatgcggttaaataatcccaggtcgataccaatgttggtattgtatgctttttcccaggaaaggttcggcacattatacacgctttggtaagcaccggggaaaccgttgtactgcgtattgatcaaataggccccaatagcgctgtagtcgcctatttccgcgttaccggtagttccgtagctggcccttaacttcaggttggtgatggcttttatctgtttaataaagttttcttcagatgctgcccaggatgcgccgaaggcatagaagttaccatactgctggttggcgccaaacttggaagatccatctcttctaaaggaagaagtgaagtaatatttataattgtagttatagttcgcctgtacaaaataggagttaaaggcgcgggctattttagtaccgccaatagacatcggcgaagaagtaccatccagtacctctactccctgcaggatacctttaccttttgcattgatatcattaagattggcctgctggaactcagcgcccaccagtccgtcgatgttatgcaccttgttgatggtatatcttgctttcaacaggttggagctgatatagctcgcagaatcctggtagtaattatacaggttgccacggtcgtcggtgccggaagaagtccgcacatcgccgttgctttcctggttgaagtggtaatactgtgcgcggttggttgagctgaaggacaaccatttggtgatgtcgtattccagtttcaccagtgcttcgagcgactgccttttatttttaatatagttatactgctggtcgtaaaggaagttagtcatatcccttccgtaccaggtagcggcggtgagcgggtttaccggcttgccttgttcgtcgtacgccttgtcccaggggagattggtatagtattgatacaatgagccgtttgaattatcgtggtcggaagtttgcgttccggcgaagttggcgctgatgcggaacttatcggtgatgttatgatccaggttgaggcgggcgctgaaacgctctaccccggtacctttcaggataccatcttctttatagtagttaccgcccaggtagaactttgttttttcgttaccaccgctggtagataattcgtagttctggttggtggcattctggaaggccagcttctgccagttggtattgatattatggagagatggatccagcgtagcgcctgcggctttctgcaggtcgtacaggtctgttccgttcatgagatggaaatgtcctgtattaagctgggcggttcctacgttggtgcggaagtttacctgggttttgccggctttacctcttttggtggtaattaccattacgccgttggcggcgcgggcgccgtacagtgtagtagcggcggcatctttcaggatggtaacgctttcaatatcgctggggttgggtaatccgcctatgataccatctacaactaccaggggagagttgcccgcagtaagggttccgttaccacggatgcggatcacgggcgccgaggcaggatctccggaagtatttcctacaaatacgccgcttactttaccctgcaacattttatccatgctgctggcagtaacgtctttcagtttagcgccgcttactgcctgcgctgcaccggtgaggtttttggtagtagtggtggtgtaacccattactactacttcttccagtttcttggtatccggttccagtttaatattgagttcagagcggccgcctattgctactttctgttgcaggtagccgatataggaaaatatcagcacgctgttttccgaaggcgcctggatagtgaacttaccggtagcatctgttacggcgccggtgctggcgccttctacggtgatcgttacaccgggcaacggatctttggtagtggcgtctgttacatatcctgttacttttacctgtgcggtaccggtgggagtaatcaccaccaggttgttttccagcacgcggaaggtaacattggagttgttgaagagttccttcagcacttcactgatctttttatctttcacatcaatagtcactgccttattcagatcagtaaagttctcgttgtagaagaagcgataattgctgttgttttcgatgagtttaaatacatctttcacgcttttattttcagcatgcagttcttttatattatcctgcgcgtatgcattagcggatacctgtaaaaaacctccgaaaatcagcagacccgtcaatttcatcatgagcaataattttcgcccggggcaaaataatgccgccaggtttgcagtggatttcataaacttgtatagattttagttaaacgataattacggcgattgcccgtcgcaaaggcaattcgccattaagtgattttcgttgattggggtaagtcgcattaccccaatttttttagtccttcatgtcgggcatgtaagttggttttacaggtgattgaatgatggttgtcccttctatccggccattaccggcttttaaatgctttattatatttttctctcagctcttcgtccagcgccagggtaactacacctttgttgatggtgtatttcagcggtgctgtgagctttagaatgttcagtacctgttccagcgtttcctgacggaaagtgccactgaagcggtattctttcagttcctgttctttaaagatcacctttacattaaacctgcgttccattgttaccgccagttcttccatggtttgagcggccactatccagttgccgtctttccaggcggtatatatttccgtattgttcacttccctgctttctatcggagcagcggtggagctgtctccgccagatacaggcgttttcaattgttcactgccgtttgacaacggttttttatacacaacatgttgatgtggtttcatcataagtccgaaaggcgtagtggttttgctgccgtctatcttcacttctccgtctaccagcgtggttactacggttttatcttccgggtatgcttttacattgaaagatgtacccagcgcgagtattctcaggtcggaggctcttaccgtaaaaggcttttgtgcgttggtatgcactttaaagaaggcctctccctccagttttacttcgcggccgcggaggttgtacgactgtgcatactgcagcttgctccctgcattcagccatacttccgtaccatcagacaattcaattttggtggtagcccctttcgggctggttaccgttaccagcgcattactgctgttatcttttttaccggaggcccaggcatacaccaggccgccgccgattaaaaaaggcaatgtataggaggcggccacacggaaatagtacctccatttgtttaccgccaatggcggttctatggccgtgctatactgcaaactatcccaggcggtgccggtatcataactcccttcccgtgccgttgcctgccacgcatccctgagctgaaggaaataagactggttctccgccgaggcattgatccagtgcgttagcgccgcctgctcatccggggaaatattaccggataaaaaacgtgcgatcaggtcatctgcctgctcctgtgtatagttaggacccatcatatagaaaacaagtagtaagacaacatttaatgccgggtagggtgacaagcgaagaaaataaatgttgttttttttaaacctctacttcaaaagaggaagtagttcgtcgcgtaacctttgcagggcgcgggtcatctgtgttttgacggtgttgatggagatgccgaggtggcgggaaatttcggggtaactcaattcttcaaagcggctaagccggaatacatcctggcactggggtggtaatttgcggatggctttttccgctatcagctccagttcggattgttcgagtttttctgccggcgaatgaccggaggcaatgctgaacagggaaatacgggactccagctgctgaagctcttcgctgccgtattgcgttttcaccttgttttgcttgatgtagttgaggcaattattctgaacagcgcggtacaggtatgctttttcagatacctggatgtccagctccctgtacttctcccatatcttcaaaaaagtatcctgcacaatttcttctgccagttcatgtctgtttacgaaatcaaaggcgaatgtacagagcgcggcgtaatactctttgaataatgattcaaaagcgggtagctgacgttgtttccggttaatatttttacttacttcctccaaagtattccttcgtccacaagattgttcactgcggcaaaagatacgtaaagtaggttcaataaaaaaacgcggatcatagacccgcgttttaccatctttaactcgttgaattacatacacaagccgccacaggtgctgattgtctgaccggttacgtaaccgctcatatcagacgccaggaacaggcaaacgttggcaatatcttccggtgtgccgaagcggcccagcggaatctgagcaatataattggcagcgccctctccttctttgaggtagctggtcatgtctgtttctacaaaacccggggccacggcattacagcggatgttacggctgcccagctcctgtgcaatggacttggtaaaaccgatgataccggctttagaagcggcatagctgctttggccggcgtttcccatgataccgattacggagctcatattaatgatgctaccgctttttgccttcatcatggggcgtattacatgtttggtcatgttatacacgctcttcaggttgatgttcattacatcatcccactgatcagggctcatacgcaacagcaggttatctttggagatacccgcgttgttcacacaaatatcaatttttccgaattctttcaatacatccgctaccagcgcttcagtttcctcgtaaacgcctgcattggatttataagcttttgcttttacacccaaagcggtgagctttgcttccagtgcctgggctttttcatcggaacttacgtatgtaaatgctacgtttgctccctgtgctgcaaatttcaaagcaattgcttccccgataccacggctggcgcctgttactatggctactttgttctccagtaatttcatgttatagttgataggttttaagcattcatatgatccgccgcaaattgcagaatttcttcgaggtatttgcggtcgttgttcagtcgtggaactttatgttgtccgcccagcttgcctttgcttttcaggaactcgcaaaaagttccttccggcaatacacgcactaccggcatgtgcagggcgatatccttgtatcttttggcctcgtaatctgagttaatggcttttaaagtactgtccagtaccgtaatgaagcggttcaggtcatccggcgctacttcaaattccaccagccattcgtgtccgccgttgccatgatcactgaaataaacaggggctgcggtgtagtcatttaccactgcacccgtagcttcgcaggctttggccactgcagtatctgaattttccacgatcacttcttcaccgaaagcattaataaacgactttgttctgccgctgactttaatacggtaaggaatcagggaggtgaactggatggtatctcctaccatatagcgccataagccgccattggtactgatcaccagggcatagtttttacccagctccacttcctgcagttgcagggtttgcggattttccttgtccagttcctccattggcataaactcatagaagatgccatggtttaggaacagcaacagcccttcttctcctaccacatcctgggctgcaaagaagccttcggatgcgttatacgtttcctggtaatgcattaaaggcttgcggatcagttttttaaattgctcgcggtaaggggtaaagcttacgccgccatgcatataaagctccaggttaggccatacatcggccaggttgtctgtaccggtgagttcaaaaatacgtttgatcagcacaatggtccaggtaggcacccctgcaatagaggttacattttcatggatcacggcgttggccatacgttctattttctcttcccattcgtccatgagcgctatttccaggtccggtgtacggatcatattgccgtaaaacggcatattctggagcattacggcgctcaggtccccgaaataggaatcgctgttttcggaaagtttgttcacctggtgactgcctcctattaccagtgatttaccggtaaatacgtcggagtcggggaaattattgtaataaagggagatcacatccctgccggaacgatagtggcattcatccaggctttccactgttacagggataaatttgcttttatccgcggtggtaccgctggattttgcaaaccatttgatgggtgtattccagagtacattctgctgtccctccatcgtacgctgtatatagggcttgatggtatcataagtatgaataggaacgcgctgtttatattcgtctatcttataaatctttgaaaagccgtactgcttaccgaattcggtatactgggcggcactgataaggttttggaatacctgctgctgcacctgcacgggatactgcatgaaatacgcaatacgccccattcgcaatcttgccagttgtgatattgcaggacttaaaattctcatataggatgctgtagaattatttttattgtttagctgcttcgtccaggtaatctttacggcgaagaataaaattctggccaagatacacttttcttacctgttcatcggctgccagctcttcggcagatcctgatttcaggattttaccttcaaacaataaataagcccggtcagtaatggacaatgtttcctgaacgttgtggtcggtgatcaggatacctatatttttgtatttcagtttggctactattccctggatatcctctacggcaatggggtcgataccggcaaaaggctcatccagcaggataaacttcgggtctacggccagggcgcgtgcgatctcggtacgacggcgttctcccccgctcaatacgtcgccagggcttttccttacgtgcgtaagccggaactcagacaaaagactttccagcttctctttctgctccgcctttttcagggtagtcatttccaggacagcggaaatattatcctccacgctcagcttccggaacacggaagcctcctgcggcagataaccaatgcccatctgcgcccgcttgtacatgggcagcttggtaatgttctggccatccaggtacacattcccttcatcaggcttaataagccccaccaccatgtaaaaggaggtggttttaccggcgccgtttggccccagcagccctacaatctccccctgggacacttccacagatacgtgatttaccacggttctgttgccgtaacgctttaccagctggtctgtatgtattcttaatgtcatatgatcaaacttagcaaaaataaacaattcattcagttagcctagttatagttatcctaagattaaaaatgatctgataataataaggggatatcttatttttgcccgcgtaattttagcaggaagctggctttatatccagccgccttcctcaaagcttataactttatgaaagtaactgaacatattgccaaggccaaagacaccctgatttctttcgaaatcctccctccgcttaaaggaaagagcattgagtctatctacgaccacctggatccgctgatggaattcaagcccgcatttatcaatgtgacctatcaccgcagcgagcatatgttcaagaaaaaggcggacggatcctttgaaaaggtggaaatccgtaaacgccccggcaccgtgggtatttgcgcggccattatgaaccattataacgtagatgcggtaccacacctcatttgcggtggttttagccgggaagaaacagaaaatgccctgatagaccttaacttcctgggtatcgacaatgtactggttttacgtggagatgctcccaaaaatgaaactttctttgaacccgacccgcatggacacagctatgcaattgatttgctggaccaggtggcacatatgaacaacggcgtttacctggaagatgatctgcaaagcggtgtaaaaaccaatttctgcatcggcgtagccggttaccccgaaaaacattttgaagcccccaatatgcaaacagacctgtcgcacctgaaacgtaaggtggaaaacggggccgattatatcgttactcaaatgtttttcgacaaccagaagttcttcgacttcgtaaacaaatgccgtgaaatgggtatcaccgtgcctattatccccgggctgaagccattaacttccaggaagcaaatgaccatgctgccacgtattttccatgtggaccttcctacagacctctctacagaaatcctgaaatgcaaaacagacaaggatgtggaacaagtgggtactgagtggctcattgcacagtcgaaagaactgaaagcctttggcgtgccggtattgcactattacacgctgggtaaacccaaggtggtgcgtcaggcagtggaagcaattatgtagcttatcctaactccttataaaagcagaagggaaggacgaaagtctttcccttttttgctgtctttcatataaaaaatgccatcacgtagatacgtagtggcatatccctataactgtcacacttttaattataactgtccaatgatcgatgtcatcttccgatggcatctttcgctaataagacgcggtaaaaaggaatgacccctatcttcttttaaaaaaaataaaaaagaccgccgtaagaggcagtctttctattgtctgtatagtatacgtactattttcgtgtaaagagatatccgacagacaagccaaaataacggtgcttttcctgggttctgtcgctggcactaacgtctaaaaagccggaagtatagtttatactaaacaataacccgtttttaaattcatagccggccagtaaattaacacccgcatctatggcgttggcatgtaactcttcctggttcgcaacatcatctccatcaaatttaatctgcctggattttttcgtttcggcgttgtatcccttataagtaacttttccgcctataccataggctatataaggtcccagccccgcaaaaacttttcctttgcccgcttcccctttatataaaaagttaacgggtaactccaggtagttataccggtagctggtagtagcttcctcgttactgcccatgcccgtcataaaggtattaacggctttggtgcctttaacactgtataacagtgccggctgaacggcaaaactcttcgcaagcgggatgtctgccagtatccctgcatggtaggcaggcagcgtccggtcgtgaaataatgtcatctgggtgcggtctttcagtttcatgtttccgcctgaaaaaccggctttgactccccatcttacctgggcacacagggttaacgaacttaacaaggttacaataatcaggatgttctttttcatataggtttaaggaatgttgtctgtcaatttgctaccggtgggtccggggaaacaagtatccaaaggaaatccggaagcttcggttcagctcttctgcatgttccctggtagttacatttataaagccggaagaataacctgccgtaagcaaaaatccttcattaaactcataaccgagcaggaaattagccgaaacgtctaccgggttagcatgtatttcagagccgtttgccggaaccgctttatccccgtcaaactttacccgttttgtttcttctttagtgccttctttgatataagtggccttgccaccaataccataagacaggccgggaccaaatcctgctacaattttaccttgtcccaatttttgcttaaacagaaagttgacaggtaattcaagatagttataccggaatttgacgatatagtaatagttcccggttgattgctccggccgggttctgtaaccagcaacgctgtaaagaagtcctggctgtaccgccaaccattttgcaagaggaatatctgctaaaatgcctgcatgaaaagcaggcaacataaactcgttccggtccggaacatcagcggggtcagtcagtttcatactggcgccggtaaagccggcctttagtccaaatctaacttgcgcagttgccatctgaacaaccagcagggctacaacaatcagaatatttcttttcatgcattttaagtataaatccgctccctgttaacaaaaaccgttccccgcgtaaaaagactaccagtcttccctgtcaaagaaaaaaccaaggcttacgccccaatacctgtttttataattattatccaccgattgatcgatatccatcatgccgtatccatattgtgcactcagtgaaaggcagcaattcaactccaaacccgcaatgaagttaaccccggcatcccagcgctgcaggttcatgttagtgccgaaaatattgggagaccccttaaaatcgatccgttgggatcccgattgcaccagtttattttcggtgtaagccgctacactgtaatcgccgcggatacaataagcggcatagggacctgcacctaccagcagcttaccaaagcttaccggcaccttatataccaggtgaaccggcagttccaggtattgcagtttcagctttgttgccccggatgtaaacaggttaaccggatgggataccgcataatccagtcccgcacctttttttatgtaactgatgcctggctgcagatagccatttttaaacagcggtacgttcgtatagaagcttgcctgccagctatccgttttttgggttcccggcgcatatccactcccggaagactccagcccggtattgatatagccgccacgaatacccaaacttacctgtgcatgtgaggtagctgtaacaaaaaatactgttacaaaaagaagagtaaaaattttcatcagtggttcggtaataaaaggattaagaatatcacagtgacatcattttgggggaaaagtcttaatgctcagtcggttattgtaggcgaaattaaacaaacgttttcataaaaataaaaaaccacccgaaattcccgggtggttaataaaaagttcatcggaagcaggttttacctgccaccaaacttatatccaacggacacgccaaaagacgtgttcttaaagctacggtcgttatcggtattatctgccgtattaaccagaccaaggtcggtattcagaccgaaatacagtcccacaggcagttcataacctacattaatacctaaaccggcatcgaatcttttctgtttcagcacggtggcttcatcatcatatacatccagatcgccaaacccggtatccttgatctttccgcccaaaccataagcgaaataaggtcctgcagataataccagcctgccggtacctacttctggtttaaacataaagtgaacaggcaactccaggtaggacaaagtagttttcacatctgtatccttgtccttgcctcctttaccggaataaagtaatcctgttccgatataaaattcatctgccagcggaacatctaccgtaaccccggcccttatgccggtaagaatagagctggtttcttttccactgtttagaacagcattttttgcagtcatgctggaaaactgcggtcctgcaacgataccccatttagcctggccaaaagaaagaccagctaccagtaatgcggctgcagataataatacctttttcatgtgtgatgtaatttgaatgattttaaaaaaagcgatacccacaggtcaggtatcgcttccctaatttttttgattgccaactaatgaatgaacctgtttttttttgcttgcttgcagttattacaatttagttccgtatttgtttattaaccagctattttccgccgaacaaataacctacagaaacactgaatacccggttcttgctcttgtcatcggtactgttgtcctctccggagttcactttggcaaaaccaataccatactgggcagagatcaggaagttgctgagttccgcaccaatctgtacgttaccaccccagtcgaaacgtttcattttattatatgctgtattcgggtcgttattaaaaggggtatcatcatcccacttaatactttctgaaccactggcatgcacaccggcaatagtggtttcatacttttgcttaccggcaacaccaaatgcaaaataaggacctacacctgcaaagaggctggaactctcacctattggcaacttagccacgaagttcagcggaatttcgatgtaagatgggttgatggtgtactttgcgtaaggattggtagtggagttattcttatctcctgtttcaagcttggtacccttggtggtataaaatacaccgggctgaaatgacaaaatctttggaactaacggtaaatctgcaatggctcccacattaaaaccggataatgaacgactatcttttgtatttccggagttatcataagtaatgttggagagattccagccagccttaatcccaactctcgcctgagacatcgctgctactgaaatcgttaacgctgcgagtgataataacatcttcttcataatctttggttttatggtctgcaaccacagagccaaagactatgccaaaggaatgttaaaagttatgaactatttggttttcaatgcgtatagaggcatatattctacgttccacactcctgtttctacagttttgtggcagtatctttcggggcaaccctgtccaggaactcctgcaattgctccacacccagtctttttgccacaattttcttcttttcatccagtaagtataccattggtgtgctgtacacatcataaagcctgcggtaattcgtttccccctgcggatctgagccatgtatccagccattaagatgatgctcatggataaactgtagccattcctcacgggtaccttccgttttaacaccgatcatggccactcctttgctcttccagcttgcattccaggcagaatccaaacggggaatctctgttttgcaatgtccgcaggtgggatcccagaaaacaaggaccgtaaacttcgcgggggtcttatacagggaaagcggcctggcagcagtatctttatattgcaacggagcggcctggcggccaatcaggtttggcgccattgtgtatgccctgtccacaattttattgagttgctcatccgtcagccagaacgcttccccaggaacgtaatatttttccacaaggtgtacaaaaaccgcgtccatacccatgtaaggcgagctctcgtaattataagtaagccaccacaacacaaacttaaaaacctctttgcttttgcgggtacgggcaatcatggcatcacagtctacaataatagaatccggatgtaccggtaccagctgggtgaaatattttttcagctttccttccaaaataggcgttctaaccaggcggtcgctttccaggtccacctcatcccagtaatgatttttaaaataatgataggcaaataaagaatccgctccggctggtgctggcggaaccaccggttccttcatcgccaggaaaatggtgctgaggatattgccgggatgttgggcaataaagctggtcctgaattcctggatcttctttcccagttcctgctgcaatggctgcaccttggcagaatctgcggtcgtgcgggcagtttgcagctgttgctggatattgcggctcagcgtttcctgctggaaaagaaatttattgtaggccaggaacccctcgttatctgggctgcccttgtatactgttttattaacaagatcgctggtgtcgatggctacgctgaaaacctgctgcttatctatcagggtttctacatactgctgtttaccgggcagtaccagcagataaatgcctggcagcagtttttccttgcctttcagcacaacttctcccgcagggcttactgctgcagagtcggccaggtaggtagatctgcccatataatgggccaggaaaaacttcccgccggtaaagtttttcagcttcacagtaatctggtaaccctgcgcctgcaggctatattgcgctaaaagggctgctatcagcagtagaaatagtttacgcataatatttgaaagcaatatgtaaatgtaagcggaaaaaagtaaaaaaggaaagcggtgtgctgagtggtaattcgtatgaattacgatgcaggattcagcatttcaattacctttgcagccgtgaggaaaaaaaacgttgttttagaaaatgtaccggttactgcttatgcggcagaaggtaaagccctggcccgtcatgatgggaaagtgatatttattgaaggcggagtagtgcccggcgatgtggtggatgttcgtcttggtaaaaacaaaaaagactgggcagaagggaaagtagttcactttcacagctattctgataaaagagttactcctttttgccagcattttggcacctgcggaggatgtaaatggcaaatgctgccttattccctccaactggagtacaaacaacaacaggtggcagaccacctgcaacgcattgggaagttggccctgccgccaatggaccctatcctgggcagcgcccataccgaacattaccgcaataagctggagtttaccttcagcaacaaagcataccttaccaacgaggaaatcagggccaacgacggcgaaatacctgtaaggcccgcattgggctttcatgtacctaagctcttcgataaagtactgaatatagatacctgctatctgatgcaggagccggtaaacctgatccgcaacaccgtccgtgaatatgcggtttcccacgaccttacgttttatgacatccgtgcccaacagggatggctgcgtaacctggtgatccgcctttgcactaccggtgaaatcatggtgaacctggtgatccaccatgaagacaagcccaacaggattgccctgctggaccatttgctgaaaacagtaccggccattaccaccctgctttatactattaatccgaaaggaaacgataccatcttcgacctggaacccaaagtctattttggtaaaggatatgcagaagagaaactggaagattttgttttcaagataggtcctaaatcttttttccagaccaacacttaccagggagaggtgttatacaaggtaacaagggattttgcaggcttaaccggatccgagatcgtatatgacctatattgcggtaccggaagcattggcatctttgtatcgcgtaatgcccgcaaagtagtgggtattgagctgataaaggaagccatagacgacgcaaaggaaaacgccgcccgtaataatgtgaataatgccaccttttttgcaggcgatgtagtggatatttgcaataacgagttttttgcacaacatggccagccggatgtgatcattaccgatcccccacgggcaggcatgcacgaaaaactggtcaataaactgctggagatcggtgctcctaaaattgtatatgttagctgcaaccccgctacacaagccagggatctggcgttgctggattccctctatacagtggaaaaggtacaaccggtagatatgttcccgcacacccatcacatcgaaaatgtggtgttgttgaaaaaaagagataataactagcaacaatgaacgagtacaggcccggaaaatttcagtacctgccgatggtgatcaaaaatctgatgatcattaatggtttggtttggttagtgcagattacgctgctgagcaaattcgattatgatctgagtcgtttgtttgcccttcactactggggctccgaactattcaaaccacaccagttcattacccatctgttcctgcatgatccgaagaacattacgcatgtgctcttcaacatgtttacgctgtggatgtttggcgccaccctggaaaacctgtggggacccaagcgtttcctggttttctatctgatatgcggactgggcgctgcactgtgccacatgggcgtactcacttatgagaacctgagcctgaacaggtatgcagcgcagttcctgaatgatcccagtttctcgaattttgtgttgctggataataagttcgacatcggcaacctcgccaacttcgatatggccagcctgaaaaatgcattggccgcccgcgaccctgcagctatagaaatggccagcctgtatgtcaaaaattatgtaagctattaccgcaatggcgctacactgggcgcgtccggagcggtatacggtatcctgttcgcattcggatacctgttccccaaccggtacctctatttctttgcaatgatccccatcagggctaagtttgtggttggcttcatgatcctgggtgaactgtactccggtatccagaactcggcaggagataatgtggctcactttgcccacctcggtggcgcactctttgcctacctgctgctaaggaactggagtaaaaagagaacagatttttattaagacaactgtattattgacgtatttttgtattgaaaaatatttgtaccatgcatgcgttggaaaaagagaaattgccccgcctctctttaggagaaggaagaaatatggtgacacacctgatggtcgttaatcttacgattttcgttttcctgttttttacgcttgtaatataccagatggaacaagtgggcgagccccggtttcaccaggatattatgacctggctgaggcttccggcagatccgtccaaattactgacccgtccctggacgctggtcacttccctatttacacacatcagcttctggcagatcttttccaatatggtgtggctgtggtgctttggcaccttcatgcagcacctggcaggccaccagcggattttaccattatatctcttcggaggtctctgcggtaacctcttttacgtggctggtatgcagctgatcccgtcctttcatgcactcgcaggcaatgaatacaccctgggcgccgccggaagtatcatggcgattgccgtaggcgttaccgctattgctccgcgttaccgcatattccctttactggcaggaggtatttccctctggatcattacccttgttttcgttgtgctttctgttggcgcactaatggcgtcttccagctatggatacacctatatcccggtactcgccggcggcggactcgcaggctggttatatatgtaccagtggaaaaaaggcagggacttgggtgctggatttaacaaactggcctttaaacttacccacgtatttcacccggcatcacaacgcattaacccggacgattttaaaaggaagaattctcccacagatgctgatcagcaaccgtaccggcgcattggcaaagtaccagaacagaaactgaacgaaatcctcgataagatcaatgaaaacggattatcgtcgctttcagcagaagaacgggatactttattacgggcaagcaaaactgaataaaagtatgacggattaaaaatacctcgaaattgcttgttcccctatgctgaaaatcattgtacgccgtaccttgctctggagtaacatttgtggtgtagctgcgctgctcctcagcgttttccttcccggtgtcaacccgggccaatggtggcccgcgggcttctccggattcttttttccgtttctcttcctgctttgccttttatataccgccgtatgggcctggcgtaaaaaccggaaatacgggtggatgaatataatcgccataatctgtgccatgcccgcagcattaactacctggggcgttcatatcttccgggaaaatattatcagcaaacaaaccaacagcgggcaattcacactgatgacctataataccagcagtatgggtttagagagatatgtaacgaataaagacaaagaagcggcgatctataacaccattgcctccggcagcccggacattctttgcatgcaggaattttacaccaatgacaaaccgggtaatgaacagcatctgcaacgcattacatccaccgggaactatccatatcattatttcacccgcgacaaaacccactgggaaagctggcattacggcattgtattattttcccggtatcccattattactgcttcggccatcccctcagtagaaagcagcactggcagtggcagcacctttctccaggcagatattgccataaacggagataccatccgggtattcaatgttcacctcatttcgtatatgtttaagggtgaggactatgaaaacatgaaagccccgaaaggtactggcctggtttataaaatgcggcgcactttcccaacaagatcctcacaggcgctccagctggcagcactgattgccgcaagtccctatcctgctattgtttgcggcgatttcaacgacacccccgtttcgttcacctataaaaccatcagccgcaatttgcaggacgccttcctcaaaaccggcgccggctggggacgcacactctcctacctgtcgccttcactgcggatcgactacatcctggcacagcctgcggtaaacatccacggaagtaaggttttccataaccggccatcagagcatttcccggttatggcctgtctttcattgaaaaaaaactaactttagtacttcaacaaagtatgacgcggtgcgctttttaagactatttacgaaaggattttttctgatcatcaatttcgccgtggtattacttttcctggcagcctgtatggcgccgtatatatccccggcctggttctggcccatcagttttattacgctggccttcccgttcctgttggggctattggtgatattcctgatcgggtggctgttttttaattatcgttatacgttattgtcactgatcgccctgttgctcggctggaaatctatcagcgcctttgtggcctttaaaatgcccgccgggaataaggtagccaccaatggcaatacccttaccgtaatgagctataatgtaagccagtttggcctgtaccgcgaaagggacagtaaatacaaccggcaggccatgtttgccatgatcaaaaaacaagagctggatgttgcctgcttccaggatttttatacctccgaaaagaaaaacgactttaataaccgcgaggatatttcccgggaaatggaactgccataccgctacttttccagtgattttaaccgcgatggcatgcaacactggggatctatcatctattcccgctttcctattatagcatcggataaaatgaaaatgagcgatggcccgagaagtgaaagccttatctatgccgatattgtaaaagataaggataccctgcggatcattaatatgcacctggaatcttatcgcttcaacgaaaaagattattctgctatcaggaaaatcaaaaaccaggaagacacgggactaaaggccaccaaaagcattatccagaaaatgcgggaagcgtatatccgccgcagtcaacaagccgatattgtaggtaactttatccggcaaagcccataccctgtaatcgtttgcggcgactttaacgacaccccggcgtcgtatacctactttaccattaaaggcgatctccaggacgcttttctgcaaaaaggtttcggaattggccgtacttttacagggctggcgcctaccttacgtattgactatgtgtttgtcagtaaccattttaaggtaaacagcttccggaaaataaactctgacctgtctgaccattatcctgtaattgccaatcttagcctgataggtagcggaaaaacagcagtagaagtaaataaataactgtaatcgattatgaaaatgtataatatttttagggctgaccgatgttgttgcctgcttgtaccaggaaaacaatttttatctttgccatccatcaacaaaaaataagatgtcagctatatggcatctgtcatttacagcatatgtcagaactaaggatatataattcattacaccgtcagaaagaagtatttacacctttacaccccgggcacgttggtatgtacgtgtgcggtcctaccgtatccggcgaatcacatctcggccatgcccgcccctatattacgtttgatgtagtattccgctatttacaatacctgggatataaagtacgctatgtacgtaatattaccgacgccggccacttcgaagaagaaggccgcgcagcggaagataaaatttccaaatttgccatactggaaaagctggagccaatggaactggtacagaaatacaccaacctgtaccactgggccatgctgcagtttggcaacctcgaacccagcattgaacccaccgccaccgggcatatcattgaacagattgaaatgatcaaaacgatcatggaaaaaggctatgcgtatgaagtagacggcagcgtgtacttcgatgttaaaaaatacgccgccaactacgactatggcatcctcagcggccgcgtactggaagacatgctggaaaccaccagggaactggaaggccaggatgataaacataacaaagcagattttgcgctctggaaaaaagcgccgccggaacatcttatgcgctggccaagcccctggggcgaaggcttccctggatggcacattgagtgctctgccatgagcgccaaatacctgggcgcccagttcgacattcacggcggcggtatggacctccagtttccgcaccacgaatgcgaaattgcgcaaagtgaaattgcacacggcaatatgatggcccgttactggatgcacaataacatgatcaccatcaacggccgtaaaatgggtaaggcttatggcaacaccataaagctcaccgaaatgttcaccggtgaaagcccccagctggaaaagccatacagccccatgaccatccgcttttttgtgctgcaaacacattaccgcggtaccctggatttctctaacgaggccctgcaggccgccgaaaaaggacttcagcgtttatgggctgcttatgaaaccctgcagaaactgacgtatacccctgccaacggccaggccattaatgaagaactggataaacaggtacgtcagtggtgccaggaatgcccggatttcatgaacgatgatttcaataccgccaaagtgctcgccaacctgtttgagctcacaccagtgatcaactccctgaaaggcgggcaaataaaaatgcatgaaatcagcgaagatactttccggttgctgcagcaaacctggaaaacttatctcgtggatatcctcggtatacaacaggaagccatcaccggggaagataataaactggacggcgtattaaaaatgctgattgaaatgcggaaggaagctaaaagccgtaaggattacgctacctccgataaaatccgtaacgaattattgtctgtaggcattcagctgaaagatgaaaaagacggcaccgtatcttacagtcttcaataaaataaacattccggaagataatgcgtaaagctcttattacactgacagcgctggccttaacggccggcgcctgccagcagaatagtcagacaaccgataacaccaccgacagtaccggcgaaagcaaggtagctaaagtggatgtaccggtacccgttttccaggcagattctgcatatgcgtacaccgcacagcaggtaagtttcggccccaggatacccaatacgcccgcgcaggagaaatgtgccagctggctgatcagcagcctacgcaattgggcggattctgtgtacgtacagcgcactaccgttaccggtcccaaaaacgaaaaactgccctgcatcaatatcatcgccagcttcaaccccgccgccaggcagcgtgttttactgctggctcactgggatacccgtccctgggcagacgaagacgcctttgataaaacaaagaagctggacggtgccgatgatggcgccagtggcgttgccgtactaatggaagcagcccggcaattccgcaaacaaaaaccggaagccggcgtggatatcctgctggtagacgtggaagattacggcgctaaaaatgacgaaaactcattttgcttaggtacccagtactgggctaaaaacccgcatattcccggctataaggcgaactacggtatcctgctggacatggtaggcggccgtggcacccagttctatatggaaggctcctccaaacaatatgcaggcgcccagatgaaaatgttctgggatgtagccaataaactcggctattctgatatattccgctatgaaaataatggcgcatttatcacggacgaccatatcgcggtaaataccatcgctaacatcccaacattcgatatcattgcgttacagtcgaacaacgactttgctcctcactggcatacacaaaacgacaatatggatgtgattgacaagaaaacgctgcaggcagtcggacaaacactgttgcaagtaatctatacacagccgtttagttattaataaccggagggtccggggtgaagagtgatgtgacgtattaacgctaaaattagttttatgcccaggtccaaaagcaccccggaagccgttccggtacattatgtagcccatctcagcaaagataaaaagctgcagaaaattatcaatggccctctaacggagctggctatacgaaaaaacatctgcctgaaactgattggctccattatgagccagcagctgtccaccaaagtagcagacgtcatctattcccggttcctcgacctctacggccgccgggagccaacagcacagcagatactggataccccgccattaacccttcgtggtatcggtttatcgaatgccaaggtaacctacgtccaaaatgtggcagcgtttatcatcgccgaaaaactgaccgacagcaagcttaaaaagatggggaacgacgaagtgattgcctatctcacacaaatcaaaggcgttggccgttggacagtagaaatgctcctgatgttttacctgggccgcgaagatgtatttgccatggacgactggggattacagcaagcgatgattaaaatctacaagctgaaccgggaagacaaaaaagcattccgggagaagctggtcaaaatctctgaaaaatggtcgccttaccgcacacatgcctgtcgctacctttgggcatggaaagataatacacccgataaataactagacatatacagtgcgtagcacggttgtaaatttgtgttatgaatgtgcagggaagtttttttaatgatgaggatgccgggaagattgcattactgaatggagagctggcttaccatccgcagttttttaacctggcggaaagcaaccattttatgcaggtattgcaggaaaccatcacctggaaacaggaatccatgaaaatgtacggcaaagaggtgttattcccacgtttaatggcctggtatggcgacactgccagctcctacaagttctccgggaacaccttctccccccaagcatggacagcagaattacaacagatacgcgatcgcataacgccagtgagtggccaacagttcaacagcgtattgctcaacctctaccgcaacggcaacgactctatgggctggcatgcagatgatgaaccggaattgggccatcacccggtaattgcctcggtgaactttggcgcagcccgccgctttcagctgcgctataaaagtgatcaccaacggaagtatgaattattattgcaacacggttccctgctcatcatgaaaggaccattacagcaatactgggaacaccaggtcccgaaaaccactaaagtatcaaacggaagaattaacctcaccttccggtttatccacccctaaaagatggcatgtactatgaaaaaccttgtattattaatcggaaatgacatcaacaacatctcacgcggccaaagctggaaagacctgctgcaggacatcatcaccttctgccacgccggcgattgcgtggaactggatgataaaaaaccttttccgctcctgtatgaagaaatctttctaaccgccagtaaaaatcaccgtatcagagaaaaagatctcaagtctttcatcgccatcaaagcagcggaaataaaggccaacccgctgcacagcgctatccgcgaactgaagccggcacatatcctgaccaccaactatgaattcacgctggaagggcaaataccattagaaaacaccagcgtcatcaaggaaaagttttacagtattttcaggagatatgaagtagataatatccattactggcatattcacggcgattgcctcaaccccatgagcataaatctggggtttgaacactatggcggccagttacaactgatgcgcaattacgtggtaagcggcaccgtgtactcttccaaagaagtacccaagccctccctgctccggcgcattcactcccgggaagtatattttcactcctggatagatctttttttcacagaagatatacacatcttcggactgtcgctcgactttgtggaaactgatctctggtggctgctcacctacagggcacggcaaaagtttcatcataaaaatgtgccggttcccaatcacatcttctactatatcccggaagaatatgtggcaacctctaaattcaaactggacctgctcaccgcaaatgatgtgaccattgtaagcctgcccggtaaagataaactgggatattacgaatctatcatcaaacaaatcgggaagacccgtcaaacggtccaccatagcagcaccaggtaataccagggcctgaaagtgagactggcagcgtttttgcaaaatacagtacaatccttcaaaagagacaacctcatgactccttttgttgttaactattaaaatctatattttatgttattggaattagcaatcactcttgccaccacctttatggccccggtacaaagcaaacaatcaccccccaaaacgcaggtcatctatgtaaaagaatcaaaggaaccctgtaccggcgtggctcccatggaatgtttgcagataaaaggagtaaatgatacagactggtcaaacttatataccaatatcagcggctttaaatatacccctggctaccgttataagcttagggtaaaaattacccgggtaaagaacccaccggcagatggctcttccctgaaatataccctcgccaaagtgctggaaaaaaagaagatcggcaataccggttcaacgcctatcaccggaaagaaatgggtattggtaaaaatggatcatgaagccatttccgatggcgccatctggatggaattcgacggcagtcagaaacgcatgcacggtaaaagtggctgcaacagtatgatgggtgcatataccacctccggcagcgatcttaccttttccaaaacagccggcaccctgatggcctgccccgacagggatgtaatgcgccgcgaaacctccttcatgaaacaaataggcgatcaaacatttcaatacgccgtagccggtcaaacgctgaacctcctccaaaatggcaatatcgtattgcaattccgcctggaaaataaagacggcaatgcttccggcaacaacaactgggcagctatcggcaataaaaaatggaccctgaaaatgatcaatgaaggagtaatcagcaactccggtgtgtggctgcagtttgatgaagataaaaaacgcttcagcggcaaaggaggctgtaacaatatttccggtgggtataccgccgttaaaaataaaatcaccttcacacaagccgtgagcacccgcatgatgtgcggcgatgcagatgtaatgcgccgggaatcagaattcctgaaacaactcggcggacatacctttacctacaccgtaaacggtgaaactgttgacctctatgaaagtggcaaattagtgatgcagttcacactggaaggtaatgacaacgatcagcaaggcaacgcctcaagcaacacccagtgggctttcattggcgcaaaaaaatggagcgtgatcaaactgaacgatgccacactgaccaactcaggtatctggctggaatttgataccaatcaaaaacgcttccacggcaaaggcggatgtaacagcatttccggcggatacagcgccggcggcaacgaaataaagttcacacaagccatcagtacccgcatggcctgcaccgatgctgaagtaatgcgccgcgaagctgaattcctgaaacttatcagcggtaacaccttccgatatgatgtggccgaacagactttaaacctgtataaagacgggaaaattgtagtgatgtttggcatgcaggataaaacactgtaaatcatttacaggtaaaaaatattaaaaaagcagcaagggttcttgctgcttttttatgtctaatccctccggttaaaaataatgcttgtctcaccactgcatatagcctgttgggctttcccctgcaaacgccctgaactcgcgggtaagatgtgcatgatcataaaagccgtggtccagcgccagcgataataagtggggattagacaatgttttcaactgctgttttaaactcagaaacctgacaatgcgtgtgaacattttcggagatacgccggctgtttgcaaaaagtgccgttcaaaattacgcgggctcatgaacgcctgtgcggccaaagtatttattgctatatcacctttcgtttgcctgatcagtgtaatactatgttgtattttttcagagatgatgtttcggcctggcaaccgctgtaagagaaacgcttccaggcactttattttttctgctatcccggaggacttcagcagcagaggctccagcgcaacatgccatccggaggaaatgtcccgcaggggaacatgatcatctgtaatcaattgcaaaggcaacccggtaaaaccactcaggccgcccggtttgaaacggattcctaacaaataggtattggcatgaagagtcgtatcgcagaaggtagtcatagtacctgttacaaaagcgttacctggcattattttcagcgccccaccacctgctgcaataacatcttcgctaatattaaaaataatatccgcacaggtatccggtaatattcgttgtagcataaaatgcggaccgccgcctgcccagtaggcatctacaaacgtggctaatagtggatgtggccggaactctttatacatagcctgcaaattaaaacattattacgaatgagggttttatacacagctccgccaatggaagaaaatcttcgcattactatctgcgtataaaaccaccatccgtaattttaattcatcacgcttacttcgctgctaccagcttgggatgatatgcaaacaacatcgcgttggatacattatctcctactgcaacaaccacaggcactgtagaagcggcctgcgctggtacctgtaccaggagggtgttaccatctgcacgcagaatctgcgcaggtacgttaccaaagttcactttgtttccgtgtttatcttcactaaaaccgtgtcctttgatgaggaggaaatttcctgcacgtccttctacagttactacttcagcggtattttctgttgaattcggggaacaagccatcatggccgtaattgacagcataagggctgtcacaaacaatttaaaatgtgtcatcttatttttcttctttttggggggtcacaaccctgttacaaataattcaccggggttaacactattgcaattgcaactcttatcggcaacagtatatattcggtattcaaacggacgcaaaggtacaatcattccttcaataaaaaaacaattcatcaaaaaaatgcgtagaattacggatacgggtatatgattttgtgactaatgcagaaagtcccgtaccggtaattccggtacgggactttctgatcaaacgcttaccagccggttatttcgccagcttcagctcattgataatattttttgcaccacccagtttgtcgatgcaccacaatacataacgtacatccacacagatagtacgattgtattcagaatcaaactgaattttatggctcagcgcttcgtagttgccatcgaaagccagaccaatcagttcaccattggcgttgataacaggagaaccggagttgccgccggtgatatcgttagtagtaataaaacccactacaatatcattgcgtttagcatctttatactgaccgaaatcttttttgttatacaggtctacgtaattttcaggcaggtcaaactcgtaatcaccaggcacatacttttctatcacacctttcatagtagttacgtagtcgtagtgtactgcatcccgcggagcgtatgattttacctggccataagataagcgcatggtaaagttggcatcaggatacctgttggcgttaggattcatctgcatcacccctttcagataggcacggcccagatcattatttttagtattgaactggttgtatatcggtagatacttacctacataatttttgaggaatgtgctggcataggcgaataccgggtcattctgcagggttaccgcatcggggttcgctacgaatgcgttccatttggcatcatcaaaaataaaggtgttggccattaacgaagccgcccaggtattgtaagttttgtcttcatcaagcggaccgtattttgctttcagcgcatcataaaaaccaatgggctgttgatctttggcgatgtctgtatagaacatacgacaggtagcagccaggattttctggtcgcttggtttgttttcgctttccaggaatcctttgcgcgctttatctgctgcctctacagcctgtttaaccgcatctttgggagcgcctggtgttaccagtgctttttccacgcccgttaaagacgctgcaaaagcagctaccggcgagcccaggataccttcattcaggtaagtgcgttgtttggcgtaaggagtccaggctttgtaggctgcctcgtaatcggaaagtatattggcaaattcaggtttgccttgtgcccatgtggcaaaagcagcttcctgtttttgtttatcggccaatacaccatgtttctgcagttgcttggtttcgccgtcaaaaaatttccagtagttggcgatgccggcgtaggaagaagccagctgcaattttactgcaggatctttcttcatctgctcaaacatggccttcagccttacatcgcggagatttaccacggaaggattttcgatagttgttttcagttgtataccataagaagtttcgtaacggttagtaccacccgggtaaccgaagatcatggcataatcattttcctttacacccttgatagatacggggaggaaatgcttaggctttagaggcacattatcagctgcataagaagcaggcttaccatctttgccggtatatacacggaatacggagaagtcgccggtgtgacggggccattcccagttgtcggtatcgccgccaaatttacccacgctttcgggaggggtacctaccaggcggatatctttatagcgttcgtatacaaacatcaggtattgattgcctttgaacataggcaccaccttcgcttcataaccggtattggcaatggttttagagataatttcaccgtatacctgttgttctttctgggctcttgcggcgccatcaagtcctttcagggcttcttccacctgcttgctcacatcttccactcttaccaggaattgtacagacaactgggcagaagcaatttcttcctgtttattttttgcgtagaaaccgttcttcaggtagttgtgttctacagaactggctgcagcaatagcgccgtagccgcagtggtggttcgtaaaaatgagaccttcattacttacaatttcaccggtacaaccaccaccaaaaataacgatggcgtctttcagggatgctttattaatactgtacaactgttctttcgtcagcttcaggcctttcttcaccatgtcgttgtacgtttgctgccccagtaaataaggcaaccacatgccctcatctgctttagcccatttgatacttacgctaagcaataagagcaaaaccagtaatttttttctcatattaagtcaggttttgttttttaaggacctcaaacctagctaatttttcgttaccgggcgcaggtataaggaccaacggcagcaaacatctgataaatataaaaatatgatcagggtctaaacaaaaaaactggaatatgttttgataaaggggtacggccggaaggctgtgccagtatttaaaaatcacaaaaaaaatcgtcggaacatgaaaaaggtattcttactggcgggcattgccgctctatttgcctgtaacgagagtagcactcagcaggaaaagaaagaagaaataaaagaagatattaaagaagccgggcaggaaataaaatctgccgccagcagtacaggcgattatttatctgagcaaaagaaacaggcggaagaagctattcaggagcgtatcaaagaaatagaccaaaccacccaggaattaaaaaaggacggggacgagaaaagcgtggctgcccgtaaaaagctggaaacactgaaagcacagatgaataaaaagctggacgacgtaaaaaacagcagcgccgacaaatgggacagcacccgggaagccgccgaccaactgatgaaaaaatccgataaagagtggaccgatttcaaacaggactttaaagatctctttaaaaaagattaaaagaaggtggccggattacttcaaaaatccacaatccttgttccttgaacattaatcttgtaattttacccggcttaatagatttcaatttgctactgtcttactatcaggaattactaacagaagccggctgtgatgaagccggaaggggatgcctggcgggtccggtgtttgccgcagccgttatcctgccgaagaaattcagacacccgttgctgaacgattccaagcagatgaaacagtccgaccgggaaaaactgagaaaggtgattgaaaaaaaagcagtatgttatgccgtggcaagtgtggataatgtagaaatagacaagataaatatactgaaagcttctttcaaagccatgcacctggcattggagaagttacagcagcaacctgaatttatactggtagatggtaaccgcttttatgcatacggcaatacgccacacgcctgtattatacagggcgatggcttatacgcctccattgcagcagcttccgttctggccaaaacctatcgtgatgaatatatgcagcagttacatgctacatatccacactttgggtggaatgagaacaaaggataccctaccaggcaacaccgggatgccatccgggaatttggcgatacgccatttcaccgcaaaacattccgtttgctgccggagcagctggaactggatttatagcttttagccgttaacgggttatctaaaagctaaatgctgacagcgatagctctgttaaccttatacttattaattttgccctgacagggaataattatgttaaagcagacacaacagcagaaattattacagaaactttctccccagcaaattcagctcatgaaattgctgcaggtccctactgtgaacctggaagaaaggatcaaagaagaactggaagaaaatccggcgctggaatatggcgaagaagcaggagaagacgagttcaaagaacaggaagagtatgaagctcccgcagaagaagatgaatttgagcccgatggcagtgaaaatgaatacgacaatatcgatatttctgaatatgtaagtgaaggagatgatgatgtggcggattacaaactgcgtgacgataactatcctgatccggacgaaagcaataaaaccatcccgatccgggtggaaacgtcttttcatgaacacttattgagccagctgggtatgctcgagctggacgaccaccagaatgccattgccgaacatatcatcggcagtatcgacgacgacggctacctgcgcagggaaatcagttccatggtggatgatctctccttttcacagaatattgacaccaccgaagaagaaatcaattccctgatcaaaaagatccaggactttgatccggctggcgtatgcgccaccgatctgaaagaatgcctcctgctccagctgaaacgtaagccacaggacgatcccggcgtgcacaacgcctactccatcctcgaaaactacttcgacgaatttaccaagaagcactacgagaagatccagaaggcattaggcctttccgacgaaggactgaaagaagccatcacccagatcatcaagctcactcccaagccaggcggcaatttcgccacgctgaataaagcagaaagctacgtactgcccgacttctttattttaaacaacgccggtaaactggaacttacgctgaattcacgtaacgctcccgatctgcggatttccggtggttaccgcgaaatgctgaaggagtatgaccggggcgataaaaaagataagcgccagaaagaagccgtattgtttatcaaacagaaaatagatgccgccaaatggtttatagacgccatcaagcagcggcaacatactttgctgtctaccatggaatccatcatggattaccagcgcgaatttttccttacgggagatgaaaccaccatgaagcctatgatcctgaaagatatcgcggatcgcacgcaactggatatttctaccgtaagccgcgtggccaacagcaaatacgtacaaaccgagttcggtaccttcaaactgaaattcttcttctccgaatccctgtctaccgacagcggcgaggaagtatccacccgggaagtaaagaagatcctgtcagacctcattgaggcggaaaacaaacgtaaaccactcagtgatgaaaacctcacgaagatgctgcaggataaaggatataacattgcccgccgtacggtggccaaatacagggagcagctgaatattccggtagcccgtttacgtaaagaattataagaaccataccatgcaagaacaagctgttttagacaggaacggaaatatacgtttggagccggagtttccaaaggcaatgaaatccctggctttaatcatttcctatctctcacatccgctgttcattcccctgctggtaacattcctggtactggaatccattccggaatatatggtcgcctttaaaccattgagcaaaaggttcgccttcgatatgctgtatttcagggtggctattatcagtatcgggttcccggtgctcacgcttttactggccaaggcgctgaaatttgtttcttccgttcatatgaaaacccagcgcgacaggatcattccttatgtagcgatgatcacttattacttctgggcattttatacttttcaacaggaaggccgggcgccaaaattctataccgcgtttttcctgggcgtgttcctgagtgtttctatcgcttttgttaccaataattttataaaaaccagcatgcataccgtaggctggggcggcataatcggccttttattgtcgctgatgtggggaatgcatatgaatgtatccattccactggtcattactttttttgtggccggcattgtagctacctcccgcctggtgctgggagcacatgaaccacgtgaaatctacatcggtttcctgattggtattgtttcgcagctggcagcgtgctggatcctcgtaaaataggtatttcaccattctatccctgctcccctgccggtaaatgctgaaacaagtcagcccaccagccagggatcagggagaacaacatttagaacggcgataaaaatttttggggtttaaccttgaccacttcaccatttcatcttcacatggatgcaaggccgcaaggcaggctaacaaacaattttaacaaacagtaggggattaacttcaacaactaaacttgacagtacaaaagtgaaactttctgcgctgatactcaagcgtataactacgctttttaaaaatgcagtagaattctcacttccgccggctaactatttttttgaggttttgttgttacgcacattcaatgcgtaatgggttcgcatctttgttatgccattaggggttaaccctttaaggttttaagaataaaattttaacaggaagttcttgaacagcacggaaaaggattactactttatttagcatttaaaagaaaatgctaaaatatttaggaaaataaaaaattagatcataacttagcagtccaattaatttgctttctaattgtgatcagctatctattaaatttgtaaaaacattacttatatgtctacagccaatgcagaaaaactgaaggccctgcgcctcacaatggacaagattgagaaagatttcgggaagggatctgtgatgatgatgggagaaaaagcagaagcgccgatggagatcatttccacgggttccctgggccttgatatcgcacttggaattggcggtttacccaaaggaagaatcatagaaatatatggtcctgaatcttccggtaaaacaaccgtcgccatccatacaatcgctgaagcacagaaaaaaggcggcatttgcgccattatagatgcggagcatgcttttgacagcagctacgccagaagactgggagttgacgtggattccctgttaatttcacagccggatcacggtgagcaggcgctggaaatagcagatcgcctgatcctctccggcgcagtagatgtagtagtaattgactccgttgctgccctggtaccgaaaagtgaactggaaggtgaaatgggtgaaagcaaaatgggattacaagcccgtttgatgtcacaggcactgcgtaaattaaccgccactatctccaaaacaaactgctgctgcatctttattaaccagctgcgtgaaaagataggtgttatgttcggtaaccctgaaactaccaccggtggtaatgcgctgaagttctacgcatccgtaaggctggatatccgccgcatgagccagattaaagatggtgacgaagcaatcggtaaccgcgtgaaagtgaaagtggtaaagaataaggtagcgcctccgttccgtcaggcagaattcgatatcgtttacggtcagggtatctccaaaacaggagaaatcatcgacatgggtgttgaatatggcgttgttcagaaaagtggtagctggttcagctatgataccaataaattaggccagggccgtgatgcagtgaaacaactgctgaatgataaccctgaactggcagcagaaatcgaagccaagattaaagtgaagattcaggaaaagcaggatgccgcttaatattgtctgctattgaattgaataagcattgaattgaaacttagtattaaacatacatagaagttagttttagttttagtaagcattgggttagtatgcacatccctgccttatcctgggcggggatttttttgcccgggagtgaagtctcccctctacttccctccaaaacaaaagccgcccctaaacggagcggctttgttttttttcactattatcttacaaacaaaagcaattaagcttctgctttcatgctcttagctgatctcttacgctcttcttcatccagtattactttacgcatacggataaagttaggagtaacttctatacactcgtcatgctggatgtactccatacattcttccagtgtcatcagtatcttaggcgcaatgttagcagcgccatcggttccgctcgcacgcatgttggtcagtttcttaccttcatttggattcaccaccaggtcacctggtttgttggtttcaccaatgatcatacccttgtatacttcttctcccggatcaacgaagaaagatcctctatcctgcagtttgtccagagaataaccggtagtagtaccagcttctttggcaatcagcacaccgttgttacggcctgggatagcacctttccatggtttgtaatcattgaaacggtgcgccatcactgcttcacctgcagtagcagtaagcatctgtgtacgcaaaccaatcaaaccacgggaaggaatttcaaattccaggtgttgcatttcacccttggtttccatgattagcatctcacctttacgacgggttaccagatcaattaccttgctggcaaaatcctgcggaacgtctaccaccagggtttcgtacggctcgcattttttaccatccacatgcttcacaattacctgaggctgaccaacggtcaactcataaccttcacgacgcatggtttcaattaatacccctaagtgcagaataccacgaccataaaccatgaagctatcagcactgtcagaatccattacacgcagtgccaggttcttttcagtttccttcatcaaacggtcacgcaggtgacgggaagtaacaaacttaccatctttaccaaagaacggagagttgttaataccaaacaacatgttcatggtaggctcatccacactgataattggcaacgcttccggctcttcagcatcagcgatagtatcaccaatgttaaaaccttcaataccaactaccgcgcaaatatcgccggcatataccttagttacctttctcttacctaacgcttcgaagatatacaactcacgcactttctgcttcttgctggtaccatctgtctgcatcaaagtaacccactgtccttcttcgatagaagcacgggccaccttacctacagcaatacgaccaaggaaagaagagtaatccaatgaagtgatctgcatctgcaggttaccttctggagtggttggctccggaacgtactggaggataccatccatcaatggagaaatatcttcactctgttctaatgaactgttaaaccagccatttttaccagagccataaaatgtcgggaagttcaattgatcctctgttgcatccagattaaagaacaattcaaaaactgcatcatgtacttcatcaggacgacagttagccttatctaccttgttgattacaacaataggtttcagattcagctgcaaagccttctgcaacacaaaacgggtttgtggcatcggaccttcaaaagcatccaccaacaggataacaccatcagccattttcaataccctttccacctcaccgccaaagtcggcgtggcctggagtatcaatcacattgatcttggttcccttatattcaatagatgcgttcttgctgaatatggtgataccacgctctctttcaagatcgttactatccatgatcagatctcctgattcctgattagcccggaatacattagcctgatgaaggattttgtcaaccaaagtagttttaccatggtctacgtgtgcaataattgcgatattacgaatgttcatatacttaaatctttagctatcagccattaactaaatttacgctaatagctacaaaaagaaggcgcaaaggtacgaaaacatagcgagaatgaaggtgtcacgttttaaataaatgtaatcatttggtcagcccggaaaacgcccttgcaataggttggttatcattgatttacaattaattatatccaaatattgtaaacaaatagttttatggcgtcaattttgccccaccccacagcgttttaaccgcttaataccgctcgcatgaaaaagaaactatatctcctcgccatcgcctgcctctccctcatcacctcccgcatatacgcacaaataccagcccaggatattaacctctctgaatataaatacccgttcccggtacatttcctgaaactgcaaatacaagggcaagcccttcaaatggcctacatggacgttcaaccctcccgtccaaacggtaaaacaattgtactcctccatggcaaaaatttctgcggcgcctactgggatagcaccgcagcagacctcagcaataacggctaccgggttatcatcccggaccagatcggctttggcaagtcatccaaaccccaacacctccaatacagctttcaacaactggcgcaaaacaccaaaacactgctcgactcgctgcaaataaccaaaacagccgtgctcggtcattcaatgggaggcatgctcgccaccaggttcgcattgatgtacccggaggtgaccgaaaaactgatcctcgaaaatcccatcgggctggaagactggaaagtgaaagtgccctatcagtcagtagataaatggtataaagcagaactgcaacagaactatgagaagatcaaacaatatatgatggacagctactacgccggcaaatggtcgcccgcctacgataaatgggcgcagctccaagccagctggaccagcagccccgactactccctggtagcctggaactccgccctcacctacgacatgatctttacccaacccgtgctgtacgagttccagaatattaccgtccccaccctccttattatcgggcaacgcgaccgtaccgccttaggaaaagccaacgttccggaagaagtgcgaaaaacaatggggaattatcctgaactgggaaacgctgccgcgaaaaaaattccacacgccacgctggtacctatcgaaggtgtaggacatcttccccacattgaagcctatacgaaatttattgcgcccctgctgaagttcctgaaagaataaccctattcctccagcagctttacgacatactccaacgcactctgattcgcaggattgtccagcgcatgcgcaatatccagcttttcccgggaggtaagatgccaggataaagccgccgccttgtcctgcttctgcggcacatactggaaaattacccggtgaaatttatccgggaaatatccttccatataattcagtaaatcatcctggtcaaaatcctgcatggcgctccagtgctgctgcatggtaaacaacggctcaaacaacaggtcgctcagatccttcgtttttttgatcggggaaatgtcattcttgcgggtatcgcggatctggatatatatcaccccgctggtattttcattgatccatttattaaacgtatataaatatcgcaacgtggtttgctgaccaaaattatcgcggataccggcgtccatcacatccacaataggattgctgggaaggaacgcattaggcagtacataaggaaacgtagcacacatacggatcgcgctggttactcgcaggtccatcgcatcctgtgccgcaaagtattgtccgaaatccaccccgtcgatatccctcacctgccgtgtaggatactggtactgcgggctgcataagtaactgactggctgcggggaaatcattaaccggcgcccgtctgcattaatagtagcattccatatcagcatgggaatgtctgcatgggcttccggctcccggtagtctttcagcgttttatccaacacactgtcagtatgctcattcagctgcatttcaaatgcataacccctatcctttgcgtaatgatttttcccgatactgaaacttctccacggtgtaataaaatcattcacggccatagcagaaaatacagaattgagtaagtcctgtgataccttctctgcatatatattatcagacaggcggataggtttcccctgctgctgttcgtaatacaactcccggaaataactggcccccagcatacccccggaggcgccggtcatcagcaccgtgtgcttcatcagccggccctgcagcatactgtccagtcgctgtaatacgtttacgctccaggtggctgaacggctgccgccgccgctgaaattcattacaattagcgggggcttttttcccgccgggaacttctttctccagttctctaatatcagcagggtttgtttcttatccgcttcgtatcgctcccgggtaaaaaattgttgcagggccgccacactgtattccggacgggccttcttctcccggtaattcaacccgtaagccttattacggttatccacccagttatgttccaccatccagttcaaaccaaacaacatcaccagcaatatgggaatagaccaggtttgcagcatataggaaaaggcgcccgccaccccgatgagaaacgcaaaaaagatgagcacactggcgcccgcaggaattctgaacacatcataatccatcatgtaagccagtatcaccaggaaaaccagcgagcaccctacggtaatcatcgcagcaaagtgatgctgcttgaggatactgtcgaggtaatgcttattgtagtgatccacattcctcgcccttctgatacgccagggcgtagagaaataattatgtaccggcagcgcattttcatctggatcctggttgggtttcaggatcatccgcaggaagtttcgcggattaccgaaacgcttttccaggcgtctgccaatatttttatctgcattaaaaaaatagaaaaaacagaagaagaatataaacaacactccgcagataaacccttcccccagcaacatgatatccggaacggtattgagctgttcataccgctggtattcccatccgcggtaaagcatactgaaaataaataccagcggtatgatggcattattaaggcaatacctgaaaaatggctgcgaagtggtggccaggaacttaaaccggccggtatgcaatataaaggtggtaatctgccagctcataataaacatgccggtggctagtcccaggatagtagtactgtagaaatttactttgcccaggtattccggcgccaggtaaagtgcatctccaccaaacaccttggcaaaaccaccgttgatggtgctgaacaggatcacccaaaaaataagtaatacctggtacttcctgaaatgcaggagcagcaactgtatagggaaagaatagtaagtttttatcagtaataacttcaccttcatcagacgattattacgaataaacctacggaaaatttacggatttatgacggcgggaatttacaccgggcggaaaatcaattcccgcttctcacgccccggctgaggaacagggtccagatcagcgacagcatcagcaacatccccacaccctggtgtaaaattccataactgatgggaatcttcacctggctgtttaacagggtcagcacgcccagcagcacctgcagcaataccaacagcaatggcaggtaacggatggtgtgtaacaggctgttagccggtgtttgtgcagctttccaccaccagatggcgatgagaatagtaatcaggtaggccagtccgcggtgaatgaattgaatggtaatcgggttatgcgcaatatctgtagcgaatccgccttgcgaaaacatgccggcaggtacccaggagccattgatgtccggccaggtatttgccaccaatgccgtatgcaatccggccatgaaagcaccgtacaccaactgcactaccagtaataccagcaaccagatattcagtttgtataaagccggaacttttaatatttctattggatgcacactcagcttcaacgcaaaccagaacacatatgccagcaacgccagcgcagatataaagtgaatggccaaacggatatggttaacatacaaattttcctcattcaggccgctcttcaccatgatccatcctatcaagccctgcaaaccacctaacacaaacaggatgatcatcgggtttatcatgctcttgttaatcttcttcttaataacaaagtagataaacggaataataaacacaaaccccatcagcctcgcccaatcgcgatgcagccactcccagaagaaaataaacttaaaatccgacaaggtaaagtggctattaatatacttatactgcgctatttgtttatagccatcaaatgctttctgccaggccgcttcattcatcggcggaaaagcgcccaataacggctgccattcagtaatggacaggcccgagccggttaaacgggtgatccctcccagcaatacctgaactatcaacatgcccacgcctatatataaccagatggccacggggcggttattttttattgtaactgcttccataaacggtgcaaaaatagggaatgaatgcctaacaagccggttaaatactcacattattttaacaaaggcgtaatgttctgttaatccgcaggtcggagctttgcattgaaaatttaaacggcaccattgtattagctaataccgccctaattaaaaaaagacgaacacattaaaaaaataatgtcatgaaacatttacgttttgttgttttagcacccaaagtagctttgttggtatttgttactatcctatctccgattttacatgctgcggcacagtcaaaaacatttgcttacaatgcagcacgactggcaaaggaaaaacctgtacgggaaactcccatcgaagctttcaacgtacatatcacgcaattgcaaaaggaccagctgttattccagctttctgtggataatccttccaacgaaaagctgacgctctacataaaagacaatttcaataacacgctgcaccgcgaaacattgcctgctaccctgcgcttcgaagcacgttacaacctcggttctcttgaggatggagactacaccttcgaaatcagaagcggaaaaaacaaactggcagaaaaagctattgccataaaaacgcagaccatgatcaacaggagcgtttccgtatcagagtagtcccacatcgcataattgaaaaatgaaaagaggtggtatccgtaaaacggtaccacctcttcttttattatttcctatctcctatttacgtactgattcatacacggcctcaaacattctttcccgggtatgcagcgccgttattttcgtgttaacgccgccgttaggatacaccctgttgctcaggaaaataaataccagccccgatgttggatccgcccacacacacgtccccgtataaccggtatgcccgaaggtagccgcagaagcactcctggcagggtacggttcccgccgggtagcattgtctttttccggcttatcaaacccaagaccacggcggctgatatggctgttatacgccgtaaacaactgcaccgtttccggcttaatatactgcacgccattgaaagatcctttgttcagtaacatctgcatgattaccgccacatcatgcgcatcagaaaataatccggcatgaccagccaccccaccaaacatagctgctcccggatcgtgcacatctccccgcaataactgcatgcggaaagaatactcacgctccgtaggaacaatctccgtcaaaggaaaacgcgttctcggcaaaaagcccgtggtcgccaatcccatcggaacgtaaaaagtttcactcacatattcgttcaacttcttacccgttaactgctccacaattttccccaggaaaataaaatcacagtcgctgtaaacatacccctgccgcggcgataacttactatccagtatccgctgccacatggtatctacatagctgttttccatgtacatctcatccgccacgcggatgccgtgggtagcgtccgggctggcgtgatagagcaccgtatcgggctgcgcattgttataaagggtttctttataaaacggtataaaggctaccagtcctgcctggtgcaaaagaatatcgcggatgcgcaatcctgctttatctgtacccaacacctgcggcaggtatacgcccagcgtagcatccaggttcagtttcccttcatcatataaccgcatcaccgataaagtggtagcgcatactttggtcacagatgccaggtcataaatagaagtgggcgttaccggttcctgtttgttgtattcgtagtggccgaagcagcggttataaataatcttcccgtccttcagggctaatacctgcgctcctggcgcggcgccgcgggcaatcatatcgttggccaaaccatcgatctgcagcaatgcctgctcattgatgccggcttccagcgcagtagcggtaggcaataaattaaacttgttcacttcataagtgatgccggtgccggaaggcaaatccgggcatacggttaccggtagttttccggatgggcccagctgcccgaaaagcaggtcggcagcggctctctgggtggtgctgtcatcttcatacgccgccaccaggtgaggcgcgtcgcagaaatactggattgcatacgggttaccaaaaacaaccgtcaccgaaggcatttccgattggagctggcggataatcagtcgctctgccatcgacaacccgaagtttccggcgggccggcggctgtagtcatgtaaactgataataaccgccttatagtcgcgctgtatgcgggatacaataggagcaatctgttgtacggactgccgcgaggtgaaaataaacgcatccgtaccgggtttgtaattcttcaccgattccacgaaagtgttgctggcatcagctcctacggcaattaccgccagcttttgctgggtcatggccggtgaaaaaggcaccagtttcttatcgttgcgtaccagggtgatggctttctccgcaatacgtttacgtaaagtatctgttttggcgttgatgtcttctgccagatgatcagtatcgatgtgctgcggctgccctagtccgaggttatatttggcgcgcaatacttttttcacgcgtccgtctacttcttcctggctgattttaccggctttgatagccttcttaatagcctccacgctgccttctgcggtggatggaagaatcatcaggtcgttgccggcaagcagcgactgtagggattcctgtccgttggtatagaattttgcgatgcctttcatttcaagtgcatcagtaacgatcagtcctttaaaccccatttcattcttcagcagtttagtaacggcattataagaaatagaggttggtgtatttggttttttatcgatagaaggaatataaagatggccaatcattacagattgcacgccggcagcaatagcttcgcggaaaggatacaactccagggaatcgagctgcgctcttgttttattgatggtgggcaggtccaggtgtgaatctacattggtatcgccatggccggggaagtgtttggcgcaggccataatgccggcatcctgcatccccctgatggtagctactcccatgcgggctacctggtatttattttctccaaaggaacggtcgttgatcaccgggttggaaggattattattcacgtccatgtcgggcgcaaaatcaatatgaatacccaggcgacggcattgttctcccatgagctttccggcatcatacgccagggtggtatcctgcatagcgcctatcatcatgttccgcggtaatgaaataacactgtcgaggcgcatgccaagcccccattcgccgtcaatggctaccagcaagggtacttttgaaatagactggtagtagttagtgagattggcctgccgcaccgggccgccctggaaaaaaatgacgcctcctactttgttatcctgtatatctttaacgacggcattaatatgatcctgcccgagattggaatgcgcgcggatcatgatcagctgggcgatacgttcttcgggggtgagcgattgaaacacactatctgcccattgtgaggctttgtcctgctgtggcgccaccttttgtgtagtcacttttttatgcctcttcttttccttaaataccaggggcgcagaaatggcgctgcctgtcatcattaggcctgtaagtcctgcaaccaataattgtttcctcatatcataaacttacaaatattcatgcggaaatccagcccgacagccctgaatatcaaagaattactaataataatcatatgattttgtcagatccaaactatttcattaaattagaataccctgttgaagatattttatggattctggtaaaaaattgaaatgtgttcactattttgtcagaatatttacatttagtttaatcaatcgtaattttaattaccaatacattcatctgtttcttatatttgcaaccttgcgagtaaagtagattttaataaaacatggtcaatctcattttatttggccctcccggtagcggcaagggtacacaaagtgctaacattatccagaaatacggacttattcatctttccacgggcgatttgcttcgcagcgagatcggtgataaaacacccctgggactggaagccaaaaagtttatggatcagggccagctggtaccggatgaagtggtgattggcatgatcagctctaagctggacgctaatcctgatacacgtggtttcattttcgacggctttccccgtaccactgcgcaggcagaggctctggataaactgctcgcattgaaaaaaacgtctatctcaaccgttctctcactggaagtaccggaagatgcgctcataaaacgcctgctgaaccgtggattaacctccggccgcagcgatgatgcctctgaagatgtagtgaaagcgcgtatcgtggaatatcataataaaacggctcctgtggctgatcactatgccaaattcggcaaattcaaaaaagtgaaaggcgatggtacagaagaagaagtattcgaactgctctccaaagaactggatgaactggtaggagaaaaagtgcagtaagcggaatcccgctgtgattaagacttttagcatcttattatacaacgcaaagattgtaagtaaagagctcctggcacatgatggtgctaattagctcaaacttcacgatctttgcgttttgtttttctgtggtaatggaccccagagtattaaaaattgagaactagtggaaaaagcaaactttgtagattatatccgtgtattttgtaaatccgggaaaggtggcgcaggcagtatgcactttatgcgtaccaagtttaatgcgcaggccggccctgatggcggcgatggcggcagaggcggacatgttattttaagaggcaattcacagctgtggaccctcctgcacctccgctggcataaaaacctgctcgcagaagacggtgaaaacggtagcggcgacaactgtaccggccgtttcggtaaagatattatcatcgaagttccactaggtacccaggctaaagacgaagaaaccggccaggtggaagccgaaatcctccacgacggccaggaagtgatctggattcccggcggacaaggcggtaaaggtaacgcctactttaaatctgccaccaaccaaacacccgaatacgctcaacccggtatgcccggcagggaaggctggaaagtagtggagttaaaagttttggcagatgttggactggtaggtttccccaatgccggcaaatccaccctcctgtctactatcaccgcagctaaacctaaagtggccgactacgcctttactacgctaaccccacaactcggaatggtggaataccgcgacaataagtcgttttgtatcgccgacctccccggtatcatcgaaggcgcccatgaaggaaaaggattaggccaccgttttttacgacatattgaaagaaacgccgtattattattccttattccagctgatagtgcagaccaccgcaaagattttgaagtattggtaaatgaactggaacaatataatcccgaattactggataaacagtttctgctggccatcagtaaaagcgatatgctggacgatgagctgaaaaccgctatatcagccgagctgccggaagatgttccacatgtatttatttcctctgttacaaaccagggcctcagtgaattaaaagatatcttgtgggaagcccttaacaggaaagtagatactaccgacgctgtagacgcagaataactgttccttccgtaaaaggggactatgcctgacgtcaatgttcgtacagtatcccgtataccatgaagatattttttctccccgcaatcgcattgctgttgctgcctgcctgccatcgaaccgtaacatccgtaaaggaaaaaccggtgcagatcgataccatgcagctgatagccatgcctgcaccaacagcgaaagttgcctccaacgaagtatacgtagtgtgccgcgactctactacgtatatccgtttcggtgactgctatttctccctcgactggatcataccggatacacaactcaacgactttgaactgcatccggataccctctacttccggctggcacacctccgtaccatcgaaggccagatgctggccgttaccaccggcgaatcaaacaggataaaagtatcacagtgctacgaaaccagcgccgttattgagcagcaaccactgctcctgtggaaacattaccgatctccctgggaaacactgttccccgaagccaacaacttcttcatctgcagaacatataccgctgccgaaaaacgccggttcccatcagccaccctccacgcattacagcaacatgtaaaacaacattattcccccgccgcttattcacgcgttgcccaaatgaataacttcccggaaccacccctgcaaattgaaatcagccggtactatatacggctggatggttgctacaaacaaacaaccaacaggatcaataaactactcatcattgatgtaaactttaatggataatacgcatgaattaaccagcaacgcaaaagcatcgccggttattcattggctgtattttcaccataagggtactcttgtttcaactattgaaaaggctgaaacaacatggcagtgcacaaacaattcctgtaatttttgcttgccaggatgggatagtttacacaacttttacagccctcccaaaaaagagggtcctgcgtaatttcatgataggtaaccggctcgaaacccaaccgggtatttagtttcataacaggtaagcccgtagtaatgctgaatatttttgacgctggataaagcagccggcttaactcaaatattttctgcttgatggcctgtgccactttcaatccacggaatgccggcgctacaattaaaccgctgttggatacaaacctgttctcttcccaggattgtatataggaaaatcctgcccatatgcccttcgccgtaaaagcaataacggccttcccttccaggatcttttcctttattgtaaggggatttcttttcgcaatcccggtacctcttgccttcgcagaggcttccatttctgccacaataggcagcgcaaaatcaacgtccatagccgtagctaaccggacgacaatttcctcatctgtttccattaccagtaagttgatattgtatgtaaagtggataaattgaatccggtatcagtgaatacatccggatcctgctcacggcatctgccaggggaacccggcaaagtaccggtaaaaaaatacgggtaatcgcttctttcacaaccgtattaccccgttcgtataaccggccggccagctgcaaacacttgcctgctgccgaaaaattctgtgccctcagctgcttatcggtatacttcgtaaagcagcccatggtttcgttaatatgatgtacggcaggaaactggtgcagttcttcttttagtgcaggtattgtgtcctctatgcaagctggcacttcaaactgattaatcatggtaacatcattttgcaggtatatgccaaatgctattccatattctgtgtaggaatgttaaaacttagcgggagcaagggtttgcaaaggaaacgttaaaagcgagagataaaaacggcgtaaaaaaccttccgtttctgaagggtgttttcaaaaatggaaaaccggaaggatgatcctttttatgctacctgcgcaggaaccgctttggatacggccggagccactgctttctttttcttcttgcgggttctgttcagccacataagggtaccggtggtagggaagatagcgcccagcagtgcgaggattaaagcaaatattttagacggcgtaccaaagatggcgccggtgtgcaacggttttattgttccccggatctgctgcccgaggttcctttgcgcaaaagtttgcgacgacaacacttttccattaaactgatccaggtagtaagtggtggtggcagcttcgtgcagcgcgtctgccggaagcaggcttaccataaaggccgcggagctgtctttcggcgcagtaaacgaataaaacagcgcatcgggaacggcatgtttggctactgccaatgccgtttcataagatatacttttaccattcgcctccactgccggagccgatagcggtgctgccgaaggcttgggagaggttcccagtgaagcatacaacgccttgttaaaccattcaaacgaccaggttaagcccgtgaaaacagatacaaaaaggaagatggaagtgtaaaaacccagtacaatgtgtaaatcattgttcacccttttccagttaccgtcccatttgattttaatccgctgccggaaaatattgcgcgttttgggccaccagagaatgatgcccgtaaccaggataaacaaaaatataagagtgctgataccggtaatcagtttacctacagcgcccgccagcagccagcggtgcagggaaaatacctggtagtaaaatgtttgctgatagctgtatagttctatgactttaccggtgtagggatttacaaacgcaatacgtcctttttctttcttcgggcccgcgccttctttttcaccagccttagcggccccttctttctttcctgtcttacctctccgctccccgccttcttttggtccaccttttttaccttcctccagctgcacctgcagcgcccgtgtggggtccgcaaacacctgtatccttgcaatacctgcacccggaacggcctgttttaccagcgtagccaccttgtccagcggtaaacgcgctcctcccggctccacgaaataacggtcacggttaaacgcttccgtcagctccttctcaaacaccagtaaggcacctgttaaacagctgatagtgatcaccaggccggcagtaaggcccaggtataagtgaatgcgccggaaaaatactttcatgtcagagtcgatcgtacctgcaaagaaaatccacgcgcggggtattatggtatcggaaccggaatattatttacgcaatacagaatttcttcagtatttctataaaataaaattgccatatgtatggtacacatatggcaattccctgtattgaaaatatcttacatcaaccctcccagcattccgccggcagcgtttttcatttctgcttcccaggaattctctgcctctttcagtgcacggttcaaagcagccagcaacaggtcttccatttcttccttatgctccggtgcgaaaagacgctccgcaatatcaatacttttcacctggcggttaccatccacggttacttttactgcgccatcgccggcctcgccggataaagttacggtagccagacgctctttgccttcctgcattttctgcttaatctgcgtcagctttccaaataaatcaccaaacatgtttcttgtgtttttaagaagagcaaatatagcagatttttaacggtggcaatcccctctgctaaatccgcactattccgtatcttaccagcacgtaatcgtatcactaataatggaaacaaaagtttgtatcataggcgcagggcccggtggagccaccgcagcattgcaactcgcccagcttggcattgaatgtatcgtagtagataaagccgtttttccacgggataaagtatgtggagacggactaagcggaaaagtgctcaccctcctggaacgtatcgacaaaggcatcggacaacgcctccaggaagcaatttttaaagcagacagctggggcgttaccttcgtagctcccaaccgcatcgggatggatattccctaccgcctcggataccaggaagataagagcaacccaaggggcttcgtttgcaaacgtatcgacttcgataacttcctcgttgatgaaataaaacgccgccccgaaatccaattattcgaaggcaaaagcatcgataaatatgagctcaaaccagacggttaccacctctccagcaaagacggctccttcaaagtaaaagccgacgtggtaatagtagccaacggcgcccactccggcttcacccgcgatgtggccggtattaaaatggaacccaaacattatgtagccggtatccgcgcctattataaaggcatcaccgggctgcataaagacaacttcattgaactgcacttcctgaaaaatatgctcccgggctacatctggatattccccctccccaatggcgaagccaacgtaggcgtgggaatgctcagcaactccgcccgcaacaagaaagtaaacctgaaacagctgatgctggataccatcgctaccgacccggtaatgaaggaacgcttcaaaaacgcggaactcaccggcagcatcgacggatatggcctgcccctcggcagcaaaaaaagaaaactgcatggcgaacgctacatgctggttggcgacgccggattcctgatcgaccccttcaccggggaaggcatcggcaacgccctgtactccggcaggatcgccgcccagcaagccgctgcagccatcgccgccaacgactattccgataccttcttcaacgcatacgacgaggcagtataccgcatcctcggaccggaattccaggtgagcaccaaattgcagaaactcatcaaatacccgtggctatttaatatgctgatgaaaatgggctcccgcaataaacagctgaaagacctgatgtcatgcatgttccatgaggtggaccttcgaaagaaactgggccagcccatgttctacgtaaaattgttatttaacagataaaagcaccactccgtcgtgaaatttttaggccaattatccgtcatcctccttttctcattcaacatgagcgcacaggtaccttccaatccggaacatacgccagcagccaccctgctaacaaaggacatcgccaataaactggtggaactgcccctgaaatgcctggacctggaatttccctataaaacagggatcgtattcaccgacagctcactgctcacaacgcctaaaaattatcatcccgctttctatggctgcttcgactggcatagcagcgtgcacggacactggatgctggtgcgcctgctcaagtcttaccccgacctggccaaagcctccgtcatcagaagtaaactggcagcgcatctatcttcagaaaatataaaaattgaacaacaactgttcagcagcgcagaaaataaaagctttgaacgcatctatggctggagctggctcctgcaactgcaaaacgaactgctcacctggaacgacccattgggaaaaaccatgagccagaacctgcagccactggccactcagttctccatcgcctatatccagttcctcgataaaatcatgtacccgatccgcgtaggagaacataccaacctcgccttcggattatgcctcgcctgggactatgccgttacggcaaaagacgaacccctgcaaaaagccatacacaacgccgccatgcgcttctacgccgccgataaaaacgcccccatacaatgggaacccggtggctacgacttcctctccccctccctcgaagaggccgacctgatgcgcagggtaatgccgcaggcagactaccgcaaatggctatacgcatttttacccggtctttttgagaacaagataagtatcctgcaggtggcacaggtaaaagatagaacagacgggaaactcgttcacctcgatggattaaacctgagccgcacctggtgcctggaggccatcgcggaacacggcggcaaaaaccagcaggccattcagcaactggcccacgcacacatggaagcaggactgaaacaggttttcagcggcagctatgcaggcgaacactggctcgcatcttttgcagtttatatgttaactatcggaaaacaaccgtaaattcatcaacaaaaatttttattcccctatacccggccgcccataaaggggtatcaatcaacatcactatactatgcacgtcataaattcccgtgcctggaagttagtattatccctgctgctgatactaacccccgccattgcacccgcccaaaaagtaaataccagccccgctccggcatggctcgtcccctttacgcccgatctctccaaaaaacccaacgccaaaaatatcagcgatggctattaccttctgctgctggaagagcaaagacatacagaactgaaaagcaattaccaacacttcatccggcaaattatctcagaagccggcatacagaatggctcggaaatttcagtggaatacgatccccaatatgaaaaacttacattccataaaatagtgatccgccgcgatggaaaagaaatcaaccgcctgcctggcgcagcattcaaactgcttcagaaagaaaaagacctctcgcggttcatctacagtggtacctacaccgcatacctgatcctcgaagatgtacggaaaggtgaccagatcgaatacgcctattccattaacggcgataaccccatcttcaacgggaaactggatagccgcatctatttcgttgcctacgaacccattgtcaattactataaaaatctgatcgttagccctcaaaggcaaatccactttaaacggtataacaatgcagtcgcacccctccaaaaatcatggaacggcctcaccgtatacgaatggaataaagtagacatcagggaaacggataacaccaactttgttccttcctggtataatccttttacctatgtacaggtaagcgaatacacctcctggaaagaggtagcgcaatggggcatgaaggtcaatcaaaagcctgcacccggtccgttgctgaccggcaaaatcgccgcttttaaaaaatcggccaatggcgaccccgctgcctatctcctgcaggcattacgatttgttcaggacgatatcaggtatatgggcatcgaaatgggagaatactcccatcgtcccaataatccggacagggtactggcacaacgcttcggggattgtaaagacaaagccctgctgctttgtaccatgctgcgcgccaataatattgtagccgacatggcctatgttaatacggatctgagaggaaccgtcagcgaatcactcccttcccccaacgccttcaaccatgttattgtacatgcggtactaaacaataaaacatactggctggatggcaccatgtcctaccaacgcggaggcctcgttgatttatgcgaaccagactacgggaaggcactcgtggtaaccgataccaccacgcaactcacgccgatcgtacccgctacccgtggcaaaattgccgtccgcgaagtttttacactgccggacgatgaaaataaagatggtaaactggaagtagtaactacctaccaacgtgatgatgcagacgcacaacgtgctgaactggctggcaccagcatgaaggacaaagaaaaatcctatctctctttttataagaagttatatggagaagtggagatcagggactccatcaccacccgcgacagcttagccggtaatacgatatatgtgaatgaaagctacctggtacacaacatctgggaaagagacagcagcaccaacaagctgaaattcacggccaacgcgcaatccttttatgacgtgctttcctatatctccgacgataaacgtaaagtaccggtgagcatccgctatccatacgacttcgattatcaaatcatcctgcacacaccggtgaagtggtcgctggatcaaacaccactgcacctgcagaatgattactactcctttgattatacggccagcatcaaagggcaacaggtcctgttatcctatcatttcaaaaccttcagcgatcatatccccgtaaagtttataccgcaatatgtagaggacctgaagaagatgaatgaaataacttctatggatcttacctggaacccaggcactgctgccacgcgtcatccggaagggaaaggaaactggctggctatcgtactggcagttttatctgccgctgcatttgccgccctcgcatttgttttttataagcattctgttacacccgccggggaagcaccggaatcgcagccgatcggcggcggactggtactgctggccatcgggttattgtttgcgccaatgggagaaatcaccgggatctgcaaaatggatgtatttgattactcctactggatcagcatttccgaccggcaggacctgggaaatatcaccctggtacagcttttcctcatcatggaaatgatgatcaatgtatttatgctggcatacagtatcctgctggccgtgttgttttttcaccgtcgtgatacctttccttttgcactggcaactttctatttcattgctactatttctatttatgcagataattccctgaatcactatttcttcaaaacagaaaaaccgcaggatattttcagcgttaattccatcctctggccattagtgcgcatggcagtatgggtgccttacctgctcatttcacaaagggctaaaaacacttttactgtaccataccggccaccacagggctaaatattatttacatacttcctcaccgtgaggaggtttacaacatacaccagtcctaataccagcgcgatacctgcaaatacaggtattcccggccaggtgctcacctgcatctcatgctgcgccagttcacctgccgcccagtattgcagccccgttaccagcagcaacgacaaaattccgattacaatatacaggggtacaaactgccgcagcaggtaccgctgcaattgtttgggagcagtacccagtatcaccagcaattgaatttcccgcttgcaggacgcaatcaccagttgtataaacatgctgaaaaccagcaaggcaaaaaacaataagatcagtccaaaaaatccaaccacagatacgatcgtttgtacaatcagccttgttttgctgaacttcagtttatcctggttcgtagtataaccattgtcctgtaaaaacttcaccagctccgggttagatggatccggcgttttaatgatcacacgggaagtacccgcggtggtggtcattccatacttttcattggcccaggacataaaagacgccggtacaagaaaggaagagatccggtcggagaagccaacaatatgccccatgtactgatcggatacctggttgttggaaatatttacctgcaacggcaatgcttttacggtttcctgtgaaatctgcggcaggtcctggctcagggaaaaaccaaagttgtaaaggttcaggaagtcattaggcaaaataataggaatagtacggtcgccctcactccatttccagtcctgccctttcacatccaggaagctatccggtactgcttcaaaaaacatatcagtagcaaagtgcaggtcgcccggcgcctgaaccactaccttatactggctggaggttactaacccaaacgactgcacgaatggctgctttcttatattggcaatttcttcgggggtaaaaatacttttagacgattgccccatcatggcgttggtgatggttttattgatcacgaggaagtcggcggtttcattctggtttttgctgctgtacagcagctggctgaagttggaatgcgcctggatggcgatgaggatcagcagcatcgcaatgcccaaaccaactgccgccatcaggaaccgggtttttcccacaccggtttgaataattttcttcagtaattcaaaaaatggacgcatgaaataacattaaagatgataatgcacatcataagggaagtgctggtcattatccaggtctgttaaaatgaacccggcattgcgggctttacattcatcggcaatcagtgcggcggcgcgctgtgtattgtcttcatccaggtggctgaagggttcatccatcaggagccattgaaaaggctgtaccagcgccctgataatggcaatacgctgtctttcgccatacgaaagggttttgccgctttgctccagcacgtgcgacacattgagccgggcggccatttcatcaatcttttccgcaggataataaggctttggctccattacccgcttcaacgaaatgttttccctggcactgagctgctcaaaaaggcgaaggtcctggaatacaatactgatatccttttgccgcatcacggctatttcgttcttattatatgcctgccatggccgatcattcacctgcacttttcccgtatagtcgtaccggatatgatagaggtaatggatcagggtagttttgccggtgccggaaggcgccttgattttcacaaaactgcctggctggaaagtgacgtcctggttccagatgtccgacgaccgttgccggagcttatcctgcaatggtatgggcatgagctgattgagctgaatctgcatagtggcatttactgttaacagtagcgaatataaatgatatattttacgcaaaagaaaagggcgcaacggatatccggcgcccttttcctggtcaggttataaattactgtgcaacggtagtatcaaccggtgcagcaaatatgctgtcttcatacgctttgtccttggctttcctggcctgcatcacttttgcagcttcagtgcccaggttgatcagctgtaccaggctattctgatccttatttttaaaggtcagcaccgcttctccatgctgtacatcaccgccatcagctttgcttacaaaggttacgtctttcaacagttcctttgctttcttggctactggtttctcgtcttcttccattttatcttcaggaattacgctggctattttttcaatgtctacataaccacccagcatgctgccttttacttttccttcgataccatcaggtaatttgatgtggcctttgccacccaggtattcctgcagcaacacgctgtcggagcccagtgtcacaaatttctcgttgatggacatcgccggcatggtagccgctgccattggatttaccactacataatgatctccttccttggtaaatacttctttcagcatcggggaagtcataattttattgaaggcatccttgttaccaactttcaggctgaagatccatttagcgtctggtttctcagtgaactcgccggggaaataaggagattcctttttggtgatagcgaagtcagaagccacgtaggtcaactggccttcaaatgcgttcagcacatcgtccatagacaggccggatttacccatcatcaggttcaccataccatccatacccgttgctttcacgatatctccgatcatgcggaaatcaaaggcataagaaatgaaaccggtgatattctgggaaggatacttcttcagcatatccatatcgatctctttcttaccatattttttatagatcgccgccatttctttacccatgtaagagtgaccgttgaaaacgattttaccgttttcaaagttaaccgtaccggtatagaaagaaccttccatcagtttctttacgttggcaggtatcatggtaaactgaccgctgttgtaaatggcttccgggtttacaaagataccggcgtcggcatcttctttcagtaacttagcgaaaggctcaatggaaccggctgtttcatcttttttcaggtgaaagagatgatccacttctgctacccaggtttttatctgcgcatcgtcttctgttgtcaccagggcagcaggaacggctactgcggtgtctattattgctgttgcagagtctattatgggatctccataatcgggagatgaagaaccgcccgggttatacttttccaggttgcttggatctactgcactgatatagataacggcagatttgttccatccgattacggcatgttgcttttcttcccagatatatttaaagtcattttgtgttttcagggagaaatttgcgatgttctttttgagataggcctcaaatttgtcggcatctttcaggctggcggtaaggctgatgtaagatttatgttctgccggctggccctggaacacaaaagaggcaaagaagtggctttgcatgtcgataccggagttttcggcatctttccaggccttcatcacttcattggaggtgtctttactttgggtggcttcaaacagtttatccatggtaataccattcgtcaccagcttggtggtcagttgtttggcattcaggtccactaccacaccagctgttttcgggatgtaccggctctcgtcaggggttttagagcaggaagacagcataaccgctgtcgtcgcagcggctaacaaaactttggaaattgattttttcataaaagcgttaaaaattaagaaaattattcggagcaacactatatcgaacatgacattcccactatcgtggtatttcattcgtgcaaaagtacgtatatttttgtagcgcatatgtctcatttttccctggcacatacaatatttccatactgattaagtttatacctttgctactaactatgaaactattactaaataccatagaaaaaccattatgttcctgattatgctacaatacatacggcccgttgcggctgtagaacactacatggaggcgcataccgccttcctgcaaaaacacttcgacagtggccggttcatcttatcaggcaggcgaaagccgaagtcggggtctgttatcttgtgtaatgcggctacccgcagggaggtagaagagattatgagcgaagatccgctggaaaggttccagctggccctttacgagatcatagagtttgaaccaaccaagtatgccaacacactgggaaaataatatttccccctgtaatgccgtgccaatcgtttttgcttctttacttccgggataattacttcataaagtagatgaccttcgtgagccatttgctactgtccttttctttgcccggaccaatcacatacatttctatagtgggtggtacaatggtcctccctttatcggtaataaagtttctgatcgccacatgcgcattggctaccttgccgtgaggccccacgtaatcggcatatgcagcctgtgctgccggcagggtaataatttcatagcccggagccggtttacttccttccggtacggggatcgcagcggccatatcagtttgcccctgcttccggtcccagctgaaaaaaatgccgcagggcacgcctggctgcaaccgggcagcggaagctgcattaaaaatggtccggaggttggaatggtaatagtcgctgattttgctgatagggatggtttttcgtacagccgcatacgttgttgccgggaaattcatctctcttaccgtcacatcaatgccattgggtgcattcgggccttttacctctgcttccgccatactcttcaggttattgagcccctgctcaaagtccttctccagtgcgcctttcataaaaagggtcattacattctgaggccggtcgtaatgggtatcaaatccccacacaacctttgttttccctgccgcttccgataaccggaaaaacacatctgactcggatgcaaacggcgtgataaaggtaagcttctgggtaaccgacttataagggtccatggacaggtgttgcagctttccctccccgatcttgctgcctttccacgagtctacagcgccaatggagccatcttcaccagtgatagtatacctggcgccggggtccatctgtttccaggtgctccactcattaaacttctcgaatttcacaatatcattccatacaattgtcgcgggggcattgatttccactgaacgctccacatgcatggtagtgggcgcaaaaaagatcagcgcaattgcaatgaacaggatgattcctatgatccaggcgagcgttttaagtactttcatgtctgtcgggggttgatgataataaaaatacatctttttattgttcaaccgacagatgatactgacaatcagggcagaagaatgtttgactactccagttctttgtcaccgttttttttatcttgctggtactgttcatccgcttcctgcgctttttcaaagtccaggatcaccgaattaatacagtaacggagcccggttggcggtggtccgtcgtcgaatacatgccccaggtgggatttacagcggccacataatacctccgtcctatgcatcccatgactgttgtccggagaataaataacactggttttggtaagtggctgaaaaaaacttggccagccacagctgctgtcaaacttggtatctgaaacaaataaagggttaccacaagcagcacagtaataggttccgttctccctgctattccagtattttcctgtaaaggcccactctgttcctttctccctggcaatatgatacacgtctgttggcagtacttttttccattcttcgtctgtcagatttactttagtggcatccgtatgggagtaaatctctcccttcttttttccatcttccattgatttctttttttccccatttttggggtaagtatagttggtataccctgatagagatagtcaaaaatatcagtttccataggtacatatgtaaagttttgattcgttaacttctcattaacactatcattgtgattactgggtcgttggccggttccttttttatctctacataaattacgtatgaacaagcataatggattgttatttcctgcaaatcaaggggctatttaacaaaacagttaattttttgtttaaaactgtctgataatcaccgatgagcaactgcatataaattgttaactttacagcaaaaggctagtaagtggcggatatcatcaatttattaccagacaatatagcgaaccagatagctgcaggggaagtgatacaaagaccggcatcagcggtaaaagaattactggaaaatgcagtggatgcaggtgctaccgatattcaactgatcattaaagatgcaggcaaggagttagtgcaggtaattgataacggcggcggtatgagcgaaacagatgcccggatgtgctttgaacgacatgccacctctaaaatacaatccatagaagatctcttccagatcaccaccatgggattcagaggagaagcgctggcctccattgccgcagtttcccaggtagaacttaaaacccgcaaaagaggcgcggaagtaggcacctacgtggaaattgacaacagcttcgttaataaacaggaaccttgtcaaactgctgaaggtaccagcattgccatgaaaaacctgttcttcaatgtgcccgcacgcagaaacttcctgaaaagtaatgccgcggaaatgagacacatcgtagacgagttcatccgtgtggccatgtcattcccgcaactgcagttctccctgacaagcaataaccaacagctgttccacctggacaaaggatcgctcaaacagcgcatcgtggccatcctgggacaacattataatgcacgcctcgtaagcgttaaggaaactaccgactacatgaatgtgtacggatttgtaggaaaacctgaaaccgctaaaaaaaccaggggcgaccagttcttttttgtcaataaccgctttatcaagagctcctacctgaaccacgccgtgatgaacgcatttgcagacatcatcccggccgacagcttcccgctctatgtattgtttattgacgtaaaccccgaacatatcgacatcaacgtacatcctaccaaacaggagatcaagttcgatgatgaaaaactgatgtatgccttcgtgcaatcggcggtaaaacactccctggcccagttcagcatcactgccacactggatttcgacctggacccgagcattcaggccctggacgcggtaagtaaacccttcaccgcccagcagcagcatgaatccatccagagccccctgtataaatcatttacacaggccaaccaggcgcacatgatcgataaaagcagcaacagcagcaacctgaagcactggaaagatctgtacgaaacaaacagtaataacgaaactacttataccatcgccccggaaccggaaacacggccggctgtaacctacgaaagtcagccgcatgccaccgcctccgtgatcgatgaacgctggcaggataccgccaccgatcaaaaagtaccggtacaggtgcaccagcaatatatcctgtcgcagataaagtcaggctttatattaatagatcagcaggccgcccatgaaagaatcctctatgaacgctaccagcgtgccttacaggaagctcccatggccacccagcaaagccttttcccgcaaaccctgcaactgcccccggcagatgcagccctggtcagcgaaatgctgggcgacctccaaacactgggctacgacctggaaccatttggaaacaataccttcatcgttcgcggtacccccgccgatatccagaatggtaacgatcacgccaccatccagagcctgctggaacaattcaaaaacttcagccacgaactgaaagtaaataaccgcgagcaactgatccgctcaatggcacgtaataacgccataccagccggcaaaatactggctgcccgcgaaatgcagaatatcatcgatgaactcttcgcctgcagcatgcccaatgttgctcccggcggcaagttcacgtttatatcatttaaactcacagacctcgcgcgtatgtttgaacgcgggaactgatgtcaggatactaaaaatccggggagacagagcaggcattgcccagctttactctccggatctttaaacaacggctctgcccgcataaacccgctctcctgatagcttccaaaccctttacagcagaggatctccagatcaagtccacctcacctccagcatttctccgtgtttagtccatgtgtaatgcagctcctatccatatgcaacgtaggtttgcgcctaccgcaaggttagtgctataccatcattctgccataaagcattcttctatctgcccgtacaacttcaggaacatcttatactttttacgataagcctcaaaccgggtggcatccggcgtaaataccgtttgcgcctgttgtgagggccgctccggccatcccagcacgttagcagccaacaggatagcaccaagcgcagaggcgtcgctttcctgctgcaggtgcatttcctggccaaagatatccgccagcagctgtatccaccccggcgcattggtaaaaccaccgctcacagagatccttttcaccggcccggcagtttcttccagggcctctttaatgctcagcaacgcaaaacaaatcccttccagcacggcgcgggtgaagtgcgccggcgtatgctggggctgaataccgatgaaggccgcggtagcatgactgttccacaccggcgccctttcccccagcaggtaaggtaaacaaaggagttttccggggtcagttaccaatgcctctgccaccaggtcgttcagcgcatccagtggctgccgcaggaaatccctcaccagccattgcagcaccacacctccattgttggaggcgccaccggtaatataaatatcatctgtcaggagataggtgaatagccggccacgggcatcagtgagtggttgggcgcctgccatccttaccgctccgctggtgccaatggtaagcgtggcatgtcctgcatccagcgcaccactgcccagctgggccaggcagccatcgctgccaccaatcacaaaaggcgtactggccgggatacccagcatggctgccatatccggcaacagcccgctcaccacatgattagccggcaccggctgtggcagctgcgcagccgtaatacccgccacgcccaaagccgtttcattccattgaagcgtgtgaatatcaaacaggccggtcgccgacgcaatggaatgatctgttaaccagcgtccgaaaaaatgatgaaagatgtattccttaataccgggaaacatggccgtggcagcaaataaggcaggctgctgctcccgcagccacatgattttgcacaggggcgacatggcgtgtaccggcgtgccggtttgccggtaaatcagccttccttccggcgtatcgcgtaatcccagcgcgttgggctcgctccggttatcagcccagatgattaacggtgtaagcgccaccccctcccggctcaccgccattatgctgtgcatggcgctgctgaaggaaatggccgccggcgcgcctcctgcctgggctaccacttcccggatgctggctattaccgcttccaggatcacccccggtttttgctcgctgtatcccggctgcgggtgactggtaccatatgcctgctgaaacaccgccagaatttttccgtccattccttgcacaatcgattttgtactgctggtgcctatatctacaccaataatatatgctgtatgatcactcataaaaaaaaccgttctttttccgcatttaatttatagatttaaaaccggtgttcttctaaaaagtctaaaatatccacgcaaatggctttcgaaatcaaaaaacaggggaaggtttatgacgtttgtattgttggttccggcgccggaggaggcatggccgcaaaaatcctgtcggatgccggcctgaaagtagcccttctggaagcgggccctaaatacgatccggccgacccggagcaggcaacacagctgaaatggtcatatgaatcgcccagaagaggagccagtaccacccgtcctttcggcgacttcgacgcatcctatggcggatgggagctcaacggtgaaccttacacgaaaaaaaacggaactgaattcgactggttccgctcccgcatgctgggaggcagaaccaaccactggggccgcatctcactgcggtttggcccccgcgacttcaaacacaaaagttatgatggcctcggcgacgactggcccattacctacgatgaggtggcgcccttttacgaccgggtagataagatgatcggcgtgtttggcagcaaagaaaacctgcccaacgaaccggatggcttctttctgcctccacctaaaccccggctccatgagctgatggtgaaaaaagcaggcgatcgtttaggcatccccgttattccggcgcgcttatcgatattaacccgctccgtaaataaagaccgcagcccgtgcttcttttgcagccagtgtaaccgcggctgtaccgtgtacggcgacttctccgcttcttcagtactggtgaagccagccatgaaaagcggacatgtggacctgtataccaacgccatggtgcgggaagtattaacagacggcaatggcaaagccaccggcgtagcttacgtagataaaacagacctgcaggaatattccgtaaacgcacgggtagttgtactggccgccagcgcctgcgaatcggcccgcttgctgctgaactcaaaatcagccaaacatcctaacggattggccaactccagcggtgtagtaggtaaatacctccacgactcaaccggttcttcacgcggaggcttcctgccccagctgatggaccgcaaacgatataatgaagacggcgtaggcggcatgcatatgtatgttccctggtggggcgataacaagaaactggacttcgcccgcggctatcacatcgaatttggtggcggcatgcacatgccgggatatggcttcggcttcggcatggaaaatatgaacggccgggcgcctggtcgtgatggccaaaccaaagcagccggtggctacggcgcttcactgaaagatgattaccgccgcttttatggctcccagatcggctttgccggcaggggcgaatgtattgcgcgggaagataactactgcgaaatagatccgaacgtggtggataaattcggtattccggtactgcgttttaactacacctggagcgatcatgaaatcaaacaggccaaacacatgcaggatacgtttgaacagatcattcatgaaatgggcggcatcgcctttggtaccaagccgggagccgataccaaatacggactggaaaacccgggccgcattattcatgaagtaggtaccacccgcatgggtgacgacccaagcaaatccgtgctgaataaatttaaccaggcacacgaagtaaaaaatctcttcgttgtagatggtggcgcgtttgtgtcacaggcagataaaaaccctacctggaccatactcgcgctatctatgcgggcatctgaatatatcgtggatcaattgaaaaaacagaatctctaatcttttaagtttttttcatggatagaagagaatcactcaaagcgcttgcactgggaacgttatcagttggtaccattttatctgccaccagttgtgaagataaaaaaacaacggctgataaaaatgatcatcccaatgtgaaaaccaccggctatggccgtactccggaagaagtgctgcgggataaatcgttaacagaacaaaagttctttaccgacgccgaaatgaaaaccatcaccatcctggcggatatcattatcccggcagatgaacattccggcagcgcctccgatgcaaaagtgccggagtttatagaatttattgtaaaagatataccggagcatcaattgcctatgcgcggcggactacgctggctggatatgcaatgtgccaaacggtataataagtcatttgcagaaagcagtgcagaacaacgtatcgccgtagtggacctgattgcctggccgggaaaagcgtccccggaaaacagccagggcgtcgcatttttcaaccgcatgcgtaatctcactgccacaggctttttcaccagtaaaatgggcatcaaggatctgaactacatcggtaatacgcccaacgaatgggatggcgtacctgacgatgtattaaagcagtacggttatgcctatgatgaaaaaacactggctacctgtctgaaaatcgaagacaggggcaagctgatgacctgggaataacgatcaaacttgctatttcataatttaaatccagaaaacttcacatcaatgattccagaaaaaaagaatgagggagaaaacggtgtttcccgcagatcattcctgagaaacggtgcgctcgccgccgccggtttcatgatagttccacgtcatgtattaggccgtggctttgtagcgccaagcgatcgcctgcgggtagcaggtatcggcgtaggcggtaaaggcttcagcgatatatctgaatttgctaaaggtccggctgatattactttcctgtgtgatgtagataaacgtcgcgcagccgaagccgtgaagaaattccctaaggcaaagttctataccgacttccgggaaatgtttgacaaggaacacaaaaacttcgatgctgtgtctgtgtccacaccggatcacacacacgccgtagcaacaatggccgctatgcagctgaagaaggatgtatatgtgcaaaaaccattaacccacgacatctacgaagcacgtatgcttacacagggcgccaacaaatacaaggtagtaagccagatgggtaaccagggctcttccggcgatggcgttcgtcaactgatggaatggtacaatgccggacttgttggtgatgtacacaccatctactgctggacagaccgtccggtatggccacagggcgttccctggccaaccacccgcgaggaagttcctgcagaactgaactgggacctgtggttaggtaccgctcctaaaaaagattacgtgggtaacctcgtgcctttcaactggcgcggctggtgggattatggtaccggcgctatcggcgacatgggctgtcatatcattgaacctcctttccgtgtattgggcctgggctatcccacttctgttgagtgcagcgttggtagcgtatacgtgggagaattcacccgcggatatttcccggaaagctgccctccttcttcccatgtaattatgaaattccccggaaagaatggcaaggaagtaacccttcactggatggacggtggtattcaaccagagcgtccggaagaactgggacccaacgaaacaatgggcgacggtggtaacggcgccttgtttatcggtgataaaggcaaaatgatgtgcggtacctacggtatgtatcctaagttgctgcctacttcccgcactacagaagcaaatgtgccgcaaactattgcacgcgtaccggaaggccactacgtacaatgggtaaacgctgctattgccggttacggcagcaaacaacagaaagcgctgagctctccgttcgatattgccggtccgcttacagaaacgatcctgatggctaacctggctatccgtagcttcgatatccgtaaggcaaaagcaaatggtaaaggctttgattacccgggccgttatatcaaactgctctgggatggtaacaatatgaagattaccaacttcgacgaagccaaccagtttgtgaaacgcacttaccgcgatggctggtcactgggcgtataaatgatatccatataaaaagaaaatgccgcgataatccgcggcatttttcttttatgaaaagctggtacatgaatcccgctattgataatcgtcttgttgtttcaggttactgttcttcctgatttcattggcaggaataggcagtaagtaattcttcgccttattaaatttacgggactggatactgtatacatggtatacaaaaggatgtccggcaatcattgatcccaacacctcaatgccaaaagcattttcattaaaagccgtttcggcatccctccacctgcgggcatcaaagaaacggtgttcttcataagccagttcataccgtctttcatatttcaacacggcccataaagcggctccggatgcagtagtagcaggcatcccggcacgttcgcgtaccttattcaatataatacggccgttcgcctcatcgccatatccaatagctgcttctgcatagttcagcagaatttctgcataccggaagaagatccaggactggtcgcctcggaagaactgggcatccaggtttttgtccataaacttacgcaggtaataaccggagtaagtaccattccagttttcgatggtactgttgcgggtatcaagtccccacacactgtcccttccattagcggcttcatatttcccggtttgtatcactcctaccgggtccgttttggcggcatcggaaggacgtggtttccacttagccccatcatataaaatggtggcgtaaaagcggggatcccggttttcatacggcgcctttgcctgggcagcattgctccatgaaaaagcagtaccatctttcatctggtagccggtcacaaaattctcaataggcacatttccgccccagttgtgatacccgttaggaccattgtacaggtcgtgagaagtacccagtaatgctttatcatattgcttaacaaagatcatctccgggttatctttatcgaggaacacccgggtatagttctctaccgggttggcggtaggctggtaaaggctgtaagtgttaaggtccattaccgcttttgccgcatccattgccagtttgtagcggtctttttgtaagccggatttataccccattaagtcattaggcactttcgcatcattgaacaggttgctggcggcgtaaagcagtatcctggatttcagggccatagcagcgcccctcgtcactcttcctttgcttgccacggcatcataggtggccggtagttgttgtgtagccaggtcacattccgctgcaatgaacttaatacattcgtcgaaagtggctcgcttcacactcaggatctcctgttcatctcccttaatattaaaagttttggtgatcaacggaacaccgccatagtatctcaccagcatgtgataataccaggcccgcataaaatgcacttcgcctgtcatgcgtgtccgcacggcttcatcggtcaaaggcacgtctgcaattttctccaggaacatattacagttacggatagccttgtagtgcaaatcccatctggcaaaatcgttgatggcgcccacatcatcggcggaggcgttaccctgcaccaccctggaggtattgtagtcgtggataaaccggctttcgtctgtcatggaggaaagcattacttcaaggaaaccgggacgcatctgtacatacaggtcgtttacaaatgcctgtaccaggcccacatctttccacacgtcattttcttcatactcggttaaaggcttcttttcgaggaagtctttattgcaaccggcggaaaccgcacatagtagaaacgctcccgctatatatctgataattgttgttttcttcatggcacattaattaaaaggttacgtttaatcccacattataaatcttggtttgtggatagaactgtccgcttccacttggcgcttcggggtcaaaaatcttcactttgtcgatggtaaccaggttctggccacttacatatacccggaggttttgcagtccaatccgtttgcaaagggcggtaggtatgttgtaaccaagatccagggtttttaaacggacatagttggtattccaataccagaaagtattctgacggtttacccagtactcacggtcacggtcgtacgctcttggccatgatccgttgatattgtcttctgtccagcggtcttttacatatgccatcgggaagttcccaatcaaaccggattctgtacgcaggtactggcttgcgcctgtagcgccctgccacagcatggtgaagtcgaagtttttgaacttggcggtcatggtcaacccgaaaatccaggtaggattttctgtacggtccatgcgaatacggtccaggtcatcaatggcgccatcgccgtttttgtccaggaagataacgtcgccagctcttgcgccgccaacgtgcgggcttttatccacttcatcctgtgttttataaataccaatggcttggtaatacagtggtgcgcctatctgtttgccggtagcctgctgatatgcgggcaggttcggcgtttcgtcgaagaacagtactttattttctgcgtgagtaacggttcctataatttcataatggaattttttgatgtcgttcttgtggctcagcaccagttcaaaccctttgttttccaccttggcaatattttcctgcggcagggtcataccggtatagccgggcatcgactggctgcggctggcgaggatattggatcttttagtcaggaagtaatctccttcaaaggccagtttatctcccagtatttttgcttcgataccgaaatcatagttgttggctacttcccaggtaatagactcgttgggcgaccgcagctggtaaaggcctttattcaggtctccgcccagcattacaccaccggcactgaatccataggtgctcaggtactggaacggatcgatctggtcattacccatttgtccccaggacgcgcgcactttaaagtagtccagtgtgcggatgctttttttccagaaggcttcattagacaatacccaacctgcggaagcaccgggaaacagccccatacggcggccttccgggaaattctgggagccatcgtaacgcatgttgtaatcaaacaggtaggtttccttgtagttataggatatacgcccgaagtaattgcggcgcgcatattcaaagccgctgccggcattattcttttctttgtcgccacccaaattcaactggtccagcttatcactgataaagtacctgcggtttgcagagaagccatcatttttcagtgtggcctgttcaaaggcgatgaagctgctgagattatgcttcccgaaagaacgtacataattcactttgaagttgacagtggtttggcgcagcgtactaaactgttccgttagttcaggcgcgcttacacccctggaacccgcattcagcttatgcgtaggatcattggcatctgccagcgtgtataatgtccagggtttaatgtacgatttgtagaagtcgaagttctgatcgtaggcaaagctaccatctacaaacaatccttctactcccggaatatttacaacggccgacatgttggtgttgatcacatagttcttatcgttggtgtaaccgattgcatttgttcctgtaacaacggggttatcgccgtattcaatatcaggtccgggcagtccgttgggccagatagcgttttctgtaggacggccgcgcatcagggatctgaaaatagacccggcgctgcgtggaggaaagttcctgttttccaggcgtcctgccaggtcgaaacgcaggcggatgtaatcactcactactgcatcgaggttagcccttacgttctgttgtttgtaattggtggcactgcttttataaataccgtcctggaataaggatccgagggaaacgtagtaagacattttctctgtaccgccgctgagcgacagatcatgcctgttttgcaaagagtattttttaatcgctgcatcgtaccagttggtattgggatagagccacggatcggagccgtctccaaatttcttgatctgttcatctgtatacttcggagcgtctcctccatactttaaaatttcgttcaccactttggcgtacgtaggcgcatccgccatttccggcagcctggtaggcgttacaaacgactggttgaagccatagctcagggtcggtttacctcctttaccgcgtttggtggtaacgaggataacgccattggccgcgcgggaaccataaatggccgcggcagcatctttcagaatggacacactttcgatgtcgttggggttcatgcgctcaaaaccatcgcgcgggaaaccatcaattacaacgagcggattactgtttcctaaagtactgcggccacggataaaaatacgggagccgtcgtaaccgggctctccactgttgttaacggcaataatgccgggaatacggccaacaagcgagttagagatattaacgttaggtgactgctgtaactcggcgccttttacagaggatactgcgccggtttttgtaacttttttctgtgtaccataacctactactacgtactcgtccagggttttctggttctctttcaatacaacattctgggttgtctttccgtctactttcagctcctgtgcatcaaagccaatgtactggaatacgagtaccgcatcttttttaacatcggttaatacatagttgcctttttcatcggaggtggcgcctttcttggtgtctttcaccaacaccgtaaccccgggcagcgggttaccgttgatgtctttaacctttcccttaactgttagatttccttgttgccatacactgggtaatggcgcgcgcgcagtgatggcgctgctggtggtcgcaaacaggcatagcaatagcatagcctttgcataacgtgggttcatgctacaagtgattttggaagatgatgaaaatttgtctgttaactagcttttcataacgacgaaacgggtattcatgtctatgtaagataaacatgaaaagtttaattattttctaaaaataaatgtctcaaatacaattattttaaaatttcttccttaaaaaaacgaataaatgtaatttctactcgtatgagtatttgagcggctaaccggagcagctggttattatattattaaaaaaaccactggcaaacagcccggcggttttttttgcataattttataccctgaagcgttatttaaacgttatagtaacatcaaccatatggttttatgaaaaaacgttactttctcatagctatcctttcaatggttaccttattgttctcctgcagtaaggaaatgagcgatgaaggagaaggtgcattaccttccaacagcaattgcgaatatgccccctatacgaacggctcctccttttcctatataaacgtaaatagctccgaagacacgaccagctacaccctcacggtttcagaagatactaccatcaacggtgtagtgtataaaaaagtgggtaacgacagtgtatttacctgctccaactgtaaagatggcatctatacgcaggtggccagcatccttactttccagggttacagcgccgacagcctcgagcttacttatctgaaagacaatgtccccgtgggcaccagctggaaagataccatcaccgtgaacaacggcggagtgaccacatccggcatcctggaatttacgattacagaaaaggatatcaccaaaacggtgggtggcaaaaactacgcctccgtgatcgctgtaaaaatggatgcctatgccattgtttttggcaacccggtttctgtgggcaccatctccaccagctattacggcaaaggggtgggactgatagaagctgatcagctgcacgacaccaccaccatcgtttcctataccataaagccttaataggctgtgcttaccatcgtgagcaaccgctctaccgcccttctcacactggtagcggattcatgatgattattcaccaatacactgaataccagcgttctctttttcttcgtttccaggtaaccgctcaaggctaccacgccattcagcgtacccgttttggcatgtactttctgttgctggtagtagttctttaatgttcccctcccgccggtggggaaaatctgccagaggcgttcctgcgggaactgttcgcgcatcagggtgagcagggttacaaagtcgcggggcgtaaacaggttataccgggaaagcccggagccatcctcccactgcggcggatgcggcaggcttttgaggttgccggtaagcaggtagctaattgtgcgggcgctgctgatagtgtcccacaaagcggaagcagccatcatcagcgtttgctctgcaaaaaagttatcactgcgctccatcatcggtataaacaacgaatctgccgggatacttttcagtattttgaagttgccggccggcggtataacggccagccctatacgcttatgcagcgtgtcttccagccgctgccgcagctcttgtacagacccggtaataaaaggaacttccgcattctccaatgccttatccttcgggttgtatttcaggtagaataaattattgcgttcgtctctcgatgtgatcgtttcgctcagggtatcatcttctgcaatatccaggtcatagaaagcaggcacaatactgttgctattcccctggtgacggatacgtaccacattaccgtacatgggccattcattcagctccggctgatagtcgtcggcataatcaccccagccccagcccgggccaaaacgttggttggtattcacaccgggtaccaggtaaatctttttagtggtttgctgcaacaactgcagcaggggttgatagtgatagtccgggtgcagaaaagatgggtctcccattccctttacaaaaagggctgtatcattttcataataccgcgccgcgggaagggaatctcccagcaactttaatcctgcatacaacgagaagatcttagtattggatgcgggggtgaaaaacttattgtcctggtattgataccagtatttcccggtagccggttcataaatacagatgcccacatgtgcctgctccattggtattttatgaagcaattctgcttccgcccatttctttatcgctgccacctgggcggttacacttcccccggttatgacggatataattactaccagtaattttttcatagatggaaattacgaattgtgcattacgaaacagggatttgtgagaagaccattttattgatcttcccccaaatccctgatccgttctttacctggtaatttttatcaggtaaaatatttggtaatacctggttttgcgtaagcataattaccagatgcatccggcataaccggtggctgcgcatcaaatgagtatgatttaggatgcaggtccagaccggagttcagcgctacattccagtcgatcacctgaccggaataggttgccaaacggcctataatagcagaaagggtggcttgtgcgcctctttccgcatctgcaaatttgtattcgcctttggcaatggcggcaaacagttcatcgtgttccgtctggtaaggattgttttccttcttcttatcaaactggtataacactttgcctttatggtccactatctgggctttatcacagaagatacgaccctttgttcctacaatttcctcgtctactttgctgggagcgtctttccagtggcggcactggctgttcattactacgccattggcataacggtactccacaaagtggtggtcaaatatttcaccaaactccttgccggtacgcacggcacggccgcccatacctcctgcggtaacaggagtagcgcccataaaccagttgcctacgtcaatattgtggatatgctgttctacgatatgatcgccgcacagccagttgaaataataccagttacgcatctggtattccatttcagtatattcaggtttgcgtggttttacccaaagtgcgccctggttccaccacacctgtgccgacagcatatcaccgatcataccgtcctggaagcgtttgtatagttcgcggtaagaattctggtagcggcgttgtaaacctactactacgttcagttttttggttttagctaccgcagcagcttccagtacttttttaataccggcgggatctgttgctaccggtttttccatgaagatgtgtttcccctgtttaaccgcttcttcaaaatgaatgggtctgaaacccggaggggtggcgaggatcactacatctgccagcgcaatggcttgtttgtaggcatcgaagccgataaatttattgccttccggaacgtttacccggctggctttgtcgcccagtgcttctttaatatcattgaagctgttattcaacctgtcggggaaggcatctgccatcgctaccagctgcacgttttcttttgtgctgagcgcctgtgtagcggcgccggtaccacggcctccgcagccaatgagggctattttgataacaccggtagatcctgagaaataattagcttttgataaaataggcatagccagcaaaccgccagcaagcaaagtagtttgctttacgaattcgcggcggccttcaccgtggaatttcttttcgttgtccataaatgaataagatttttagatttttggatgttgaatctttctagcgtgcacctttatattttgcgatcatctcttcaaaaaatgctgtggcttctgctgctgttggttgtttaacgggtcttactattctgaagccaacaaagggggcgtctgcattccaccaggagcttttaggaatctgtgggtcgcggcggttccagatggggtccgacttcaggcgggcggcgctgcggagcagcggggcttcatcctggaaactgccgcctttcagcagccgcggggttttagcagttggctgtgtccagggatcagtagctgccgcgttggctacgccattttcgtcgtattgatccaatgtccattcttccacattgcccagcatatcatataatccccaggcattgggtttcagctgtcccaccttatggtatttattatcactattgccctggaaccaggcatactctttcagctgaccggcgtcggcgccaaaaggatacgcggtggtggaacctgcccggcaggcgtattcccactctgctgcggtgggcaggcggtaaaagacaccggtttttatatacagccactggcaatacatcagggccgcatactggctcatactgttggcggggaatccaccggatttacccatgcccagcgtaagatcaatatatggcgggctgggacgggtcatcccgtctggtgtgggtgttttatccttttccgcatcagcatatatatcgtattcgtcaaaagtaacttcagtggcgcccatccagaaatcagacacgcttaccttctttgccgggccttcatctttattccttcctttttcactgtcggggcttcccagttgaaagctccccccttgtataggtaccattttaaaactaacatcggttccggggatctgctggctataagcttcgaacgcctgctttgattgtgctaaaacaacaacctggctgagcaatccgcccagcattaaggtcacatacggtttaatcatctaacgtgtttgaaaatataagtgggtgaatctaaaaaaaactaacggggaaagcaatatttttttatgaatgcgaaaatgagctgatgaattgaaaaatttttatcaatattagtatttccttagaaaagcgattaaatttagctccctgtcaattatacaatcaatcaaacgttatggaaagaagaaaattcctgcaaaacggcgccctggccggtatttcagcgctggcaatgggaggcatcagcaacactgcacaagccgccggcgataacaatgccagcctggccggaaagccgtttaacatgaactatggcccgcatgacggcatgtttaaaaacagcgccaatggcggtaacttcctggaccagataaaatatatgtacgatcagggattccggtctatcgaagacaatggcatgctgggacgctctcctgaggaacaatccaaaataggcgacctcctgaataaattagggatgaccatgggcgtgttcgtagtagataccggcaataactggaaaccttccctggccacaggcaaacaggaatttaaagatgcctttattaaaacctgcaaagccagcgtagaaacagccaaacgctgcaatgccaaatgggctaccgtggtacccggctactttgaacgcacacttcctatcggtgttcaaaccgcacatgtaatcgacgcactacgcagcggcgcggaaattttcgaaccgcatggcctcatcatggtgctggaacccctgagcgataaccccgacctgtttctccgtaccgccgaacaaagctttgaaatatgcaaggccgttaaaagcccttcctgcaaaatattatacgacatctaccatatgcagcgcaataccggcaaccttattcctgtaatggactggtgctgggacgaaattgcctacatccagatcggcgataaccccggtcgtaaggaaccaggcaccggtgaaatcaattataaaaacatctttaaacatctccataacaaaggatataaaggtgtattaggcatggaacacgggatggccggaaaaggaaaagaaggcgaagacgcactgataaaagcataccgcgaagcagacagctttatataaccactgatatttagctgttggcagcagattacatgccggccgccaacagctaaactttgccattcactttttttttcgctaacttaactagtaaaatgatctacaatgggtttcctgcttcgtatactagttagtgctttggctgccatgttaaccgcttacctgctgaaaccggcagtaaaagtagatagcttcatcaccgcgctgatattggcgctggtgttagcactgttaaatgccctggttaaacccctgctcattttactcacgttcccggtaactattgttaccctcgggcttttcctctttgttatcaatgccctgatcatcctgctggccgctaaactggtacccggttttaaagtggacggtttttggtgggccctgcttttcagtatagttatgaccatcatcaacagcgttatgatcagccttgccggcggtaacaacgattagccattacctttactgcctgttaaaaagccaattcatgcactttgaccggtcagacctgaacgatgcgcaattacagtctttctataaagcattggtatacccacggcttatagaagaaaaaatgctgctgttacttcggcagggtaaaataagtaaatggttctccggcatcggccaggaggctattgcggtaggcgctaccctggcgctggaagcagacgagtggatactccccctgcatcgtaacctcggtgtgtttacaacccgtgaaatgcccctccacaaactactgcagcaatggcagggaagtgaaaacggctacagtaaaggtcgcgaacgctcctttcactttggcagcaaagcacatcatatttgcggcatgatctcgcatcttggcccccagctgtctgttgccgatggcattgcactggcgcaccagctgaaaaaagaagaaaaggtatccctcacttttaccggtgaaggcggtaccagcgaaggagaattccatgaagcgctcaatgtggcggcggtatggggcctgccggtcatcttcctgatagaaaataatggctacggattaagtacccccgtcagcgaacaatatcattgcgccaacctggtggataaagccattggctacggcatggaaggcgtacagatagatggcaataacctgctggaagtatatcaaaccatacgcaccgcaagggcctatgccatcaaggaacagaaacccgtactgatagaggccatgaccttccgcatgcgcggacatgaagaagccagcggcataaaatatgtgcctccggagctgtttgaagcctggggtaaaaaagatcccattgcgcaatatgaatccttcctggtgcaggcaaacatcctttctgcagaaagtattgccgccatccgggaagaactgaagcatgaaatagatgtacaggtggccacgggctttaccgatgtccctttttccgccgatacacaaacagagctgaatgacctctatgccccggcgcccgctccggtagccgcttctgggccgtcttcagaaaaacggtttatcaatgccttatctgatggtcttaaacaggcgatggaacaacaccctgagctgatcctgatggggcaggacattgcagcttacggcggcgcttttaaaatcaccgaaggcttcctggagcagttcggcacaaacagggtgcggaatactcccctctgcgaaagcgcgataatcggcgctgcgctgggcctgtctatcgggggattcaagagcatggtggaaatgcagtttgccgattttgtgacctgtggctttaaccagattgtgaataacctcgccaaaatacattaccgctggggccaggcagccgatgtagtgatcaggatgcccgccggtggcggtgttggcgccggtcccttccattcacaaaccaatgaagcgtggtttacccatgttcccggcctgaaagtggtatacccttccaacccggcagatgcaaaaggcttgctgaccgcagctttcgccgatcccaacccggttctgtactttgagcataaggcactgtaccgcagcatcagtgggccagtacctgataattattacaccattgaaataggaaaagccgcgctggtaaggcccggagaagatatcagcatcattacctggggcagtggcgtgcactgggcattggagtatgcccaacagcacccggcgctttcgatcgctatattggacctgcgtaccctgctcccactggattacgccgctatccgggaaatagtggccgcaacgggtaaagtgctgatcctgcatgaagacacgctgacaggtggcttcggcgcggaaatcagcgcctggatcgccgaacactgctttcctctcctggatgcaccggtgatgcggtgcgccagcctggatacccctgtgccttttgccggcccgctggaaaaaaattttctcgccaaagcaaggctgggcaagtacattcagcaattaaccagctggtaaccgaccgtatgattgggaatatgcattgaaagttttaatttgcatccggaataatataaaatcattatacaatgttgatgaatcttttaacagtagtacacaccaccaacttctataaagttggcgatagtatcggaggcttcctggctcctgtggccattatcgtttttgctgccatgtttatctacgcatgggttaagtacgcaaagatctaattgcaatagtttttcacatcgcattataaaaaggggccatctcaatgagatggccccttctatgtttagcgtattattcttcgggaggtatatattgattataatagtgccttgtgtaacgtaaattctcttcatcaaaacacacgaggatcacttcctctatttccgtgtttttctccaggtacttcacgatggtatccatggctattttcgcggcaagatctttagggaaatggtaaatgccggtactgatattggggaaagcgatacttttcaaatgatgccgggccgccagctccagtgaatgccggtagcaattggccagcaggatatcttcttcccgggtaccattgttccaaacaggtcctacggtatgtataacatgttttgccggtaaacggccggcagtagtgattactgcttctccggttttgcatcctccctgccgggcaacaatagccctgcaatcattgagtatttccggtccgcctgcacgatgaatagcgccgtctacaccgcctccgcctaaaagcgaagagttagccgcattaacaatggcatctgcctttactttcgtgatatcaccttgaatgatactgatctttctatgtgccataggattatacagttcttacatataccagtttcccggttttctttccactttccctgatgtctatttcaaagtccggaaaactttttagcaattgcaccagtttattgaatccaaagttacgggagtcaaaatccggttgtttcttcagcaacaggttccccagttcgcccaggtaggcccatccgtcttcgtctgcaatatcattgatactggtggatattaaagataccagctgcttatctgctttactgatgctgttccgtttatctttagtggtttttgtggttttctctgtatctgttttcttttctcttacctgtaaaatttccaggtaaataaatttgtcgcacgcggccctgaaggcgctgggtgttttttgttctcccatgccgtatacaatcattccggcctcccgcaagcgggtagccaaccgggtaaagtcgctgtcgctggatacgaggcaaaagccatccaccctgccggtatacagtatatccatcgcatcaatgatcatagcggaatcggtcgcatttttaccggaggtataactgtattgctgaatgggagtgatcgcatagtccaggagcacccctttccatcctaccaccgtgggttttgtccagtcgccgtaaattcttttaaaggtaggattaccatacttggctatctcttccagcatccctttaatattatgatacgggatgttgtcagcgtctatcagcactgccaggcggaggtctttcgtggtattatccattgttttaatttttgggttgaaggggaacaccaacaaatgtagccaattactgaaaactaaaaacgtgccggctgcagttatttactgccaccagcacgtcagttacttcaagtgatctgtttagctgaggtatgcgcggatcatccaggccagcttcatgtgcttttgcagcatttgtgtggcaaaatctgcggctcctttatctttatatttctcatcgaattcatcgataagcctgcgcaggttacggataatggtttcatgatcatccagtaattcctttagttgttttttctgatcgttggaatactccgactccagcaggttggtcagtttcaatacatctgcatagcggccttctgcataatgtcccaatgaacggatgtattctgctacttcatcgccaaagtcctgcagctcttcatattgtgcttcatagaacttatgcatttccatgaaattacttccttcgatattccagtgagaattgcgtgttttagcataaatcagtaattcgtcggccagtactttattcaattctaatgctatttgttttgtgttttctgctgaaacaccaatgtttgctttcatatcattgcgtttttttggttactataaatttaatatttccctggttaccgggctatgatgattatcataatttaacaaccggttaatataaacaggctactgctgatttttgttcatgagatcgccggggtggcaattactttgctaaaattgtaccatagttcctaattttgtgtacatgtatcagtcgaaggaaagcatctacacgctgcattttatactactttgtcttagcaatgcgctcttttctgccagcttcaatatgatgatccctgagctgccggcctatcttacccggatgggtggcgcggattacaaaggatatattattggcctgttcaccttaatggcggggctgtcgaggccattcagcggtaagcttacggatacaataggacgtgtaccagttatgattttcgggtcgctggtatgtgtagtgtgcagcctgatttaccctttaatcagtactgtaggcgcattcctgttactgcggttcttccacgggttttctacggggtttaagcctacgggcacttctgcctacgtatccgatatggtgccggttacgcggcgtggtgaggctatgggtatggtagggttattcagtactatcggtatggctatggggccggctattggcggatacgtggcagtacgatggaatattaacatcatgttccagttgtctgcggtgtttgcgttgttgtctgtagttattctcataggcatgaaagaaacccttaccaataaacagccgttccggttttccctgttaaggatctccggcagtgagatttttgaaccattggtttggtcgccggtgatcatcactttccttacttatttcagttatggcgctattctcactatcatcccggatttcagcgcttacctggggataagcaataagggtcttttctttactttctttacggtgagctctatcgggatccggctattggcgggcagggtatcagatcagtttggccgcgtacctgttttaaagatttcagcgctgatgatggcaggttccatgctgatgatggcactggcgcacaatagcatattactgctttcctcagcggtggtatatggaatttccgtggggctgaactcccctgccgttaccgcctggacggtagatcttggccggccggaacaccgcgggcgcgcgcttgccagcatgtatattgctatggaagccggtattggccttggtgcttacttttcagccttcatctataataatcacgcgactaatttccctcttacgttctatatatttgcgggcattacgctaatggccactttatatctcagttttatttataagccccggaaggccgcagacgctattcactaacatctgcatcagcaatcccggttgcaggaattacggtaatctgctcttcttcctcaggcaatgacaagtctgctgccggatctgacatcaaatcttttggcagcaccttcttattatcaagccccagtttccgcattctttcggcgcggcctacgagattgccattcccggtggaaagcttattcatagcgctttcataaacattctggctacgtttcaggtgttccccgatcaggcccatatcttctgcaaagcctacaaacttatcatacaaggcgcttccctgtcgcacaatttcttccgcattcttattttgtttatccagccgccacatattatcaatcacgcgtaaagtggccagtaaagacggcacgctcaccagtatgattcttttacggaaagcgaaatcatacaagtcctcctccacctgcataatggccagggcataagccggctcaataggaataaacaacatcacaaagtcggtggtgttcttgtatagcgtatgatacgctttggcgctaagttccgttacatggttcttcaccgattgcaggtgcatcctgagggcatgctttttttcttcttcgttggtggcactgcaatattgttcatatgccttcagcgatactttggaatcgatcaccagttgcctgttttcaggcaattgcaataccaggtcgggtttcctcagttgccctgtttcgtcacgctgcgcatcctgggtaaaataatgcactcccttttccaatccggaagcctccaataccctttccaggatcatttccccccagtttccctgttttttagtgtctgccttcagagcgttcgttaagttattcgcctccttggacaatgtttgattgagcagtaacagccgctgcaactcattcttcaattcggtgcgctgcgccgtttccgctaccagcgattgctgcacactactgcggaagttatcaattttctccgccagcggcttcagtacgtcgtccattttcactttgttctgctccatgaacgtaccggaaatacggtgcaacagctgctgcgctatattctcaaactggattttaaaatcctgctgtacctgttgcagccgctccttttccccgctcaactgcagctggagatatttattctgctccatgatacggccctgctccgacatcagcaccgaaaactcttcgtttaaccgttccagttgttcctgcttctcttttactaacatccctttatcatccagcatattctgcaggtactcctgccgggcctccagcaggttatatttttcctgcagggccgcctggctggcttgccaggcctgctgctgctgcgccagcactgcttcctgcacccgctgctgctgtttagccgcgaataaaagatagccaagcaccagtatcgcaattcccgaaatgactattagtatgatcatgataatttcctctgaaagcaaaataacttattactacgcactgaatctgcgttgcggtgaacagataacttcttcaaacatcattaaaaaagcaggaacaaccggaaatgatccgcccgttcctgctttcaatattataaaccctgttataaacgttcgtacagcttacgcagtctttcgcgggtcatcagctgctgccagtctttacccagcgcgttttcccacaatggggccatacccagcgatacattgatcatggtttcaaactgctcatctgtcaagcctttggtgattccctgcggaatatcaatcttatgctttttcaccatctgcttgaactttatcactccctcaggatagaattcttccagcttatcaaacacaatacagttaccaataccgtgcttggtacccaacaggtaggccaaaccataactcacggcatgcgccacacccacctgggaataagcaatactcatcccccccgcataggaggccatcatgagtttctcgtcggcatcgtcatcccattcatccttttgcaggaaaatttcctcacacagctcctgtgccttttcaccatatgatttactgaacgcattcaggtaagtaccttccagcgattccacacagtgaataaagcaatccatcgcagtataaaaacgctggtttgcctccacggtgctggtcagcgcagggtccagcacaatctggtcaaacggcgtgaagtcagaattcatacccagcttacgggttggtcccgttaacacacaggtacggctcacttccgctccggtaccggaaatagtaggaatacccactttatatacaccggctactttcacaagatcccatccctggtaatcagcagaagaacccggattggtcatcatcagggataccgctttggccatgtccattacagagccgccaccaataccaatgatcccggataccataccgaattccgctttgagctcatcacggatcttatcaaccgtttttgttttgggctcatcggtcacatcaatcaccacaattttgtccttgccttccagcggaagacgggccaaaaaatcattcttatcctggaagtactcatccacgaagaatatcatgggagcatcgcctatgcgcctgggggccagtatttcacccagctgatcaaaacatccgctgccgtaaactacatagtccaccattttaaaattcctgaatttcatatatccgtgttagttaggtattataaaagttttgctgccttttccaggtcttccggcgtatctatttccacgcccatataagaagtcactaccattttcataggaatgccattctccaggtaacgcaaacattcaattttttcggccgcctccagtggcgtcatcgccagctgggtgaaatccagcagggtttgtttacggaaggcataaataccgatatgctcgtagtaaatgcttctgatctctttattccgcggatagggaataacggagcgggagaagaataatgcgttgaagttcttatctaccgccaccttcacgtaattaggatcttctatggatgcgggatctttcagttcctgcatcagcgaagccacctgtactttctttccttcttccccttcaaataccttcaacagcttttccagcggctctttctgtgtaaatggctcgtcgccctgcacattcactacaatatccacttccatatctacaacggcttcagctatacgatcggtaccgcattcatgctcttttttgctcataacggctttgccgccgttacttacaatttcattatagataagatcactgtctgtcaccaccattacatcgtcgaaaacaccggtgtttactgcagattcataggttctgagtatcactgttttatcccccagcttagccatcatcttacctgggaaacgggacgccccataacgggcaggtatcaacgctatttttctcatgtagtatggttttaactgcaaaggcgcaggcaacaaatatacattgctgcccggcgccttcaccagatcaattataatgcgcttttaactgccttcaccagtttctctgctctttcccggatctcttcttcgctccagcccaggttaatcggggtggaaatgtttcttccgatgatatcatctgaagcagggaattctttggttttgtaaacctccattgcctgtttcagttcttttgcaaagggagttaatacatgcccttctttaaaatgctgccactggcggatgtaatgccagttgttatcataataatggaaagcggccagtccggcggctttcattgcagcagctgcttttgctgcctgggctgtttccggcaggaaaaacgacaggaaggtagcgctgtcgccggcttcatccggcaaccggcggaaggttacacccggcacagtggccagtgcatccttgaatattttcttggtcttacgctgtatttccaggaacgtatccagcttgcggatctgcgccagtcccactgcagcatgcaattcggaaatacggtaattgtaaccgataaatggatgaaggtcagcgccacggtctaccccgaggtgatcatgaccatggtccgtatacccgtcacatttagtataaatgtctttattattggtaatgatggcgcccccttctgcacaggtgatcgtttttacgaaatcaaaagaaaacgtaccggcatcgccaatggaacccagcgcttttcctttataggaagcgccaaagctctggcaggcatcttccagcaggaacaggttatgctttttacaaatggcctgtaacgcatccagatcggccattgcgccgcacatatgcaccggcattactgcctttgtacggggagtaatagctgcttccaccgctttggggtccagggtcagggtatcgtccacatctaccagtaccggtgtggcgcctacggaaaataccgattcaaagctggccacaaaagtaaaggtgggcataatgatttcatcgcccgcgcccaatcccagggcagccatagcggtggttaacgcggccgtaccactggaggcaagctgggtatactgtacattcagtttatcgcaaatagcctgttccagctcctttgctttccagatgcctttacgcggaccgtcgaatccgtaacgcatcattattcctgtttccagtacgtcgtttacttctttcctttcctcggctccaaatagttcatatccgggcataaactgttgattttaaaatataatttgaatgagtgctttttcaatagtgctgcaaagttactataataggcattgcgttacatcggaaaaactgtttatcttttgctaaaaattcaccatgcgttttatactgttccttaccctgttgggggttttagccggaatgcccgctcacgcgcagaaagccctgcccgccgatcagcaacagattgctgcactcatggccacgcaaacggccgcctggaataaaggagatatcgacggcttcatgactacttactggcattccgattccctgctgttcatcggtaaaaacggggttacctatgggtggcaggccacgctggaccgctataaaaaaacatatccggacgccgcggcaatgggcaaactggatttcaaattgctggaattcaagcccctggcttccgatacctacctcttaatcgggaaatggcacctggaaaggactataggcgacttacagggctacttcagcctcatcttacaaaaaataaaaggacaatggaaaattattgctgaccatagcagctaaaaaaaccatcccaggaataggatggccgctatacaccacaacattaaagaagttctggacttctttttctttagaagtaaagtttaaaagttttcatctgatatggtaaaatgttcaatgctttgatttcttactggcttcactatccctcaccgctttgttctccttttcaggtttatcagacaaatcgccatgtaagggattacggttagtagtgcctttatcctggtctaatatgtctaccggtttcttcttcctgtcacgatactcaccggtatgatctgtttccttctttttcataatctctttttttgaagatgaaaatatgggagatacaccatgggaatcacaaacactattccaccctcaaaacaggccattttgacgagctggcgaagggtgtccggggcatcagttccacaaaaccctgatgcacagtgagaaagaataacaacacaccggctgcggaaatattgcagttctgattaacattagatttacaaaaactatgatcattatctcatatctacgcactatcttcgatgcctcaaacaagttttaacccgtaacctctgatcagccacgagtagttttaatcaagttcctgcctaaagccaattttttagttttaatccaagtcctgtttagaacccggtatctatttactataactaattactggttatgcccgggaaaattatgcgcgttgccaccgctctgatggctgttgttatttattgcagttgtactaaaaagactgacctggcgctggatacgccggaaaaaacacctcctgcagatacgtcggtggtgcccgaaaacaaagtggaccgcaacgccctcttactgttggtaaacggattacgcaaccgtggctgtaactgcggtacagaatcgatgcctcctgtaggcgcccttacctggaatggcctgttggaaagagcggcttatgaccacagcaaagacatggtactgaataaatatttcgaccataccgggctcaatggttccacacctggttcccgcctcgatgtagccggatacaaatggacctattatggagaaaatatagctaccggcagcctgaacgaacaagccgtgatacttggctggctaaacagtccgaaacattgtcacaatatgatggatgctaattttaaagagatcggtattggtcgctataacaacgactggacaatggaattgggcaggaggtccgttgccaactaaatcagggggcgctcatctttttgcgccacatacgccatacaaagtaaagataggctgccatggaaacgccaaaccagctgtagaagaagatcatcctgccaggagtagactcctccggcacagcaaatccaaggtacaacccgaggaatacattgatcatcaaccagaaaaagccaataaagatggtccgcattatttttatgaggaaatgaaacaactcataatccatcttattgggatccggcgccggtttttcctgttcttcttccataatcttttatatcagcactactaaggtatgcacagtttggcaaggtctgtactgtcgcccttaaatacattaaaatccacagtggtccggatgccgtttacccggccgatgtcgctgtgctgccaaaacaaccaggccctgtcggaacgcggccgctccttctgatagtaatgcgcgatccacaaaggatagcgatcaaattcgctgccaagataggtttcgtaaaaatgaatgttagtgtagatgatgggttttaccttgtataccttttccatttcctccagccagattttcgccgtgctgcggataacggcggcaggctggttgttgctggtttcgatatccagtaccggcggaagatcccctgactgcaggtcggccacattgtggaagttaatggcttgcttcaacgggtcacgggtagcataaaagaaatggtaggcgccccggattaaaccagccttacccgccttgtcccaatttatcctgaaggcggcgtcctgccgtgtaataccttccgtggcttttataaaggcaaaggatatacgaattttatctacctgcatttgttttactgccgcccagttgatgtctttctgaaatttagaaacatctatcccatgtatcttataattcaccggcatgtcaattccaaactcttcatagcgtacaaatttcacttgcttttcccgctggcgccaccataaataagccactgcggccagtactaccagtaatattaataataatcggatccggatgcttttcacttttgcttctgttagttgcagggtaattgggtaaggatgctgtaataaatgccggcagtcctattttttacagcaagtataggttataatttgtttaaagaagctacttttacagcggtcaagtgattttttatgcccgattttaacctgaaggatacccttaatttgttttcaaagtttacactgcgccgcggtttaaatgccggcaaagtacttggaagctatttcatgagcaagtggaccaacaaaccggttcagtggggctatcctatttctatatcttttgagcctactacgtcctgcaacctccgttgccccgaatgccccagcgggctcagggcctttacccgccctaccggcatgctggaacaggactttttcaggaaaacgatcgatgaaatttccaaagaactgctatacctgatcttttacttccagggagaaccttatctcaatcccggtttcctggacatggtgagatatgcagccgataaaggaatttacaccgctacctccaccaacgcccactacctcacagacgccaatgcgaagaaaacagtggaaagtggactggacaggctcatcatctctatcgatggtactacccaggacgtatatacgcagtaccgggtaggcggccacctggataaagtgatccagggtgcaaaaaacatcgtaaaatggaaaaaagagctgaattcatccaagccttttgtctttttccagttccttgtagtaaaacccaatgaacaccagatagaagatattaaacggctggccaaggaaataggcgtagaccaggtgcggtttaaaactgcgcaggtatatgattatgaagaaggcaaccgcttaattcctaccatcgataaatactcccgctaccatcgcaacgaagatggtacctacgccataaaaaacaagctaagcaatcattgctggcgcctgtggcattccccggtggttacctgggatggcctggtagtaccctgctgcttcgacaaagatgcacagcacaggctgggcgatctgaaaaaagaatccttcaaaacactgtggcataataaagagtatatccgtttccgtagccaaatcctcgaaacccgcaaaaacatagatatctgcgctaactgcagtgaaggcaccaaagtttggggataatcacctgctgcagaatttttttctcattgacattcaatccattaactacatttatagtttaatactacaaaaatagtttttaaactacagaaatagttatagattagtgttatgaaaaagctatcccgtaaagaagaagaattaatgcaggtaatgtgggatctcgaaaaagcatttgtaaaggatgccatcgagcagctccccgacccgaagccgcattacaacaccatcgctacgctcatgaagcgactggaagataaagggtatctcgcccaccatgaatatggtggctccttcgagtattaccccaccattgcaaaggaaagttataaagacacttttatgaaaaaggtactcaatactttctttgataactcctatctcaatatgctggcttatttcgctaaggaagaaaaaatcagtgcggaagacatgaagacgctggtaaagatgatcgaaaaagataaaaaataacgtgtatgcctaccctgtttatatatattctgcaagcatcctgtgcaatgacgcttttttatctcctgtatatcagctgttttaagaaagaaacattttaccggtataacaggatcgttctgctgagcgctttcatattctcagcgatattgccgctgcttcccctccctgcatggcaatggacgcaaaaatcaacagaagccgcaacaccggtaagcgtttactttagtgataacgcgcacgcatctacgccggtaaccggtgtcgcagtggaacaccactggtgggacccgctgatgcagcatggcggtaccatattggtagcagcatacataacaatagccgctttcctgctgttgctgcatatactgcagctcttaaagattcgccgcctggtgcgggcaggcaatgtatacatgcgtaataacatacgttatgtacagctccccggaataacagcgcccttctcttttctgagaaccattttcttcgatcctaacgcacatgcccatacggaattgcaacatgttctcaaacatgaagaagcgcatgtacagcaataccactctgctgatatgctgctatcagccctctactgctgcatttgctggatcaatccctttgcatggcgttgtaaaagagcgctgcagctgaacctggagttcctggcagatgaagccgtcatccaaaccaccgacgccccggatgcctaccagtacagtttactgaagataggcctggccggcagccgcgtaaccatcgtgaatcatttcagcaaatcattcattaaaaacagaatactcatgatcaacaaaacccaatcaccccggctacgtacctggcggtacctcctgctgctgccggtatttgcactggcagcgggccttctggcagccacttctccatcatcaaaaaacgacgcgggcactaaatacctggccacagaaaacgaccggctctatggagtggttacgccattaacttctgataaggacttcgcggagatgaaggatgcattggaaaaaaaaggtataacgctgaacatcccgaccctcagacgtaataagaacggggaaatcacagcaattgatttcaaactggtgtcgggtacctggtcaatgcgggaaacaatggaagttccgtttacaccttatttcttttattgtgctgagaaggaaggcggaataggtccttttccaatgaagaattgcccccggcacctgcaggaccttgcattggcagaaggtaatggagccgctaaagggattactaccgactccacctttttgaatcgctttccaggtggagagcacgcataccgcaaggtgtttgcaaaaaatgtccgctatccgagggcaagccagcaaagcaaaacggccggtgtggtcaggctgcaatataaaattcagcccaacggtgtcatcaataatatagagttgctggaaacgccggataaagcacttggcgatgaggtaaaacgtgttttagaacagctccctacctttgcagcggatccttcggggaaaactgttaccgtttccctgcgcatatcatttatgctggataatggcgcaggtggatttattaaaggatccgacgcagataacgcggatataattgtagtgggatacctgccgaaaccgatttcctttattcagccactgtctctttcttttttcgacgacccttcgtcaccttgttaaacaggttgatacctagttgaacacctataaactcaagtgctgtcattaatgccccggtagcaaaattcttaaacttaccacttccccaggccatcttagccacattcatggctacgttcagggcaccgctatgttttgcgctaccggggataacagcattcagggccatctttttatagttgtccctgaaaaaatccaccctgtttcccatttcattttccagctgcctggacttcatttttagccgggtaatttccagctccagtgattcgaagctgtctattttcttactcatgtgtaaacatttatcattgtttatcctttcatggtgttttcagtggcttcttcatcaggaacataccccgaatctacaggttgctccggatgttcctttgtccgctgattgtgaatatgattggaatgctcatcctggtccgtaatttcatctaccagttcagtaatcagcaatttagccagtggccgctgtatcagctgcttacggaacaataaaataaccaggaataacaatataaataatcctgcagcacagctgaaaccaatggtaaaactattggtcatttccccgatccagaagcctactaccatgcccaggaacacaatcacaaaaaagaacagcaggaaagccatcaaaagagagaaaaacaatcccaacgcttttgacagctttcctgctgcctggagcttaatcaggtccagtctggtttccaggtattccctggctacttttcccgtttgggaaaaatagttgctgaaattatcttccatgcaaatcaatttattcaaatggggttatgccaactcattctctaactcatcctggaactgatctttcttctttctccatttttctttcagcttttcagactgatctcttaatttttctaccagctcatcttttttatcggaattgaggaaataccctactgcaacgcccacggctgcacctacaataaatgaaaccacggctttggaactgttactcataactaaaggtttttaagatgttataaattaggttttcttttttggtaacagaggtgcaacaaacattattccataaatgacaattgaataaaaagctgtgttaaacctccgccaaataagaacaagctctccgtaattttgtttagggtttataaaagtataacggtgcggccggtctgttttttgacataccggataattacacgatattatgtactatgagctatcttgacaacgaccgccttaaacaaattggctttttactcctgatcctatttcttgctgtgctcctgtttatggagatgttcaccttttttcccggcttcctgggagctgttaccctgtatgtaatcagcaggaaatggatgttcaaactggtagaacaacgtaagtggagaacaaatcttgccgctgcactgctgatggtactctccttcctggtgatcctgctgcccataggcatgctgataaacatgctcggggctaaagccgcttatgccgccaaccactccacagaactcatcaacagcctcaaacaaaccaatgcccggctggaaaatagcctgggattcggcctgctcaccgcagaacggctgcagaaaatacaggaaaatatcaccgcctttttacccgggttcctgggcgctaccttcaatacgcttactaccattgccctgatgtatttcatgctgtattttatgctggtaaacggccggaaaatggaagagaacctctatgagtatattcccctgaaagataaaaatgtggaaagactgggtaaagagttcaacactttggtaattgccaatgccgtaggtatccccctcattgcggtggtacagggtgttatttctctgatcggctatttaatttttggaatcccccaaccttttttctggtttgtgatcacctgttttaccgcaatgttgccggtgataggcgccgccgctgtgtatgtgccactgggagtttatttactggcttccggcagcacctggcagggcatagcggtgctggtgtacggattcggcgtggtgggcacctccgataacgttgcgcggatgttgctggcaaagagaattgcagacgtccatcccctcattactatattcggtgtaatcattggcgttagcctgtttggtttcatcggcctgattttcggccccttactcatctctatgtttatccttttgctggatatttacggaaatgagtttgtgataaaaagaagggatatcgcgcagaagaaaccggccaccgatacagatgtccgcgatacgcccggaacaaggtaatcagcggtaataattattttcggagatataattaatcacattatcaggtaccataaaacggacagattttccttctttcagccattttcggatatctgtagcggagatgtccagcataggcgcatccagtatttcaatccgggcgccaaaggtgtctgttatttcatgccccggccggcggtaaacatagatcggataatttttcacgatctgttcgtaatttttccagcgcggtaaattctgaaagctgtcgcttcccataatgatggcaaattcctgtgttggaaatttctcctgcaaatacgtgagcgtgtccactgtataggacggccggggtaacgaaaactcaatgttgctggcccgcagccgcacttcgtctttgatggccagctccaccaggtgaaagcgatcatgttcattcagcagggccgactgtggtttcagcgggttatgcggcgaaaccaccagccatactttatcaagatcagtattgtgcgctacgtaattggcaatgatcaaatgccccgtgtgtataggattaaaagacccaaaatacaagcctattctcatgttttcatcgtataaattgccaatggctacttcataatgcgtgtaaaaataggtatttatagcgggaacatggaaataaggcttattccagtggtttgaattgttcaaacacctggccgcagttcttgcaaaaatggatcgcacggcacaacgtagagccgaaaggagaacgtaaataagtttgttcgctgccgcaatgcgggcagggaacctccatcataagttctgggcttacctctcccgtcaatactttgggaggggctatgccaaaggttttcagcttttccttggcggcaggcgtcatccggttgctatgccagtgctcctgtttgtccacttcaacgctaacggctataccaagttctttttccagcactgttttaatgttatgccggatataactcaccgccgggcaggccgcaaaagtgggaatcattttaatatgcaccgccgagtcattcagatccacaccggtgatcattcccagatccactacgctcaataccgggatctccgggtccatcaccgtttccagtgctgcatatacatcggctatcgtaattgttttggaagacatcatttaccagctggcctccgtatccaggttaaacacttcactcatttctctcaataaaggctgcaggtgcggcgtatgaagtccatgacggccgccatacaccggaacaatagcacttatctccggcaggttcagggaggcctttaccaataccgggtaaatccgatccagccagcgatggtacaatcccgtttcaccaggatataccttgtcttcaatcaaagcctcttcatatagctgcgagggttcaaaaattcccgccgccagtgcaatcgtttggtcgagcgcctgctgcatacggtcgtagctttcttctcccgcccggctcagttgcataatccatgcatttgcatgcagcgtatgatatttcagctccccctttacttttttgctcaatagccggaaaggttcataactgctgtcctgtaaactttcataacggactgattcggccaggtcaaataaaaagtgccgcatcaggctgaaatcatattcaccattaggcatctctaccaggtgcgacgacttgaattctttctccggacggagaaatgcaaatgtatccggatcttttcctccgagatcttcatgaagcatgcgatacaacgcccatgcatggcctattttgtcctgcgccatggaagaaaaagcaatatcttcttccatcacaggtcccaatcccgtccactcagaattacgatgtccctgaatcagttcatcgtctgccatttttataatcaggtctgttagtgctgcgttgttcatttggattgtttgaatttattgatcttctccatcactttaaagccactggcatcccggtaggttttctccatattgttggcaaacatatcttcatcttccacatcaaaggccagaatgtctgcacttttcacgacccagagattgacacattttttccggcgggcaaattgctctttcgcaaaaaccagtgccagctgcgggtccggcgcatgtacacagcccacgtgctcatgatgagcgcctctcttctcctggtgaaatacctcgtatatgttccagttctctccctcctccactttcactacttccccggccgggcccagtttcagcctgtttacacggggatctaaagaatcgttagacatgaatatttgaatagttttaatgataaagtttgatgccgctttctctgccggcacatcctaggccaccggcaatacccgtttttctgttggtttcatgagcgctttgcgtacccaacggcccttttcttctgcccacttgcgcacctgcagccgttccatattacagggtccgccgccgttaatcacccggaaaaactcgtcccagtcggggtccgtgtattcccaacggccggtctccccgtttttgcgcagcgcaggatccggcagagtgaggcccagctcccagatcttaggcacataggactccaggaattgattccgcatatcatcattactcgccattttcactttccattgcatcagtttttcactatgactggaacttttgtccggaggaccaaagaaatgcataataggctgccaccagcggttgagggcatcctgcagcatttccttctgcgccggcgtacccgttgccagttcaataaaagcgtcatggccctgtttgaggtggaagctttcttcgtaacaaatacgctccaatgccctgcaatagggaccatacgaacccttcgcattggcaacctggtttacaatggctgcggcatcaatcagaaatccgataacagctacatctgcccaggtttccgccggataattaaatacgttggagtacttggatttaccgctgagcaggtcgttaatcatcgcctcccttgatttaccgagtgtttcggccgcattgtacagtaactgcccgtgccctatttcatcctgcactttggcgattagcgccagtttgcgcttgaagcccggcgccctcgtaatccaggtgccttccggtaatgccccgataatttctgagtgagcgtgttgttcaataaggcgtattaactgcctccggtattccaccggcatccagtcgccgggttctatcttttcccctctggcaatacgttcctcaaaagcagcgagcttttccggctcatcatgctgctgttcttcccgcaactgatttctgttgggttcgtcgaaaatatatccaccgccgtacatagtgcgattgttttggtcgctagtaaattacggaaaaaagaccgtttcagcaggaattgattgttaaaacagcggtattcaaatgttatagaatcgccaaatttttccgtcatgaaacagatagccggccattcccttaattttattaccttctaaccgataatgctgtctgctgctaccatactgagctttttgctattgttcaccgggcataaaaatccacgcccggagggccggcattataccgtcatacagctgaatttcgaagaaaaacaaacgcccgcaccgcccggatccgatactatttattatgatttcgaaagaaaactgcaatgggaggattttcaggcaaagccttcgcccaacggccccagcgctgcagtttcctacaccagctttgcctatgagggcaacagcaatctcgtaaatgataccctccggatcacgctaaaccttcaggtgttctttataaaaagcgcgtcgtgggtaaggccggaagcaaggaacagctatgccctggcacatgaacaacttcatttcgatattacccgcctggtggtggaacggtttaaacagaagctccggcaaaccgcattgaaccgcgacgactacgatagtatcatacaatatcagtaccttcagtctttccgggagatgaaccgcctccagtaccgtttcgaccaggaaacccaccacggactgaacgctgcagaacagatccgctggcgggataaagtaaatgtgggcctgaaaaacaacggcgtgcttccggaagaactgggtattgaaggcattaacttccgacccatacaataacaacccgttttaacgtttattcatagcggttatgcagcataaaaaaggatctatgcaaccaaataatttttaccactcattgctcactggcttagtgctcatttttttgatgactgcctgtaataaaaaagatagtaatgccccgcgaaaccgcggaggtgatggcgtaaccggctccgtcaacgacagcgtctttttcatcgcaaaagatatatacctctggaacgacgttttgcccgactcggcaacattcaaacccaatcaatatgcaaatccgatcgtgctgtttaacgcattgagaacctataaaaaagacgcttccggcaataacctcgacaggtacagctttgtagacaacggcggcacctccagggccttacaggaaggaattgcgggcgatatgggctttgaagtcggctatcaaacagattctaccttgtttgtggtgtatgtataccccggctctccggccggtaaagctggtattaaaagaggctggcagttaattgacgtaaatggggttacccgcttccgggtaaatgatggtactacggataatatgctgaataccgccttcggcagcgccagcgcctcctggggtttccgtaaaccagacaacactacccagcagtttaatttaagccgtgtagattataagctgaatcctattctttattctcacttatatgactttaacggcaataaaatcggctactttgtttttaataacttcgtagcattatccgacgtaaaagcgcagatagactcaatttttgatgcttatacaaaggcaggaataaagcaggtggttattgatctgcgatataacggtggcgggcttattgaaacagcagaatacctggccaacatcctggtgcctgcagccaaaagcaataccaccatgtattcccagtatttcaataacaacgtgaatactaacaattatggcccctacttcaaatacatgaaggccgtaccttattatcccagcgtaaactggtcggatatcttctacagcgaagctactacctataaaacagcgaagttccaaaaaagcggcgcacttgccttaaacaaagttacattcctgggtacacgtaataccgtatctgccagtgaactgctgtacaatgtgctgaaaccggtaatgaccaccaagctggtaggaagcaacacttatggcaaacctgttggtttcattaatatctcttttggtaaatatgatatgtacgcggttaacttccagacaaaaaactcggctaacgaaggcgattatttcagtggccttccggcagatataaaagcagaggatgatttctcgctcgactggggcgccctcagcgacccgttattacgcgcggcactcattgatatgggggttgacgccggttcactgggccgtgcagcaaaattaaacggaaacaggctggctgtaacacctgccaacaggctggaatccactaaatttaaagggatgatacaaaccatccgccaatagccggtagtttcttttgcggaactaccggacttcatttttacatcgttttagcgccgctatatttgttctccggcatatcgctgtccagtttcttcaccacttccagcaccgcctgtactgccctgtaatagaaagaatgattaatgcgcgaatattcatcagagagatgatggtaatccgggtgatcttccacgccgaagtacaggaacgggatcttttgtttaaagaattcatactgatcgctctgtttcgtccagtcgtctgtaccactttccggtttatcatgaccagctattagtttcacgctgctgcgggcagccacatcatcggtatacttcttcagatccggaaactggaatgtgccgcatacatacaattcgtttttgtcgttatgggcaatcatatccatgttaatattctgccggatttgtataagtggcaccggggactgtgctacaaaggctttagctccctgaagtccttcctcctctccatcaaaagcggcgaaaataagggtataacggggcgggtgcgttttaaaataagcagccattgccaataatccgcctatgccggaagcgttgtcgtctgcgccgttatacacggtatccgcaccatttgttttggaggtaataccaagatgatcataatgcgcagaaataacaatcactgtattcagcttaccggggatatagccgtacaggttagtccccataattttcttatctccttcctggaaatagaaaggatattcgtaggtatcgtgataagcggataagccaatttttttgaagcggtcgaggatataaaattgcgccatacggctgccgcgggtacccgttttccggccttccatcttatcggcggaaagcgttttcacatctttcatcaattgcatggaatcaacggaagtttgcgcaatcgcaggcagcgcaaaaagcaggcaaaagctgtaacaaagccatttcataaacattgcatttatggttaactatacctgcaatgtacaagatattatttgaagatattaaagatgatcaaactgcacacataggccagtgcagtcatgtaaacaagttgtatcagcgggtatttccaggatttggtttcacgttttacaatggccattgtactcatacactgcatggcaaacgcataaaaaatcattaaggacaacccggaggccagcgtgtataccggcgctccgtcaggccaggtagccgacgacagtttttcccggagagtagcgttattgttatcaggatcttctcccacactatagagggtagccatagtacccacaaacacttcgcgggcagcaaaagaggtgatcagtgcaatgccgattttccagtcaaatcccagcggacggatggccggctcaatggcatgaccgagtacccctgcataggaattggataatttggcagattgaaattccttattcaacaccgctgcttcgggagattcagcaggcactttcgcgagaagttgttcatatttggcatgtaccggttccattctgctggcaggaccataagaagccaggaaccagaggattacagatattaccacaatcaccttaccggcgtctttcacaaatattttcgctttctccaccatggtggttcccacattggcccagcgcggggagcggtaaaccggtaactccatgatgaagtaactcttttctttgatgcgtacaaacagcttcatgatagccgcaatgaagatggccatgaagaaacccagcaggtaaagccccatcataataagtccctgcaggccaagaataccgaagatccgcttgtcggggatgaccaacgcaatcatcatggtataaataggcaacctcgcagaacaactcattaaaggcgttaccataatagtgataagccgttcctttttattctcaatagtacgggtggccatgatagcgggtacagcacaagccactccgctgatcagcggcatcactgactttccgtttaatcccacctgccgcatcaggcgatccgtcaggaaactgatacgggccatgtagccagtatcttccagtatggtgatcaggccaaacaggatcatgatctggggaataaacacggcaaaaccgctgataccagccaggatcccattgatgaagaagtcggtaactttattgtcggggaggatattgctcagccatccgctcagcgcgccaaagccgccttcgatccagtccatggggtatgaagccagccagaaaatgctttggaacaggaggaacatcactaccagcaaaattacgtaaccccagaaacggtgcaacaggaggtcgtctattttttcagaacgcaattgcttctgcagcggatcattttccactaccgtcgctttcatgatatgtttgatccggctataccgctgcatgatctcttcggcctgaatctttgttttattaaactggtatgtttccagtgcgccatgaatcgcctttttctgtgtaatgtctataaaaggcagatcgtctacgttaacggctatatgtaaagcgccgtaatcacttttcaccggtactgttttacgtacctcgtcaatcacgtctttagccagcgcgttgttattaataaaatccctgggaggagtgctgtaatgggaacgcatcgacaggtctattactttcttgatttccgtaacccctttattttttcttggattgatggctactacgggtacgcccagttccctttccagtccgtccaggtctatctccactccctttttacgggcaatgtccatcatggtgagggctataatgaccgggattttgagatcgatgatctgggaacagaataacaggttacgtttaaggttggaagcatccgctacaatgatcacgaggcggggggtatcttcgttttgctggttaatcagcacatcataggtaacatattcatcggcgcttttcggatacaggctataagttcccggcaggtcgataatattggctgttacgcctgatactatctgagctatcccggtttttttatctaccgttacgcccggaaaattacccaccttctggtttaagccggtgagcgcattaaaaagggaacttttaccactattcggattacctaccagcgcgatgtttatgggagcctgcattccttatcttatcctatttattaatattaattgctgaagatgcaaagttaaacattaatcagccggcggaatgatccgatcgggaaaatctcagaatggtaatttgccggaaaagataaagcgaaaacagtggcttgttttcgctttatctttttaaaaattaattatttatatagattaactgtgaaacatgttaatgagggaataagccaggaaagatacatcgccttcgatgggctggttctttttcaccgctttaactgcattttcagcggcgggtcccttgtaacggtagccttcattggaagagtcggtattcgccttttccggcgccggtttcttttcgttgacgtcgtcggtaccatcgggtgtcattttcaggttcaatggtccgggctggtcattatcgaaatcgttatcccagtcgccattgtcgttacggtcgtaccggctaaagtcatagttacggtatacttcgcggtctatttcaatattctttcctaccggtactttaatggttactgtaatacgctgaccgcggtacttggagtgcggcggcagggaaaacccttccggcaggtacaatacagagtcctgttggttcaggtggaacgctatatcatgagccagcatttttgcctgttgaacggtacggcccctggaaaagcgggatacatctaccgagaaactgtcggtcgggcttttttcaacccttatccggatgtagttaatcaacacggtatcgtctgcgatcagtaagtgatcatcaaagaaactgatgtcgtcgccattgatttcagacaggataccaggcgttcttttcagtatcagcttgcctttcgatggctgttgaatggctattgcttccgtttctgttgccggtcttctgaaatcttttacaaaggacgtagcaatgatggcggcgaaagtcagtccaagtaaccagaggaaggttaaggtataacctgcatagcggttgccttcttttacaccggtgagtttacggatgatgaatataaccagtgcaacaatcgggatgcctatgagcaatccaactgcaggccataacaatgcgctttgcaccggagcgccgagtaacagatccttgatgggaaaaagggccgcggaagtggctgcaatggctattcctgccactatcaggcagatcagcatcactacagcgaagaagtaaaagaaccctttggtaacagctaccaacactttacctaatccacttgccaggctcacaaaaaagcgttcgatatcactacctacctgcttgccgcggccctgagaaaaatttcggatatcatctcctacatttttcacctggcctttcatatgatttaattcttcctggatggtggacttgatagtgttcagatccaccttctctcctctcatttccagcttttccgctgccgtgtcggcagacggagttgctatccagaggatgaagtatacaaggataccggtaccaaagccaccgatcgccaacagggcgaatatgatacggaagatcaccggatcgatattgaaataagcgcctaacccgctacatacgccacttagcaccttattttccggatcgcggtacaggcgtttgcgtgggcggggaatatatcctgcaaacggatcgtcttcctttgtttgttgagtgctttcgccggcagcgtcgtcgaattgctctggtgtacccatggaagcttttactgcaattacatcttcatcagtaatacaatgagcgccttttttcaatttatcctggaatatttcagcaatgcggctttcaatatcagacacgatttcatccccgccttcctctttcgagaaatattttttcaggctcccgagatactgattcagtatctcatacgcgctatcctcgatggggataaggcggcctgaaaggtttatgttgattatctttttcattaccagttgattttaggttttaggttagtcttcctttacaggggtgtactattttgtgttaattgatgcaccgcattggccagttcgttccaggtactttccagttctttataaaaggtttcccctttatctgtcatggaaaaatacttccgtggggggcctgagctgctttctacccagcggtaagtgagtaattccgcattttttaatcttgttaataaaggataaagagtgccctccaggatatccagctttgcttccttcatcttttcgatgatatctgaagggtaagcttctccttgcttaatgacggacaatatgcaaaactccagcactcccttcctcatctgcgattgtgtgttatcaatgttcatggcaagtgagctttaatgtttttttctaatggtggtttctgatcagttattaaagtgtttgatagctattctttcaactttacgatacaaaaataggaaacttttactactatgcaatacacaataccatagaaagcaaaataacttgtttagaacgttacccggcaaagcctataaaacgcaatacagctgcggatcttacagaaaaatcaggctataacaccggctgcaggataatgatgaccggttttcagccgggataaacggaaaggaacagttggggccgcctttttatgttaaaatcctttaacattattttaattgggattttttaccatttatggttaacctctattacatttgcattaagcgtattatacacatgaagaaattaatcggcatattcctgctggcactgatggtgtcacaactgcttccgatcaaggaagtagggaagctgttatttaataaccagattgtggaagaacacccggttgattgtggtggtgatcatataaagattgcgaaagagctgaaattttgtaaacagtttgacgagattcagtttaacccattactcattcttggtattttacaatatcatttaatggaagatattcccagcaaccctgctcaggaaatacacgcccctcctcccaatacgcacatcgcgtaatttcgttttgcagttgtcattacaacagctgtttttctattttatttattactgattttttcaaacactgcccgcgctacgtgtatccattaaggcgatacctgtatgtagccgttaacggggtgtactattacatcattgtagcttccacggttgcagcattggctgctatccggaagtgtgatccctcaacggaaaagcaaattttatgaacaagcaaatatcaatattctccaatataaaaggcgatttttcagccggccttgttgttttcctcattgcggtgccattgtgcctgggaatcgccctggcctcaggagcgcccttgtttgccggtatgatttccggtatcatcggtggcctggtaatcggctttttaagcggctcgcaattgagtgtaagtggtcctgcagcaggtcttaccgctgttgtactggtggctatcaccaaacttggcgccttcgatgtattcctcctgagcgtggtaataggcggcgccatccagcttatactgggattaatcaaagcagggacggtagccaactacttcccttccaatgtaatcacaggtatgcttaccgctattggtatcatcattatcctgaaacagttaccgcacgcatttggctatgatgccgattcggaaggtgatttcaactttattcaggtagatggcgaaaatactttcagtgccctgctttccacgattaaccacattaatcttggcgcaacattgatcaccattatctccattctcattattctgtactggagcaagatcccgaagctcaatgtagtgccagcgccactggtagcagtaattaccggcatattgctgaatacagcattttccggcagtgagctgctggcactgggatctaatcacctggtaactttaccggtagccggtagttttggtgatttcgtgaaccagttcacgctcccgaatttcagcgccatcactaacaaagatgtttggattaccggcgctactatagcaatagtagcttccgtggaaaccctgctgaatgtggaagccaccgaaaaactggatcctctgaaacgccatacttctcctaaccgggaattgaaagcacaaggtattggtaacatgatcagtggcttaattggcggtttaccaatcacctctgtaattgtacgctccagcgctaatatcaatgccggtggtaaaaccaaactggcaacaatgacgcatggtgcattattactggtttgtacggccctgatccctgcattattaaataaaattccgctggctaccctggcggcagtattgctggtaactggttacaaattgtgcaaaatttccattttcaaggaaatgttcaaaaatggtaagtaccaatgggtgccttttgttgtaaccgtattagccatcgtgtttaccgatctgctggtaggtattgcattgggtatgattgtaagtgtgctcgccattttacgtggtaatatgaaaagctcttactatttccgcaaggaaaaataccacagtggcgacagcatccgcctggaactggcacaggaagtttctttcctgaacaaggccagcatcctgcttacgctggatcatatgcctgaaaatattacactggtgattgatgcacacaaaactgcttatatcgattttgatgtattgcagaccatccgcgaattcaaagacatcaaagcgccacaaaaaaacatcaaagtaatcctgacgggatttaaatccgtgtacaacattcaaaatacaccagacctttctgttgaagaacagtcgaggctgaattccccgcaggtacacactatttcttccggtaaccataaagagttactgaaagagctgcagttaaattaaaggcaggtacacctttaatgtaaaaacgtaacggaaaccatgcttacatccgttcatttttcaatttcaaaaaatgacaattatgaagacattgaataaaatatctcaagccaatatatctcctaaaaaagcactggaattgctgcaggccggtaacacccggtttgtggaaaaccttcgcctgaaccgcaacctgctgcaaatggtgaacgatacttccgacggacaatggcccatggcggctatcgttagctgtatggactcccgtacctctgcagagctgatctttgatcagggattgggcgacatcttcagtatccgtttagccggcgccgttatttccgataatgtactgggcagcctcgaatatgcctgtaaggtagctggctccaaattcatcgtggtgttgggccatacgaaatgcggcgcgatcaagggtgcctgcgattccattgaaatgggtaacctcaccgggctgttaaacaaaatagccccggctgtatttgcagagaaaactattaaacaggaccgcaactcccataacggcgaatttgtggaagcggtaaacgcgatccatgtacaacgctctgtgcaggccattatggaacaaagcaacattctccgtgaaatgatccagaaaggagaagtcggtattataggcgcgatttacgacgtagaaaccgggatcgtaagctttatggagcaaacgctgatcctggaaaataacataccggaaggagcaacagcagtagctgtttaagctgtccgccttttatagaagagaataaatttgctttttcataaaaagagggagactctgataacacgttagatcaattatttaaaggcattgatctggctgttatcagcggtctcctttttttatatctgttgcaaccgcgcggcagcctgttccagcgtagcctgtttcttcgcaaaacaaaaccggatgacatgatcatcttttccgtcctggtaaaacgcagacacggggatcaccgccacaccaaattctttggtcatacggatcgcaaaatccttatccccttcatctgatatccggtcgtatttcatcagctggaaatagcttccctggctggccagcggggtaaaacgggtacctttcattaactcaaggaaatagtctcttttctgctggtaaaacgccggtaactccaggtaatgagatggcgtttccaggaattttgccagtccgtactgcatgggggtatttacagaaaaacaaaggtattggtgcaccttccggtactccttcatcaggtgctccggcgctacacaatagcccattttccagccggtattatgaaacacttttccaaaagagaaggtaacaaagctattcctgaaaatagcgggataacgcaatacgctgtgatgctgtgcgccgtcgaaaaccaggtgttcatatacttcgtctgataatacgatcaggttaaactcatccaccagtttttccagttcctgcatatcattttcctgtaagatgctccctgttggattatgcggggtgttcagcataatcatcctggtgtggggtgtgattttacttcttacttcgtcccagttgatccggtagcccggaaacgaaagggaaatgagcacgggcactcccccgtttaccaatacattgggaatatagctgtcgtaggccggttcaaaaatgatcacttcatcacccggatgtatacacgtagcaatggccgtaaaaatagcataggtgcccccgggtgtaatggtaatttccgaatcgggatgtacctgctgctggtaaagactactgatttttgtggcaatagcattacgcaactgcggaaggcccggcataggggcatattggttatgcccttgctgcatggcttcatttaccatagctttcagttcatcactgcaatcgtaatcgggaaatccctgggagaggttaattgcctggtgggaagccgccagtgcggacatgacggtaaatatggtggtgcctacgttgggcagttttgagatcattgccggattttttgatattgaaattcagacatctgctggtgagaaagtcttttcagccactaaatatctgaatttcaatatcaaaaatcacaaaaatatttacaggaacttctcgcctttgttgcgcttgatttcccctacatattctttgatctgttgttcattttcttttttgcagatgagcagtacatcgtttgtatcgattacgatgaactcatccaggccctgtaacagcaccagtttatcgttaggtactttcaccatgcatttggtagcgtctatcaccaccacgtttttaccctgcactgcattgccgaggtaatccttttcgaggttctcataggcggaagcccaggtacccagatcactccatccgaaattggcggggatcacatatacgttgctggctttttccatgataccgtaatcgatagagatattggtacactgcggatatactttctccattacctctttttcctggggggtattgagtgcgggtgtagcctgttcaaacagttcatctatctccggaagatattgtttaaaagctgccaggatagtttttacattccatacaaagatgccggcgttccagaggaaatcaccgctttgcaggaacgttttggccagttccaggttgggcttttctgtgaaggttttcacctggtatacgttatccgccacgtgttgtggttcaaactggatatagccgtaaccggtatccgggcgggtaggtttgattcccagtgtaaccagggcgctgtttttctgcacaaacagcagtgcatttaaacaggaattggtaaacgccggtccatccatgatcaggtgatctgccggggcacaaataatgttggccagcgggtcctgtttatggattttatgggaaatgtaagcaacacagggagctgtatttttacgggatggttcgctcacaatattggctgtgggcaactccggcaactgatcactcaccttgctgttatattgatggtgggttaccacgaatatattttcctttgggatgaactgcgcgaagcgttcataagtccattggagcagggtttttcctgtgttcaggatatccaggaactgcttgggattgtctgtgcggctatggggccagaaccggctgcctattccccctgccattattgccacgtaaaaatggctgttcagctgtgtcatttctaaataattccttctctgattaaatcatgtaagtgaataataccttgataccgttcaccgtccattaccagcagttgggtaatatcgtgctggcgcatcatctctaaagcgttgatggccagttgatcctgctggatcattttcgggtgaagcgacattatatcttttgccgttacagctgctgtaggaacatctttctccagcattctgcgcaggtcgccatctgtaatgataccctgaagtaatccattttcatccactacggcagtaacacccagcattttggatgaaatttccacaatcacctctctcaatgagctgtttgctgatacctgcggggctttgtgctgtttgctgagatccccgaccttaaggtacaatttctttcctaaagcgcctccgggatggaacttggcaaaatctgcagcagtaaatccgtgccattctatcaggcaaacggccagggcgtctcccatcaccagctgtgccgccgtactggtagtgggcgccaggttatttgggcaggcttccttactaaccgtggtattaagtacaaaatcggcttcctgggctaaaaacgagcttgtattccccaccatggcaattaaagtgttgccaaagttcttcaccaggggaacaagcacctttatttcggcggaagtaccgcttttggagatgcacattaccacatcttcctcgcggatcatgcccagatctccgtggatggcatctgctgcatgcatgaaaagggccggcgtaccggtagaattaaatgtagccactattttctgggcaataatggcgcttttaccaatgcctgtcaccaccagtctcccctggcattgagcgatcttttcaacaactctttcaaaatctgcatctataaaatgctgcaaatcattaatagctgatgcctccatcgcaattgtgcgcctggctacctgtcctatattgatagtttgattccttttcatgtcgatttacaaatttatcattttttaaccagcactggagcggtcaagtaatttatattgatactccgcgcttttttaagtaacttcgtgtcccctaaaaaacatataaatatatttcgtcatttgttggttctttagagttaaaatttgaatgcaatggctgttgttaaggaacgtttgatggatgcattacgcgaacacttcgggttcgattcctttaagggaaatcaggaaaaaattataaatagcatcctctcaggcaaagatacttttgtgataatgccaaccggcggaggtaaatcattatgctatcaactaccggcgctgatgaggccgggttgtgcgctaatcgtttcaccccttattgcgctgatgaaaaaccaggtagacctggttagaggctatagcagtaaggacaatgtggcacattttctaaactccaccttatccaaggcgcagatcaagaaagtgcgggccgacctgacggcgggaaaaaccaagctgctctatgtagctccggaaaccctcaccaaacaggaaaacctcgatttcttcaaggaactggaaatctcttttattgcagtagatgaggcacactgtatttctgaatgggggcatgacttccggccggaataccgccgcctgaaggaaatgatcgaccagatcagcgataacctgcccattattgccctgaccgctactgctaccccgaaggtgcaaagcgacatcgtaaagaacctgtgtctgaacaaggccaatatctttatttcttcctttaaccgcccaaacctgtattacgaaatcaggcccaaacgcaaaaaggatcaaaccatcaaggatattgttaagttcattcatcagcataaaggcaaaagcggtatcatttacacgctgaaccgtaaaaccaccgaggaactggcggatatgctggtagccaacggcgttaaagcggtagcctaccatgccggcctggaccctactacccgggcacaacgccaggatatgttcctgcatgaagatactgaggtaattgtagccaccattgcattcggaatgggaatcgacaagcccgacgtacggttcgtgatccactacaacattcctaaaagcctggaaaactactaccaggaaaccggccgtgccggcagggacggactggaaggacattgtatctgctactactcccataaggatgtgcagaaactcgaacaccttatgcgcgataagtcgctcagcgaacgtgaaatgggcgcacagctcattaacgaaaccgttgcatacgccgaaagcgccgtatgccgccgccgggttatccttcactacttcggagaacattacgaaacggagaattgcggccagtgcgataactgccgtaacccgaaagaaaaaatagaagtcagaaaccgcgtggtgatcatgctgaaagccatccgctccctcgaagagcgctttggcagcgaatatgtgatcaatatcatcaccgggaaaaccagcccccagatcagcacctaccgtcatgataaactggaggtgtttggagaaggaaaagaatttgacgcgcacttctggaactccctgatgcgccagatgatgctggaaggactgatagaaaaagatattgaggaatacggcctgcttaaagtaaccgataagggcgccaaattcctcaaaaagccctactccatcatggttgcactgaatcaccagtttgatgaagacaccctggatgaggaagaggaagccgccgcggaagcacaggcatctgcagaccccgcattgtttgaaatgctgaaggaactgcgcaagaaagtatccaaggaaaagaaccttcccccgtttgttattttcctggaaacttccctggaagatatggccacccaataccctactaccgttcaggaactggaaaaaatccagggcgtgagcaaagggaaagctgttcgctacggcaaacagttcctggatgtaatcaccaaatacgtagaggaaaataatatcaccaagccggacgatttcgttatgaaaagcgtggtgaataaaagcgggatgaaagtatttattatccagaatatcgataagaaaataccgctcgaaaccattgctaaaaataaggaactctccctctcccagttactcgacgaaatggaaaccattgttgccagtggtaccaaactgaacatcgattactgcctggatgaagaactggatgattatgcacaggatgaaatcatggagtatttcaaaggctgcgaaacctccagtctcgccctggccagggaagaactgattgaaaatgattattcgctggagcaactgaagctgatgcgtataaaattcctggtggtatacggcaactagtccggctataagtacaactgatgagcattaaacaaatacaggaaacgattgcttccgggagggagaaagtagtatcacacccgttatacgcggagctgcaaacattggatgatgttcgcacttttatgcagtatcatgtatatgctgtatgggacttcatgtctttattgaaaggactgcagcaacaacttacctgtgtaaatgtaccatggatacccgtgggcaatgccgctacccgttacctgatcaatgaaattgttaccggggaagaaagcgacgtggataaagaaggtaaccgctgcagccattttgaactgtatgaacgcgccatgcaacaggctggcgccgataccagcccgatagaggcgattatagctgatataaaggctggaaagcctattgaaagggtgctggccaccgccgaccttcctgaggccataaagggttttcttagctttacatttgaagtgattgctaccggtaaggcacatattatggcagcggtgttcacctttggcagggaagacctgattcccgacatgttcctcgcactggtaaaagacctcgatcagaagtttccgggcaagctggataccttcatttattacctggaaagacacatagaagtagacggtgaccaccatagtcaactggccatgcaaatggtcaatgaattatgtggcacggacaaaaataaatgggatgaagctgctgaatacgcccgccagtcgctgtattggcggcatgaactttggagcagtattctcaatgaaaaagtgatttcgtaaaattttctcaaaaaaattttgcaattcgaaagaatgtattacttttgcaatcccctcacgagagagggcaataaaaaacggatggtgcggtagctcagttggtagagcaaaggactgaaaatccttgtgtcgccggttcgatcccggctcacaccacagaagcgggaacattactgtaaaaggttttgttcccgtttttcatttcccctaaaagccgtaccaggcccgtcatttggcggaatacttcattcacccgcggggttcgacactgttcattttcctattatatagaattggggtaaaaaaaattaaaccttattggttttgctatctactaataagtctggcagactttttttacgacttttaaataatggaacattggatgtatgaataatcttccggcactataatactgcgccatattaatggagaagaatctttcaggcttatatgtaactggaacgctttacttttcatagtgtaagcaattataaacggtagacatctttattggaatatttcctggtatttattttcgatttcaataacctctttatctgtcaaagcttcgaactcttttgctctcgctctttcagatagttgtcctcttccttgttccagaaaacggacaagcaaagcaactgttttatctggcatttcaaagtagttgtccagataatctttcataagatcatacttttcgagataatcaacttcttcaggaatggtttgctcgatggtttgctgaacgcaactatataaaaactccacctgcttggttgcatcaaaataccggtaaaaatcaattgtatcattcagtacttcaacgttattattttcagtgggtttccattccaccaaattaagacgcggccttgaaaaaccctctaacacccggcggtactcatccaatcgctccaaaatgatggcagaaacaggaaagattattccttttgaaatatattcttttcttaaaagcacatgatggatcaggtaccggtgaatcctaccgtttccatccgcgaagggatgtataaatacaaatccaaaagcaatcaatgctgcagctaatacggcatcaaaggaaccatccttttccaatttttggttggcagcgatccaaccatctattaatgcatcaaggtcctgccatttggctgaaatatgatctggaatgggtgtcccatgtcgtctgtcatgttcaccaataaacccttcgtgatcgcggaatcccatcttggtgaatcgcgggttatctattactatctgttgtaaccggattagttcgtctttcgagattggtgtttgacctgcctgaccgatagcccgtccccaacgctgtgcccggttctgcggtggtctttctccttcaatggcataagacgcttttgaatcttttaataacaaaaaagccgatgttctcgccataacatccgggtgaatttttccgatgatcctttttatctgttgggataaatcaagactgatatattgctctaataaagcagtctttctgatcataggacaaaaatctttaacgccgggaaggttatttcttatccgatgccttttagaagtctccagtctatcacgacaagcatattgaatgtcttcatcaaccaggttaatataattaccagctatcagatcaggaatttccagttgaaaacccatcaaccactcgtacaagaaccatattttcctgctgtattggcccgttggttcattgctgatcaccttactaatctcttctgcatccagcttttcaaataatttttttagtagcccaagttcaattccttcatactttaatgcaaaagtcaggtgccccatgagagtatcttcaggcatatgtctgggtgtaaaaacaatccattcttccgttttgtattgcttgtgcttttggcttataagagccaggatatcaggaagcggagcctgtaaattataggcctttaatatcgccccatatcctactaaataacctttttcaggcgaagttctctcctgaaataccgttattaattgtgaaaagctgttaattcccatcttatttcatgaaatatagttatatctaatttatgaaaattatttagaaaacatgaaatgtgattaaaaattaaggctatttgtgaaaactagttatttgatatatctaatatattcacaaatttctgagtgaatggctcactcatatgaaaagcccaacttgtattccgggtaatctttaatatctcattcgctcccacttattcaccgcaagcttaccccactcaatgattttgcaaattttcgaacatcccctgcaaatagatctggttgttccattgccgtaaagtgtcctcccctgggcatttcagtccattgctgcacattaaagagtcgttccgcgaattccctgggagccggtacaacgtcttgggggaatatagccacgcccgtaggaacttccactttcttaatttccatacttttttcctcctgttgtattgaaacggccgcctcataatagaggcgcattgctgaagttattgtttgcgtagcccagtatatagtaagattcgtaagtaattcatctttggtaaaagtattttcaagcttgccatcacaaccactccaactaaagaacttttctatcagccatgcagcaagccccacaggcgaatcattcaatccatatgccagcgattgcggcttcgtagattgtattacggcgtaacctccttcggtttgactccattgctgaccggtttgcacgtatttcttttcagatgccgtcaacgcatccggggagatagagaacagatgacgccaggggatatcggtaagatgaatacctttaagaatttgagaattattaaccgcaatttgctccgctatggtgctaccccaatccccaccatgcactataaaggaggaataacccaactcctctgtcatcaattttgcaaacaaggatgctatgtgttttggattcatacccggcgatgtcggaatatccgaaaaaccatagcctggtatggatggaacaaccacatcaaaggaaaacccatcatcaggagcaaccaacagcggaattgctttcaggaaccgcataaacgaatccgggtaaccatgtatcaacaaaagaggcacgcttgttttgcctttgcctttttcatggataaaatgaatcccttcgttgtcgatagcagttctaaaatgcgaaaacgaattaaggaaggcttcattctttttccaatcgaagttatgcaaccaataatagcataactctttcaaatatgttgtgtttgtgcccgttttccagttgtcgttgttaatgtcattggtccagcgtgtcatcgccaggcggtgacgtaaatcgtcgagtagagatacgtcgatgtttataacataaggctgtttcataatttctgtttatcctctcccaacaaaaattgtgacaccttgaattggctgattccgatttatcagatgaatgcccaaatagaacgtttcatcattgcccttctatgttaacggttattccaagtattcgtcctatggcctctttcacctcctccgcccgctcattaaaccgcaaccccgattgtgtcaccaatctttcaaatgtatgaatacttccattttttaccagctgctgcagttgcaacatactctccgggcttatcacttttttatcataccagctcgaatataaaacaaggtagtgaacctcaaaagcagactggttaaaataagacacgatttgcccgatgtcaaatgcgctgttatctattaccaggctgaggctaaaaagaaaagaggtatccgatactgcatgatactctataaccgatttaatgcggctgagctggtcgtctgaccggcagtacgggtccggagtatttacgacaataaatttctccttccacaaagcatccagttttatgggttgtttgaagagataaaaccgctttcgctgaaacaagttttgtatcgttcttgttttgcctgaatgaggatcaccaacaatgacaaataattttcgtgggttaaaattcattctcaaaaaaacacggaaaacatcaaaaaaatgttaaccaattgtgaacggactatactttttctgccagccaggcaatcaattgcgcacaggggaaaagtaacagctgtgcaagtaccgttccggcaatacgggcaattaccatataggcaacaaatcttctgaaagcgccctgtgaaagcttccctaataccacatcatccgtgagtatagataaatgcggatcaataaacaataccatcagcaccgtggccataccgtttataacacccgataaattactggctgttgttctgtattctggattcagatatgcagcatacacacacgataaaaccgaaattgttattactgcgctggccaatacattgtagataaaaatacgccagggcatatccctgttagcaggcaattccaggaattgctcttttgtgggcatccgcatgctctctttcatgaactgcataccggcgccggataagccaacataaaataacctgggaatagatttatgtacactaaaatgcaccactgccttagacaataaccgctgaaaagttgggatcaacagtgcgccaattatagcgccaatagtacacgacagaataatatacctgaatatctccatattggaggaaagcccctgtttcaggtcccgttctaccgttttggccagtaacggcgcctgcaacgtattggcggtgcgggataaaagagcaaggatattaaataaagaaaaggtaatggcaattctaccggtttttacacctaccagtcttacagcataagacaacgtagttatcccgttaataaacatcgtaaggataagcacaataataatctgagtggccattttagtaatcctttaaaggattactaaaataatcattattccgttctcaggctctttaccgggttaatagccgctaaccggtgagtcatccacacaatgatcacccctaccagtattgccagggttaagcccacaatcaggaaaggcaataccccaatgttgatccggtaggcatagtccatcagccagccatgtaagagataccacgataatggccaggcaatgatattggacacaacaatgattcctgaaaactcttttataaaaagcaggaggacgtgtaagcccgatgcaccgagtacttttcttattcccatctctttattcctctttgcaatactcatagtaacaattcccagcacccccagcaacacaatcatcagtgatactgcagtggcagcctttgcagccttccgcatttgtgtttccgtatcgtataactgcgctatactatcatccaaaaatttgaaatcaaaaggagcatccgggaaaacctgctgccattttcgttgcaatgcagccacttgcgtcgccgtatttccaggattaaagcggaacgataaatagcggtatatatttattccccgtaccggctgaaaataaaccgggcctatggcatcatgcagacttccaaaatgaaaatcccgggtaacaccactcacatacagcacctggttaaaattatgcaaccgcagcggcttattgatggcttcttccgcactcctccaacctaatgcctttaccgccgcttcattaataataattttggcagcatcttccggggcgccattataaaagcttcctgcatccagtttgatatcgtaagtggcgaggtagcgctcatctgtaataagtgacaccgccgaaacagcagtactggaatcattttccggcctgtaaatcctgctggcgccactggctgccccgtcggggatcacataggcaaaggtggcatcttttatttccggcattgcccggaactcctccctcattcgttccatatgtgctactcccgctatggtccagtcgcgcggcacggcaacagtcaccaacttttccttattatacccaaggtctgaattgaaaaagaaagccacttgccggtctattacaatcgcagcaataaataccacgatggctgtcacaaattgtacggttacaagcgaccgcctgaataataatttctcctttacatcctttaacttccctttcaatgcggttacagaaggttgcgcagataatacaaacgcaggataaatacctgccagtaagccggtaaacaggattaccaacaatggtaacacggcaaaccaggcaggaaaagaagataacgctggaatgtctttcccgatcagttctccaaaccaaggtcttactataaaatacaaacccagcgatacaataaaagaaaaagtaacgactaacaccgactcggtaataaactgaagtattaactgcagccgctttcctcccatcgcctttcgtacgcctatctcctttaatcttgttaaagaattaccgatagaaatattgacaaaatttataatcgccatcagcaggataaacaatgccactaatgaaaatacggtgatcatttttctcgccagccctttattcataaggaggtaccagtgcttcaaagataccggcgttacctccagcgtacgttgaatttctgcgtccgtattggtagccaataatgtttttattggcccctggagctggtcagcagtaacacccggttttagcattacatagcccacaatatagggcgataaccagctgttaaatccaaactcccttccaaaataacgtatgctggcgggtgaaagaaatatttcatttccgggtttaaaaaagttggtgatggtattaaaaggaagatcttttattacagctgttacttcaaaattatcattccttccatcgaaggattgtatccttactaacttccctaccacatctgttttgccaaaatactgctttgctttcttctccgtaagcaccaccgcatttggcttatccattgcggtgtgcggatcaccataggcaaccggaaaattaaacatctcaaaaaaagttgaatcccctggctgtgccccttccctgaaatgcttatctcccactgaaataacaacattgattccatcgtgggcataagctttttccaccagcgagggataattatcctgcagtgccttggttagtggtcctaatgttgttaactctgttcctgtttccggatttgcccatttgcttctcagtagaaaaatgcggtcactattcttcacaaagtggtttacctggtattctccccaggcatatgcaccgatcaacaatacaaatgtgatcccgatagctaatccccagatattcacgatagcaaaaaaacggttcttcgccatatttctccaggcaatcagaaagtagttctttatcataaacaaatgaatagtggtttgttcttcccgcgaaaaaaatgccgcaccccaacgtattgatgatcaataaccttataaaagatttttgtccggtaccggacaacttttgttcacttttgtacgggcacatcctgaccggaatagtacctgtctcccgtaaattaccatatacatcctttctttttatttgtattttgtacacttattcctcgttagtaaatattaaaacatgagaacactgttttgcataagctttctattgttaacccactgggtatctgcacaggaaaaaaatatccgcattgctacccgcaacattagcctggtatacagcattaacccggaaggccggttaatacaacaatacttcggacaacagttacagcccgatatggcggatacccttgcaaaagggaaacaggaggcctatataaccgccggcatggaaagcctgctggacccggctatccgcatcgttcacaacgacggaaatccttccctggagctaaaatatgatacccatacatccgcaaaaaccagcgatgacatcattgcaactaccattacacttaaagatcccgtatacccggtaaccgttatcctccactttgaagcgtactataaagaagatattatcaaagcatggacggaagtaaagcacaacgagaaaaaaccggtacagctaacagcctacgcctcctccatgttgcacctgaaagcagataaatactggttaacgcaattccacggcgattgggcaaaggaagctgatatgcaggaacaatatcttaccaccgggatgaaaatcctcgacagcaaactgggcgtaagggctaatatgctgcaatcgcccctgttcctgctgtcattaaatcatcctgctgaagaagagaatggagaagtattggccggaacattagcctggacaggaaattttaagtttggatttgaggtagatgaacacaactcactccacattaattccggtattaatccttacgcaagcgactatacgctaaaaccaaacgaagttttcaccacgccggcattcatcttcaccctgtcggccaaaggcacaggacaagccagcagaaactttcatcactgggcactcaactacggcatccttgatggacattccccacgtttaaccctgctcaataactgggaagcaaccggcatggacttcaacgaacaacggctgaccggtcttttcagcggggccaaaaaactgggggtcgatctgttcctactcgacgacggctggtttgccaataaatttccacgcaatgcagacaacgcaggcctgggcgactgggaacacaacaccaccaaacttccgcatggattgggctacctcgtacaggaagcagaaaaacaaaacataaagttcggtatatggctggaaccggaaatggtaaatccaaaaagtgagttgtatacaaagcatcccgactggatacttcgcctgccaaaccgcgctgaaaactattaccgcaaccagatggtgctggatcttaccaaccctacagtacaggatttcgtgtatggtgtagtagataaaaccatgtcggaaaacccgggcatcgcttatatcaaatgggattgtaaccggatgctaaccaatacctattctccctacctgaaagaaaagcagtcgcacctttttatcgattatacccgtagcttatacaaagtgctcgacagggtaagagcgaaatatcctcacctgccaatcatgctttgctccggtggcggcggccgaacagattatggcgccatgaaatacttcaccgaattctggcccagtgacaataccgacggactggaaagaatttatatccagtacggatactcacacttcttcccggccaatacaatggccgcacatatcaccaactggggcagccaatccctgaaattccgtaccgatgtagccatgatgggcaaactgggatacgatatcaaagtggacgattttacagagaaagaattacagttcagtcgtgatgcagtaactacgtataagcgtatcagtgatattgtgtggtatggcaatctttaccggcttatttctccctataaggaaaacagggcggtattccagtataccagcgatgatcagcaaaaaagtattgttttcagctacctgatgaacattgcaaaaaacgacgtatttacactcgtaaaactgcagggactggatcctcagaaacgttaccgcatcaacgaaataaacctgttcccgggaacacattcttcctatcattttgataggctctatagcggcgatttcctgatgaaagaaggcattcagctggtacctggcaatggcagatcactaagcagcaacatccttgaaataacagccgaataaagtaccgtatatttaaatggcctgtttccggtaacgatggaaacaggccattttcttttgaaagaaaatgaatcgcaggtgatttattatcttcaatacttcaaactacagggatatgcttcctttcgccaatatgccttatggtaatgcccctggatactgctttccgctaacggagatctgtatgtatatccttttgcttatttgcggctggcacgccctgaaaaaaggaaccgcacatatggcgtggttactgggggcactgtgtttcgggttgttgctggaatatgtaaatgtagccaccagcagcggctatgtgtacgggcaattctggctcatgttgggcaaggcgccgcataatattccgttttgtattggctgtggttgggcggtcattatttattcgtcgcgtttatttacagataactttgggttgccgttatgggcggcagcggcgctggacagcctgctggcattgaacatcgatgcaagtatggatgtggtagcctatcgcctgcatatgtggcactgggattgggtgggcaggggctatccttcggaaacgcttaccggtcaatggttcggcgtgccatacgctaatttctatggctggttgctggtggtatttttctattccctctttggccggctgctggaaaaagtagccgtcacccgggtatggaaggcattgctgcctttactttccattctcctttcacaggctgccctgtggatatccttatttccattggccgatttactgaaacaggcatttggcatcagcagtatgcatcggctcattgccttgataatactactgtcgttaatggtagcaacgggttttgccaggagaaatagcaccagtgcccattactttccgctggccgcatggattgttccgttatggttccacgtgtatttcctggcctggttattcctgggtgggttctcccgcgaaaatagctggatgacggctttctcgctgctaaatgcaacgattggtatattgatacacgtacccatgttgataaaaaagcagcctgtaactattttaacggaaacatgttaatattaatacttaaataatttttactggtgaaaacactgatcggttatctaacaggtgcagaatggcatatttacatcaaaataggcagtatcgtcttactgatccttattttcatcggattgattgctaccattctgcttgaaaaccgcaacccggtaaaggctatcggttacatcctggtgctggtatttattcccgttgttggtttaattgtttactactacctgggacgagacctgcgtaaaagaaggcggtttacgctgaaaggcagtaaagatgaagtattgttttcgaggtactgggagtcacagaaaccactgatagaacaaatgcaggtagaactccggcggctggcaggaaataaacaggagatttcagccatgctgcttaatacgcggcagtctatcctcagcaaaaataacagggtacaactactgatcaacggagaagaaaagttcccggtggttttcagcgcactgcgtgctgcgaaacatcatatccatatagagtactacatgattgcagatgatgatgtgggaaatgaagtaaccaacatcctgatcgaaaaattaaaccagggtgtacaggtacgttttctgtacgacgatatgggcagcgaccggatcggggatattcctgaaaggttaaaagcacatggcgccagtgtataccctttttctcctgtgcttgtagatttttatctgaacgccaattacagaaatcaccggaaaattatcgtggtagatggcaaggtcggctttgtgggcggcatcaatctcgatgaacggtacatcaacaatggcaagcatcctactttctggcgggatacccatctgaaaattgaaggcgatgcggtaaacatactgcagctgcagtttctgatgagttaccgttattgcagtaaagaagtatttccttttgcagaaccgttctttggccggtcagatttaacgggtacctgctttgtagatatcgttgccagcgggcccgattcagaatggcctgttgccatgcagagtattcttatggctattaatattgccaagagaagaatcaggatctctaatccctattttattcctactgaagagctgctcaccgcgctgcaaatggcggcgctggcggggaaagatgtacagctgatgctgccgttaaaaggcgattcctacattgtacaacatgccgccctctcctatctgaaacctttgctggcggcaggtatcaaaatatatttttacacgcgtggttttattcacgcgaaaacgatggtgatagatgataatctcgcctgggtaagttccgttaatttcgacaaccgcagcttttatctgaattgtgaaataggtgctttgatctatgatacagaggtggctacccggctgaataaggtgtttgaagaagaccttttatattcagttcctgttcaggaaacccgctggaacaggcgcaatattctaaagcggtttatggacgctgtttgtcgcctccttacaccgctattataagccctaatccttgtcttcatccaggttgaggaactcaccgttatcttcttccagatcttcgtgtctgtcgcctcctatgctgtaaatattgttttcctcatcctcctctccgatagcttctgcttcatcgtcgagttcagcaccgggaatatcaaggtcatctcccactttatcctggcgccaggtttcttcctgttcattattttccctggacttctttttatcaggcgataattcactgtttctacggaaagagccggttacctcgttaatatccaggtctacttctttatcccggttctttttgttcatgatatcttcgctggcagggtattcggggtatccaggaaactgatcatcttcatttttagatagttgttgatcttcctttccggttttattctttttgttgctcataatcaaatcttttattgagtaggaaagcagaaaatgccgtgccacataaagcagcaggcattgtatcaggatgataacaacgcagcagaatgattgtttacaggatggatcagcgtttttttcctaccaggtttaactgtactgataagccggcagagtacagtttcacctgtcccaatccgaccccatgcaggggaatttttgcatatggctgtagcccaacaattaaccttcttccggcagggtgctggtaaagggcgccaacattcagtatggcaagataatgctggttttcattatctaccgttctttccttttcgggagaatacttgtatacatattcatacttttctttcagcataaaatagttagagataccgagtgtggcactcaccgtattattttttacctgtaagaatgtatagttgatattcactggtatatcgagtacatcacaattcgcatttaccttaacaacaggatcccacggattattgtaaagatttttataatcaccgtttgtagcgccatatagcttcttactgtatacaactccacttgtaacaaaccagtgctggctaaaataataatgcgccagcacaccagcgttaaagccgacgtttccatatttaaaagagggcgcaacgttcagatctggtccgaaagttactcctatatacaatccttttgagttgatcttccgacgtacgggttttttatcctgatccggctgtaacttagtatctacgggtatttcaacaggtcttcctattttcgtatatacgttaaagttattactgttctttgttttcagcagatcaaaagcggtgtgattaattgttgggggtacacctttatcatttcctgtttcttttcctgcatctgcagtaatatctggtgtagttgttttttccggtatatcctgacctgttgttttatttgccttcggcagataggtgtttgtctgcgaaaaggtttgctgacggccggtgtttacggctgttgtatttgtttttggcagatggattcctgacggggaaatcgtttgctgttgggcggaattttctgtcgtagtatttgtttttggcagctgtttacctgatgataagtcgctgttttgctgcgtttttgttgctgttgacgtaattgttcttgttccgggcagttgtactgcactgctatccggcgtggcaatacgctgtccgtctgttgtgatggtatgctgttgctgatcctgtgaagaaactattgttgcacgtgaaaccgctttatccgttgctgatggttgcatgatccaccagcctaagccacccagcacaggcaataacaacagccaccaccagcctgctggtcgtttcttattatttcctgcatcaagcttcgattccatttttttccatgcatcctggtcaaaaggaatatcagcttcattcagcttattacggatactattttcaaacgcgtcattcatttttgtataagggcatatttatgtctattccatcagcagtgctcatggatgctttaataattctttctttcagtattttctttgctttaaatagattcgatttggaagttccttctgagattcgcaacatacctgctatttcctggtgctggaagccttccattatatacaggttgaaaacagttctgtaagccggaggcaaagcctgtacatgtttcagcaattcatcataggatagtttgtcaataattttttcatccgttcctggttccggtacctggttgatatcatcagtaaaaaccagtttctttttacctcttaaaaaatcgatggcggtattcaccataattctggccagccatgttttaaaaggccgggaggtatcgaatgtttcaatgtgttggaatattttaagaaatccgtcgttcataatttcaactgcctcatctctgttctgtgcatatcgcaaacaaatgctgagtccatacccgaaaaagttccggtataacgcttcctgactgctgcgttcttttctgcagcaaccggcaatcacttcattaatattattcagctcatgcacaaaaatattcttacctgcttttggtattaggtgctgttatttttttgtcagggaataattgtttaaataaactccaggctgaagatagatacggtggaaaatcaaaaaaggttgctttttccggaaaaataaagttctggttcaaaaacatgcatttttagccgtttttatcccttttaccccttttctaacacttatatccaccaaagaagagatcattaaaatttaccgcgtttctgaaggtcgattttcgggcatttttggtcattttttgtctgtgcccggtgataaaccaaaaaaaacgggcagattgtaaaaacaacactacccgctataaaagctttatatttttatcgtcccatataaaccatcaggatttgtacatcacttggattaactccactaatgcgacttgcctggccaagggtatgcggacgaattttattaaatttctgtcttgcttcgttcgacaatgaaaccagttttgcataatcgaaattggaaggtatcacgagatcttccagttggctcattttctgcaccagttcattttccttttcaatgtatacatcatacttgatctggatttctgcctgttccaaaatatccttactaaatccggcgagtgcctgtcctattttttccacctggtctttcatggcaaaaatatcgagtcccggacgtaataaaatctggtgcgctttctgtttttgggttaacggagcagatgatttctctgcaagtagtccgctgatttcgtccggctctatggacaattctttcaggatgcgcttaatttgttctacgccttgtcttttttcctgcaccttctgcattctttcttcagaggccagccccattttatagctcctttctgtcaggcgcaggtcggcattgtcctggcgtaacagggtgcggaattctgccctggaggtaaacatacggtaaggttcttcggtgcctttattaatcagatcatcgatcagcactccaatatatgcttcacttcttttcaacacaaaaggtgcttcttcccgggccttcaggtgggcatttatgcccgccatgataccctggcatgcagcttcctcatatccggtagtgccgttaatctgcccggcaaagaagaggttttgaacatgcttggtttccagggagaactgaagctgggttggtggaaagaaatcgtattcaatggcatatcccggccggaacatccggcagttttcaaatcctggtaccaggcgaagcgctttcatttgcacatcttccggcaaagaggtagagaatccgtttacataaatctccacggtgtcccagccttctggttccacaaataactggtggcgttctctttctgcgaagcggtttattttatcttcaatgctggggcaataacggggacctgttccctggatacgtccctggaacatgggcgacctgtcaaaaccagtacggagcatttcatgtacggcatcgctggtataggtaatccaacaacttctttgttgtgcgggtttaattctttcgacatccaaataggagaatccaacaatctcttcatcccctttctgttcttccatttttgaataatcgaggctccttccatcaatacgtggaggtgtacctgttttcaaacggtcgctttcaaaacccagggaaacgagttgttctgtaatgcccgtagccgctttttctgctaccctgccaccgccaaattgtttatccccgatatggattacaccgttgaggaaagtcccgttggtgagcaccaccgccttcgcctggatctcatggcctagtccggtaacaacgccgtggcatcttccatccttcactaaaaggccttttaccatatcctggtagaagtccacattcggtgttttttccagtgcttccctccattttgcggcgaaaagcatgcggtcattttgcgtacgggggctccacatagcggggcctttcgaccggttgagcatacggaactggatcatagactgatccgttactatcccggaatatcctccaagcgcatctatctctcttacaatttgtcctttggcaatgccccccatagcggggttacagctcatttgagcaatggtttgcatattcatggttaccaacaaaaccttggaccccatattggcagcagcggcagcggcttcacaacctgcgtgtcctgcgcctacaacaattatatcgtatgatggaaacataataactttagaaagtgcaaaattacgtagaagaaaggagaatgtggttgccaatgtgaatgttccacgtggaacattccgtggaggattcaatagctcatccttagcatcttctttatcctgttaatgtttcacgtggaacataattagcgggcaagagatgtaagttcccattagaaaaggatgctatcctgattcaaaaccttttcattagttatgaatcacctattagaagatccggtaaacatcagaagtatgacgacgaatacgctctttttttcatcgattttaattatctcttagtctttccctttagacacttattcaaatcctcctctcctcgcataataatacactggagaatcccctgcgggaagtatctctttaagttgtaaaacacttcctccggaaatgaaaattgcttcccgggtgatgggtacctatatctttaagaccctccaacaaacagggaatccaaagcacgattatcgtttgtagctcttgcagtttcttgatacaaatgcaagaagcaattaagaatacacttgagacaccccggctcaaagtccatccactgtcatagaaactcagttatataaaatctggtaaatgctgctctcctgcatcatttattacgcagataaagctactcttagcatggaaaaattgctcaatagtaattctgtgataacaagccggctggcagaaaataaactccaggaaaccaggcatcctaggtttctctccattatctaaatcctgtaccttttcaatctgcataactaaatgcaaaagcctacagtttgcttctggtattatcaacagattcctcaaacaacatctataggcaaagccggaatagcagtcctaaattggctcacaggcatggaatatcaaatgatattcagcagagctgcgcataagaagaatgtccctatccttccaaagcttgttaacatcacttggttgttttggaaaaagaattgaaggtcctgtgtcgctaaattcggtaaagagtaccaaatgtcttaccatcaacaaatacggctgaggaaaaatacagcggcgcctacctcctatgagcattaccactatagccatcatctaaaccaatctggcgatatcatgttcacttaaaacggcatgcatagatcatcatatgacttgatagaaatcaaaagtccagatcatgaaggaaacagcattaccatgcttattatatgcccggttccccccttgtgaattacgcccacctcttaaaccttacaaatcaaagctcggtttttaaataaatccctttttagatgttccacgtggaacatctaagtttgttctttcttatagtaaatcttttattggaggcacttcatgaaatgtaaagaattctgtccttgcttatgaacaccataacagaatatctgccggaataagattaacggcgccattcgcaatattaaacaggaaatcgtttcacttgattccaagcctattcattcccataaccctaaatgggaatcccctcccaaaatgctacatgcagaaaaattgaaaagatttataagcacaacacttgcctagcggataatatccagtaacacaatgttgccctggttgtactgtacaaacatataaccaaatgcctcttaccccggtcaatatcccttcctcctgccccgttatatcggaggtccaggccaaacgaaaactagtgccgtaaaccaaatacaggatttacaacccacactgtaaacttatttcaggacttaaaacctaaacagtaaactttaaacaggatcatcaagcaaaaatgcaatccaattccaggacctttgaataaaagatggaaaatcaaaaagaaagccttggttactttgttactgtaaagctattactgcaccgaaaagcaacattgtaagctaaatctgtgttcgacgctggggggtgtaaagtttttccagtataaccaccctgagctgtaaggttcttttcggtataaaacagggcatagtgtattgtaagtgtatgggaagtgtataatgagtgtatgaggagtgtattgtgagtgtatgggaactatatgggaactatataggaactatataggaactatatagggactatatggggactatatggggagtacgacacatacgctactcctaggtaactgagaagtaactgagaagtatccgagaagtataccacgggtaataacgctatatgcaggatccccaggttttataacgcccaggttaatcatctccaacgattccaaacaatgaatgttccacgtgaaacattgtaaggctcaaaagcctatttactaccaaaatactttaccaggtactcatcctctttacttctcataaggacagcgtcctttttacttttgtctttaaaaccacataaatgtagtgcaccgtgaaaaataaccctgtgcagctcctgggctaccggtaccttaaacttatctgcattctccagcaccctatccacgctaatgtatatttcaccttccgtaatggccgggttctcccccatttcaaaagttacgatatccgtatacgtgtcgtgctgcaaaaactgtttgttgatctccaacaagtaagcatctgaacaaaaaacgtagtgtaaactctccaatccctgtccttctgcagaaaaaagatcacttaaaaacacctttagcttcctcttttcttttaaataatcctttacctcgtgcgatgtaaactgaatagccatctatactgaaaaaatttatgtagatgtaaaagtaaagtgaaattttggattggatgacctttctttttgcatattggctatacagcggtaactttgcttatcattcataagtatgctccccattgtgctggtactaagtttaaacagattaacaagcaggaaatgaaaaaaggcattataaaactatcgtccctgtcgacaggaaaaagcgcgatcattatagaatttgcgaaagacgatcttcatattaaactgatggaaatgggctgcgtaccaggtgaaacagtaaaaattgaaaaaattgccccgttgggagatccgatttcaattatggtggctggctataatttgtcacttagaaaaacagaagcagatcatatttgggtagaggaaatttagttttcctctacttttttcttgtttttatccccaaaaaccaagaaaattttataacaaaaagagcattttccggaaaaaacacacttttaccgctatttttccacacattcttgagcttttttcttccttcaatgaaattttgatggactcccccacttattaacaaatcttccaaaagaaattcagctttctctttagtttcttagccgaattttccctgatttattaataattttccttttttacccctattccgacattttataccaagaaatttttgagggaaattcttcttcttaatgtcgccggccagattccgttgtgaaacattaacaatttgcagagcgtttagaatgaatccagccaaaattctccggcgttcccctgcacaattgaaaaacacgcaaatctcagcaccttctcaaagcgcctacaatgcatccccagtgtataattcccgaggtataaaaatatccccgattctcaaagcctacccaatgagctgagcgcgcctccgttttacaaaacctgatccgagccacgaagaataaaaatattcaattctcagcgccctcctgagccgctcagaattacaccggaatatcatatccgggcttatacaacaaatcctgtcgaatattagattctcagatcactacttgcatcctgacaatcgcctgaaaatttccagcgtgcatttttaaaagcgggtaaacaaatattcaattctcagggcactacaagtgaagtgagactgcgatgtaaattgaataaacaggaacaagtgcaaggagctattaaatatcagattctcagcgccttgacaaagcgctgagaatcgcatgaaatatgtgttgacaaggctaccccaatcaacactctattctcagcaaactacaagtcagctgagaattgcatgaaatataaaatctcgggataaccccagtaaaaagaaaaagaatcaatcctcatagccttctttaaaaatcaataagctgccgggtcagaaagcatttatttgtttcaaaaaacatggctgaagatctcctaacaacagaaatagaaggtcactaaagagagaaaaaccgtatggatcaaggtagttgcaaaaaaaataaggggttgacattgtaatgaaaatcaaaaccatggggtatccctgtcttctaaaaaaatattgaactgtcagggccttaaaaaaataactactgagacttccttaaaagaaaaattacacacacgattccatgcaaataagaaatatctcattctcacgccaatatcaacgcgctgagaatcaaatattctctcaaatccttcacttacccaatacctcctttttatttttaattctcagggcactaaaaaactatttcaaagggtttttaacatcaaacaaatcaggggtccctgtattgttgcgcttttatggagaatggtgtagtccaatcacagataagagattctcagggcctttgtaacacgctgagaattaatcggttcgtacatacatacgaaggccgtcagaatacaagattctgacggccttcggtaaatacctactttcctatatataaaaaataaaatttaaatagtgttgttaatcagtcagttaaactaaagcccggcttgtgcactaatttccagcatacgctcaattggctttttagcggctattctcagactttcttccattgtaatttccggttgttcgtattccatgcacagatacaatttctccagtgtattcagtttcatgtgtggacagtcgttgcaggcacacgcgttattgggcggagcaggaataaatgttttgcccggattttccttttgcatctggtgcagtataccggtttctgtaacaacgatatattcctgcgcatcatctttctgactaaacttcagcaaaccagtggtggatccgatataatccgcaatagccaaaactgccggttcgcattccggatgcgctatcactttagctttggggtgacggattttcaattttgtgatcttttccagggagaaaatctcatggaccatgcaggcgccgttccataaaaccatgtctctacccgtttttttgatcagataggcccctaaattcctgtcgggggcaaatatgatcggctggttgtgtggcacgctttcgatgattttctcggcattggagctcgtgcaaatgatatcgctgagcgccttgatacccgcggagcagttaatgtacgaaatcacaatatggtccgggtaacggtccctgaacttcttaaacagctccggaggggcactgtcggccaaggaacaccccgccttcaggtccggtaacagcactttcttctggggactgagaatttttgcggtttcagccataaaatgcacacccgcgaaaacaatcatgtcggcatctgttttggcagcctgctgactgaggcctaaactatctccgatgtaatcggcgatatcctggatatcgggttcctggtaatagtgagccaggacgatagcgttttttttctttttcaaattttctatcgcttcaaacaaatccagagaaggatcgactgatatatccaaaaatccgttgcgttgcaaattttttttcgcgtcagcgatttccataatcatagctatatacttctttaaatatttaaaagaaaagcccactactattagggctgtgaatatgtggaaatttaatttccagctcacgtacaaatgtagttgttattcctttttattacgctttccacacgaaattaacatgccatttccgcgccaatactgggttttactactttcatccacatacgtggatatcctccaaggttaaaatctttttcgtgtgtagtgtattaggaaaatgttaaaagaagacatttcgtatccacatttccacctccgggtttttaagggtaaatttaaccacaataacaaaattagttttacctgtggacagaggcaccttttcccaccttattttgcgttttacaggggtttttacacatcaattgtggaaaagaatctcttggagatgaaaaatggtcaaaatgcatacgggcctaaattagccccgttttattcacaaatttatgtgaattagaaaatctgcttttttcacatttgtgaataacctttttttaggttttgacacttaatttcggccaaatacctgctgtaatcagtgtttaaaaatattgggcccacaaaaaaaaggaagatgttaattggcccttcatgtggaaaacctgtgaatgttacatagcccacaaaagtgttataagcacctgtaaccctttactgtattgagtttcagagtaaaaaatactcttttgcagttacagtttatttattctatttttgctatccttaaaaatgtagactatataatatatgtcagtaattcagaaaatcagggacaagtacgccgtcatgatcgttgtagtgatttgcctggctattgttagtttcctgttgcaggatgccttttttggcaaaagttctctatcccgtcgcgataccagcgtgggtaaagtaaatggtgaagatctcgatttggcagagtatcaacgtcgaattcaggacgcagaaaacaacgcgcgtcagcaaatgcctaatattgacgaacagacccgtcagtatatccgcgagcaggtttggaacgaatttctgaatgaacaaattatgcaggctcaatacaaagtattgggtatcgacgtaactgaggcagaagtggtagaccaaatcaaaggtaaaaaccctaacccggttgtggtgcagcaatttacccgcgatggccagtttgaccgtaatgctttgcaacaggctatttcacaggcaggcagcaatccacagatccgtgaaggcttgcaccagctggaaagctatattgcgaaataccaggagcgtttgaaatacgtgacccttgttaaacaaggtatctactatccaaaatggctggcagcgcaacagcaaaaagataacagccaaacagcgactgtatcttatgtaagcgttccctatgctaccatctccgattccactattaaagtaactgatgcagaactcgatcgctttatccaggatcacaaacaactgtttaaagtggaagagtcccgtaaaattgaatatgtatcctttgacgctatcccttctgctgccgactcagcagctgctattcagcagataatggcgatgaagctggaactggatactacaaaagacaatatcgccggttttatcaaccgtaattcagatattaaatattacgacggatatatttccaaaaatgaagcaaaagttccgatgaaggattctatcgtgaatctgcctgtaggaactgttttcggaccatactacgataataacctgatcgtttttgcgaaaatgattgatcgtaaaaatatgcccgacagcgtaaaagtacgccatatccttatcgcttccggcgctcagggtggtttaccggattccatcgctaaaaaacgtgcagatagccttgagctggctgtaaaaggcggtgcagactttaaagccctggttgaccagttttccgatgatccgggtagcaaacaaaccggtggtgaatatgagttgactccatcttcccaatttgttcctgaattcaaagacttcgccttcgatggttcaaaaggccaggtgaaagtagtaagaacacagtttggttaccatgttattgagatcctggatcagaaaaatattggtcctgctattaaagtagcgtatctcggtaaatctgtagaggccagcaaagaaactaacaacaacgcatttagcgctgccagcggttttgccggtaaaagcggcactgctgctgcttttgagaaaacagtacaacaggaaaagctgaataaaagaatcgctgataatgtacgtccaatggatttcgtgatccccggtatcggacaatcacgcgaactggtacgctgggcttacgaatccaaacaaggtgatgtaagcaaggtatttaccttcgatgataaatacgtagtggctgttttaaccaatgtacgtaaagaaggtactgctccgctcgcagatgtacgtccccaggtagaagctgaagttaagaaacacaagaaagcagaacagatcatcgctaaactgcaaactccggctaccctggatgcagcggctaaatctactaaccaaccggtgctgaatgcagaaggcgtttctttcgctactccattcatcgcttcccttggctttgagccacgtgttgccggcgcatctttcaataagaactggggcactgcaaaagtatctgctccaattgaaggtaatgcaggtgtatatgtgattaaagtagacagcttccagccgtctgcccaaccagcccaagatatcgcttcccaacaggcggcttacgaacaaggtgttaaatccatgctggatcaacagctgttcgaagtgctgaaaaagaagagcgatgtgaaggatacccgtggtaaattcttctaaatcactacattttttactgacataagaaaagggaagcactactgcttcccttttttatttcccccttttagtgcctttctgcccttattcctattcctgcgccgatattcgtaaatttgtattcttaaatagggacaaaaatggaagaaatcataaataaagtagcgcagagtggactggaaaccattgatttagaacagttttacccaaaaggggaaattgttgtttttgatatgaaggattacctgtttatggagctcattctgaaagaaaaggatttccgggcggctatgcagtcgcacgactgggagcaataccgcggaaagaacgtggggcttatttgctctgcagacgccgttattcctttatgggcttatatgctggtgatgaccaacctggaaccggtggcggcctatgctgctttcggagacgcagcatttatacacaatacattatatctcagaaacctgggagaaattgacctttccgcttttacagataaaagaattgttattaaaggatgcggtgataaacgggtaggagaaattgcttacgcggaaattacacgcctgttgcgcccggtagtaaagagtattatgtatggagagccttgctccaccgtgcccgtgtataagaagaaaagctaaaaccagcctcttttccggaaaaataataccatcagcaccaataatatccccatacctcccaatgtaaaataatatccattgggggatgccagttcaggcatatgctgaaaattcattccgtagataccagcaagcagtgttggcggcgccattaatgtagttaccaccgccaacactttcatgatttcattcatcttcaggttcaactgcgtatgatacatctcctgtaagttcagcaccatatcgcggtagttatccgccagatcattacattgaatgatgtgatcgtagatgtccttgtagtatttagttactttatcatccagcagatcgctctcacttttcagaaagccatttaccaactcccttaccggagcaatagcccgtttgaacaggaaaacctggcggcgtaaataattaatccgcgccaacgtacgggtgttgggttgatgttgaaccaggtcttccatcatttcaatccgttcccccagcttatccataacaatgaagtaattatcaataattacatccagcaatgaataacagaggtaatcggcgccaccattgcggatcctggatccggttatcagcagcttggcccgcacagggtcaaatacatcccgtgcagggtcctcctggaaagagatcacaaagtttctgcccagtacaatactcacctgttccaggtcgatagatgaggtttcactattgaaataaatcatgggaagcaaacaaaacatccggtcattgatttcatccatctttgcccgttggcccacactcagaatatcttcctcaagtaacgggtggatgatgaattgttcacataccgcatgcacctcttctttcctgataccatcaatgttgatccagcttaattggggagcgttggcatatttaaaggtgtcctctattttgttcagcaccagctctgagcaaagattaatattataatcaaaaacagtgatcttggttttttccaccggcttgcgggatgggactccttccgccggattaaagttcatgatgcgttgcttcttcaccttgaacgggtttagtacttgtactacgccgggaataggcaatttatttttgaaggccatatatgctgatgttagcaggattgattaccgaatttaaagcaaaaatccgttaatagtagtgagcggaactatcataccgggttaattctatttgtttgaagggaaagagattaggtgccgcggttgtttgaaatcactcgtacggtgccgaaaatatatgcgtaatttaaatcctataggacatgtggactatttgtaggtgtttgataaatgagattatttttttagagagataaaaaaagtcgcccgtcatatttacagccgggcgactttttttcaaattctgtgaaggataacaatatccttagaactttggcaactcaattaccggaggagtgccggtggcagggcgttcaaacaaatcgccatactgtgcattggctggtttgaaaccactgttccataaatagaaccatccgttttctgagccgccgccataatcaagcctgtcttttgctttagcggtggcatcattggagaatttggccttggtaagttctatccattcgccggtattggttttaatccagtggttaccgaaatatcctttgcggccaagatgaccattttcaaaagagaaattttccaggaaggaataaaggtgtcccatgtactttccgtcttttggcgccctgaagctggcaatcagtttccactctttgtgttccggcacataaaagtatgcggtgtaagtagtggtatttcccgttggcacgctgtgcatcaggaaacgataggtgtccccggctttccagttgtacacccaatggctatgtccaccggtgccttcgccgccaaacccgctggcgtctacactgtctccttttgccagcattactacctggtcttcatactttaccttgctgcgttcctctggttctccaccggcatcccatacagaaaaaataattcttctttctgtgggagaatttacctgcataccaaaatagcccctgtgaaaaccacaggacatgaaataggtacccagtttatcttctccttccggcaccttaatttctccataaaaccattctacatttttaccttcgggaacaggatagtttaaatgtacagaagccgcacggcgccagggtttggcgttatactgcatatcttttaccgcggatccggaaaggcttacgctttttacatctgcatatatacttcccttcttctccactccttttaatgacacacagtaaaagcctgctttttttattgttgtttgtaatacgggtaccgttacaaaatctgtattgttaggtatgcttactattttttgagcgccatttacggaaacagataccttactttctgcatcggcttttgccagtaacgacactttgagggtgccgggattcgccacatggaaataaaaattaacggtattgctgttatccgtccagtttacaacgccgtggcgttcactgatttctacatgttcttccaccggatcggcataggcggcaaagccgggaagctcagccacaggcgcctgtgcaaaggccctgttggcagcaaagcaaatagccagcgatgctgcaaggagtgttttcttgttcattgttcttaattgtatgtcaacaaataaagctgcatctgcttccaaatgcaattttgccggaaaaaaattacaatcgaatgagattcctttttatatcccatgcaatcaacggtatgtgcattaatttatacaggcgcaaacgtgctgatcttgtgagaggtaccgtgcacgtaggtgaatgcaaagggaattgtttttgtggcagatgggatgctgccgcggtatttatctgccggaggcagcatattccaaaaactataaaatattattttatggcaaaccagttaaaagataagagaatagcggttttggtagcaaacggatttgaagaagtggagcttacaaagcccgtggaggcgctgaaggaggcaggcgctacagtagatattatttctcccgaagggaaaactgttcgtgcctgggcggaaaaagactggggaaaggactacccggtggacaaggacataaaagaagtggtggcatcttcgtatgacgcgttggtattgcccggtggtgtaatgaacccggaccgtttgcgtaccaatgaccgcgtggtggcttttgttaccggtttcttcgacgaaagcaaacctattgccgccatttgccacggtccctggacgctgattgaaaccgatgaacttgatggccggaaggtaacgtcttatccgtctttaaaaacggatcttgaaaacgcaggtgcattatgggtggatgaagaagtggtgaccgataagggattggttaccagccgtacgccaaaggatttacctgcgttttgtaagaagatgattgaagaaattgcagagggtccgcatgatcagcgcggcaatgaagcacgtaaagatggtgtacatcaattgggataatacccgggaacaggagtgagcaacctcactcctgcttttattttttcttctttttgtatttcacttctacattagccaccccagtgttcagcatgcctattttggaggcggctttgtgcgacagatcaataatgcgccctggtacaaacggtccgcggtcattgatacgaacctttacgctttttccatttgcgatattgataacagtaacgcgcgttccgaaaggaagtgttttatgtgcggcagtaagcgaccgctggtggaaggtttcgccacttgcggtacgttttccatcgaatgagttggcataataggatgctttccccgtttcggtaattttccggctacaggaagaggcgcctgtcattatcaggataatgaacagcaatacccaattgcgttgtgagggtgcagggatatacatgacggatagcgatttagacaatgacctaaaaataagtcaatttcccgacgctttcagtagctcgtggcggggaatttgatgaatggcaggcggctgaacaatgtgagagatcagctgtttttatctggcactcatcctaacaaattacttatggcaacacttgtagcggatcaattagtagatatgctggcaaatgccggtatcaagcgcatttatgcggtaaccggcgatagtttgaatcacatcaacgatgctgtgcgtcgtgatggacggatccaatggattcatgtccggcatgaagaagtgggggcttatgctgcaggagcggaagcacagctgaacgggctggcttgttgtgccggcagcagcggacccgggcatgttcacctgatcaatggattgtatgatgcgcaccggtcgggcgcatcgctggtagccattgcgtctacctgcgctaccaatgaatttggcagcgactatttccaggaaaccaacaccattaagttgtttgacgattgcagtcattataaccaggtagcggcaacagccgagcaggcaccccgcatgttgcaggctgccttacagcatgcggtgcataagcacggcgtggcggttttaggattgccgggagatgtagcagccgctgatgcaaaggagatccctactgccacgaagctgtatcatcctaagcccgttgtttgtccgtcggcaccagaattaaagcagctggccgggttactcggcgatgcgaagaaaattgcgatctattgcggcctgggcgccgtagaagcacacgatgaagtagtggctttgtcgcaattgttaaaagcgcctattgcatactcgttccgcgcaaaaatgggtattcagtacaataatcccaacgaagtgggcatgacgggtttgctgggattggcatcggcttataaaagcatgcatgaagccgatgtgttgttactgctgggaacagattttccgtacacgccatttattcctgagaaggcgaagattatccagatagatatccagccggaaaggcttggccgcagggccacactggagttaggtttgtgcggggatattgcagatacactgaaagcgcttctgccaatgctaaaggaaaataccgaccggcaattcctggacgaaatggtagcattttaccgggaagtgcaaaagaaaatgcagacttatgtagaagacaccggcaaggagaacgccatcagccctgagtatgtagcggctaccctcaataaaattgcagcagatgacgctatttttactgtagatacgggcatgaccaatgtttggacagccaggtacctggaaggcaccggcaaacgtaccttgctgggatcttttaaccatggctctatggcgaatgccatgccgcaggcaataggagctgcgttggcgcaaccaggccgggaagtgtttgctttgtgtggcgatggcgggttaacaatgttgctgggcgacctgatgaccattaaacaatatcaactgccggtaaaagtaatcgtgtttaataaccgcgccctgggcatggtgaagctggagatggaagtggcggggctccccgattggcaaacggacatggtgaatcctgattttggggcggtagcagtggccatgggcttcacagcgtttaccatccgtaaaccggaagaggtggaaagcatattggcccaggcagcaaaaacggcaggacccgtgctggtaaatgtatttactaatccagagtccctggctatgccgccaaaagtggaatttgcccagatgaaaggatttgcgctctggatggggaaactgatcctcagcggaagatatgaagatgtatttgatgcggtgaagtcgaactacaagcacctgaaagatgtgctgtaaatatgaatttatggggagatgatttcaggaccatctccccataatattaaaacggataaccgatggcaatgttaagaatgagattttttttgcgccagtcgggatcgctgaaatctattttatcaaacacccagcgttcgttctccggcaggtaaggaacacggaatgggatagccagatcgaggcgtactactacaatagaggcatcaatgcgcaaacctaccccaccgccaacggcaatgtctttataaaaagtattgaaggcaaatttactacccggcttgtccggaacatctttctgtaaccagatgttaccggcatccacaaaggctgccacattaaacacactggccacgtgcacccgcagttcagagttgaattccagcttgatatcgccggcttcattagccagcaaggcggaagtatccacggcggggttgtgataagatcccggaccgagggtacgcgccctgaatgcccggatgctgctgctaccaccggtgaaaaactgttttacaaaaggcagggtggctgagttgccatatggcaaaccgtatccaatcaacaggcggtttacccattgtttgcctttgcccagctgccagtagtggcgcgcttctgcagtgaatctttcatactgcgcaaatgaattcccaagtaatgttttttgcccggtatcatttttcggaatgatcaacccggcaatgtttcctgagatatctatattgccgctcaggtagaaactgtgtacccggttggcttgctggttattgtaggtgatcgtatagttgccgccgaggataaattgtttttcaatagcgttgcgctgacttggatcgtttgccaggatactgtcgtatgccggtgttgttttggtaggcaacacataggtaagcgcaacgggtgcaaagatatgactcaggtattgtgtccgttgccacaggtattgcagctgtagcgtatatgcgttaaggttatacagatcggcgcggctgtataactcatagctggcgcttattcttgttttaggtacatagggtgtgcggatgttcaatccacggaagggtgtgatgaacctcggaaaagtaacagctgcttctgcaccgaggccatacgaattggagcctcctgcatttttattaccggtttgccattccagtccgccacgcaacccaatttcaagcaatgctgcagaatggagccagttgcgatttttagcggtaatctgtatttgtgatccaatgaacccgttagatttagaggtaccacgtagttctgtttgaagggaacggcgtttatatggcgtaaggaaaagttttgcgtccagccacccgctgtcgagtgccacccggttgtttaccatggccctgtagttgttggcctgggaggtatcacgggcgtaggtgctatcgcgccggttcaggttcctgccggaggtatcgcgccgcctggagctgtccctgttgccggtaacattggggccgccgcccactaagttgtgaatagaggtatcccttaccggcgaaaattgtccctttacaaatttgaatacgcccaggttaatcagtctttgcagggtaatattatgtgaactcaggcgatacaggctatctggccgtaaaaacacggagcggtcaaatgcggatgatttaaaccggtgggcggagtccacaatgtaaatgcccttgtatcttaccggagttccctgtgtagaagcggagtcgttatccagcgaatagtccgggaacagaacgatgtcatgcatcctgtaaggccggagcgccagcagtggcgtgttgtcttttatctttacaaagaggtcaaccgtaccgctattggtactatctacctgtaccagtaaataatcaggtgtaaaataataataaccttgttctttcagcgcggcgtgtatccgttcccgttcggctttaactgaatcgagcgaataattggcgccaatgatcaaagagctttccggtttggtataagtaacggttttaccgatggcgctactatctgtcaaataggtgacacttttaatggtataccggtgattgggagtggctgtgtatttgatggaagcttttttcttgccagataacttaatagcagaaacaacgccggcctggaaatagccgttatccaccaggtattcttccaatacctgtgaggtgtagtcgggttttgcctggctcagcaacacgggcggttccccccattttcttcgcagcaggtagttcaatcctttccctttgggttcattgcctaaattgtacagccacaacttaatgggcataccgagaaatttacggttcctgttgggacggattcttttatccattccttccatgagcgagctataatctttcggtctttttttagtaatggtgtcagtgatccattttacgtcgctgccagtatatagccggtctccttcaggtacggtacgtgtggtactgcaggagctgactgccaggattaccaggcataacaggctacagcaaataatgatatggctacttacttttcgcatcaggcgttgtcgtatttttatcgttcttctttttggtatcgcgtaaccgctgttttttagtatcagttttggaccgctgcagaatttcgcggaactcatcataatccatgatcagtgcaaaggcaactcctgtttccactacctgtccttcgagcactgtttgactgtcgttgcgctgatatacccttatccggtaacgtccgtcgcgggtaagtttatattctacggagatatcaccgatcagggagctggcattttgctggcttccctgcaacatgatattggaacctacggaaacggttaagcgatcattaaataactgtttggaggcgccaactttcaggttggtggattcctgggcggagccggaggaataatcttcctggttctgcaggtcgaagttgagatccactcctttgatcaggttgcccgccatgttattgagctgttgtgaaagtattttacttacactgtttttcgctgcctgtcctactccaccgccggagccgccatcgagtgtactcatagggtcatccgggataaaggagttcagcaccagcagtcccattacctgtttattcagctcagagggcacctggttaatttgtttcaggcggttatatggtgttccgttcagggtattcctgtcgttctctgccaggtccaggcggaagctgatatcaggcttcatgagattgcctttgatcatcaggtatacctggaagggcatccgttgtttataggtatttcgttgttcggcagacatgctttgaagctgatctgccaccaggtcgtaggccggcgcattcaccgtgtatttggcggtgatatccaggtcggcgctggtagcgtctccattgaacgatacgaagctgcccttttctatatcgaaagagcgtttaatgagctggttcagtgacatctcgtatttaccttccgttatttcgtagcggccggtaagacttaacttactgctgggatccagcgtggcattaatgctggcggtaccttttgcctgtacataatcaccgttttgtgaatcgatgataattttaaggacagattccggagtaatatcgaggttaccggataagaacatgccttttaaccgcgtggttttaaaccgaaggctatcttcacgggcgagtagtgcagaatcgacaggattggatttatccacaaattcgatcacgccttccctgttggcgagtcccggctcctcttgcggcagcgtcatggtaacgctggatttgtcgcgcagctttacgatggcatcaattctcggcaggtcgagtgtgccgcggatcttcactttactatctatataagcgggtccataaatccactggtccgggttttgctgccggccaagagccatgaagttatcggcagtaacatcgaggttaaagctataccgggtgaaattcctggtattaatgcggccatctaccaccagttcattattggcgctgtcggctattaccaggttattcagttgtattcctctttcatccagtacaatatcttcatccggtaaatggaaagtgctgccgatcatggttaccatgcctgcagcattatcgaaatgcaggcttcccaatactttgggggccgacggtgtacctgtaatattgaactgcccggtggcactgccggacattttagtaacattgcccatcgtgaatggttccagcgaggcgatgctcagtttattgatatccagctgggcattgatagtagtgtcgtaggtgccgtccacctttacatcattatcgttgccggttaatccggctgtaagtttatattggccagggccgctgttttccacattggcgtctaatgttcccatgcgtgtattcttcaccgttagactgtctactttcagcgtggcgtgaatcagtggtgtttggttccagttacgtacagtcgcttctgcattcaggatgccgttggccagcagggtgtctgttgccagtagggcggtgatggtcgacaatttaaaattggcgatgttggcctggagtgcaggagtggcgctggtatcaggcttggtggccacctggatggactgatcgccctgcgacagtttgatattcgccgtatccggtgcgccatttttcatccggagaatattgttctctgccacagtccattcctgtttgtttaacagcagtccgggtttgagtgacagctgcatggcattatctttcaggaacgtaaaaatgccgcccagtttatacttgggctgccgtttaacatcatccagtactacgtcaaagtcaaccacaccagtgttggcataagccgtaagataggtatgttgcagcgggaatgtagggtgcgccatgcgggccaaagatgccccgagccgcaaagaggtgtcctggatagatacgcctatgcgcaggctgtcgacctgcagggaatcataattaattttcggaagatatgcgtttgcgatcagcaggctgctgtcgctgttgaggcggccattcatcaccagcggcacttccatgcgcagtgttggaatcatctggtgtaaattctttggccactgtaaagaggcattccactgcagtgattgtccgccggggacctgtacaatagcgccggaatcggccggcattaatggtttattgataatattggcgaaggcggcccccacttttgtataatcgatatggccgttggcgctgatcaggccaaacggactttttaaggtgaggtattgctgatccttgtattcggctaccagggagatgctgtccagcggaaatacctgtccctgtgtggctatctgccattttgttaaaaaggcattgccttctatgcgctgtggttctatgctgttgaaatctgccaggagattgccctgtaccgttaacggttctgaataccaatgggtggcatacaggtcggctttggccagttccatatttactttcagtccctggatggtagtatccaccatttgcccgctgatatcgaaagtggcggtgatgctgctatctgcgctttcgccctgcgcttcaaaatcgcctttgttgataccggcgattacgcttacgtcgtgatacgtataggcgttataggtagcttcatccagttgtgccgtggctttggctaccatttgttttagcgtatagccctcaccggtagcgctcagtttgccggacatccagccgtaggtagtatcgtatagcattgctcccgggtttatgcggaagtatggaatgctgatggtgtagctgctgcggatgctgtcggtaatattgacgaggcgtgcgttgatattggcgttggcggtttcgcttttcagttgtaattgggtaacgaggtccttcatgccgcctttgaacataccggtaatcagcatgttttccggcaggcgtggcgtatccgggagggtacccgcgggtagccaggcgcgcaagggtttgttgcccgtttgtatataaagcgcaggaagatcggcgctgagcagatccgggtttgtagcatggagcacctggccattgtctgttttgatcaggttgccttcatgatcgttgacgtagagctgtttaatattcagttctcccaggtttccttttaatatagccgccagcgttagttgtttattccatagctggtcgaatgatttgtttttgcgtgcgttgggaacgaaggggagccactctcccagtgctacatgcacagaatcgagattggcatccagtccgagctggtccagatggtcggaaatgccggaccaggaaggcactgttacgatgatctgtttgcggaaaatgcttttattggtttgcagcaggaagttgcgcagcgccagtgtataaggcgtgaacaatacgtccatattggctttgcggatggtaaaaccggacttatcccgggcagtcaatgattttattcccaccataatactatccggcttataccggatatggctgattttactggagaattgagttagcagcaggtgattatagtcaggatctggtcccgcggctttaggtgcggggccaccgttatcgtagcgcagggcaagtttatcaagatttacctgggtggcaaatacctgccaggtatttggcgtggtatcgtttggcgcggcgggaacggagtcctttccggcaaccatcattaccaggccggcggtgttgctgatggaaagatcgcccatctgtatacgggtagagtcctggtccaggttgctgttgcgtaattgcagggcgcctattttccaggcggtggtaataccggagccttcatctgcatacaggaaatgactgttgttgatctgtagttttttcaggagcagatggagtgatgcgctgctggtatcggccggtggtggcggcggggcggcagaggtaacagccggggcgatgtacttttgccggaaaaagcctttcagtccatcgagggtaatgcccctgaacgcgtaaatgccatcatctatgaggaggtcgtccggatcaatgtgtaaactatcccaggtgagcactgcagacatgccgccctgcgcatcttcatagcttactttcactttacgaaatgaaatgtctttcagccggaattgcaaggtggtgccggtttccggcgccagggtatccttatccccggaaggggttacaaaggcatctatggcaaactggtaattaaaggcggaatcgccggggtgccggtaggcatttaccagcagggtgtcccactcgagtttatctattttcagttcattgctgatcagcgacaggaggttgtaatgtactttgagggagccggtataaaaaagggcctggttggcggtgtcggccacatatacattccgaagttccaggtactgccagccacgtgcgcgcaggtagccgatctgcactttggtgtgcagttttttccggaggtataattctccctgttctcttaagtaattctggacgccgttcagttgtaataataaaacagccattacgggcaataggagcaccgcaacaataatccatataagccatcgccaccaggggcggccgtgtttttctccggtttctgctggttctgtcactatgatgtattacaaaagtaaattactgaatataaacgcaaaagcacgtttatggtttactttgccggcaggatagtgcaaccgggcgcttgcctgcgggtacaacaaaatccatacctcaggggtaccggcaacgaatcgttattgcaagaatacatcaaatacggtaacggacatactttttttggcgatggaaacagaatggggtgagtagtaatatgcacagattggcgaaaaggaaatggaccggacgggttggtttttattacttagttatcctgattcagggcatttttatcttctttttcaattcttctttttactttatccacatcttctgccgggggaaggctttctggttttacacctctttccaggagcacatttctaacggcggtattgttgtcaacatgttcttcggtaatatcctcttctcctttcaggtctttttccagtacattatgactggtgagttctgtggcgaggtcttttgctttaatggtaatagtgggaaggaaatcggccaatgccctgttttcgggaatgaccagttttctcttcatatcgcgggtggtaaatcctccgaaaagagcctcatcgcccttcgagcggatccgggcaaatcctttatcgtccacccctctttcgtaaataataccggataatgccttttctgacttcgatagcttttcccgggcattaatacggtcaatatccagcaatcttttttcaacaatttcctgtttgcgggtttgcacggcaaagtaggtttgggcaaatgcaatcggatctttttgggtgtcgccactttgagcgatcaggtagcaggcgtaacgggtaagcgcgatgtcctgaagttccctcgttgcatcactgccaacagcgaccattttgctgatgtcagcaaaatggtctgaaaccaatacaccactgttttcacaggaggcttttgctttgtcaattactttcaaaaagtttctccactgcgtatagccaagaatttgctgcaattccctggcgctccagcattcgatacccttgtgttcataacaagcctgttcaaattgtttaaacagcgcttcaattaattcttttttcatgaaaaaatatttattcatctcacaatattgtaataggcacaatataccaaagccataacagcagtgggttaacgaaacttaaacagtatcattttgaaagaagaataattactttgttccgggtttattccgttgattaaaccggaagatataatactccagctgatctttcttttccctgtcgcccctgaattcgtcgagcaatacgctgtcttgcgggagaatatattttttgagattgtaggcagatagttccaatatctggcctgtcaccacattcagcacttttttgagtaccaccggtgtgctgatgctgtttgttgtcatatcggcctggtttaaatagccccgggagggttggatgccgtgcagggcatatatgcagtagtagccgatttcctgtagtttattaagaccgttgtctttgatgtagatgttccttccgtcgcaaaagccccagtagtttttcagtttgtgttcctggccggcgccatcccggagcaccaattcattcctgttggccagcagatagatctgcgcggcggagctgcggttttttataaccaggtctccttcttccgaaggattatttgattgaaattcctcaaaggttttatacaggcctttctttagttgaggtgcgtctgtaatcagcacattttgcgctgctacggaaataccgagtaacagcaggttccaaaaacacaacagttgtttcataataaacaaatgtattgggtttaggaagtgaggttagccggaaatagctgaacaccggctttgtttctgctgatgtttgaattatgtctttaaaatcaggagagggtggcgttaacagcaggcattaagcagaagctggcggtttcccgggagggaatcctgtcttttaaaaaaatataggccgggtaaaaacccggcccggctgaaggttacaacaaaatctaaacctgcttatgagaaaaattttgatttacagttttgaattataaagccattgcctgcagtgaatggtctttgctttccagctgggagctgcccatcaggaattcgtccacttttcttgcgcactcacgaccttcgcttattgcccataccaccagtgactgtccgcggcgcatatcgccggcagtgaacactttaggaatagatgtcaggtagtctttttcggtagcttttacattaccgcgttcatctctttccacttccagctgatccagtaagccggtatgctgcggatgtacgaagcccatagccagtaaggccagttcgcagggtacatctctttctgatccgggaacttccgtgaattttgccggtctgccgtcggcgctggcggtccattgcaggtctaccaggcgcagggctttcaggtggccgttatcatctccgataaaggatttggtggcgatggcccatttacggtctgctccctcttcgtgggaagacgatgtttttaagaccatcgggtaggtaggccatggcatatacggcgtacgttcgcccggaggttttggtaataactccagctgtgtaacgctgttggcgccatgacggttactggttcccacacaatcggagccggtatcaccaccaccaattacaattacatttttgccggttgccagtatatcgctgccttctactgcaatattgcttactcttttattctgctgcttcaggaagtccatcgcatagtgtacgcctttcagctcacggccctggataggcaggtcgcgtggaatggtggaaccaccagccagtacaattgcgttgtattctctcagcagatcattggtactaacgttaacgcctacattggcattgcattgaaacaccacgccttcttcttccatcagtttcacacggcggtctactacccatttttccagtttgaagtccggaataccgtagcgtaaaagtccgcccggtgcatcgtcgcgttcaaacacggtaacggtatggccggcatagttcaactgtgctgctgcggctaaaccggcggggccggaaccaataacagctatttttttgccggtacgcatacggggcgcttttgcctgtaccaaacctttatcgaaagctacttcaatgatgtgtttttctatttcctcgatagctaccggaggctggttaataccgagcacacaggcgctttcgcagggagccgggcaaatacggccggtaaattccgggaagttattggtcgaggacagtatatcatacgcttctttccaatcctggcggtatacggcatcgttaaattccggtatcacattacccagcgggcatccgctgtggcaaaaaggcacgccgcagttcatacagcgggcagcttgctgatttaatttattatcggggaagcgttctacaaattcattatagtgaccaaccctttcccggggatccgctttcccgggcagctcgcgtgtaaattccaggaatcctgtaggtttacccataattttcctccacaagtcccttacctgcaagggatattttgatgatgaatgttaattgttcaattaatgacctactttctgaccctgtactttgtctgatttcaacgctgccttgtattctttcgggaacactttcacaaaatgacgcagttggttttcccagtctttcaggataaacttcgccacggtgctgtttgtgtaggcgtgatgttttgtgatcagatcctgcaacatggctacatctgcctgatccagcggatcgaggtcaatcatatcccggttgcagtagttggcgaaagtgcctttcacatcgtatacaaaggcaataccaccgctcatacctgctccgaagttgcggccggtttcacccagtatcaccgctttaccaccggtcatgtattcacatccgtgatcacccactccttctactactacggtagcgccggagttacgtacacagaaacgctcgccagccttaccgcggatgaaagcttcaccggaagttgctccatagaagcaaacgttacctgcaatgatattttcttccgccttgaatcctgcttctccgtgtggatagaggatcagtttggagccagacaagcctttaccaaagtagtcattggcttccccttccagttccagcgttaaccccttagtggtgaaagcgccgaagctctggcctgcagatccgataaatttgaaatgcagggtgtcttccggtaatccttcgctcttgtagcgtttggatatttcgttagacaagatggtaccgatggtacgatctgtattttttacagggaactgctgatataccctggctttcttttccagtgcaggctgtgcagccttcagcagttgccagtcgattacctcgctgatgccgtgatcctgttcttcctgtttgtacaggccggtttcggcagaagcttcttctttatataagatcggtgacagatccagtttttgtgttttccagttggtgatgttatcacgcatctggaggcattctacctgacccaccatttcattgatggtgcggaagcccaggtctgccatgatttcgcggagttcttccacgagataggtgaacaggtttaccacgtgctgcggatcgccggtgaagcgtttgcgcagttcaggatcctgggtagccacaccaacaggacaggtgtttacatggcatttacgcatcatgatacaaccttctaccacgagggcagcggtagcaacaccccattcttcagcacctaataaggtagcaatcgcaatgtcgcggccggttttcagctggccatctgtttgcagtactaccctgctgcggagcttattttttacgagggtctggtgtgattcggccaaaccgagctcccatggcaaacctgcgtgtttgatggagctttcaggagaagcgccggtaccgccatcgaaacctgaaaccagtaccacatcggcgtgtgcttttgcaacaccggcagcgatagtaccaacaccagccttggataccagcttcacgctgatacgggcggcacggttagcatttttcaggtcatagatcagctgtgccagatcctcaatagaataaatatcgtggtgaggaggtggagaaatgaggcccacaccgggtgtggagtgccttacttttgcgatccactcatccactttatggccgggcaactgcccgccttcgccgggttttgcaccctgcgccattttaatctgtaattcgtcggcattggtcaggtagtagctggtaaccccgaaacgggcgctggcaacctgtttgatggcagaacgcatagagtcgccgttttccagcaattcataacgcagctcatcttccccaccctcaccggtattgctttttgcgccgatacggttcatggcaatggccagtgtagagtgtgcctcatgggaaatagatccaaagctcatagcaccggtagcaaaacgcttgaagatgctggatgctggttctacttcatcaatggaaatagaaggacgattctttttaaacgtaaacaggctccgtaaagtggctgctttttcgctttgatcgtttactgcttttgaatactttttgaaagcagcatagtcgcccatacgggtagccagctgcagatagtgaatagtagtggggttaaagagatggaattctcctttacgtttccactgatatacgccaccctctgttaaacgctgcaccggtgtttctttacgaccgtagcccatccagtgtttagccagtgtttcacgggcaatttcatcgagccccaatccctggatacgggaaacggcgccggtgaaatatttatcaacagttgcctggttgatacccaatatttcgaagatctgtgcaccctggtatgattgcagggtggagatgcccatcttggagaatactttcaggaggccgtcacagatagctttgatataatttttcttcagtttatctacgtcgagcgcggtgtccagtttgccattcagcttcatatcgcggatggtgctgagggccaggtatgggttgatggcggttacgccaaagcccagcaggcaggcaaagtggtgtacttcccaaacatcaccggcttccacgatcagtcctacctggccacggtaacccttgcggatcaggtggtggtgaacggcggatgcagccaggatagatggaatggcggcgtgttctgagtcgatagcacggtcagaaaggatgatcacttcaaaaccgtcttccacggcgtctaccgcgtagcggcataagcgggccaatcctttttccagggagccgggcttaccgtctgccttgaaataagtgtgcaatgttttggcctggaataagccggtatcgatactgcggatcttttccagttcgtggttgttgaggatcgggtggcgcagcgccaaaccatggcagtgcagcggatcttcatccagcaggttaccgttgttgcctacaaaagtagccagcgacatcaccagtctttccctgataggatcaatcggcgggttggttacctgtgcaaataattgtttgaaatagttacagagatgttgtggctgattgctcaggactgccagcggagtatctgtacccatggagccaacaggttccttgccatcaattgccattggggcaatgatgtgatccaggtcttctgtgctgtaaccgaaagcgcgctggtatttaaagatctggtcgtgttccaggtgagtaaaggttactcttggttccggcagttcttccaggcggatcttatatttattcagccattcgccataaggttgctgggagcagatctgttgtttcagctcttcatcacctatgatgcggccctggtccatgtctacgataaacattttaccaggttgcaggcggcctttctctttaatattttttggatcgatgggcaatacaccggcttcagaagccatgattacgcgatcgtcttttgttaccacgaagcggctcggacgtaaaccgttacgatccagggtcgcgccaataattttaccatcggtgaaagaaatggaagcaggaccatcccatggctccataagggaggcatgatattcatagaacgctttcttttcttcgcccatgtcttcgttgccgtcccaggcttccggtaccagcatcatcattacatgcggcagggagcggccggtcatggtgagcagctcaatcacattatccaggctggcagagtcggactggccttcttccacgatgggaagcagcatttccatctcttctttgctgaaatatttggaaataaagtccctttcgccggcgcggagccagttaaggttacctttcagcgtattgatttccccgttgtgggcaatgtacctgtaagggtgggccaatctccagctggggaaagtgttggtggcaaaccgggagtggatgagggcaaaagccgacaccattttctcatcgctgaggtctgtataataatgacgcacctggtaggtggtcagctgacctttatatacaattgttttataagagagggacgcaatgtaaaacagcgatttctctttaggaacggtattgcgaacagttttggaaacgtagttacggagcacaaacaatttgcgctcaaaaatttccggatcgctgatatgataaggacaggcaataaatacctgttcaatttccggttctacagaaagggctgattcaccaataccatccgggcgtaccggtactttacggtaacccagaatttccaggcccagtttctctgcgctgcgttgaaatatttcacggcattcttcacgccagcgtggctctttcggaaagaagaccatgcctacaccgtattttccaaactccggtaaggcgatgcccagtttcaggcattcatcatacaggaactcatggggcgtttgaaacagtattcctgcaccatctcccgtgttctgctcacaaccgcaggctccgcggtgttccatgttttccagcatggttaaggcatcacgtataatatggtgggatttacgacccttgatgtgggcagtaaaacctgttccgcaggcatcatgttcaaattccggacggtataaaccttgcgtttgcttcacttcatccatttggtttagattttttgctttggcacacccttcccttctgacttgcgccgcgggtgatggtgtacgatataattcgggaacggtttaaagatactaaaggaacgcggtattttttgtataaacttttgttagacggttaaaatttagaaaaacataaaaagatggcggtaattgttagaatatttgaaaaaatggctgctccctcaggacaaattggttccattttaaggctcagaccggcacctttaaagtgacccggattataacacttttgtgcgaggtgctttttcaaccgccctgtattatatttgaatgataccctttactaacataaacgcctataccaattttatgctcccaaagctattcatgagtgcgtttttagtgtctgccggatttctgctgccggcccgcgcacaggatgccgccgaagcgccggctgccatctcacaaaaaaaagtaagcctggcgaaggcctccccctttaccgccgacagcctgcaggcgaaagtatccggaattgccattgtcagcgcggtatgggataccgcccgcattggctttttacaaaccggacttttcaataataaggcagaagccatccctgataaggaaatgggcaggtacctgcaggagttcgtaaacaataccttcggaggcatattcacccccggtaagccccggcttatatgggtggtagaagatcttcgcattggggaacgtactcagatgatgggagaaaaagcctacgtccgtgtaaaggcaaccgcctacgtacaaaccggcgacgacacctacaaattgctgaaagccatggatataacacatttgaacaatggctttgatgtaacccaccagcaccggaacaatatctcaaatgcattcaaggaattttatgcggccggcgccggggtcctggattcagtgctggcggacgccgggccgggactctcctatgccgcgaccacaggaatttatgcaaaaaagcgggaactgccggcgctgaaggaccctgttatgaacgatggtatatacctgtcattcgccagtttcctggagaacaagcctgatatcctgcaatatgaaacaaaagggaaagcgggcaaagtaaaggtgtatgctattcccggcgatggccagaaaacaattgttcctgccttatggggtgtggtaaaaaacggggcggtgtttaaatacaatgataaatcactggtagggctttcccgcagcggttatggctatgtgatcacttcttatttgtcggcctatgaaaggaggcaaagcgctattataggcggggccttaatgggcggcgttgccggcgggttgctggggtctactgttgcactgcagcacacagatgccttcccggaattaaaacttcctgcagaagccaccgcgatagatatggaaacaggcgcactgattttttaatgcgcctgtttcccgctgctatggctcgaaaaggaattgtacttttccatttaactgccgcatacgcagtggctcgctgatatgactctcattctgtaatctgtcgagtgcggtgacgatgtaggtatacagcttccctttcacataagtgaggtccttaaattcaggatcggacgattgcgacaggatgctgataattttcgtagggtcgctgacgttaatcgcttcgttttgctcaaaccggtacaggacatactgtttggtgtggccgctggtatcatcatctgcccagtgtatttccagtcctcccggccgttcaaaggcatcaataaagtaaggcgcttcgggtgtttcctttggcagccacggcataatgggccgtaatgcagggtacttataaagacgggtacgcaacgcatcttcaatgcccagcgggttgccgcggaaagaggccgcactgtaaaaaatactgccctggatagtgttcagtgttctcgcttcttctatttgtgccggtaattcatttggatttttccaggccgcattgctgccaatccggtacacgccgtggccaatatacacgtggcggccatagccatgttggctccaccagttcagtaatatttcgtagtcggccagccggtgtccgcgctcccaatagatctgcggcgccacataatcgatccagccgtttttcagccatttcaggatatcggcaaacagatcgtcgtagttggtttgaccgcctttggtataggatccttcctggtctttgtctttgttacgccaaacgccaaagggactgacaccaaactttacccagggtttttctgctttgatggctacgctcagcatttttatgatggcatctgtattggcgcggcgccagtcatctttcatcatattgttgccatacaggcggtaggagctgttatccgggaattcttttcccggaacccggtaaggataaaaataatcatcgaaatgtacggcgtcgatatcgtagcgttttaccacgtcgcggataaccatcgttacatattcgcgcacttccggaatgcccggatcaaaatattttttattgtcgtaaacaacgaaccattgtggtttcaggcgggtaatatgattggctgccacgctgctgcggcttgtattaaatacagccctgtatgggttaaaccaggcatgaaattccatgccgcgtttatgcgtttcttccaccatgaactgtaacggatcatagtacgggtttggcgcctgcccctgcacgcccgtgaggtattcagaccagggctcatatggagatggataaaaggcgtcggtagccgggcgcacctgcaccactaccgcattcataccatttcgctgttgctggtcgagtatggcaatgaattcctgcttttgctgctctgtactcaggccccgccgcgatggccagtcaatattttccacagtggcaatccacaccgctcttagctcgcgtttggggggcaattgcgcccatgcctgctgcattccgataatcaatagtattgcgcctgctataaattgcttcaacatctgcctgactttttaaccgtaagatgcgaaaatagcaaaaagcagggctgatccgatacaaatatgtgattcttatgaagatagggaactaatctttctccatcttcagcttcgtagcaggcgcctggtaatcttccggcaaatattctgttgggaccgtggtcatatttccatcgcggtgtgcaatgaaatgcggcgacataatttcaatacccgcagcattaaactcatctatgatatgccggtgcagatcagaatagatgactgccattttatgggaatgatcggtatatacattgatttcgtaagcgatggcaaaatcatccaggctggtttgtaaaacaaagggcgttttgtctttcataacgccgtctgtttctatagcagccttgatcagcatttcatgtacttttttccagggcacttcatagccgatagtaacggtagtatgtaagatgaggccaaggtctttgctggatgtggtgaagttaatggtatggccacttaatatgctggcgttgggcactgtaatttcttcgttcttaatcgtgcgcagcctggttaccagcaggttcttttcaattacatctcccgtaatttccccgatttttacccggtctccgatcttaaaagggcgcatgtacgtaattacaaaacccgctatcacattggaaatggcggaagaagaacccaatgaaaacaagatgccgaggaaaacagaaacgccctggaatatttttgaatctgatccgggcaaataaggaaatatgacaacgaacataaaggcgtacagcaggaacttgatcccgcttccggtgggtcttgcccaatcggcataaaaacctttgagcgagaggttgccggtggccacttcttccgagagatagttcaccagttttaccaggtaccgcgtgataagataaattacgatgatggtgagtaatttgggaagataatgcaggaagcccaccaggatggatttgatgggggataatgtccagttgatcagtttatcggcgatgccttttgtccatggaaagatgctgaatacaaagggcagcgtaatataaaagacaaaaagaatagccacgatccttactatacgcaacgcgttaaaaacaataccgatctgcttttgctggttcagcaaagcgtaatcttttacttttacgcctttgaaatagcggtctttttcacggacaatccttttgcgcaggcgtttgaacaagcggttgatgccgtatacgatagcggaaaatataacgatgatcagtaacagccaggcgatcctgacaaggacattctgcaggctgctgtctttcttttcctgtaatatcgcgttgcgtacagcggcggcatacttttgcgcaacaggttctttttcctggtccagccaaagagcgtcgtcatttgttacgcttagcagcaccagttcattataggtaacgtctatattgttttcgttgggtataactttaattgaatcaggtataaaaaagggatcgtcggccagctgcgacagtttatgttcaatgtttgctgcacggtcgcttgggttcagtggtcccagtttgttataaatatagaagagggtatcacggcggaagggtactacgggaatgcctttgctggtagctttcagctggataatccgctggcgggcagctacttttttcagggagtcggcctgttcaaaagcggagagtttctgttgcagttcttttttgcggttgtcgttgtcgttactgatcagcagcagttgttgctgcagctgttttttctgttcgtcgtccgctttctggagagaatcgttttcccggagcaggcgggtggtaaggatcagttgtgagtttgtgagggagtcgcgggtggctttgctgctatcattttgtgcgttgcacagcaaagccaaaccagtcagaatggtaataaagtagagggtaaaagcagttttcattcccggagcttttctttaatgtacggaaaatccgggtagtaaaacgcctatatcttcctttttgtatactggctgtagtccggcaaacttgcttcgtattcctggtgcatgagcggggatgtgaggaggaagtcggccgatgcgcggttgctcgccatcgggatattccacaccacacctaagcgcagcagggctttgatatccgggtcatgaggcagggcttccattgggtcccagaagaaaatgattacatcgagttccccggtggccacgagtgcgccaatttgctgatcgccgcccagcgggccactcaggagttttcttacagatacatccagcgcctgttctatcagcagaccggtagtgccggttgcatacagttcatggcggctcagtaccgttttattataagtggcccattcaattaactccgcctttttgtggtcgtgagcgatgagggcaattcttttgcgggcttttaaaacttttgatgtttgcatatgtgaccacaaaagtaataagtgacgcgcaataattaaatctaatgttagtgtttatcgttgctgtccagaacagccaggtcgcggtcaaaaatgtaaagaccgcccttgtcttccccgatcagttttaatttatcaagaatatgccgggccaggcgttcttcttcaatttgttcggtcacataccattgcaggaaattgtgagtggcatagtccttttcgctgaggcacaaatccactaggttgttgatctctttggaaaccagcaactcatgactaaacacttgttcaaaaatggcatgtatgcttttgaatttcacggtaggttgctttaatgcaggaaccaggccatgaccacctctttcgttaataaatttcaggagcttcagcatgtggcccctttcttcatcggaatggcggtacaggaactgggccacgccattgtacccctgcacctctgaccaggaggccattgccaggtaatattgggaggaggctgcttccatttccacctgctggttcagtgcgtcataaatttttggagagagttctttcaataacataatgaaaaatttgtataatatgaagaagatcgaggtgtgacggggatatcaccgggaactataccgggattgtaaatttcgatagactacatttagatgcatcccggaaatctgcctgaaaaatgctacctttgcataagtaaattaggataaaatgattaaaacaggaaatccaatcatcagcatatatacggagatgacgccaaacccggaaaccatgaagtttgtggcaaacaagcttctgtaccctggcaaaagcattgatttcccggatgaagccagtgccaaaccgtctcctttagccatagagctgtttagcttccctttcatcaggggcgtatttattatggctaactttattacgcttacaaaaaccagcgaaactgactggaacgatataattcctactgttaaggccttcctgaaagaatacctggaagactcccgtcctgttatcaacgaagatgaggtgattattaccaaatctaccgcgagcaatgaagtgagtgcagacgatacagatgtggtaaaacggattaaggaattacttgaaaactatgtgaaacctgcggttgaaatggatggcggcgccattcagttcaaggactatgaaaatggtacggttacactgatgttgcaaggttcctgctcaggctgcccctcctccatgattacgctgaaagccggcattgaaggcatgatgaagcgtatgatccctgaagtgaaggaagttgtggcagaagcagaataagccatagttgagtgaatgatagtgttaaacgaaagcacagtctttatggctgtgcttttttttggcgtttaaccgggaaataaatgccagctactcctatacaacacaagcaaacagctacaatgagaaaattactactgatcgttaccggcatcgccctcgccctgcaaccggtacaggcgcaaaaaaagaagaacgtggacagcgcatcggctgttattacctatggtttcagcagcaatgggaaagccatccccggcaacgaacagcaattgatgattgatcatcaccgtgcacacattgttagcggtagcaggaaacaaaaagaagagcagttcctggaattgcaggagcaggctaccctgcaggtgttaagtcttcccaacggggaagtatatacgttaaaaaaagccttttctgaatataccaccccggagttactgccggataccgctactatcctcggatatgtatgtaaaaaggcaaagctgcttatccgttccaataccatagaagtatggtataccaatgatctcccgctgaaaggcactcccaatcttactattgcgcccggcctgggcctggtgcttaaaacggtacgtaacggcaacagcgaaacggttgcaaagaaaattacctggcgtaaaataacggctgaagaactggcctggccatccaataccggtaccctagtaaacgatgccgcgtatacacggcaggtaatagacagccgctataccaccctccccgtgtttaaccaggaacagatcagctggggcaataattcgcctaaccctcccggtgagcaactgaaccaaacctatcatttcgcgggcggcaccgtgatccttaaaaaagtaagcctgccggcagtgaagaagggccagacattatttgcggaactcacgcaatactccaacggggatgcgtacgacagaaccggttccgtatttatgatccccgcagataaagccatctctttcctggatggtttgcaaaagggcgttgggacgttaccgttatttacggctaaaaacggcaagcaataccagggcatggtggccactgataattatttgccggcactggaagtattgcgcttttttacgccattcggcgtacggcagtttaacaaccaggtaaagattgccggttacaactgggcggactctgtgatttacaaacaagacatcactgagctgcacagccgccttcagggcgatgtgtggctgggcgtatatattggcaattacgataaaggcgggcataaagtaagtcttagtcttaaatactacccaggcgatccggaagatgaaaaccggccgtcagccaactggatatacccggttttcaataccaccaacctgatggaaatggccgggcaggagtatgctaccctgtttgataaagactccctgaaagtaaccgtgaccattccggaaggggttaaaaatattcagttaaggttcctgactaccggccatggtggctggggcggaggcgatgagtttaatcctaaacagaatgaaatttttgtagatgggaaacgggtgtatcattttattccgtggcgcacagattgtgcgacctatcgtttatctaacccggcatccggcaactttggcaacgggctttcctcctctgatctaagccgttccaactggtgcccgggcacgcttacttcaccggtattcatttcgctgccagatatcactcccggacagcataccatacaggtggctattccgcagggaaagccggaagggaccagccagagcttctggaacgtatccggtacactgatcggagataaaaaataatttttccgggatgcagtatctgctgcatcccggatgccataatccggaattatttatccactttcgcactatgaacgatttataccagggcatattagaaggtcttcaccagatgacctggctggaagcagtagctgttttttttgctgtcttgtcggtcatctttcaaaaaaataataacatactggtataccctaccggcatcgtgagcacgggtatttatacctatctcctgtcgagagagcatttcaagctatatgctgatgccgcgctgaacgcgtattacctggtgatgagcgtatacggctggatctattgggcaaggaaaggcccggaggagccggcaacgccggtaatgcgcagtaccagtaaagaattgaccaccgccgttttcattgcactggccggctggggaattttctatttcctgctaagccgcttttccgattccaatgtgccggtgatggatgcctttgtatccgctactgcctgcgcgggtatgtggttgctggccaggcggaaactggaaaactggatattcctcaatatttccaacctggtagccatcccgctgttaatatataagcatttgtatcttactgccgggttaaccgtctttttatttaccattgccatattcgggtatcttagctggagaaaagaagtgttgcaaagagaaatgtctcataaatgaagaaagtagttgttataggacctgaatctaccgggaagagcaccctcagcgaaaagctggcggcacattttaataccgtatggacgccggaatatgcgcgtgagtatcttgatcaactccaacggccgtacgaagaatccgatctgctggaaattgccgccggccagatagcgctggagcagcatatggcccggcaggccaatggggtgttgatctgtgacacagacctgtatgtaattaaggtatggagcgaacataaatacggccgctgtgatccgcggattttacagcaaattgcccgccagcagtgcgatttgtatctgctcacctatgttgatttgccgtgggaagaagatccgcagcgggaatatcccgacccggaaatgcgccattatttttatgacatttaccgggaaatcgtcagtaattccggtgttgaatggaaagatatcaggggtacttatgaagagcgggaagccctggcaatagctgccgtgcagcagttactgaaccggccctgattattttctgccggtaaccaactccataatatcagggtccggcgagaggttacgcatttgcaccagtatcttacgctgccggtaagccgtgatccgcgcaggcggattaatggtatatttaagcgggttaggtaaacaggcggcaatcatagcggcttcctccctgttaaggctcgcggcgcttttttgatagttggcctgggcggccgcttccaccccaaacacgccctctcccatttctgccacattcaggtacacttcaaggatacgctgcttaccccaaattttttcaatcatgaaagtgaagtatacttccagccctttgcggaaccagctgcgtccctgccagaggaaaacattttttgctacctgctgactgatcgtgctggcgcctttgatttttttgctttgctggttgtgcttcatcgccttttcgatggatttgaagtcgaaaccattatgatctgtaaaaagctggtcctcgctggctatcacggccagtttggcgtgttgtgatatttcatcgtaattcacccaggatttctgaagttttttatctgttccccaaaggctgaaccagctggagatttctgtaatggtaataggcgggttcacccatttcagcaagaggatgtataaaaattgtgcaacaattaaaaccagtactactctcttcagtctcctccacgttctgggaacaatgccttttaaattcattgcgtaggtttagaaaaatcgggacgaaaggtaggctaaaaacctgaaagtgaaacacaatcgttaactttatatatgctattaaacgtacacccggataacccgaatccccgtcatttaaaaacgattattgaatgtttaaaagacgggggaattattatttatccaactgatacggtttatggtttaggctgtgatattacccaacacaaggccatagaacgtattgcgaggattaaacagatagatccgaaaaaagcaaacttttcatttatctgttacgacctgagtcatttgtcggactacgcgaaaagtgtggatacgcccattttccgtatgctgaaaaaggcattgcctggtccgtacacctttattttgcctgccagccgcatggtgcccaaattattaaaaacgaagaaagacaccgtgggtatcagggtaccggacaataatatttgccgcactattgtaaaagaacttggcaatcccattatgagtactacgttgccgatagaagattacgtagaagaatatacggacccggagatcatttatgagaaattcggtaaccaggtagatattgtaatagacggaggacccggcggtatgggtttttctactgttgtggattgtaccggtgcagaaccggtgttggtccgtgaaggcattggcagttttgaagaaatatcctgatatatgcagcgatggtggataagtgtggtttgtttattccccggcatgatagccggggcgcaaacgcttacgttgaaacccgcagccccggtgttgtcggtggcagtgaagccactgccgtttacgttgtgtgatactaccggattcctgttaaaaccggcaacactgctttccgcttccacccggaaattccccactcctgttcctgtaactgccccggtttaccgccttgcagccgatgaatattaccagcagcactttggttttttttgtaagaaagagtgggtttggcaaaaacaaacaggcgtgccgctcaagttccgtttaggaagctattcttacgcccagcaacaggaaggaaaacgttaatttcttttactgtatttgttttggaagataataattgacgaagtcaataattattagttgaccatggcaaatattttttaaaaagataaatatgattagccaggataaaaagggccactaaacggccgattctgataaatattttggggagataaaagcgaatatatccgcttatatctcccccaatcttttaaaatcaaaactgatcaaatcaagacaatcagtataatcaatctaatcctgctccaagacaatttaaaatcgccggaggcgatcctatttaatccccagtttctttgcaacatctgctggtaacgcttttttgtttaccatgtagcaggtggttttataggcaaagtaaggctcagaagcgtagaaatatccctgacccggattatcggtaccccaggagtttttcacgcggaagtatttgtttccgttctgatcttttaccaggcctacaatatgcataccgtgatcatcctgtgtttcgaagttatcgaaagcctgttggcgtacttcaggggtgattgttttttctttgcctggttccaggaaagcattttttctttcttcggcggtcatatccgtccagtctttttcaggaacgatagccagtccgtctttaaaattgaatcctttttcgcttacatcagcagcccatgcaatggaatagccgttcatgatagcattttcagcgatggcggtaaagtcattcaggtttacgttatatactttttcccagttccagttatccggtacttccagtacaaactgtgaattgtacgggtggtgtgtgaaggaagaaatcagtacgtaatcatcggcgttcaggcccagttcttttgcgaaggtctgcggcgtataggttttaccgttatactggaatttttccggagcgtcgcccatataggcattcaacacgccatcgaaagcttttgaccagtcggggttgatagtgccctgtgcattgcctattttattcaccataccttccaggaggctttccatttcagcgtggttgtacattttacctttattgccatcgtaggctgtttgtggcaccagtccatattcacgtaggcagagcagatcatccgggaaaccgccgccttcaccgaagttggcttttccatgcatgcgtacatagttagcggctttcagcggatacattttgcgtaccacgtacatttcactgaggttcagtcctttatttttaccggtgcgaagtatttctgattcaaagaaagacaggccggaaaaagaccagcaggtgccggtacggccctggttttgcacatcacctgcgtcgaggttctttaaaacggtaaactgatagtggcttccctctgtgttggtactgctttgtgcatatgcgcctacgctgcaaagcatggctgcacacattatccatttcttcatgagtatatcaatgattggtttaaaacaaaggaccaaaaataagggaaagcgggtatttgacagacgaaaagatggatgaacggggcttgctacagctacttttaaagattgttcacgtgaattacagttatttctcctggtaatgattgcgggtgatttcccattcccagagatcttctccttctttatttttaaatgtacctacaaatcgcatccccgctttttgtaatattttaacggaggcgttatattcttcttcagtgtgggcaatgacccggtgaacataagaatgtccgaaggcaaagcggataaggccttcagccatttcagtgcccaatcctttttcccggtaggcggctgttatttcataccccatttccacaagcccatcttcattgggcttgcctttgaagccgccggcgccaatcagccgtttatcggcgcggtgaatcaccaggtaaaagaaccagccaagcatggcggggtcgttgcgtaatttatcatacgccaccagaaccatttcgggatactccgtccaaccttccggaacagaaatgccaagcaggtcggccaggtgatcgttgccctgtaatagcaattcgaaatgctccagtgagcacggcaacaattgtagtcgaggtgtttggatcatgtttgaaaactagtaaactgttttgggaaatacaatagcggcttttagcatttaattcattagcttttagcatttaacaatcccgccggggaaatattcccgcgaatcagatgttacctgctaaaagctaattgccacagccgaatttagtgcgcctccagccagttattgccggtgcccatttccgcttcaaccggaaccgacagcggtaaggcgttacgcataagatctaatataaggggtttaataatctccagttcagaacggtgcgcatcaaaaaccaattcatcatgtacctgcaacagcatgcgggacttgaggtttcgttctttgaatgctttatgtatagcgatcatcgccagtttaatcatatctgcagcagtaccctggataggcatgttaatggcgttcctttcggcaaagccacgtaccaccgcgttagaggagttgatgtcctttaaccagcgtttgcgtcccagcagggtttgaacataaccattttctgacgcaaattttatctggtcatccatatattttttgatagatggatactgtgcaaaatagttatcaatcagcattttggcctcactgcgcggaatgcccaggttttctgacaggccaaaggcgcttacgccatagatgatgccgaagtttacgcttttagaattgcggcgcatatcggacgtaacttcttccaggggaacgttatacacttttgctgccgtagccgcgtggatgtctattccctgctgaaacgcggccatcatttctttgtcttcgctgatggcggcaataatgcgtagctcaatctgcgaataatcggcagagagcaacacaaattcctcgttgcgcggaatgaaggctttccttatttcgcgacccctgtctgtacgaattgggatgttctggaggttggggttattggagcttaaacggccggttactgccactgcctggttataggaggtgtgtatccggttggtgcgcctattcagcaataacggcaacgaatctacgtaagtggatttcagtttgctaagctccctgaaaataaggatgtcctctactattttatgtttgctggaaagcttttgcagtacatcttcaccggtggcatactggccggtacgtgttttctttgctttcgggtccagttgtaatttttcaaacaacacttctcccaattgcttgggcgacgccagtttgaaacgaacgcctgcctgttcgtacacactttcttctgcccgtttgatttctatttccagctcctttgaatagtctgccagcgcggtggtatcgagggcaatgccttcgtactccatgtcggcaagaactttcacgagtgggttttcaatatcgtagaatactttgtccacagccttttcgggcaacagcggcgcaaatctttctttcagctgcaatgttatgtcggcatcttccgcagcatattctttgatcttttctatttccacatcccgcatgctgccctgtccttttccttttttgccaatcaaggattctatggaaaccggctcatactgaaggtattgcgcgctcagcacatccatgctcctgcggccttccggctcaatcaggtagtgggccagcatggtgtcaaacagggtggtggtaatttccatgccgtaccatttcaggatcagcatatcatacttgatattctgcccgatgagtacaatggaggggtgctggaacagcggtgtaaattcatgaatgatggcacgggcagcagtgttgtctgccggcatgggaatgtaatacgccgaaccttttttaaaggaaaagctcatacctacaatttccgcatcattggcgtcggtgccggttgtttcggtatcaaaagacacttctgactgttgcagtaattgctgcagcagggccgttcttttttccagggtatcaattacctcgtattcatgcggggtgttgtgaatatttttatctgccagcaggatgttgccggtttccactgtttctgtggtgacggttacttcttctgtaacaacagtgccgaagagatctgtttgtaccacccgcgctttagcttccacactggcgctgccggcaaaaccatctcccagtattcttttaccaagtgttttaaattccagctccatgaaaatgtcggtgagctttcctttatcgcaatctttgatacagaaatcttcttcatggaaggtaaccggaacatttgtgatgatagtcgccagttctttggacagcagggcattttcacgaccggctttgattttctctcccattttaccgccaatggtatcggcgttatccagcacattttcaagggtgtgatattgtgccagtaatttcatcgctgttttttcaccgatgcctgcaatgccggggatattatccactgcatcacccataaggccgaggatatcaatcacctggtgtacatctttgatctgccatttttcacacacttccttgggccccatgatttcttccttgttgcccatgtatggtggcttgtagataaagatattatcacggaccagttgcccgtaatctttatccggggttaccatataaacggtgtagcctgcatctgcggcctgccatgcgagtgtacctattacgtcgtccgcttcatagccatccagctctactacaggaatattgaagccttcaatgatccgcttgatatccggtaatgcatccagcaggtcttccggggcatcttcccggttggctttatagtcagtataagtggtgtgacgctcggtaggcgcgtgcgtgtcaaacgcaacggctatgtgagtaggcttttctttattaatgaggtccagtaaagtagtggtaaaaccaaactgcgcattggtatttcgacccgcactggtgatgcggggattcctgatcagggcgtaataagccctgtaaatcagtgccatggcgtccagtaaaaataatttcttttccattgctaaacctacaagatttaatttgaatctgcaaaattaagatagtactaccatatacggtgaggatgtaactttacaaataaaaaaaatcaaaaaagaatgaataaaatttatcatttgtcgacctgcggaacctgtaagaaaatcctggaagaaacgaaggcaaaggagcgcggatttattttgcaggacatcaagaaagataagatcacgccggcgcagctggatgaaatgaaggcgctttccggcagttatgaatctttattcagccgcagatcgcagcagtacaggccgatgggactgcatgaaaagaatttaacggaagatgattaccgcagcctgatattacaggagtattcttttctgaaacgcccggtggctattaccggcggaaagatctataccggtgcggaggtgaaaaatatttagcaggagaacattttacggatactgaagaaaaaagggacggctgaattcagccatcccttttttaataatctcagagggattgtacgaactgttgtacgacctgtttgtactggttcatatcctgttcatgatgaaaagaccggaaggggaagcgggctgcttcgtccagtgccgttttcaggtgaaaacgttcctgcggaagcgaatagaagtaccctttctccatcaggtattcacccaggtatacctgctctgattgtccgggtgtagggataagaattgcttttttattcaatttggccagatccatgagggtggtatacccggagcggcttaataccatatctgatgccagcatggcatcgtttaattcgctggcgttgaggtgattaatttgtgtaacaccgggggccacctgttcatgttgcgggatgccgggttttccacttacgatcagtgcggtgatggacaaggatttgatctggtccaggatcagtttttccaggttggtgcgttgtggctccggcccggagatcagcaccagcagatcgtacttcttttccacgcccggtttttgctcaaaccggctaagacaaccgatataagtggtatgcgcaggtaattggccgggatgcgccagttcgccggagagattgttactgccgggataatcgggaatccagcaggcgctgtatttgttaatgaaacgataatttattttttgcagggtccgctctatccaatcgccaaaaggtgttttaatcagcagttggtgggtaatgaaaacagtggggatatttttgtgatataaaccgaaacggttgtctgaaataactgcattgatttgatactcagcgactatcttcttcagccatcgttgttcatagtttaccgcacggaaaattttaggtatttgctgaatgattttcagtccaaaaaactgtcctttttgtgcatattggatacggtagccggggagcggaagtatggtcagttgcgggaattcctgctgtagcagggcagcgtgtttgccttcagccgcaataaaaacctggcaacctgcgtttagcatttcacggatgagcggaatatcccgggtggcgtgtccaaggccccaatccaggggaacgattaaaatttttcgggacgaaataattgtggacaaatattttaaaattttttacgaatttagcttaaattacaaaagggcattgttaagaaaaggtaaacacttcaggaaggtattcaaaaatagccagtatataattagcagtatgaaaagtataaaatggatcgtagtcttttttctttgcggatgcctggtgatggaagggtgtaaagtttttaagaaaaacgattgcggttgtcctaccatgaataaaaaaagaatgcactaatacgacgatctgtttgatagcaacgacgactttgacaacgactgacaactaaacaatttttgccttatctttttgaactatcctttgatacctggccaaacaatatttcggggaacagtcaaattttttattcatgaaacctgtagatagagatttattaatcctgctacatgaagataggtacacggaacagcagattcaatctgcggtgagacaaatcagcgaaatgctttcgttgattgagacgatggattatctctgtgcagttatggaagttatggattgtaacaaaagccggattaccagcaaacgaaccgtgctggaaaaagcaatttcacgtaagtcgcataagcctttcgaatttattattcacaagaactagtagccttacctctacaaattcccgttatagtagctttgacccgctgcccttatctgcctggttttgcttttttttaaattcttgttgtacgtttgccatcaaataaacgcaatttactgatggcagatttttcgcatctgcaggatttcctacatcctgtttcaaaggcatttttaaacgatgaccaggaatacgatccattccaggtgggcggtgtaattgacgcatacgaagatgaccatcatccggatatagacgcagcagatattattctgctgggtgtaggagaagaaagaggcagtgcatccggcaaaacggatacacacggtcctgatgccatccgccgcgaatttttccgcttgtacaactggcaccgcgatattaaactcgcagatgttggcaatttgttgccaggtgcatttcttgccgacgcatatgcagccatgaaaactgttgttgcagaattattagccgccaataaaaccgtgatcatcctgggcggttcacacgatcttacctacccgcaatataaggcctatgcggcgcagcaattaattattgaagccactgttgctgatgcgctgatagacctgaaagaagactccagtatccgcagcgaacgctttttaatggacatactcacggagcaacccaactacctgcgtcactacaatcatatcggtttccagagttattttgtacatccgcggatgttagaaacactggataaacttcgcttcgactgctaccgtcttggccgcatccgtgaaaacatggaagaagcggaaccggtactgcgccattcagacctgttcagtcttgatatcaatatcatccggcacaccgatgcaccggctaaccagctttcaccaaatggattcagcggtgaagaagcctgttccctggccagatacgccggcatgagcagccgcctctcctcttttggtatttacggctaccgccccgaaaaagataaagaacacctcaccgcccggcaaatttcccagatgatgtggtactttatggacggacgcgccgtgaaaaataaagaagccctgctggacgaccgcgatgctttctgggaatttcatatagccttttccgatatagaaacagtttttctgaagagcaagaaaacaggccgctggtggatgcagctccccgaccgggaatttgtgccgtgtgcgtataacgactacctgatggccagcaacaatgaaatgccggaacgctggttgcgtcaccaggaaagactctgaccgttgttttctccgtacaggaatgttccctgtacggagaaaacactaaatattgagaagggtagttaatctctctttgatgaaagctgctttatgatcggtagaaatcatttcatcatccaatccttccatcgtgcgtttatgcatcttttctacccgctcatctatcttcctaaaatattcttctttctttgtttcccacgccagctgttctacctggagcttttgctgccgcccggtattcaggctggaatagagatgccggagggtggtattcagtaaactatccagttgtttatagtaggtaacagcacagttgtacatgttgtggctgttgccaaggcattgctggtagcggttttcaagtgtgtccagcgctgtttgttgtgattgggaatacgctttcgtgcacaggaataccgcgagaaggatgatcaggtttcgcatagggactgtgtgatcatcaaatatacaaattatatttaataatatactagtatcagtaatccttctcaaccagagggcttattaattgcccagtttatcaccgatagagccggtacagatatctccctgtggcagcccgttcagccagactctcagggattcggtacgctgattcgtcagttcggtgaggtaaccggcgcggcacatgggaaatgcgctgccatagcttttggctgcagcggggtacattgcctgtacctgcgcatcgcggaattgtatccagagccgctgcgcgtctttcaggtttttaatgaatgctttgttggcggcatagtctttcaggatcagctggtaaatatcattcagcttcttgtcggcctccttatattcctggccggcttgtttattcatttctgactgtgactgtgaaaaggcggccatgctgcctgtaatcaataaaagaaaaagaataagagatttcatgttataaaggtttgaagaatttaaaagcatataccattggcagtttttcttccattccccggatatagaaacggccatctttttcaattgtgttactgaaacagttatagggagaataatcaaattcctggaatacctgcaactgcaatccctgcgcggttaatgccgtaactatttcactcagcggatggttccaggaataggaagtatgccggatgccgctgccgccatcggtataagttccggttgtttcttccacaatggtttgggtgttaaaatagctgtagatgatctctttaatgttgtcgtcaaacatccatataacaggatgaaaatccgccatcacgaatgatccgccgggcttcagaaaatgatttactacagcggcccatttgtcgaggtctggcagccagccaatagtaccgtaagaggtgaatacgatgtcgaaagcgccttccaggtgatggggcgtgctataaaggtcgcagcaaatgaagcgggcttttttctccaatccggatttaatggcgagttcgtttgccaaagtaatggctgcatcggaaaggtccactcctgttaccgtggcgcccatcctggcaagagataaggtatcttgtccgaagtggcattgcagatgaaggatctccttttcctgtaccgtttcaagtaaccgcaattctatctctttcagtgaattttttccaccgaggaagccgggcaggtcataaaaatcagacttaacgtgaacgcccgtacgtttattccagagctctttgtttgttgaaagataatcaggcaatgggtccatgaccatagtatttaaagggtaccttaaaagttctttgattcccggtggaagggataatacaggttatccaaaaataaaaggtttccgttaatggaaaccttttattttttagcgggatatttctttttaaatcactaccagctcataaaaatcgcctggcgtgaaatattgttttgccagctgctgcaattcttccgcggtaatggttttaatagttttgatgttattatagaagtaattctcgtccaggtcgttcaggatgaggtttttccagcgttggatcagctggaaagcgccatccaggtcgccgaggatggatccgatcatatagttgcgaacgaggtccaattcctctttgggcaccggttcgttctgcaggcggagcagttccttgtaaatttcatcgatggtagcttcgcaaacatcgcggccggcctctgtttgaatattcagggcactggtttgacggaagttatacaactgtgaataaatgccgtaggtataccctttttcttcccggatgttgctcatcaggcgggaaccaaagtagccgccaaagatggtgtttaacaccagcatcttcgggaaatcgggatggtaacggttcgggaaatgacgggccacacgcacggcgccctgtaccccattttcgtcattaaagatcctgaattttttctcttctgccggctgtattggcagatcgagtttaaccaggtgagtatccccgttccattgggtggtgccaaaatattggttcagcaacgggatcatgttggcgggcaggttaccagccacaaagatcttgcagttgttgtaagtataatgctttttatagaacgcctgcagtccttcagattgcaatgcatcatatgccatcatggagcttacgcggccatatggatggaattccccgaacaggtatttatcaatgaaacggttgcctacaaaatcgcatttcagcaggtttactgccagcttttgtttctggttctgcttatacaggttcagttcttcttccgggaatattgggtccaggatcacttcctgcagcatgggcagcagtacttccgtgtgcttggtgaggcagtgaagcgtataggttgcattttcatggtatgcattacggttcaggtaagcgccgtgatagtcgatgttttcattgatttgttgcgacgtatgtttgctggtaccatttttcatgagaaagttggtagctgtagcttccaggctttcgctttcgtaccagctgcctgcaggaaataccagctccagctgtaatgtttcctgttcgtcagatttcattacgtataccgggatgccattgtccagggtgaactgttcatatggcttcagttttatatcgaaatccaccgcatctttaatgggaggggcaatcgttctgttcatcgtgtcttatttaaagggtgagggccgaaaacaagccactgcactaatttgcagcgtaatagtaaatggtatttgaattcttctcatcaaaaagcagtttcgcttcctcatgtatttctgctgcggttaccacttcataattttcaaattcgtggttcatcagtgcggcatcgcccagcagttcgtaaaatgccaggttattggcacggttgagtaagctcatgtcttcaaaggccagcaagctttccacgcggttttttactttttgcagttctctttctgagatgacttcctgttgcagtttttccaattcctgctgaatagctttttctgcatctttcatttttactccttttaccagtttaccttctatggttagtaagccggcatcgaggctgccaaaatgatagcattcaatattgctgaatagctttttttcttttaccagtacctggttcaggcgggaggagctgccaccaccaaggatgtcggagatgagatccgctgcatagtaacgtttgtcggtgcgggcgtacatgtggtagcatttatacagtgcatccagtggtacattggcttttacttccagtttatgtgctgctgtttgcgcaggttcaaccggcaggttgcgataatacttttcgccggaagggatatcaccgaaccatttttccgcgagcgctttcacctgctccacggtaacgttgccgcctacagagaggattgcgtttaccgggcggtagtacttaaagaaaaatgcttttacatcttccagtttagcattctcaatatgtgataattctttaccgatggtcatccagcgatagggatgagtagtgtacgacagctcgcgcattttatgccatacatctccataaggtttattgatataatgttctttaaactcttccgatacaactttgcgttgcacatccaggcttttttcatcaaaggccagggagagcatgcggtcactttccagccagaaaccggtttcaatattttctgccggaagctgaatgtagtagttggtcagatcgctggtggtgtacgcgttattttcgccaccggccatttgtaacggctcatcgtacgagggaatattgatggacccaccaaacatcaggtgttcaaacaggtgggcgaagcccgtttgtgccggattttcatctctcgctcccacatcatacagcacatttattaccgccatcggcgtcgtatggtcttcgtgaacaattaccctcagtccgtttgccagcgtaaacttattataatggatcatatctttttattggtcaatacggtaaaaatagggaattacggtaagctttcagctcaaagcggcaaaaagctactccaggtacagttccttcttgtcgtaattaatggtaagcgtgtagtctttccagatatcataaccaatagagccggctacttctgtaaatacgccgaggtcgtctatatccttgctgtagctcaccggcacattggggatactgcggccgcccatttccagtgagggcaccgaactattgatatagtacaataccttcaacatatcctgtacgcggtctgtattgatggtggggagcagggtattgagtttgtatttatctacatagggccagttaaaaaggatgccgtagtcgccgccggtggtgatgtgatagtggccgggtaaccggcgaccatcgggcagctggatggaggcgtcaataaccggggtgctgaaattaagctgaaaatgcagcagcctgccggtattgccggtgggggttttgccggccttgtacagtacgagttgtttggcccggtagtctattttaacgatgtatagctttagcaaagcgattcctatgatgccgtccaccggccccagggtactgaggttttccaggtatactttcacataaggtaaccggagttctttgagataaagggcatttagtgtagccagttctgttttggccatcgcattgttggtgccggttaaaaaggcattgccggcatttcttagctgtagtttagcggcagtagcgagattcattaccgttacttctgctccgctgtcgaaaataaaatgcagggtatccgtactaccggaaacggtaacaggaatgatcaactggcggtttaccagttcaaagggaatgacggctaccggtttgctgttatctgttgctgctactgacgagcctctgcgctgggcatgggcaggcattagggcatagctgaatacgatggttactgtcaataaaaagcgccacatgacacaaataacgtcaaagaatactttttattggcaattttttaatgaggagttctttatcccggctcaccaggcaggtagcgcgtgtgccgatgtttttcagtaattcgcggaacagctgaagatttgggcccaggttattattgatgcccatgataatatcgcctgtccggaagccggctttttccgcaggtgatcccttgataatatcggttacttctacctttccgtcgatcaggtagatgatcaaaccggtgtaagaatagtcgaacatatcacggaaatgcgtgttgggcagcatgtatatttcctttttgctgtagttgagggtgatattgaaacggcgaagcaaatcgttccctatcattccgccaagaaaaggataagcggtaacgttgcttttatcgtcaaacacataagtgggcacattccggaaactatagttgccgatacggaattcatttaccgtggtgagcgacatggtcatcttccctcccaggccctgtgcttctgtttgtatgatctttttggtgcggcgttttttgccttgtaatacgctgctgtcgtttacaaactgggatgacagcaacaggcacataccggcgccggtgtcgaaataatagcggttggtgatagtgcgcacagcgttcttcagcggagcagatatcaacgggatctgcgtgagagaaggacgtagcagttgacctccccggggataagtatattttcctttggaataaataataatttcttctgtatcgtagtctattgtaacaatataccggctcagtaagctatacccgatgatgccatctacctgtataccgtacacctggctgatcagttcataatcgttgatgtggaaatcaaggctgtctacctttaatcccgggagtttcagtgagtgacgccgtgcaaaggataccggtttggaactgcccagcccttttatgatccggtcggaaggttccatgcttattcccagcctgaggcaggtggtggtatcaagtgaaatgcctgcgctgccggtgtcgagaatgaactgaagcgtgtccggataattgctgaccagtgcctggatgactactactcccccgtaatattgtttgaagtggaagcgcgtgagcagcatggcttcgcgagtactatcgttttcaggcgtggcatttccggcttgggtgctcatcgatataccggcggctgccagaagcagcataacgtgtaacagaattggtctaagcatacttggttgatgcaggggatgtgtatacctataaatttaacattaaatagtgttcgtataaaatatttttattacaggcggttaattgcctaaatactacctttgtcaaagttattcagggttagaaatatagcacatggaacttcaggatttatacaaaaaggcgcagaactttgagtttctgacagcagcagagggcgtttacctgtttgaaaatgctccgctggcagaattgatggaaatagccaacgagttacgcaagcaacaggttccgcatggaaaggtaacctggcagatcgacaggaacgtaaataccaccaatgtatgcacggccaactgcaagttttgtaacttttaccgcattcccggccataaagaggcctatattacgccaattgaagagtacaaaaggaagatcgaggaaacccttaagtatggcggcgatcagctgctgttacaaggcgggcaccacccggaactgggtctcagcttctacgtaaatctcttcagggaactaaaacaattatatcctgcattaaaattacataccctcgggccccccgaagttgcacatatcaccaaactggaaaaaagcacccatatagaggtgctccgtgccctgcaggaagcgggtatggacagtcttcccggcgccggtgctgaaatactgaacgaccgcgtacgccgccttatctccaaaggaaagtgcggtgcacaggagtggttggatgtaatgcgtgcggcacacaagctgaacattgcctcttcggcaaccatgatgtttggtcacgtggaaaccgtgctggaacgttttgagcacctggtggatatccggcaggtacaaagcgaaaagccggaaggacactatggctttaccgcgtttattccctggactttccaggatgtggataccctgctggcaaggatccgtggcgtacacaacatgactacctcggaagaatatatccgcatgatcgccatgagccgcatcatgctgccgaatattaaaaatatccaggcatcctggttaaccgtaggtaaacaggtggcgcaactttgcctgcacgccggcgccaacgattttggctctatcatgatcgaggaaaacgtggtaagcgctgccggcgccccgcatcgctttacctacctgtctatgcaggaggcgatccgcgaagctggttttgaaccgcagttacgcacgcaactgtacaaattcagagagctgcctgctgctatcgaagagcaggtgatcaactactaatgcagcggaggttgtcttactcaggattacgctgattagcttttggagatttggggagaatttagcggaggttgtcttactcaggattacgctgattttatgattagatttttgggattggggagattggtggggataacagggttggatgaagattgcttaaagatggacggtaaaatgctttgtgtatactttgtatatgcttagtacatgcttaatacatgcagttaacacggaggtgatgcggaggtgacgtggacttgatgccaggatcgcttaccacagggctttacaggcgaaattttttcgggcgttatatggaatactaccctattaagagaaacggtgcgctgatataccggtgaaagtgagtgaacgacattcagtaaatctttgctgtaaataccgctcagcttttttaaattatttaaggaatattgatggagaaggccgtttaaatttactgaattttccgaaaatcctgtaaaaagctaaaaatataccaatattccatagaaaatgccggataccaaattaaaatccggccagtgccttcatcttccaaaatccttctaaaatcaaaatagtatcagcaaaatcagcgtaatcagtgtccaagacaacctcctctcccatctccgcaaatcccaaaatctaatcataaaatcagtgtaatcctgagtaagacaacctacgctaaattctccccaaatttccaaaagctaatcagcgtaatcctgagtaagacaacctacgctaaattctccccaaatctccaaaagctaatcagcgtaatcctgagtaagacaacctccgctgtgcataaactattcattagcaaattattaacaagtctcaaagatttgttaaaactgccggggtgatgttacaaattgctctgttccacgtctaacagatacaaactaacaatcaaactaaaggagggaatatgaaaaagctgggtcttatcatggcaggatttgcaatcatcgccatggcagcctgttcaagcaccaaagtaacgtcttcctggcgttccaatgatgcacagcaactgcaaaaggataataaaataatggtaatggcgctggtacctcagagagatcgtaccctgcgcagccagatggaaaattacaccgtatcggaactgagaagaaagggatataatgccatgtctgcactgcagacctatggccccaacgacatggctaaaatgacggaaaagcaggtgttgaagcaattacagggaagtgatgtaaaccagatcatgaccattgtaatgctggataaaggcagggaaagaaactttgttcccagttactcaccttacggttattatggcttctggccctattactctatgtggtcatccaggatgtatgctcccggatattatacttacaataccaagtatcaatgggaagccaacctgtatgatatgaagagcggacaaatgttgtactctgtacaatcacagtctttcgatccgccaacaacggaaagaatggccgtattatatgcacaacaggtagtaaaagatatggctaaacaacagttgttagcaaaacagtaacggtaataaatagagaataaacagccgctggctcttagtttttatacaataaagctaaaggtcagcggctatttactgcccgcaggttggattttacgggaaatcggtgtaagtttaacgcccttttaaatccagttatgttcgaaataaccgttaatgaaaacatatacctccggcagctccaggtgcaggatgctcccttggtatataaacaactggatgcatcccgtaaaagcctgcgcagatttttaccctgggtagattataataccaacgaagaacattccctccgctttatacagttgatgttacgcaaagctgaagaacaggaagccattgcgctgggcgtatggtacaaggagcaattttgcggggtcattgatctccacggatgggaccaccagttgcagaaagcagaaataggttattggataggagaagagttccagcggaaaggcattgctaccgccgcgtgcaaaggacttatttcctttgccttcagaaaactccacctgaataagatagagatccgctttgtattgcagaacgaacgtagcgggcaaatcccgatcagactgggatttgccaaagaaggaatattgcgccacagcgccaaactgcacgggcagtatgtggatatggtggtaatgggtgtactgcggcaggactggaaatattagcttttcagctgcttacgcactttactgtgcttcttaccataaaattcatagatcaccatgcctattgccatccatacgatgagacgtaaccaggtatcccagggcagaaaggccatcataacggcacaggtgataatacccattaatggcacaaagggaacccacggtgttttaaatgcgcgcggtgcatccggcatggaataccgcattatccaaacccccgcacatacgatcacaaatgccagcagggtaccaatgctggtcatctcccctactacccttaccggtaccagtgcggcaaacaaacttacaaacacacagaaaaggatattcgatttccagggagtacggtaacggggatggacatccgaaaatatctttggcagcaggccatctttagccatactgtaaaatactctcgattgcccccagagatccaccaggattacggaggtataaccgactatgatggcgaggataatcatttgcccaagccatttgtagggcgtgtgcgcaatggcaatggctaccggcgctgcgctgtttttaaactctttatagggcgccagtccggtgagtacatgggaaaaaagaatgaacaggaccgtgcataccgccagtgatccgagaatgccaataggcatattacgccgtggatttttggtttcctgggcggctgtgctcacaatatcaaaaccgaggtatacaaagaagatgacacctgctccccgcaaaataccggatatgccatattctccaaaggtgcctgtgtttttgggaatatatggggtgagattagccggctgtatatacttccagcccagggcgataaaaacaagcactacgcccactttgagcgacaccactatcgcgttccatatggccgagcctttggtgccacgcatgaggatcgccgacatgaggataatgaccaatgctgcagggagattgaaatagccatgggtggttacgccgtttgccagcgtgatggtttcaaacggggagtgtgaaaactgtgcgggaatgtaaattttatatcctgcaaggaatgctaccaggtaattggaccagctgatagccacggtggcggctcccacggaaaattcgaggaccaggtcccagcctatgatccaggcaagccgctctcccattgtcgtgtaggcgtaggtgtatgcgctgccagccaccgggatcatggaggcaaattcggcatagcaaagaccggcaaaagcgcagccaacaccagccactataaaggagagtgttactgccggcccggcgttattgccggctgcgggtcccgtaagggaaaataatcccgcaccgataataacgcccaggcccagcatcagcagctgaaagccattcagcgtgcgtttgagggtatctttgctttcactggccgactcgttgagcagccatgataaaggctttttgtaattttggttcatgttatataccctactggtttagtagactggtccgcgaaagtaggatatatttatgaatttaagccagatcgcagattcctactgcctggcggagcgatgcgatctggtctttatgggcaggaataaactcctgggccacgtggcctttaaagccggtttcgtagatcgctttcatgatggccggatagtacagctcctgggtttcgtcaatttcatgacggcccggtaccccgccggtgtggtaatgcgcaatataatcgtggtggtcgcggatattacggattacatccccttccatgatctgcatatggtaaatgtcgtatagcagcttaaaattgggagaacccactgatttacatagctctacgccccaggcggtatgatcgcactggtagtcgtggtgatccactttgctgttcagcagttccattaccagcgttacctttttcttttctgcatagccggtaatgcgttgcaggcctttggtgcagttttcaaggccctgctgatcgctcatgccgttacggttgccggaaaagcagatcaggttggtgaaaccggcttttgcggtttcatctatataatgtttaaaatattcttccagtttatcgtggtgggctacggtgttaaatcctttgccgatattccaatccgggccattactggccaccatagcggtgatcatgtcatttttcttcaggatgtcgaagtctttcggatcaacgaggtcgatggaatgaatgccgatttgtttagcagctttacacagttcatccagtggaatgttataacaccaggcacataccgagtggttgattttgccttttagtttttcatctactgccagatcgtgtgcagataccctgctggagagggatgatagcgcggtggatgcgaatgccattgtggctactttcttaatcatatcgcggcgtgagttttcctgatgcataaaaaaggtttgctttaaaactgccatcaatgtaggcgaaattatgtttacttacaagctcctgccgcctttttaaggcaaaagggcgtggaaatacggattttattttttccgtagaaccaaccgcgctcatcctgcgtttatatagtaacttacagttagtttggaatttggtaagtaatttgtttatgtattgaaaagcggaggttgatatggaaaaaaaatatactcccagtttatggatctgcatcctgatggacgtgttaggatgcgccagttacgcagttccggtattaggagacgtcagtgactttatctgggccccgatttctgccatcattttctaccgtatgtttggtggcacgattggtactttcggtagtgtttttaacttcatggaggaattatttccaggtacagattttatccccacgtttactctttcctggatactgaagcgggtaacggctccaagaagaacgatgtctatttaaattagtctctaaataacaagggcattattaatcatacggattaataatgcccatttttatatagatggtcaacttagaagcctcttggtctcatgccgccgcggccacctcccggaggaaagcccatcatacggttgcctctttcgcctttgccgctattaccgccaaacttattcaggaaataggtgaagctcaccataaagtattgctgtaatacattgctctgtacgtcctggatgtagttgtctgccacggtgcgggatacactgatatattgtctcaacaggtcaaatccctggatcttgatcatcccctgtttctttggaaatacatactttgatacgttggcgttccacatggtggaggtgaggttataacccggctgccggccacggttcattgtacaggtgatatcgctgccgatcaggaagccgagcgggagattgatattgaaatccgtgttgatattgtaatccaggtagcgggtatcacttgcaccggcgctggcctgggagtagttggtggcattgaaattaatgctgccgcccagtgaaatatcaaacaattccttgtacatatagcttacgttggccgactgtgataactgcaacgaattggtgttgctgttaatgccattgctcacaattacatctttattataactcacggaagttcctgtgttcaggttttgccctggcgttttggataagggaatggagttgtgtaccatacccgaaatattgtaattaccatttacgtttaccggtctcacggtttgcctgccggtttcaggatccagtgtagtggagttgataattttatttaccgtataaccgccgttcaaccgggcaaacattccccggaaggtgatgttgttaaacgagttgtagttaacgctgaggttattggtaaaagatggtttcaggtccgggttacccagctgtatatacaacgggttactgttgtccggaacgggcgccagctgttgtacagatggttgctgtgtattaccgttgtagtttatgcgtagccgtttgttcttggaaaatgtatagttaaaagatgcctgtggggagaagttaaccgtgttttgtgtgatcaggctgtctttccccttcaggaatgaatacgtgttattatcaaggctgttaaacagcacattcagtcctatggaataatcatatttcagtttgttggtgcgtatggcaaagccggtctgctggttcagggtactgttggtaaaagaattgctcagtgagtcgttcatgatgttgtactgtcctttcgcatcatcatagtcgtaagtatattttgtgctggtgctattgtattttgtgataccataatttgcttcgaggaagcgatcccttcccaacggttctgtgtaggtaacattcacgccttcgttgcggctattggtatttatttgattgcgctggttgaagttaacgatgctgtcggcagaaacataattgatacttgattttacatagttctcctggtcattatcgctgttgttgtaattaaagttaaggctcagtgtgcggcctgcttttctaaaccgtttgcggaacagcagtgagccgccataattttcattgttgccctggccatcattgtaagtgagtcccctgttcaatgtatccttattggtgttcagcgacaggttttctgtaacgctgtagttgttgccgtttgtaagggaataggttggtgaaaagatcagtgaatgaaaggagtcgatcgtatattccaccctggcagaaaagcggttgttactgttatctgtttgagaggtggaattggtattgtcgtagttggtggtggcgttgccttgtttatcggtactgaatgtttgttttgctgttttttgttctgtattattcttggtatcattaaaaaagtagctgccgttcacgatcaggtttttgctgaagtcctggttgaaattcaggccggtgttccagttgcgggtgataccgctgttgttgccgccacccatgagctgttgcatgcctcttccgccgccgcggccaccacctcctcttccgccaccggcagaactgaagctcatggcatcctgttgggtatagcccatattgtttacgttgttaccgccaccgagcaacgacatctgctggttttccctgaagcggtttaagctgagggatacgccatagcggtcgtcggtaccatagccggcagtagcgcggccaaacagtcctttctttttatcttttttaatggtgatgttgatcgttttttctgtttgcccgtcgtcgatttgtgtgaattgagcctggtctgatttgcggtctatcagctgtactttgtcgataatattggctggcaggtttttggtggccagtttggggtcgttgccaaaaaacggtttaccatctaccagtaccctggtaacggtttctccctgtgcggtgatagcgccgtctttatctactgtaacgcccggaagtttctttaaaaggtcttctaccactgcattttcgcgggttttaaatgcatcggcattaaattcaagggtatctttcttaactacaatgggtggtttttcgtccagtatttctactgcattcaggtttactccttttaataccatagggatgttgccgagggatatttccttatggtcctggttaatctgcaatgatttattgataggtttatagcccaggaagcttacgtacagccggtatgcgccatcggcgacgttggtcagttcaaagttgcctttgttgtctgtcatagtggtggtagcaacgctggagtcttttgcattcagtaacactaccgtggcagcgggcatggcatccctggaggtagagtcagtcagttggcctttaatctttccttgttgtgcctgggcctgtacatgtataatgcccaaacccagtaccagcaagagttgtataagtttcttcatatatgaatttaacaggaaaggggaagttaggatgaaatttatttattgttgttgccgcttacgtaatttctccatttcctgtcttctgatttctctcatttggtcggggctcactttttctgcacccgcgggtatgctgagatccgtatctgttacggctttcaggctaacattttttgcgatgaaggcgcgtttgccgccttccgcagaaagcacaacggcattgctgtcgggtaataatccgttcaccggggagaaagcgaagggcaattcgttggtgtaccaaacggtgtacgtatcgtcttttagctgtatggtggcctttttacaggtatagcccgcaattttttttgttttgtcggacgacttgttattagcggtaaagatgaagtcttcttctgtgtaataagttttcttatcatcaccaaaggtgctgaacacctgttcatacttcttattggccaggtctacatactgggcgttgccaccccgtcccatgcccatgcccataccacctgggccttgtctgcgccgggtgctggtatctccgtcggggcgctgtcttctgccgccgaagccgccgccttcaggccgctcggtggtgagcttaccgaggttgttgctgaaagtaaatacctgtttgaaggtgatgacatccggaatttcgggtgcgtcgtcgccaccgcgctggaatccgcgcatgcgttcgggatctgttttggcggttacttcatattctatcactcctgattgctgagcatatacctggctggtggcagatagcagcgtggctgctgcgatgaataaacggatagttcggttcatacctgattgattttagtacaaatgtgaatcttcgtcttcattttttgggttaaaaagctttatttactgttatttactgttaagggctgtctgtaagcgttaatcttccttatttactgttaattactgttaagggattgccttcttttccccgtggaatggatagttttgtaaggatcttaaaatctttcatgcgacaaagaatcagaaatattctcatcctcatgtctgtttgtatcctcggaatatttctgttccaggggtactggctgtataattcatacaaattaagagaggaacagttcaataaagagatcaatgaatcgctgcggatggctgtgtttaataagcagttttctgatgtgcgccgctatatccgttactatggtaaagataaagattcgttgaagtcgcctatgcgcggactggcagatcagctggaagaaataggcatgcctaaaggcaggcgtttcaaggggcagcatttcgaccgctaccccgagcgacctccggcagctgcttttaagggcgattcttccagcaggatatatgtggatacactggcccggcagatctccgagttcctcattaccagcaacttacacgacgatagtaccaatcttaaaaaactggactctgttttcaaagtggagctggccaatcgccagatagccacgccctatgaactggatacttttcatctgaactacagcggttttgaaagggaaacgtttagagacagcatccgccggagggaacccaggcaaacggcgaaaattccttttaaccccgccagcaacttgttcgtacaggccagcttcgattcccccctgcagtttattttacaaaagatgatctggaccctgctcagctcactggtattactggtgcttaccaccctcagttttatttatatgctcagaacaattctcaagcagaaaaagctgtcggaagtaaaaaacgattttatcaacaacatgacgcatgagctgaaaacgcctattgctaccgtatctgcggcagtagaggcgttacagaacttcaatgcactgaacgaccagcgtaaaacacaaacgtacctggatatatcaaaaaatgaattgcagcgcttatcagatctcgtggaaaaagtactgcatattgctgccgaagaaaaagaagatattgaattgttccgggaggaaacagacctgaatgaagtaattgacaacatcctttccaaccaccagcttaaagcaggaaagcagctacagttacgctatgataataacctggccggcaaagccgtatttgttgataaaacacacctggccagtgcgattaataatctcgtggataacgcgattaaatattccggcgaacacgtacaattatacctgcaaaccagcatggaaaacggtatcttaaagatccgggtaaaagatagcggcattggtatcccgaaggtataccagggcagtatctttgataaatttttcagggtgcctaccggcaacctgcacaacgtaaaggggtttggcctgggattaagttatgtgcggaaaatagtggaaatgcatggcggctccatacatgtgcaaagtgaaccggacaaaggcagcgaatttaccattatcatcccttctgcttaaccatataaaagagatttatgcccaaagtattattgatagaagatgaagtgcagctcggacaaatcgtgaaagacagccttgaaatgcgggggtttgaaatgctgtacgcagccgatggcaaagaagggctgcgtatataccagcaggaacaccccgatgtggtggtgctggacatcatgatgcctaacatggatggatttacggttacggcagaaatccgtaagcaggataaattcacgcccatcattttcctgaccgccaaatcgcagactgctgatgtggtgaaaggttttgaactggggggaaacgactacctgaaaaagcctttcagcatggacgagctgattgttcgtattacggcgctgctgaaacgttttggcgataaccccggcaccagggaaatggaagaaggcgctgtaaccatcgggcaatatgttttcaactacaccaagcaaacccttgcccgcaataattccatcgagttcctgtcacaccgcgaggcggctattttacggcggttatacgataacaaaaatgaggtaatggagcggaaagctgtattgctcgatctttggggagatgataattttttcaacgcccgcagtatggacgtatttatcacgaagctccgccggtatttgaaagatgattcccgtgtacagatcgttaatatccggggagtgggttacaaattgattttttagtggttcatggccggatcggattcaaaagtaatgtacacacgggtgccttctacggtgttctccgctcccggcagatcggagatttcaatgttaaattgtttatggtacatggcgcggtaaagggtggccctttccatacatatttccatgcccctggaatggtggttgttactttttagcccgtcgtgatgatattgcagtgcctgtacccttccgataccgttgtctgttacctcgcacgcatacaggtccggacccagctgcatccactgaacgtgtagctgcctgtttgtacgcttgtgcatcaggccatgccagatagcattttccacaaaaggttgtaccagcatacagggtacatacagggccgccgcagagatctgcggatcggtatagagcgtatactcaaacccgttattggtgcgcaattgttccagtttgaggtactgctccagcagatcggcttcttcctgcaggggaataaaatctttatcagccagcattaacactttccggagcaggccggcaaaacgggaaatatattcctgtgccagcgccgtttcgccggtcatgagggcggtgtatatgccgtttaggcaattaaactggaaatgcgggttcacctgtgatttcaggttcaccagttttagttctgtaatttgtgtgcggagaaggagcattgcggcatcctgctggtggctgttttggatcaaagcttcgctactgcctttgagaagaaggtaacgggaacggtaatgcagacaaaggagaaaaaaaatgacaatgccggctgcagccagtatcagcataacagtgtgtgtggtgacaggcataaccccctcgatttgctcatgaaaatatacgtcatttccgtgaaaaaaggagcaatggctaaacctcttcagtttacacctaaacgcttatctttgttgtttatggaacagttagtacagcaaatagcagcctacaaagaagaaatagcggcttttacgcctgccggcgcagcggatctggaacagtaccgcataaaattcctgggtacaaaaggtatcgtgaaagctcttttcggggagatgaaacaggtaccgaatgaccgtaagaaagaattcgggcagattttaaacgaatttaaacaactcgcggaatcccgctacgagcagttcagcgatctgaaagatgctggtggcgccgatgccggcgatatagattatactttaccggccgcgcctcaccggctgggcaccaggcaccctatcagcctggtaaggaataagatcatccgcatttttgagcggctgggctttaccattgccgaaggaccagaaattgaagacgactggcacaacttcacggcattgaaccttccggaaaatcatccggcccgcgacatgcaggatactttctttatcagcaaaaatcccgactggctgctgcgcacccaaacttcctccgcccaggtaagggtaatggaagaaggcaagctgcctatccgtatcatcagcccgggaagagtataccgtaatgaaaccatttccgcccgtgcacactgcttcttccaccaggtagaaggattgtacatagacgaaaacgtttctttcgcagacctcaaacaaacgctgtatcactttgttcaggaaatgtttggcgagaatacgggcatccgtttccgcccctcctatttcccgttcacagagcccagcgcggaaatggacattgtatgcttcatttgcggaggcaccggttgtaatgtatgtaaacaaaccggctgggtagaaatactcggttgcggaatggtacatccgaaagtactggccaactgcggcattgacccggaaaaatattccggctttgccttcggtatgggaatagaacgtattaccatgctgaaataccagattaaagatctgcgcctgttctctgaaaacgatacccgtttcctggaacaatttgaaggagcagtataaatattattaccaggctatttggctattacataaatgcagcggaacttcccgctgcatttatgtaatagccggatgaaaaacctcaaaaaagtgattcaaactattgccgtatgcggcgcaggtactatgggcgccggaatagcacagatagcagcctacagcggatttactactttgttgtttgatatccggcaggacggcctggacagggcaaaagcacagattgagaaaagcctgacggttgccgtggaaaaaggaaagctggctcctgcggataaagacagcatcctgcaacggatccgtttcaccgcagctatcgaagactgtgtagccgatgtgatcatagaggctattgtagaaagaatcaccgccaaaacagcactcttcaaccagctggccgccatcaatactgcagaaaccatttttgcttccaatacctcttccctgtctgtttctgaaatagcctcggctgtaagcgttcatccatcaagagtggtgggtatgcacttttttaaccccgcccacctgatgaaactggtggaagtggtaagcggaaaggaaacagcaccagcagtagcagacactatttatgaactggcggaaaagatgggtaaagtgccggtaagggtaaaagatgctcccggttttattgtgaacagggtggccaggcattattacctggaagccatgcatattgcggaacagggtcaggcagatttcagcaccattgaccagctgctggaagcagccgggtttaaaatgggtccttttgcattaatggacctgataggtaacgatatcaacctggcggtaacgcaatccctgtatgatgcttttgagcaggcgccccgctttaaacctaatgcgctgcaggaacaaagggtgaaggatggtaagctgggacgtaaaacaggattgggtttttacaggtacgaacaataacaggttttagttatttttgaacctctttttggaaaaaagaattttagtcttcatgattttagtcaccggcggtacaggttttttgggtagtcatttaatccgggcattggttgccgcagggaaacctgtgagagcattgtaccgtaaacaaccttcaccccggttgcaggatatttcagataaaatagaatgggtaccaggcgacatcctggacgtgtgctcgctggaagacgctatgacggatgtaacacaggtatatcactgtgctgcagttgtttcttttcaggcagcggataaagaccgcctgctgaaaattaacgccgaaggcactgccaacgtagtgaatatggcattggatgccggcgttaaaaagctcctgtatgtaagctctgtagccgctatcggaagagcaaagccaggtgcggccgtaaacgaggaatgtgaatgggaagacagtaagaataattcccgttacagcatcagtaagttccagggagaaatggaagtatggagaggtattgcagaaggactggatgcggtaattgtaaacccttccattatcctgggtgcaggcttctgggaggagggttccggcaccctgatcaaaaatgcctggaaagaatttccctattacacacagggcgtaaatggatttgttgatgtggaggatgtggtaattgccatgatccggttaatggacagcgacatcaacgaagagcggtttatcctgtcggcagacaactggagttatctgcagttattcacccatatggcgcaggcgctcggtaaaaaaccgccgcatattgcggccaagccctggatggccgaagcagtgtggcgactcgaaaaggtgaagggaatgcttacgggcaaacacccgcttatcactaaagaaacggcccgtactgcccagctcaaagtatactacgaaaacaacaagatcttaaatgccttaccgggattccgtttccggccactggaagaaacaatccagcatatttctgccgcctacctccgggagcgcggagctggtttttcgcgggattaacgcggatgttgtctttctcaggattaaacggattttactgattactttgattttactttttggattttataaaggatttttaatgattcggggagataaaagcggatatattcgcttttatctccccgaatcattaaaaatccaacgtgatcaaatcccctaaatcagtaaaatccgtttaatcctgagaaagacaacatccgcgcgcgccacttaaaaaaggaatgcagcgatagccgctgccagtgttttggagagttcgggaggggcgtccctgctcatccatacccggggtttttcgcctggtattactgctgcgatgggttgcccgcggtattgaaactcgtagcacacactttcgtaggaatttaccttaccaaaacggttatgggcggtaatgcgtatatctgtatccgtagaccgtaacacgcctgccggtttgttttcattcagctccaggtaatgagggcttttaacgatcatttcccagcgttttaacggctcattcctggtgccgttgatcaatgtgtagcgaaggtccgttgctcccggcaaactacttaaataagccggcaagtcgcggttggagaacacaatggctgtagtgttcatggtttgtatcaacaggtgttcctcattgccgttcagataaaaattaaaggcgtttttagggtctttaacgaaggtggcttccgctacgccgtttttacgggaagtagtggaataaaggccaaaagaaatggttttagcgctaagccagccgtctttcacctttaccgcccattcctggtcgctggtgtatagggatgatttaacggcagtgggtttggtggtgctgcaactccaaagtagcagggggagtaaggcggcaaacaaatacttcatgaagcgggtggttttgaatatgctgaaacgccgggaacaggtgatattgtttcccggcgttgatgattacctggtttctttgagtttctcccacatctcggggatgcgtttgatccaggcaagttctttcttttttaccctggcatcttctaccggggaaccaaaatatgttttgcctccttccacggaagccggcaccccgctttgtgcgagaataacagcgcctttcccgatggtaagatctttattcacgcctacctgtccccagaggatcacattgtcttcaattttagctttaccggcaatgcctacctgcgcagcaatgaggcaatttctgccgataacggtaccgtgacctacatggatcatgttatccagtttggtgccacggccaatgatggtatcgccgcttacgcctttgtcgatggtacagccggcgccaagttccacatcgctttcaatgatcactcttccgcaactttccagcttatcatagatcacttcacgctccgcccttttcttaaagtaaaaagcatctgccccgagtaccgttcctgcatgaataattacgttgtcaccgatctcacagtagtcataaatcgttacgttgggatgaatgagacagttgcggccaatgcgcacatgattgccaatgaatacgttgggttgaataacagtgccttctcctatcacggcgctgtcgctgatggctttggttgctgcctcaaaaggcctgaatcttttaaccagttttacatacgcactgaatgggtcgtccagtaccaaaatcgccttgccttccggacaatctacctttttgtttatgataatgatggttgctgccgactgcagactggcgttatagtatttctcaaagtcaacaaaggaaatatctcccggtgtaaccttatgtatttcattgatgccagtggccatcaggtggctgttgccaaccagctctgcgcctatatatgctgctatttccgttactgcaacaggtgcttcgaacttcatatactctgaattattgaataatgtttaagagcaacaaaggtagtaaatcggcaattgcaaccatcaaaatatgaaggcatgataacgatgatcggaaagtttcgatctgctgttatccacaattattttcgtagtgtgaataaaattttttgtaaattttttcttttgtgatgaaattctttttaatattgtgtagggaattttgtttccctgtacttactaacccattcacataacaagaaagtctgattgttccaacggtcagactttttttattgcctctgaaacccgcatgaataaagcgttacagcagatcacatttttatcgcactaaaattcatcactacatcttcttctttctcatccccatttcccggtaaatggataacccggtagaggaccccgttttttcaatttttgggtttttctggcctaaaagcgaaaaaaaaacgcggattttgtctttctcaggattaaacggattttactgattactttgattttaccttttggatttataaaagattcggggagatataagcgaatatcctcgcttatatctccccgaatcttttcaatcctttataaaatccaaaagagtaaaatcaaagtaatcagtaaaatccgtttaatcctgagaaagacaaaatccgcaatgctttatatggcgcggctaaacaattgtgaatgtggtacttgtcgccacagccgggcatcaaaagccatacaaatgttgcggataaaaggcctcccctcaggcgttaccaccaccttctgaggcagtacctgcaccagcccgtcgcgctccatctcctgcaatcgctgcaggccatcaatgatcgcatcacactgcgtgtctgccttgttccaggtagtttcaaatcgacacatcagctcatgaatatgctttcgcagcaacccgtcttcttcgttcaggatatgaccgcgtacaaccggaaactcccctttgttcaccaggtcctggtaaagatccaccttcttctcattttgtgcataagcataccagctgtcgccaatggaagaagctcccaaaccaaccagcaacgatgtgggagaatcagtataacccatgaagttccggtgcagccgcccttgcaggaaagctttgtgcaaggcctcttccggcagcgcgaaatgatccataccaatctccgtataaccattgctgtcgaacagtaacttacccagttcatacaactgccgcttctcttcatcttttggcagatctgcttctgtataacgacgctgaccggttccctttatccagggcacatgtgcataactgtaaaaagagatcctgtcggggcgtaaccggacaaccttatcaatcgtatgctgcatgcttgtaagcgtttgcaacggtaaaccatagatcaggtcgaagttgatggaggtaaatccaatcttcctggcgttctctactacggatgccaccattccaaaaggttgcaaacggttaatgatttcctgtacccgcatatcaaagtcctgtatgcctaaactgatcctgcggaagccgaggttatacaacgattgaagatgctccggcgtggtattgcccggatgaccttcgaagcttaaactggcatcaggcagcagctccgcagtgcggtaaatgccattcagcaacatcgccagatgtgctgcactgaaaaaggtaggcgtgcctccgccaagatgtatttcccggatgcgcggacgcccgccgaaagtatccacatacagctgccactctttcagcagggtttcaatataaggcccctctaccccgtggttaacggtgatgtgtttattacaaccgcaatacgtacacatactctcacagaaaggcaggtgaatgtataagctgatcccatctttaccgttcgattcgaggaatgattttttcaacagcgttttccacttctccggatgaaaagtttgctcttcccaatagggaacagtagggtaactggtgtaccgcggtgcggctacgttatatttactgatgaggctcatgatgtaatggtttatgacaacaattttcaactacatgttcactattgggcgtcagcaccgggctgatgtaaggaatgcccaggtttagtccccggaggatcagcaacacgcccatgatgctgatcaccaccggtatcaaactgcgcatccggttacgcacctgcatattgaccaggtgactgaaccaggtaatacccaccattgcaggtaaagtacctgcaccaaaggcagccatgaacaacatccctttcagcacatcaccggaggcaacggcgccggcaataccgaggtacacgagtccgcatggaaggagtccgttcagaaagccaatggcatataaagtatggaagcgctgttgccttaacaggctgcccagccggaattttatttttgaagtgaaaatatccgggagatgcctgccttttgttaatcttatgccggcgtatttcaatattaccagcacaagcaataagctgccggtgatgatcgacaaccattgctgtaatccacccaggtataactgtttgcccagccatccaaaaagcagtccgaggatggcataagcactgatgcggcccgcgttgtataacagtatgccccctaatttgcggataccgttaagatgttgtaccggcagcgttaatgcaataggaccacacatacctatgcagtgaaagctgcccacaaaaccaagtataaatgaagcgatcatagtgcgtatatcttttgtaattttttaaataactatcctgctccgttatctcaattaatatttaccagttgttcctggtagtatggctggtcgttcatcgtccatgctatcttcactttgtacggccccctgatgaataattgccggctcactaactgccgtcccgattgatccggttgaagcggcatcaatacatccttgccggaatcagaaggccggtaaaaggttactttaccattgagcgctttgttccgcagctcagatggaagagaaatcattacacctgcgtcttcctgtgatatagtaacaggagcagataatcttccggcattttcttttccatcaattacctgctggtatttcaattcttcgccgtagtaatcaggcgttaccatatcaatcctggtatgcatgcttttggtaacaagcgtcagaatgccggcggcaaatactacaaacactataatgatcttatgtccccagttcatggtaataattttttaagatgtgaatgcgctgtcttgtttattgtaccggtcctaaaaacgtggtgcgtaaacgggtaatccttttgttgtgttcatacagcccgatgtataaagttgacttacgctgatgcacggaagctttgggcaatacaataaagaaagtaccctccccctgcccttcggcctttatatgaatcacggcattgcctatcatggacaccacgccgttttcgttttccagtttcaacccgagcggaatatcccggccggttttattgaggagtttaatacggtacaggttcgacaagctatcagtgcctctttcctggtacaacatacctgctgtgcgcataatagtgccgcttaccggtttccggctgcccagcataaagctgatagcagtaagcaataccaccaacaccccggagtatactttgagccgcggcgtaaaccgcagcttttgtttgctggcgatgccgttttcggaagcataccggatcagtcctttcggccggccggtttgttccatcatgaaatcgcatgcatcaatacaggcggtgcagttcacacactccagctgggtgccgttccgtatatctattcccgtagggcaaaccttcacgcactgcatacagtcgatgcaatcgccgtgtgccctggaatcgtctttacggaactttccacggggctctcccctttcgtaatcgtacgccaccaaaatggagttcctgtccagcaataccccctgcaaacggccatacggacatacaatcgtgcagatctgctccctcataaaggcaaatacgccatagaacacgcctgagaacacgatgatggcgataaagccgccggtgtgtgcagataacggctcggtgatgatcttacccagcgctttagccccgatgacataggcgaggaatatattggcaatgagaaatgacagggcatagaaggcaatgtgcttccctgttttccgcatgattttattggtattccatggcgactgctgcagcattttttgcgcagcggcatctccctctatccagtattccaggcggcggaataacagctccataaaaatggtttgtgggcacatccacccgcagaagagccttccaaaggccatcgtaaataccacaataaaaagaatgaatgccagcatagccagcccgaaaatgaagaagtcctgcggccagaagatggcgccaaaaaggataaactttccctccaccacattcagcataaataaaggcctgccatttatggaaataaacggcaggctgaagaaaacactaaaatacaggagactcacccaactgcggatattataccagcggccttttggctgctttgcgtatatccagttgcgtttgccttgcccgtcaacggtagctattgtatctctgaaggtgctgttagccataactgctgctttattctttctgcccctgtggttctttggcattcggcggattagtgccgcgtaacgttttgatatagcaggctacctgcgccagttgcttgggcgaaaaatcttcctgccaggatttcattcctttatcggccacgccgtattttattgttttaaagacttcattgagtttgccgccatgcagccagtagtcgtcggtgagattaggccctactacaccctgtccctgcgggccatgacaaggcgcgcagttggaaacgaacatcttttgcccggcagcgatatcagccggatcggtgagcatgactacattgttttcatcgatgttattggcggcttttttcaggtattcctgtttggcaacagccgctttttcttcttctgccgccagctcttccagctggctgggcgccgagtgagtaacttccgtacgccagaagtatacgatgccaaagcaaacggtgaatacaaatccccatttccaccagggaggtgtagggttattgagttcatggatgccatcaaaatcatggcccatgtcttcctctgcttctgccaccgcatccacggtccgtgttttattgattttttccagccatgatacccggggtttaccaggcgccactgctttcgcgggtgtacgttttcttttgatgcccaccaggtagcgcaacaggaataaaagactgatgatcaccgccagttccagtataataaccgatatcagcaggtagaaagaagtttgcgacagcctcgtaaaataaggactggcagcagtagtggccgtttgtgcaaaagcgttgctgctcaggagtgacagcataacaacaccaccagttattaaagctttaccggcatctttcttcatcttttccctgaaaatatccatagcgcccagcaccgcattagccaggatgccgatagccagtaatagtcctcctgctaccaccagtaataccagggctaccgggtcagataattctgaaggggtccccgctccgccatctgcaaaggcagggatactgcataataaaccgccagtgagtagctgtataaactgtttattcattgtttttcttttattgggcatttgtgtcgtcattatctaaaggaatacggctgatatgatccaccattttcttatcggctttaaaagcccatagcgaggccgccacaaaaaaagtggtaaacaacagcagcgatgccatcgggtaaatactgataccggctatagatcccaggtaattaatgaacttcatgacgttgcggtttagaattcagcgttattggctaccggtgcaggttttggggtcgacttaatatctttccccatcctttgcaggtaggctattaatgcaataatttcacggtctgctttaatgggcagcttatccttttgcagggatgcggcaatgccctgtgcctgtttctccaggtcggcaatagcctgttgttcgtagccggctgcataaggcacccccagtttccgcatcacgttgatcatggcaggcgttttacttttatccactctttcttcaaagagccagggataagccggcataatagaacccggcgacatggacgtaggatcgagcatgtgattaaagtgccaggagtccggatacttgccaccaatacgcgccagatcgggaccggtacgcttggacccccattggaacggatggtcgtatacaaattcgccggctttggagtattcgccatagcgggccacttcatcccggaaaggacggatcatctgtgagtggcagttgtagcaaccttctctcaggtaaatatcgcgaccgtgtaattccagcggtgtatatggttttacgctgctgatagtaggaatattgctgcggatcaggaaggtgggcatcatttccagcaggccgccaacggctaccactaccaaactgaataccaccagttgtatagggcggcgttctatccagttgtgccagtgcgctttaccatgtgtaacaatctctttgggtaatgcaggtgcttccgctgcttcgttggcaataaatgcacctttgcggattgttctggtaaggtttacaatcatcagtatcaggccgctgatatacaacatgccacccactgcgcgcagcgcatacatcggaacaatggtggtaactgtttccatgaactggtacttcagttgtccttcttcggtaaactgtttccacatcatactctgcgtaaaggccgcccagtaaagcgggattacataaaagataatgcccagtgtaccgatccagaaatgcgtattggcccatttgcgggagaaaagctgcgtaccaaaaatgcgcgggatcatccagtaaaggataccaaaagtaaggaacccattccagcccaatgcgccaacgtgaacgtgtgcaatggtccagtcggtgtaatgactgatggcattcacatttttcagtgacagcatcggtccttcaaaagtggccataccgtaacaggtaagcgctaccacaaaaaatttaaggatagcatcctccctcacccggtcccaggcgccgcgtagggtcagcaggccgttgagcataccaccccaggatggagcgatcagcataatgctgaaagccgttcccaacgattgggcccattcgggcaaagcggtgtacagcaggtgatgcgggccggcccagatataaataaatatcagcgaccagaagtggatgatggaccagcgatacgaatacaccggcctgttggcggccttaggtacaaaatagtacatcagccccaggtaaggcgtggtgagaaaaaacgccaccgcattatgtccgtaccaccactgtaccagcgcatcctgtacacccgcataccagctgtaactcttgaacagggataaagggaattcaaaagagttaataatatgtagcatggcaatagctacccaggtgccgatatagaaccagatagctacgtataaatgtgattcgcgcctgcgcaggatagtacccagcatgttggcgccaaacactacccagataagggtgatggcaatatcaaatggccattccagctctgcatattctttgccggtagtgtagcccaggaacagggtaagggcgccgccggcgatgatggcctgccagccccagaaatgtattttactcagcagatcactgaacatgcgggctttacaaagccgttgcagggaataatatactcccatgaaaataccattgcccacaaatgcaaagatgacggcattggtatgtacgggtcttaacctgccaaaagtaatgggggcaaatcccatgttaaggccggggatcaccagctccagcgctgcccataaaccggccagcatgcctatcagcccccagaacatacaagcgtaggcaaaccatttcaccgtgcggttgtcgtaataaaatttttcgagtgacatagtggtatttaaaggtgttgataaatgcgtttattcgttaacgttatcgggcttatcctcgaagaggatgcggtgcgccggtgaaaaatcatcttcaaactgcccgttttttactgaccagataaatgctgccaggaatcctatggctaccagtaaactaacaccgagtaaaatgatgataacgctcatggctatttatttaatgagaataaacctggctgtttccaacgcctgcagggcatgtatttcgttggcgccaaaggaaaaaacatcgccggattccaggatggttatttcttcgttgagcataaatgcgatcctcccttccagtataaggatcatggcatgggccggcgatgtatgcggcggaatctggtgcccctgctgcataatgagcagggtggcatcaaagcgttttgttttcaggataccacaactcttcactttttcatttcccgctatctgcattacgttcattcctttcatggatggtgtattgtgatgtaataccatacttcttttccggcatgcctcacccgttgcgtgtaaacagccttttcagcggctgtttacacgcccatttcatccgggcttatctgaggttgggcttagatttactgtgtatgtttcatgtgatagcaaaggtaacagcactgcacctttactactatgactttactcaatcaggaatatgacttttatcattcatttgctgtagtgcattgctgtaaagctttttgccctgccattcgctgcaaccgaaagtgatcaggataatgctgatagaactggctggcatcaggacagcggctaccagcggcgataaaattccctgcaccgcaaagtataaaccggtgatgttatagaggagtgacaatacaaaactaaagaggataatacgcttgttggctttgcataagcggatgaaagaaaacagcaaaggcagttgatccgcatgcagtataccatcgctggcaggcgtaaagttgttgctgtcttctgttaatgaaataccaatatcactttgtttcagcgcaccggcatcatttaatccatcaccaatcatcattaccttttcgtttttcttttgcagggagatgatataagcgagtttatctgccggttgttgctcaaaaagaagggtggcatcgttgcccatcaaccgacctaattgtgggagcgtatgattattatctcctgatagtacagataatgggtaagaagtttgcagctgctgcatcagttgccgtaaaccgttccggtagctgctgcggatagtaaataatccgtacagtttttcgttgatggatacgtacaccacgcttccttcctgctcacttttgtggtgtgcgcccgtgaagcctgcattgcccagccggataaaaaatccatctacccatccgcatacacctttgcctgtaaagtgctgaaagtcgtggatatgccgcgatgcgggatccccgcaatactgaacaatggcccggcttaaaggatgggtggactgcgctgcaagggtagctatcatcacttcctgtataggtgtaagcgcattgccgtaatagataaccgagctgcctgttttgccggtgagcgtaccggttttgtcgaatacaatatgtgtggcgttggccatgttttcaatggcttgtgcattacgcaggtaaaaccggtgccggctgaggattcttaaaatatgtccgttggtaaatgaagatgccagcagcagggcacaggggcaggcaatgatcaggatggcggtaacagcaggccatatacgcgcaggttcattcacccaccagtaagcggcagtagcagctgcaatcaacaacaccgcccacgtaaaatagcggctcagcaggtgaacaaaagacacctgtttttccgctttatttttcagttcatcacggttccataagctggtcaggtaactctgcgctacctctttaatggtaagtatttcgaggttaccattaagctgtctgccgccggcataaataatttccccgatcgatttgctgaccggcaccgattctccggttacaaagctgtaatctatcagggcttttcctcttacaataatgccatctgccggtaccagttcattgttgtgaatacggatggtatcgccggttttcagctcaggaagcgtggtaggaatttctttatcttcccttataacgcttacggctataggaaaataggcagtataatcccggtcaaacgaaagcccctggtaagttttatcctgtaatattcttcctatcagcataaaaaatacgatgcctgtcatggaatcaaaataccccggctgaccgttaattacttccacaaagctgcgtataaaagtaacgaagatggcaagcacaataggtacgtctatattaaggaatccatgctttaacccgttccaggccggcttataaaatgcctgtgcgctgtaaagtaataccggcaatgccagtatcaggttcatataccggaacaggcggttaaatatttcatcaagaccaccggcgctggcaaaataatcgggaaaactcagcaacatgatattgccgaagcaaaagcccgccacgcccagctggtataccagctgccggttaaccgcaggttttttgcgttgcagatcctgcaggctgatgtacggttcatacccgatggcggttaatatttctgccacccttcttaaagaggtgccggtatgtgagtagatgatcaatacctctttcttactaaaattaacggtgacccgctgtacccctttctccagccggtgcaggttttcaagcagccataaacaggaactgcaatggatttgcgggatataaaaggaaacatgcgtgtgggtatcatccctgaatagatagagttgttgcgctattttttcgtcatcgaggaaagcaaacttatcgcttcgcacggctacccgctgactgataccaggtttgctgttaagatggtagtattcacaaaggtcgtattggttcagtatttcgtataccgttttgcatcccatacagcagaatactttctcctgcagggtgatatcgttgtcagtacagttttccccgcagtgatagcaggtggtattggtttgaacatgcgaagaaacggccatcagtcaatagttgtgttattgcaaaagtaccggtcgcggcagaagggcgcaatgatatgcgtcaagcgggaatatgatatttgtcaggattggggctactcctgcaggtttgcagttctgataatttcggccaggtcaagcaggcggatctttttgccttccagttctatcatgccatcttttttgaattcagaaagcagcctgatagcggattctgtggctgtgcctacgaggttggcaatttcttcacgggagaggcgtacgctgagggtgtggccatctgcttccagtccgtaagtttccttgataaaaagcagggtttctgcgaggcgttcccgtaccggcttttgtgccaggtgggttattttcaattcggctttgcgcagttcgctcgataagatgcgcatcatttcaaatgacagggatgcatctttctgcagaatattgagaaacaggtctttaggtataaagcagatagaagaatcttcgagggctgtggcggtagcagtgtacctttcgttgctcagcagggctttgtagcccatgatatcgccgtctttgaccaggcgtataatctgttcccggccgtcatcaccactgtgcgagagctttattttaccgtcgtttacgcagtacacaccgaagggataggctccttcatggaagataacctgtcctttcctgtatacggagcatactttggcttctgcaatctgatcgagattgcattgttccgccttgcagaatattgatgagaagcgatccttgcaatgatgacatgaaggattgtggaacgatgtagccataatcaatttgcaaaagtactaatttacggctccttaaccaaagcaaaagcattcgtgtctctttattattatattatatataaaccatatgaagtgttaacccggtttacaccggaaggtaacaaggcctgcctggcggattattttaaggttccttcggatgtatatcccgtagggcgcctggattacgacagcgaagggctgctgatccttacaaatgataagacattgaaccagcaactgctattgccgcagcatgcccatgaacgggagtactgggtgcaggtggatggcgccgtaactgcggaggcggtggagcagttggcggcaggggtgcagatcaatgtagatggtaagatgtaccgcaccaaacggtgccgggcagaaatatttgaggaagaaccgttgttgccgccacggaacccgcccatccgtttccgtaaaagtattcccgcaccatggatcaggatggtgctgcaggaaggcaaaaacaggcaggtgcgacggatgactgccgcggtgggctttcctacgttgaggcttgtccgttaccgcatggaagatatcaccattgcaggcatgcaatcaggagagatggtggagatgagcaaagaagagatctacaggaagttaaagctaagggcaaagtagtgatggcggctctcagcgcactattagcatagtcgcgtctctgaggtggggctgcagctcccgtcctcctgcacccgctttttgctttaagctttatgctttcagcttttttaactaggtttgtcacctacaaatttctattatgctgaaatcaatgaccggcttcggaagggcagaaagcgcaagaggcgaaactagtatcgtagtggagatcaaatcgctgaatggaaagcagtttgaggtgaatctgaagttttctcctttgttaagaccctatgaatttgacatccgtaccctaatgcagcaaacgttgcagcgcggcacccttgatgcaacaatcaatatccgccagaatggcgccacccgcccggttgtgatcaatacagaccttgcaaaatattattaccagtctatcaccatgctggccaaccagctggaactcccccagggagatatgctcaacgtgctgatgaaattaccggaagtggtaagtccggcttcagagcaaatgaccgaagaagaatggaaagatgtggaagatacactgcgtgaagccctgatcgacctggatacacatcgccaggatgaaggcctcatgctggaagccgatctgaagttacgcatagaaaacatcgatagctatatgcagaaggtccgcgaactggacccgctccgtaaagaccgtatccgtcagcgcctcgaaggattgctggccgagcatgtaggaaaagaaaatgtggatggcaaccgcctggaacaggaactgatcttctatctggaaaaactggatatctctgaagaactctcccgcctggaaaaccacctccgttatttcacggaaatactgaaagacagtgactctgccaaaggcaagaaactggggtttgtgttacaggaaataggccgtgaaatcaacactaccggttccaaagccaatgatgccggtatacagcaatgggtggtgctgatgaaagatgaactggaaaaagccaaagaacaagtattaaacgttttatagtaaggcgaataccgtatgaacaaacttttcctggccacagcaggcttgttacttttggctgccgcctgcatgccgcctaaaatggacacttacgagaaaaacctggagatccccaggcatgagtgggcatatgattataaaccgtcttttgaagtaaaaatacaaccggaagatactgcgtacctttacaatatctgcgtgaacgtgaggcatacggatgcttatccgtacagtaatatctggttattggtaggtacacagtatcccggtgacagtaccataaaggaacaacgggtggaactgccgctcgcagatgtaacaggcaaatggtccggtaccggactggatgatatttatgaacaccgtatcttcattcagcaacgggctgtttttaataaaccagggacctataagtttacctttgaacaaaatatgcggcaaaatccgctcccccatgtaatgaatgttggcttgcggattgagaaagccggcacaaggccatgatgaaaagaatttccaataaaatgcaggaagggaaatccgtttccttcgtttattttttagtaatggcgtacacaattgccgcactggtttggtggggcattttgctgttcaggcaaagtgaacagatccgccgctttgaacaacaaaatctttctttgcgggtagacagcctcgcacaaccggtagaacatcagctgcaactggagcggatcaacaaagaagagcgtatgcgctcttttaaatacctgggcgaaggcctcatctttttagggatcattttactcggcgcactctttgtataccgggctgtatggaaatatatgaagctcagcaggcagcaacagaattttatgatggcggtaacacatgaactgaaatcacccatcgctgccgccaaactgaatctcgaaaccatccgtaaacataaactcgacgaagaaaaacaactgaagctgatcaataatacgatccgtgaaaccaaccgcctcgaccagctgtgcaacaacatcctgctggcggcgcaactggaaacacataaatacgaggtgtttaaagaaccgctggatttttcagccctgatagaaaacagtatcaaagacctcgatggccgcattggtacccatcagatcatcgcggatattttaccggacgtatggatggacggcgataagctgactttacaaattgtactaagcaacctggtggagaatgccgcgaaatatgccccgaaaaataccaccatctctgtaaaactatttgaaagtaaccagcaactgaaattacaggtgatcgacgaaggcccgggcatcccggaagaagagaaaagcaggatcttcctgaaattttaccgtgtgggtaacgaaaatacccgcaaggctaaaggctccggactgggcctgttcctgaccgctaaaatcgtggaacagcaccacggacgcattgaagtaaaagacaatgtacctgccggcagctgctttgaaatatcatggcctgaatattccgttcaaacggcgtaaattagatgacggattgatgaataccggaatccggattcgatgtaaaatcaaacaataacacatgaaggaagcgacaaaggcatcaatactgctggtggaggatgaagaaaatctccaggaagccctgaagctgaacctggagctggaaggttacgaggtcaccgcagtggacaacggcactgctgctctcaaagcagtaaaaaacgaatatttcgatctcattatactggacattatgctgcctgaaatggatggtatcgcggtatgcgaaaacatccgtattcaaaataatgaaatccccatccttttcctgagcgccaaaaacagcagcgccgatcgcgtgctgggcctcaaaaaaggcggcgatgactatatgactaagccctttaacctggaagagctcctgttaagggtggaaaagctcatcgtaaaaaataaaaagatccaggacaaagacagcgtacccaacgtataccgctttggcgataacgtaatcgactttgccgcgcaggaatgcgttggtaaagatggaaaacactacgaactgagtaagaaagaagccatgctgctgaaactgctcatcgaaaataagggcgaagtagttacccgcgaaaaaatcctccaggtggtttggggttataacgtatatcctactaccaggaccatcgacaactttatcctcaatttccgtaagtattttgaagaagatagccggaattcccgctatttccactccgtaagaggagtgggctataagtttacggaagcctaaataccagccgtttggcaaatgcagcagtagataagtataaccatctttgctgtatttgctaaaggctaaatacctgtagcaaacagccacttttcacctcattctccccagtttcctttaaaatccgacctcgtagtaaatcccactttatagtggagattaattagccgatatttattgagcttataagcgtagagaagtacttcctataaacctagttagtgacacattataccgatatcgtctttgctgcggagtggcccttctggctgttttttttgttaagtctcgttaccctaatagtattttttaccctgcgggaaagaagaatcaggagagcctcagcgaaagaaatcaccaagaaccatgcgttgattaacctggagctacatgctttccaggcgcagatggaccctcattttatttttaatagcctcaatgctattcaccactacatccttaccaccagtacggacatggcctccctttatctcacccgcttttcgcgcctcatgcgcctcatgatcggtaatttcaataaagaatggatttccctgcaggatgaactggatgccctggaactgtatatacagctggaacagttgcgctttgatgaacagttcgattaccagctcatcgtaatgccggaagtaaaccggcagtttaccctcatccctcccctgatcatccaaccctatgtgcaatatgccatctggcacaggatcctgctgcgccccgaaaaatcaggcggactgctccggatcaccatctccaaagaaaatgaccggctccagatccagctggaagataatgggatactgatcactgaaatgctcgacagcaccggcgaacggcaggcctccggcatcgatatcgcttcggaacggctgtacatgatgagcgaaaaatatcacatgcaggccagcatcaaatccctgcagatgtatgacgaagagcgtgaaccctccggtaaccgccttattatcagcatgcaacatgttgccgcccggcagtccctagccggatagcctgaattggaaatgtccggcaaattgcttaatttctacatggattaatagaatcaatgaccatatactttccacaacagtaaatctgaaaccacctttcattaatctgatctcaaatgcgtaccattatcgtggacgacgagaagcatagtcgggatgcgctgcacatgatgctggagaggtattgcccgcaagtttctgtacaagccgtttgcagcagtggtcctgaagccctgactgccattcatgaactacatcccgaactggtattcctggatatcgaaatgccgggaatggatggttttcaggtgctggaagccagtgaatatcactcctttgccgttattttcatcactgcctatgatcagtatgccctgcaggctattcatcacagcgcgttagattatcttctcaaacccatcgatagccaggaattaaaagacgcagtggaaaaagccagcacccaatccaccgttattaccgccggaaaagtagaagaccttctccgctttctgcaacagcacctcaaccaggacgaacggctggcattgcccacgtcagacggactgcgcatggtagttgcaaagaacattatttattgcaaaggtgcgggcatgcaaacccggttgcatttacaggagccggaaaagcccgtaatggtatgccgcacgctcgtggaaatggagcaatggctcgcagataaaggatttttccgcgtacacagcagcttccttatcaacctgtcttttatggagaaatatattaaaggagatggcggggagatcattatgtccgatggctacagcgttccgctggcacgggacaagaaacaggacttcctgcaaaggatcgaaagactataaccgcctgatatagttacaactgatccagccgtttttcccatcggccagttcaatcttacagaagtcgcgtgtggcatcggtgatacgcactttcatgccctctcccacttcaaaggcatccttgctgttttcatcaggcgacgttttggccctgatgttaccgttcattacaacacccgcttcatggttgttggaccacaggtaagtatctacagacatgatcaggtataaggcacacaatactcccaacacataagtgccccagcgcaaaaatttatttctccatccggggatatatacattgagcataatggtggcaataaacaaccagaaaaagaggatagtgcctgtagcccagccgttggctttatgaagatgttgcaattgtaaccaccactgctggaaaaataccatcggcagctcttccacaaaaccatttactttctgattggcaatagcgaggttatgtttcaccgcagcgtcattgggcgacaactgcaatgctttctcatagttataaacagcctgcccggttttacctgctttgtaccaggcattgccggcattaaagtaaagtgccttctgcgtatgaccttcatccagcaactgctggtaaagcctggcagcttctgtaaacttgctctggttaaagagtttgttcgcttcttcaaaccgttgttgctgattctgtggcggcgtttgtgcgcggcttccggtgaaagagagcaggcatataacagccaataataccggtttcatttttctgtagttcagcatttcgcctttcgttaagtagttagttcttcaacgcatcttccaggttggtgataatgctcaccgcctgttcatatgtaccctgcattttacggttatcctgtccgggtgcatataaagccacttcgcaattatcgatcaggttaaacaggtcgtgcgtattgctgccgttgatatgacgggcgctcagcttatcctgtatcagttgtttactcagatcggccattggtattttcagtttggaactgagataaccccaaacggcgcgggaagtttcttcataaaatgccttgtccttgccttctttcagataacgggcagccagttccaatcgtttcagggctaccttattggcgtagcggtgtttcagcactgcggcgttggtggtgttgtagtctttgcggcgtttgtagaaaataatacctgcagctatcagcagcggcaataacaacaggatatagaaccatgggctgagaataaaccagctgtgattttttgtccagtcgaggataccggtttcatttttcaccagttcatttttaccggcgccataatcctgtttatcctgcttaatatgtttgccctgttcgatatggatatcgaaaggttgggaacgcaatgttttatagctgttggcggcggggtcaaagtaagagaattctactgccggtatggtgtgatcgccggcttcctgcggcatcagcacatattcaaaagtacggctgccggaaagcgggttgctgttcttttcaatgtcgtctgttacttttggatcatatttttcaaagccggtaggcgtttccacctttggagagttcaggaggtttacgtttccttgtccgctaacggttactttcagcgtgagggcgtcatctgtggtaagcttcttcttatccactaccgctgtcatgttaaagttacccacagcgccgttgtagctgagcgggcgcccgtcgaccggaaccggtttaacattgatctttatcggattgctttggattttgtagggaacatcctggtattccacttccgggcggttaaagaaatcatcaaagaaaggatctctgaatgcgggatcgttgaagaaatcttcaaagggatccctgcccctgctgccaccttttttgctcaccatttttacaaggcgcacctggttgtccacttctacagggtccagttccagggtgcccgactgtagtgggaaaagcaatgttttgcggatggtaaacactttatacggaatgccgttaaccctttcctcggtagcctgtggcgggttaggcagctcaatatccttggcagaaaatcctttgaatgccgggactttagttacactggaattggttggaaggcgtgtaaaaagtttatacgtggccgttagttgttctccttcgtataaattggttttatctacttctactttcaggaaaatatttttcttcagcttttcattgatgtcttctcctttcttcaaaataccttcctggatatcttcgttaccaccgggggagccgcgatgcggcgggtagccggcagaaggaggtgcggcctgctgctgttgttgcgcattgccctttctgacttcaattaaaaccgggtttgattttacgatattcccgtttacacgggcctgggcgccggcgatggtaaaactgcccacatgctttggttgcagcaggtagcttagtgcaatgtattcagaccgttttccattgaaaatagattgaccctgcatttgagaggggccctgtaatacttcaaaatccttgaaactgggtggtgtaaagctggagacgtttacgccgttttccagcataaactggatctggaatggttcatcctgcgtcacggcattattgctcacagtggtagtaaagcggaaatcctgggcgtgggcacaagctaccagtcctatacaaatcaaaatggcgtaaatacacttccttatgcaaaatctgtacatcataattatgtcaacaaatttaaccaaagccgcgccggaagcgctgtaaggccccgttaaaagttagttaaaacattttaatatgttcttatttagttatccggagaaagaacaattaccatccactaaaaagccaatataataagatgtttaaatatctcccaacataggtctcagtacaatttcctctacaacggtttgtttggccattgtccatgcggcccatattacgctggctatatcttcggggggcatcattctgtcgggaggggcgtcaaagccttcccaggaagcggttaaggttgggcccgggcttaccgccgaaaccccgatgtagtgtgcctttagctcctccctcaggtttttggtgaagccaagcagggcatatttggtaatgctgtaagcgccgccattggggtatgcgcggtagctggcagtggaacacatgttaaaaatatatcctttacgccgggtgatcatggcgggtaataatgccctggtaagatgataagcgctgtatacatttaccgccatcatcttttcgagtaacccttcttcttcctggtgaagggcgccaggtacaaaaataccggcattgttcaccaggatatccacctgcggaaatgccgcatttattttatctgcaaaagccagtacctgtgctttatctcccatatccaccacctccgccagcaccgttactgccgggtttttccgctgaatatccgctttggccaaagccagcgtgtcggcatgtcttgcacaaatagccacattaaatccttccagcgccagtttttccgctatagcctttccaatccccttgctggcgcccgtaattactgcattcatagtttctttcattgatgcagtaaaataaggaatttactttgaatacaccggcgccttccacccatctctgaggtattttgtacctttgcgccgtcatgaaatacaaacatcttttctttgacctggaccataccctctgggactttgaaacaaatgaacaggaaaccttgctggagctttataacaggcatggtttagagagcaggggaataccatcttttgaggcgttttccgtttcttatgtggatcataacgagcgcctgtgggatcgcttccgtaaagggttcattacccgccgggaattacgcgacaagcgcttccgccttacattgatcgactttaaaataggagatgaaaaactgacccagaaaatcagcgaagaattcctggaaatactgccatataaaaaagcattattcccggaagcaaaggaaacgctggaatacctggcagcaaaggaataccctatgcatatgatcaccaacggtttcgaggaaacacagttgctgaaaatgaagaatgccgggatcgaccactatttcacgcacatcgttacatcggaagtggcgggcagcttaaagccttaccgggaaatttttgattatgccatcggcaaagccaataccagtgctacagaaagtattatgatcggagatgccatggagctggatatcaagggcgcccatggtgtgggaatggaccaggtatattttaatccggctaaaccaccggttgattttcaacctacctatgtgatcgggcaccttggggagctgagaaatattctgtaagaaagaaggagatgtgataaccacatctccttctttctttattgtgctttcgcttttgttttggtagcggcagccattctcaggctggcggttttagacggctgctgacaacagcttttaccttttgcggtagttttacacgaggcagccgaacaatcctttttagatttagcggctgttttggttttctcctgtgccagcgctacgcctgctatcagcagtaaggcagtcaggccggtaaaagctttctttatcataataatgccgtttagctactaaagatacctagattttagcaataacagtaatgccaccctgcactacctgttccagctgtaccgctacttctgtaccgataggcaggtaaaggtctacacgggagccaaacttgataaagcccatttcttcattctgatttacttccatgccaggtttcaggtagttcacaatcctgcgggcaagtgcaccggcaatttgtcttaccaggatatccgttttaccgttaccgattactacggaatgcctttcgttttcagtggaagactttggatgccaggccaccaggtatttgccggcgtggtattgcgataattttaccgtacccctgattgggttccggtttacatgcacattggcaggactcataaaaatagacacctgcaaacgcttatccttgaaatattccggctcatatacttcttcaatgaccactactttaccatcgcagggagaaacaaccagcgaatcacctgttgtatattgacgggagggaatacggaagaatgaaacgatgaacaggaagaacgcaagggagataatggataccgtccagcatagcgccggcgcgttaccgaaccaataaaatactgctccgtttattaacgccagtaccaggaatacaagggaaatagtagcaaatccttcacgatggatcttcattgtttttttattagatgtttgatttatgtgtttaatctgggtgcaaagttactttaattcaatttttttagaatacgaatattttgttaacgtattacagcataaaaaactgaacatagatccaggcgaagggagccgccagcagcagcgaatcgaaccggtccataaagccgccatggccgggcatgatccggccggaatccttcacgccggccatccttttgagtttcgattcaatcaggtcgccaatggtgccaaatatggcggcgatgagcgccagcgctatccagtgttgtaaggccaggtactggtagccccagaaatggccataaatgccggcagtagctaccgcgaggatcatccctcctaccgtcccttcaatcgtcttttttggagaaatagccggggcaaaaggggtacgccctatcagcgacccaactatataagccatagtatcatttatccagatgaatatgatcagcagcaaaggaatgagccagccgggagcggtgcctacgttttcgggtgtatagtgaatgttgatggcattcatccggatatggatcagcaacccaaacggaataatcacatacaatagcccgatagccgaatacccgatattctttaaagaaaaatctttactcatcaatacttctcccaaaggcattaccagcaggaaaataacggctgtccaccagccaatcagcccggtgggcatgccgcctatttgaaaattatctccggtaaaagtaagcaggatggcggctcccgcgatggtagcgccccatttatgccagggcgaaacgccggcatagtcagcatcgatcccacgcagcagcctgaagtactcctggagggcaaaacagcctatcagaaagaaaagcaggaaaaaggtgtagtcggcccataggatccctcccagcattactgccacaaacacaagcgcagaggcagtgcgggtgaaaaatgtcttcattatggttgtatctgttgattaagttctacccgcaaaagtggataaaaatagcctacggagcaaatcccgttctggaactgcccgggggcgccattccacgggagctgtcacttacgcttccccatctatttcattaggatcgccggtaggcaggttgttgtgattgtgtacaagatccctggctaattgttcctttgattcatgtacatacaattccacctgtcccggcagcgtgatattataggaagacgactgacggttgagtaaaaccgcctcaatgtcgttgtccagtaacataccctttacaatttcggcttcaaatggcctgtcgctcgaaaaaactttaacccagtccttctccataatgattgtttttagtgtcttttattaagattaaaaattttcgtctgttccaatttcatccacctcttccccttcttttttatccacgggatctgtcatcagcatgggggtggattttttacttaacgcccaaaacagtccaatggttacgggaacgcttaaagcgatataataccattccacgggagtgtttttcatcggatcgtcttttatcatgccatgctggaacaggtacagcagcgttacctgcagcccgttgttcaggatatgggcaaagatgcttaaccacaggttaccactgatcacgtagatagctcccagcgcaaaacccattaacacacggggcagaaaccccagcatttcgccatggatggcgctgaataagatagccgtgataaatacactcagccatacctttccggtagctttaataatgagccgctgtaaaacgccgcggaaaaacagttcttccgcaatagccggtacaatggctaccagtatcatgttaatgaaaagatctttcagggtaggcatcttcagcataatgcccagcagcttttccgccatatcctggaggtcgcgggccgattgggaaataggccaggtttcgttccactcacccagcaggctggccaatggtaaactgccgtacatagccagcagcgccagtataacctgtaagccggggggcgttttaagccccaggtatttcatcggataaggctgccagaggtaggcaaaaattgccgccggcacaaagaaggcgaccacggtataaaggaattgtgttattttcagatagccgatcgagttagggtcggtaagcgtgccggtttgaagcgcttccagcgtttgaccggtaacacctggcgtaattgcctgaagcgcataaaggtacagggcaaagaacccaaaggaaaagcccaggaaagagacaaactgcaatgaaacgggagactgcttcagataaccggacataagaagatactgtatttttttgcgtaaatttacagcgcgaaattaagtttttgcagatgcttaccgcttaccgcaactgctgaacgatagccgttactgcaaagaaatcctgcttgtaaaagaaatagtatataaaatattaaaataataactccggcaaaagctgctgtggttatataaattatggtgaagataggaaatattgaattgggagaattccctttattactggcgcccatggaagatgtgagcgatccgccttttcgtgcggtgtgcaaggataatggggccgatctcatgtatacggagttcatttcttcggaaggactgatacgtgatgccatcaaaagccgcaaaaaactggacattttcgactacgaacgtccggtaggaatccagattttcggcggagatgaagaatccctgtcgctggccgcacaaattgtggaagccactaatcccgatctgctggatattaacttcggctgcccggttaaaaaggttgcctgtaaaggcgccggtgcgggcatcctgaaagatattcctaaaatggtaaaacttaccgctgccgttgtaaaggcaaccaggttgccggtaaccattaaaacccgcctgggttgggacgacgacaccaaaaatattgaagatgtagcggaaaggctccaggacgtaggcatcaaagcccttactattcatggccgcacccgtacacagatgtataaaggcagcgctgactggaccctcatcggaaaagtaaaaaacaatccccgcatacaaattcctatctttggtaacggtgatatatgtacgccggaacaggcaatcgccgccaggcagaaatatggcgtggatggcgttatgatcgggagagccgcaatcggctatccatggattttcagggagatcaagcattttatgaagacaggcgaacatttacccctgccaactgttttggaaagagtagaagtttgcaaaaaacaccttcaccagtcggtttcctggaaaggtgaagtagtaggcatactggaaatgcgcaggcattatacaaattacctcaaaggtttgccgcatatcaaggaattcagacaacaattagtaacttacaatacattagctgagattgaggaagtactagacgcggttgtgttacaatacaaggaccatatattcgagcgggccgctccccaattagctgcacacgattttctgccggctgataatgaaatggccggttgtaacgtttacggataaacggataaaccccaggatataaaaaaaataaaaaatactttcacatgaccacaattaaaaatctgaaaaatgaagtctggaaagacttacagattaaaaacaaatctgccctgcgtaaaaaatacgccgtttcaaacatggggagagtgatcagttatcatgaaagtaccgaagatggtaagctgctcacggggtctaccgtagaaggctatacggtattaaacgtaaagcccgcagacagctaccagtcactgtacctccacagggaagtggccaaacttttcagcaaaaaaggaggacgggcacataaatatgtgatacacctggactacgataaaaaaaataataaagcctccaacctccaatgggctaccaaggaggaaatggaagaacatcagcaaaaaagtcccgccaagctcgcctacaaagaaaagcaacgcaaccgcgtgaaaggactcaaactgaatgttaccaaagtaaagagcatcaaacgcctgctgaataaacccggcaagaaaacaatgaagcaaatcgctgaacagttcgatatcagtgaaatgcagctctaccgcattaaaagcggcgaaaactgggggcacgttacactggattaaagcctggtttaccaggactgatcatatatgatgttgtctgacgatggccatactaaccgtatggccattgttacttggagccgtaacgtatagtacctgccgttagagtacgcctctgctcatctcccccaataccttccggtaatgagcgctatcctgcaacactggctcgtatcccagcaatatcacctgttttcgtgcacgcgacaacgttaccaacaacttccggtctacctctatctcctcttcttcccagttaaactgccccaggcactgcaacgtttgcacctgcgctgcatgatataccgccagcgacacaatgataatatcgttttcagaaccctggaaccgctccacggtatcaatattaatgtcctgcaacgcttcatcatccgcaatcaactcccggatcaagctgatctgcgttcgccatggcgttaccacccccacggtatctttactgaaacccgcaccataacggttcttcaggtgatgcagcagcgacactacccacgccgcctccgtcctgttcatcttggaactcggctcatacgggctgccaataaatacttttcttcctaaagataaaacccgctcccagcctaaattctcatgaccgtcatacaaatcgaaaccggctttttgctcctctcttccggaagataactgaccagcatagtaatgatttaccaatgccgcaatgctgtcatgcatccggaagtgggtattcaacatgccccaggcatgccgccactggctggttttacagcgttgtatgagccgctcgaaaatagaggtccgcaaatccccgatacccagctcctgtaaacagggcgctttcacctggcagaaatgcgcttcctgcgccaccaccggcggcaactggttctggtctcctatcaggataaatttacgaaatggcatcagcaaccccagtagctgtggctcggttaactgggaagcttcatccacaattaaagtatcggcaggaatccccatcattgtaagctgctccagccgggtggccatagtagccaccgtggctacaaacacacggtgactggtaatataattccgcgcctcatccagggagccttccaggcaatattgccggagcgtgagtgaagcggaggagttacgcccgcccatacggagatgcgtaatatttttagccgtcagcttatggcatatttcttccaccgccttgttggtaaacgcaacaatgatcacatggtgatcctgttttaccatctcccccactatagtagtaagcatggaagatgttttaccggtgcccggcggaccctgtaacaggtaataatcctgcgcctccagggcatgctttaccagctgttcctggttaggattaaacatggccggagtagtgtgctgtaaaggataccagcggggtgtagtaagccccaacagcatattggtacgctcacggtaaagcggggaaatcacatgaaaaagcgacgccgttgctatccagtagttggattcataaatatcatgctctatgatccactcatcaaattgccggaaaaagtcgagcgtcatctgccggttattcagggaaaagcttaactgatttttcccgagatcctctatcctgcctttcagcaactgttgctgcaacggctgtagttcagtgctggtacgcggataaataatagcggtatctcccttgcggaaattatggctaacgggaacgactatattaaataacacggagctgttaacagtatcaaactcccggaagcggagcgctggtataatattgaagcgggatagcttatctttttcctgttgcagccatagcgctgcaaagccgtctgcatcttcctcccggttaatttctgaaaacatgccgcacttcgcctgcaggtattcccgcagcataaaggcgaggaactcgtgataataggcctttgccacaggaggcgccgtttgccaggcctgttcaaaggtggtgaaatgcgcagcactgaaagaaggcaggcccagggcagctgcggtggtgatagtggacagtatttcaaattccccgcccgcaagccgcagcaacatacccacgacttcattgcgcaatagcagcagatcattttcggtgtgatgtgtactgctcacgtttcgcagaggattggtggcggcggcagaatacaggatggcggatcctccctttcgttgacggccaaaagcagagcgcagcaggagattataccccactacctgcatttcgtggtttttccaggtattaaagtcggggcatttcccgcttttcagctcaaaaatctccttccggtattcatcggtatcatcttctgccatgagatccagtcgcccctgcaaaccgtactgggcggacaaaaaggtgggttctatcttcaccggtttatcctgcagttcttttacggtattatgcaggttgccccagtgttgctgccggatatcgcgaaacatgtcgttgatcttttcccggccgtaagcggccgcctgcagtacattttctgccacggcttccacaaaagagcttttgaaatctatgtcccggttgcggagcatttcatccaggagggcatttaccaggtttcccttaaatgccgccgggctggattgctggggagtaagttttttaacaagatataatagccggttaggtcctttatgggtgaaacattctgccaggtcgctgatatctatcagcagatccggctccagtacaacctggctttcgctggtggtagtgtattcgtgtccgttggtcccctggcggcagtggagtacgtgaatggtgtcgtaagggcgtagcagtccatgcagggatattaccgcttcagggtccatatgttccagcagcagctggaaatctccctgctcgtcattttttacatccagcagcagggtatattttccgagcgtggtggtggtgagcgtgcctactgtggtaaccatacatttcagcaatgccaggctgccggggcggtgttgccatgcaagcgacagtttatgtgagcctgcggaggcgtatagtgcggtgagttctgcaggcggcgctatttggtagcaccaggccacagattccgtaagggctttgatgcacaggaggtgttcggcgtcctgcaggggaaacattccccgtgtagccttattagttagtatgcggagcgccgtcagctgctgatggatatccggtggcacggattgccggtcgaaataaaactgcatgcgtgcaaacaggtttccgaaagagcgggtttctttgcgggtcagctcccggaaaaggatttccagtatctgtttatagtgacgggttttatcttccgtatcaggaatgttgtgggcttcttttattctggcgtaaaacgcagttgctgtatgtaatgcctgcatatccgcaagttaatgaatcgttgccgtttgcatggatgcagcatttgttatacctttcttacgatttataatgtaatcttcattttttatgtcagccaaaaaaatagccattataggtggaggaaatctgggatcggccatcgcccagggattgctgaagagcgggttttcaaaggccggcgatatcattgttaccaagcgtaacaccagtacccttacggatctgcgtgacgcaggtgtgcggatagaaacggacaatgatattgccatccgcgaagcggaaattattgtggtagctttaaaaccgtacaatgtgcgggaagtattgcaggagttcaaagggtcctttaacccggcaaaacatatactgatcagcgtggttaccggcgtaagcatcgacgacctggaacatgtggtacccggcatgccggtagtgcgggccatgcctaatacagccatcgccatacaggagtcaattacctgtatttcccataaacacgccaccgaagaacagatccggtatgtaaaaaccatgttcgatcagctgggagctaccgtaacgatcgatgagaaactgatggatgccgccacagtgctgggcgcctgtggtatcgcctttgcgctgcgctatatccgggcaaatatccagggcggtattgaaatcggatttgatgtgcgcacggccagtttaattgccgctcaaacggtaaaaggggctgcagagctgctgatccgtgaaaaccgccatccggaagaggaaatcgacaaggtaactaccccgaaaggctgcactattgccggtcttaacgaaatggaacaccagggcttcagttcttccctgatcaagggaattaccgcttcttacaataaaattgtgaaagactaatctttacggggatactcgaagaagaggaactttttctttgccaggtcaaaatctttccaactatcggtgtctgcctggataccaaagataccggtagtaggtacattatctatcctgatttcttcggtgaggtaattggcaaaatcggtgatgcctgggttatgggcaaagatagccacggcgccgaagtcgtcatcaattttggtgattaccttcaggaaggtggcggcatagcagagatacagttcttcttccagcaggatcgcctgtttgggataactccactcattcgccattattttagcggtagttctggctcttttggccgggctggaaataattaattccggcaccatgccgcgggtaataaggcgttgtgccatttcgggcgcgttcgcttttccccgtttattgaggggccggtcaaagtcatccatatccggatcggtccagctggatttagcatgacgtataagtagtaatgttttcatgggctgaaaacctataattaactattacgaaaatacagattttacaggaagttaacttgttagacttatacagtcaggaggaagggggttatttaagataaaattaacatgaaaacaaatagtcatttaaaaaatcagagatctgattattcagctcaaaagaagaatttcttctgataaccaaatgaccagatctctgattatttatacgattaatatcctctttcgtttttgccttccatatagttcatgaatgctttattcaccacacggttgccgcccggagtagggtaattaccggtaaagtaccagtcgcccaggttgttcggacaagccagatggaggctttcgatagattgataaatgacttctatttctgctttaataccgcctgggttgaggatttctgcgatcttggctgagatctgttcaggggtaaacggcttatagatattcttcactacgttttgtgcgtgaagggtattggtgcgttgcagttccttgcagaggccgtaggcttcgttcaggatatgttccttgccatgatctttcaggagggcaatagcggcctggaaggctacgaaatcgcccatcttgctcatatcaataccatagcaatcggggtagcggatctgcggcgcagaagatacgatgatgatctttttgggtcctaagcggtccagcatcttaacgatactttctttcagggtggtaccacgtacaattgaatcatcgatcaccaccagcgagtcaataccgggtcttaccttaccgtaggtgatatcgtacacgtgttgtaccatttcattacggctggagtcttcggtgatgaacgtacgcatttttacgtccttggtggctattttatcgatgcggatacggcggttcaccatttcggtgagcttttcctcatcaaaatcattaccccaggaaaggatgcgttctacttttattttgttgagatattcttccagtccttttaacaggccatagaaggctacttcagcagtatttggtataaaagagaagatggtattgcggaggtcattgtcgatcgcctttaatacggtgccggacagatgacggcccagatcagtgcgttctttgtatattttttcgtcgttaccacgggagaagtaaatcctttcaaagctgcaggccttacgttctttaggttcgagaatttgttcgatggagtagtcgccgttgtttttaacgatcagcgcattacccggcatcagttccagtacttcattttcgcctacattgaaagtagtgcggatagcggccctttcggaggcggctacaatcacatcttcattaatatagtagtaagaaggacggataccatgtgcatctcggatgacgaaagcatcgccggagccgatcaggccgcaggtatggtaaccaccatcaaacatggaaaatgcctgttgcaggatctttttgatatccaggtcgttgctgccttcattgtcctctttagcgaggaaatggtgtacaacttcgagcatggcggcaaggtcactgtttttgtgtacttcgccgggttgtgccttggaaaactcgaacagttcgtccgtgttaatcagattaaagttaccggccatggcgaggttgcgggcaggaatggtattgtagcgtacgaagggatggcagagttccacgttgtttttaccctgggtggcataacggatatgtcccatcatgagttcaccgagaaaacgaacatggcctttcatcaggccggggtatttggtgatttccggctgatatttttctatctcctgtatctcatcacgtactttcgcgaaaatatctccgatggcttgtggagcagcactgcggatacggtgcatgaaggggacgcctggttcggtattcagtttcacggtagccaaaccagcgccatcctggcctctgttgtgttgtttttccatgagcagatacagtttgttcagcccatagaaaacgctcccatatttttgttggtagtaggaaaacggttttcttaatcttataaatgccagaccgcattcatgtttgatcgcatcactcatggcagaaaattgaagtcgcaaaggtacgccaaaaaaggagaaaaccagaaagcgattgtaaagctatcagcctttgcctattcagtatcagggcataaaaaaagcggagataagagcttccgctcctatctccgctttgtataaatagtattgttattgcttggccagggcagccatccactggctgatatggttacagtctttgtattgatcatctacgtgaacgtagaaggtcgggatcttttcgatgagccatttgttaatggcttccgcgcgtttgatatccagtgttctttgctggatgcgggaataatcatctgtaaggttctcccggtgtggctgggtacgtgttttcaggtatacgatccgtactgctgcacggccgttttcgtctgtatactgtacgggggcggaaatctgacctgctttcagggtatcgagcatcattacgatatccctttcggttggatcatccagctgatcaatagtgatcagggtgcttccgtcgccggttttggactgcatcataccgccatcaaatttggcgcttggtgcgtcgctgtatttagctacggcttctgagaaagtgattttgcctgctacgatgcttttacggatggaatccagtttggcagtgttgctggccaggtcggatttggttactgcggctcttacgaggatgtgttgtacagtaacgttatcgccggagcgtttcagcatcatgatcaggtggtatccgtgttgcgacttcaccggggaagaaatttccccttctttcaaacggaaggcagatgccaggaagtcgggatcccaggtatttttatcattacggttcagggtatacacacctttgttatcctttacgcccggatcttcggagtacaggatagcgagggagccgaaatctgattctttattctgaacgcgttttttgaaatcgaggaggcggtcaatggcgtattggtccatttcgcgggtagctttgggctgcagcacgagggtacctatttccagttctgactcgtaaaaatggaggctatctttagggatagcgtcaaagaagcgttttacttctgagggtgttacttttaccggttcaatgattttgttacgcattgcctgggccagcaaaccttctttgataggctgacggaagcgttcgcgaagctggtaaatggagtagccggtaacttctttcattttctccttactgccgtacatggattcgaagtagcggatacggttttccatctgggcttccacgtcgccgtcacttaccggtaaactgtctctttccgcctgtaacaccattactttctgggaaatcagcatttccagtgttttgcaagcagcatcaggcgccagattgccatcgggtgagttgtgttgctgatcgctgagtgctccgtccatatcggatttgaggataattttatcccctacaacgccgataatcttgtctgccaccagtttctgggccgtagaagcctgccatagcagcaaggcacctgcggataatgctaaaagtttcttcatacaaaagcggtaaaaaccaaaaataaccatttaaaagtcagtagcatagggaatgtcgatggatttaacaaaagtttagataagctgccgccttttaaccataagcatcttagccaaaaaaacagcgaagaaaataacgatgataggttttacactatggatcgttcttttcttcgctgtatgttattttaaagcgggtagtttttggctacaggcttcttataaagttctcttcacttctacttcttcaaacccttcgatgttatcgttaggtctcagatcgctgtatccgcggacactcaaaccacactccatgttagcggccacttctttcacgtcatctttataacgtttcagggagccgagttcgccggtgtgaaccacgataccgtcgcgcaccacgttgatacgggtgtttcttgtcagcttgccatcgataacgaagcaacctgccacggtaaccttctcgaatttgtaagtttcgcgcacctgaacgttgcacaccactttcttctcgatttttggttccagcataccttccatggcgctcttgatttcgtcgatcgcgtcatagatgatggagtagttacggatttcgatattctctttctccgcgagcttggcagcctgggaggaaggtcgtacctggaatccgaggatgatggcgtcagaagcggttgccagcaatacgtcggattctgtaatctgacctactgctttgtgaacgatgctgatcacgatttcttcggtagacagtttctgcagggagtcactcaacgcttctacggaaccatcaaagtcggctttgatgatgaggttcagctgtttaaagttacccagtgccaaacggcggccgatttcatccagggtgatatgtttcttggtacggataccttgttcgcgaacgatttgtgctctgcggttagccacttctttggcttcagattcttcggagtacatcttgaacttctcacctgcctgtggtgcaccattcaagccgagtacctgtactggcatggatggtcctgcttcttccattttctggccgcgttcgttgaacatggctttgatttttccgaagaaggagccggatacgatggtatcgccctgacggagggtaccattttgtaccaggagggaggcaacgtaaccgcgacctttatccagggtagcttccacgatacttccggaggcttcgcggtcgggattggctttcaattccagcagttccgcttccagtaatattttttcgaggagcacatcaatatttaatccgcttttggcagatatttcctggctctggtatttaccgccccagtcttctaccaggaggttcatgccggccagttgttccttgattttctcagggttggagccttctttatccactttattgatagcgaacaccattggtagtccggctgcctgtgagtgggagatggcttcttttgtttgcggcatgatagcatcatcagcagcgatcacgattacagcgatatccgctgctttggcaccacgggcacgcatcgcggtaaacgcttcgtgacctggggtatcgaggaaggtgatctttttgccgctggcagttgttacctggtacgcaccgatgtgctgggtgataccaccggcttcaccggctaccacgtttgcactacggatgtaatcgagcagggaggttttaccgtgatcgacgtgacccatgatggttacgatcggtgcacgtggaaccagatctgcaggatcatctacttcatcttcatcatcggtttcttctgcatcttccagaccaatgaattcaacttcgtatccgaattcgccggccaccagttctattacttccgcatcgaggcgttggttgatagataccatgataccgaggcccatacatttagagattacttccgcgaagcttacatccatcaggttagccagttcggatacagaaacgaattctgttacctggagtttgttgtctccgtcgccctggttaattttctggttggctctttcctcacgtttttctctacggtgtttagctttcacgtttttaccgcgaccgccgccaccgagcttggccattgtttccttgatcttattctggatctcgttcttatcgatttctttttcttcggtagtacgtttatcctcaccgcggtgttgacctggtctgttgtagccgccaccctggcctggcctgttatagccaccgccttgtccgggtctgttgccgccaccacctggtccgccacctggacggttgtaaccgccaccttgtccggctggtctgttacctccgccgcctggaccgccttgtccggcgggcctgttatagcctccgccctgaccctggccttgtccggcaggtctgttgtagttacctccgccgccggtacctgtgttggtgccgcctggacggttatgggtacggttatcgccttgcggacgatttccgccgccctggccctgatgtcctcctccgcggctatcgtggtgagggcgattgccgccttgtccaccatgctgatgcgggcggtgttcgcctggggcgccgccttctttgcggtcaccttctttaaagtctttaggctgaacgggttcaggtttcttttccacgatgatacgcttgcgtttgcgtttctcatcccggctaaagttgctgttcttattattatcgcgtctgtcagactgaactggcagctcaattttgccgatcactttagggccggtcagtttttcggcctggatgttttcgatcaccgcagagccagcagcctcgtcctgtgcctgtggggcagcggggggaggtgttggtggggtgttttcggcagtagagggtttgcgattttccgtttttacgacatgtttaacaggaacgtgcgccggttctttgactgcagccggttttgcggcttgtaatacttcttccacttttttaactacaggtttatcttcaaccggtgcggctttttccgttttgtctgtcgtatcggtcttttctgttttcgctactttctctgctgatggagtgttttcggctttaggggcctgttccacgttttcagctttatcagctttctcaactggtttttcagttggtgctgtagttgcttcctgtacgggaggggcaggaacgggtttaggttccggtttttcagcaactgggggagcgggtgtaacgggagccggtttttcttcttttaccggtggtttcactgcttctggttgcggagccggggtttcttcctggtctgcttttttagcaactggttttttattgcggtttaatgcgtccagatcgatagtggtgatcactttagggccgttgattttcggcgaatccgttttcttcactgcgtctggttctgccggaggaggcgttgccggtgctttgggaacttccgcaacagggggagctgtaacaacgggtggttcaggcttcggttcagctttttcctttgcgggaggcggagttgcctgggcaacattcgcctgtggttgcagttgcggtttaggggtttccttaactggttccggtttaggttcaggttttgcttcctgtttagcagcaggagcagcctcttctttttctttggtggtattctttttagccgccgcttccgcttcctccttctctttcttcttcatcgtttctaacacgcttcctttaggcagggctatctggtcgcttttgcgcttgttagccttgtcctgctggaactccgactgcagtgctgtgtacataacagccgtaagacgggcattgggagaaccaaagccgtccatatcaaagcctttattgccaaggaaatcgatgagggtctccttaccaatattaaactctttggctgcagccagcaatcgtggtgtgttgtttgttgtttcaggcatatcgtatttcgggcctcccctgtttcccgtttcttcaaaacgggatgtttttttacgtttaaacaataactcgaaaaaatcaattccctttctaataaggcctttacctgggaagggttgtggctcggctttattctttgtcaaactcttcctgtaatattcttcttacatcctgcactgtctcttcttccagatccgaacggcgaaccagttcttcaacggtcagctccaatacgctgcgggcagtgtcacaacctattcgtttaagctcatctattatccattcttcgatttcatccgagaattcttccagatcgatatcaaattcagactgttcctgcgcttcatcacggaatacatcaatctcgaaaccagtcagttcacaagccagcttaatgtttactccttttttaccgatagccagtgatacctggtcagggttgaggtaaacggaagcgtatttgttttcgttatccacttccatgcggctgatcctggcgggcgttaaagaacgctggatcaacaattgaatgttggtggtaaagttaatgatatctatattttcatttctcaattcgcgcacgatgccatgtatacggcttcctttcatacccacacaggctcctaccggatctatacggtcatcgtaggattcaacagccactttggctctttctcccggttcacgaacaattttcttgatcactataagcccgtcaaagatctcaggcacctcaatttccagcaatttagccaggaaggatggatgtgtgcgggagagaatgatgagtggggcattgtttttcatttctaccttcttcaccaccgctcttacgttctccccttttttgaaataatctgtggggatttgttcagacttaggcaaaattaactcattcccttcatcatcaagcaataaaacttcttttttccaaacctggtatacttcaccgtttacaatttcacctgctttgtcggcatatttctttaccaggatgttctttttcagatcgccgatacgggcagataaagtttgttttgccgccaggatagccctgcggccgaaatccatgatctctacctcttcatataaatcctcaccgacctgataatccggttctaccttaatagcttcggaatatgcgatctgtgcattatcatcttctacttccccatccgttacgatggttcgacggcgtaatatttcaaggtcacctttttcggtatttacaatcacgtcaaaattctcatctgagccatactttttccgcagaagcgttttgaacacatcctccaggaccttcatcaatgtaggacggtcaatgttttccgcctccttgaactcggtaaatgactcaatcaagttaatactagccatgtttagttgttatattttaaaacacgatgcacacctttatgtgctttatttcattaagttttaaatcagttgacttcttttcttttttcttgccaatcagttcctcgatgttaatagcatcttcggttaccgtttgcagggtgccctcttttacagagccatccagcagggtaacttccactttgcgtccaatatttttaaggtattgtctgtgcagtttgagcggttcatccaggcctgcggacgaaacttccagggagaaatcgttatttgggaacagttcagccgcttccagcaaaggatataactgacggttgaatgacaccagcgtagccaccggcacccctttatccccgtccagaaagagcttgatattgttagtgggcttaattctgatgtctaccaaaaaattgtcgggattattcgccagcagtccttctgccatttcccggatagtttttatcacgtgttcgtttgccatacaaaaagcgcgaaggggacaatatctcgtccccttcgtttgaatcatttttccttatacaaaattaggattttattttgattgaaaaactatttctttaacttgtatgtaaatatttatgtaagatgctctgccatcattcatatgtgtttttaaaatatctgacgtggcgaccgctttctggcgaaaaataaatatcgaactgctggcatggcccctgggcctgaccctcctgtatatgatgccgcccgacgaaaatgccggcagcctgtgtttctttaaaaatataggtctccctatttgccccggttgcggattaggtcatggtatccactattttttacacggacaatggactgcctccatccaacaccactggcttgctcccctggtagtagccgtgctgctgtaccgcaccgtgcaactggcccggtatcaatatactgatttcaaacaatcataaacccaacactatgaacgacttttcatttgcgatgctccccggaattgaagccgaggaaatgatgtggctacaggaactgaccaagagctattctgccgaaaacaagcagcggttcctggccgtataccagggcagacgcaaagatccgcaaacaatccttatctgcagcctcataggtttcctgggcgtagccggtgtgcaacgcttcctggtagaccagatcgccatgggaattgtatattttatcaccctcggtttctgcggcatcggtaccattatagatgccatcaatgcccgcaaaatggcctggcagttcaataaaaaagaatccctggcatcagccgctttactcggactttaaacgctcccagaaagttaaaaaaaccttaaaatgaggtggttttcaggaggtcgaaaaggatattccgctaccttcgtgtcactatgtttagattttttctttctatatttctggcctggctgctgtacaaactggtattcgacctgatcataccaggctacagggttaccaaacaagtgcgcagacaaatgagcgatatgcaggatcatatgcgtcagcagtatgaacagcaaaacggcggaccaaaaggtccacaacctcctcctaccccacaacccaaaaatgtggataagggagattacctcgattttgaagatgttaaatagaaaaaggccggtgcatcaccggccttttttataacacctttttaggctgaaaaatatccataatcgttcggggcgcctgcagatgaatggtttgcaaccctaccgccttcgctccttctatattgggcaacgtatcatctataaacaacgtttcctccggcaataacccgttttcctccatcaccatcaggtacgactccttgtccggcttgcgatgtcccatcaggtgcgaatagtaagccctgtcgaaaaagctgcccagcgaaggaattcccctgctttcctgcaacaaccggttgaaagcctccaggtgtatcgcattggtattactcagtaaatacaggttataatgctgccgcaactgctgtaataactgcagccgctgtaaaggaaaatcgagcaacatcgcattccaggccgctgttatctgctcacccgtaaccccctccggcacatgacgctgcatttccgtcagaaattcttcctcggaaacatgtcccgtttccaggccattaaataagctggaaccatgaaactgtgaatacaactcattgaagttcttcacgccaagagcaataaatgcctcgttggtaagctggtagttgatgttcagaataacgccacccaggtcgaaaataatgttctttatgccttgcatgccgcaaatttattaagtatatgcgtaagcgttgggattaaaaaaaaatttaggttaattcaataaaataattaattttgccgtcccctgaaaaggggaaattagttcttcggaacaggtcctatagctcagttggttagagcacctgactcataatcagggggtccctggatcatgcccaggtgggaccacgcaacaggaaaggctttcagcggtgagacgcggaaagccttttttcatttgatacatgttaactgcccattttaatattattctatagaatacgcttaattaccaatcccatccctcaataaggaagcctattgaattataacccagtaacatttctcaataagtttttattacgcaaatagggtacatatcctatgcctattttcaagtaaatctttgttaaccacaaacccttatttatgacagttacgtccattaatgcccttaaaagcctgagtactccccaggcaaacactatttaccacgttttaggctatgcaactgccaacgatggcggtggcggagaattctactgggacagcagcgacaccacttctcctgaaaatggaggaacaatttttattgcttcaacaggtcgttggaaaagactacatgacggcgaattaaatgtaaaatggttcggtgcaaaaggtgataattctattaatgattctccggcaatcaataaatgtcttgactacgccaaacagatatttacgaatggaggcaaactggtgttccctaggggccgttatcgcatctccgaaaccctgaatatgaccaatgccactttttggcagattatcggagaaggtgccacaattgctcctgatagcgccattaccgccattaatatacaggctagccgatctacctacactggattgaatattagtttcgagtccctacactatgatcagatcaacgagaactgcgttgctatctggctccacaaaggtggcagcaccgtaaatgaccaggtgaacaacaccacttttgagtgttttactattattggcgctcatactggtatcaaatcgacaccaaataccggcctgatttggcagttggattttaaatctatttacttcgatatctatgaaggggtttcctccatacaggcaataggatttgatattgccagtggttttaaccagggaggcagcaccaccataaggatttcaaaatgttgcattcaaagctttatagtaaaccgattgaacagtaataacgaaccggtttttccaaaaggtgttggatatagaggatatagaatttactattctacagatgtttatattgttgattcttcctatgatggttatctgggcgcaaccctccagctgaatcaaaatggccagatcatggatattttttcgaaaaatattcatatcgatggatttcactgtgaggccctaacaaatacgctaaacgccaataatacacaagccccgttccggatcaacagtaccggatttctcgatatcaagaatgttgtaatattggattcctttatgaattgtggaggtccaacggctgccggtgcctggttccttttctttggtggtggcgtttttaactttggaacctacaacaacaacaacatcggttctgtagacaatacccccatttacattattacactcagcaacttgctggatggtgatgatgttaccaataaaagatcccagatcaatttatccaattcaatacagccatctcaggttcacctgttgaacaggaactataacagtattcattttgattctctggaagtaaatggtttggttactgctgtaacaggtactgctccggttacaattttaaccatgccaactacacgcgcttcctgtatgattgctgtaagaggattctcacagatagatggcacttcttattttatcgactacctggtaatatcccgttcaaggaccagtggaatcgtgaaaataaaatcactactcaatgataacaatagttatacaagtgtcgtgaatacttacagcgttacatctgatggaaatatccagcttgctagaaatatttccactggtttttgggtaacggctaaagttgtaaacatgatctaaccagaatagaattacgtcaggcgaaggcaattcagctttcgcctgactattcgccatatactacggaaaggaatcggtcaatcacaatgattgaaattatgtatcacaattactcccatctccccaaattaccacccccaccccaaatgaacccaaaaaatacccgtttcagtcatatattcaccggatattcagtcagctttaccgtttgctaagtggatgtaaacccaggcgtctgataaagatagctttggtacaataaaattattgtatcatgaaaagaacagtttatctatggttgctgctttgcctgccctacctgctgcccgcacaggacaagcccggctactttgccctgaaacccggcgactggtttgatatgcagatcacgaagcataaggataataattactatccggtaatggagccattattacagtttcaacgccggtatgtgctgcggtaccggttgcagaaccagttgcctaatggcaaccagcaatacagcatcactcatgaaagagtggtagcatatactccatatgatcagaagtttggctggatggggtacgatagttattatccgccttataaacaggggttagacaaaaagccgcctaaagggatgttccggctggaaattacagccaacggcgaaatcgtatcattgaccaccgacaaagatcaaccaccgttgccggtgttgatgacgagttatagtcctcagaagcaggtcggcatatccatccgttcaactttctcacctatgccgccggaggagctgcgccccgcgatagaagcgatgctgaaatggcgcagcaccaataacggcatacccagcctcattcccgccaaaaccgaatatcaatacgcccagttgcttaccggcgcgtcctttccggttgcaggcaatgcattgataaaaggcacgttggcacacgctcacaaaaagcaagtggaaattgaactgggagacagcaccctcagctttcctgttaatagccggggagaattttattgcccgttgctgttaacaaaaccggaacgccggtatattgctatggaaaataacggagggtatgttttcttagcgcctggcgatacgctgattattgaagcagatgctgatacttccctgcgacccagaaagctgtcgggcagtgccaaatggggttccatgctggcagaggatatggatagcatcttttacggtgccgagggcatgaataccatgtacagaaacaaaacattgcaggaagtgctggccgcacaggaaaacgcaaatgccagattcaaagcagtgctgcaaagctatgaggggaaagcatctcccgaaagtatcgactactataaaaccaactggcaataccgtattgcggatgactggctggtttttctgtataatcatggctaccgggtagccccggaaaaacggccatttgagggcataccggaaatgattaccaccggtattgataccatgccggtgacaatgaattcttatcacgacaatcacttctccttctatcatcaatacctcgattggctcctgatttatcagcagtcacgcatcggactctctgctggcggcagttcagaagaatcttccttttacagtaattactttgtcctgctttctatgctgaagggatacccgttgtactataaattatcaaaagggatcagcgagagcatgaaagcaaatagctttgcaaaaaatcagcggctgaaaccttatttcgaagactttattcgtaactgcgacgacagcagcatcattaaacccattataaaagattggaagttcatggaacactgggcgccgggtaatacagcgccatacccaatcctatcgctagccaatggcaaaacgtatgatttgaaaactcagcatggtaaaacgacctgccttatatttgaccatgccagctactttcaggatagtgcgttggttaaaatggttaaaaagcatcccgaagtaacctttgtgttcgcatggatcaatgagcctggccttaaccgccaacatgatccggaactcgcaacactgcccaactttaacagtattgaaataaaaaaccagggagataaaaactatgaagtatatgggatatccgaaatgggcaagaaaaatgttgttgtactggatcaatggggaaaaataatatcagatcatatctattccgacgacaacttatgggatgacctgaatacggccatcgatgatgccgcaaaagcaccgcgcttttcggtcctgcaaaaagccggcgtgatgaatattattggatggagccttggctccatcctctttactgtgctggtgggcatctggatttaccgggtgcgcattcagcggatcaagcgggcggaggccatgaaaaccgcgatccgggagctggaaattaaagccattcgctcgcagatgaatccgcattttatttttaatgcgctgaactccattcaatcgttgatcaacaccagccaacataaagctgccaatacctatcttgtaaaattttcgttgttattaagaagtgtattgcataatgcggaaaagaatatgatcacgctggcagatgaactggctaccatacgcctttactgcgagcttgaacaactgcgttttgatttctcctttgaaatagatatccctgaagaactggctactgacctggtagatatccccggcatgattttacaaccgctggtggaaaatgcgatcctgcacggtatttcttccaaaggaaaagcaggcttactccgcattacggtgggaaaacaaggcgcggcattactgatcgcagtgtacgacaatggcccgggatatcatccggaagttggtaacggcacgcataaaagtgtaggattaaaactggtacaggaaaggctgcagctttttagtatcgccggacaaacagccagtttgcatatcagtaacggaaacggcacaacggcattactcactattccaattgaaagtgtatgaagataaaaagtattcttgtagatgatgaggcaaaaagcagggataacctgcgcgtactcctgggcgaatactgtcaggctattgacatagtcggggaagccgattctgcggcgagtgcgctcaggctcatcaagcaactggaaccagaccttcttttcctcgacattgaaatgcccggaggctcagggcttcagctgctgcaatcacttcctgccaacaggcgctttgaagttatttttgttacagcctatgaccactacggtattgcggcagtaaaagcctgcgctatcgactatgtgctgaaacctatagatgtactggaactttccggcgcagtggaaaaagcgatcgcacagattgtaccccagcaggaaaacagccgtttacgggaactggtagccaatatgggcaagcccatggcagaaaaccgtattgcattcccactggccgataaaattatttttgccctgccggaagatatcgtacgcctcgaagcggcaggaaactacacgcatgtatacatctccggtcaaaaaaaactgattgtttgtaaaaccctgaaagaatacaacgacctgctggctgataaacattttatacgcacccaccagtcccacctggtcaacagccacaaaattacagcctggataaaaacagaaggtggcgccatttccatggaagatggcagccaggtgcctgtttcccgtcaacgcaaagaagaagtattaaagctgctgatgaaatagctaccatgtgtcctgatcaagtccacctttaagccgtgcttaagcccggtatgatccgtccctaaagcgtcacggccttctttattttctccgtttctgcggaagtgtcttttacccgcaacgacaggtaataatgccacaatatcatcgtggcaacggtccggtaaggctgccatgctgccgatattcccagtagtttctctggaggagtgtctttaggtaatttcttcacctgcttgagtgcatttacggcggccaggtctccaatggggaaaatatccgcgcgttgcaatacaaacatcaggtaaacatccgccgtccagttgccgattcctttcagcgctaccagcgctttccttacctcttcatccggcagcttttccatggctttagcgttgaatgctttgctttgaatggcctgggctaaaaaccgggcatacgacatcttctgccggctgaaataacaggcctttaattcttcgtccgtgagttccagcagtttggcgggtgtaatttttgtgagtttctctcttaatttattgagcgccgctaaggcggaagccagcgatacctgctgttccaggataatgtgtatcaggctttcaaatgtattgggtcttgtccacatcggcggatagccatatgttttcacaatgaaggctaactccggatcctgggtacatagttgatcacagatggagtgaaagttttctgttgaaaaggtatgcaacacttatttctggtttgtggaaagatagtataaactccccacgtcagcaagtgcctaaaacaacgtaggactaacactgttttctagttgaagtaagcggtttttgttggctataccacctgcaaatccgactaattttccggaagcgcctatcacccggtgacagggagcaataatagaaatgggatttttattggctgcaccgccaacagcacgtactgctttcggatcaccaatttgtttggcgatctcgccataggtcctcgtttcaccgaaaggaattgtcagcagtgctttccatatcttcttttgaaattccgttcccacaaagtccagttctacagtaaaagaagttcgctttttggcaaagtattcattgagttgttcttctgcctggcaaagaataggatgatgtatatcgtttgcaccggcgcttatgggtacgcggtctgcaagttcattttcccacagcactgcggccaaacctttgtcactcgctatcagcgtaagctgccctacgggagaagtcatttttttatgatagtatgtcatctttttatttttttatgatgatacaaatttaccatccacacccatctgaaagaacccgtttcttgcccttaatcctattaaatggccatttgaggaacatagcctgccctgaaggcattcaccacagaggccggcgttaaaacaggtagtttcccactccccggcaaagggatgccttttgcataaccaccgggcgaccataaatacagcaaccccttattaagaagataaggctcctccccgatgcgcacaaatgtgccgtcgggcaggttttccggatgttccccgaatgtaatctttaggttatgctcatctatcctttctgcatgaagggtgctatctatctctttaataagtgttttttcattaaaccctttatccggattacctttcaaccaaagggatttaaattgatgcgcttctgctttgcggcattcaaaacaaggccggtggccggcagcaaaggaagttgcttcatccataaaaaagagttccgtataccggttaggagccattacgggtcttctcctgtttttaaatgccaacatacaagtaatccaggtcttgatcttataaggcctgacaatttctttgttgtcgttgtgtaaaacgccccggttacccataaatagtcccctggcctctgtcctgataatattaccggatggatcaactctgttctgcaacatgccgatgcactttaaattatgctgaccacaagttacatatatccggaaagaatattgatgaaatactaatttatttagtattattgctaaataaattagtcatgagtatttaaaccagctgtcaactatgcccgcagataaagcagctattattgccggcttgcaaagggatattctccatttgcagggctttaaacaagccagtaatacgagtgtggatatgggacttgggcgggttacagctgcttttccgaatgcaacatttccaaccggagcaatacatgagtttatgagtgcggcagcagaacatactgccgcggccaccgggtttatcggtggtttattaaatgcgttaatgcagggcggcggcgcctgtatatggatcagcacctgccgcacgctttttcctcctgccctgaaaacctttggtatcgagcctgaacggatcatctttgtagacctgaaacgggagaaggatgtactctgggcaatggaagaagcattgaagtgtgaaggactcgccgcagttatcggggaagtaagagatatcagttttaccgcctcccgccgcctgcaactcgcagtagaacaaagcagggtaacagggtttattattcgccgggaatccactgctgttaataccactgcctgtgtttcccgctggcgcatcacaccattagccagcgaaccggaagatgggttgcctggtgttggctatccccgctggaatgttgaactgctgaagatccggaatggtaagcctggcacctggcaaatagaatggtctgccggcaggttcaggttgatggatgagcaattgtcttccgcaccaccggaactgatccgcaaaatcgggtagtatggccaggcgttttgtttccatatggtttcctcatctgatgaccgattggttaatccgttgccgcccggcgttgcaacaggaagcgtttgtgctggctactcccgatcatggccggatgattgtaacagcagccagcagagccgcgcagttgcagggcatcacaaagggaatggccgtggcggatgcacgcgcgctcatcggcacactggaggtaattgatgacaagcccgggcaatcgaaccgcatattaaacgcactaggggaatgggctatccgctttacacctgtaaccgcaacagatccccccgatggcctgctgctggaagttaccggctgtgcacacctttggggcagcgaagaattatatctgaaagatatagtgaccaaacttacgcatattggataccaggtgcgtgcaggcatggccgatacgattggcgcagcatgggccatgccacggtttagtcaaacactggctgtgattcctgccggtgagcagtctgctgcattaatggacatgcctccggctgcattacgactggaacccgctatctgcgaaaggttaatgaaattaggcctgcgcgaggcaggaagctttataggaatgcccagaacagtgctccgccggcgctttggccaggagctgctactccggcttgatcagttcaccggacaggaagatgaagtaattcagcccctgcagccggttgaaccctaccaggaacggctgccatgcctggagcctattgtaacaggtaccggtattgaaattgcgctcaggcgattgctggaagccctttgccaccgcctttcccaggaagaaaaaggtctccggaacgctgtgctgaaatgctataaggtagacggggccattgaacaattggagatcggcaccgggcatccatcacacaatatcaaccacctgttcaaattgtttgaggcgaaaataccaacgatcaaaccagacctggggattgaattatttgtactggaagcgcctaaagtggaagaggtgcggcccttgcaggaaacattctggaatgctgcagggggactggaagatgtgagtatcgcggagctggtcgaccggctggaaggtaaggctggcaagggaactgttcaccgctatctgcctgctgaacatcattggccggagtggtccgttaaacccgttaccagtcttattgaaaaaacagctacttcatggaaaacagacaggccccgtcccattcaactgctttccaaacctgaaccgatagaagtagcggcgcccatacccgattatccaccgatgcatttccgttataaaggaaaagtacataaagtaaagaaagcggatggccctgaacggattgaaagtgaatggtggctgcaacaaggacagcaccgggattattatgtagtggaagatgatgctggcagccgctactggttgttcaggctggggcattataccggtgataaaccccatgcctggtttattcatggtttttttgcgtgagaaaaaagaggagatatgagctacacagaattacaggtcactagcaactttagctttttaagaggcgcgtcacacccgggagaactggtagaacaggctgcagcactgggttataaagaaatagcgattacagaccgaaatagtcttgctggtattgttcgcggacatgcagctgcaaaaaccagcggtatacgcatcatacccgcctgccggatcgatctgctggacggaccttccttacttgcttatcccactgatacacaggcatacggacgcctttctgcattgctcaccaaaggcaatctgagagcagaaaaaggacaatgtcacttatacaaaacagatgtatttgaacatgccgccggtatgaaatttattgcattatcacccgcatccctgaattcaaggtttgaatttgatgacgccttcagcgtagctatgaaagagtaccgggaggcactgggaacaaacctctatcttgctgccacccgctcttatcagggagatgattttaaaaagctacaccgtctttcacagttatcttctcaatataatattcctttagtagctaccggcgatgtacattatcatatccccgaacgtcggcagctgcaggatattgtaacctgtatcagggagaaatgtaccatttataccgcgggttatcgtttgcatgaaaacgcagaaagatacttaaagccacaacaggaaatgttacgcctcttccggcaatatcctgatgcgatcctgcgtacaaaagagattgcagaaagctgttgtttttctcttgatacacttaaatatgtatacccggaagaaattaccagcaatggccgcacaccactggaagaacttacacatttagcatgggaaggcgccagggagtacttcggagatgatatccctgaaaaaattactactgcgattcactatgaactctcttttataaaagagatgaattacgcatcttatttcctcaccgtatatgacatcgtccgttttgcgaggcagcagggaattctttgccagggccgcggttcagcagcaaattccacggtttgttattgcctgggcattactgctgtagatcctacaaaaattgacctgctgtttgaaaggtttatttcctccgcccgtaacgagccccctgatattgatgtggatttcgaacatgaacgcagggaagaagtgattcaatacatttatgaaaagtatggtcgccaccgcgccgccattgtagccactgttacccaacaaaggcaaaagggcgctatccgcgatgtaggaaaagcaatgggcttgtctgttgatactatcaatcgtctttctgcttccgtatgggattttaccgccgaatggctggaaggggaaggccttgcagaacagggatttgatcccagtgatgcgcatctgcggaagatgctggaactcacgcaggagttcatcggttttcctcgtcagctggggcagcataccggcggctttgttatcacacaaggcgccctctccgatctgtgtcctattctgaatgcacgcatggaaaacagaacctgtattgaatggaataaagatgatatcgatgttcttggctttcttaagatagatgtgctcgccctcggcatgcttacctgtatccgcaaagccttcgacctggcaaaaacgcatcacaatcgtcctcttaccctggcaagcgtaccgcaggatgatcctgatgtgtatgaaatgatcggccatgccgatactattggtgtattccagatcgaaagccgtgcgcaacaatccatgctaccacggctaaagcccacctgcttttatgacctggttattgaagtagcgattgtaagacctggacccatccagggcgatatggtgcatccttatctgcgccgtcgcaatggagaggaaaagccggattacccctctcctgaactgaaagaaattttaaaaaaaacgttaggcgttcccctgttccaggaacaggcgatgaaaattgctatagtagctgctggctttactccatcggaagcagatgaactccggagaagcatggccactttcaaggcagccggacaggtaagccggttccgggaaaaactggtgaaaggaatggttgcaaaaggatacgaagctgaatttgccctgcgtgtttttaagcagctggaagggtttggaagttatgggtttcccgaaagtcatgccgccagcttcgccttgctggtgtacgtttccagctggctcaaatgtcattacccggatgtttttgcctgcgctttattaaacagtttgcccatgggcttttatcagccggcacaaattgttattgatgcccgtaaacatggtgtggaagtaagaccggcagatgtaaatctttctctctgggataatatactggaagaaaaaacaggtaaattatgcgcactgcgcctcggctttcgccagataaaaggcattggccaggaagatgtacagtcattgattgaccgccgggatacaggctataccaccatccatgcactgcgggatgtaggtgttacactgatcacgctggagaaactggcagatgcagatgccttcaggtcgatgggacttgaccgccgtcaggcgctctgggaggtctccgcacttcacgaccgacctgttggtattttcacaggccagccatctgaaagcgctgcagaaacccaggtacagctccctgaaatgacagtatcagaacatgtagtacacgattacagcgccaccaccttatctttaaaagcacatcctgtaagctttgtccgggaaaaattacagctgctgcatatcgtgtcttcaaaagaactggatggcgtcaagaatggcgcagcagtgaaggtagcgggtcttgtactggtacgccaacgaccgggcaccgctaagggtgtttgctttatcactatcgaagatgaaacgggttgcagtaacctggtggtctttcaacaactgtttgataagtatcgtaaagaaatcctgcaggctaggttgctgatggtggaaggtaccctgcaacgcgaaggcgaggtggttcacattattgtatcctgttgttacgatttgtctaaattcttgcgtcagctacttccttcaaaaacaacaactccgctaatgcaaccaccatcaaaaacggatgaaatatccgcgacgttattttctgaagccaggaattttaaatagatgcttataccccttccacacccagcctgtgccggaatattccgcacgggtcccactttccttttacacgctgcagccgctcataattatcctggtagtaaaacatatgccacggcacacctgatttattaaattgttcatccgccatatcagcatcgggatgggcaatcaaacatccgcctgtttgctccccgggtacaggtgctccgcctgttgctgcaaacagctcctgataaatattacgggtccatgcaacagacttcgcttcatctgccgcatctaaccagccggatgtacaggcagtggctaaaatcgagtcccgctgtgggaatgcggtagcatccgctgctacagcattcatcttgccaccaagaaaagcgacgccaacagaacctcccggcacatcattatgctccgtcagatgccggtatatggttccgatttgtgcggctgtatagggtgcacgtaacaaggcatcttttactttgaaagcaacccgcatgtctatgaaaatatccggaaaaggctgtaacgcaaattccacccaacgcatcggttttcgtatagctcttcctgttatacccatgcctgcggaaactgcggctgcaaattcttctgctatttcttccggacaatcggataacacggccttcaacataattttaccagtcaccttattggaaaggtaaagcgtggcaaacagcctgccggcttccgtgtctgtactgctgtgcatcttaccccactctccgaaattgtccagcaattgtttaaatacccgctcatctatctgatcccagtcccattccatctccattgtttccagtacttccggcgacttgggtagtaacagggaaggatcacgcgctgttacaccgggtgcccggaaccaataacgggtaacaatcccgaaattgccggtaccacctcctgtatgcgcccaccagagttcacggttactatctgtttcttcccttgtagcaatcaccttttccacctgccgcgcattatttacccaaagcacttctactgcatacaggtaatcggctcccagcccatgatgacgatgcagaaaaccaaaagcccctccggatatatgccctcctatcccgatggccggatgctgtccggccgggagtaaaacaccccactcgcggtccagtgtttcaaacacctctcccaatgttgcacctgccatcacctcaatcgcattcattccttcatcatagcggatcccctttatgttggaaatatcaatcactatttctacagcaggatcacccacaaaattttcaagacagtggccgccgccgcgtaccactacccgtttgctattgtccactgcatattgcagcgcgtctttcagttcatcgacagtagttacaggaatgatcccggaaggatgccccttccatctcaggttcgcaccacgatcgttccactgatcatatgctgcatctgccggagtgataatactaaaattcatattgacggctttaaggtgaaagtgaaggtaagggtgcaggacatcccaaatataatagtaaaaagcggtagcaaacaagcgctattttttatttaccggcatcattttatatacctgcaccaaggcggaactatcggtgctgagcgtatctattttgctgccattccaggttaaatgatagtaatcataggattctacggcaacggtatcttcaggaaccccatactgactggagctaaaattttccaggatcgcctgccagccattgtccggagaatgatacagccaggacttttttatcagcacatcaccgggcgtcgccaaattcttctgccagctcagtttcaaaggtgatggttttggttttcttatggtaagcaaacagtttaacggaagaagattcgtattcagaaggagacctggtaaccaggccaattgtattggcatccaggttgaatttatagcaggcgtaaaaaagataatcttcattatacctgcgatcgctcagcaacggctgtagctggctatcgatggcagtacctttaaaatgccaggtgtcaggatcaccaaaagcgccgggtaaaatttccagggtgtcctgttcaaatgctttgtaaagatggattaaagagtctatatcagaagggatggtatcatctgcgatcgtaaccgttgtattatgttggcgggcgctatatatacaggctgaaaagaacagcaacagcagaaaaggcaagtatttcatgcccaaatataaagaagaccccccggaaaatccaggaggccgttcttattattacaaatccacgttaattaactgattaccattatcaaaggttgcctgctgtacagtgcaacgctctgcgggaatcgaggatccttgcggatcaaagcgtgatataggtgaaaggaaagaataaccagttgacactaacgatagcggactaccattaacggttatacttttttggtccccaaatccgtggagtaataatttaatgtggtgaaatttcgatgcataattgccacttactttttccaggataatttttttatccgcgggatgataagcgatagtccgttgataatacactcctttctcgttatcaaaagtttctccgtcatcttcataataaacaaaggtattttgtttatcacctttgtagatgtgcaggaaaagcgtatctgacggcttttcggaagtattttgtatcaacgattgcatcgggatgatactgctttcttttacatataccggcagggattttatattcagcggcgtaataacttcctgcttcccggcggtgatggtgtcgttataaaggttataccattttccctccgggaaatagatggagccgaattcttttgtgctttcaaagggcgctaccataaaggcattcccgtacccatactggttctggaaacgggtgtcgtaaacattggcgtcaaaggtattggtgagcgccagcgtacgcataacgggcatgccggtacgagttgcttcaaacatggaactgtagaggtagggaagcaagcggtaacgcaggtttacataattgcgggaaatttccagcacctcttcgccatatgcccatggttcggacgacttggtatttacccctgtgtggttacggtagtaaggaatgaaggcgccgatctgcatccagcgggcatacagactcacggtagcattgccggtaaaaccgcctatgtccatacctgagaaaggcatgccgctaacacccaaactgttcatcaggcgaactcccagcaacatatgatcttcttccgcgcggttgtcgccggtccagatagcactgtagcgctgcgagcctgcgtaagcggccctggttaacaggaacgggcgtttctttaattcctccctggagccttcatagctggcgcgtaccatttcaagaccatatacattgtgcgcctgctggtgggttaccggatgcccctcgtaatcaaagatcacgttgttaggcatcttttggccccaggtggcaatttcattcatgtcgttccatataccacgcacaccgtcacgcatatacgattttatctggcctttccaccagtcgcggccctttccactggtaaagtccgggaagtggcaccagccgggccatacctgcccggtataattttgtccgtcgctatatttgataaagatgttttctttttttccgctctcgtaagcagcataaccttcttctacttttatgcctggatctacaattacggtgagtttaaatcccatatcattcagctgtttgctgagttgttggggattggggaaacggtttttgttccaggtaaacagtttgtaggcgtccatgtaatggatgtcgagggtaataccatctgccgggatttttttctcccgcagggtttgcgcaatccgtaatacttcggtgtcggggtagtaactgtagcggttctgctggtatccgaggctccacagcggcggcatgggcatgcggccggtaagattggtataagacgtaatgatatccgccatttgtgggtgatagatgaaatagtaattcatctctcctccccttgcgccaaaagaagaaaagcggttgttgctggcgccgaagttaaaatcgctctggaaggtattgtcaaagaaaataccgtaattgatatgatgatgtatccccacgtaaaaagggatggtggcgtatatgggatcctggttggcagcatagccaaacttatcagagttccagttcgtatagccttctcctttacggtcgaggttaccggttttttcgccaagaccaataaaccgttccccttcctgcattttcttgtaggtagttacttcatcgccgatccaggaagtagtcaatccttcttcatcctcattaatcacttctcccgaaggggtaagaaagcggatggcaaaaggatttttagaaatacgcagttgaagggaatccgtggttacattgatttcattgttgttttgtgtagtctgcaaccgggtgctggttggtttggcaattaccgcataagaaaaatctgccgcaagcggatgctgatccattcttacacggatcacagaagcactgtacacggtgatttccgcgaacgcgttttccgcactgatttttatctgttgccctgagatgctgaccgtatttattttaccgatcttttttacctggttttgtgcctgggccgacaggcaggaaagcagtaaaatccatcctgagcgccttagcagagcttttgtatacataagaataattgaattgctacgcaaaaaactcccctgtcgcattagctatgtaatgcgtagcaggtataaaatatatttgggagaaggatttgctgcggtggcagggccggatagccctgcccgcaacaaaagaataattatcagtaacccgggttttgtaccaggtttggatttacagcaagatcactggttggaatcgggaacagcaggtattttggatcgcttacagttttcagctgccatgcgtccaggtatttaccaaagcggatcagatccattcttctccagccttcccaatataattcacggcctctttcagcaagcatcttggtgagatcaatgctggtgaatagcgtagcgccgcgtttcgaacgcaggtcatttacaatcaggagtgctgccgcggtattgccggttctgatcagcgcttcagctttcatcagcaccgcatctgcataacggaaaaatacgaagtcgttggtggcattgctaccgctggaccccatgtcaggaggatatttcaccaccctgataccagacatttccacttgtgtgccggtggctctcaattccacttcgcgggtgaagataagcgggcggttgcttctatccaggatcttcttaccggtctgatcatattgctggcccaaaaggaaacctactttcaaaccggaaacatttgtaacgcctgcatagtcgccgcctctgcgggtatccgttgcttcgaatgaatcgtagaaatcagataaagtggtaaacccattccatccgctggggttctggctgtagtgcagggtacacatccaacggcagtaaacgttattgccgctacggttattactaaccccggggccattcagttgggtaaagatattttcggtggattttgcatcgttatcccttgcaaaggtgtcgaaatatttcgcctggagggtataaccgctgcctgttatctgatcggccagggcaatcaccttttgcatatctgccgcatcgaaggtgggtgcttttctgttcaggaaagcgcccttattcagatatatcttcatcagcaggaaacgggccgcatcctggctggctacataagcatccttggctgtaaccctgtctggcaggttgggcagaatagcattcaattcagagacaatgaagtccaatccttcggcagccttgaaaacttttggtggcttcagcaggttttcgcccggctcgcgatagggtacctgaccgtacaggtcaatcaccgcaaacattgagaaggcacgcagaaaacgtgcttctgcttcctgtcttggtgaaggatggaaattcaatacattggtagcgctgaactgttccagcaacagggcgctgaaggtattctgaatatgtgagtgatccggtgtccactggtgttggtgaagagcgcgccatacaccgttatcatcccagtcgccgccacgtgtgggtccgagcgcttcatcggtactgatttcagacatgccccatgtctgcgaaaaatcctggtaggcattctgcaggttatcgtaagcagatcccagcagctgggatgctttgatcagtgaatctgcctgctgctgattcaggttgctccccaggtcttcatttaagctacaagccgtgaaaccaatggcactggctattactatggctgttttaattatatgttgagtcgtcattgtggtctttttttagaagtagattataaggtaaactgtacaccaagcataaaggttcttgcagttgggtatggagagtattctataccaaatgaacttacaccatttatgtttttatcggtatttacttccggatcaaatccagtatactttgtaattacaaacaggttctgaccagtcagggatacggcagcagctttgaaaaccttacccacaggacctaggttataggagatggtcaggttatccagtttcaggaagttaccgttttccaggtagcgggaagaagcggcgggagagttcgtttgtgcttcgccgttaccaaccagtgctttggcgatgttcctggagccaaggttaccgatgggtaataccgtgttggcagtgttgttatacacctggaaaccaaaggcgccgtgagagctggcagaaaggctccattttttataggctacttctgtgttgatacccagtaatactttcggattcgggtttgtcatgtaataaagggtgttgccgttatcggaataaatgctcacccctttatcgtcgaagccttcaaatctgcggagatagaatgtatttaacgggtagccgttcgccaggcgctgtgaggttacaccggatacgccttgtccgtcgatggaaccggtattaaccgtaggaccggaataaccagacatttcatttttcagccaggtaccgtttacacccaggttccacagccagtttttagactggatgatatttcctttaagagacagttccacacccgtattcattactttacctggtaagttgatccagtaactggaggcaggcgccggttgaatagccgggaagctgaacaacaggttggtggtgtttttgaggaagtaatccacagtaccgcttatccggcctttgaggaatccgaaatcaacaccaacgttcagttgtttggattcttcccatttcaggtctggatttggtacgttgatgagactggctttgccgccggtggttaaaccgtactgagcttgtgccgcaccggcaggaaattcctggttaccagtgatgccataaccggctcttaatcccaggttgctgaagaaggtgttatccttcatgaagccttcgttggaaatattccatttggctgcaaaggaagggaagtaaccataacggttgttggagccaaacttgctggaaccatctgccctcattgtagcagtgaggagatatttatcttttgcatttatagttaccctgccaaagaaagactgcagctctgagctaggattacggaaagagttgatgttggtattcacctgttcaggtgtctggaggatatccgtgtaatctaccgcgttagtaggaaagcctcttgcgccgatacctacaccggagtaagcaaatttctgatattcatagcccaccattgcgccgagattccagccaccggaaaactctttggtgtagttcagggtattattgaataactgggtagtcagctctgcggtattataagcggcaataccttctcccagtacctggtcgatgttaatggaagaatccagggaagcccttctttgaccaacctggtggtttacgctgtacatcatgcggtattcccagttgtcgttgaatttgaagtacggggaaatacttgccaggatataactgatgttggctttatcgttataaccctgcgacatgttcattgggttgatcgcctggtttttagcgaggatgttcagtgatccgtcgggtttagtcaatggaactgttgggttccattgtaatgcctgaccgatcagacttccggtgaaaccggcgttattggaaataggcgccaattgttcactggtttgtgccgccatgatgccgtagtcaattcccaattgtttgctttccaggaatttgttctggccactgagggaagcggtgtatttcttcatgcctgttttcttcacaataccctgttggtcctgtaagccaaaggatgccctgtagcggctggtttcacttccaccgctcattgctacctgtacattttgggtaacgcctgttctgaggatagagccaagtccgtcggagctaccgccgccgtcgccggtaagattgtattcttttaaggcagcacggtattcatctgcattgagtacatcaagctttctcatgatgttgctcatccctacagagtagtttacgtctactaccgtaggaccggttactcctttttttgtattgataatgattacgccgtttgaaccacgggaaccatatatcgcggtggcagaagcatctttcaatacttccatggtcgcaatatcattactgttgataaagttgagcgggttggcgtccggtgtttgtcccaatcctgtgaggttcagggaagggcgggccacacggccatccaggggtactccatccaccacataaagcggctggttaccagtacggacagaagatacgcccctgatccttaccgtggcggaggcgccgggagcaccgttattattcagtatcatcaatccggatactttaccctggatcagctgatcgggagcggaggtgatacccttattaaaatcagcggctttcacctgggctatagcgccggtaatatcctttttacgggaggtaccatagcctactaccaccacatcagtgagggttgtattttcctgtgccagctgtacgtttatagttgttttaccagcaatgctcacttcctgggtggcatatcctataaaagtgatgatcagcgcggaggcttcaggtggtgcagttactttaaaaaccccatcggcatcggcggatgttccgcttttggtaccttttatctgaacagtagcgcctgggatagcaacgccgttcctgtcagtgaccttaccggtaatggtcttgttctgtgcacctactataccttgtattgctaaaagcaatgagcacaaaaaaagattcttgatggatcttgttttaaacataaagtggattttttgagcagttatgtaatactgcttccgtggattaaatgtttttcattaaattttaataatggaaataaggcgttgtttgccggggatgcccgcaatttgtcaacgtggataatgtttgttttttttaaatcgaccttagccgttctgtcttctttagtggtttttagttctcctgttagaatttagagttttggtattatcattctactgattcaaagtaaaaaatcaatcagcagggtaacaagttttacagttaaaatatagaaaataaagccgaataaaccaaaattatctcacaaataattttgataatcagacggttatgattatatataaataattaatatattaatggcatgagacggtttttcccgctttttacagggctttaatgctcataatatgggtttcgaactcttcgcttggaataagcgcgcgctttttgatcctggttttataggcataaatagtgttcacagaatactccaggatacgggcaattttttcgttgtcgttgataccgatacggatcagcgcgaaaatccggatgtctgtattcagcagttcgttttctttcaggatcacctgattctccttgtcaaaaagcgcgttgaactcagccacaaaatgtgggaatattttaaggaatacccggtcgaagctggtaaatagttcttctctctcctggcggatattgatattatttacaaggaaccttagctctgaaggcttattatccgttaatttttgctcaagattctgttttagcttttctattttaccgatgtaggaagcattgatgttaaaacaataccccacgtactcctctttaattttattggcttcgagcaactggttgttgatttcctgttgtttaagattggctgcggtaataatgcgctgcgcggtttttaatttttgtacctgccggaacaccgtaatggccagtatcaccaacgcaaccagcaacagggtcacaatagcggcatagatcagcagtgacttggttctttcttctgctgtaatgatccgttcatgctcaattattggtaaaatactacttaccattacctttctttgccttgcaccgtaaaacaccgcttccgaaatagcccgctcaatacaatgagatgcattctttacatcacctctttcaaaaagcagggttgccaggctgtaggcggccatcgtttctttggtagaagtctgcagatccgcaatggccgacctggccatcaggctgatggcggtatccttattaccggctgcatcataaatagagcccagggtgcaggccaatatagccagttgccgccctgaaataccaggctggttcagatccgggaaaatggccagcgctgccggaatgttacccagcttgaatagctgcaatcctttattgtatcggtactcaacagagttgggacgcatcaggtggagggcagaatccacaaatgtactggccactttaatataggcgggggtataatacttatcctggttatagtctgccaggtcgaaatacaaccggctcttcatcaagaaaaactccactcggatactatccggagcgccggtagggtcaatggtattaataaaagcagcagtttctgtaaacatgcccgatgacaataaaacatatcccagcttaatccgggcatcggttaacaataccggatcatgcaactggccggccaatacctgcagctgctgggcatatgtaaatgcggaatcgaaattaaataccttgtaagcattatataattgccggcaaataaggtactggcgggcaggatcattgcctgccacctgccgggtaagttttatgctgtcaattccacggagtttaatggaatcataagcagccgatttcgccatcaccttgttgagctccttcagaagactgtctaccggtgctttggcataggtatgtatagagaagaataaacataaaatcagatagccccgaattcgattcataataagttagaatgataaaaggtcacaggtcaccgctaaatttaagcgacttttttgatataatgcggggagccggtttattttaaaccggctccccatcttccttctatcttcctttaatattaaagtacctttttcagggtataattaaggctggtttgtatagttttctggtcggcacccagtaacaacagctcattttcattcacctgctggtaatagcgctggaggtttctgtctttattgggattgaggtgaatcacggtagctcccgggtcaacagcggtgccatgcacaatggtataaatgccttcactggcaaaggtctggttcttccccttgtaggtctctcttaatgtgaaatgatcatccggttgcctttggagggtcagctccgtaacaatgccctcacaatcagcacagggcaacattcctgaataagtaacgccggaggcagtgtctgaaggagagtttactgctatactatccggctggccggttttggcgccggaatgctgacaggcagccaggactaccagcagcaacaatagtggcaagtgtttcatatcgggggttttctgattataaacaaccggtggtcattattgttttacgggataacttcgaacaggaaaaactggttttcttctttatcagaaaaattattatctgctacgaacaccaggctccgatgcccgttaggcaaaacaggaccataagtaacgccttcaatgttatctatatatttcccaaggcgcacaaaatccagcagtaacgttttggccgctggcttaaaacgggtatccgcctgcagggaattaataccgctgatatcagtagcattgctaagatcggtgataaacactttaatggtacaatcctttacgccactggaaaatgacctttcaatggttaatattttattattgtccaacaccatgatatctgaaatgccattcactttgaacgcattttcaggaatggcgggaaacgccaccggctctagtttatacgcatattgcgccaccggttgccgggtgttgttgtcaaatttaaggatacgggtataggcgccctgccctacttcggctctcggaccatcttcataacggggttcttccaggctcacatacaggtatttataaccgggggtaaatcccagtccttcaaatacaccattgcggcgtggcccgttctctgtggcctgcatcctgaattgcgatggcagcgcgaatgaatccaggtattgcccgttcatgcggatctcataaatacccggattggtaagaatggtatctttttcgtttacaatgcgttcgccttcgctgctccacaccagccgttgctttttactattataccgcatcgcttccgggtcgggcgtaagcgagggattggttttggtatcgggataaggctgtccgttgggttgcaacaaaggagtaacacctgtgaactttatactgtcgaatgatttatcggaaaagtaaagccgggcggtataaaaacgcgccgggttcagtgcggagcggtcatcacaaataagataatattgcccggtagaaggggcgtaatcaataccggataaaccaccggttactgtaccattgaaaggaagattatagggaacaatatattcaccgataaattttagctggccgatggtattggcagcggtagccgctttacgggtggtgttgcagctgaagatgcccgccagtacagggaggatcagaaaaagcaggtattttttcatgacggcaagttaggaaatctcctgcattcagatcgccgcgctgcatgaaggatttgttatgcgcacggaaaggccggcccgaaagagccagccttttctacatctgaccaactatatagcgtacttaagattttataaacaaagaagcaatgggtaatacctgcgccatcgacaatggttcatcaaatgcttctgatgcgctgttagccccgatgttaccacccaatgcggcaatgtccacccctgcctgcatggttaactcctctcctgcataggaaggatttaccgcggtagtagcgatgccgctttggttcagggtaatccagggtttaagtgcaggggaagcacccagcgtacccaatgccctgcgcatcatccggatatgggctgcatggcgtgcttccacagaatgtatattcagtgccgccgtgagcaccgtattatttcccgataaatttcctgcctggcctttataggcgcgaacgccggtatcttcaaatgtttgtgcgatagccaggaagaaattgtaatcggtaaaaacggccgggaaggtgccaccggcggtgaagtcgaacgcaggaccggcaggcgcgccacccatgttactgagcacacttttcaaaaaaataacgtgagcggtttcatggttcctgatggtagtgagggcggcagttgcagccgcagtaggtatcaggccgggcgtggctaccccttttacataaaaagcctcttcaagatattccagtgtaagggcgtatttcaatacatctgctaccgaagtaccggtagattgcgcatatgttttattaaacatgctgcccagtgcaaacggaatagctgcgagtgcaattttaccgctgatattggtaaattgtttcatggcattgcggcgggaatccagccggtcgtatacatcaggatcgattttttcgatttccttgaaaatattgaacaggtccatataatcagattttaaacagataaaataataatagcagttgctttacttaggtaatgtgtttgtattgatcctggttttgatatacgttttggcaatgttgaaaacgtctatcggcgtcctgcttttatccagtccgtttgcatctattacatcgccggcagcaaatgatcccggctcaatcaggtcccggatataggctgcatgacgtgcttctaccgacactattttgcctgcgagaccgagatataccaatcctgttgaagaagatgaaatatactgccctgcgccgttgtaggcggaaacacccaggtcttcaaatgctttagccgttgccagtacgctggcccttttggtgaagtcaatggaactgaagtccacctccaggccagcgatggcattggttgataaagcggttttgaaaaactcgcgatgccctatttcatgatttctgatatctttaaaaaaatcaagttccgtgtcggaaatacctgcgtagggtgtaagcaccacctgcgaatagaaggccgcctccagctgctcaagggcataagcataatttagtacagctacgtcacctgaacccaggctcacaccggagccccccatattgttatcatcttttttattacagctggcggcaatggcagcagcagtaacaaatgcagagcccatgccgaggtatttcagaaagttgcggcgctgcagattaggcataacttccttaccctcctcctgagaggggttcttgagaatgtacataagagaaagttttaggtgaatagataatacatgatcacaatgccctgttgcttaacagtggcgggttttaaagatgcctggaggtatgctcgcacaggtatctgacgaccatatacggggtgcgacaaaaagcggttttaaaaaaggtaaaatattttcagcacgacggaaatggaagggataacaaaaaaatccccgtctaattggtaacgaatcaccaattagacagggaagaataaagtgcagcgtaatcctataaggccctgcctctgattatatttacaaggatggcaataatagccagcacaagtaaggcgtgtattaaaccaccggctgaataaacaaagaatccaagtatccatcctataatgagaattacggcaattaaataaagaaggctgttcatgtcttaaggatttggttcgcttattatactagaaaatttatgccaataagataatcgctttgtatacagctatttcccattgctgacaccgctccattgtggaaccttctccaccatccgagaaaaaaaaggacgggaaatagcaggctctccatctggaaataccttgtgctaaagggttttatagtatggacacatttttggaaataaaatggttatattataagactatttttttaaccataaatttttgatcatgttacaagaggaaaagttggtcacacttttaagcgatctcgtaaaaatcaacaatgaccggatagaaggatataagcaagcgcaggacgccagtgatgacgcagatgtgaaggcgttatttcaacatatgatcaacgacagtttaaaatatgtagcagaactaaacctgttattgagagcgcagggcgcagatgcggaaactgatactactgttagcgggaaactataccgcacatggatggccataaaaactacgtttacaggaaaggaccggtattctcttttttcctcctgtgaatatggggaagatgccgtacagcgtgcctacgccgatgccctcagtatggatgtagccatgccctatagtatgagggaaatcattggcaatcaacaggcaaacctcaaggaagcacacgatactattaagagctaccgcgatgtagtaagtcaatagcatgctgtgcagacagctaccgcctgttctttttgttcaaatcaacccattaagcggttgttcaggatagccatattacttttagattcatgaaattccaatcatacttatattaataagtaatatggcaactacgggattttcggtacagggctgcttcctcatcgtttgaagcagccctttttttatattggatatgggagattttttgtgaaataagcccctaaaaacagcgaacaggaaccggttctgttcaatggcagtattgctgttcattttgttcagtttagccaggggcttttggaattcaaagacctatactatctttgaaatgattgagagaagtatctcttgtattacttttaacctccccatgaaaaacaacaacaataactaccaggtggtctaaccaaccaccttttttatttcccctgagaaggcaggatcccaatctttccaaaccggttcaaatccttgttcccgtagcataccggcaatagtggcggcgctccggtcgtcagatatttcaaattgctccagtgactgctgatccaccacatagccaccaggattggtttttgacgcagcactcatggctgtcacgcccagatgcacaatgttattccggaatttttcctcttcccgggtagaaatactaagctccacttcctggttgaagagccggtaggcgcagatcagctgtaccaactcccggtcgttcattactactttcggtgttaacccgcctgaaaatggccgcagccgcgggaaggagatactgtattttgtttgccagtattttttctcgaggtaggccaggtgcagcgcggtaaagaaactgtcggtgcgccagtcctccagccctatcagcaccccaagccccattttatgaatgccggcacgtcccagccggtcgggcgtttccaggcgatagtcgaagttcgactttcgtcctttggggtgatgttttttatagtcgtcctggtggtacgtttcctggtacaccaacacagcatgcaatcccagttccgcgagttcccggtaatcctgttcgtccatcggctgcacttccatcgaaatattggcaaaatgcggccggagcagttgcaaggtctttttaaaatagtcggtgcttaccagctggttagcttctcccgttaccagcaaaacatgctcaaaccccatctctttgatagcagctgtttccagcaggatttccgcagggctgagggtttttcgccttatcttgttatcgagactaaatccgcaataggtgcagatgttctggcattcgttcgacaaatacatcgggatatacaactgcatagtgttcccaaaccgctgacgggtgagcgcctgactgatagccgccatttgggagaggtaaggcgccgccgccggggaaataagtgccgcaaaatcttccagtgaacggcgctggttatgcagggcctgttccacatccctggctgttttagcatagatgccggcctttacctcgttccagtcatactgatcaaatatgcttttaaacatacggaaggattaataagatgataaaataattatgcttcatcaagaaatgcgatcaacggactggaagctaccgcgtgctggctgctggcaggtaaaccagcttcgtaggccatgcgccccgcttccactcctgctttaaatgcggcggccatctccaccgggttacgggccacggctatcgcggtgtttaccagcacagcgctggcgcccatttccattgcctgcacggcatgggaaggactgccaatacctgcatccacaattaccggtatattactttgtgcaataatgatttccaggaaatcgaaggttttcaatcccttattgctgccaataggagcgccaagcggcatcaccgccgcagtgcccacatcttccagccgcttgcataataccgggtcggcatgcacataaggaagcactacgaaacccagtttcaccagctcttccgccgccagtaatgtttctatcgggtcgggcatgaggtagcggggatcaggatggatttccagctttatccagttggtttccaacgcttcacgggctaactgtgccgcatatacggcttctttggcagtacgcacgccggaagtatttggaagcaggtgtattcttgaatgcgccaggtgccgcagcatatcatctgccttattatccatttccacccgttttagcgccacggtgaccagctcactgccagaggccagcagcgcactttccatcacctggggagaagaaaatttaccggtaccggtaaacaaacgggaatgaaattccctgccggcaataattaatggctccatgtggataattgttttaactgttgatgaatctggttcacaacggcccgtttgtctgttgcatgtgtaatcagtccgctgacggcaataccgtgaataccggtttccatcaatgccgggatatcttccggcaggataccgccaatggcaataactggaatgcctatatttttttcttttaaagattgcaggatagattgataaccgctgagtcccaatatggggctgagattttgcttggtggtagtgaaccggaacggaccaacacctacgtagttggcgccatcctgcacatgctgcaggatatcttcaagggtattagccgtgccgccaacaatcatgttgcagccggtaatagcacgggccgcggcaacagtcatatccagtttgcctatgtgtacgcccgctgcatttaccgctaccgcgatctccggatagtcgttgataatgagagacgcctggtaacgatcgcagattttttttgccagctccgccagcggcaatacggtggccggtgattcgtttttgatacgaagctggatccatttgcagccggcgtcacaggcggcgagtatattatcggtatgcgatggttgcgatatgtaatgtaagttgctgatcatatgtgatggtatcctgttaatgatgaatgactggccaataaattttccgtatatactttaccgttagcacatgcttccggtagtgaaacgccgcgtgccaaaccagcagtgatggcggccgacagcacacagcccgaaccatgttttggaaatacttctttctgtacaggaggaaaggtatggatcacatcaccggtataaagtatatcgtatcccggtttgtttttatgatgacctccctttagcagtaccgcgcagccggcagataattgccgggcggctgcttctccatccgtaagccctgttaacaacaatgcttcgtcgtaattaggcgttaacaggtaaatttcggccagcagttctttccaggcctgctggtgaatgctgccgtggaaagagaaacccgccgacgcttttaataccgggtccacgatgatacgtataccgggcgataattgttttacctgtcttaccagctccagcaaagactgtatatccggcatgatacctattttgcagtattgcagccgcgtactgcataacaacggttttgcctgcgccagtatatgcgttaccggtatccactccactgatataaattgtgcaggtgtttgcaccgtactggcagtacaaacgcccattccgtttaccatgtgttgttcaaatgttttgatatctgccagtaaacctgcgcccccgctgggatccagaccggcaaagctcatcacgtaaggtcgctcttgttccatagctgttgaatacggcagtaattttccacggcttgcgccggtattttccagatggctcccagcaaagctgcaccatcaaattgccatggttttaataaatgtatattgctgtgatccacgcctcccaaagcaagcacccggcggttgtttttatcaggtaacatcccttgtacccggccatgatagccaggttttgagatactgttaaataccgggctcagtaacaatgtttgaaagcgtttgtccgttagcgttataccttccggcgaatgaatacctgtgctgttttccttaaaattttccggagatagataactggttagtggttccgtttcaccggcacctggagccgttttttcgttactggtcgcagcatctgataaaaaccgttgtatcccctctctgctccagtgtacgcccgcgaggctatacctggcagcgagcgcaccatgatcactgataagtacgcggttgtaatactccggcggcagcttgtccagtaaagcggcatactgcccggctgaccagccaggctttcttaacagtacccgctctactcccgcagttaataaggccgcaaggatatccacttcttcgtgtatacgttcgggtgatgtgatgatccagatcaaatatttgtgtttaaatgctgtatctacaggtaaatttcgccgccctgttctgcaaaagctgcggccttttccttcatgccggcagtcatggcgtcctcttcttccaaacctttttgcgcggcgaagtcacgtacttcctgcgtgattttcatggagcagaagttgggaccgcacatagaacagaaatgagccaccttcgcgccgtctgcaggcagtgtttcgtcgtgatacgagcgggctgtttccggatccagggccaggttgaactggtcttcccagcggaattcaaagcgggccttgctgagtgcattgtccctgtgttgcgcacccgggtggcctttcgccaggtcggcagcatgcgcagcgatcttataggtgatcaccccctgccgtacatcttctttatttggtaacccaagatgttcctttggtgttacataacataacatggcacagccaaaccagcctatcatggcggcgcctattcctgaagtgatatgatcgtagccaggtgcgatgtcggtggttaaagggccaagtgtgtagaaaggcgcttcatgacagtgctccagttgcttatccatgttggttttgatgaggtgcatgggtacgtggcccggaccttcaatcattacctgtactgagtgtttccatgctattttggtaagttcccccagggtttcaagttctgcaaactgcgcggcatcattggcatcggcaatactgcccgggcgtaatccatcgcccagggaaaatgaaacgtcgtatgccttcatgatttcgcaaatctcttcgaaatgtgtgtacaggaaattttccttgtgatgcgccaggcaccatttagccatgatggagcctccgcgggaaacaatgccggttacgcgtttggctgttaacggtatatatctcagcagcacgccggcatggatggtgaagtagtccacaccttgttctgcctgttcaatcaatgtgtcgcggaaaatttcccatgtaagggcttccgcttttccgttcactttttccagtgcctggtaaataggtacggtgccaatgggcacgggcgaattacggataatccattccctggtttcgtggatatttttgccggtgctgaggtccatgatggtatctgcgccccaacggcaggaccatactgctttttccacttcttcttctatactggaagtaaccgcggagttgccgatgttggcatttatttttacaagaaaattgcggccaatgatcatgggttcactttccgggtggttaatattagcggggatgatggccctgccggcggcaatttcctggcgtacaaattcaggggtgatgaactttacaggtgtgttggcgccaaagctctggcctttatgctggtcccagagggggttgttttgctcaaacagtttgtcggcgcattgattttcccggatagcaatgtattccatttcgggtgtaatgatgccttgttgtgcgtagtacaactgggttacattttgaccgggtttggcgcgcaacggtttatgcgtgtggctcatcaaaggcatcttgcctccttctttcatcagttctcttacaaagggactggtatactccgggagttgctccacgtctttccggctgttgatccatgtttcacggatgcgcggaataccggtggccacatcaatatggatattggggtcggaaaaggcgccgctggtatcgtatacaacaacgggggcgttaggaacggcttctccgttttttccatgaatgcgtgtatccgtgagcgttattttgcgcatggctacttttaccgggtggatcgttccgtccacatatattttttctgaagcaggaaagggtgtgcggctaagtgccacaggctgattatgcatgatgtctggtttttttagagatagaaatgccggtccgtaatgatgcatcacggaaaagactatacgaaaaatgaaatgcagggtttagccgccctgggtagcccggataatagtaatattatcggctgcagatagtggttggttttcccaggaggttttcggtatcacctggttgttgacggccactgcaatgcctttttgagcagagatctgaataaactgtaagagtgcagcgatggttgttcccggctgcaccgcataaagtttattgtttacatgcacttccatgttaattggaatttaagtgaaacaataaactttaaggatgtggaaagatgagaaaggttcagttacttttccctacggcagtatgaactgcttcaggtactgagggtatcatctcagtttatccttcatattggataaacacccctaaagtgtagatgtaaaagtaatggaaatatttaaaaattacattacaaatgatgaattgtgtatttttaaattatggtacgattcagtttaatgtgtttattgatactggcggttgcctgtaaggggagtaagaaggaggcggagcaggaagaattacaggatgacagcagcctggttagtataatcgcagacagcagtaatgccggcattactgacagcattgctgctgttgcggatacgctgcatattgacgcagctaagctcataggaaagtggatacagcccgtagcgggcctggataaggaaacgcagggttttcagcttagaaagaacggaactgccagatccattaacatgtacacactggtatacgaaaaatggttactgacacacgacaccctgctgttgtggaatcattctgaaggtgtaaaagatacctccacgatcgtggatacaactattataaaagaactgtcagacacctcactggtattgtttcctgtaaaagccgccgaaggctacgtggaaaaataccatagaagcaattaattatatagctgccagagtcctaccaggcaggctactaccgccataaatacgccggcagcagcgagctgcatatcgtcaatattttttcttcctatatacagggaaagaagaccaactactatagctactgagcctgcggtaactgcataggaaggcgtgtgtgtactgaaagcgaatgctgccgatagtacaccaatgatgagcgctgatatacaggctgtttttgttaatgctgttgagtgttgcatatattcgaattttaaagaacaggtgaaggaataattatttgcaggtattttatttatgctgactactgatcttttccttcatcacgggattatcgtgttcccagggcacttttaacagggatcctatttcctggtagcgggcgtcctggtattcatccagtccgtatctgatcgccagtgtatccggtacttttataaaagtgccgaagaggcgatcccatatagaaaatatattggcataattagcgtctgtttcgggctggtaatgactatgatgtaccttatgcatatccggtgatacaatgatccagctaagcgcgttatccagccatttgggcagatggatattagcgtgattgaactgcgacattaaggccgatatggtctggtataacataatcatccagaagggcactccgagaatcataatagcggcaaaaagggctattactctccataggctttccaccgggtggtgtctgagggcggtagtggcgtctatctgtgtatctatgtggtgaattttatgaaaatgccacatccaggccgttttatgctgtacccaatgtatgagccaggccccaataaaatccagcagtaataatgccagtatggtgtgtagccacagcggcagttgggtcaggtacaggatgccgaactgctgggcgctggtccaccgggaagcctttacaataagaaatgccagccctgtatttacaatcaccgtggttaatgtaaaaaagagattggtaccggcatggcggtagcggttgctgctaaaacggaaccggggggctatgccctcaatgatccataacaacaatagcccgctcaccaggatagcagtacggtatactgacggaatattttcaaaaaaacttaccatatcatggtaatatatataacggtctttttacgctatgctgtggttctccttaaccaggccaacaaaatctctgcagtggatatgggggatgtgatcttgtaatacgcagtaaacatatatccgttactgttattacccttgcgttactgtcctgaatcctcgggtgtgttccaaccactgattccggagaaaaattacaactatttggggaatataaaaaggcctcttttaggccacaggcaaagaaaaaagcaacctctttgtcagagattgctttatgtatgagtttttagctataagtatttatctttttagcatttagctaacaaccgccgattagttgttcagcatcagcggcattaccagcataaggaggtcctcattctcttctttttcggatggtctgaggatacctgctttggtggcagtggccagatcgatggagatttcatctccttccgctgcattcagcatttcgatgaggaatttcgcattaaaagcaatctgcatatcatcgccggtgtactggcagttcatgcgttcgttaccttcaaaggagaagtccacatcctgggcagacaactggagttcgctgccggtgatgcttaaagctacctggttggtgctcttattagcgaatacccccacacgtttcaaggcgttctggaaatcgctttttaccacggtgaggcggtaaggattatcttttggtattactaccttatagtcagggaaacgggcatcgatgaggcggcagatcatctgtgcgccttcgtgttgcacgaagaagtggttctggctataagctactttaatttcagtttcgttatcaggcagggctgatttcagcaggttcagcggttttttaggcacaatgaaggtgtctgcctgcgggcactttacgtctgttcttacatatttcaccaggcgatgtgcatcggtggcaacaaaagtaagactgtccggagccagctcgaagaatacgcctgtcatagcaggtcgcaggtcatcgttgctcaccgcaaacagggttttattgatggcggtaacaagacctgtagcagccatggtaaaggaggtggtatcatccgcagcgggttctttcgggaagttctccgggttttcccccatcactttatatttaccattgtctgaagtgatttctactgcgtaggagttcaggtcaatgtggaaagtcagtggctggtcgggcagatttttgagggaatccatcaggatttttgccgggatacagatccgaccgctttccttggcttccacctccagcttcacccgcataacagtttccaggtcagttgcaactacagtcagttcgtttttgtcaatcaggaacataaaatcctccagtataggcaatactgtgtttgaattgataaccccgctgatctgttgtaattgttttaataaagtagaggaagaaacaataaatttcatggtttatataagtttgcttatcattttttgttgaagggtaacctttagggcatgccgccctgattttctcctggcacctcacataaaaggtcaaatgtactgtaaacaaagatagaaagttttgtcgttctccctaatttcatcacatcttatacactaagataacgtggttttacacaacgatttgcagtcattcatatatttctttttagtataatactagatagaaagaataaaaataccccttctggttagatgagatgcaataaccagtgccatttattaacggaagtgaaaagaatttacctattcttttaaattatcttcaaatcggttacttttgccgcgctgaaaaattattacaaaccaacaaaaaaaagcaggttatgaaactgtctcatttagccgaaacgttgattggatccgaaatcattaagttagcagctgaaataaaggagaaacaggccaagggtgagaagatatacaacttcacgattggcgattttgacccgaaggtatttcctatcccggttgaatttgaacaggaaatcataacagcctataaggagcacctgaccaattatcctcctgccgatggtatcgcggagttaagacaggcagtaggtggttttatagctgagcgtgagggtctctcctacgatcctgcaaaggaaatcgttatttcctgcggcggtcgtcctatcatttatgctacattcagaaccatcgttgaccgtggcgagaaaatagtatacgccacaccatcatggaataataaccactatacccacttcctggaagcggaacacgtagtgctggaaaccaaggcagaaaacttctttatgcctacggctgctgaactgaaaccgctcctgaaaggtgctaccctgctggcgctctgctctccgcagaacccaaccggtaccgctttcggtaagcaacagctggaagagatatgcgacctggtactggccgaaaacaaaagcagaggcgccgatgaaaagcccctctatgtattgttcgaccagatgtattgggtgctcacctttggtgaaacacaccaccacaacccggttaccctccgcccggaaatgagggattatacgatcttcatcgacggtatgagtaaagctttcgctgctaccggcgtaagagttggctgggcgttaggacccgcacacgtaattggtaaaatgaaatccatcctttcccatgttggcgcctggagcccgatggcagaacaaaaagctgctgcccgctacctggtacagaaagaaaatgtggataaatacctgcaacactttaaaggcgaaatcgaagaaagactggtgaaaatctacgaaggcttcgacaaactgaaaaatgcaggtcataaagtagaagccattgctccccaggctgctatctatctcaccgttaaatttgacctggtaggcaaacaaacggctgatggcactgcgcttgcagatcaggccgctgttacctcttacatcctgaatgaagctaaaatagccctggtgccgttctatgctttcggatccgctaaaaactctccatggtaccgcctcagcgtaggtacctgcgtgaaagaagagatcccggcgatgtttgagaaactgcaggctgcactcgaaaaactgaaatagcggagagatcgccttcggcgattagaaattgtcttggagcaggattacgctgattttactgattagcttgatttttattttttgattaataacaattaagggagatataggcggatttttttcgcttatatctcccttaatcattataacaaagtccgataacaaataaatcaaaacataatcaaatcagggcaatcagtaaaatcagcgtaatcctgctccaagacaatttctaatcgccgaaggcgattactcggctatatctcccaaccctgactttctgacttttatcttcgaaaagttaaatgggtgttaaaaggtcaactttagttactatttcaaaaaaagtccctaattttgaccttgaaactaaaaaagtcaaaaagttaatgcacacagaagctaaagatgaaatgagggataagatcctggaggcggctctgaagcgttttactcattatggcgcttctaaaacaacgatgaacgagatagcagatgaccttcactgctctaaagcatcgctgtattactatttccccgataaaaaggcgatgcacattgccgtgttgcaaaaaattgcggaagcatattttcagcaaatggagaaggaagcagttcaggtgaaatcggctgccgaagcattatataatatcattgatctccggaaagattttatcagcaaattctgccggctggaaatatttaaaatattacaggataattctgcgctcttcctcgaagaaaagaagaaggcaaaacaacgggagtttaatatccataccaccatcattaaagcaggtattgcatcaggagagtttaaagtaaaagatcctgaaaaaaccgcggaactattggtgctggctgctatgggattgcgcttttctgtgcccgatcatatccgggaagacatggagctggatgaagaaatgatggaccaggtaatagaaaaacaaaaacagttactcgaaattttcataaaaggaataaaagcataaacggaaatcatggtagtgagagaaaggatactggaaactgcgctgaaaatgttcaggacatacggtgtgaaaggagtaactatgtttgatatcgcccgcgactgtgggatttccaagaaaacagtatatgagcatttcgaagacaaacaggcgctgatagacgaagggatgcaacaactgctgacaaaccatattaactacttccatgagtgtttgcaaaccacagacaatgccatcgaagaactggtgcgtaacatgaagtacgtcaccaatctggctaaaaccctgaacccggtaatgctgcacgaaatccagaagtatcatccggatacctggcgcagtattgagagttttaagtcggataacatgctttgtaacatcaaaaagaatttaaaaagaggaatggcggaaggcctataccgccagaaccttcatatagatattgtagcacgtatgcgccagctgcagctggaggcagcttttgacccggagcaataccccgcagatcaatttgaaatgcatgaggtaatggaacaggtaacggcccactttatactgggaattgccactatccggggacataaactggtaaaccagtacctgcaaataaaagaagaagaataaaactactacgctaagatttattttatgaagcgattaaagttaacgcttgtcctcctcatggggataggggtatataacggctatgcccaaacgcaactgaccttacaggaagcgctgaggtttgcattgaacaacaataaacaattggccaaaaccaaaatggacgaagaaatgggtaaatacaaaacccaggaagtccgctcccaggccctgccacaactgaatggtaacgcttcttatacagacaacctgatgctgcagaaatcgctcatccccggtgctgtatttggcaaaccggatagttccatactggtggcttttggtgttaaatacaatgttaccgtaggcgcagaactcagccagcaaatctttaatcaggcagtgtttaccggtttgaaagcttccaaggcaggagaagaatattataagatacaaacggaacaatctgttgaaaatgtgatctataatgtatcacagctctactaccagctgctggtaacacaggaaaagatcatcaccatcaacagcaacatcgagaagcttacgcagctggtaagcgccaccaaatctcaatttgataacggcctcgccaaaaaaattgacctggaccgtatcaaagtgaacctcatcaacaatatgacgcaacgtacacagttgctgaatcaatatgcaacgcaaaccaacaacctgaaaaaggtaatgggcatgccactgcagtcaactttcctgttgccgcccgcttcactgaaagacattgaaaacaaagccgccggtgtgttacagtatgatgatatgaatcttgccaacagaacggaatacaaattattgaagaaacaggaagaactgcagttattccagaagaaagcttaccaggcagaaaattatccctcgctgtcgttgttcggaagatactcttacaacgggatgagtcagcaatgggctttttcgaaagaccctaccaactcaaccagctggtttggtgcagcagccatcggcgtatcactgaaggtacccatcttcgatggctttggccgccgctccaaagtgagtcaggctaacgtaaccctgcgtcagctgggcaagcaactggaagacacagagctgaccctcaacaccgactacgaaaacgccaagctgatggtgcgtagcaacttatctaccatcaccacgcaaaaggagaacgtggacctcgccaatgaagtgtattattctactcagaataactacaaacttggcctggcaggcctgacggatctgctgaacgcagaaacttcgctggcagatgcacaaaacagttataacgaagccctgctgcaatacaaactggcagagctggagataataaaaagcaaaggaagtttgaaagacctcctgaactaaacgtataaacgaaaacaacgatagaacacacaaactattttgcagatgaaaaagtttataatctggggcttggtggcagtaggtgcagtagtactgatcatgtggaaactcagcgctaacaaaaaagcgaacgaggctaaaacagaattcgtaaaacaaagcaatatcggcgacatcccggtgctggtacagaaagtatcccgcaatgatttttcccagggattcctggccaatggtaactttcagccagtacgcgaactgacgtacctcgccgaaaccgccggccgtattaccaaactgctcgtagatgaaggcagcgtggtaagacagggacaacccattgcttacattgatggtcagcttttaaataccgacctcgaatctgcaaaagctaacctcaaccagctgaaagtagataaagaaagatacgagagcgcgttccagaccggaggcgttacgcagaaacaaatggatgatgcacgcctgcaatacgacattgcgaaaacgcgctatgaggctgccagccgtcgcgtaagcgatacttatgtgaaagcgcctatctccggaattattaataaaaaatatattgaacagggtgcttacctctctgtaggcaataaaatgttcgacatcgtggatgtatccaggctgaaactgtcagtatctgtaccggaaggacaagtggtaacactcaaaaccggccaaaaagtacaggttacttccaacgtattccctgaaacccagtatgaaggcactattacctttattgctgcaaaaggcgataactccctcaactacccggtggagatggaggtccgcaatattgatggaaaagacctgaaagcaggtatgtatggtactgcacatttcgtagatccgaatgcggccaaaacaattttcattgcccgcaccgcatttgtgggtggcgtaaacagcaataccatttatgtaatggacggtaatgtggcaaagaaacgcaaagtagtggctggccgcattgttggcgaccaggtggaaatacgggaagggctgaacgaaggcgacaccgtgattaccagcggtcagattaacctgactgaaggcgctgttgtagtggctcagaacggcaaaaagtaagcgaggaaaatgtatctggtgtttgaccaaatttttgcaacatgaagattactgaagtatcaattaagcgacctacgatcgtggtggtggtgttcaccatcctcaccctgctgggcgtgatgagttataaatcgctgaactacgagctgttgccaaagttcagctcccctatcgtaaccatttctacggtatatcccggcgcctctcccaatgaggtggaaagtacgattaccaagaagattgaagatgcggtagcatctatggaaaagatcaaaaagatcatttccaaatcttctgaaagtctttctgttattaccgttgaactgaacaacgatgcggatgtggatattgccctgcaggatgcacaacgcaaggtaaacgctatcctggcagatctgccgggtgatgccaagccgccgtcgctcaacaaattctccctggatgaccttccgatcatgacgctgtctgccaccgctaaaatggatgacaaacagttttacgacctggtagataagaagctgcagccattattatcccggttaccgggtgtagcccaggtatcactgattggtggccaggagcgcgaaatacaggtaaacgtagatccaaaaaaattgcaggctttcaacttatctatcctgcaattacgtcagctgatcaccaacgctaaccttgactttccaaccggtaaggtgaaaactgccaatgagcagatcctgatccgtttggccggtaaatataaaaacgtagaccagctgcgtaacctggtgttgaaaacaactgaggatggcacacaggtgcggctgacagacgttgccgatgtacaggatgcccagaaagatgcggatcgtattgcccgcgtagatggtgttagtgcgattgccctgcaggtgcagaaacaaacggatgccaacgcggtaaccgtaagtgaagaaatgaagaaggccatcagcaaaattgaaaaagattatgctgcgaacgacctgaaaatgctggtagcaaacgattcctccgactttacactggaatctgccgactcggtaatacatgaccttatcctcgcggtagtgctggtggctgttgtgatgctgttgttcctgcacagtatccgaagtgcgttgtttgtaatgatttccattccggcttccctcattgctacgttcatcggtatgaaattgatgggcttctcgctcaacctcatgtcattattgggcttgtcgctggtagtaggtattctcgtggatgatgcgattgtggtgctggaaaatatttaccggcatatggaaatgggtaagaatcgtgttcgtgcggcatttgatggtgtgaaagagataggcttcaccgttacctccattacgctggtaattgtggtggtgttcctgcccatctctttaactaatgagctggtatcaaagatcctgcgtgagttttgcgtggtggtaatgatttccacgatgcttagcttgttgtcgtcgtttatgattgtgccgctattatcatcccgctttggtaagctggaacatattaccggtaaaaacatttttgagaaattcattctctggtttgaagcacagctgcagaagttcaccaactggatgaccagtatcctgaaatgggcgctgggtcataaaaggatcaccatagccgtggcagttggtttattggtagcttctttcatgctggtaggtaaaggctacatcggtggagagtttattcccaagggcgaccgcggacagttcatcgtaatgctggaaatgccaaaggatgcatctgtagaacaaactaacctggccacacgtactgcagaaaaatatcttaataaaaaacaggaagttacccgtttgatcacaacagtaggtcaaaccagtgaagatggttttggtaacgcgcagtcaactgcttataaagcggaaatcaccgtaatgctggtgggtccggaacaccgtttggatgcttccgatatctatgccgccaagatcaaaaaagaactgaaaagtatcttacctggtgtaaaggtaaaaaccacggatgtaagtatcctcggcaccgcagagcgggcgccggtagagctggtggtgatgggtacggagctggacagcgtaatgaactacgctaaaagagccatggatacgctcaaaactatcagtggcgctacagaagtaaaactgtcggtagaagatggtaacccggaaattaatgtgcaggtagacagggataagatggccgcactgggcctcacactggatgccgtgggtggtactatgcaaaccgctttcagcggtacagccgatgactctaaagtaaagttccgtcagggggattatgagtacgatatcaacatccgttttgatgatttcaaccgtaagaacctggaagatgtatccaatatacagttcatcaacgataaggggcaactgatcaagctgtcgcagtttgctgtgataacagaaggctcaggacccagtcacctggaaagaagggataaaaacacttctgtatcagtgcaggcgcaggtaatggggcgtccgtcaggtacggttacccaggaattttccgacaagctggcaaaaatggacaagcccgccgggatcaactacatttttggcggtgatgcagaaaaccagggcgactcctttggtaccatgggcgcggcattgctgatctccattgtgctggtgtacctgatcatggtggcgttgtacgacaactacatttatcctttcgtggtattgttctctattccgctggcgatcatcggtgcattactggcactggcactcaccaacaatacgctgaacatctttaccatcatgggcatcattatgttgatcgggttggtggcgaagaatgcgatcatcctggtggattttacgaaccagatgaaagagcagggccaaagtacttaccaggcgctgattcatgccaaccacgcacgcttgcgtcctatcctgatgactaccatcgcgatggtgatcggtatgttgcctattgcattggcaacaggtggtgtggggtccattaaaaatggattggcctgggctatcatcggtggtttgatgagctccatgttccttaccctgattgtggtgccggtggtatacatgatcgtagatatgggtatggcgaagctgggaatgggcaggttgtccagcaaacgttatatcaggcaacgtatggtggcctcttatgaagaagtgcctttaaatgaaattcattcgaattaaagatatgttactaacagtgtaacagttgtaggtttaggtaatagccggagtaatcatactctggctttctttttttcttgagaagtacgaaacctgccatttggtgtattattattttcacgcgacctcaattttgttctttgttcgcgatttgcgaacaaagaacaaaagccgtatctttaagatatgagaggtcataatggaatgcgtccccaggacgtagtaatcttattgaaaatattaacaatgcgggataattggcagtacagggatctgtcaaataccttgtctattagtatttcagaaatatcggagtctttaaaccgcagttgtatcgccggtttaatagacgagccgaggaggaaagtatttcgtatctcattaatggagtttattcaatatggactgcattatgtttttccgcagatacctggtcaggttgttacaggaactcctactgctcactcacatccgttttataaaaatcattttgccagtgaatccaattatgtctggccggatgatcaaggctcaatgagagggatgttaattgaaccattacataagggagtagtgaaagctgtaaaagaagatgccctgttgtataaagctttggcaagtatcgacataatccgtgtgggtaaatccagggaaaaaaagctggctatagaagagctcgggaaaatcatattaatatgagtcatagagaaaacatcaccaggataaaagcagtttataacgctttggaagaattaaaacgggaagttgtatttgtgggaggcgcgaccgtctctttatatgctgatagaaaaggagaggaagtaaggccgacaaatgatgttgatattttgattgagttgttgaattataaagggtatcaacaattggaagataaacttagagaaaagggattttcgaatgaccaggagtcgaagataatatgccgttataaggtactcggtatcgttgtagatgtgatgcctacttcagatgaaattcttgggttctccaataagtggtataagcagggatttgccactgcaatggattatcaattggagcctgaagggaatgtaaactatatcatcaggatatttaagcctgaatacttcattgctaccaagctggaggcttttaaaaaccgagggaaagctgatggaagaacaagttctgactttgaggatattgtttatgtttttaacaatcggaccacaatttggcaggaattaaacaatgcagataaagatgtgagagattatctccataaatcttttacagaattaataaataatgtttatctggatgaatgatagatgcaaatatggatttttcggaaaaaggacgaactaaatttattatcgataatatcaggcaatttgcatcattatagtaattgtggaattctttgattttaacaataaattctttccttttcacaaccccgtttatctctccacagtttatatttgcagcaaatacatttattcctgacagttctcccaaaaaacgatcaacagacagaaaacatgctggtggcggataaccagccgaaaataattccactgaaagactatggattatgagatgtaccggaaagtgatttacagccacttcccggtgacagattattttcttgctaaaagcagcatatgcgaaacaggaaaagggataggtaagggtacactatttttgcacgggcgcatcaattgtaccttaccttccagcctgttattcacaatccactcgttacgccaggtagcagacaaattatccagccgcaggccggcttcttccagggcggctttccagtcttcataattccaaaaacaaaacgtttcatgcatttcactgagccagttgtcgtggtaatcctttttgaacaggaattcacacgcattttgcatggacaactgtgcataagtttgtcctgctatggttacccattcatagggtaattgaaagccttcctggcggcggaagtccttcgagaactgcttgaacagcgctttggtcgacagctttcccagccaggcggccagttcatgtgtatcggcatgttcgggtaattcgatatcattttccccatcggtttcattgagccagagcaaaatggtttcgtctttgttttccggtcctactacatcccggtttatccagacgccgccgggaaccagttcattataacggttacgtataaacgcgatcaggtcttcccggctgccgtatgattctatttcatgggtgagcgaagaagtatgaatggtattcatgctgccggcttcaaatacgaggctggtcactgcatttttttgcgagaagaacacggatgggttggcgaattcgccgttatgttttctttgaagacagatatcatacaaatgacgggatacctctataccgtagaaatcgcattcatgcaggcgatcatcttcgcaggccatttttatccacgaaccaacggcgcagccgatatcgccgatgttgcccggctgaatatagggagctgtttcccggtatttctgggcggcgatgtcgtccatttgtttcacgtatacgttatagtcacgcgtagcagtaagatcgccgtctgcgccaatgataggatctttcaggatatgttgcaccttgtcccctacattgtagagcgaccagattttgaaagaagccgggtgcatctggtcgaggatggttttgttttttcgccagtcgccggcctgcgctaccagctttacaatatcccagggcatgggttgcgtgaactggttgctttccgggtcccactctgccggcagtatggtgaagccatgtttgatgtacatctcctttactgcggtggagcaaataacgagggtattggccggggtgagggaatggatcccttcactggaatgccgtatagtctttaccgtatattctgtaaaatcattgatcacgcctacatcgtcgataccgtatacgtataccggcacatccagggagttggaaaattcctggatgatcatagcgcggaggtagaatggcaccgggttccgtttggtgcctaaatgattggcggaggtaactgcgaagatcacgccttctatttcctgtgcgactaacggttggccatacacgtctttttcgccttccagtttacatttgatcaggcggttcaggtatttgaactgaaaatctgttagcaggtgatgccggccggggatgagtaaatacatgccatgaagttaagggaatgcgatgattttttgtatacgtattatgcaaaaataacagagggtgtatcgtagatctgatacaccctcctgaggaaaacacggttggaagaaataagaatacgttataatgttgcagtttttctgacttcatcaaaggtgtagctgagtgttacttcaccattttcaaataccgtatgtaacaggtcggcagatgcaggcgcctcttcttcagacactgttttgaaagtattgttgtcttttatgagtctgagtttcccggcttttgattttttgaaagaagtgcgtaactggccgctggcgtctagttccacgggcatcttctgaacattgatggcttttccgtttaccacagcgtaagcgcatttgagggcaaactcctgggtgtcgcggtttacacgttgcagtaaggcgcctcccatgcccaacaccaggttttctgcgctgatgccggcctgcttcaaggcttccagtatgccggggatagatgaatagctgatgccatcgccctggattacccttacctgcggaggcagtactttaaatcctttttcattggtgctatagccgaatttatccatcagtatggtgaagatacggagcagggtttgtaccggatcgccgctatcagggcgaattaccagcgtgccttctcttttgaggatctgttcttttaaagcagtgccccagtattcttcacaggccctgaaaatgttgtaggaatcagatacacaggcgatagtgccggtaggataactatccaatatatgtttgaatatttccagttctccttcttctccaagaagtgtaacaacggagtgttcggtagccgggatagataaaccgggtgcggcaggggcatcgtaatatttcttcgcaaatacggagccggggatggtgtcgctgcccgcaaagcttaccaggtgggcactcccgccgataccagcgctttcaacagagctggcgccacggaatccaaagtcgttcagcacaaagtcgataccgccgaaggcagctgtactggctgtttcttcataatatttctttactactttttttatttccctggatacggatgccacggtgcaggggtaccacacctgcatcagcagtgtttcaaggaagttggtgagccagaagcattccgggtcggtgttttctatggtcatcagcacatttcgtacaggcactaccgtgccttctgccactgctttgatacgaacggggagtttaccgccgtatttatcgatgatgtattcaaagcggctgcggtcaaatacatctttccggccaaacacttctgtgaggatggtttcggcctcgtccagtttttctttggtgaataccaccccgctcaggtattctttcagaaagtattgtaagccatagaaaacagtttcttcaaatttgccgccgcggctttccagataagagtaaatgaattgtgtaccgggaatgtacagtttatggtgggaatatttataagcatcggccaggaggatgagattttcctttgtcatgtctcaaaagttttagtcttagtcaatatatttttcggtcagttttgccagcaggggaatatgtgtatcattgatctctcctctggcaattaaaccaggtatatccgttaccgttatccagcggatttcctgtaagtcatcgccggcggtgggttcgccatatataaggtctgtgctgaacagcgtggtgatgattttgtttacttcgctgcggtagcgccagtcatttaccctgagggaagctacatattgcatgggaccggtttccaccgcgccgcattcttcctgtaactccctggcggcggccatttcgaagttgtcgtctgttgggtcggaaaaacctcccgggagacgccatacgttttcgtttggcttgcggcccagcaacagttctttcttatcgttcctgaacaatgcaatatctacagtagcatatacagaaggaaagagattgtaagtattgtagatgataccggcgcggaattcttccgtatcaaacaccttgtcagatatcgcttcccgcatggcggtggcgttataatcctgtaccggaggcagggcttctgttttatatttgccggagtaggtatccataaagctgttgcggctgccgtacagcaaaaagctttcgtgcgggaagttgttgctgagcagttcatccagtttctgtgaccatacatcatcgcttttctgatcactcaggggcagtacaatgatttccggaaattgctgcttgatcatccgttcacgggtatagtaatccagtgggtttttgcggctgcctctcaccgggctaacgccgagtatgatgagtacgcggttgtgcttttgtttcacctggcggatgagttccaggtgcccttcatggagggaaggcgtttggaaccgggcgataataactcctgtgggctttgtgttttgcatatccgagctattttgtgtaattgttacacaaatatagaaaccgtttctgtatttccaaaatatttcttgtaaaaaatacacaaaataggaaatgcggttgctacaggatattaatatagggattattgcagggaaaatggcatgtggaagaattgccggcatgccgtggctgttcaatctttaaccggcctgtatgatgcgacgggtctatatttcaaacgtcattccttctttcttcagcttaaaatacctggcttcgtcaaagctgaacagctttgcgggcctgccctgcgatacctgtttctgtttttcgttatgggcaatcaatatcccgagatgattaatcttcttctggaaattgcggcggtcgataggccggtccagcagggtttcgtaaagtttttccaggtcggcgatagggaatttattatccagcagttcaaagccgataggctcgtaacggatcttgttgcggaggcgttgtacggcaatattaataatggcggcgtgatcaaaagccagtgtgggcaggtctttgatattgaaccatttggcgtcttctgcatcggaactggcggccagtttgaaattggtgggatttaccagaccgaagtaagcaatggatactacccttccgcgcgggtcgcggccgggtaaaccaaaagtatacagctgttcgaggtagttgatatttacgccggcttctgtcagcagttcacgggtaacggccgcttccagcgcttcatcgtccagcacaaagccgccgggcagcgcccagctgtgcaggtatggctcaatggtacgcttgattagcagcaccacgatgccttctttgggaatatatccaaataccactgcatctacagttagtctgatgttttgtatgatcggcaaactcttatctgattattttgcttgaatgtaatgttccagttgggcagtgcctttgtgtaaatttacgaacaaaggatttttctgtggatcaaaaacgatgatggtgctttgttcccagatatcctgcggggtgggcagctcaatgatcacttcctggccgttttcgcggtggaaaagcaaactgtcttttcccgccatatgtcttttatactggtgctgatccaggtaatcagtcagctcttttctcaattgcagtacagaatcggtcagcgggttggaggccggcttgaactcgcggtacacgtagcacttttcggtgataacgtcgtaggccgatctgtcggtggtgcgttcatcgttacgggtatggttacacgcaaacagcaacaaagcaactcccagtagtgataatatttttttcatgatctcatagctttaatgttcgtaacaatcatagttgcgttgccggtaaattttcccgtcgcggaattctatgatagtgcaaatgaatgctttcattatttgtccccggcggaaatgcccggcatccacgcctatttcccctgtccatttggcttctaccaccagggtatttcctgattccactactttcagcacgctgaagtgctgcgatttcaaaattattttattggtgaccatgctttccagcatgatctcaaagttccgttgtttaatttcattcgagagctggtttggatattcagtctgaataatatttggatgaaagatcctggcaaattcaacgggatctgctgaaaagctctccagcagctggaaataccggtatataagcgccagtttctcgtccatttatagggataaattgaaattttacgaatgacgtatttatgcgaaaatatacatttcgcacttatatgtaacctgcaaattttgaagcgatcttaattcgggcacctcactggatgctgctgaaggcgagtttatccctgttatttgttttgtcgatgatgttgtacaccagcttcagcacatgcagggtgccatcgtagttcactttatctgcggaagtatttttgcagaaatagagtaccggtatattttttttgtagaaagatgcatgatcggagttgctgataccactggaatcatataccagtggcagctctttgccggcagcttcctgaacaatggccgaccatccgggcgatgtgccggtaccaccgatctgtaatgccgtacccgggttcagggtgccgataccatccatattaatcatgtagttcacctgcgaaagatctacggtactgtgggacgcaaagtaggaagagccggaaagtccctgttctttccctgaaaaggcgataataatataattgttgttatgaagacgggagcctttcagtaagcgggctatttccagcatggcggcggtgccgctggcattgtcttccgttttgtcggtggtttcccagccgcggtaatcgtaatgcgcgccaatcacgatggttctgggagctttattgttgatatagccgattacgttggtgccattacgttttatagttttgaaggctacctgcatgtgaataggaaatccatccgcgtcgtcagcgctcagttttttgctgacgtcggcattaagccatacggccgggatgccggcggctttgggacgttcggccagccatttcattacttcgggagccgtttctttgccattgtaaaataccacaccggtggcgccggatttttcggcagtctgtgtttgctgtaaatactggtctgacatgcttttccggccgtcggtatccagttcggctgcattgatcagccagatattatcgggttcgttcacccccggaatagcttctcctttggccgatttgccggcactgaaaggcagtggcacaaattgtttacctgcttccagtttgtttccgccaatggtcatctgacagtctgccgacggttcacgggtttcttttactgtaaatgcctgtaaaaaaccatcctcgcccataggcgtcaatcctattttctgcatttgcgcagagatataggcggctgccagctgttcgccaggagcaccggtactgcggccttccagcttatcgctgctcaggtaactgatgtgtgtttgcaggttaccaattgttttgcggtcttcctttttctgggcatgaacgtgtatggttacaactatcaatggtaacagccaggtcttctttttcacagcgaatctgttttgggtgttgcagcaaaattacgaattacagacggcccaaagcacatcggcagttaattcttttgactatatcattgtattttaagtatttataatgtatgcctttcgtcttaaaacagtcataccccgttttatgttggccgttcataatttccaaatcgctatttttgccccgttttaaaaacaaagtatgaaaaacacgccttttacagagaaacacattgcgctgggcgccaaaatggctgcctttgcgggttacaacatgcctatttcctacactggtattaacgacgagcatcaggcggtacgtaccaacgccggtgtgtttgatgtaagccacatgggcgaatttattttaaagggtgaaaatgcgctggacctgattcagcgtgttaccagcaatgacgcttccaagctcactgccgggaaagcgcagtacagctgcctgccaaacaacgaaggcggtatcgtagatgacctgctcgtttattgtatcgaagaaaataaagtatacatgctggtggtaaacgccagtaatattgaaaaagactggaactggatttcccggttcaacaccaaaggagtggaaatgcacaacatttccgataaaacctgcctgctcgccatccagggccccaatgctaccagcatcctccagccgcttacagaaaccgacctggtgaacatgaagtactacacctttaccaaaggaacctttgcaggcgtaccaaatgtagtgatcagcgctaccgggtacaccggcgcaggcggcatcgaaatttattttgaagataccgacggagcagccgataagatttgggatgccatcttcgcagaaggcactcctaaaggtctgaagcctatcggtttgggcgcacgtgacacacttcgcctggaaatgggattctgcctctacggaaatgatatcgacgataccacttctccaatggaagcaggtttgggttggattaccaaattcaccaaaccatttacctccagcgagttattcgcaaaacaaaaggcagaaggcgttaccaaaaaactggtaggctttgaaatggtagataaaggcattccccgccacgactacgaaatcagggatgctgcaggtaatgtaattggccgcgtaacttcgggcacccaatcgccctctatgcagaaggctatcggtctcggttatgtgaaaacggcttttgcagcacaggatacagaaatttttattgcagtaagagacaaggccctgaaagcaaaagtggtaaaagtgcctttcctgagctaggaatatgtatgaatagccggttaaagttgttaatttcggtgcctggaaagttttcggtgcaccggaatttttatattttattaccatatctatgcctactattcatttaactaccgttatctatgctcccctggagcgggtctacgacctgagcaggagcattacgctgcacaagcgaagtatgtcgcaccggcaggaagatgcgataaaaggccgcaccaacggcctgatatcttataatgaaacagtgacctggagagcaaagcacctgggaaaaatgagggaactgaccactaaaatcactgccatgcgtcaaaacgagttttttaccgatgagatgactgccggcgactttacccatatgaatcatgaacattactttaaaccaatagagaatgccacggtgatgattgatattatggactttggcgccccttatggttggttcggaaaagtatttgagcggctctacctgcaaaaatatatgaccaggctcctgcaggaaagaaataataccattaaggattatgcagagagcgaaaagtggcgggtaatccttgattaaagcaaaacataactgaatgacagatagcaacaaacccagcctggaagtatgtttatctccggcattattacatttgtttgatgtaaaaaacagcatcgtagttatcatagatgtactgcgcgctacctccaccatctgcaccgccctgtacaacggtgcttcccgggtaataccggttgccagcgtggaggaatgtgtgaacatcggccgcgcgatcagcggtatcaccgccggtgaaagagatggcaggatagcagaaggactggcatacggcaattctccctttgaatatccacgcgagttcgtggaaaataaaacactggtactcaccaccaccaacggtactaagctgctccacatggctaaagatgccatacaaatcattaccggttccttccccaacatcagcgctgtttgcgattacctggtggcacaaaaccagaatgtcatcctcggttgcgctgcctggaaagaccgtgtgaacatggaggataccttgtttgccggcgccgtggtaagccgcattaaagagcactttgacgtaaactgcgactccgccattgctgcggaaacactttaccactccgctaaacacgatatctataccttcatgaaacaggcctcccactacaaacgcctcgcgcagtacggcctggaaaaagatattcactactgtcttactgcagacggcgccaacgtgttgccactgttcagagacggggaactcattgcagggtgagcgcggattttgtctttctcaggattacgctgattatactgattttttggattttatcctttggatttttaaaatgattaagggagacataagcggatatttccgcttatgtctcccttaatcattaaaatcaaatatggtcaaatcttagtaatcagtataatcagcgtaatcctgagaaagacaaaatcctactcctttggggcgatacctttgttcagtgcaaaaaatatggttaccagtaacatcgtcagcggataggaaatttcggcaaagggcgcgccgctggtaattttaaacagcgttgccactaccatggtaagtagtaaggcaattgccgccggccgtacaaagaagccggtgatcagtgcaatgcctcccaggaattcagccatggtagccagaaaaccccaaaccgccggccagaaagtaatacccattattttcaaggtgccgccaagaaattcccaggtaccggcgccgccggcaattttcataataccaaaaattgtgaatagtacgccaatgcctatacgaagaataagaaatgccagtttgttgttgtttgtcatagaaaagagtttaaaaatgtgatgcaaaaataagatgatgaaccagggaagtcgatggataaaatgtgttttgtattggactttttttaccggccttgtttcattggctggtcagccaggtggactaaattttggagcatccatgaaataaaaacaaatggttctgttatgccggcttgttcgctttgaccaaaaaatcctatattctgtttcctaaagaggatgatatgacacactatatctgcagcacctgcggggtgcaatatgatgccacagaaaaggcgccggcatgctgtcctatttgtgaagatgagcggcagtatgtaaaccccggcggacaagcatggacgaccctggaacaggtgcggcaaacccaccggaatattatagaaatggtggcgtccgatctttatgctatttacacaacgccggattttgccatcgggcagcgggcgcatttattgattaccccatccgggaatatcctctgggattgcatagctaacctcgacgcctctacgattaatattattgaaaaactgggtggcatcaaggctattgccctctcccatccgcattatttctccaccatcgtggaatggagccatgcttttggcaacattcccgtttatgtacaccaactggatgcccaatggctacagcgccacgacgatgtgattaaattatgggcaggcaatgaattgccgctgtgggacggcatccggttggtattatgcggtggtcattttgccggcggcaatgtgttgtattccccggccggaaagggatgtttgcttgtgggcgatgtggtgcaggtatcttccgacaggaaaactgtatcggtgatgtacagttatccgaataatattcctttatctgccaccgaaattaataccctgcatgccgccataaaaccgttaaactatgatgcgatgtatggcgcttttggaaaatatattaaaaccggcgccagggaggctgtcgacttttcactggaaagatatctgaaacgtatacggtaaacgattgataaacaagcttctatatttaaaaaaaattatgttgaaaaatacgcgttacaccgccatagtaaacggagagcggttaacgggttcttaatgagtgacccgcgggttattagaaattttctgcttacttttgtggattgcctttttatcagctgttaagtttttttgatatatctagtaacccttttgctgataataaaaagcgggcaacaacgtatagtatgtcgctaccccatttgctaaaatatgtttacaacaacggcactgatgaagtgatccgcagggggaagcgtattttttcggccgggggcgttgagctcatcgaggcagacccggtgctgaaaacagctaccttccgcgttaagagcgacacacatgccaattattaccgtgtttccatcaataagtatggagaaactaccggtatgtccatccggtgccaatgcccttacaacctgggcgacatctgccggcacgaggcggcagcactgttccagctccaggaaatgctggacaaaaatcatttcgagagcttcgacacacagtttgatcagcagcatacgctgattaaaatgaagtctatcgatatcaaatccattaaactgcttacctccggtactatactggcagaagcagaggaaattgccaagaaacatcccgccaaaataagcctggcgaaagatgaaaaggtagaagccctgctgaaagtcaatggagaagagttcccgctgatcattcaacggaatgaagaacggttttttgatacgcattgcacctgcgatgaaacagaacatgcactgtgtgtacataaaacagccctcttcctgcaactcctgcagaaaaacggtccgttttatttcgataccctccgcaactgggacaaggaaaagaacaagctgctatccttatacggctattctcttaccgacgacctggacggaaagtttgccttctcctatatggacggcaaaccgtttttacgtgtactggaccccaccatcaaacgggtagatggcgccgccgcaggcagcaggcaaccggttacggctcccccgccaccggaagaaaccattaccattacacaacggctggcagcggttttcaacgccaacgaaacattatacccttatttcaaaatagacctggtaagcggcgaaattaacgaagagcaaactgccttcgtatcactggccagcaaactggatcttaccaaatacgtcgacttctaccagttcaaggaaaaagaccgggaactgatagcgcctatacgaaaattacagggcagcgaagtcagcaaatttctcagcaaaaattctccgtttgccggtatctgggaaaatataacgcacgaaaatgcagaagaacttcccacggaaacaaaagaactgatgctggaatacctgcatcctaaactcgccaaactgttcccacagctggcagagcatggattggtatttgaactgcccaaccggcaggcgtttaaaacaaagaacctgcaacaactgcagataggcgcggacaggctcaaactggtcattaaaaccaacaccggcgatacgcatgtagacatcaactgctacgtgaccatcgaaggagaactggtgaatgtgtctgaaaacgaatgggaaagcccgttgctgttcctgcacaaacagatgatctatttgtttgaaagcccgcaggatgccctgcacgtggagctcttccgtcaaaacggtcagctgcgcatcgctaacaaagactggcccgcttacctgaaagactacctgctgccattgagccgtcagtacgatatccagttcgataaaggactgctggcagaactgaaagatgtaatgcccgagccacgggtattcctgaaagaattgggcgaaacttttatcatacaacccggatttgcttaccgcggccaggaagtggagtggaacgatgagagcaagatcacggtgcaggaaggaaataaagtactcatcatccaccggaataaagaagccgaagaaacttttgtaaataaactccgcaccttacataccaacttcgcgcaacacgataaccacaattatttttacctgcgtgctaaagaagcgctgaaaaataactggttcttcctgttcttcgatgcactgaaagaaatgaatgtgcgagtgttcggattcgataacctgcgcaactttaagttcagttcgcataagccggttaccaatttacagatcagctccggcatcgactggtttgatgcacagattgaagtattgtatggtgatcagaaagtaagtatcaaggatattaaaaatgcgctggccaacaaacagaactatgtacagctggcagatggctccctgggcctgttgccggaagaatggctgcgcaaatattccctgctcttcaaagttggggaagaaaaagataaaggactcaaactcagcaaatataatttcagtgtcatcgatgaactctatgaatttattgatgatgaagcagtagtattggaacttgaacaaaagcgccggaaactgctgcagtttgatgaaatccgcaatattgccctgccggaaaacctgcaggccaccctgcgcccctaccaggaaagcggtttccagtggctgaactatctcgatgatatcaaatggggtggtatcctcgcggatgacatggggttgggtaaaaccatccaggcgcttaccttcctgcagtattacaagaacaagcacggcggtaaaacaatggcgctgattgtttgtcctactacactgatctataactgggaaaatgaaatcaggaaattcacacctgatatcaggcatcatattcaccacgggccggcacgattgaaatcgtctgaagagctgagtaaatttgatgccatcattaccacttacggtacgcttcgcagcgatattcaactgctgatgaaactggagtttgactatgtcatcctcgatgaatcacaggccattaaaaatccgcagtcgaaagtaaccaaagctgcacagctgctccagacaaagaacaggctggcgctgagcggtactccgatgcagaataataccttcgatatttatgcccagatgaacttcctgaacccgggaatgctcggcagcgtggactttttccgtaacgaatttgctacgccgatcgataaattccaggatgaagaaagaaaagaacatctgcgtaagctgatctatccgtttatccttcgccgtacaaaagaacaggtagcgaaagatctcccggaaaaaatagaaactgtaattttctgcgaaatggatgcggaacaacggcatatttatgatgcctacaggaatacctatcgctccaagatcctcggtgttattgaagatcagggtatggaacgctctcagctcaccatcctgcagggcctgatgaagctgcggcaaatctgcgattcaccggctatcctgaatgatacggaacagtatccgaaccattctgtgaagctgcatgaactcacccgcgaaatttctgaaaacatcggcaaccacaaagtgctgatcttctcgcaattcctgggcatgctcggattgatccgcgaccggatgcagcatctcaaaataccttatgaatattttgatggcagcacttccaccgttgatcgtgaaaaggctattcagaacttccagaacaacgacgagtgccgcgtgttccttatttcactgaaagccggtggtgtgggtctgaaccttactgctgccgactatgtgtatattgtagatccgtggtggaacccggcagtagagcaacaagccattgaccgtacccaccgtatcgggcaaacgaagaatatcttcgcttaccgcatgatctgtaaagacaccgtggaagaaaagatattgcagctgcaggaacgtaagaaatcattggtgaaggaaattatttccgacgacagtggttttgtgaagaagctgacgaaagaagatgtattgtacctgttcagttagatattggcagcctaaggattatgtactaaattagatccatgagactctcaaaagaagatatcagaattattcggcaatactttacagataaacctgtaaagaaagcttttatttttggatctcaggcaagaggagaagctaatgaatatagtgatgtcgatatattggtagagctggattattccaaatatataggattaggctttgttaagatgcagcaggatcttgaggatcaattgcataaaaaagttgatttaatttctgaaaaagcgctgtcgaaatttatcattccttttatagaatcagataaaaagttgatttatgaaaggtaagatgggcgataagctacggttacaacatattgcagaagcaataaaagaaatcgaatcttataccgccgggaaaacactttccgatttttttgaaaattctatgatgagatttgcttcagtaaagcaaattgagattataggagaagccgcaaatttgctgacccaggaattacgtgatctttatgcagatgttgcatggaggcaaattatcggacttagacatatcctggtacatgaatacttcggaatagacgcagaagtaatttggcaaatagtagaaagtgatattcctgttttgaaagatagaatagaacatattttaaataatctggaatagaaagtattaatgaagttataagagagatattttcctttcaaggaagatatctctcttttttattgaagttgattccctgaaactctttcatttttgcatacaccctgccatttctgcatggtttggccaatgaacatcttctccctatctcccctgaaaattatttaataccctgattaataactacttattcccttttgaagcactcattcccaatgatggcactccgctggtattacctcatttgtatcaaacaattgattcatatgctaccagattcaaaaatctctcaactgataggtttacagattccggggttaacatttcccgcagaacagcaacaacctgcaaagagttccatcagtaaggtgatccacacttttgctgattataccggcaggatgatccggagtgagcaacttcatgaggtgaaacgttgttttaacgtggccgctgtattgtatcacaatggaagcaatgccctgcgtaacgccatcgaaagcgcgtttatgtataccctctctcccctactctgcggaaagcataaggaactgcttcctatatcactgaagaacgtaaggattcagcatttacaaactatagctatttaaacacttttatgatgatgactattctcctggtgctggcaggattggcctgcttcgccgtattctttaaatcggtcgactatttcgaaaagatctaactaaaacacttgttatcatgactgcattatttgttttgtcacttttcgttttcggctacatgatctatgtactgttaaaacctgaaaaattctgattggagatattactcccacgcctatacgcaaaaaagcttatttaaatgacaacagaaatcttaggcgtaatcgccacctacggcatcacgcttttattggcctggcccttgtcgaggtacattgttaaggtattcaggggcgatcgtacctggtccgattttatggcgccgctggaacgcctcttttttaaaatttccggtatcaatcctaatgaggaaatgaactggaaagagcatttgaaggcattactgaccatcaacctggtatggtttgtatatgccttttttgcgctgttcttccaggacaagctgccactgaacccggatggaaaccccggccagtcggccgacctggcgtttaataccgccatcagcttcgtggtaaactgtaacctgcagcactattccggtgaaacaggcgttacttatttcacccaattatttgtactggccttcctgcagtttgtgagcgccgctaccggtattgcagcgctgatcgtggtgttcaaagccatgaaagaaaaaacaaccactaagttggggaacttctgggatattttcctgaaaacaatcacccgcatcctgctgccaataagcatcgtaattgcactgatctttgttttcaatggcgtgcctgccagttacgccggcaaagaggctattgttactatgcagggcgacaccgtgaatgtgtctcatggcccggtagcagggtttgtggcgatcaagcacctcggcaccaatggtggtggatggtttggcgccaactccgcacacccgctggaaaatcccaactacgttacctggatgacagaaatggtggcgcaggtactcattcccatcgcaatggtatttgcactggggatgtttattcaacggaaaaaatttgcgatgatcatcttcgggatcatgaccatcggtatgatatgcctgctgattccttccatgcagcaggaaatggccggtaatcctgccattgcccacatgggtatccagcaggctaccggggccatggaaggaaaggaggtgcggtttggagccgccgccacagggtactggagtacagtaaccactattatttctactggttccgtatgcggctggcacgatagcaccatgcctatgacaggtttaatgcaactgctggggatgatgctgaactgcttctatggcggttgtggcgtgggtatcctcaactattacatctttattattatcgcggtgtttatatccggacttatggtaggccgtacgcctgaatttatggggcataagctggaagcgcgggaagtaaagatcgccgctattattacgctgttgtcgccgttcctgatactggccggtactgctttatcatcgtgggtattgtcacaccatccggatgccaactgggcagtgaagccatcggcctggttaaataaccccggttatcacggcttctccgaaatgctgtacgagtatacttctgccaatgccaacaacggttccggttttgaaggtttgggagatggaaacgttttctggaatgtatctaccggctttatactgatcctcggcaggttcctgcctatcataggaccagtggccattgcgggtttgatggcatctaaaaaatatatacctgaatccgccggtacgctgaaaacagattcactcacttttggcgccatgaccttcgcggtgatcgtgatcctcactgccttgtcttatttcccggcgctggcactgggtccgatcgcagagtatttttccctgtaatttttttaatgactgactaccatgaagcatgataataaattgtttccgaaagaattggtgatggagagcctgaagcagtctttcgtaaaactgaatccgaaattaatgatcaaaaacccggtgatgttcaccgtggaaataggtactgccgtaatgctgatagtagcgctgtatgcactctttaccggtaataaggaacagggcagtgcggcgtataatgtcgccatctttatagtactcttccttaccgtgttgtttgccaacttcgcggaagccattgcggaagcgcgtggcaaagcacaggccgaaagtttacgtaaaacaagagaagaaacaccagcaaagaaagtagaactgataggtgaaatcttcaccaacgaaatcaaaatcgtatcctcctcttccctgcgcaaaggcgacatcttcgtatgtgaaccgggcgatattattcccgccgacggcgaaatagtacagggccttgccagcatcgacgaatctgccatcaccggtgaaagtgcaccggttatccgggaagccggcggcgataaatccagtgtggtaggcggtactaaagtattgtccgatcatattaaagtacgggtaagcactgagcccggtgaatctttcctggataaaatgatagccctcgtagaaggcgccagcaggcagaaaacgcccaatgaaattgcgctcaccatcctgctggccagcttcaccctggtatttatcattgtatgcgtaacactgaaaccctttgccgactacgcacaaacaccgattaccattgcggccttcatctccctgtttgtatgcctcatccctactaccatcggtggtttattatcggctatcggtattgcgggaatggaccgtgccctgcgtgccaatgtaatcaccaaatcaggtaaagccgtggaaactgcaggcgatattgatgtgctgttgctggataaaaccggtaccatcaccatcggtaaccgcaaggccactaacttctacgcgaccaatggtatacccacggcggattttatccgcctctgcgcactcagctctttatcggatgaaacaccggaaggtaaatccatcgtggaactggcgggcaaagatgtggtgagtaaattatcggtgagtggcgccagcctggtgaagttcaccgccgaaacccgcagcagcggcatcgatctacccgatggcagccgtatccgcaaaggcgcctatgatgccatcaggcggctcgcggaaaaagaaggattttctttccccgcggaaacactcgcaaaagtagaatctatttccaacgacggcggtacgccgctggtagtagcgctcaacagcaaggtgcagggcgttattgaattgcaggatattattaagccgggtatcagcgagcgtttcgaccgcctgcgtaaaatgggcgtgaaaacggtgatggtaaccggtgataacccgcttacagctaaatatattgccaccaaagccggtgtggacgacttcatcgcggaagccaaaccggaagataaaatgagctatatccgcaaagagcaaaacgagggccgcctcgtagccatgatgggcgatggtaccaacgatgcgcccgccctggcacaggcagatgtaggcgtggccatgaatagcggtacccaggctgcaaaagaagccggtaacatggtggatctcgataatgaccctaccaagctgattgaaattgtggaaatcggtaagcagctgttaatgacgcgcggtacccttaccactttctccatcgccaacgacgtggcaaaatattttgctattgtgcccgcgctgtttgtggcttccataccagccttgcagggcatcaacatcatgaaactgcacagccccgaaacagcgatcctgagtgcggttattttcaacgccatcattatcccgatgctgataccgctggcccttcgcggcgtggcctataagcctatcggcgccagcgcattgcttcgccgcaacctgctgatctacggagttggcggtattgtagcgcctttcatcggtatcaaactgattgatatgctgatagcgcttttcatgtaattgtaaactgataaatttttaaagagatgaaaaaatatctttggccttctgtaaaactcacactgttactggtggtattattgggaggaatatatccgctgttcattgccggcgtggctaaaatggctcccggaaaaggcgatggtatcaaagtaatgtataacgggaaagtagtgggctatgaaaacattgcacagaaattcagtgatgataagtatttccagccacgcccttctacggtagattataacgctgccggttctggtgggtccaataaagcagcgggtaacccggattacctgaaaacggtacaggaaagaattgattcttttatggtacacaacccggatgtaaaaaaagaaaacatccccgcagaactggtcactgcttctgccagcggtttagacccgcacctcactcccgctgcggcttatgtacaagtgccgcgtgtggcgaaactaagaggcattcctgcggacaaactgcaacaactgatcgatgccaataccaaaggtcccttgatgggactgtttggactatctactgttaatgtgttaaaattaaacatagcgctcgacgatatgaagtagcgcgcagttctattattccttacctctgaatgtcctgtgaacaaccttttaactggtggcctgtcgcagcaggttaccagtgatctaccaacacgaacctatatatttaaaatgaagaaacttttattactggccggtgcactggcagttgccattactatgtttgcccaggacgcaccgccacaagagaaaggaaaagtaaccttttccggctatgcagaagcatattacagttacgacctgaacaacccggccaatcatacaaagcccgggttcctgtataactacaatcgccacaatgaattaaacctcaacctggggatggtaaaagccaattacacatcagaccgtatccgtgccaacgtagggctgatggccggcacctatccccaatacaacctggcagcagaacccacgctgatgcagtatgtatacgaggcaaacgtcggtatccgtataggcaagaacgtttggatcgatgcaggagtaatgcccgcacacatcggttttgaaagcgccatcggaaaagattgccctacgcttacccggagcatcctcgcagagaactccccctattatgaaaccggcgccaaagtaacctggacgcccaacgacaaatggtcgtttgccgctatgtacctgaacggatggcaaaggattaaaaaagtggatggcaaccaaacccctgcttttggtacacaaatcacctttaagccaacaacaaaaatattgctcaactggagcacttatatcggtaatgatctcccggatagtgtacgccagatgcgctactttaataatgtttatggtacctttagcataacggataaattcagtgtcatcgcaggattcgactatggattacagcaaaaaactaaaggatcatccaacttcaatagctggtacagtcttgttgtaattgcccggtacgcctttacagataaatttgcgatggcggggcgcgtagagcagtataatgataagaacggcgttatcatcagcaccggtacaccggatggcttccaaaccaccggctattcacttaacctggattttaccccggtgaataacgtgatgttccggctggaaggtagaacgtttaacggaaaagacaacacatttataaaaggaacagaattgaagaacacgaatacagcgattaccgcatcactggccgtatggttctaactaaataaataatgacagataaagaacactccgtacagcaatttcttaacctggctaaccgcgccggcagggggaagtttaagatctacatcggtatgagcgccggcgtaggaaaaacgtaccgtatgttgcaggaagcgcatgccatgttaagaaatggggtgaatatccagatcggttacatcgaaacacatgggcgtgcggaaacgcatgccctgctggatggattaccgcaaataccccgcaggcaggtattttacaaagggaaaatgctggaagagatggatctttccaccatcctgctcctgtcgcccgactgggtagtggtggatgaactggcacacagcaatatccccggctccaaaaatgaaaagcgatggcaggatgtggtggacctcctgaatgcagggatcaatgttatttctgccgtgaacatacaacacatcgaaagcattaaccaggaggtgaaatccatcaccggtgtggaagtacaggagcgcgttcccgacctcgtgctgcaaatggccgatgaagtggtgaacatcgacctcaccgccgatgagttgatcacccgtttgaaagaaggtaaaatttatgatcgctctaaagtggagagcgccctgagcaatttttttcaggcagataaaatcctgcaactgcgtgaactggcactgaaagaagtaaccacgcaggtggagcggaaagtagaaatccagattccgcgtaacttacagatgcgccatgagagttttctggcgtgtatttctaccaatgatgaagtggcccggaaagtaatccggaaaacagcgcgactggcggcctattatcacgccgattggtttgtattgtatgtgcaaacccctggcgaaagtgccgacaaaatcgcgctcgctgcccaacgtcatcttattaataacctgaaactggctacagaactcggtgcggaagttatacaggaacataacgctaatgtatcggaagctatcattaacattgcattggaaaaacatgttaccactatttgtatgggaaaaccgcatatcagtctttttcgtatcattttgcgcaccaacctgtttaaccagttgttgaaaacgctttcttccaacgatatcgacattatcatattatcatgagtacgttcagattaaaaacaaagattacgcttggggtattgttcctgtacatcatgctgctggtggtgagcatactgggctattactatctgaaccgcctgaacgaaaaggcgaagtttattctcaaggataactatgaatcactggagtattcgaaaaatatgctggtagctttggaagatctgccggctcatcgtgctgctgcgatacaaactttttccgataatctcaaaaagcaacaggccaacgtaacagaaagaggcgagaaagatgcaacggcagcagtaacccgcatttttgaactattgcaaaaagattccacagtagaaacaggcgccataaagaaaaatatctacaccatcatggatctcaatatggcggctatcgtaggaaaaaatgaaagggtaaagaaaaccgcagacaatgcactgctttacattgccatcattagcgggctttgctttgtactgggctttacttttgtgtataatttccccgggtacattgccaatcctattggtgcgcttacccaagggattaaagacattgccaataaacaatacggcaaaagactctactttaaatccggcgacgagtttggcgatctggccactgccttcaatactatggcccagcggctggatgaatacgagcacagtaacctggcgcgcattgtatttgaaaagcaacgcgcggaagccgtgatcagcagcctgaaagatgccaccatcgggtttgatgtaaataatgtgatcctgtttgccaacacccctgccctgcagttactgaacatccccgagaaggatctgatcgggcagccggcggaagaaatatccaaacgcaacgacctgctgcgtttcctcgtgaatacaaaggaaaatgcaccgctaaaaatagtggtggatggaaaagaatgtttcttcacccgcgaaacaacagatatcaggcatgaggaaaatcgtataggctatgtagtgatcctccggaatattaccacttttaaagaacaggatattgccaaaacgcattttattgccaccatttcccatgagctgaaaacgccgctggcggcctctgatttcagtattaaactgctggaagatgaaaggacaggcgtactcagtacggaacagaaagagctgctcgacagcctgaaacaggacaaccggcgcatgataaaaattgtaagcgaattgctggatttgtcgcaggtagaaagcggcaatatacaattacagccgcagccggttaccgccatgagcattgtacaatacgccatggatacggtgcggaaacaggcggctcaacgcgaagttaccatccgcacagaggtgccggaaaccttgccaaaggtattggcagacgtggagaaaaccgcctgggtgctggtgaacctcttaaccaatgcaatccgctactctgctcacggcgctgccatagaactaacggtaacgcctacaggaacagaaatggtatcgtttgcggtacaggactacgggaaaggtatcccggaagctttccggggtaaaatttttgaaagatttttccaggtgcctggtatgaaagggcagggaaatggcctcggactggctatttcaaaggagtttatcgaagcccagggcggtattattggcgtaaatagcgaggtaggaaaaggcagccagttttatttcactttaccggaagcatagtgctgtcagggttgctcaatatgcgcttttaccaggggcacatgctgataatagaaggtagtaagttcctccagcctggcgggaatgctgtcgaggttttcctccagccgggcatctctctcaacagacaaggctatatctgatgcgtattgcatgccaaccatgttcaggttaaatttcatctggtgcgccagcatataaagtggttgccagtttttttctgccagcagctggtgcatctctgaaagcttttgcgggatgctatccagcagttcctccagcattatttttacatgttctttttcgccggacatcatgccgtatgcggcggataagtttagttcgctgttgggcatttcagtggttttttctttgtcagtggctgattccggcacttgttccccgagtcctttcaggattttctgaaacaggtcggagcgatcaaatggtttggacacatattcgttcatcccggcggccaggcagcgttccttttctcctttcagtgcggaggcggtcatggcaatcatataagtccggatgcctttccggcggatggcctgagtggtctggtagccatccattcccggcatctgtatatccataatgatgcaatcgtacgttttgcagtccagcatttcaagggccgatttcccgctgttaaccacgtctgttctggcgccggcatttcgcagcgtatgaaataccacctgttgattgatgtcgtcgtcttctaccaccaatatcgtttttccctgcagtggtttttctgcctggtgcagggggcctttttcatttttactggtcattgctttgttattgcgggtgaacggcagttcaaaatagaaagtagcaccttcattcaggtggctgtttacccggatgaatccatgttgaagggtaatgagttctttggtgatggctaatcccaggccggtaccgccaaatttgcgggcattgttagcatgtgtttgggagaagcttttaaagatcagttcatgttgttccggatctatgcctatgccggtatccgttatttcaaagcccagccggagtgtggattgttctttatcttcctccaccagcgatactttcacggttactttcccggcgggagtaaatttaatagcgttttccacgaggttggtcaggatctggttaagacgcacttcatctcctaaaaggcaaggggggatggcggtatctatctcatcaaaaaacaatagttccttttgttgtgcctgtagtttcaggggaaagagggcattgtctattacttcgtaaatatccagcggttcatgtaggagcaatagtttgccggcttttatttttgagaagtcgaggatttcgttgatgatcaccagcaggcggttggcggatgttttgatggcgccggtatactccatttgtatgggagataactggctttgctgcatcaggaggttggtcataccgatgataccgttcatgggcgtacgaatttcgtggctcatattggcgaggaacatttcctgcgcgctgacggcctcctgtgcaaggttgtttgcattttcaatggcagcgatatagttgtttttttcggtgaagtcctgtcctatgccgcagataccgatcatttcaccttctgcattccggagcgggaatttagtaatgagaaagtgataggtcttatcgttcacggcaaaggtctgttctgattttatcctggcgcctgttgctcttacctcgcgatccaggctggtatagcgttgtacccagtcgtatggcagctctgcatctgttttgccgataatatcttttttatctgcgccgtgtatttcggtaaaccggttatttacgagcaggtatttcccgggcatatcttttatgaacatcatggatggcataaagtcgaggatagcgtccaaccgttcctggagatacattacctggtcttcgttcctttttttcttatcaatatcccttacaacgcattgaaattcctttacgcggccatcttcgccatataccagtgcgaccatttgttccacccatttttttgcgcctgatttggtaatgatttcaaattcctgggaggtatagtcgtcgcctgttttcacctggttggtgtaaaaagcttcgagccgtttccaggtatcttcttccaggaacagggaataatgtttgcctaccagttctgtattgctgtagccggtcatttcggtggcccctttgcttacgtaagtgaaggtgccatccagccgggctttatagaggattagttctgtttcttccgccagtcgcaggaaggattgttcccgtttatgcagctggttggttttctgtttcagtttcctgaacatccggtataagtaccgcgattcgcccagcagcagcaccagggtgaacaggctgatgataatggtggtccagaaggagtacagggtatagcgattgtctttatcgatccgtgcaatcagtttacgccggttttcctgcaggaaattattcacggcggctcttacgttttcccggaaccgggtgttttccggggcggtgatcagttgcctggccagtgctggttgagtggctgctattgccagtatccgttgatgataactgattttttgttggagaagggtactgaaattatccagtattttttgagagagcgtatcaccgggcatgctggcggcaacagacttcaggatgtgcagcatgctgtctggcagggcataattggcggcgggtatggtggattgccccctcagcagcatgtcacggatgctgttggtatagttgttatccagcatggctacggatcttaccttatctatcagcaggttggtttgtattatgtcttccgctgcgctcctgctcctgtttttaacgatccaggcataataaacaaagcccatgagcgccataaatactgccaggataagtaccagcactgtattcacaatttttttcatgcgaagtttttcaacggctctttaatagcattggcaggggttatgaggttggtgatggattatttattcaaaataggatattttgcggcaatattgttgttcatcttgttcaatccaacgtatggaccaggaaaagattatggtggtcaatatttctttttctgttactttcggcgtgcgaatgtaggaccgggtgaatgttttagcaatactttaacggattgtctttacaatcattccattatatttgcctaatattctttttcctaagtatgtatattatatgaagaaaataatttttaccctgggtctgatagctgtttctattggagtttttgcacaggatggtggctcaccgatgaataaggcggttaataaagttacccattccaacgactttttaatggtacagttgtcatacgatggctgggcgggtgcgcctgacagtattaagagcggccttaacaggggttttaatattgccctgatgtacgacttcccatttaagaaatccaaactgagtatggcagcagggttaggtatcagcactagcggcgtttacctgaaagatcatacgatggatatccagggaaagctgaatcctaaccaggtatctttccctacttcttcggctaaaaagaataaagtagcgaccacttacctggaaattcctattgaattaaggtatcgcagtgtgccggacaacgccaataaaggcttcaaagcggcaattggtgtaaaagtaggcgccctggtggatgctcataccaaagtaaaatataccggcgccaatggcagcaaggatattgataaagatgccaacaggggattctttaacccatggcgctttgcggcaactgcccgcgtaggttatggtaactttgccttgtttggcgcatattccctgaatccaatgctgaaagacaacgccagcaataacctggatatcagaccttaccagatcggtatttgtttaagcggattgtaacagcctacgggcttttatatagagaaaacggcccgggtttaacacctgggccgttttttattaggagataatcagagcgatctcttgttttttaccggttattcacctttgaatacaggctttcttttttcgaggaaagcctggatcccctccgcgttatcggcagagttgccggcaatttcctggcaatatgcttcatactcgagtacttcatcgaggttttccgtcatgcctttggtgagcatttttttcatgagtgcaatggctttcgtaggtgcggcagcgtagtaagcggtttccgcctgtacggcggcatccagttcggcagccggcaccactttgtttaccaggcccagttttaatgcttccgctgcgctgattttactggctttggtagccagttcaaacgcccggtggtagcccacggtgcggggcaggaaatacgaggagccggaatccagtaccagggcgatgtttacaaaaatttctatcatagtagcttcctcgctggcaatgatcacatcgcaggccagtgcaatggaacatccggcgccggccgccacgccattaagccggcagataaccggcttgggcatattgcggatagcgcgtataatggggttatagcgtttgcgcagcgattcgctcaggtcgcgctttcccgactccatagaagccttgaggtcctgtccactgctgaaagccttgccggcgcctgttaacactaccaccctcactgccggatctttttctgctttctttaatgcgtcctgtagctcatagctgagcggatcattaaacgcattgtatacttcaggcctgtttaacgtgatggtggcaataccatcctgaatatccagtaataaagcagccatgataatatggttaataagtgatttacagggtttctttcagccagttgaagaactcgcgctgccatacgatggcgttctgcggtttcagcacccagtggttttcttccgggaaatacagcagcttgcttttaatgcctttcagctgcgccagctggaaggcctgcaggccctgttcaataggaacgcggaagtcgataccaccctggatgatcagaatgggcgtattccatttattggcgtattcacttgggttgaaatgtttgtagccattggcattggcggggtcccagtaagcgccgatatcccagttggcaaaccacagttcttcggtagtaccgtaccagcttttcaggtcgaataagccatcgtgggcgataaagcttttgaagcggttttcgtgtacccctgccagcatgtatacggagtagccgccgtaactggcgcctacagcgcctaagcgggctttatccacataactttccttgctcacatcatcaatagcgctcaggtaatctttgatcggttgcccgccccagtccttgctgatagacgcattccattctacgccgtgacccggcatccctcttctgttgggggccaccacgatgtaaccctgggatgccatcagttggaaattccagcggtaggagtaaaactgcgatacggccgattgcggtccgccctggcaatacagcagggtcggatattttttagcaggatcaaaatccggcgggaagatcacccaggtaagcatatccttaccgtccgtggtttttacccagcgcttttcaattttgcacatgcctattttatcgtaagcggctttgtttacgctggtaagcggggtaacggcgcctttctgcaggtccacagtaaacagttccgctgcatggttcatatctgtgcgggacacaaccagggtgttaccggattgtgccagcatatcgttgatatcgaagtcgccggtggttacctggcgtatatgcttttccgttgtttgggcaatatttttctgcagggcaatttccagcagctgttctgtgccttttattacggccaggaaatatatctttttaccgtcgttgctgaagcgggaagaagcagcggtgccatcccagcccttggtaaggttggtgataacgccggtagcgcgatccatgatgattacatcatttttatctgcttcatagccatcgcgggccatgcttaaccaggtgaggtatttgccgtcgtggctgaaggtgggcgccacatcgtagcccatcattccttcggagagattgcgggtggctttggtatccaggttatattcgtagatatccgtattggtgctgatggcgtaatcttttccgaattttttcttacaaacataaattacacttttcccgtcgtggctccagatcatatcttcagggccaccggagggcatttgcgggcaatcgtgtggttcttccgccataatatctacgggcgtacctacttcgccattattgtaagtggcataaaaaacgtgggagaaattgccatcttcccaggtatcccagtggcggtagttcaggttatcgtagatctgcacattggatttcggaagatccgcgtagtggtcgttgccggacatcttctttatttttacttctttcgaaaacaaaatatgcttcccgtcgggagaaatgcggatgttttgcattccgccgtccacgttggttttttgcaccgggtcagatccatcggcattcatttcataccactgtcctttgagggagaaaccaattttgttgccgggtaatacggctacatctccttctgcgccgggtgtttgcgtgagttgctttgcggcgccgcctgccagcgggatcgcatagaggttcttctcgcttttgttctctgccatattgatctgagatacgccatagataacggttttgccgtcagcactcaacgcctctccactcacccgtccaagttgccatagcaattcgggtgtcatcttatcctgggctactgccatagttgatattaatagtcctgtcagtaaaaaaggtttaaacatgatatcgaaaggttgttttggatcgggtaaatgtaggaagaaatggcgtagcgattaaattctctgtaaatttgcttcaaattctgaaataacttgattgagaaaaaacaagtagtacaaaaagaggaaagagccgtcatagttggtgttattaccaaagaccagacagagcgccaggtgaatgagttcctggatgagctgatgttcctggcggaaactgcgggagctacggctgttaagcgctttacccagcggctggcgcatcccgacagggccacctttgtagggaaaggtaagctggaagaaatccagcagtttattgcaggcagggatatatcactggttatatttgatgatgagcttaccggctcacagatcgccaatattgaaaaggtgctgaaagtaaaagtgatcgaccgtagtgacctgatcctggatatcttcgcgcaccgtgcccgcacggcgcaagcaagggtgcaggtagagctggcgcagtaccagtatatcctgccacgtttgcgcggtatgtggagtcacctggaaagacaaggaggcggtatcggcagcagggggcctggtgaaacagaaattgaaacggatcgccgtattgtaaaagataaaatatcgctgctgcgtaaacgcctggaggatatcgaccgccaatcccttacccagcgtaaggaacgcggcgaatttatccgtgtggcgctggtggggtataccaacgttggcaaaagcaccctcatgaacctgctcagcaaaagtgaggtgtttgcagaaaacaaactgtttgctaccctggataccaccacccgtaaggtagtattcgatcaaacgcctttcctgctcagcgatacggtagggtttatccgtaaactgccccaccacctggtggaaagcttcaaatccacgctggatgaggtacgcgagagcgatatcctgatccatgtggtagatatttcccatccgcagtatgaagagcagattgaagtggtgaaccgcacgctgcaggaactgaaagcgtttgagaagcccaccatcatgatctttaacaagatggacctgtacgaggccaacacctttgataaatggctggagccggaaatcaaacaggatatcctgaacaccctgaaacaggactgggaaacaaaaacccaggggaattgtgtattcatttccgcattggaaaaaaggaacatcgaggaactgcgcaaaaccatcctggacaaggtaacccaattgtacaaggagcgcttcccgtataaaaccgaattcttctactaatggccaaagaatattcctggtataaattagaagaaggccgtttgccctttgcagagaaacagattagcgtaatggaggtaaatggaaaaaaaatttgctgtaccctgcaccaggggcagctttttgcctttgcatataaatgtccgcatgccggtggcattatggccgatggagtgatagatgccgccggtaatgtggtatgcccgctgcaccgttataagttcagtcttaaaaacgggtacaatagcagcggggaaggatattacctgaaaacgtatcccatagagcagcgtgaagacgggccctggctgggcatggagaaaagcggctggttctggtaaaataattatctttttgttaagagtgatcgtcgtatttgaagtaaccggtatatgcctgtaacttttcgttatgctgactacaactgttacacgctcatttgttctctctgaaaaacaagtatggctgctcatcaccgctatgctgatactattgcagtttagtgccctttttgtacccatcctggaacccgacggcgcgctgtatgccggcatcgccaaaaccatggtgattaaacacgactactggaatctttatgccgatggtcatgactggctcgacaagccccacttccctttctggatggccgctatcagcttccagctttttggtattcatacctggtcgtataaattgcccgccatcctttttttgctgatgggcgcctggtacacttaccgttttgcacttcatttatatgatgaaaaaatagcccgctgggccgtgtgtatcttacttacggccgaacatcttgttatatccaacaacgatgtacgggcagagccttatctcacgggactgattattgcggcagtgtatcatttctaccgccgtggcatcctcctgggcgccctttttacggcctttgccatcatgacgaaggggttgttcgccctggtgccggtttgcgctgctattggcggtcatttactgtttacacgcaactggaaagagctgtttcactggcgttgggcgctggcactagtactgatagcgcttttcattacaccggagctgtatgccctgtaccagcaattcgaccagcacccggagaaaattgtattcggcgctaccagcgtatcaggcatccgctttttcttctgggacagccagttcgggcgctttatgaacaccggtcccatcaagggttccggcgatccattcttcttttttcatacactcctgtgggctttccttccctggtcggtgatgctgtacgcagcggtcatcatcttcataaaaaaatggaaacagcaaaaggaatactactgcatttgcgcagccctggccacttttgcattgttttcactctcccgtttccagctgccgcactacctgaacatcatctttccgttttttgccatccttaccgcccattatattttatcgctgcaaacagaaaaaggactgaaatttttccgggttacgcagtatactatcatcatcctgatagccgttgcaggcgtagtaatcgaccttctgtacaagccggctatgcattatgcgtggctgctgctggccgccgccctgctcctgctttacctgctgctgcactactggctggataaatctacccggcaggccgtattttaccgcactctttccatcagcattctgctgaacctctacctgaacactattttatatcccgatatgatgcaataccagagcggaagtacagcggcagcctatgctaatgctcatcttcctggtaaaagcatcggcctgtatcaggcaaactcctatgcattcgacttttatttgcaggcgccggtgttacgtcctgattccgctactgcactcgtttttaccactcccgatgccgtgacttccctgcaacagcagggatatacctgcacagtgatccggtcgttcccccatttttatgtgagcaaactggatttgccatttgtccgcaaggcgacgcggacgggcgctttaggggaaaggctgctggttgcagtgaaaaaataggattgtttaacccgctatggcggccggtttctaatttttttctaaaaaaaatgaaataagattttgcaaaaatgaaaatttacctatttttgcaatcccaaatcgtgcaaacgatacgggaaacactcctccttagctcagttggttagagcatctgactgttaatcagagggtctctggttcaagtccagaagggggagcgaagaaaaagaagccttacttagtaaggcttctttcgtttatagaagtggaggttgagatatgatggaatactcttcatttcatggagcgtaccaatgaattaccctctctttttcgtatatttgacaagtgcgaaccaatccggacatagcgaaaccagcattatcccgccgtgcatattgggatattgacttgagaacgttggattttgaccgttacccagagtttaccattatcagggctatggagaggggtacatccaatgatatcagggagatatttcgttactatggaaaagataagatacgcaatattgtaactaattctgaacacttgctgccacgggcacaagtcatctcccgcagactttttcatcttcgcaatagtgatttcaaatgctctaccgacaaactacgagcgatgaacttttcgaagttttaatcaaactaatgaacattgccgatctttccgactttaggttggttggaggtacggcattaagcttattaagagggcatcgggaatctgtcgatattgatatgttctgtgatggtccttacggacaaattccttttgatcatattttgaaggtgatcaacttaaatttcccctatgtagaggaaatcaatgctattattggcccctctaatgaagtcaataaccaggggctttacctttttctgggcgaagatgagcagtgcagtattaagacagacattctttactgggatgctccgtttttgtatccggtagttgaagaacaaggtgtccggatggcaactattgaagatatagcagcaatgaagctggacgcgatttcacggggcggacgaaaaaaggatttttgggatctgtcggaaatactggagacacatacaatgacacaactactggagatctacgagaagaaatatccctggttcgaaataagagatgtcatcgttggtttaacaaacttctcagtagcggatataatgccggaccctgtgtgcttcaagaataaaaattgggaagaaattaagtcggaaatggtgagggcagtaagtatataacgttacgtaacaatatcagctaattctatattataccctttgaaaaaaatgggctgacccgaaagcatttcgcttcctgatcggcccattttatataaaagccttaattatacttcagcttaatcgtcaccttccaaatcccttctttcagaatagacatatcaaaccagtaattgaaatagtcgccgttgatttcaccattgttatacatatcaattctcagcacctgccctgctacgaaaggcagcggaaaccccgctatttcgagttccaggtgatccgggaattccgtgtatttggtaggattgttcaggcccaggttatgccagtcttttaaatctgttacgccgggggtactggaatagtcgtatccgaataataatttcgggtcaaccgcggagccatcttttttcaatacgtacaccagtattttgttgccggtatttacctggcgctcaaatgttacatcgatgccggtgagtttaccgtcgatgccggagaaccggtaggtatagggcaaagcgtagctcacgtctattgtcagcgcagcttttatcaccctttcaccggagctgttctttactttcacatctatggtgtatttcccttttgtaagcagtaaagtatcggtcgcttcggggtatatcacaatgttgccattctccgggttgatgtctattgccgggcgatttaccttttgacgtttggtatccagttcctgcaccgttttttctttcccggtgtattccgcctgccagaagtaggtatctactttgtagcccattactttatcggcgcgcttgccatcctccgtgtaaatgccgtcgatggtgaattccagcggcttggtggattcatcggttaccatggcgccggattgaatcagcgacgcgcctacggctactttaatggaaggattggtatatttcagcgccggacttaaaaagccgtcgctgctgtctttggtgcatgatatagcgaacagggtgacagccagccatagtatgcacgttatttttattgatattttcatgataaaaaatagttaggattatctgaaatatttctgcttcaatccggcagcgaaactggagccgtaggttaatacatgtactactgcattggcggtaatcatgttgtgcgtttggacactaccggtatatttgacggagtccatacctggtatttttacatgctgatactccacgtagaacgcggatgtttgtaaagaactgccggcacttacaccacctcctttgccataaataaacaggctgtcgccgttgagggctttgtaaaatttcgatttatcttttaaggcttgttccagtgttatttttacattagggatgatgaacctgccgagtaatttcagcaaggtatctttcccgatgttttccagtggtcttagcgcctgccggtcgtcggggttgaagttcatttgcagccgcatcacggcgttgttaggcgctgcgaaaaaagtgatgttggactggtttacgatcgacttggcatctgtgaggtcaatgattttaaccagggaatcgaacatgtggttggacctgcttttcaggaaatcgtatacgggcatgttcttttcggcttcagattgctgtgagaggccaccatccacgtaatagtcatttttcctgcacgacgccagtacaagcacggcgcctgctgcaaggagtatagctgtttttaacgaagtaagtttgttcatactatatctttatcaagaaatgggagtaattatttccagaactcattctgtgtaatcatgaaattgcttttggcaatgataccctggtcgattggtaacagccatgcgccttttttgaaccagtcgccatccgtaattttcgaatccttatccagctttcttgttcttaccaggtcaaagaaatattgcccttctccaagcagctcttttttacgttcaagcaggatggtatcctgcaggtttcctccgccggtataaggtgtggcaaatgcgcgctcccgtactttattaagaagtacaatggcttctgctgttcggccaactgccggggtggcgagggcttctgcccgcagcagcataatatccggcaggcgggtgataataatgttagactcgttgatgttctgggtagaagtatcaccttttaactgtaaggttctgtattttcccaggaagatgcggtcttcgttcacgccctgcaggtaggtttcgcggataaaccaggtaaataaccgcgcatcccgcgcgccgggtgtgaacatcacattgatctgttgcctggtagggcacagtaagtaacggtcgcttccgccgccgccatcggattggtctttgtaccagggccttcccaatgttctgttgtatacgcggttcttttgtacttctcttaaattggcatcgaagttaaactcaaagatgccttccgtcgatttgccaataaaaatgctgaggagattggtggtatctgtaaccaaactataagggcctttggtgattacgctgtcgcataatttctcgcagccggcaaagtcctgcaaccagcccagcacatgtgccttgatagcccaggccgcgcccctgcttgctcttacggccttgtcgccgtcgccatagtccagttccaggttgctgatggctacatccaggtctgctttgatctggttgaatacatctgcctgcggcgttctggataaattatccgtgttcacgcttttcaggttcagcggtacatctccccaaaaacgaaccaggtaaaagtaagtgagcgcccttataaagctggcttctccaatatgtcttttccgcagtgactcatcgtaggaagtaatcgccgggatcttttccagcagcaggttacattgtgcaatagcagtatagaactggttccagttgccgccaccgttattgaataaagcggatgccgtattggtagcgatgttggtttctacgcgtacgttcgaactttgcgagtaactggaaaatacatctgcacgcacgtcgcccatgaggaagattttatccggcactactgtgcgaagcagcgagtaggcactggcgatgcctttctcaacatcggaagatgaggtgatggcattggcagcggtaggaagttctatgatctccgggtcgagtatttttttacaggaaaataataatgcgagggaggccagtagcacgcacacaattttgtttttccgggtagttattattttcatatgcttagaattcaaagtttaagccgcagttgaatttgtaggggattggataaccgttgcccaggtcatatccgtatggatccacgttttccggatccacgccggtatattttgtaagaatgaacacgttgctcatgcctccgtatacgcgcagccggcggatgtttatccggttgagcaatgcagtggagaagtcgtagctgaggttcacattattcaaccggataaagcttccatcttccaggaacatgtcggtattgatttcgtagttgcctataaaatcataactcgacgtaccataatatctccagggatttagcacgggatatttggcattggtgtgttccggcgtccagaaatccaggtcggaaacatccagcaggtttctttgtccgccgggatagtttacgttttcactggcggtccagcttactccgcggatacggtcggcttttactttgttgaataccttgttgccgacagaatagttgaaaaatacatccagctggaggttggagttgtttttaaatttatagctgaagctatgggagaaacttccggtaaacttaggattcggatcgccgctgtataccctgtctgagttatccagcacgcctatcctgccatccccgtttacatccagtatccggatgtcgccggcgtggtaagggtcttgtgaggagaaaccgctaacgttcgggaacaattttttgccggtatatttattaacaggaacggatgcatcatcgggatacacgcccaggtatttcatcaggtagaagccattcaacgggcggcctatttgcaggtaaggctggccaacagcataattgctcctggacacgcttctgccgaaatcaggaagtttggtcagctcatttttgttgatggcgccaataaaggttactgaatactggaagtttttgccgggtttggtgatgtacccggtgatagctgcttcatagccatagttacgtacggcgccgctattaatataccgtgatgcgtatccgctggtaccgttcaatgcatcggggaacaggaaaccatcggtttttttatcgtaataatccagcaccatggtgatgcggctattcaggaattcaagatccagtcctatgccgcggtcttttgtagtttgccaggtgaggttaggtaatgcaatcccgttgccgccgccatagttaggcgatagcaatggaataccgttgtaggtagcattgtcgccgcttttagtaagataagcgcctacagcgaggtagttgtcttcatactgcgtaccggatttccccatgctggcacggatctttccgaaatttaaccagcggccgatattattgcggacaaatttctcttctgtaaatacccatcctgccgaagcagaagggaaataaccccattggttatccttgccgaacttggaagaaccatcggcacgtactactgcctggagcaggtatttcctgttgtagttataagacagcctggagtaatacgacagcaacccatattgaagattatgcgtttcgagtttaagatttgcctgcgggtagccgagtatcacctgttgcgcatcacttggaccgccggtggcagcaccgtaaatgttattgttttcgctggtgttaatggtgttacctaatacaaggtcaaaggaatgttttgattcaaacgtatggtataaacggagaaatgtttcgctaagcagatttactttttcctgtgaataataagaggcggctgctttcagatcattcctggtggcagaaggctcaaatgtccgcgtgcggtaaaattcatagttgccggatgcgcgggaagtaatgttgaggaatttaaaaacatcataacttacttccagttgcgccagggctctcctggtgaggtcgatgttcactcctttgttgtaagattcgaggaaggcatcaaaaaatccgctgctggggcccggacgaaaggacgacgaaaagttattgcctactacggcggcattataggtatcacctcttttctggctcgcatctgtttggctcaggttggcccggccggttacggttaatttcgacgttggcttaaatatgccgttgtacgtcagtgaaaaacgggagaagtccgaaccgagaacaatacctttctctttataataatccacacctaagcggtagctggcgttttccgtggctccgctgataccgaggttgatattcttcagatccgcatcacggaaatataacttctgccagtcggtggagttgttataaaagctgttcaggctatctgatagctcaatgggcagatcggtataaccgccacctactttagaggatttgtattgattgtacagtgcaatcttgaaatcgcgttctgctttaccgcctaatgttttacgaagggacggataatagctcaggccatattgtgtatttaaggatacaataggcttaccgatttttccgcgtttggtattgatgatgataacgccgttcgcgcctctcgatccatagatagcggtggcagaagcatctttcaatacatccacggactccaggtcgaaggggctgaagccagccagtacgctggtaatggcctggcgcgggtcggaaggattaaaaacatcctgttcaagcggtacgccatcaataataaagagcggcgtacttactacgccggagttggcggagttggaaaatgaagccagtcccctgatctgcaccatacttctgccgccgggcataccggaattattctgtaccaccagcccgggagccaaaccctgcagcagtccttctatagagccggacggtttattttgcagctgcgatcctttgatggtggatatcgcggaagttgtttcccttcttttctgtgttccgtatccaacggttacattcacttcctggagctgggaggcggaaggctgcagtgtgatcagcaggttttgcagggtgtttctcaccagctgacttttaaactctttaccggcagtggttagcacgccgtcgtttaagcggagcagcagggtgttgaaaccaattgatgaaataacgatggtggcatcttcaggaacgccgttgagtgtaaacttaccattttcatctgcggtagcgccttgccgggagccctgtactatcacggtggcgccaatgattggctggttgtcggggctcaggattttacctgacaacgatacaacggcggcctgtccctggcgggaagagagtaccgtcacaattttatcgtttatttcaaaagtgaatggctgatctttaaatacttcctccagtgctttctgaagcggcgcttctttgatattaacggttaccggcaaagcgttccggttaaaccgggcatcgaaaacaaaggaataattcgtttgggctctgatggaagcgagcacctgttcaagcctggcatcggtaacccgcaggcttacctgctgtgagaaaacagcagcggctgttgccagggaatagaaggccgcaagcattaggctgcaggcataacgcttccaatggcccacaaagtggccacgtttaatttccataaatgtgattttaaaggattgactgttggttgataaaaaaaacggtattaatgcgcggttaatacccggttattgctcatttttagttttatgtcacttgttttctctatagctctcagtaattgtaacagtggtgtactgcggggcagctgcccatataattttgcgtttggaagggatgaataatccacttcaatatcataccagcgctgcagttggtgtgcaacagcgtgaaggtcggtgtctgaaaaataaaacatgtcagacatccaggagatatcttccctggtatctgttttcctgatttgcagctggttattctccagtatggcctgttctccaggattaagcaactttgcttccgttccattcctgggatcaatctttatgcggccttctaccagggtagttttaatataagattcatcggcatatgctttcacgttgaaagccgtgcccagtacagcaataacctgctttcccgttactactacaaatggttggccggcatctttggcgatatcaaaatatgcctcaccggttagttctaccttgcgctgaccatcgctgaaaatggtaggatagcgaagggacgaagcggcatttaaagaaacccgtgtaccgtccggaagtatgatcttatagtactttccccgcggcgtggtaagggtattaaatacaatctccggctgcgctgcatcgttttctgttggcctggcataggtaagcgctccttttccactgttcactgcgtggatgcccttttgctcaattatttgttctgttgcggcactgtcgagggctacctgtctgccgtcagacaaagtaagcattacatgtgccttagcaggtggttgcggtgttatttgcgccatttccctgttggcctttactggtggcgcgggcctgtaaaataaatggtaggaagccagccctaataacaacgttacagccgcggcggctgtccatgtaagtgttggcctcaacttaaatatactactgcggttgccgggctcattcaccttgttaatgcggtccagtaaagcgtcggcttgctgtggtgaaaacaagtcctcctgcggggttgtttgcctggcgccccagtcaaacagttgatgataaagctcctttgcctcaggatctgccagtaaaacaagcagctcttcccgttcttcttcggaaatgctgttgttaacggctttttggtataagtatattaacctgtcttcctgcataatagcggcttaaagtaggtgcccaatatataagacagtaaagggggcgtaaaaggagatatggagatgaaaaatttatttgaacaaccggatagccagcagggacaagaaaattgtttccctcactttcatataccggtaaataaatttaatcgcaagctggttatatttctttacagaatcggtggacaaattcatccggtgggcaatttccgggttccggtacccctgcgcccgcaacaggaaaactgttttctgctgcatgggtagcgcgtcgatagccttatccagcatatcgaggcggttatcaggatagcctggcgccttatcttcctgcttttgggcaaagagcgcatactgctcctgcttctttctttccgccaccaggcttgtcaggtaattaagggtatgatttcgaagaagaataaaaaggtaagcgttgaactgttttaccgaagtgagtttttcccggtctttccacagctttataaagatgtcctgcaaaatttcttctgtttgttccatggagccaacaatcgtataaacaatacgcccggcctgatttacatagccgtgaaaaagcctggcaaatgcttgctggctgccgccggcaatttgcgtcagtatttcttcttcattgtcgatactttttaaccccatgattttatttacagaattggttgatatttttcaggcaaaaaagggagtgagacaatattaagtatttcatataatatttccatatgcaattttagcaaagaaagatggtaagttgaccgaaactactatcgggcagtccccttcctccgtaggcgatttctacatcacccaataaaaatcaatataacctgcacatttaatcaaatatttaactagatttgccgccgatgttcacaaaaaggtgagcatctataagacatcttcatctgaatgggcttatagtcatattcctccttagctcagttggttagagcatctgactgttaatcagagggtcgctggttcaagtccagcagggggagcaaaaaagcctggtaattttaccaggctttttttattggaagcagtgccattgcacgcccactcacgaaggattttctttaacttccggattaacaatcgttccataatggataaaagcagcaaatttatagcggtagaaggtttagatggcgcagggaaatcaacgcagatagacctgctgacgaaatacctcgagtctaaaaatgagaagaccaggtttgtacatttcccgcggagcaaccagggcatgtttggggaactcatcgctaaattcctgcgtggtgaatttggcgacgtgaaaaacgtgcacccacagctggtagccctgttgtttgctgaagaccggaaagaatttgccaccaccatcaaccaatggctgagcgatggttattttgtactggtagacaggtacgtgctgtcaaacattgctttccaatgcgctaaactccataccaacgaagaaaaacaatacctgcgcaactggatcaatgaatttgaatacaactataataaaatccccaagccacatttctccatttacctcgatgtaccgttttcgttcaccgagtcggcgctgactaaaagacgcgcaaacgaagaccgggaatacctccagggaaaagatgatatccatgaagcggacttctccctgcagctggccgtgaaaaaagaatatgatgcactgttggtagccgataaaactattaacaggatcacctgctataatgaagcggcacaaatgcgcccgatacgggaaatccacgaagaaattattcagctggtcaacagccaggtgcagttataagatcccccctttcgtgtagccatccccgctagcatctccccaaaaatatttttaccggctgtaagtaattaccggttgtatacctgtcctcgtatgtgagcacctgcgcaaaacccggttccactgttatgagcgcgcaggctcatcccctattgagttatacggctttatatacgactggctgagcacattgaaaacctgatatctttttattccacaaaactgaaaaacatgaaaactcaaacacttttccgcagcacctgcatggcagtgctcctcctggcatttatggttaccggctgtaagaagccggaaatgatcaaatcttccgaaaatacccccgaaggcactgcttccggcctggtggcaattaactccgttcaacccgtaaaatctgaagcgctgctggcaatgcaatgctacaacaacgcattttatcatcagtacggctcctatggcccgtcgtttaaagcctattactattcagatgtaaaccaaaccggccggatggatttctggcggcaggcagaagccatcgaaaccctgattgatgcatacaatatcaacaacgatgcagacctcaaaaacaaaatggtgtacctgtacaacggtatgcgcgatgcctatggcctgctctggacctccaacatctacaacgacgacgtgatctggggcgcattaatgtgcatccgtgccttccagatcaccaacgacggcggcatgaaagatatggccaaaaacaatttcgatatggtgtggaaccgcgcatgggacaccaacctgggcggcggcctgtggtggaccaccgccaacaataccaaaaatgcctgcgtaaatgcgcccgccgccatttgcgctatgtatctctaccaggctaccggcgacgcgacctataaaaccaaagccaaacaaatcgtcgactggatggtcactaagttgtatgtacccggcaccggcgaggtgaaaggcgccatgaacgctgccggcgtaattaccgaaggcgcccgtacctatacccagggtacttttatcggcgcctgtagcatgctccataactcctacccctccaataactacaaggcaatgggggctaaagccatggactatacgaaaatcagtatgtgcaacgcacagggcctgctgccggatgaatatgacaacgaagactgccagggcttcaaagccatctttgcccgctgggcctgcaggtttgtaaaggaccatagctaccagggtacttatgcctcctggcttaactacaacgccgcggaggcatggaactaccgtaactccaatggtcttatgtggggccagtggtggcacagaaccccggataactacgtgaactcgtttgaaactacctgcggcgtggctatgatgaatggcgtctggctgttttaattccccggcttttgtttttcttccgggagataattaatttgtgtgaaataaacctatatctaacggttatgatgaacacaaaaagaatcgcactgctgctgctcgtaatattttcaggcatcatcacacaggcgcaatccctggaggatatcgttaataaaaacgtggcggcactcggcggcgccgataagttgaaaacactgaaaacccagtatgcagagggtaccatggaaatgcagggaatgaattttcccttcaaaagatgggtattgcaggacaaagccatgcgcctggaatttacagcaatgggtaccaccaatatccaggtattaaccgatgccggcggttggatgcagatgccggtaatgggtaaaactaatccggaagatatggactccgccaccattaaggcgttgggcaaacaactggatctgaccggtgatttttaccgctataatgagaaaggtaacaaactggagctgctgcccgccgacacagtgaatggcgctaaacttgccaaagtgaaagttacctacaccaacggcaacgccactacctgctttgtagatcctgtaacgggtaatgtgttgagaacatccaattcgctggaaatccagggacaacagatggacctggtaacagacatcagcaatttcctgaaaacggcggatggctataactatggtaccgctatttcacaggaaccagtaggtataaagatcagcattaccaaactggaaaataatgtaccagtggatgaaagcatcttcaaaaagccataaaagtaaaaggctggtctttgcggaccagcctttcttattttgtaagtaatgattccagcaactttatctttttaagatccggcttcgtagtaaatattccctgcccgctcacattcctgaccccgcgtacaaagcaatagataacgcctccaaactgcttctcataattaaagccaggaatccggctttccaggtatttttttaccgctaccgtataaatgaagtactggagatggtaattgttttcgttcatcgctgccgctaaacccgccgcatcgtagtcggccacactgttgcccaggtaattcgatttccagtcgaggatataatacttcccctggtgctcaaagaacaggtctattttcccattcataatgccttccagctcctggctgctgtattctgaaaaccgttttacgcttatgcttacctggtcgtctgaaagattattgagcaggttcgacttaaacaccggcaccgggaaatcaaattcaaattctgccagccgctgctgccgccctaccgctgccagctggaaactggcgccatcgatatgtattgtagagtacatcacatgttgcagcatttcgtgtagccgttcgagatatacctcccgctggccgggcacaaatttccggatggcttcttccagccagtgttcccatttactgctatcggagaagttgatgctttcaaagacgaagtgcagcaggttaccggttttagcgcctctgcgcagggtggtaaatataaagttatcgtaagggtcggcttgctggaaggagcgcacccgtggctggtgttccggctttgccgccagcatggtatagctcatcttccgccagttttgttctttcaattgaaaggataccggcgcgaggctcactgccagctggcctttgtggagctgctggcgatagctttctgccggcgtttcgggtacggggccctgcagctgtatcagggaggcatccggcgcttcggccgccagtgctttcaggaaaaccgacagcgacgaatctttaaaagcgtgataacagtttttaaagagataacatttatatactgcgcgggtaatggctacatatatcaggcggcggttttcctgttcctgctggtgctgataggcttttaactgctcttccgtgagcagggctttttgtgtgcccaggtaatcgccggttgccggatcacggaaactcacaaattcaattttcgatttctctacaaaatccaggaaaggcgccatcactattttgtattccagccctttacttttatggatggttactatgttcacggcatcttcatcactttccacgcgctgtgcatattcatctccatcggtggtcatgccgtcgatgccgcgtttgagccaggagataagatcgcgcatggaaaggtttttccggctttgcacctggtgtaccagttctgatagctggtacaggttggtgatgatccgttcgccgttttcagtgtggccatcgagcaatacctggcgcacgctgaaatctgcaataaactccatgagcgccgtgtacgcgccatcgcgctgccataaggtgcggtacttggcaaacaggtccagcatggtttcatcgtccagttgcaggatggtttgactgttgtagccggtaaatgaaccgagcaatgcgcggttaatagatgagcggtccggtgtttccatcgcttccagcaggtgcagtaattgctgtgcctccgcggacctcagcaccctggcttcgtcgatggtaacggccgggatgcccaacttcgccagggcatgtttaatgtccctgccttcctgccctgtgcgcacgagaataccaatgtctgacggaacgatggagcgggagccctctttattttctatgcggtaatccttattcagcagcagctgcgcaatttgcgcggctacgctgttgcagatggtttcttttttatcgcaggcaattacttcaataggtgtatccggtgtattgcctttatagagatagcctttcttattattatcaggactgtgtacttctatatagtcaatgctgtcgctttcctccgtgaaatcaaatgttggaaagtccggggtgggtttaaagaatacgttcatggcacggatcatgttttccgacgagcggaaattctggttcatgtcgtaaacatgttgtaccccgttgcgggcattgaaataggtaaatatgtcggctttgcgccaggcgtaaatactctgcttgggatcaccgatgtagaacaggatcgtgttctggccgaaggcccgatcgaatatttcaaactgttctttatcggtgtcctggaactcatccacaaaaacggccttgtatttattttgcagggaagcgatcagttcttcgttgttattctttactaaagcggtatgcaggttattgatcaggtcatcatagcccatcatgttgctgcgctctttgaaggcgcgtacctgttcgctgatttccttgatggcggcataatacacctgccggcggatcaattgttgatgctccagcagttgtttgctgatttcatctgcctggtcaattgccggtaataagtctgcaaaaactttctcaatgtatttggcgctgcttcttttactccggatcctttttaccagcagctccggttgggaaatcagttcaggccattctttccgggtattatgattggtagcgcaggctgcggtaagatgcgcgttgttggcagtaatgtatgcatacaacgcttcgttggcggcctgttcttttgccgttaactgctgtagctcctgcatccattgttcctgcagggtttcgctgatatcgtcgggagtatcttcccggtagtccaggaatttctttccgctgagatgttctttgatcacgttgagcatctccgttttcatgtcctcatcccagatctgttccagcagggcagcgttgagcgtggttacactcctgcgccagaatttattcagttcgttttcaataaccggcgtgagatcaggtaccatggtggcgccaaacagctggttggtttcaaacgcaaattcattcagtgtttgctggcaaaagccatggatggtaagtacagccgtttcatcgagcaacaggatggcgtcgcgcaacagctgctgcacggggcgcggatcatcgaagtcgattacgctgaacaccaggtccataattttctgatcgctgatttcctgtccacggcttactttgtacgcctgccggataaacagccggatcctttcttccagttctgctaccgccgcgcgggtaaaggtaaccatcaggatttctttgacagacagcttttgctccagtatcaaccgtaaaaccagtatggcgatggagtacgttttaccggtgccggcgctggcctcaatgaggttgctgccttccagcggaacggtgcctgcgtcaaactgtttatatataatgctatcgatcatttctctttatcgggtgtttctaaataagccggcagcagggttgttaacggcaatatcagcagctcataaatatcgaggtagccggttaatgcttcttctttctcaaaaaatccctgctcatatacctgcacgagatacgggtccggcgattcctgccggtcgatcatcccggatattttatccctgaactttttaaggtccatggagagccaatctttttccgtgatttccaggtcggggtaaaaggatattattttgctgaagcccgtcttataaacttttacaatttccgttaatctcctcaatgcctcttcagatgttaatgggatcgcctggaaagcatcttcttttttagcgccggaaatatagcagaggtctgttaccacgcctgccgcttttcctgcgagataacggagataggcctctaccaggtatttgctctctttttttgaccacgacacctgcaccagggtttgatcaaagattcgcagatttcctttcagcatgctgttatctaccggtaattcaacggtaatccgtttttcttccgcgcctttggtaacggcttcgtacaggctgcgcacgggtactaccatttcttccattttttgaatagaaacggtagccatattgcggagcggaagtttgcctttttttaccagcgtggtttgcagcgcattctttttatcgccggcagccggcagcagttcatttttaacagaccattgctgcagcctgttgagaccaaagatctccgtttcgctgagcagcagctggctgtcgttataccggatgcccagtactttattataataagcccggaaaggatttttaaagaagctgatcagttcttccagggtaatttcttcgaaggttaagggagtagtaattttattttcgttgagatatgtttttttgccggtatccttattgctcagataggaaaaaagacggttatctgtaccggcatatttcctgctgaagctttgtaaaggttgcaaggtaaccagttcgctgcgcacggtttccggggctgctgtaccagcttctatatagtctaccagttcgtctaccagcacggatggcggaagatcggtattatcctttgcatctttcccgatatagctgatatacaggtattcttttgctgaaagcagggtttcgaggaacaggtgcttatcattttccttcacattacggtcgcctttttgccggtctttttccatgaggttaaagctcgacttattttcacgacggggaaacttattgtagttcagtcccatcagcgccaccactttaaaggggatactgcgcatcggaatgagcgagcagaaagtgacgccgccgtttacgaacaatcctgcgcgggtgctgccggtaagcgtgtccaggaagctgtggctaaacacttcgaaggttactttttcgctcataaattcgttcagcgcgttgtaggcggtgagctgtttgatgagggtgttataatcttcgtcgatatcatctactggttcgtacacgatattatgcaataccctttcggtataggcaacccactccacaatggtgcgtgggcgccgcctgtcgaggatagacgacatgagcacttctgcaaaatggcagaagcggatcacatcgtgcgcgtcgctgccttcggtaatatccaacgggaagaagctgtcttccccgaggccgtattcttcttccccactcatgcaaataccaaacataatgcgttggataccgtattgccagctcacgaaatgcgtttcttcctttttgctgccgttgatgccgaagcggatattggcggcctcaataatccggcggatcagcaccgggtcctggaggttaaagcgtttgcggatataggagaagtcgagcagctgcatcacggcttccgatttgaagttttcctcattcatggtgaggaccgcatgcagggcgttaaagagattgtcgttgtcggtgtaactttcatccgcaatcgtataccggaaggtataaggcgcgttgttgaaaacggctttgatatagggcgcataggcatctatatcgcttaccattaccacgatgtcgcggggcgataaggcttctttccgttgcgctaccaggtgtaccaggtagttgtagagcacttccacttcgcgggctacggtgtagcaggcgttgatggtaatggagccgtcgcggatatcctgcggtgtgatcagctgccggtcggccgtggtggctgccgcggtgaagatatcgtattgtattttatgcaggagactatccggttccggttccacggtatcaatttcttcgtacgcgttgatgaaggcatcgtatgcaaagaagaggccgaagctgtcctgtattacccgtccccagccggtgaggagggcgttgcctgctttggagtcctggatatctttgagacctttttgccgccagcgggccagttgtttttcgttgcggtcgtcgaaccagaatacaaccggagaagggttgatgatatgaaaatgcacgtctataaaagacgacagttcgtgcaatatttttacgtgataagcggtgatgatggataagccaaacaggtgtacgaccggcatgcgggtgagcagtcctgttttcgggctgttgctgcggagggcgtcgaggataaaattccctacgatggttttatccggaagcgagccgccggagagttgttttacttttacccacagccagtgttgccatccggcggtggccagttcgggggtatcggtaaaggtccatgcctggatcatttccgggcggtacacctggtactggtcaaacagatcggctactttttctgcgagggccatacgtttcaggtcactttccgtttcatcggccgtatagtaggcggcaactttcgggtatttggcgatgaactcttcctggccgagcagtttaaataccagccagctgaggttttgcggcgacagcacttctgaatgcggccctcccagcactacgtacagctggtagagcaggtcgttgggctttaggaagcggcagttggctgcaatgcccaggtggctggccagctggagtttcagccagttgttcatcccttccgtttgggtaatgatatagtgaggctggaacacactgttgcctgcatcgcggaggttttgggccagtccggatgataaactgttcagtgagttcgaaacttttaaaaacaatgccattgataagtcctttgtttgcactccgccattcccgaagcaggtgatttaatttgcagctgcattcacttccctgaacctcgaggcgatgccggaggccctttccacgaagcgttctgctgccatgagtattacctccggcgttccctgtacatacactttattttttgcacggcttacagcggtatacaacagctccctggtgagaatgggtacatcggtggtatccggcaacaataccagtacttctccgaattcggagccctggcttttatggatggtcatggcaaaggcggtttccgcctgggttaaatagccgggcagcacggcttttaaggcgccggtgctgtcttcaaaccaagccatgagcacgccattttcatctgcacgaatgatgccggtatcgccattgaacaagccatgttcataatagttacgggtaaggatcaccggccggttttcatagaattccccattggcggtgatgagttttttatcgaataaatatttttctatttgtttgtttacggcgtaaagtccctgcggcccttcccttacggcagagagtacacgctgcgcgttcaggagcttgagcgcggccgcgatatccttttctgcgatgaaagcggcgtagccggcaatgaagtcttcgaacagcggtaccgaagcatccgggtcaacgactacctgttcatctgccgaaggcggaaaaaaagaagttattaccggtacattattactgatgatagccttactgaatttaccaatgcctttgtcgccggtgaaacggtgactgcgccgcagttccacgagatgctggaacaacgggtgatgatcatcgttttgttctgctgctgcgggaatctgccggttttgttccggtataaaactattgatcagctgccggcggccggaagtaaagcggttcaggtgttcctgtgcctggcagaggtctccgaacaggctgcctgcttccacggaggccagctggtctttgtcgcccagcaaaataaggcgcgtatccggatggatggcgtccagcagtttggcaaacagggccacatctatcatggagcactcatcgatgatcactacatcgtagttgagcgggttatctttattgtgcctgaaatacgggctgccattaacagacttcagcaaacggtgtatggtagccggttgcagctgcccgaacttttcagagatgggcgcatctacttcgatagtagtattacgcaggctttccgccatacgggcggcggctttaccggtgggcgctgccagcgctactttcaacgccggatcggtggcaaacaggatggccagtattttagcgacggtagtggttttcccggtaccgggaccgccggtgatgatggtaaaattgttcagcaccccggtgatggcggcggccagctgccagtcggccggatcgttattatcattgctgccggtggcggcaaatagtttactgatcagcggttgctgttgttgcaacagggcaatcctttcaggcaattgtgttttttcctttaccaggaattgtcggatactttgaaggaatgcggtttcataccggaaatagcgttgcaggtacagccggttctggtaaattacaaagggctgtttatcgttgccctccgtacctaccagtggaatactttccagcaattgattgctggtttctattttctggtaggattccgggagattttctttttctgcggctattttatcgagatgaagacagatgtgcccttcactgcctttctttgataacagataagcgtacggtttcagcgccggtatatcaaaatactcggcaaattgctggtgtacatcattcagggtgggtatgtttcgcattcttatctggacacttgaaaagattaaagtacaactttttctgcttcccctgaaacactatatattgtagggattctaaacctatttctatacactatgacaaagaaattgctaacccttagcaccgtttttttatttgtttgtttgcatgccagcgctcaggaagatctctggagaaaaccaggtcagctgaaagcaaatatttccctggtgggtgctaatgtaaattacgaattgcgtttgttaaaatatgcgacccttaacctggaagcgggaattgaaatgggagtttcctattctaatggtagctatttaggagaagaatgggagtttgcgctttacccggttttttcggcggagttcaggcagtactatggtattgcccggcgggctgagcggaataagcggatagataacaatgccgggaattttttcagtttcacgggaggttaccagggcagtcctattacgactacggactattattctccccgaggcacggctgtttttacaccagcgtggggaatgcagcgcagttggggccgtcatttcagttttgaagcccgcttcggcgtttcctttgtgccggacgatggttatagtaattcggtgtatcccagtgcacgcatcaactttggctatgtaattttgtaaattagctgcttaaacagtgagatatgtcatccaggatagttaagcaggtaatagtgatgcgcaaggatttgaatatgcgcaagggaaaaatgattgcacaaggcgcccatgcttccattgcttttttgacgcgccatgctaccatcgacgggcatacgctgcaaaccaatatcaggaatccggaagaggtgtcggagtggatgacgaaaggttttacaaagatttgtttgtcggtagattctgaagaagacctggaaagggtataccaacaggcggtggaagatggtttgaatgccacgttgattacagattcggggttaacagaatttggtggtgtgcccaccaaaacctgttgtgccatcgggcctaattcaaatgaggagatagaccggatcacgaaggatctgaagttgctttagtcttcgtctcctaccacatccgtttctacaaccctgcctacctgtccgtcttccagccgtactttgataccgcgggaatgataagcagcagaggtgagcagatcctttacaatgccgtaggtttttttaccgctgcgttgatcttttttcaggatgatggccacttccaggccagggtagatatcttttctatattgtccgtccataattgcaaagctacagattttataaaaacggtggatcatatgctgacccaccgttttttatttagggatgaagatttgccgcagctgatctatcagtacaccgtttccactgacgctgatactgttgatcttttccgcgattttttccacatactccatttccttcaatttaaacagcatgggattgtcttccatgagtttggcggtattgagcaggctcctggtgctggcagtttcttcccttcgcatgatgatattggcttgtgctttcttttcggctaccagtacctggttcatgatgtctttcacatcacctggcaggatgatatcccggataccgaagctggtcacgttaatgccgagaacttccgcctttgcgcttactgctttcagtatagctggcgccagggtatctttcttttcaagcaattcatcgaagttcaggacggcgatgtattcccgcaaagccagctggaactgtacatacagctgccgttcgtattccttgttttgtaacacggctttattgatatctgtaacccggtactgtgcccatgcgttgattcgcagtgctgctttgtctttggtcaggatttcctgtccatttacttccacctgcaactgccgggtatctattttactaacggtgatagtgatgttattcttccaccagcaataaacgcctgggtacagggtcatggcatacttaccatctaccagcatcacggcctgttcgtggttttccacgctgaaggttcttacgtaaggcgctaccagccggtggcacaaggtagaccggtctatattttcagtgatcgctattttagcgatatctgcgcgaacaaatttgttgtcgatgatatttttccagaaggcatatctgccggcggtcaatacctgcttcagtaatccattttcgtagtgcagcacaatttctgtttcttttacttccactacctgcaatgcgttggtgacgtctgcatcctgcaggaggatgttcagttctaccggcgcgatgaatggcttgttgatatcgtagatggttacatcttcgttgatcagccagtggcggcctaccggcagcattcgctggtaaacgccgtttttaaaaaccaggcctctttcgtaggcgttgatggtaactcttttcattttctttcatttgggggtgttgataaataaagccagtgctgttgcccggatgatgaacacggaaaaccaggtgttgatcagtgcttattcatcagttagggcggaagtgctaagtgatgataaggggctgatgtagtccttgtttgcaggtgtttaccctcctgcggcatcatccttttgatgaggcggcggggcggtgagccctggctttgtttgttgttgtaaaggatttacagtccttctgtgattgtctattgctctaaccgatgagctaccgtttttcaaggacggaaaggattcgaaccttctacccatagattctatggcgggaacagtgttttgcggcaacagcatacagttcgttattacggctgcactgcggagtagtatgatactcctgcctgggttgctttgaagaacatctgttcccgtcttcctgttgaggaagcttttttagcaaatgctttccatttgcggggtggatgaagcaggagtcgaacctgcacgggcggtgcttcaaaccgctgctctaccattggagctattcatccggttagtgagtagctatgctgcttacgcacctattttgtaaccctgattggactcgaaccaataaccttctgctccaaatgcagacgcgctaaccaattgtgccacagggctttttgtgtagtccggattggatttgaaccaatagccagctgcgtataaggcaggtgctctgaccgttgagctaccggactgttttgcgtctgtgctgctgcggcggctcttatcgggcataaaaaaaccgggcgttcagcacgaccggtttctacgtatatacataagcgttacttatgttcgccgacaccggtgtcgttgatgaaatatttcatagcgatagcaaaccgataacaatggtttgttatgatcgttactaaattgtatgttatgagtatgcatttgcatgcgcattttagttttttagtacaaataaaaagccccgcaatctcttgcggggcctgtgttatatcgaattcgttatttcaacttattcttcagcataacatgccccgccactggtatagcctggtatcagactaaactggtgttttgattgtatgttaaaaattgagcggtacatgtttgttgtttttttgttgatgcaaaggtgaggatatttttttaatatctccaaataaattttaaaaatattttttggatagataaataagacagcatttataagcagggagaacttcgtttatgcgtatactttatttcatgttaaactggtgtttattaatgaaatgtaaatatctggcatattaacaaatatttcggactgctaactttatcaaatgtttgttaatgctgattaacaaatgaagatcatgtatacttacgaaaccctttattgtagtagattttgttgttttgagagttggaacttcactttgatttttagaattaaatttttccgttaagatttcgggtttagtgatgaatagtttttttctttgagttattaatcggagtgtatgagagattatcataaatatatttcaggtaaacggaaagcatatacgattatgctgacgccttgccgttcagcactcttagctaatttattatcacctgtaatccatttaaccttctatgaaacaccgcattctacatgccgatgacgacactatattttccggcattgtaaaaaaaatcctccatcagcaaggacttgaagtatatagcgcttttgacggagagcacgcatggatgctgtttaatggatgctgtttaatgaaatgtcatttcattcctgtttgttggatattatgatgccccgcatgaatgggattgatcttggtgaacgtatacgtagcagggatagccagatacctatcttctatttatccggtgaagatctggcactggtatcagcagaagtatttggcagaggtggtgcaaatggctatttccctaaaacttttaacctgcgtgagttgacaggcagattgcaggcatctcttatctacaccaataattacatcttatgaaaggaactataagggtgccttattattctcccggagataatgagttttacggctcccacggaaggccaagaaaagttgcaccggaaattaagaaggtttacagatgcctctatgataaccgcaatgaactaataagcatggaagcaattatggatacggttttcggaaaggagcatcacgatattaataaattgtacgtatacatatccaggctcaagcgcattattaaagatcacccgggttcaagaattcataatgtacgtggtaaagggtataaattaattgtgccatgacttcctgttgccgcaagggttttttgcctatttatcccaatattttttgtgttgttggtatgttttcctaaccagatattttattatattcgttactgtttagtaaacccaaaatataaccgttaaccaaatttatttactacaaaattattaaccatgaaactccacagaacattgcatcatcctgatggtgggcgttcattagcagaatatgaaataagagacaataatgtttttaccactatccaccacgcgggcggatcccgttccctaccctggtatgaggtgcgggaggataaactatatcctacgattcaccatccgcatggctggagttcttttccctggtttgaaatcaatggtaccagtatccggccatccattcaccacccaaagggctgtgacggcttgccgtggtatagaattgtataacctctgaagataatgggtttatggaactagcctggcagtgatgccgggcttttttgtggatagcaagttcggaattaggaacttgctatccagttagctattgtacctctgcaaccttctccgtataattttttactgtatcaattaaatggtcagcatggagaaaaatgtcgtccaaagatgttagctcttttttaatttctgttttgtcgctcttgaagagcccgatttgtttcttattattattaaggtagagccggcaaatcggttttctgttattatcgtcatacaacacagcgaagtaggattgggcatctctataactgatttttatgatcggtactgttctacgtagtattgattttataatattatatccgtcaagctcctcttgggttgttgctattttggcttcggattctataactggttcaatcaattcaggtttgttttgctcaatttcctccgttttgagcgcagttttcaatctttcggtaatgagatcactgatgtaaatctgaaaagctttttttgttaattgtgtaaattggtccattaccttttgagtcagaatgccattagtgtatacatgtttagcaaaatgccttacaaagtcaggacctgggctattgatttcattaccgatcatgcttttgatctggtttagatacttcagttcactggcggtagatacaatagtttctgtatcaaaatagtttttgtgaaactttttcagttcttctatttggttgtccctgatgtcatttaaatcaaatataaagaatggtttttcatccattttattgggcgcgtcgagatctgtgtaaaatcgggattcaaagccgttggtcagaatagagaacttcgcttttgtagtgtggaaatatctgaataattgggagttgtgtggatcaagattagatgaccagtgcttgcactcaattaagataagtggttgcccgtctttcatgatagcatagtccaccttctctcctttttttattcccagatctgccacaaactcaggtactacctccaatgggttaaaaacatcgtagcctagtgcctgaagaaatggcattacaaaggaatgtttggtggcttcttcggtttgaacgagttctttgtgtttgaggattctttcagcgagctgcttgagaagatctttaaaatccataagtaaaaatgtttgtgatggagtaattagttttagggaattagccattgccgagaggcaacagcgtattaagttaggaaagatttggggaattagttctgttcgtaggcaaaataaataaaatggataagggtaagaagagtaatgtggtttagggatactttatattataagttttgatgatccaataagcagtgcctttccacgttttaatatgaagaagaaagtaagctattgatttttaataaattatgaatatgggcggatgtacaggttaataatctctaataatacggccttacttctcggatacttcttggatacttctcagttacttaggagtagcgtatgtgtcgtacttcccatatagtccctatatagtccctatatagttcccatacacttcctatacactcctcatacactcatgatacacttcccatacactcccaatacactatgccgtcctgatttagggttgaatcgtcctgaaatagctttacaccttagtgagataatcctgaaataggtttacaccttgtttcttaaatcctgcatttgatttacaggtaaatttcgacattttttacaaataagcattgaccccggcgtctggatcttttcatgtgcgcccggatcctgatgtttgcagccagctatatacccccatacagccagctttggggccaatgctgctcatttgaaatggaattgatatcagagcgatattaccagcgcttcgttgttattaggcgcttttgacaggcttaaaaggtaattggcgtccaatagtcttaacagctcgttgtagagcagaagaaggtcagccctgtgttgggcgtcctcatattgggtgtcctccgcagcgagtgtttccgaaagccacagccacagtgtttgtcgtgctgcagcaggagggaacagttcgcaaaagcggttaatggcgagcatgggatcagtagattccggcccggataagtgtgtgtaatgaaaaaaggattgggaggtttgcataacaatagattttttgattagtacaaatttatataaaaatatcaatattagggatattaaaatcagttaaatggttataaatatgttattgagggatattttttagaatcataatgagaattattctgcctaaattgatgataaatatgcttttaaagcttttttatgagtgttaaagtattcaacaggataaaggcagtattggctgagaaaggaaaagcaaacaaatggttagctgaagcgatcgacgttaatgtaaatacggtttctaaatggtgtactaacaaaatccagccctctgtggaaactttgtttgtgattgcagaagcattggacgttgaagcaagagaattgctggtattaagaaaaaccaaataatctactcctgacccaagtgatcgcattaaatgttacataaagaaagtcttgccctccttcgccaacaaatccccattggcgcccgccacggtcttaacctgcttaatcaaacaaatggaaacgtagagcaagcaaggcgtttatttgaagacgaaatggttcaggttatcataaataaaacggccgttgcgccggaaatagccagaaagcatttgataatctgtaattatgatattgccggaaccatctccagtattgacggggagcgctttaccttatcccagcgcatcttaaaaaaaacaaagaataataaagaagaagccttgaccctcatcgtacaaagcattgaatccactgagaatatccagcggaaattttggctgcctttagaagaactgcgacatttaccccctcctgtatattgtttgttagtactgcacgattttttaagttatgaagattgggaaggctttagcagcgctatttactttcatccggatatagttgtttcgcagctggaaacggtgcttaacctgccacaggttgctgatcatttacgcattgcaaggaaacgtagcgatgaaatttatcagcaatataaagggcaaacagaatcggtaattgccaataaggtggctggagatgcggagttttctaaacacgagtcaggatttatggccggaagatcgttgattgttgaccggctgtacaatttggtggtggataatattgggttgtttccctgaacctaatcagacctggaattttacatcggtaaatcagtccaggccaccgttgccccaagctgctgcagattatcaatatgcttttgtaagtgtagcggaaagccatttgctaccagtacatcctgttgggccagtctgactaatgcttcctgcggaccaatattccagatcttcatgagatatttggccacctttactttgttgggaccggcgtctgtaacgaccagttttccgtacctgagcaatgccgggtctatttctgtgctttccgcttcttcatcgtcccattcctgtatggtcgtgtgaagttccaaccagaagggattctggatatctgtagaaagttctacaagctcaaggcaggccgttttatctttaccagccttttccatctgttccaaaaagtggcccaaagaaacaatattgaaaccaaggtcaatggcatcccatcgccccgctccatgcaacgcataataaaccgggaagcccggcgcttcttcattcaggtcaataaaaaaaggatcatccatttcgttgagagctataacgtaccagccgggctgccattcaccttctttagttgaagtcagatcttcccccgaaagaccgtgatacctgaaaccgctttgaaactcctcccattcctcctttttggggtaatgaaagggcaataacatagtgcgcgtctctgtttggttttcgataaactgcagaataagctgtgggatgttcaatggcattattagtatagctttggcatggttgatagcagagatgttagggaccttagtaaatttaaatcaatcaaagatcaattgttaaattaactcttccgcctaatccaaccgttacaatttcctgtaaagtggaaagtctaatttctttaatgtcgttctcaatttttgatatataagatttattcttccctacttttgcaccaagttgctcttgtgttaaacccttagcgattcttgcgtcatgtaataaagcaccaagtttaaaaactttatatccagcttcgaattcttcgcgtttttcggttcctcgtttaccatgatgtttacttatgaagtcatcaagggatgtgagactagtatttttgatctttttcatattcactttttattttcaaggctcttgtaatttcattcttcggtgttttctgtgttttcttttgaaaaccattcgccagtacaattaatttccctttatcaaagaaacaaaaaatgcgaaaaatgtcagtaccatgctttattctaacttcatataatccttctgttccttcaagatgtttcaaatatgattctggcaccctttctaattcttcaattgcttttaaagtccagagtattttatcctgaacattttttctctgaccattgaaaaatgtttcaaaatgagtcttgtagaaagctacttttcgatatttctttgtttccacgattgtaaagatacgtaaagttcccctaaaggacaactaatggtttttactactatattcacatagatagaatattataatgttttataatatacatatgatattaagaatgaattagattcctttagatccgcatcattcgctcgcgcagtccttcaattgacaatacatttatatccttgtgtagcatccggtggcaattggagcaaaccaacgccaggtcttttaggcttgtttttgtagaagcggttatctttgaaagtggtgttttgtgatggcattcaataaatcctttaccaatatccccgtaagaatcataaaaatcaaatccgcaaacttcacaaaggagtttccccttcttttttaatatctcatctttttttagcttaatgatagcgggcgcgcgttctctcactttgtggagtttatataagatggaaccttcttctacgctgtcttccaccgtttgctcatcttcttcaatatgaagtatttcttctttgattgatggatctgttacggcattggttatttcaatagctaatttttttagttgatctcttttgtctttgaactcattaaacagtatttcatcaagcttggaatagcttttcaatcctttgcctggagtttctaaagacataaaattagccagctttctagctaccccatttacattcctgaactttagtggatcaggacgttcaaggtcaagaggaaggcttcttaataaatcgcttaaggcaatgatcttgcggtttttgcgatcaatactccctctatccggagaaaaataaagatcgagtgcaagtataatttcatccctatgccactttggattgcttttcatagtacaacgatgtatggacgctcaaaatcacgatgggtatagcttgtcttgaaatgatatttataatatcaatatgatatacaaatataaatatagaatacctatcaccctttgctaatccccccttttctccctatttttactataatgtccacgcacctaccaaaacaatctcacctccaactgaagtcattatttgacctgctatacctgcgcctttgccggtttgccgaccttttgatcgcggattccgccatggcagaggatatcgtgcaaaaagtgtttataaattatgagtatgaagacgatgatttcccggccatcaaaatgttcctgtacaaagaagtgctgaatgcctgccacgcgcataaaacgggtataaaagctgcctttataagggcggaagtaggcggggaaataaaccgggctatcgctgcactgccggagggctgcagtaaagttttcaagcttagctatgtggaggaactgaaaaatgaagagattgcagcggagatgtcgatgccggtaagctgggtgaaaacccagaaagcgagggcacaggagttattgcactggcgactgaagccggaaacttttctcgtattaaacttcttcttatccattgcagaataatctggaatcatattaccaccggtcccggttaataataaagtattgggaaaacgcactttcagcagcggaaagtgaggagctggaggcgtggatagatgccagtgaggagaaccagctgttgtttgcggagttaagcaaggaagctactttgaaggaagagttgaaacagatgggcaactattatccgcagcaggcctggaagaaaattcaagccgcaagaaaggaaagaaaacaggtgccctgggcaggggtggttgccacgttaattatgttgctgctggccattacgttgaagtggtgctatctccgcgaggcactgcctgctgataaaaagacggagaataggggtaccagccgttgagctgcgtcctgtagtgaaagagggatttcctcttctttccgccataggtttttataaagcgtctccttccggaggcgctttatttgtatccggcagcctgcaattcaaataattcggcgtaacgtcctttgcgggccagcagttcctcatggctcccgatttccaccagcgtgccgcgttccagtactaagatgcggttagccatgcgcactgtggaaaaccggtgtgagattaacacggcggttttatcacgggtaagatcagcgaaccggagaaatacattgtattctgcccgggcgtcgagggcggaggtgggctcgtccagtatgaggagttgcgcgtctttcatgtaggcccttgccagcgctatcttttgccattcgccaccggagagttctatgccctggttaaagcggcgccccagcatttgttcatagccgagcggcattttttctatgagtgggaaagcaagactttgcctggccgcatcctcaatcatgggaaggttgttgctttctgcgatattccccacggcgatgttctgggaaaccgtcatctggtaacgctggtagtcctggaatataacgcctacctgcgtacgcagttctttaagatcatattcacggagatctataccatccagcaaaatgcgtccttctacggggtcgtagaggcgggataatagttttaccaacgtggttttgccggcgccgttctcccctaccagcgctaatttctcgccgggatgaagggtgaagttaaggtgccggatggcccatttgtcggagttaatgtatttaaagcctacatcttcaaaagtgaatccctgttgaataggccgcgggaatgcccggggatgaagcacaggaaccattttaggctctatctcaaaatattcaaacaggtcgcgcaggtaaagggcgccctgtgtaacactggaaaaccggataaggataccctggaaggtggtacgcaactgcctgaaagaccccgccaggaaagccaggtcgccaatggttagatgcccctggatcgtttgcaggatgatgatcacataagcggcataatatcctgcggcgccaactaccgcgaaagcagttccccagatggagtccctgatctgcagtacttttttatcggtataaaatttattggagatgaccttaaagcggttgatcaggaaattggaaagatcaaacacctttacttctttggccgtttcatcgctggcgccgagatagcggatataatccagctcacgccggtcggacgtttggccccaggccagtttataatacaggtcgttgaagtgcgattcattcaggaacgccgggattactgccagcagcaataataatatcagccagggattgaagaataccagtcctgccgccaggaaaacaatcgtgatgatgtcctgtacctggctgagtacctgcgccagcagcacggttctgccggaggtttgctgccgggcacgctccagcttatcataaaattcagcatcctcaaattggtcgaggtccagcttggcggcatgttccatgatcttcaccgaagtatggttggcaaagagatcacccaaaaggccatccagcaaggaaatagcgcgacttagcgcatcggataatatggccagtccgaattccagtgccaccagttgccatagccaggtagtggaatgccctgcatctttggtgaggtgtaccacctggtcgatgatcagcttgcccacatataataacgataacggcatggcagattgagccaccctgagaatagtgttcgctatagcgagccctggactggtttgccataccatcctgaaaaatgccggtaggttgcgaagagctgccagccgctctttgaaggttaatttctcgtctttccccgggcgttttttccggggcgttgccattgcactcataccggtaatttacgaaaattgcttctccaaacataagcgcattatctaaaaggatttgttttaaatttgagttcatgtgaataaaccagaatgctatgttattattgatcgtttccttgctgatcgtttgttgtgtgattgttgccggcgttgtatacgctgtaaatgagcaatccaaacaatgggcggcatcagaaaactaatactgcgctttaattgagtaccggatatctgagctgaataaataaaaactacaatagagggataccccttccaggtgcgttatacctgcgtactatagcttttatttaattagcaattatcgatatgcgtgaaaaaaggaatgtgctgacttacctggcagaaaaggaatggctgatcatgagtttatggttcggcctgtcctttatcggcgccttcatggaagtatcccggaataattttaataattaccgcatatttaaagacgtattttttcacgtcattcaccagcagccactatacatcccctacccggccgattattatgatgtaaatctttatggccccttattcagcctcgtaattgctccttttgcaggtttggaaatccacctcggagcgatgttgtggtcgctcaccggttccgctgttttattttatgccatccggcaactgccactcttacgcatgcaacagaatattatcctgttgctatgttcaatggagctgatgggcgccagcagctggttccagatgaaccagttcatcggcgctttcattatcctcacttttgccaatacggttaaagggaaagaactttgggcggctttctttattgtattaggaacgctgacaaagttttatggtatcgtaggacttgcattcttcttctttacccccaatcccaaacggtttatcggttacctgtttttatggggcgcggtcatgtttgcactacccatgatcatatcttctccccaatatattattcaatgttactttgattggtatgctgcgctggtacacaaaaacgaactgaatgaaggcgcgaatatcctgttccaggatatatctgccggaggctttataaaaagggtatttcatttaccggacctgagtaataatgtagtactcattcctgcggtagtacttttctttttacaatatacccggttagcagatcgctacaattcccgttaccggctgtatatactctgctccacactgatattcccggtacttttcagcaccagttcggagtcgcctacctacatcatcgctataccggcggtatgtatctggtatgtaatgcagccatctaccagaaggaataacatatttatgtttttcctcatcttcctgatcagtttttcccattcagatatacttactccctggttcaggagaaatattgctatgccatatgccgtgaaagccttgccatgcctggtattatggctggtgatcgtctatcagacctacacccggaaatatctgtcaaaaaaagatgtttctcccgcgcctgtcaaggaattggaacccgttgccgtattgtgaaaaaattaacgaaaaaagtaataatccggacgtaaattgccggattattaaaggtttttgattatgaacacgggattcaagataggtagtgcatttgcgttatctgctatgctgtttcacggcattcaaacaagtgcacagaagaagtcagcatcattgccaggctttgttgaaagtaaatcagttgcttcagtagatccttatatcggctccgggggccacggacacgtatttgttggcgccagcgttccatacggcgcagtacaaacaggtcctaccaacattgtaaaaggttgggattggtgctccggatatcattattcagacagcgtattaataggcttttcccagatgcacctcagcggaaccggtatcggcgacctgggcgatgtactcattatgccctacaccggcaaggtgagaactaaccgcggcacacaggaagatccaacttcaggatacggctcccgctactcccacgaacgcgaaactgctcgtcccggctactacgccgttcagttggacgactacaatatcaaagcagaactaaccgcttcagaaagagttgcttttcataagtacaccttcccgaaagatcaacctgccaatattatcatcgacctgaaagaaggtatcggctgggatgcgccggtagaaacatttatccgccaggtagatgaatatacgctcgaaggataccgctactccaaaggatgggcggaagaccaacgcctctggtttgccattaaatcaaatgtaccggtgaaacaattcctggtatttgatggagataataaacaaaccggtaaagaagtaaaatcgaaagaagccaaaggggtgattgtattcgataaatcgcccggacaggtaatgctgaaagtaggcgtttctcccgtaagcagcgaaaacgcactggcaaatataaaagcagaaataccaggctgggacttcatcaaaaccattaacagcgctaatgctaaatgggacaaggaactggctaaagtaagcattgaaacaaaagacgaagccgcccgccgcgtattttacactgccatgtatcacaccatgattgatccggccttgttcaatgaccatgacggcagctaccgcggcaccgataaaaaagtatataccaatccaggcttcgataactactccgtattttctctctgggatatttatcgttcctgcgcgccactcgccaccatcctgcatcctgaaaaggtgaacagtttcgtgaactccatgctcaccatccacaaacaacaaggcaaattgccggtatggccgctgatgggcaatgaaaccaactgtatggtgggctatcacgccgtaccgcctattgtggacgcttacctgaaaggatttaaaggattcaacgcagaagaggcttttgaagccatgaaggttaccgctaaccgcgacgacctgggcttgaaatacgtaaaggaattgggttacatcccggcagataaagaatacgaatccgtttccaaagccatggaatacgccatcgacgactggtgcattgcagccatggcgaagaaattaggcaaaactgccgacttcgaatactacaaaaaacgcgctgcttactaccgcaattatttcgatagcaccatccgttttgtacgtccgcgtatgagcgatggcagcttcaaaacgccttacgatccgtttaactccgtccacgaaaaaggcgacttcaccgaaggtaacggctggcaatacacctggctggtgccacaggacgtggaaggactcatccaactcatgggtggcgacgatgcgttcaccaacaaactcgacagcctcttcaccgccaaaggcgatatgggcgcagaagcgtccagcgatatctccggtctcataggtatgtatgcgcatggtaatgagccaagtcatcacgttacctacatgtacgcattctccggttatcaatggaaaaccgctgaaaaagtaagacaggtaatgaaagaattttacttcgatcagccggaaggtcttgctggtaacgaagattgcggcgcgatgtcgtcctggtatgtattctcctccctgggcttctaccctgaaaactccgccagcggcacctatgtattaggcagcccgctgttcgacaaagcaactattaaagtaggcgccggtaaaactttcacggtacaaaccatcggcaatagtgcagagaacatctatatccaaagtgttacccttaacggtaaaccatatacgaagagtttcatcactcaccaggatgtggtagccggcggaacgctggtagttaaaatgggcaacaaacccaacctcagctttggtaaggctgcagcggacagaccatcaaacgcgctttagcggaggctgtcttactcaggattacgctgattttattgattttcgggatttgatcacgttggatttaaaatgattatgggagatataagcggatattttcgcttttatctcccataatcattttaaatccaaaaagtaaaatcaatgtaatcagcaaaatcagcgtaatcctgagtaagacaacctacgcgttaggcgttctcgcccagcacgcgcaatacctctggtgttacgttgccgaagatggaaacgcctgccgcgccgttttggatggccagttttacggcttcggccaggtcggcgtagttgccatggaagtccggaaggtacaggcctgcgtataatggaaaggcgccatggagccccttcacaccttctgctaccgcatcgccgatccagctcacgttttccctgtaaaagccatgatagatcattgggcagatggcgttcaatggccagtttgtccaatcctggcgtacgatacgtttggcgatttcaggagtagggaatactgctgcggaaattggctttttatgttgccgggctacctgtgcgagattgctcaccacattagtgatccggtcgtagcggaacttgcgccaggaaggactttgatcgggatgctctatttgtaaaggatctgcgccatgtttttctttataggcattgcggcattgttcgcaatagcagaaatcgtattctggcaattccttcgactgatcaataccataattactccagaggttcacgggtaatatcacatcgcagtaacggacatagtcgagatggatgccatcgacgtaatccagtgaaaggattttttccacctggtctttcagataattcactacctccggtttgctgggacatagccagcggtagtaatctacatagggaggatggttggcgcaggattcacctttgcggttttgcgcataccattccgggtgactagcaagcagttctttttccccgcgattcatagtccacatccagcggtgagcgttgatgccgttggctttagcggttttgaaatgcagttcgctatcttcctcaaacataatatccgtgatccctgcttttctgtaagcagcgtatcttgcttttaagacagcggcggtatctttatgatccggattgatccacacgcggtgttgcacggcattcttttccagcgtgggcgctgtttcttttgcagtagctgcgctggccggcagcgtagatttcgccagtgccaatccaccgatgcccaatgattttataaaaagacgtttatccatagcgcttattttctgttactatacactttaccttcctggttgatatttacgaaaccagcaaaactactaccggtaacgctggcgttatactgtaatgaaatgccttccattgataacgtatatacttctttattagtaccggtttgtttttcagagatcttcagctcttttaagtttttagcataacggccattggcttgcctaaattgtagttgggcgctgtaaatctgccagagatattgtttggcttcctccgccggaggtagctggaaagtagtactggctttgctggtaaacaacagataaccccaccgttcaggcgcatgcatattcacaattccttgtggtgaccaaacccagttgtgttctggctgctgttgttttacgtacttgccgttcttaatatcagtgtcccactccacccgcgaaaaattgatgcgccacaggctattttctgcgggtcgttggtttttattgaagaagctgagggcgctgaaaggcacggccatctctactgtccactctttatcggtatccgacggattattaatagtgccatcaatatgtatggcagtgataattcctttggtgtcccagttgatcagcgcctctcccatgttgcggtaaggcttacccataaacaggtccatcacggtatttaaagcattgatttctatctcgtagtattggtgggtatctccatcgggatctataaatacttcaaagtcattatcccggaaaataatggcgtcatgctccaccagtgttccccagatatgtggctcctgcagcgtagctgcgatataaagatattgctggtcccacatcatcttcaccctggtgcgcagtgccggcgccggtttagcgtcgccttcaatatctttgaaatcttccgtccaggcggcttgttgccaggcggcttcatcgagtttaccatcgatcactactttgtttttcgtttcctggcatacgtagtggcggggtgtttcgtgtgcgggtttatacaattccagcccggtttgagcggaggttgtcttactcaggattagactgattacgctgattacactgataaatttttttataatttttatattgagatgatcttttttcatttgaaatttccgttgattaaccttttaaattctaagcttggccggccaaagttaataagtaatcctgtttctacattatatgcttcaagatagcttctaacctgagacaaatgcacttgttctgttattgttaatgcttttagttctacggctacaacgctttcgacaataaaatctgctctccttccccctacgtgttgtcctttatagtataaagggatttctttttctctttcaaagagaatttgtttttcactcatttcaatggctaacgcgcgctgataaattacttcctgaaatcctgatcccagtatacgatgcacttgcattgcacaaccaatgattttactagtaagctcagaatgcttataatttggattaatcatacattatgtattaaggttaaaacaaacaatgacgcgaatttaactattccaataactaaaaaaaagagccggataaaacatccggctctaatcctaaaaattaaaatcaaattaaaatcaaaaaagtaaaatcagtgtaatcagcgtaatcagtctaatcctgagtaagacaacctccgcgcgcgttaccatatgcgtacgcgcgcactatccgcccggtacatgccatcccccggcttcacgccatacacttcgtagaaggcgtccacgtcgctaaaaggcccgttcaccctgaatttggcgggagagtgtacatcggtcagcacctgcctggccagcgactcttttttggtgtggcccagccagcccagggagtagcccatgaagtaccgctgcgacggcgtgtatccggcgatcttttcgttcttcttatattgtgctgtttttttgaacgcttcccatcccagcaggataccgcctagatccgcgatattttcaccaagagtggctttgccgttgatgcgtaaggtatctactactacgtagttgttgaattgttttaccatgacggatgcgcgctcattgaattttttctcatcgtctttggtccaccagcttttcaggttgccggcggcatcaaactggcggccttcatcatcaaacccgtgtgtgatttcgtgacctatggtggaggcgccggcatagccgtatacaacggcatcgtccagctcttcatcgcgcttaccgggaacggtgaagataccggcaggcagcacaatttcgttgttgctggggttatagtaggcgttgtatgtttgcggcgtcatatcccattcattgcgatcaaccggtttgccgagtttgttgatctggtagttttgccaccactggtgggctgcttcgatgttctgatggtacgattgttccttgatatccattgcagtaaaatctttccacttatcgggatagcctactttcttggtgatcttggagagtttgtataatgctttttgcttggtgctatcgctcatccagtcgaggtgttcaatgcgtattttcagttccgcacggatttcttctaccaggttttcatatctttttttggcggtggtattaaagaactcttttacaaacagttggccgagggcctctcccattgcgctttcctctgcgtccagcactcgtttccaacgcggtttctgcttgtcttgtcctttgagaagggtgccataaaatgcgaagtcggtgttggcgatggtatcgctgagatgttgggaggccgcgttgatcaggttccacttgaggtagtccttccaggtttgaagtggctgtgatttaacggcgttgctcaggttggaataaaattccggctgaccaacaataatggtatcggcgaatttgctgatgccttgttgtttgatgaactcattccagtcgatgttgccggcaattttatttagctgggtgacagccatcttatggtagttggcttccggatcacggagtgcttccagtttgcggctgtttttagccaggtttgtttccagttgtacgataccggcagccgcctttttagcggcggtgctgtcgtagccaacaaattgcagcattttagcaacgtgaccgggataggcattccggatgttggtggtgcgtgcgtcggtgttgaagtagtagtcgcggttgggaagacccagcccgccttgtgccagctgcacagcgatgacgtcactgtttttggcgtcctgcccgatgtacaggctgcagaaggcgccggtgttgatattcagcttggaggccatttgcaccagctgcgggatggtggtaatggcatcaatggctttcagctccgcttcaataggctttataccttcctggttgatgcgcacggaatccattccgctggtccagaaggcggcaatttttttagagataggatcggtaggattttctaccgctttttcattgatgatacgcaggcgtttgtacagttcttcctgtaccaggttaccgatgccccatgaactgtattctgctggtatgggattgcgttttatccagccgccgttggcataatcaaaaaaatcttgggtgggatttacggtgctgtctacattggcggctactgcgtcggggatggaagatgcgtcggtgccgggttgtttctgtccctggttacatgcagcgaagcaggtaatggcagccagaccggttccggtgaggatggattttatcataagctgttgagattttgttatcggaagaaaggtaattattttttatcaccctgattattaaaatgggcttaacggcagcaggagaatataaagtaaataatgtattttggtacaaagtcatttccttacctgcaacgcttatgatcaacaatttaaagactggccgcattttatctatcgatgctttccgcggcattactattcttgtcatgattttcgttaacagtgtggcgggagtgagcggtatcccttcctggatgcagcatgcgcatggtaatgaagaccggatgacctttgtagatgtggtgttccctgccttcctgtttatagtggggatgtcggtaccttttgctatcaatagccggttggcaaagggagatactttctggcagttgcagcggcatattgcctggcgtacattgggtttgtgggtgctgggtatttttatggtaaatgctgaaaaggtgaatgcagctgctaccggtatgagtggcgccgcgtggtcacttttattttatgtatgcgctatactggtttggaatgtttataaatttaaaaacgcatggctcgcatggtgtttcaagggtgcgggcatgataggattgatcatcctggcattgattttccgcggaggtgaagatggaacggagcgattaaccccagattggtggggtattttggggttgataggctgggcatacctgtatgcatgtatcatttaccaggtgtttaaaggtgcggccggcgccatcatgctgatgattgcggtatgtatcgggtattatattttatgtaaacagccgttcatgggagaatggggctggcttacatcgcaggcaggtcatgctgcgcatacttccattgtgttgtcgggaatgttgctgacattattttattttgatgaagacctgggcctgaaaggaagtaagctggtgtcgcgggtaacgggataccttattttactgttgatagccggtgttttgttaagacctgcttataaactatccaagatccaggctacccccagctggtgcctctattgcagtgctatatgtgtggctgtattttccctgttatattttctgatagatgtaaagcaggtcagtaagtggacggctttctttcgcccggcaggttccaatcctttgctcacttatatcctgccggacattgttttttatggcatgttgctcgcggggatcagcctgccggctgtattgggagaaggactgccgggtattgcctggtgcgctttttttgcagtaatcatgctcttcctggtaaagggattaaacaagctgggaattcgcctgcaactgtaacaatcttacacactgcttcgttataactctcgtaatgtagaaaaatatctacgtgaaatacatccgtaaccgggtatagcgcgtaaatagttgtggcatttcgtttgtccctttcattcatgtaaacagattttgcatcccaaaagttcccccatgaaaaaaattgcaattgtattagcgtcagccggattgattttagctatcttagcgcagtacgccttagtcaacgactggatgtggttcaaagtgttccacacccttgggtttataggctacatattgatcatcagcggtcttgcttgtttttgcctgtggttgattcatcagttttcccgtgatgaaaaaaacaggataaaacgttactatcatcgccagcacgatgaaagcgaagtgaatactgcacaacggtaataacgatatgtctgacttcttcacacttaaatttgaatacaacgggcatccgcacatcctggatgtgcaaaccgctcatcagcaattcaaaacggtttataaggtagccgttcaggaacatgaaattacttttgagcctgatgaagaaggctacgtacgcgctgtttccagcaagcctatgcacgatcatttaaatcctgtagatgtaggactgctacatcatgtggcagaactcattatccagcatattcagcaataaattattcctcatcaattttttctccccggatctcgtcacgcaatgattcagggtcccatccctgcccttcatccagccaggtttttacacggtcggaggaaatgagcttttccatttcatcgatacgttccttcatggaactgatgtattgttttttatcatcgcgcaatgcagataagcctttcagggtgcgttcatcctggcggaagaaagtccgtgcggcacgttcactccggtaagcccttccacccagcatacgcagggcatccacgccaacacgcagggaagtgtctaccgtttcgcggtaaatatgtagtacgcccaggtccatcagttcaaaagtatcttcattattttctgcccttaccaacagttgcagatgaggaaaataccgttgggccattctcactatttccagtgtttgttccgcatgatcagtggcaatgatcagcatttttgcatctttagcgccggcggcaaccagcaggtcataacgggacgcatctccataatatactttaatacccaggttgtgcagcgcatctacccggtcggaatccaggtcgaggatagtagcattaataccattggcccgcaggaaacgcccggtcatgctgccgaagcggccaaagcctgcaatgatcaccgggttcttttcgttgatctcatctgcttccctttccgcttttacttctgagcgggtataatacggttgaatcactttttcatatagcagcataatcagcggggtaagcgccatgctgatggctactactgctgttatcatggcggtcatttccttactcatcagccgcgtttgactggtaaacgacagcaacacaaacgcaaactccccgatgtctgcgagggcaaaagcaaacagcaggttctggtcggtgctcagcctgaatatttttcccagcagcaacaacacaatacctttcagggccatgatccctactaccaagcccatgatcagccagggctgttccatgatcagcctgaaatcaatagatgctccaacggcgataaaaaataagccgagtaacaatcccttgaaaggttcaatatcactttccagctcatgacggtattcactgttggcaagtaccacgccgcccaaaaatgctcccagcgcagagctgaggcccaccaggttcatcagcacagcaatgccaaccaccatcagcaaggccgtggcggtaaataattcgcgtacacgggtccgggcaatgatacgcatcagcggccgcaccaggtacatgcctgcaataatgatgatggctactgcgcccagcactaccagtgtttgcgcccatccgggtaaattatccctcagggaggcgctgtgtggagcggcatctgctgcgacattaccagcgagcaatggaaatatggccagcatcgggatcacggcaatatcctggaacagcaacaccgaaaaggcgctctgcccggcagatgtgcccatccaccctttttcattcagcgtttgcaacacaatggcggtagacgacaacgaaaggatcatgcccagtgccagcgatgtgttgatgggttgtcctaccaggtaggcaatgcccgcaatggcagcggcactgattatcacctgcagccctcccagcccgagaatggaggaccgcagccgccacaacagcgccggttccagctctatccctatgaggaacagcatcatcactacaccgaattccgcaaaatgcataatatcttctccctctcttcctataaaacccagtaaagaagggcctatgataatacctgcgatcaggtagcctaaaacagctcccagtcccatctttttggccagcggcacaaacacgatggcagcagccaggtataccatcgactgaaatagtaaagaatgttgatccatattatctggtttgagcgggtagttgaagtatttgacggagattttccaggccaggcaaaggtgtaaggtcaaatttatcgtcgcggagacgttccagcacctgtttcaactgggccgtatcttcctggatatctgaaatatcctgccggtgaacgccatatatcacaaaaggagccgcataatgcatattgcataatttggcggtttgtataaaaggcagcaggaattcatgcacggtatgtccgtggtgaccatccggttgataggaatgttcggcgccccctgctgtgataatattgctgaaatactttccctgtaaggctttgccggtatgtccatatgcccagccgtgctccagcaccaggtcgatccactgctttacaatagctggtgcactgtaccagtaaaaaggatgttgcataaaaataatatcatgctgctccagcaacttttgctcacgggctacatccacatccagatcagggtattgttcatacaggtcgttgaaagtaatccccgggatatttttaaccacccgcagcaactgggaatgtaccctggatttttccagggcgggatgtgcaaaatttatcagaactctcgccattattggattttcgtataaaggaatttaggtattttgtttcaaacattgtccttctgtgataacgaattccgtatcaaccttccgaatactcctgtaaaagcagccggtacttattgaggatactggatttggagataaagcccaccagttgttgatcctgtattaccggcaggttccaggcctgggccgtatcaaattttttgatcaccacgttaatgttatcttttaaattaaccaccgccggcggggcgtgcatcagcttctttacggtaacggtatcgtacagttcaggattaaacataatcggcctgatttcatccagcgtaataacgccttcaaacagttgttcgtggttcactaccgcaataatattccggctgccttctttcaccagttctataatatcccgcagggtggcgtcaatagaaattgtttgcacatctttttcaagaaggtcctccattttcaggagtagcaggatgtttttatcatgggcatgcgtaaatactttgccatcttttgccagttctttgatttccggggagataggtgaaaaccattttgccatcaggaaagaaatggtggaaacaatcatcagcggaataaaaagatcgtaccccgagctggattcggcaatcaggaagatggccgtcagcggggcatacattacaccggccattacgccggccataccaacaatcacgaggttggtaaccgggatatcggtgaatcccatctgctgacaaaccatggcgtaaaagaatcccaggaatccgccggcaaacagtgatggtgcgaagttcccgccgttaccaccgctttgtatggtgacggaagcggccaatgctttcagcaggcacacgcagccggtaaacaccactatcatccagctttgcaggggaagataccggaaaaaactgttttgaagaatggcttcgccattgccggcagccagtgatttcacgctggagtagccttcgccgaataaaggaggcagcaccacgcagagggcggataccagtacaccgcccaggagggcgcgttgtatcgctgtccagttgagggagtggaaaaagtgttctattttttgtgagatgaccacgtaatatcttgcataaaatccgctgagtatgcccagggctatataataaggtacgttatgataattaaaagcaacccttgactcgaaatgaaacagcgcttcttcctgtaaaataattttagagagcaagctgccgcaaacggctgccacaatcagcggcatgaaatcagaaaacaccacgcccgtgagtaatatttcaaaagcaaacatcatcccggcaatcggagcattgaatgctgccgctataccggcagttgcaccggcagccagtaacagcgtacgttctttataacctagtttataggtacgtgcataattggagccaagtgccgcaccggtaaccgcaatgggactttccaatccggccgatccgccaagccccacggtgatagcgctctgtaatatctgtgaatacatttttacgggtgggatcaggctggagttccgggctatttcgtgcaggatagcaggaatccctttcctcgattgccccttgaaaaaccagatgaccatgagggtagtgagcacaattccgaggaacgggaacactacataaaaaataacctgtgtgctgaaatgtactttataggtgattacataatggatgtaatggacgaggctttttaagacgacgcctgctaaccctgccgaacagcctaccagtatacctgaaagcaggaggaactggctgcggctcattttgctgtgtaaccaatgtaatatgagctcatagcttttggcactctttaaactgtattgttcaaaatcctttttgaatcgaaaaaagctatggtatttccgcaggcggttaaattgactcatgcggcaaatttaaggatcaaagctcaatcagtgcataaactttatcattcatataaggaccgccagggcgacgggccgtgtaatccaggttaatccagtactctcctttcagctcgtgatagtatatttctttcacggctggcttcggaaaaagtgtgatgatagcctgcttcatgatttcaaactcttgtttatcaccacagtaaagctccgggtaggcatggcctttcaccagtacaatacggcatcgtgccccgatcgattgcaggcaggaagtcatgaggatggaatggtcgtcgcagtcgccccccaaaccattttgaatggtttcctgtgcagtggcgaagtattcgtcgcggcgggaatccagcacatatttaaactggccgttgatataacggaacagggaaaggaaccgggttattttcccgtatttataaaaatattcgtcgtaataatcgagggagtgttttacggagaagttgcggaccaccgagtcctggaagttgattttttcccgcatgccgcgtacggttttatcgcggtagctttctacccttctcggataaagactgaggatatccagttgtttgctgcctttggtgttgaggttgccctgtaccatgcctttataatcgttgagcacattataaaaggtatagcggtcagtaactttgttaatgaccattacactgcataccagtaagaagatgggaataatcagcggtctgaagacccagcggagcaaatagacaactatgaaacccgctaccacggccaataacagatcgatgtgccagccgttcgctacgatgggaggcgtaaagctgttgatatagggtgccagcaataataaggtcaacaaactcaatgtgttgaacaatatattctgtgctatggtatatttgctttcgtctatggccattatgctacgcaataaagcaaaattatgccataatcacctcgcaaagtttgaaacggcctgtttgaaggaagtacttttccggatgagttctatttgctgaaccgtatcatttttctgtttatccatttgcagttgctgatagattttgttcagcaatccgaaattcatcagcgctaatactttgaaatccagtttttgtgcgttttccacagctgtttctgcggtgcggatagctttattgaattcgtgttcattaaaatatacgcccgcgtatagtaatttctgcacagattccaggtattttccgccgaaataatcagcagaatatttcttgatcacctggtcggtgtgccggcagatccgtgcagcggaagctgtttggcccaggccgaggtaggcttgtgcctgccagcagagcagcatgaggcgcagtgaatctgttttacggtgttgtaaagaaggatatgtttcaaaaatccgggtggtaaagctgaggaggtgttcgttatctcccagcagggtgaacacgatccccatattacggaatacaatttcctggggttcactgatgggtttcttaccaccactggtgccggtccagtagcggaaatagttatagatcttttcccggatatcttcgtttataataccaaatttgaggaattcatagatgaagagctggatttcataaggtgttacccaaagctcgtcttcaaattcatcggctgcgtagattttcttaatattattgagttctatttcgcactgttctgcatcgagttgcagcagggccattgtaaataatttgctcctgattttgagcttgtcttcccgggcttcagcaagtcccagcaaagcgttaagtactttgcgtttcctgaaatgaataaattcgtcactgataaaagggccaatagggttcttcttgaagaagcccgcggggaagatggatttgagttcaccctggttgttgccatcatgctggtagtgtaatacgaggtattccagcaggtgggatttttctatgttggataatggtaaatgcaacattttgatgatgccatcgatctgcgcatggttgatagcgtagcggagcagccatctgaatacgccgatgcggtaaggcgactgtggcaggtgttcgagtattgccattagcaggggctcatttatttcctggccgttttctttcaggtagtgcatggccacaaaatattcgagcaacatggtatgggcaaagcgcaccttcacattgaacataatttcctggctcaggttttcttccaccaatatattatcggccagtagttctttgtaggcagggaacagatcggcattctgggtgagcagcaaatttttatctgcgtagatccctgttctgccgaggtcgagcagggtgagtaatttttcaatgatttttattttgaaagaattgctttgcgaattgaacacgcggttctgaataaagcgcgatacaatttcgaacaggctaaggtgttcatctacaaaggtttgatccgggccgctgttgagctgacaaaatagttgcaggtaataaggataacgcagtttttgcaggaagttttcagaaaacagccgtacggtagcgggatcaaactggtggttataaagaatagacttcacttcctgttccgtaagccggggcatattgatattggtttcctcatccatttcagcgcccaggtaccaatagcgccggaaggcggggtattgctgggagtgctggaatatttcggcccaggtactgctccggatggaaaggatcactttcacccaggggtataagtcgttggaatacacaaagtcttccagtttggaatatagtaggcggagtttctcgccggctacggcgatttcatcgaagccgtctattattaatataaggcgtccgccttttttatcgaagtggctggagaagtattcgcggaagttttcaccattaccgaggttcatctggttatcgagccaggaggaaagggagaatcctttcagcaggaggctgccggccgcatgagcatggatgaaccagcaaacgtcctgtttataacgggcttctttgccaaaccagcaatgttctgcgaggtgtaccaatgccagcgacttaccccatcctgatggcgctattaacgcggtagcggcgtagtcgctttccaggaatttttcgatgtgggcattacagaagggccggtgaacggtatacggaaaagcaatgccagagcgatttttgagggttagcatcgtgtaatgggaaactgcgtctgccttgtttttcaggtcagaccattttccattatccaatgctacggccgaagtagacgcattggtggcagtggaagcggtgttcatcttccggtagtgatgttgctgaaaatcttcccagtctttatattggcaatattgcgaaagggtattcagggtatatctggagaagctgtgttgagcaacagcaaatccgaacacccttttaagcgtagtttcgcttaccagtttcgtggtgttatccaatatggactgagagagatgtttgcaatctcctggcaacatgacttcaacaccgaacctgcggagaacttcattctgcagggtaatgataaagtcataggatagatcaatcataggggacaataaatggattttcgaattgtcggtacctgtttaattacgtatcgtatttgcgtttagattttcggaagaccgaatgaacaaaatgaacagaaaatattaaattgaattatatatatgaaaataactaataaaattaattttattattagttgtcatctggatatcatatataaatatgatgacgtacagcataatgtttctatatgagtatatattatatattattttccagtactttgactgtaatgaaaacggataaataactttattagccagccccgaaatttttctttttcctgttttaaatgcaatggtcccttattttcctgcctgtttttctccaactcctaccttccgaatgaacaaaatgaacagtaaaaacgaagattgaacaaactgaattgtcagtcggaaatgaacaagaaagacacatccagaaatcagcccttcagtatacattcgtagcgttcttgtaacattcttttaacaaatgatcgcaaggaagtatacttttttatcaaccagtatcccttccccaagctattcctaacctgcctgccgcccttagagttttgttgtaatgcaatgaaactgaacaatttttattcaaatatttgatgctatgcattcaaaagctactcctaatagcccttttactgcccttttctgtttccctagctctgcagggaaggaagctgtgaaaaccagcgttgcccacttttttcataaagccgggtcaatagcttggaaaagttttctgctactattattactattcggtataggcgcgcgggacagccaggcgcaaacctataccacgagggtatatgccaatacacaagtaggcagagcctccggactttgcatcggttgtggtgtaacaaatggtacacaggcagtggatggctcccttactacagcctccactatttctacattggtaacactgttgggcgctacagcctcacaggacctgatttttccggctgccgttaccaataatacccctgcggtagttaaaataggtactgccggcacactcggcacgctggtaaatttaaacctgcttggcggcgtttatgtacaggcctacaatggcagtacgccggtaggtggtactgtctttgccaataactcagtattaaccctgttggcaagtggcaaccaggcggaaatatttttacctgctccaggcggcacatacgaccgtgtaagagtaacagtagatggcggattagcaggagtagccggtagcatacaggtattctcagcatattatgatatacctgcttcaggtacaataaactgtggcgctgcaatagatgtgctgtacggcgttaccgggcaggcagcttcacttggagtagtaaccaatcctgctgctgcaggtgatggtattgttactgcagccaattatgcaacgctgagcagcgttgttggtgcgttaggcagcagtgcccaggttactgcagtattccctggtctctctaaagcaggtgattctatccgtgtggtagtgtcagatcctgcttcgctgcttaccctacagctatttagttctgttagaattattacttataatggaggtattgtagttgataatattcaggccgatggcaatttattgcgcctcaatcttctttcaggaggaggaaatttacaggcgttaactttccagcctacagcgcctttcgatcacgtaacagtgcagataggctccgggctggcaggcgcactcgcctccctgagagtacatgaaatacaacgtttcccggcaggtccgtcaacagctggtgggatattgagaactacctgcctgaattcgccgcttacattgaatgtaagtagtccggaagcaggattaacttatagctggtacgactctacccaaaccacagtggtagcttccaacagcaccagttacagtcctcctgtaggtgttgccggaagtttccgttattatgtttccgccaccaggatcggctgttcaaccgaatcagccaaaacgttggtgactgtaaaggttaataatttctctaacgctgcagatattactgttcctgccactacacagggctgcatcgcggataccgtaacaattacccctacttctgcaaccgttaataataacccggtattcagctggtataaaaatgctgataaaaccgggcctattacaaatggcctgatagaaggagccgttaaatacagcatcgatactaccggaaaattaaatattaccggtcttgctgcaggatcatacacctattatgtaagcgtatcggacagcgatcattgtgaaaatgcagctaacgccctgaaggcggctccggtaactgtatccgcgcaaattgcgccaccggtactttcccaaacgtacgcggtaacaaccggaataccattggtgttaacagccacaccagtatccggcgctactattgaatggtacagcgataccacgcaggcgccggttgcagtaggcaactccatcaccctgcctccgtttaccagtcctggtgtatttacttactacgcaggtgtaaaaactaccggaggttgtacgtctttccgtgttcctgtggtcattaccgtaaccggccctgttaccactaccagttgtaacgtgcccaccagtcaggtaaccggaaccacattgggttgtgtattgtgtagtgttgtaaatcctggatttgatatagatacggtttctacgaatttcacccgtctcaatataccggtaggtttattaggaggatcagtttatcaacaacttatcttccctgctgcaggcgatgcaacagacagcattcgtcttgatctggcttcaccaggcggactggcagatgtaagcttacttggcggcgctgtagttaccatttataatggaacaacggttgtaagtacacacactttatcccagttgctcactttaagattactgagcggaacccgctactatgctacagtggccgctggtggtatatacgaccgtgtggaagtgaaacttacgggcgtagcgaatctgcttacttccctggatatttatggtgtacgctctcttgtaccggatcctgttattacagccggcaatctgaccgtatgcgttggcgagcgcgctgtatttacagccactccagctgctggtactactgttcagtggtatgctgattcaaccaccaatatctccctgggcaatcagccgacatttacgaccgatacgttaagaaccgccggtacctttacttattatgtacaggcaatggatggtacctgcgcgaatccaaatcgtataccggttaccgttaccgtgaacgcattgggcactgcagctgatattaccgttgcagatactactaacgtttgcggaagtggtgctgccacactcacaccaacaaccgcaggcgtaacaactcccgtatttaaatggtatgcagacgccaataaaacaacgcccattaccaacggcactgttattggtggcgccacctttgctataaatgcagccggcagcctgtctgtcactggcctttcactgggtaatcatacttattatgtaagcgtatcaggcgccaaccgttgcgaaaatgcagccggcagcctgaaatctgctactgtaaaagtaactacccctcctgcacctcctaccctggttcagtcatacaccgtatccaccggcttaccattaacactggtcgcttcaccggctccgggatcaacgatagtttggtaccgcgatactacacaggcatctattggcagcggcaattctattaccttgccgccgtttactacgccgggtgtatatagctactacgccggcgacagcctgccaggtggttgtgtttccagccgcgtgctgatcaccatcacggtaacaggtcctgttactaccaccagttgtaacgtgcctaccagccaggtaaccggaacaacttttggctgcgtgttgtgtagtgttgtaaacccaaccaacgacatcgacaccgttagtgccaatttcacccgcctcaatataccggtaggattgttgggaggcgctgtttatcaacagctcatcttccctgccgcaggtgatgcaaccgacagcatccgcttcgacctggcttcaccaggcggattggcagatgtaagtttactgggtggcgcagtagtcactgtatataatggtactactgtggtaagtactcagaatttatcacaattagttactttaagattattaagcggtaaccgttactatgctacagtacctgctggtggcgtgtatgaccgcgttgaaataaaattaaccgggttagcgaacctgcttaactccctggatatctatggcgtgcgttccgttgttccggatccggttattaccgccaaaaatgtggcagtatgtgctggtcagcgtgccgtattcaccgccactccggccgctggtaccactgttcagtggtatgctgattcaaccggcggcgtttccctgggtaatcaacctacattcacaacagacacgctgagaaccgccggtacctatacctactatgtacaggtaatggacggcacctgccctaatccaaaccgtatcccggttacagccaccgtaaatccattggctactgcggcagatattaccatagcagataccacaaccagttgtggtagcggaccggcagtgttgacaccaactgcagccggtgttactacacctgtatttacatggtatacagatgctaataaaactacgccgattgtaaatggtgctgttattggcggtgctacctttgccatcaccgcaggcggtcagcttagcgttaccggccttacaccaggtaatcacacttattatgtaagtgtatccggtgctaaccgttgtgaaaatgcagccggaactttgaaggctgctaccatcaaagttgtcagcgctccggctccgccaacagtggtacagaattatactatcagcaccgggttgccgttaaccatcaccgcaacgcctgctccgggcgccactgtgctgtggtatagcgatactacgctggcgccaattgctaccggcaattctattactttgcctccgttcgcaagtccgggagtatatacttattatgtaggcgatagcctggcaggtggttgtttatccaaccgtttgccaatcgtgattacagtaactggtccggttatacctgccagctgtaacgtgcctaccagccaggtaaccggaactacgctcggttgcgtgctgtgtagcgttgttgatccaaacaacgacattgattctattcctactaatttcacccgcctgaatataccggtaggtttattgggaggttcagtttaccaacgcctcatcttccctgcagtgcgtgcggcatcagacagtatccgctttgaactggcttcaccaggcggactggcagatgttagcctgctcggtggtgcagtggtaactgtttataacggctcaaccgttgtaagcactcaaacattatcccagcttctcacgctgagaatattgagcggtacccgctactttgctactgttccggcaggcggcgcttatgatcgcgtggaagtaaaactgacaggtgttgctaatctgctcaattcactggacatctatgatgtacgtgcagttgttccggatcccacagttaccacacaaaacgtggtggtatgtgctggtcaacctgccacattaacagtaacaccggcagcaggtacaactgtacgctggtataccgattctactaccactattataaagagcactttaaatacatacatcaccgacacgctgaaaacagcaggtacatttacctattatgttcaggcggttggcgcaaatggttgcgcgaatccaaaccgggtgccggttagggtaaccgttaacccaatcagccagtcaggtgatatcactatcgcagatactactactgcctgcaccagcggaccagcagtattgactccaactgcagcaggtgttaccgctcctgtattcaagtggtataaaaatgcaaacaaaacatctccgattaccaacggcctggtagaaggcgcggtaagctatgcactggatagcacaggcaacctgaccatcactggcttgactgccggcgcctatacttactatgtaagtgtatccggaaccagtcagtgtgaaaatgcagccggtacattgaaggcagcaacagtacgtgtggtaccagctccagctgctccggttgtaaccggcgatgtggtggtaaccaccggtgtaaaagcggtattaagcgctcaaccggtaccaggggccactattgtatggtatagagatgcgactactgttcagggtatgggtgacaccatccaggtaggaccatttaacacaccgggcacttatacttattatgcggcggtaagaattgccggcgcctgcgaatctgcccgtgcaactgtaaatgtaaaagtaacaggagttgtgattccttctcccgattgtaatgttccaaccagtcagacctcaggtactaccctgggttgtatcctgtgtagtgtaaataatcctactaatgatatagacagtagcaaaaccaacttcactacgctgtctgtacctgttggtgcgctcggaggctcagtatatcaacagctgatcttcccgcatgcaggatctgcagcagacagtgttcaggtacgtcttggtaattcagtaggactggcggacgtaagtctcctgggaggtacactgatttctctctataacaataatgtactggttaaaacagacaccctgtcaagattgcttaccctgcggttactcaatggccagcaattcctggctaccgtagtagctcctgctgcttacaaccgggtagaagtaagaatgaaaggtgtactgaatctcctgaattcaattgatatctatggggcaaggattatatatcctaaaccaactgtaaatacgacaaatgcaaccgcttgtatcaacagcaaggctacgctttctgtaactcctgcggccggcacatctgttcggtggtatgctgattcaaccagcagcaccgtattaagcacacaaaacagttacactactgatacgctgaaagtagcaggtaaagtaacctactatgtagcggtactgggcggaccagacaattgtcctaacccggatcgtatacctgtaaccgttaccgttacacctgctcctcctgtaccaggagttccggctaccgtgaatatttgccctggttcaaatgcgtctctgcaggtttctaacccggatcatcaactgacctacaactggtacaatgtgccaaccggcggtaccaaactgaataccgacagcggctttgtatttaatgtaacagcggttaacagggatactaccttctatgtagaagcggttagcagttgtggtgctgcatcaggcagacaagccatcagcattgtgatatctgcttcattgagcgcgccggtgataacgccaaatccggattcaactgtagtaggcagacaaactgcactgacagcaacttccaatacagcaaatgttcagtttgtatggtatgcaagtcaggctggtaatgacagtctgtttacaggaccagtatacactcctcctgtatccaatgtaataggaaccgttacctattgggtggaagccaggttaacaggcggtgcttcctgcaaatctatcagggtgcctgcagtaatagtttacggacctgaacctggtccggatcctggtccatgtgaaggcgcttctacgcaaacaatcggcggcagcggattactcatattgggtaatgtatacaatcctgccctggcagtagatggcagcttaagcaccggatcttcactggtaattaacctgggcgcattgaacgcacaggtatggcaaagaactaaattcaacggagtatctgctcctggagataccgtaagggtatggctgtcgaacccaagccaggtgctttctgcagcactgctgggtggtgtgcagttaacaacttataatggtaccactcccggagattctctcctggtaaataacccgctcattaaactcactatactgagcagcaagagacaggctatcctcgaatttgtaccgaccaaagcatttgatgcagtagaagtaaaactgaaatcaggcatactcggtgcattaaccacggtagacttcaattacgcacaacgtgcactggcagctccgaaagttcagtcagcacaggtaacagtatgcgcaggcggtaccgccaaactggatgtacagaatcctgcagcaggcgttacttatcgctggtacaccagcaaaggtgtttatctcacaggtaaagatggtgtatccttcaccaccggcaccctgactacagatactgccttcctggtagaagcattcaggaacaattgcgccagcagtggtcgcacaagggtggatgtaaaagtggtggcagcacctgcgcctccggtagtacgttctgcgaatgtggaagtatgtgccggatctgatgcccaacttgccattaacaacccggtaagtggatacagctacgcatggtacaatgtggctactggtggaaccagactgaatccggttccggacagcggcttaacatttactgtgaccaacgtaactgcacaggcaatctattacgtagaagctatcaacgatagctgtaataccatatctgccaccaaaacagcggttaccgttaaaacaggtacatcattggcgccgccaacagtaacacctgtaaacgacaccgttgtgattggccagcgtccgctgttcattgcaaaagcagatgcggctaacgcagaattctattggttcagaacacaaacagcaacagacaccttatttaaaggtgcttccttcgaaggtcctgcgtctaccgccctgggaaccgttacctactgggtggaagcagccctgccgggtgcagcaacctgtaagtctgcaaggatagcggtgaatgcaattaccgtaactccttcaggtcaggtgccatgtgaagccgctaccggacaaacaattggcggatccggcttgctggtgctgggtaatgtatataacccgcaactcgctgtggatgcctttacaagcacaggatcttccctggtgataaacctcggagctatcaatgcaacggtgttccagaaggtaaccttcaacgggttatctactccgggtgatactgtaagagtgaaactgtctaacccaagccagatcctttctgcagcggtgctcggcagtatacaactcactacctacaacggtaacaccccaggtgattccgtattaacatccaatccgatcctgcacctggatctgctgagcggtagcagaagcgctatcctgtggtttgtaccaaccaagcagtttgacggtgtgcaagtgaaactcagatcaggtatcctgggagccttactcgatgttgacttcaactacgcacaacgcgttattgctcaaccgaaagtacaggtgaacaacgctactatctgtaagggtagtcaagctactctcagcgtaataaatcctgcatcaggtatcacttacagctggtacaacagccagggtaatcatttactggatagtattgcatatgtaacgccaaccacactcgattccggagtacatacttatacagtagtaccaaccaggaacggttgtccgggcgccgcatctgcagcgataacagtaaccgttcagggatcaccatcagccccggttccggaagccaataatgtatctacctgtctgaatacaccaactaccctcagggtaaaagctgtagcaggtgttcgctacaactggtacgacgcagcaacaggcggagcaacattggtaactaacagtaatgaatatactacgccggccagtctgcaggcaggtatctataacttctatgtggaagcagtgaatgcaggtaactgcgctaacgacagcggccgcaccagaattacactcactgtagacagcgcctcaacagcggccgacattcagatcacagataaagtaatctgtgccggtgatacagcggtattaacaccaactaccactaccgtacagaaccctgtattcaaatggtacgctaatgccgacagaaccggtccgatcacgcagggtgtaagcagcacaggcgtattaagtatcacaggattaatgccaggaacatacacctactatgtaagtgtaagcaacgccggcaagtgtgagaataaagcaggtgatttgaaagcagtaaaagtaaccgtgaataataccgccacaccatcagacattgtggcggcagatacaactatctgtgcaaacactacggttaaactcacagctgcttccactactgtaacaaacccaatatttaaatggtatgcagatgctgccctgacaacattccttgcatcaggcgcaacatatactaccagtgcattgagcgcaaccacttcttactatgtaacagtagaaggaagcaatagatgcgcaaatgcagccggcagtgcgaaagaagtgaaagtgacagtaagtgatataccggctccgattattaccgcatctgccatcagcatctgtgtaggcgataccgcaacactgagcattcagaatgtggataatacattgacctaccgctggtatagcgcagcaacaggcggtacattactgttcaccggtccggtgtacaaggtaacaggcctcaccgcatcgaaagacttctatgcagaagcttctctgggtggatgtagcagtgctgccagaacgaaggtgtccatcggtgtgggtgttgctccaacgccaatactggaaagtaataatgtaacagcatgtcagggtggaacagccgtactgaaagtgacctcttctgtaaataatatcacatacaggtggtacaccacattaaccggcggagtagctgtgtttacaggcccaatctttaccgtgaataatgtgaccgctaatgcaacctattatgtggaagcaaccggtgacacttcaaattgtggtaaaccttctgtaagagctgccgcgaagatcaacgtagtaccggtaccaccggctccagtactggtaagcaacagtgcggaagtttgtaaaggccaggatgtaacactgcagatacaaagtcctgcagcaggagttacctacgaatggtttgatgcagcaacaggcggcaataaagtgaacgaaggaccaacgtttaatatcacggcactggattctacagtgagctactacgtacaggcactggtaaatggaggctgcccaagcgcaagcagaacgaaggctaccatcaccgtgaagagcgtaccggcaacacctgtaattgcatccacttccctgttcgtttgtcagggtggcagcgtaacactttccatccagaatcctgtggctggtgttacctaccgttggtacagcgccgcatctggtggtacgttgcttgcaacaggcaacagctacgcaaccggcgcattaaatacaagtactgatttctatgcagaagcgaataatggtaattgcagcaatagtgtaagagcgaaagtttccgtaggtgtaggacaagcgccaacaccaatcctggaaagcaacgcactcactatctgtatgggaacttccggaacactccgtgtaacctcagctaccaacggaataatctataaatggtatacttctgccgcaggtaatgattctgtaggtgtaggaccggtattccagacaggaccgctcaatgccagcatggattattatgtgggagcaaccggaactacgggtcaatgcggtaatccatctgcgagggtgaaagctaccgtaacagtagtggctccgccaacagctccggatgtagtagcctccgcacttaaaacatgcgccggcacaggtattactgtatcagtgaaaactatcaaacctggagttacctatcagtggtacgatgctgcaacgggaggcaacctgctttcttctgatgcagtgtacagcgtaccggtggttacccagaatactaccttctatgtacaggcgaacctgggaagctgctccagcagcagaacagcggtagcagtaaccgttgacccaactccgccaatacctgaagtaaatgcggataacctgacaacctgcataggcggtaccgtaacattcagtatcaagggtgcagacgcttcattgacttatcgctggtatgatgcgcagaataacggcgtattcctcgcaagcggtacttcatacgcaaccaaaccgctggccgtaaataccacattctatgtggaagcattgaacagccagggttgcagcagcggacgcaaagcagtaacagcaaatgtccgcaacgatatagacgcaccattggcagatccgctgacagtatgtagcggacacacagcggtactttctgtgaaaggcagacagccgggcgtcatttacaaatggttcaccgtattacgtggcggaatagaagtatttaccggtgcagatttcactatcacaccaacagtaagtaccgtatactacctggaagcatctaccagtggcggttgcatcagtgcaagcagaacaagggtggaagtaaccgtgaatccgtcgccagctgctcctgcagtaaccagtgcaagcattaaagtttgtaccggcctcacagctacgctgaatgcgctgaacccggataatacgctcacttacaaatggtatactgccgcaagtggtggtacagctatctccacaggtgcttcttatacaacacctgctgtaaccgcaaatcagatgtactacctggaagcaaccagcaataatggttgttcaagtccaacacgtaccgcggtaagcgttgaagtaacacttccgccagccggaccacgtgtaaccggaaacgatccggtatgtccgggcagcacagccatactgatggctacttccaccactacggatgtcgatttccgctggtactcagtggccactggcggcacgccgataaccacaggtgcaacatttgttacaccagcgctgaatgccaatactacttattatgtagaagcatttacagcgggtggttgcaccagctccgccagaacaagggtggatgtcagcctggcacaaccgctgcctgcaccagttgtaacagtggataacacaacggctaccgctatcaccttccgctggtcaccggttacaggagcacaacgctacgaagtaacagtagacaacggcgtcacattcacagcgccaagctcaggtgcaactggtaccacacatactatctccggcctgcagccgaaccagagtgctacgatccaggtacgtgccatcggggcatccacctgccagaacagtgcactgtctgccgcagtaacggacaaaacgaagaacccgcaaggcaacaacatctatgtaccaaacctcttcagcccgaatggtgacggtataaatgatatcgagtatgtatatggaaccgccatcgcacagcttgaattcaggatctacaaccagtggggtcagttggtattcacatcgaaagaccagcgtcagggatgggatggtaccatgagcggacagaaacaacctgtaggtgtgtatgtatggatagtgaaggctactatgcaggacggcaccgtgatcacgaagaagggtaacgtgaccctcatgagataatgatgattcatcagcaagatcaaatcaaaaataaaaccggggtgcttcaaggcatcccggtttatccagaaatacttaaaaatgttcctatgaaaaggatttttatagttgcaatgattttatggagcagcctattgccccgcactgctgttgcccaggttgatccgcacttttcgcagtattatgcgtacccgttatggcttaaccctgctctgacaggtgtaatagatggcgactaccggattagcgctgattatcgtaatcagtgggccaattatgggaagccattctcaacagtgggcatttctgcagatgccgccacagataagaacatcggtgtaggcatcaatgtaatgaacatgtcggcaggtgacgcaggctataacttttttaatgcaatggccagcgtttcttataccggtgtgaaatttggccgtaccaaaaccagtcagctggtgtttgggattaatgcgggattgatcaacagaagactggaccctgccaaattccagacaggcagccagtatcagccggtaaccggtttcgatccaagcatatttaacggagaaaatgtaagtaatacaacctccaatcaatttgacgccggcgcaggggttgtgttttttgatggtaatccaaatcatatcctgaacccattcgccggatttgcagcgcaacatctcacacaaccgaaagatccgttttcttccgatggcaccgaaagaaagctgccagtgagatatcttgttcacggtggtaccaagatcaggttgaatgacgctgtgacgcttactcctactggtctttacatgcgacaaggcaatgccgaggaaatcgtggcaggtatgtatgcgcagctaatggtaaatcctgaattcgacttcctggtagggggtaactaccgcttcaatgatgcggtgattccttttgccggtttccatttcaaaagctttgtactgggattaagctatgatgccaatacttccaacatgcgccgcctcgtaaatggcagccagagctttgaaatatcactttcttttatcagccgcaaaagaagaacgcttaacgaagaatactttatttgtcccaggttataatctatcaaaaaccggatcagaatggaggcaaaaacttatacagaaaaaagaaatggaaccctcatgaaaaaaattactctctgttggctggtgatttttgcaggaataattagctctatacaagcgcaatatgtttatgattttaaacatactgcggatgttttttatagctcacgggattattattccgctgcacagtactacaataaggcactgggcactttcaaaatcaagccagagcaggtattgccctatacagttgcaggcgctcctcccagtggtaaactaaaagattatcaacaggtagtagcccggttggccgaatcctaccggctcttctacgactatggaaatgctgaaacctggtatgcacagctggttgggtttaataacccggcatatccccaggcacgatattggtatgccatctgcctccggtacaatggaaagtaccaggaagcactggatgaatttaaaaaattcaaacaaagctacaccgtcgccgatgaactgtctgtaagaaccccgcttgaaattgcctgctgcgaattcgcactttccgaatccaataaggaaccgagatttacgatcgtgaaaactgccggcaatgttaatgaaggcggagcaaactacgcgccggtgatcctggatcccggcactttaatgtttacctcttcccgtgctgagaatccaccgttgccaaccactgttaagcaacccacaacaaaaaaacaagcaaaaaaaggaaccccatatgtaaatgacctttacacagccaccggaagcggcaatactttcgacaacagccagaaggtaaaaatccctgccgccaaaggattcgatcagggagtatctgccattacccccgatggtaattcactttatatcacccgctggtctgtgaaagatggcgtgaaacaatccgctatctattttagcagtcgccagaacggggtatggtcggaaccgaaaatattaggcgagaacgtaaatgttgcagggtataattctatgcagccctatatcacggccgatggaaaatacctgctgtttgcgtccaacaggcccggaggtatgggtaaaaatgatttgtggtattgcatcatgaccaacggcacacccggtggagcgcgcaacatgggcactgccatcaatacgaaagatgaagaacaggcgccattttacgatgcagagaaaaacctgctcgtgtttagcagcgatggccgcgtaggtttgggagggctcgatttcttccagagcgagggcgatttcggcacctggtctgctcccgttaatatgggaaaaccattgaactctcctaaggatgatatctattatacggcattggataatacacatccctttgcagccggcttcatcagctccgacagggaatctatctgctgcctggaagtattcagtattaaccgcatccgtaaaatagcaagcggtttgatcatcgactgcgatactcatcttccactggaaggggctactgttaccctgcttgatactgtgaggaagaaaacaatccgcaaagttaccctggacgccaccggaaggtatacttttgaagtagacccacagcgcttttacaaggtaattgctgaaaaagataactacttcaccaaagcactctattttaatacagattctttagtgcggatagattcaatggataatcccacactttgcctcaagcattacgaaatagaaaaaccaattgttcttaataatatctactacgatttcggaaaggcaaccctccgtgaagaatctaaagtagtattggataccgtggttgatatgctgaacgataatccgaagttaactatcgagatgagcgcacataccgatagcgtaggctccgtgaaattcaatgagaaactgtcgcaggcaagggcccaatcctgtgtggattacctgatcagtaaaggtatttccgcggaaaggctcattgctaaaggctacggtaaatccaggccaattgcaccaaactccctgcctaaccacaaagacaaccctgaaggacgtcagcttaaccgcagaactgaattcaaggtgttaaaaagacaagttcaggtaaaggtggaagatggtaacagtagtagtcaataaagttttcccttaaaccggctgttggtagccggatccttccatatcctgtaataaccatttagaaagccggccccgtggtcggctttttgtttgatgatgttgcagtattttattattaggattccttattaaatatattgcaggagaaagcatgttcattttgtgaacatgctctcaatagttttaatgtaaatttttaacttcctgattagttgcttttgccaaagagaccaatagcaatggtatcagcagctttcatcactttcagatgagaactcagttctatcgcattgttatacttgaatgcagtatctttctgaataccgcctggttttgaaaccttgatagatttcactttcgttaaaagatctattttcagtgcagcaccagttcctttaaacgttcctttcagcagggtatctgttttaggagccgcagcagtaccggctatcaggtaaacgccgtgatccgcatccttaacgtttttggtgagattcagtacaacattcacactgctatctgtgttctcggtgatggtaatatcacctacctttttatctctgtctgcgccggctcctttcagatcaaacgtcttggaacgtggtgttggcggagggggcgttggattatcatcatctttacaggaacttacagtaatacccaatacagtagcgatcactactcccgtcaggagtgtgtttttgttgaacataagcatgatttcagtttttatgaaggttttacgattgtggttttgtaattgtaatgtttgtgatttgtgatcttgttttaatataggttttcagcgcttactaggaatgttaaacggaggtggaaataaaaagttacagctataggtaaagtattttttaaatattttttttcgcctgcctgtaacctttacctattgtggatcgtagcgatcgcattttctctttgaaagaaaatacctgttataactgatgttgatccgcctatttgaaaagatggtttttgatgattgaaaaattaaattacatttgcgaagcatcataagatgccagaactgatagcatatgaaaatttaatcagaccacggtacttccgtttgtcgccctcccacttttcctgttttagtttgcagtgccaatggtgcactgttcctcattgttatttttcaaaagtaagttatgcctcttttaacgaacgcaccgcagcgtatacgtcgtttttttcagttatttaagatagccgttaccggtagtgaaaaggaattcaccactggaagtatagaccgtgcaatatttctgctctctattccgatgatccttgaaatggccatggagtcattgtttgcggtagtcgatatttatttcgtaagtcatttgggtgtgaatgctattaccacggtaggacttacggaatctgtgctcacgctggtatataccggcgctatgggattgagtatggcggcaaccgccatgattgcccgcagaaccggtgagaaggatcctgatgccgcagcgcatgcagccatgcaatccttatacccgggattgctcgtgtctgtactcatcagtatagcaggaatattttttgcgaaagatatattgctggtaatgggggctgccaaagaagtggctgactacggctacgaatatacgcagataatacttggtggtaatatcgtcatcattttattattcctgatcaatggtatctttcgaggtgcgggtgatgcggcgctggcgatgcgctctttatggattgcgaatggcctgaatattatattatgcccgctgttaatttcgggatgggggccggttcctgcattgggcctgaaaggtgcagctatagccacttttattggaaggggcacaggcgtgatgtaccagttatatcacctggtaaaaggaaaagacctgatccgcattacaaaaaaacacctggctccggcatttccgttgattggcgccattcttaaaattgccgccggcgctactgcgcaaatgctgattgcttctgcaagctggattttcctggtgcggattatttcatattttggaaaagatgcggtagctggatatacgatcgctatcagggtggtgatctttaccatattgccagcctggggaatggcgaatgccgctgctgcattggtagggcaaaacctgggggcgcagcagccggagcgtgccgaaaaatcggcctggagggctgccttcttcaatatgatcttcctgggtgtggtggcagtagtatttatggcatgggcgcctgccatcattggtttctttaccaccgatccggtggtaatcaactatggcgtgcagtgtatccggttaatgagtgccggttatgtcttctttgcctatggtatggtgcttacccaatctttcaatggcgccggtgatacgcgcacgcctatgttgatcaatatgtttattatgtggttattccagatgccgttggcctatacactggctatatggcttaaaatggggcctgttggggttttctgggctatggccatatcggagtccacttccgctttggtggctatatggctgtttcgccggggcacctggaagcaggtgaagatttagcttcctgctttctgtataagtagttacctttgcgaggtttgcattaaatttttacataataaaaataactcaataagcatgtcactcacagtcgtaggcactatggcgttcgatgaaatcgaaaccccctttggaaagtcaggtaaaatcattggtgggtctgccacctacatcgcatgggcagcgtctaatttcgtgcagcctattaaccaggtgtctgtaataggcgaagactttcccgcttcagagctggatgcgttgactgctaaaggcgtagctttggatggcgtgcaggtgaagaagggtgaaaagtcgttctattggtccggcaagtaccatatggatatgaatacccgcgattcactggcaacagaactgaatgtactggccgatttccagcctgttattccggaaagctaccagggaagtgagttcctcattcttggtaacctgaccccacaggtgcagatgagtgtactggatcagttgaaggaacgtcccaagctgatagtgatggataccatgaacttctggatggaagtagcactggacgatttattgaaagtactgaaaagagtggatgtgctgatggtaaacgatggagaagcccgccagttaagtggggaatactcgcttgtaaaggctgcccgtaaaattatgtctatggggccccgttacctgatcatcaagaaaggcgaacatggcgcattgttgttttacgaaaatcatgtgttcttcgctcctgcgatgccactggatgacgtatatgatccaaccggcgccggcgatactttcgcgggaggtttcattggccacctcgctaaaacaaaggacatttcctttgaaaacatgaaaaccgctatcatcgtaggttctgctatggcttctttctgcgtggaaaagttcggaacagaacgcatccgcgaaattacccatgaagatattgcggcccgcctggagcagtttgttcagctggtgaacttcgatatcgacctggtgtagcggaggatcgccttcggcgatggaaattgttttggctcaggattacgctgattatactgattttttggatttgatcagttttgattttataagattaagggagatataagcggatatattcgcttgtatctcccttaatcttttctaaaatctaaataaatccaaaaaataaaaaatcaagccaatcagtaaaatcagtgtaatcctgagccaagacaatttacaagcgccgaaggcgcgcctacttgtaaatactattaagaacggccgccaaccggaggccccccttcagcagctgttgattcaggtcggttacaaaaacgtaattgtagcggtagctgagcttggcatcgggttgggtataagcatataccctgtcggagagctggtgtgagtcaaacatccagtcggcgatagaaccctgctgcacggccttaatttccgctgcagacgcaatgtccagcgctttggtgtattctgtataactcagctgctggaaatcgatcaattgttcgtcccataccttatgcaggttggaaggtttatcaaaccacataaccgcgattttgttgccgcccatatcttcatcacggcctacgtggagtggctgatgcatatcgcccatcatatgaaccaggaaggtgagtgcaaaccgttgtttgtctttcggcaggttacggtttttcagatcctttatcatggcctgtgtttccgtgtacaggttttcaccgctggctgcgctcaggagctgatcaaattttgcccggtcaatattgcccggaaaatcgaggtagtgccacttactggtatgatcgtactggtgtgtagtgtctgatttgataaaatcaggccagttggcgatcatcgccaggctttcgcggcccaggatattcgtaatggctttacgcgcctggggggtaagatgaagccaggctatttcggcggtaatacggtgcccgttggggccccaggcaaaggtggcaatgggtaacaggaaggccagtatcagccctattaaaattttttttctcataagtcctttcttgattgtggcagcaaattaaagcttcttttttaacactttcacttccatattctttagtatttttacagatactgctcaaatacaatttcaatatgtcttttaatatacatgctccatacgctccagctggtgatcagccggaagcgatcaaacaattaacaaaaggaatcgaagaaggcgaaccgtttcagacgctcctcggggtaacgggttcgggtaaaacttttacagtcgctaatgttatccagcaggtgcagcgccctaccctggtgctgacccataacaaaacgctggtggctcaactttacggcgaactcaggcagtttttcccggagaatgccgtagaatattatgtttcctattacgattattaccagccagaggcgtatatgccggtaagtgatacctatatagaaaaggacctggccattaacgaggaactggataagctccggctgaaggctacgtccaacctgctttccggcagacgggatattattgtggtagccagcgtttcctgtatttatggtatcggtaatcctacagactatgaaaatggtattatccgcattcagaaaggtcaaacggtgagtcgcaataccttgctgcatagcctggtaaactccctgtacagtcgtactaccggcgattttaaccggggtaacttccgcgtaaagggcgatacccttgatattaacctgccttatgtggattatggttaccggattactttttttggagatgagatagaagagatagaaaccattgatgtgcaaaacagtaagcggatcacagtggtagacaacgcggccatttttccggcgaacatgtacctggctccaaaggatatgatgcagcagatcatatatgaaatacaggatgagctaaaagcacaggtagaatattttaaagctaacggaaagctgatagaagcgcagcgcctgtctgaccgggtaaactatgatgtggaaatgatccgtgaactgggttattgcagtggtattgaaaactattccaggttcctcgaccgtcgtaagcccggcgcccggcctttctgcctgctggattatttcccgaaagatttcctgctggtggtggatgaaagccatgtgaccattccgcagatcggggcgatgtacgggggcgacagatcccgtaaactgaacctggtggaatttggcttccggttgccttccgcactggataaccgcccgctgaacttttatgaatttgagaatatggtgaatcaggccatatttgtgagcgctacccccggtgattatgaactgaagaaaacagaaggggtagtggtagaacaggtggtgcggcctacaggcctgctggaacctcctattgaagtgagaccaagtgtgaaccaggtggatgatctgctggaagaaatagacaagcgggtgcaaaaaggcgaccgcgtgctggtaaccaccctgacaaagcgcatggccgaagaaatggacaaatatcttggacgtattaatattaagtcgcgttatatccattctgaggtagacaccctggagcgaattgaaatattacgtgacctgcggttaggtaatatagatgtattggttggggtaaacctgctgagggaaggattggatttgccggaggtatcattggtggctatcctggatgccgataaggaagggtttctgcgcgatgagcgctctcttacacaaacggcgggtcgtgcggcacgtaatgtggacgggctggtgatcttctatgctgataagatcacggagagcatgcagcggacgattgacgaaacggatcgccgccgtgagaagcaagtggcatttaatatagaacataatattacgccccgtactgtccgtaaaagcaaagaacagatcatgggacaaacttccgtgttggaaatcaagcacttcgatgaaaactcaccgatggctatccatgatgaagtgctgttggtagcggaagatgcgatggcttatgcaaaatcctctgcagccaatgtaaaaaccatcccacagatggagaagtcgattgccaaagtgaagaaagatatggagaaggctgcccgcgatcttgatttcatggaagccgcccgtttgagggatcagatgtttgcaatggagcgcgaattactcgaaatgaaacaataatcggcttcgcaaattcagaacattatatgcaattatttgtaatataaattagttgttccagcaattaaagtgattaattattaatttatatattattgtttaccaggtgtttgcgcggcttgttcccttattacagtagcgcgtgcacctggcaaatttgaaaattgttaacctttccttaatattcttctaatattactgatattcaattatttagattgatattttatcttcctgaaagccgctatatcttaaaaaataataattaatattattataaattataatatcattgatttaatcctaattatcgtacctcttattcaaatatttctatttttagacccttctatttgatgttttaaatttcggacctacttttatttaagaaatttaaaaatcaaacgctatgaagaaaatatcttttcaggactatctccccttcattttccttgcgctcatcgcaatagttggaatttttatgcctgccctcccaagttttgctgatgccagcaaatataattccgctgatatcgcctggattcttgtagcatcgtccctggtatttttgatgactcccggtttgtccttcttttatggaggcatggtaaataagaagaacgtgatttctaccatgatgcaaagtttcattgctaccggcttaatcagcatcgtttggttagtagttggatttagcctggcgtttggtaaatctgttaatggcattattggagatcccagtacattctttatgtttcagaatgtaggatcaggagctccatggagcctggcgcctactattccgctgttactgtttgcgctcttccagatgaagtttgcaatcatcactcctgcactggtagttggagcagtagcgggaaggatccgtttcacttcttatgtattgttcatggtgttattcagtttgctgatatatgcaccaattgcacactggacctggcatcctgatggtattctgtttaaattaggagtactggattttgccggtggtactgtggtacatatttctgcaggttgcgctgccctggcaggcgccctggtactgaaaagaagaaaggatcatatcgaaaagaaagaattacaacctgcaaatattccctttgtattactgggtaccggtttactctggttcggctggttcggtttcaacgcaggttctgctttgagcgccaacgccctcgcagcttccgcttttgctactactaacacagctactgctgctgccggtttagcgtgggtattcttcgatgtaatccgcggacgcaaaccatctgccctcggcttctgcatcggtgcggtagttggtctggtggctatcactcctgctgctggttttgttgctatcccgcaaagtatattcatcggtttcattgcctctatcatttctaatattgcggtacactggaaatccaaaaccagcattgatgatacactcgatgtattcccttgccatggtttaggtggtatggtaggtatgctgctcaccggtatcttcgctaccaaggctgtgaattcagctggtactgatggctggctttacggcaacttcgaactgttcaaaaaccaggtattgggtctgttactggtagtaggttacagcttcactgtatcttacggtatcttcaaactcatcaacctgattcacccgctgcgcgtatctgaagaagaagaagaactgggtctggatgttacacagcacaacgaaaactatcatccttctatgatcagtatctccgacaacggttcactgaaagaagaagacgaactgattcactcctgaaaaacaattcctttcagaggtatcaaaaatgagttacagttctttgagtacgatctttatcaactttattaaacgcatatactttacgttgtaagaacctggaatggataattggtagttaaacttgctgtaaataagtgaaactcgcaccaatcattgattactgattatccattccttctatttttctgaatgtagcatcagaagatactgtagcacgcacccccgaaacaatccgtgagaaaaggccgcattagtacttaccattttatcaaccaaatttataagtatgaaaagaatgttaacgaccttatttgccatgggcagcaccctcgttgccatggcacaatccacgacagatagtacatctgctcccgcgtttaaattatcaggatctgcagatgtgtattataaatacaatctcaacggaaattatactgataataaaaccagctttaccaactcccacaactctttcgaattgggaatggtatcgctgaaagtagaacacggatttaaaaatggtagcatcgttgccgacctcggcttcggcaaaagagccggagagttttcctataacgatgttcccggctccgctaatggcctgtcaatggctattaaacaattgtatgtatcttaccaggtagctgagaaagtaaaaataagtctcggtagtttcgccacccacattggttacgaactggtagatgcctacgccaacaggaactatagcatgagctatatgttcagttacggccctttctttaatacaggcgtgaaggcagatattgccatcacctcttctttaagcgctatggtaggcgtatttaatcctaccgatctgaaatcagttacccttaacagccacaaatatattggtgctcagctgggctttgctccggcagaaacacccatcaaattatacctgaattacctggaaggaaaagatactttcggtatccagaatcatcaggtagacctggtagccacttaccaaatcaacaccgtattcggtttgggatataacgctacctacagtacctataccgacacacgtgcacctaaaagcacccgcgaaaacgcaaaatggtggggcaatgcgctgtacgtgaacctcgatttcactgacaagatcggattaacagttcgtggagaatatttcagtgataaagacgggcttaaagtttttggagccgtaccggatggaggtaatgtagttgccggtacactcacctttaactataaggtaggaaaccttactattatgccggagttcaggctggataaagcctccgcagatattttcagcaagtcggatggtaaacctgctgatatcacatccaatgttttattagccgccacctaccacttctaaaagttgcattcaaacaggtgcaggagtttgccacgggaagagatcgccttccggcatacatcctgcatctgtttttttaaaacccctcccaatggcccctcaaaattcaaaaaaccataaatgatttgtattatcttgctggcaaaaagaagtaatgttgcagccgtccacgttaaaatttcttaagtcactcaggctgaataataataaagtctggttcgatgaacacaaaaccgagtacatggcggccaaggccgattttgaaagcatggtacagcagctgatagatggtttggcaagacaggatgccaccatgcaggggctccaggtgaaagactgtgtgtttcgtatttacaaagatgtcagattttcaaaagacaaaactccctataaaaccaatctcggtgcttctttccaggcaggtggcaaaaaatcggcgtttgccggttattattttcagcttgaaccaggaggcaatagttttgccggcggcggtatctggatgccggcagcccccgaactgaaaaagctccgccaggaaatcgactataatttccgggaatttgaacaaatcatctctaataaagaatttatcaaacactttgggaaggtagagggggatgcccttaaaacagctccgcagggatatcagccagataacccggctatcgcgtatctaaaactgaaaagcgtgattgtgtctcacccgtttacggatgaggcgtgtgtacaacctgctatggtaaaggaaattctgaagacatttgcactgatgcaacccttattgcagttcattaaccgcgccatggactaattaatgtaaagtagtttattagtttatcagatagttaaccttttaatagttgcctgttactaacatgtaaacagtggctgcaaacatcattaaaaagtacaccgcagccaatacccagtatccaaaccaatagatatgcaaatggttctttattctctcctggtaatttcatgatagcggactacctgataaactaataaatacttctccggcttaccccggcttaattcttgtgaatcaggaattcgaacggccgcgctttgcgattctttaaaagattttccttgtccgtgcgcgcgtgagcaaaacgttgattgtaaacattggccacttcaataatcggtataattccgtcaagcgtatcctgctgatcaacgatgttcatgatcctggatacttgtgaagagaaattagtgctccactcttcggtgaacttgtgcattaacagaagctctcgattggtgttggttttcataggacttaagggtgttttctgattagaaaataacgaaaaataccggcatctctaaaattggacttctcttctttttcaaagagttaagttggcataggattattactaccaaaattggattttatcccgcacaaatcaatactacttccgtgtaatttttaaggtttgtgtgttatgcttttgtaacacgcgcaaaaaagagcaagcggtaaaatgcttgctcttaacgagttataaatatattttcgtatagtcatatacgggaggtgctattaagagtggtatactcctaaattacatagcacaacagtatgattacagccagtttttaccggtaaggtattctgctatctgcacggcattggtagctgcccccttgcgaaggttgtctgctactatccacatattcactgttttaggctgtgtttcatccctgcggatacggcccacaaacacttcgtccttatcgtgtgcatcctttggcattgggtataaagccttcgacggatcgtctacaacgattactccaggtgttttttcaagcaatgccctcagttccgccacatcgtattcattttcaaactctatgttcaccgcttcactatgaccacccattaccggaatacgtacagtcgtagccgttaccaggatgctgtcgtccctcataattttcttggtttcatttaccatcttcatctcttctttcgtatagccgttatcgagaaacacgtctatctgcggaataacattcagatctatcgggtaagcatacgccatttcaccggtaataccttgtctttcattcattaactgcgtcactgcctttacaccggtgccggttaccgactggtaggtagataccactacccttttgattttatatttttcgtgcaggggtttcagtaccagcaccatctgaatcgtagaacagttaggattggcaataattttatcttcctgcgtaatagcatcgccatttacttccgggactaccagtttcttcgtagggtccattctccacgcgctggaattatcaattacggtaatacctgccgctgcaaatttaggcgcccactccagggaggtactgccaccggcagaaaagatagccacatttggttgcattgaaatcgccgtatccgcactcaccaccttccaggtcttgcccttaaatgttacttccttaccaacggacttctcagaagccacgggaatcaattcagtaacgggaaaattcctttccgttaacacctgtaacatttttgagcctaccagtccggtcgctccaactacggcaactttcattttgttttacatttttaattttggaagcccaaaattaacatatagcccccgcttttcataacattaagatttttttttaccatttacatggcattaacaccagatgatcaacagaatgctaagtttgaaagctataaaataattgttcatgcggttacccattgtttgttcctgcctgctgctgcaggccctcaccggttttacccaggcgccggctatttatgacgtgattatccacgaggtgatgcccaagcccactcctgtagcaggtttgccaccgtatgaatacatagaactgcggaatatcagcactgcacctgtgcaacttagcaattggcgtttagcagtaaataagcgggaagtgctgctgccagtgtatttgctgcaacccgacagtttgctggtgctgtgcgctcaggcagcagtgagcagttataacattcccaatatcaggggaatagaccgttttccggcagtggcagacgacagcgcgctgattattttatatgacgcattcaaaagggtgatacatgcggtagattatcatcaaggatggtacgcaggcggaaaggccggcaagggcggaatcagcctggaaatgatcaatacggcatttccatgcagcggaaaagtaaactggatggccagtactgcccctgccggtggcacgcccggttccgtaaatgctgtggccgcgaacaccccggatctttccaaaccagacctgctgtttgctgccattgcagatagcatgcgggtgttgttacagttcagtaaaacgctggatagcgtgctggcagcagatcctgcgcgttatcagattaccggtggaatacacataacggcctgccgggtacagcctccgctgtttaacagtgtggaactgcaactggatgcagctatccgcccggaggaggtatatactattaataccagcggactggcagattgcaatggggctaccagcagtatctacaacagtgcaacacttggtatatcacaaccaccggctggcaacgacgtattaattaatgaagtattgttttacccgcccaccggtattcctgaatttattgaactatataacgccagccgcaaagtggtgaacttaaatgagctacgcctttgcgcacgcaccgccggtggcggattaggtacttttaaaaagataaccaccagtggccgtctgctgatgcccgggcaactgctggcatttaccaccaacaaggatttgctttgcagttattataactgccggtcgccggaaaatatccaggaagtaagcggcctgccctccatgccgctcgacggtggggatgttgtgctgctgcgggccgatagtacagtgattgatgaattgccatataccagcgggcaacacttcccgctggccagtgagttgcagggtatttcgctggagcggctggcgtaccagtttcccgcttccgatgccgccaactggcactctgccgctgcttcagcaggatacgcaaccccgggatggcccaattcccagcgccggggcaatgcaggcgattcgttgaatattgtattattgccggaagtgttttcacctgatcatgacggaacagcggatgtaacacagctttcctggcaactgcccggcccgggcttcatgggcaatgttaccgtgtatgatttgcagggcaaaccggtgagatacctggcccgcaatattttgatgggaaataccggatatttgccgtgggatggaattggtgaaaatgcagtagttttaccgtcagggatttatatattttttatagagatatttaatcttcagggctacgtaaaacgctgtaaacgcacggtggtcatggcacgaaagttgaattgacgcacgcccccgttgcccgctttttgcaagctaaaaatagccgcgggcaatctattataattatttatatttgcgcttcctaaaaatttgaacatgcagtacagagaaattgttgcagtaaccggattgggcggtttgtttcagttagtagccagtaaacaagatggcgccatcgtaaggtcactggaagataaaagtacaaggtttgtatcttcccgcgtgcataattttactccactggaaagtattgaagtattcactaccggcgaaaacgtaaacctggctgaggtattcaaagccatggaggaaaaggcagcggcgcacccgcctgtagccggtaaagcagacaacaatgctatcaaagcttatttcaaaagcgtattccctgaattcgatgaagacagagtgtatgtgagtgatatgaagaagatggtaaaatggtttggtatcctcaaagcaaacgatctgttgaaatttgatgagatcctcgccgaaggtgaaggagaagtggaagaagtggcagtagaagaaaccgctgccccggagaaaaagaagaaagcagctcctgaagcttctgaagaagcagctacagaagaaaagcctaagaagccacgcgctaaaaaggccgctgaaaaagaagaaggcgaaacaggcgctgaagaaaaagcacctaagaaagccaaagctaagaaagatgacgcaccggctgcagaaggtgaagagcctaaaaaagctgctaagccacgcaagaagaaaacagaagaatagtaaggatccgggcggtttgatgatcaaaacaatcatctgccggcaaaatatttcaggcttctatttacagagatcattttctgtaaatagaagcctgaatcgttttcgccctccgatatttaacgattcttttagccggaaacaccgggcattagcgtaaaattgcctaaatttctacatccgaaaaatttataaataacagatagcatggataaactaagtgcagatataaagaaactaccgcgtacatttctcccggaagattttaaagtaaccacctgggataccctgcagccttactttgaagcgctgaaggaaagaaaaatcaacagcgcgcaagacctggaaaaatggctgaaagacatgagtgaactggaagcagtgatcagtgaagacgcttgctggcgccagatccgcatgacctgcgatatcaccgataaatcgctcgaagaagcctttgcctacttctgtatggaaattcagcccaaactgcaaccctatgcagatgcgctcaataaaaaactgctggaaagtccgtttgtaaaggaattagaccccgacctgtataaaacctatctccgcaatgtagagaaacaggtgaaactgttccgggaggaaaacattcctatccaggcagaactgagcgtaatggcgcaacagtacggcgttattgcaggtaaaatgaccatcaaagtaaaagaccaggaatataccctgcaacaggctgctaaattcctggaaaacagcgaccgctccctgcgggaagaagtgttcaccaaaaccggcgcccgccggctggaagacaggaaagcactggatgacctgtacaccggattgattttaaaacgcgaccaggtagcaaagaatgccggcttcgcaaattaccgtgattataaattcgaagaactcggtcgcttcgactatacaaaagaagatgccttccagtttcatgaagccattaaagcgcacattgttccgctggtacaacagatcctggaaaagcaaaaagccaaactgcagctggacaccctgcgcccgtgggacacagaagcagaaccagtgggcgtgaagccactggagccattccatacaggtgaagagctggtgaataaagccattgctacttttgatgaactgggccccttctttggcaattgtctccgggtaatgaaacaaatgggacgcttcgacctggaaagccgcaacggtaaagcgccgggaggctataactgcccgctggcagaaacaggcgtgcctttcatttttatgaatgccgccggccaaatgaaagacctcaccaccatggttcacgaaggtgggcatgcggtacactctttcctcagtcatcacctcgcactcagcgccttcaaggaatacccaatggagattgcggaagtagcgagcatgagcatggaattatttaccatggactactggaacattttctttgatgatgaaacacagctccgccgtgcacgcttgcagcaattggaaagagccatcaccatttttccgtggattgccaccatcgataagttccagcactggatctacgaacatccgcagcacactacagaagaacgaaccgccaaatggctcgaaatactgaatgagttctcccctgctgtggttgactggagtggtcatgaagattaccgcgccatcacctggcaaaagcaactccacctgtttgaagtacctttctattatattgaatacggtattgcacagctaggcgctattgccatgtggaagcaattcaaggaaaacaaaacccaggcgctgaataattacgtacaggcgttaagtttaggtaataccaaaacgttgcctgagttgtataaagccgcaggaattaaatttgatttttctccggcctatgtgaaggagctggccgattttgtgaaagcggagatagaaaagatatagtaaggatgcctttgttaacgttccgcgtagcggcattaacaaaggcatttttttatttacaggatttacaaaccccactcaccactacttccacattatgcgctgcataacctttgggaagctgtatctgcggcacatcagtttcgtctaaacaaatggtattgccgcattcttcgcacttgaaatgaatatgatgatcgtgatgatggtgctctgaacactccgacttacataaagcgtagcgtacagatgtatctgtagtgggtattttatgaatgattcctttgtcgaggaatgtttgtaaagtacggtatacggttacacggtcgaacgactgaccggccagcttttcaaaatcgctatgttccagcgcaccgttgcttttcatgaacagttccaggatccttgtccgggtttctgttacactcagcttgctttcgcgcagtatactgccaattcgttctgttatttgttgtttggtgcccatgatgaaaaaaaactttattcttccattaaacggtctatgtcttcaatcaatttatctacatcctgtttttttgtgccttcatacaaaccgcggatttgtcctgttttatcgaccaacgcgaaccattgggtatgtacaaaatcttcttccccggtatatacgccatcgtctaccaggtagccctgcctggccaaccggtaaagctgtttcttatcgccggtgaggaaccaccagtttttggaatcagcgccatgtttggcggcatatgcctttagtaccggtacgctgtcgtgttcgggatctaccgtatgcgaaaggatcaggaagttgggattgtctttatacttcgcatataccctatccatgttggcattcatcttcggacaaataccggtgcaggtggtaaaaaagaactcagatacatagatcttgccttcaacatctgcttttgcttttgtgcggccatcctggtcggtaaaggaaaagccggggatggtatgtcccggcgcgcccaggtgaggcaatttatcttttccaaagaaggtccctgtttctcccttaataatataacccgcataggtcaggaagcctgcgctcaacaacacaaaaaatgaaatcagtataattgctttcttcgacataggtatgattccttgttttattcgatatacaaaggtagcacatagttaacagatgcccatcagtaccacccatctcttatttttttaacacgcctgcaacattttatagttgaaaaaataaattatctgaagataatagatattttaatttgcaacatcgttgcaaatttacgtagttttgtccggatagaaaaatgggaacatggaagtgaatattttaaagaagatgagtttggacaccattggaataggggcttccctgttgtgcgccgtgcactgtgccttactccccttgctgctcacggtattaccattgataggatcgcatgtactggaaaatgaaatgctggagtatggcttgttgtctttctcctttggcgtgggttgtttatcgctggggcgcgggtatttcagacttcaccggcgcatagcgccgctgctgatcttcaccgcgggatttgccttgttagtgggagggcacttcggggtggccggcgggttctggacacccgctatcatctttgccggcgcggcgggagtaacgactgcgcatatattaaacctgaagcgttgtaagcaatgcgccaatgggaaacacggggttcataatcacctggggccatcatccggtaaacagcatttgacagcagagggattataacaatttgattgtaaaacagcagggtcgtatcacccgggacttataaacagtgccacaactaaaatacatagtcctatagcaatataatttatcacatatggaaaaattacctgttacggtgctgagtggttttctcggcgcggggaaaactacgctgcttaatcacgtgctgcacaaccgcgaaaatcttcgtgtagccgttattgttaacgacatgagcgaagtgaatatcgacgcgcaactggtgaagaatgaaaatacgctgcacaaaacggaagaacgcctggtggaaatgagcaacggctgcatttgttgcactttgagggaagacctgctgaaggaagtagctgcactggccgccgaaaaacggtttgattacctgctgatagaatctaccgggatctccgaaccaatacctgtggcgcaaactttttgctaccaggatgaagccaacaacattgaccttactacggtaagccagctggatacaatggtgacggtagtggatgcgtataattttatcagtgactatagcagcatgtcgttactgcaggacagaagcttaacggatgatgcggccgaccggcgcactattgtgaacctgctgaccgaccaggtggagtttgccaatgtgattgtgctgaataaatgcgacctggtaacaaaagaccaactgggcaacctaaaagccgtactgcgtaaactaaatgccactgcccgcatcgtggaatcaatcaaaggccaggtgccgttgaatgaaatactgcacaccggtctttttgactttgacaccacttcccaaagtgccggttggcaggccgaactggaaaatgagcatacccctgaaacggaagaatacggcatctcttcttttgtataccgcagccgcaaaccctttcaccccgaacgcttgtggcagtatatcaatgaacgctggcctggtaatattatccgcagtaaaggattgttttggctggcttcgcggccggatatagcggtgaactggagccaggccggcggatcactgcgcgcagaaaaggcgggctactggtggtgtgccattccccgggcgcaatggcaaatggatcccgaaacctatgaactcatcaccaaccgctgggatacccgctttgcagacaggtataatgaactggtaatcataggccaggagctggatacgcatgatatcatcattgatctcgacagctgcctgtgcacagaatccgagattacaaacttccgggatggtcatctttttaaagatccttttcctggtatttaggctaatctaaaaaataattaagacaagtataaaaatagaagatagttttgttgaaaattaaattggaagtgtgatccattgttactatccgtgaaaacactgtactaaagtttaaaacctacattacttatacgcatgaaacaagtatctacattactattcttcttattaatcattactacagcatatgcccagcaaggcatggtgaaaggctcggtggtgaataaagaggggaagccggtgcaatttgccaacattgccattcctgccctgcgtaccggcgctacagccgaccagcagggtattttcaatataaaaaacctggcagcaggtacttatgatatcaaaatatcaatggtaggataccaaacggttaagctgaagaaacaaattaccgcaggtcagacaacggtattgaatgtttcactggaagaagatctgtcgaagttagatgaagtagtagtaaccggtgtatcccgcgccacggctgtccggaaaaatcctatacccattgccgttattggtaagagggaaatgaatatgaacgtaaataataacatcatcgatgctattattaaaggagtaccgggtgtaagcgcggtaacaaccggccctaatatttcaaaaccatttatccgtgggctgggctacaaccgtgtactgacgctgttcgatggcgtacggcaggaaggacaacaatggggggatgaacatggcattgaaatagaccaatacggcattgcacgggcggaagtggtgaaaggccctgccagtcttacctatggctccgatgccctggccggcgtgatcaacatgatccccgacatcccggaactgacacccggaaaattacagggcagctttctcactgattaccacagtaataacgggatgataggttcttcacttggattggcttaccggcaaaacgactggaaatatgtattgcggggcactgtaaaggcagcgcataattaccgcaacagcgtggatgggtttgtatacggcaccgccttccgggagtataatctctcggcattggcaagggtagataaatcgtgggggcattcccagttcggcgctacactttatgacaatacacaggaaattcctgatggcagccgtgattccctgacccgcaagtttacaaagcaggtgaaagacagtggggatgatataaaagaccggccactggtgccggaaaatgagctgcgcacttacaccattaacccgttgcatcagcgtatccagcattaccgcgtgtataaccattccaaatggaatgtgggtaccggcgatattaatactatgattggcgtgcagcaaagtatccggcgggagtataatcacccggagatgcctgagcagcctgggctgtacgtggtactgaatacattgaactatgatgtgcgctacaatttgccggtaatgaacggattggaaacaaccataggggtaaacggtatgtaccagtcgaataaaagtaagaacggcaccgatttccccattccggattataacctgtttgacataggcggatttatttttgccaggaagtcttttggtaaggtagatgtatcgggtggtatccgctacgataaccgctctatccgctggaatgatttctacgtgggacccaataaacagaatggctttgagcagcatgcgcagctgccggataccgcgggagcccatctgcagttcccttctttcagtcatcagtataccggtatttccggcagcctgggtgctacctggaacatcagcgagcgggtgctggtaaaggccaacattgcaaggggctaccgtgcgccgaatatcacagagattggctccaatggtcttgatccgggggcgcatattgtatacctgggaaaccgtggatttaagccggagttcagtttgcaggaagatattggcattcaggcctggttgccggatgcggatatcagtgtggagttgtttaacaataatattgagaactatatctaccaggcaaagctatatgataataccggcaacccggtggtaattgtgccaggtaacgctacttacaagtaccagcaatctgccgcgaggttatttggagcggaagtgagtgtgaatctccatccgcggagtattgcctggctgactatgaataacagtatcgcctacacgcaggggcgtaaccggaatatggaactgattagtacgcatggcgacgaggcgcggtatctgccgtttataccccccacgcatatacgcagcgagctgaaggcaaccacccaacgcaattatgggatattcaccaaagcctatgcccgtgtggaggctgatattatcgctgaccagccccatttttacggggtggatgatactgaaacatttacgccgggatatactcttttcaatataggcgccggttcgggtattcttaacaaaaaagggaaaacggtgtgtgaagtattcctgcagctggataatgtggccaacgtagcctaccaggccaatatgaaccggttgaaatattttgaatactacagctcctcccccaatgggcggctgggcatatataacatgggcagaaatttcagcgctaaagtgattgtaccgttttagggaagattaccatagtttaagtcccattttaatacctatctggagacttggcagtatgctgaccattttaccatcgttcagtgatactttgtcgtcgtcgaaatgataggtactgtatttatagattttactgcggatacctacgccgatgaagggatccaggataaagcggtcctttttgaactgccggcctattaaaagctgcaggccaattacggttttatctccggagttggtgtaggtaatattactgaaggtattgtcttcattaggatagaacacctttttaacgaataatacaggttcaaagtaagtgccggctgcgcgggagggcgacatttcctgtgaaataagatacaggcgtgcgcctacgcggaagccaaggccccggccgtccacaaattgttccgtactgatgtctggttttttctggccgatgtcaatctttttcgccagcacataatccggataatcggtatagataccactgatacctacctccaggctgaatttatcagttatttcctgttccaggtaaatatcgagttcattaattaaggtggtgggatttactttaagaaaggtgtttttgctcaattgtgttttaccatcctgggcagaggatgataaaataaacgaacaggataaccatattaacagcagtgtctttttcatacagttgtaagggttagactggcttcaggacctccatccgggcgtttgtcagctttcagaaccggtcaataatcgttccacaattaccggaaaccactgatgttccagcgcttgcactttacgtgctaccgactcgggcgtatcttccggtgtaatgataatgcgttcctgcagaatcgtttccccgtcgtcgtatttctcgttcacgaagtggatggtgatcccactttctttttctccggcagcgataacggcttcgtgcacgaaatgtccatacattcctttcccgccaaattttggtaacagggccggatggatattgataatgcggttaggaaaagcctgtaccaggttagcggggattttccataaaaatccggccagcactaccaggtcgatcttttgctcttttaataactggatgtatttatctgaatggaggaaggcctccttttcaatgagtatactcgtaatgccttcgcgttcggcaatctgtaaaacaccggctccgggtttgttacatacaattacggtaaccctggccttatctgactgtttgaaatgatctataattttctgcgcgttgcttcctgcacccgatgcgaatatggcaatatttttcaaaatctcttactgtttgagtagggtacaaaaatagataatttagcagggatttaaagtaatgaatataaagaggcccccaacatgcctggaatacgcttcaggcatgctttataccagcctttgacacgcctttgaggtggacttgatggggagttgaggtggacttgatccttatttgagatattccccgcagccctggtatgttttgtctttcacctgaacctgtacggtattgggtttcatcagtccgctcatatcgtcggtgcaaacggtgttgcggatacttaccgtgatatccggtgtggtatacacctttaaagtatcggtattgggttttgcagggggcagggttgcctgcaggctgtcgccgttaacgttgttgaaacgtatttttttgttatcaagatcgaggctccagaagggttcgttgccgttggcggtgaaccggatgccggcttttgtcttttcggcgagcagttgcctgcggtcgccaccctctacgggcttgaggatatagttgctggccagcacaccttcaatccgtttgcctttggtatcgaggaggaggagttttccttcggaggcgaggaaggaggtgctgtccgttttcttttggagcattacggtggagtcggaggtttgtttccaggtaccggtttccacggaggctatcccctgtcctcttccctggtaagccaccagttcatgaaacgtatgatcgtcaaacaaactgatctggtagtccataccggggcagtcggcgcacgggagggtaccctggtaggtgccggttattactgcgggggtggttatacccggtgtgcttttttgcgtggtgctatcgttttgggtggtggaggtattattattattacaggccacgaaggcggtaagcaaaacggggaatatgatactttttttcatgggagcgattttttcggtggtggattgaacattctggtccgccggcaggttataaaggtaaaaataacaactctcgcagaaattaactgcgctgacagataatatattatattgtgtgttgaaggatataggggaccactatttgattttcatctgcatatattataattatatccccgcaaaccttgccccacgttatgatgtagacgtgcgcccacagaggaattgaactttcaattaaaataataagttttgaaaggaaatattaaacaaagtgtttaaataggccagcagcaagactttcagctcaatcgttgttcaaaaaacgggttaaaaacagcattctataagacaataattttttttaattgttggtaaattgtcaacattctgtcttatttttgctggcacttttaagaaactttaggtcaaatctaaactatataggctgtgtatcgtcgtgtttccattcttttgcgcaagcattttgtgagtgtgcttattctatgcgctagtatagtaattccgttttcttctgttaaggcagcggatccagcgaagggtaaagcattattccaaacaaattgcgcttcctgccataatgtccataagaagctgacaggtcctgcattagcgggggtagaagatcgctggcccgataagaaattattgcaccagtggatccataactctgcgtctgtactggctacgggagacaagtatgctaatgctctgtacctggagtacaacaagacagcgatgacgccgtttcctcagttatccaacgaggaaattgacgacatcctggcttacgtaaaagttgagcagagcaagacaactggtcctaaaacatcaggtgaacccagtccagatggtgctgaagacaaaggcaatgacaacagtttactgtttggtatcattacactgatccttgcagtagtagcgctgattctcatgcagatcaacagcaacctgaacaagctggctggtgataaagagggtgttcctactccggatcctgttcctttctacaaaaataaagcttacctggcgctgattatcctggtgctgttcatggtaggtggttacttcactattcagggggctatcggcctgggtcgccagaaagactatatgccggagcaaccaatcttctacagccataaggtgcatgcgggtatcaaccagatcaactgtttgtactgccacgccggtgctgagaagagtaagcatgccatgatcccttccgagaatatctgtatgaactgtcataaggccattaaggaatactccggtcctgagctgacaactgcagaaggtaagaaggtagatggtactgctgaaattgcaaaattatacgattacgtaggatgggatcctgaagctggtaaatataccaagccaggcagaccgatcgaatggactaaaatccacaacctgcctgaccacgtttactttaaccactctcaacacgtggttgccggtcagcaacaatgtcaaacctgccacggtgctatcaccgaaatggatgaagtacatcagtttgccgatctctctatgggatggtgtatcaactgtcaccgtactaccaaagtgcagtttgctgacaacaactattacagcatcttcgaaaagcttcaccaggatattaaagataagaagatcgatagcgtaacagttgagatggtaggtggtactgaatgtcaaaaatgtcactactaggaaggatttagagagattttctcttaatcagaagatatcaaatttataaacgtaactcgttaatataacatggagcaaaaaaagtattggaaaggcttggaggagttgcacaataccgatgcgcatcaggaaattgtgaagaatgaattcagtgaagaacttccgttcgagagtgaaggcctgttgaatgctactaccccccgcagggattttctgaaatatctggggttcaccaccgctgcagccgctattgctgccagctgtgaaacaccggttaagaaagcgattccgtatgtaaacaaaccggaagagatcaccccgggtgtagccaattattatgcttcttcttacgccattgatggcgaatacgtaccggttgtggtgaaaacccgcgaaggtcgtcccatcaaaatggaggggaatactttatcagctatcacacagggcgctacatctgccaaagtacagggcgctgtattaagcctgtatgatactgcccgactccgtttcccatctatcggtggtacggaaacaacctgggcagaactggataaacaagtaggtgcagcactggccggattaggcggtgctcctgttgttttattaagcgccactttactcagccccactaccaaaaaagtgatcggcgagttcctggcaaaatatccaaactcccgccacgtagtatacgatgcagtttcttactccggtatgctgcaggcaaatgaagcctcttacggtcaaagagttgttccttcctaccactttgaaaatgccaaagcgatagtgagtttaggtgcagactttatcggaacctggctgaaccctgttgaatatgcccgccagttttcttccacccgtaagatcaatgcacagaaacccgaaatgtccaaacttttcgcgttcgaaagccatatgagccttaccggtgcaaatgcggacgaaagatatacacacaaaccttctgaaaccggtgcagtagcactggcactgctggcagcagttggcggcagcgtaaccgctccggctattgctgacaaacgtgtagcagatggtatcaaaaaagcggcggaatcactgaaggccaatgccggtaaagcactggtagtaagcggttctaacgatgtaaacgtacagatcattgtaaacgccatcaacaacatcgttggcgccaatggtactaccatcgatttcgcatctccatccaactaccgtcagggtatcgacagcgacatgaccaaactggtaagcgatatgaacgcaggcagcatcggcgctgtactgatttatggcgctaaccctgcttacgactacttcgaatctcagaaattcgcagaaggtctgaagaaagtgaaagtcgcggtatcctttaacgacagaaacgacgaaacaactgaactgtgtaaatatgtagctcctgatcatcacttcctggaatcctggaacgatgctgaaggaagggcaggttactatagctttgcccagcctactatcctgccgctgtttaaaacacgcgctatacaggataccctcctcacctggtctggtaacactactactacctgggctgactacctgaaaaatgagtggatcagcaaactgggcggacaggaagcatgggataaagcattacaggacggtattgttgaaccagctgcagctcctgctttaggtggtgctacatttgccggtgatattgccggtgctgcatcgaagatcggcagtgccaagaaaggtggtaaactggaactggtgctttatgaaaaagtagctatcggtaccggcagatctgccaacaacccatggttacaggaaatgcctgatccgatcacccgttctacctggggtaactacgcctgtatctccaacaaactggctaaaactttctctactcaattaggtgatgattacgaaatcaacgcagagaagaaagtgctgaaggtgaaagccaacggtaaagaaatcgaactgccgctgctgattgttccgggtatgcaccctgaagtaatcgctattgcagtaggttacggccggagcaataatgtaggaagagctgccggtggtatcggtaaaaatgtttatccgcttgttagcttcaatggtcagaacttcgactacttcgctgttgacgcaacagtagaggctaccggtcaaaaagaaattgttgctttaacgcaaacacataatagctacgaaggtcgtccgatcgttaaagaaactaccctggaagagttcatcaagaaccctaaagaggtaaacgaagacagactggaactgaagaaatttggtcctgacttccgtaaggatgctaccctgtatcctaattacagctaccctggtatcaaatggggcatgtctattgatctgaacacctgtttcggttgtggtgcatgtacaattgcctgccaggcagaaaacaacgtttctgttgtaggtaaagaagaggtggctaaagcgcatgaaatgcactggatccgcatcgaccgttacttcagcggggatgaagagaatccggaagttgtgttccagccgatgttgtgtcagcattgcgataacgccccttgcgaaaacgtttgtccggttggcgcaaccaaccacagctctgaaggtattaaccagatggcttacaaccgttgcatcggtacccgttactgcgctaacaactgtccttacaaagtacgtcgcctgaactggagagactggaatggtgctgacagctttgaaaacaacctgtacgatgtagctgatatgaacgataacctgacgcgcatggtactgaacccggatgtagtggttcgtagccgtggtgtgatggaaaaatgttctttctgcgtacaacgtttacaggaagcgaaactggatgcgaagaaagctggtcacccattgaaagatggagctgctaaaaccgcctgccagcaagcttgtggcgctgatgcgattgtatttggtaacatcaacgacaagaacagcgaaatctataagattcgtaacgagcagcaggtagacaggatgtactatgtgttggaagaaacacacgtactgccatctatcagctacctggcgaagatcagaaacaaggatgccgctcctaaagcagaaaaagagtctgctcacaaggaagaagcgcatcacgcgtaatggtcttaaccggtaaccgttaagaaaaagacagaaagaacagaatctgagatcataacaaaagacaagggctagtagctagaagctagcagctaaaagcttatagaatatgcatttaaaatacgaatccacactgagagaacctttggtagacggggttaaggattatcaccaggtaacggaagatatcattagtcccattgaagggaagcccggaaaactgtggtatgtaggctttttcatctccctgacactgttgggctttggtgccttttccgtgttctggcagatctatttcggtgtcggagtatggaatctgaataaaaccatcggttggggttgggatattaccaacttcgtatggtgggtaggtattggtcacgccggtaccctgatttccgcgatcctcctgctgttccgccagggttggcgtacaggggtgaaccgtgcggcggaagcgatgacgatcttcgcggtaatgtgcgccggtcagttcccgatcattcacatgggtcgtgtatggatggcgtttttcattctgccttatccaaatacccgcggtccagtatgggttaactttaactctccgctcctctgggacgtatttgcgatctctacttattttaccgtatccctgctgttctggtactctggtctccttccggatttcgccagtgtacgtgacagggctaaaacaaaattgcgcaagttattatatggcgtagcagcattcggctggaccggttctaccaagcactggcaacgtcatgaagcgctgtcgctggtactggcaggtttggctactccactggtattgtctgtacacacgatcgtatcttttgactttgcgacttctgtaattcctggttggcatactaccatcttccctccttactttgtggcgggtgcgatcttctccggatttgcgatggtacaaacgctgctgatcattacacgtaaaatattacatcttgaagaatacattaccctgggtcacatggaagccatgaacaaggtaattgtgttaacgggttctgtagtaggttgtgcttacctgactgagttattcatggcatggtatggcgctaacccttacgagttcgctactttcttcaagtatcgtgctgccggtccgttaggatggtcatattatatcatgatgacgtgtaacgtggtaacgccgcaggtattctggttccgtaaaatgagaagaaatgtaatggtgactttcgtaatgtccatcattgtgaacattggtatgtggttcgagcgtttcgtaatcatctgtacttcactgtaccgcgattacctgccatccagctggtcatactatcgtccgtcctggcctgaagtaggtttctacatgggtactttcggtttgttctttacctgctatttcctgtttgctaaatatttccctgtaattgcactggctgaaatcaagtcaatcctgaaaacatccggtcagaactacaaggagaaaatggaagtgtacgaagaagagcctgcagagaaatttgctcatgatgtggctcacgcacattaatagatgaattaagagaacttattacctggaatttgaatttttaaatatatggctgttaaaaaatttgttgtaggcttgtttgacgatgaggcggtattgtttccggcagtaaagaaagtacgcactgcaggatacaaattgcacgatgtatacactccttttcctgttcacggcctcgatcatgcaatgggtttaagagaaaccagtctgcacacagccggtttcatatatggtatcactggtaccactacagcattgggtttcatgagttgggtgtttaatgtagactggccgctgaacattggtggtaaaccacatttcccgttaccagctttcattcctatcacctttgagctgaccgtattatttgcggcggtgggtatggtgatgactttctgttatctgtgccagttaatgccgggtgtaaagaaacacatcttccatccaagacaaacagacgataagtttgtgatggtaatagagctgacagaaaaaaccaatgcggaagaagtaaagagcttcctcgctgctgcaggtgcacaggatatcaatgagcagaaggctgaagcaggatggtggttcggaagatacgataaggacgatgagccttatctccgtaagattcagaccgcaaacgcttaattaaaataacagctaaaacataccgttgcgacattaggatttgagcaagcaagaactaatgaaagctagataaataatttctgatgaaaaggacttccaacatattgattgtagccgcattggcaactggagctttcctggcagcctgtaacagaggggagcataacagaaagcccggcaggatttatatgccagacatgtatgaatcccgtgcgtatgaattttacagtgctcgtttgtcaggcctgaagccagtggaaggaacagtaaaaagaggagaacttttgccataccatctgaaagaatcagatacggcactggctaatctggtaaagaatccattaactattacgccatctgatctgaaggaaggcgaacgtttatttaatatctactgtggtatctgtcatggtactgcattagatggtaatggtccgctgtacaaaggtggagatggaccttatcctgcagctcctgccaacctgattgccggtgcaaaatccggttacacagaaggccgcctgttccatgtaatgacttatggttataacatgatgggtagttatgccagtcagctcgacagagaccagcgctggaagattgctgcttatatcaagagtaaacagccaggtgctgccgccccgtctgctgctcctgctaacgatagcactgcagctaaataaatgagttaaactgaatttcaatcaagtattttaatatacagtaatgaaagaccaatttgtagtaccggcaagattaaaaaagaccagcttcgtgttaatgggcgtgggcttgctgacgttattgatcggattaattgcgtttcgaggtgagaacgcgacacggttttgggccggtctgttgcaaaacagcagcttctttttgctgattacattggcgagcaccttctttatagctgccactaccctggcacatggtggctggcagattgctttccgccgtgtacctgaagcgatttcaatggccgttcccgttttgtctgccattttatttgtgattgtaatgatccttgtttttggtggaaaagaagatatttaccactgggtaaacgcacatcacgtagcggaggacaagatcctgacctggaaatctgctttcctgaacaaaggattctttaccgtagctactatcctgacactgggcctctggatattctttaccctgaagctccgcaaaatgtctatcgaagaagatggatgggatctgcgtcctgaaacaggccgtaaattactctggagaaataccgttgtatgcggtggcttcctggtagtatttaccctgagcgttggatctaccacaccatgggtttggttaatgagtattgatgcacactggttctctaccatgtacagctggtacactttcgccagcacctgggtatccggtctgtcgctgatagcactgttcgtagtatatctgaaaaaacacggttatctcacttatgtaacggaagagcacctgcacgatctgggtaaattcatgtttgcattcagcattttctggacttacctctggttctcccagtacatgctgatctggtacgccaacatgccggaagaaactgaatacttccagccgcgtgtttggggccagtggagaccaatctttttcctgaacctcctgatcaactttgttactccgttgttgttcctgatgaaaagggacaccaaacgtaactatactgccatcgttttcatcgctattgtgatcatcttcggtcactggctggatttctggcaaatggtttacccaggcaccgttaaaaccctggtattcccttggtatgaattcggactcggactcggtttcgtaggactgatcatcttcctggtatctaaccagctgactaaagctgcattggttccgaagaatcatccttacctgaaagaaagtatcattcaccacacctaatagggtgatcaaggagattaggcaaaagaaaagcattagataacttaattatttcatatagcaatgtcaggatttttagcagtcttagttgttgttctcatattcatagtcatcttccagattgcgaaggcgagcgaatatgtgtccatattgaagggagaaaagaaagcgcgcgagcaaagcaaccgtataaatggtttcctgctgattgcattcctggtgctggggcttataggagtgtactactgtaatgatttgctgaagggcaagatcctgggcgaatctgcatcagaacagggcgaaggcgttgataccctcatttacgtaacactggccatcaccggtatcgtgttcgtggttacccaggttgcattgttctggtttgcattcaaataccaggagaaagaaggacgtaaagcattttactttccgcataataataaactggaagttatctggaccgttatcccggctattgccttaacagtactggtggcttttggtttgaaacactggttccagcttacctcagaagcgccaaaagacgctgctgtggtagaagtaaccggcaaacagtttaactggatcttccgttatcctggtaaggatggcgcattgggtcgtcgtgacattaagaatattgatccttccgccggtaatgaactgggtctggactggaacgatcctttgaacaaggatgactttatgcctaccgaactgcacctggtagttggtaagccggtaaaattcatcattggttcccgcgatgtaatccatgacgtaggtttgcctcacttccgcatgaaaatggatgcggttcccggtatccctactaccctgtggtttacgcctaagtttactaccaaacaaatgaaggaaaaaaccggtaacccggatttcacctatgaaatttcctgcgatcagatgtgtggtagcggtcactactccatgagaggcgtgatagtggtggaaactcaggcagaatatgataaatgggtagctgcccagaaatcgacatacagcctgacacacgctgacactgcagctccggctgcgcctgccggcgaagccaaagcagatagcacacaaaaagcagtagctgcaaatattcagtaagctgtaattttgtgtagaagaatttttgacggagtacaattaaaaactaaaaagacaaactgacaaacgacgatacttcccgggcgttagtttataataaaccgaaccgattatgagtaacgaagcaacattgcacagtcaacaggaggtaatgcacggagcgcatgatcatcatgatcatgagcaccaccatgaagacagtttcatttcgaaatatgtgttcagcatggatcacaaaatgatcgccaaacaattcctgattactggtatcgtttgggctatcattggtgctttcttctctgtactgttccgtttgcaacttggttttcctgatgccactttcccctggctggaaagtatcctgggtcattgggctaaaggtggccgcattacagcggaagcttactatgcactggtaacaatgcacggtaccatcctggtattctttgtattaacggccggcctgagcggtaccttctctaacctgctgattcctttgcaggtaggtgcacgtgacatggcctctccctttatgaactgtttgagctactggttcttcttcctggccagcctggtaatgatggcttccctgtttgttcaaacaggtccggcttccggaggttggacgatgtacccgccgctgagtgcactgggagacgcttccatcggttctaaaataggtgtggatctttggttgaccagtatggcgctgtttgttgtttcgcagctgctgggtggtttgaactatatctccacactgctgaacatgcgtaccaaaggtatggcgatgaccaaaatgcctttgactatctggtcattcttcttcactgctgtattgggcgtattgtctttccctgtattgctgtcaggtttcatcctgctgctcatggatcgtcacgctggtaccagcttctacctgtctgatatctttattgctggtaaagcactggcaaatgaaggtggtagcgctattctctatcaacatttattctggttcttaggtcaccctgaggtatatattatcatcctcccggcgatgggtatggtttctgaagtactggcggtaagttcccgcaagcctatctttggttacctggcgatgatcggttccctgttcgccatctgtatcctggccttcctggtttgggcgcaccatatgttcgtaacaggtttgaatccgttcctgggtgcattcttcgtactcttaaccttattgattgcggtaccatctgccatcaaggtatttaactggatcactactatctggaagggtaatatcaactttacgcctgcttccctgttctctatcggttttgtgagcactttcatctccggtggtttaacaggtatctggttaggtaactcttctatcgatattcacctgcatgataccatgttcgtaatcgctcacttccacattgtaatgggtgtatctgcgttctttggtatgtttgccggtatttaccactggttccctaaaatgtatggccgtttcatgaaccagaccattggttatatccacttctgggtaaccatgatcggtgcttacctgatcttctggccaatgcactacgaaggtatggcgggtatgccaagaaggtactatgatgtatccggctgggcttccttcaaacaatttggtggtttgaatgagttcatcactatcgtggtaatcctggtatttgcagtacagctgctttttgtgttcaacttcttctacagcattttcaaaggtagaaagatgaccacacagaatccgtggaacgcaactaccctggaatggactacacctatccatgccggtcacggtaactggcctggtgaaattcctgaagtataccgttgggcttatgactatagcaaggatggaagagatttcattccgcaaacagagcctatcggacctaatgaatcagcgcactaaaatatagttcggaattccggcaggaagacacctttcaggcgaaaaatcttccttccgggattttgttcactgtgatgtttgtaaatttgttccggacttaaacccgggatgtggctagaaaaaaaatgttgcaagaaaactccataaaattgtcgtcatcatatgcggtagcaagcaaggtgaaagattactctcagttaatgaagtttaatctcacctttatggtggtattttcatctgtggttggttacctgctggtgcctggcgtggagtttaacttagtaaaagttcttttattatttgctggtggtttgctggtttccggatcagccaataccattaaccagatttgggagaaggaaacagataagctgatggcgcgcaccgctgttcgtccattgccttccgggcgtatgcacgacaacgaggcgatagccctggctgcggtaaccggtgttgccggcctcctcgtaatggggtactgctttaactggttaagtgctgcattgagcgggttatctttggtgttatacggttttgtgtatacgccctggaaaaaatggaactctcttgcggtgctggtaggggctattcctggtgccatgcctcccctgatcggttgggcagccggcgccaacaatctgagcgaaggtggctggtcgttgtttgctatccagttcctgtggcagtttccgcatttctgggccattgcctggattgcgtataaagattatgcgagggcaggttttaaaatgctgccgggcagcggagagcccaacaagtacaccgccatacaggccgccatgtacacgttgttgctgattcccgccggcgtagcgccatacctcctgaagatcactggaagcatttctgccatagtggctattctggcgggaggtttcttcctttacagggcagttaacctgtacagaaagaacgatgttcctgcagcgagaaagctcatgttcggatcttatatttatctgacaattgttcagctggtacaactgctggacaaagcgtaaaatgaaaagaggagtgatggatactatgacattagaacaacgtaagaaaatacatccgcataaatattccttatggatcgccatgggtagtattaccatgatgttcatagggtttaccagtgcttacattgttaaaagatcccaggcaaactggctggcatttgaactgccgcatattttctggatatccactgccgtaattttaaccagcagcgtaacaatacacctggctttaaagcagttcagagaaaggaatatgcagcgttacaaacaactgatcaccctcacagcatttttgggtgtggtgttcgcggcctgccagtggataggattttcacaattgaagtcggtaggactgcccctcaacgggcctgtttccgcttcttttatttatgttatcgtaggagtgcacatgctgcacgtgctgggtggtgtagtagcactgcttattatgtttggcagggcttacagaacccgtgtacggacctacagcgcagtgcccattgaagttgccgcaacatactggcatttcgtggacgtactgtggatttacctgttaatttttttaagtatcgccagataaactttgtaaaattttataaaacaaacaatggatacagcagttacagcgaagaaaaaatggtgggccggaggatattctccctttaatgtgagctatggtaagttgatgatgtggtacttcctgatgtcagatgcgttcacattcggcgcattattgatttcatatggtaccatccggttttccagcccgtcctggcctgatccgaatgaagtgttccgctccttccctggcatgggccatgccaacttaccgttggtatttgtgagtttgatgaccttcattctcatcatgagttctgtaaccatggtactggcagtacacgccggtcacatgagagataaaaaagcagtggccaaatggatgatctggaccatcattggtggtatcgcgttcctgagctgtcaggcatgggaatggacgcatctgtaccacgaaggtgcatggtggggtcgtaatcctttcatgaatgttgacggtacactggcatctaccaactttaccaacttcttctttactattaccggtttccacggtttacacgtaacttccggtgtgatcctgaatatcgtaatccttgccaacgtactgaaaggtacttatgagcacagaggtcactacgaaatggtggaaaaagtaggtttgtactggcactttgtagacctggtttgggtattcgtattcacctgcttctacctgctctgagtaaaagacaggcagaatagtacaaggtttgttgttgattatttggaatctgatttttagaatttatttaatttaaataataatggagcatacacatactgaggctgggcatgaagctgcacatgccgattcatctaccaaaacaatctggagaacgttctggatcctgttgtgtatcacaatggtggaagtaggtctggcctttttacatctggaaactggtttcccgagcagggtattcctgaatgccatcttcgttggtctcaccgtggtgaaagctttctatatagttgctgaattcatgcacctgggtcacgaaatcaagaacctgatccttaccatattgattccgttactgttatttgtatggtttatcgttgcattcctgtatgaaggggattcctggaaaaacatgcggaaagacctgaaaccaggtacgccggtggaagcaccaaaggctcctgcaaaagaaggacatcattattaatttcatcataaactatcaggatcatctctcgcagggctttattaggagtgtcgttggctatattggtgccgcttttgggttatctcattgtagatcactacggaaaaaatgtggtacctgtacccggatacttcatcccggaaagagtagatacgatctctgaagatggtaaagtttcatacgataccgtttttcataagatcagggattttaaacttaccaaccaacttggagaacaggtgagtttgaaagatatggaaggaaaagtgttactggttgatttcttttttacctcctgtccaagtatctgtcctactttaacaaagaacctgaaaaaggtacagagcgcttatgtaaagaatgattctttgctgcagatcctctccttttcagtagacccggaaagggatacggtagataagctgcgtaagtacgcctacgaataccagataaatcccgataactggtggctgctcacaggtagtaaaaaagaaatctacgacctcgccagaaacgacttttttgtttctgtaacacagggagacggtggtccggacgactttatacataccgagaagctggtattaattgacaaaaacaggaatatccggggatattataacggtcttgattccaatgatgtaaaaagatgcgcaggcgatatcgccatattgcatctggcaaaagaaagacaccgaccgggttttggagccttcctcaaaaaactgttctccggagagaagtaataaaataattataaaggaaaggtgaataaggaaaggttgttcacctttctttattcaccttttacattttagtggatatggaacttaagaacagaaatctcaatacgcctatcaccatcgtatcgatagttatacccgcattggtggcgttattgtttgtgttgcccaagccggaaatgcatcctggttttgatatcaggatactaccgctgttccacgctatcctcaataccagcactgccgttttactattggccactttatattttataaagaacggacatgtaaaagcccataagatcaccaatttaattgcagtgggtttgtcggccgtgttcctgctgtcgtatgttacttatcatgcgttggctacagaaacccggttcggcgacctggatcacaacggtattgtggatgccggtgaaaaagccttgctgggcggtatccgttatatttactatttcctgttgctgacacatatcgtactggcggctattattgtgccattggtgcttttcaccctgctgcgcggcttccagaatgatattccgcgtcatcgcaaaattgcccgtattacgtggcctatctggttttatgtggcagtaacgggtgtgattgtttatattatgatttctccctattaccactgatagaattaaggagatttttttaagacagatagcctaattttgtgagatcaaacaacaatactatgaagaagacaggtttgtttttactgacagtgtttttgacggtgatgagcggatcagtaatggcgcaatgttccctgtgtactaaaacggctcagcagctgggcgaaggcccggcgaaaggtttgaacaatggtattctgatgctggccctaacgcccctggctatcataggttttctggcattccggtggtggagaagtaataaagaagcctgacaattttcgtataacccaaaataactatgattacctacagaaaggcggatatcacggatatcccgcagttagtgcatttgcggctgcagtttctgaaagaaatttaccctaagtctgataactcccaggatgccgtgttgaaggatcagctaagggtctacttaacagaacatctctctaaaaacaattttgtaaactggtttgccgatgcagaaggcaaggtggtggccagcgcgggcatagttttttataaccagccgccgctgtaccacaaccttgaaggcaaagtggcctatattctgaacgtatacacgcttcctgccttccggcggaaaggtattgcaaaagcgctgctgcaaaagatcctcgatgaagctaaagcacgcaataccgggaaggtgagcctgcataccagtaaagaaggacgtttattatatgagcagttcggctttgtggccggagacaatgaaatgacctgccagttgccccgtgttcaataataacggctactcttcgcggagtttgaaaacaggacattccattcttaacccaccgttgtttaaagagatctttagtttgttgcagtggtaacccttcttttcgttgagatgctcacagttaaagcacataggctgagtggaaataatttcctgttgattcagctggtaaatcagctgcatgagctgctccagcagtccggcctggtctttcaatggcagctgtgctacggttgcgtgcagtggatccgcaaattgctctactttcctggcaaccgcttttccttcccttaccaggtgtaaagtgtggctccgggtgtctgtagggcttgccttacgagtcaggtagttcttctgttccaatgattttaccgcatcgctgatggtggctttggtcatgttaaagtacgatgccaaggtggttacagtacgtttttcctccgggtagtgcagtaaaaaggtaagtacctggatttgtatgggactaagtccatactgagttgcttcctgccataataatacgcggaaggcttctgataatcgctccagggaggccactactttactaggtgtgtcttctgcctgctgtgcagggctgaatgtggaaactttccccatatattcttgctgtccttatagttagtgtggcaaggtacaatataaatatatggtgtgaaatagcatattagtgacattcctgagtgaatccggcttttttcagtgacaaccctccaattcatggatataatagcctttttgccggatctgggtttcccagcgtggtataatttcagtgatatgacaaaagcggcagtctttccgggaaacaattaacccctctccttttttggtttgaagataggtattgccataattcagtacttcatcaaaggaggtttcctttgtgacgatgatatcgaaatgaagatatctcccatcttttttcttaacataagtgtcgaatacagcaacttccataggaatacttttgatactaacgtaaatggttacactaaaaagggagttgtcggggttgagggtatacccataacaatacactaaaacttattgctttgaaccaggcctgctgcatacgttctacttcagcagccgggcgcccgtgtttacttaaataaggccggcctgcttcggaaacggggtatataaaagaagacaggtaacgtaagtataccatgggcaacgggtccatatcatgctccgctgaagacctgaactgaagctgtgcagcaatccgctcttcaaactgccaccacggcttgccttcctggcggttacataaatcagtgatccatttacggaaatgcggacggagcgattgcaggtaccccacgtcgggagcaccgttcctggtaaaataggtggcgagataattattctttagtatggtatcataccagttattcagaatgtcttctgtatgtgcagcgaggatgtttcctgccatcatcaggtattgctcgtcctcatgggtgaataacaacatcctttttaatctgaccagggtttgtgcatccagtgagggttgggggttatcagcgccagctgtgccttggtgcatagcgtcattcatacatgttgaattttggtttccgtcacggattggttattacaaatataataaggttgcctaactaaaacaataaatataatgacgtatattcctatacgttagctattaaatacattaataaaaaattatttgtgattctacaatgaactatatagctttgataatctggttgataatacccctttcatgattaataagctatacgcaataacaaaaaacggtttaccggttgtaccggcagcagcatatgaacctgcagatgtacccggtaaaaaggcatcgcgcactttgtatctttctgttgcagccatagtggcagcagcgggaggcgctgttgcagcatggggcattaacgtcataatccatgcgattgcttcactggtttactacggggaaatagatactgcatacaggggtatcgaaaatacagaacgggaatggtggatcattggtattccggtggcgggcgccctgttccttgttgccatagcccggtatacttcgttcctgcttcgtgcattgggattgaccgttgccatcggggccggtaatccgttgggagtagaaaatgccgccatgttatttaacgggggcttaggcgcctggatcggtaaattatttggctgcaccagtgacgagtgcagactgctttttacagcaggcatgtgcagtactttaggcagcctctttggagcgccggtggcggctgtactcctggcattggaagtgtttctggcagaatggacgcttgccagtatattaccggttgcagccgctgcagccactgctgccgcaggaagctacctgtatcgtggcaccactcctgtattaagctttacagcactgccggctatgagtgcaaaggccatgataggctatatgatagtagctttaatagtgggattgtgggcaagattaagtacagcattgtaccatcttattggtaaatggttcggcgtgctaactaaatacaatgcctggtatttgttattggcggcattgcttacgggtattattggatatattttcccccggatactgggcaccggcgaaggttatgtgcgtgacctgctggaggcacacgtaacgctggcgattctttttacactggcctttatgaaatggatcgcctggattttcttctccggcgccaacaaaacaggtggtggtatcattccattgctgatcattggaggcgcattggggttgttgattggagcgcccctgcaaatggcttttccgtctttaatgattaatgcagggattgtagtgctggtggggatgggagctatgctggcgggtacttcccgggcggtgttaacagctattatattactgctggaaatgacgcatgatattaatgcagcgcttcctgccatacttgcctgtatcctggcttatggtattgctgtcttcaaacgtaaaaaacgacaggaactaaccagggcataattattaattaattctgcggagcgcttcccgcctgctgagtggcgccagcgtgtgactgtctgcgaattttcgcacactgccggggtttgttttagcatactcccgcaaggcccagccaatggctttctggataaaaaactctttagaacttgcgcactgttttatatagcggtacaacagctgttcattggtatgttgcttgtatgcgttctggtgtataatggccgcacgctgcagccacatattttcactattgatccatcgattggtagtggcgggccattcttccccgaattttttcagccacggaccggcgaggcacgacacgatggcatctacgctatcccaccacgatttatgaactatcatgtattcaaagagatggatatcttctgcgcgccattccttgtttaacatttgcataaaatctatggcagcgtattggtattcacgttccggttttttccacaatgcttttatcagcaccggcatatcaccaatggcgggtaatccatatgttgctttcaatcctttgttgataagacggcgctccggcgcagttatacccaggtattcaaactggttgcgcatatacgctttcatagcaaccgcgttgtccggattggcggccaccaggtatgcatccgtgatcagggggaggtagcgcatgtatgcttagcttttagtgctgatataacggtaaaggttaaacgctttttgccggataagttcctgtatttcctgttggagggtttgtttagagatatctctcatacgcctgtgttgtatcagttgccaggctttttccgccagcagcaggatatgtttttgttgttgatgggagatgatagtgtgatgtttttcgatggcctgtataatttcgtgtatgcctgactgttgggtggccacggatttgatcaccggaatttcccagtcgccctgatgtttactatgtgcgagcagccggagatttttcacaaaagcatctgcattgtcgcggtcagctttgttcacaataaagatgtctgcgatctccattaaccctgctttcatggtctggatctcatcgccggcttccggaactactaccacaacagttgtatctgctataccggctatttccacttcactttgacctacacctaccgtttctataaagagatagtcgaatgcagctgctttaataagatcactcacctctataattttaggacttaacccgccaagggcgcccctggtggccatggagcggataaatacctttggatggttgaagtgttggctcatcctgatccggtcgccgagcagggcgccgaaattgaatggcgaagaaggatctaccgctatgatagctacgcttttatcctgttccagtaattgagtaatgagtgcatttacaagcgtgcttttacctgcaccgggagggcctgtgatacccactactttggtgtggtcagtcacgggtatttgttccagcagctgttcatatcccgttgcttcgttttcaacaagggaaatgcaacgggccagtgatttgatatttccgtttaagagtccgggtatatgctgctggtacattttattgtttacagaatttaaagaacaaaaataagcggtatccctgtttacgcgatcagcgaccggtaaatatcaagatattgtcctcctatctcctcccatctgaagctgtcggcatgctttttaagagcagccattggctgggtagcttcgtaatgggccattcctttattgaaaacatcccgcatgtaggcagggtcaaaattttcgaaatagtaggcgaggttgccgccaatttcgggcaggctggttttatcagaaaggaatactggtttgccatagtgcatagcctctattacaggaatgccaaagccttctgcaatagacgggaatacaaacgcggcgcaattgctgaaataccagtatttgcttttctcatcaatgggaccgataattttaacccggtccagcacaccgtaggcggctgcttcctgcaggatctgtttctgataggtggtatttgcgtttcctgctataatcaattcataatcagtgtctttcagcagtcgcggaatgacatgaaagttcttcttgggtaagatggtgccaatggtgaaaagaaacggccgggaggggcggtaaagcggggcgttaaaggaggggaatgattttacatcgcaaccgttataaataacgctcaatggagtatctcctatttcaagatgttgtaaaacatcttcctttacataatttgaaatagtaataagatgatcagctttattgatcatccgctgcactttggccagctggcccgatattttgtgtttatagttaggcttgtataagaaattgagatcatgtatagttaatacccgttttatgtcgggtgatgaaggaatgtagtcagataactggtaggtggtatgccagagctgaatatcttttgaatagggcatccagagtttatgccatgctttttgtttgtagtgtgcctgatttgaaaaaagtgtttctttataggagggcagatagaagtacaactcctcgggaggagagatcagctgcatcagagtttggccaagttcgctgcaataagtatatagaccgttgttcggatatttcattctttcacagtctatcacaaatcttggcatgttaatcagtttgaataattgtcaggtatatatttatatataactaaatgcttaagcgaagatattacaactttttacgaaaaagagataattatctttcggccttttccagataaatttatcagcctggcgtatattggtcgtcagtccgatggcgaataattaatacagatgacgaattttatctccatatttccgcttggaattgtagtgtatccgggagagcagttgaatctgcatgtttttgagccccggtacaagcaattaattgcagcctgtttggccgagcaaaagccgtttggtattccagttgtaataaataaaaaaattatggaatatggaacactcgtccaaataaaaaaggtagaaaaaatatatgagagtggggaaatggacataattaccgttggagacagtgtttttcgcattttggagcatgtttcggaaattccggagaaattgtatgccggggccattgtaaactacccggagaataatgaagccggtaataaccggttgctgcaggaagtattgcatggcgtccgggaattgcatgctatcctccagatccataaatcgtttaagaaagaagacagccagctcagttcatacgacttggcgcaccatgcggggctgtcgcttgatgaggaatacgaaatgcttcatcttttctacgaagcacagcggctggagtacctgaagcggcatttgcacaaggtaattcccatgatggcggagatggaaaggctgaaagagcgtgttttattgaacggtcacttcaggaacttatctgccgataatttataatttttatgaagatgcccgcctgacttgcttttccgggcatcatgaccgcaactttaacgtgcatttaacaggtggttttttggatttttttgcttcccgccttaaaaagtagatatttgcagacccatattttcactggaataagggcttaaactcaattctgatactaaatgcattggacaaaagtcagtattctttgcctgcttggaagtttttttctattggcaaataaggctatcgcacaggacaattcaccatattcccgctacggattaggagatctgcataataaccagaacacggtaaaccgtggaatgggaggcgtttctcaggcttatagtgatccgcaatcagtcaactttattaatccggccagctactccagcctgctgcttactacctttgatgtaggagtggaaggtggcgcccgctctatcacagaccagggggcaaaatttagttccggattcggtacactctcttacctgcagttgggtattccgttgattaccaacaaatggggattaaatctggggcttcgcccggtaaccagggtttcctataacatccaggaatcaggtaccggtaccttctttgatacattgaggattccgctcaccagcaaatatgaaggaagtggcggtctataccagttatatgccggtacaggtgtgcgttttggtcatttcagcgtgggtgtaaacctgggttatctgttcggtaacatcgagaacaatacccgtcttaccttccctgatcctaccatgtatgcttcccaccgcatgttccgtacttcctacaacagctttttctataaattgggcgtgcagtacagggccaagctgaaaacggatatggatctgacgtttggcgcctccggaagtttgaagcaaaatatgaatgcccgccaggaaatactcaatgaaaccgtgcagttcgacgcatcttccaataactatgttacacaggataccgttcactatgcgaaaggcgacaggggaactgtggtgtttccgcaagagtttggcgcaggtatcatgttgcgcaaatttgataaatggatggttggggtagactttaattccagccaatgggagaattataaaaactttggtaataaagattccctgcagaattcctggaagcttgctatcggcggacagtttgtacccaatgcaactgcactgagcggttactggaacagggtagcgtatcgcctgggtggttactatgggaaagattacctgcagctggaaggcgtaaatatgcctacaatgggcttcacggtgggcgctggtttacccgtacgccgcatgccttattccaaccagtacagtatgatcaacctggcgtttgaagtggctcaccgcggcaacaacgaaaccatcctgaaagaaaatatctaccgtatatcgctgggctttaccctgagtgataaatggtttatcaagcgtaaatacgaataacttttttgcacagcgcgtattttgtctttctcaggattacgctgattatactgattttattttttaagatttggggagatataagcgaatatacccgctcatatctccccaaatcatttaaaatccaaagtgatcaaatccttaaaatcaataaaatcagcgtaatcctgagaaagacaaaatacgcttatatctccgctgcattaagctgaaagcgaattcctatctttgaagtattattcattcaaatgattaaaagagccatcttattttttattatagccattgccgttagtagctgcgaaaatgatattgatgcggtgatggaactggattccaaaaaggcagccaccgaaaacgggcaggatattgtaatcatattcagccagggtggaaaggtgaatgcaaaattaacggggcccactatggagcgtggtttggataagccaacctatgtggcctttaataacgggctgaaagtatttatgtataacgacagcctggggctggaaagcacattatcggccaagaaaggaaaatttatggaagatgatggagatgtgttcctgtcggatagcgtcattgtaattaataagaagggcgagcgcctggatacgaaagagctgaactgggatcctaaaagaaagatcttctactctactaaagaagtgtttatcaaaacgcctaccgactcgctgcatggatggggactggaagccaaccaggatttcagtgtaaagaaaatactaaaggtgagcggtcctattacagtacaggacagtactgctgccctcaactgatctcactaacgtaaagctatatacgaaagaaccccacctatgcaggtggggttctttcgctttaacctattttttaacctaaaatttgggataaaaagtcaataattatgccagtttgccatgttttccgcattgtttgttaccattcataacatttgaagataatttataagcgccgctggcaaagctgttttaaacttcagccgggatggctatattaggcgaaaaattagcgcatggaaactatcagctggcccgattttgaaaaagtagaaatgagagtgggcactatcctggaggcgaacgattttcctaaagcccgtaatccttcctatcagttattgatagattttggcccggaaacgggaatcaggaaatcctctgcccagattacccatctctaccagaaagaggacctgatcggaaagcaagttgtggcggtggtgaactttccgccaaaacaaatcgcaaactttatgtcggaatgcctggttttgggcgctgtaggcgataacaaggaaattgtattacttcagccggacaggaaagtgcttaacgggcaacggatagcctaaatagatttgataataaactgtgtaaacttctctatcttctaattatcagttaattatagatatttaaatcatataattctgaattttaataatattattattaaaataatataataacacattatccattatcatcagtttacgaacaataatacatcgttcacggaaatgaaacctattcctaaaatcggcggtatatctttgttctaggtttttcataggatatggttaaaattattacaagggcggtattcttaccagcccttttttttgcttttttccagtcctaaagccgaaaaatggcaaaataactgtttaaacaccttcttaggctgataatcaatttattgtatgcctgtactcacataccagcttatcatgaagtgttttttgccctcatacgttcaccttcacttttgatacgtttaccggataaaatatatcattcactagaatggccatcgcagtgtgataaaaatcggccacctttggtataggtttttcaataaagatatggttaaaatttttcggggctgtagtcttgcagccctgtttcttttttctgaagtcctatttttccctctgcctttctctttctccggttattttccaaacagataaacaacattacggcttaacaaacagatacaagcgtatatctgtatgttaagccgtagcggttttatagcagtgtgcctatttagtgaatagcgccggataaggtttatccaggaggttattataaataaagcggtaagactcaccggaagaatgaacgcttttcaagccaccccatccgtgacgttcgccgggatacagcataaactcgaaatgcttattgagattttccaatttatcgatcagctggatacagttctgcatatgcacattgtcgtccattgtaccatgtacaatacggatcagccctttatacttatcggcataggtcattactgaggtagccttatagccttcgggattctctgcgggtgtatccatatagcgttctgtatagtggctgtcgtacaattgccagtcagttaccgcgtagttggccatcccataattaaatacatcggcgccataggtgagggccatacaggtcatataaccgccaaagctgccaccggtcatgcatattttgccggtgtcggtccagggttgggaacgaagccaggtagcagcgtccatataatcctcgatttcgtgtttacccagttggcggtgaatatagttcatgcccattttgccgagctgtccgctgctgcggttgtcgatggctacctggatcacgccttcctgcgcccaccattgctgcacattaccatatttccaggtatcgtatacggtaccggcatttgggccgccgtaaatgctgatcaggaccgggtattttttacctggttccatgtgcacgggcatggtaatggtaagaggaagtaccagtccatcgcgggttttgtatgttttcaatgctgttttggccaggttgaaatcgtcaaagttttctcctttactatcgcctaattcccgcaccagcttgccattgttgtccagcagtgccatttttgaaggcgtttgcaggttggaataagtagtaataaagtatttacctcccggcgccagtttgattacattattatagttaccgttggttaaacgggtaagcgcgccggttttcatgctcactttatacagatcgaagcgggtggaggcttctttgcgggcggtgaagtataccagttgattcttatcatctatctgaagtacttccttcacggtccagttaccggaagtcagttgttttttcagggagccgtccatattatggagatagagatgtgaccagccggttttatcgctttgcagcaggaatccctggttattttgcacaaaaggaacggcatcgaaccaatcgatccaggttttctgcttttcatcatagatttcctttttggcgccgctttgcgggttgatgctgtatattttgaggttgtcctgtccgcggttcatccattgcatccacagctgccggctatcgtcggtccagaaaggcataccaaagtactgatcgtcgttttcattaaaatcggcccaaacggtggggccacccgtaacgggtaccacgcctactttcacagcgggattggggtcgccggctttgggataacgcgtgttttccaggtatccgtgctgtcctttttcgctgtagatagggaataccggcactttggtgtcgttaaagtgcatgtaagcgatctgccggctgttaggactccaccaaaaagcgcggtaatgtgtgggacgacccaggatttcttcataatatacccaggatgcccatccattatatattacatcagaaccatcggtagtatagcgggtttcctttttggtagctacttccacgctgtataggtcattattgcgggtaaatgccacatattttccatccggcgacagggttggattcttttcctctgcgtcgtcgttggtcaaacgaactatgttgccatcggcggctttatagaatacatccttttcacgtatttctacactgggaccgtctaccggggccgtataaatggtggctttgccggtgcgggcatctacagaccatgcctgcatgcggccatttgcctcatccgggcgcatttccaggtaatgttctccatctgcccagtcgcggatggctggtaatggtttggtgatatgggtagctttgcctttaaaagcctgttcataggtgaggtcctgcttttgctgggcctttaaacagggggcagtcagcagcagtaagcctatactgccgatagtggctggttttaaccattgttcgcttctcatcatttgtaagatatcaggtggttgttttgttgtcgttagcggacgaaaataagcataactaaaaaatagcggtcacaatttacacaaacgggcggcgcgtgcaagccggggacaagtcaaataccaccagatatgaaagatttccccgcgctggttaaatagggctgtaaatggcagtggaagcggttatctttagtctggttttcataggatatggtcaaaaaataagagggctgtagtcttacagccctttttactatttttgcactccattagtgcaattaaattactacatgacacaattatctgagcaagagattatacgccgggaaaaattacaggaactgcataacttaggtatagacccctaccctgcagctgagtacccggttaatgatacttccgtaaatataaaagccaattattcggaagaaacaaaggaacaattccaggccgtatgcctggcaggccgcgtgatgaacaagcgcgacatgggtaaggcctcatttgtccaggttcaggatagcgtaggccgtatccagatatatgttcgccgggatgatatctgccctggtgaagacaaaagcggttacgatgttgtaatgaagaaactgctggacatcggcgattttatcggggtgaaagggtatgtatttattaccaaaaccggtgaaacctctattcatgccacagaaatcaccatcctgagcaaatcgttgcgcccattgcctattgtgaaagagaaagaaggagaagtttttgatgaagtaaccgatccggagttcaaataccgccagcgttacgtggatctggtgatcaatcccgaagtaaaagaggtgttcatcaagcgtacccggatgatgcaaacgatccgcgacttctataataacctgggttacctggaagtagaaacgcctatcctgcagcctattcccggcggcgctactgcccgcccgtttgttacgcaccacaatgcgctggatatgccgctctacctgcgtatagccaacgagttatacctgaaacgactcatcgtaggcggttttgaaggggtatatgagtttgcaaaagatttccgtaacgaaggaatggaccgtacccacaacccggaatttacggtaatggaaatgtacgccgcttacaaggactacgagtggatgatgcgcaccaccgaatcactgctggaaaaaattgccctcaccttacatggcaccaccaccgtgcaggtaggcgatacaaccattgattttaaagcgccattccgccgggtatctatgtatgaagcgatacaggaacataccggttttgatatcgccaatatggatgaagcacagctgcgcgatgtatgcaaacagctgggaatccacgtggacgccaaatttggcaaggcaaaactgatagatgagatctttggtgaaaaatgcgaaggcaattatattcaacctactttcattaccgattacccggtagaaatgagcccgctcaccaagaaacaccgcagcaaagccggtttggtagaacgctttgagctgatggtgaatggtaaggaaattgccaacgcctacagtgaactgaatgatcctatcgatcagcgtgaacgttttgaagaacaggtgaaactgatggaacgcggggacgacgaggccatgtatattgactacgacttcttacgcgccctggaatacgggatgccgcctacctccggtattggtatcggtatcgaccgcttaaccatgctgatgactaaccagccatctatccaggatgtactcttcttcccgcagatgaagccggaacaacagaaataaaatcatcttaataaaataaaaggcgaatggctacggtcattcgcctttttgttttatataatataaatgtggcattaaattttcatgaagcgttcatataccaatgcacatcgttaactttaagtagtgcttattagtatcttaaaattagcccatatgaaaacaattttagtacctactgatttttctgataccgcttataatgccgctacctacgctattgccctgggaaacagtttagaggccacccgcattgtattgtaccacgcatatgagctgattgtaccaattccggatgtacctacggcgattccgatggtgaatccggaggatctgagagacgccagcctggaaggtttggaaaagatgaaggcagagctgacccctctcatccgggaaggtaccacgctgcttacacgtgcggataacaccctgctggcagctactattgaagaagtatgtaaaaatgagaacgccgacctgattgtaatgggcattaccggcggcagtaaactggaagaagtgttggttggttccaataccattgacgtagtgaaaaataccagttacccggtgctggtggtaccccaatcagcaaagtataaacccatagaaaaaattgtttttgcagcagacctgcggaaggtggcggaaaccactcccgtggaaccattgaaaaaactattgcatatttttaatgcggaactgcatgtaatcaatatagatcatgaaagcaggcatttcagcaccgatacaccttttgaaacactgatgctggataccctgctggaagatttccatccggagtaccatttcatcgataatcccaatgtagtagcaggaattgtggaatttgccgaagaaaataaggcagaccttattctcactattcctaaaaaacacggtttatttgaaagcatctttaaacgcagccgtacttccaaactggcgtatcaaacacatataccactgttgactttacacgaataatttatacttttgaaagatattaatatttataataacactatgcttaaacgttcattattggtattgctgggtttctttagcctgcaggccactcaggcccagttcctgaagaagctgggtaaacagctggaaaccgccaccaacaagagtagcagcacgagtaccggtagtggtacttcccttgctggtttgactgaatctgacgcaggttccggaatcaaggaagctttggctaaaggcgtggctgccggtattgcaaagctgaataaaaaagatggtttctttggaagtgatgtatataaactgttactgccggaagatgctgtgaaaattggcaacaccttacgggcaattggtttaggcagccaggtagataaggctatcctgcaaatcaaccgctccgcggaaaaagcagtgggctatgccgcacctatctttgtgggcgccattaaacaaatgaccctcaccgatgcactgaacctcgtgaaaggaggaaatacatctgccactgatttctttaaaagcaaaacaacagattccctgaaaaccgctttcatgccggtgattaagaaatcgctcgacagcaccagcgctacccgttattatgcggatatcgtgaataactacaataagctgcctactaccttcaataaagtaaatcccgacttacaggactacgtgaccaccatggccgtaaatgctttatttgaccagatagcgaaagaggaactggccatccgtgccaatcccgcagccagaactactgacctgctgaagaaagtattcggagcaaaatagtaccaacgataaaaaaggaaaggggcagagatgatgatctccgcccctttccttttttattttgcggcttaatagctgccggccagtaatacctgccatgctgcggctacctttccttcatccagcaacttctttgcataatagtgcaactctttttccatttcatccggtgttacgctgtaatactggatgatatttttgagatgatcatcatgaaaggcggcatctacaaaaggaacttcatgaacattacccagttgccccaggtggttgccggtaagaatgtggctattcctgatggccaacggtaacgcatcaacgccgatgcccagtttggtattaggttttgctacctcaaatacggcatcgccggaggcccggcaatagtagtcgcctcccatacgggctaccaggtctattttatgcggatctattttaccattgatatccagtatgttttcgttgatatgcagcattaccggctcgcagataaccaggtttcctgcgccgccaccctgcccggtttcaatgatctctcttacaatacattctatttgcaccgggctttcttttacccggaaaggctgtactttttcagatttcaacggcgtaaagccggctttttcaaattcatttacaccagcgggatattcgcagctcgacaaagaggcctgttgcaccataccataacttaccatgttgatgaccacctctttggtggcgtatacattttccagtgtatgctttaccgtgttatcacgtacgcggcgcgatggtgaaaagatcagtgtagggggattggagccaaatacgttaaagaaactgaagggcgacaggtttggctgcccatccgcatctattgtgctggcaaagcaaatggggcggggagaaaccgcacccaggaggtaagcatgcagctcacttgttttcacctgtgatggatctatctgcatggttatgcttttttcttaagggccagcagcgaaaagccggtatcttcttttacgatagtattggataaggtacctaagccggtaacttccatttccactacatcaccaggttgcagccattgttcggtatagtccggatcattcagtttgccggtaccgttcagttccaggaagcagccggtgcccaccgtgccactgccgataatatcgccgggcaagatgttaacgccataggcgcagcgttccacaatttccgcaaaggtccagtccatatcgcccatgttgccttcactcactgggatgccgtttactttgcaggtcattttcaggttaaagttgttgccggtatgtccgtctttcgccggtattttcaagggttccagttcatcggcagttaccagcatgggacctactacggtgctgaaatccttgcctttggcggggcccaggttaagcagcatttcttccatctgaagggtgcgtgcgctcatgtcgttcatgatcatgtatccaccgatatagtcatcggcttcagcggcggtgatattacggcctgccttacaaatgacgatggctacttccagttcaaaatccagtttttcaaaatggtcgggcatgcatacaatttcgccgggaccctggatagcgttatgattggtaaaataaaatatcgggtattgatcgaattcggggatcatgggcaccttgcggttgcggcgtgcggccgcaacgtgctgacggaaagcatatccgtccctgcaggaagtagggaatggtacgggcgacagcagctgtacgctgtttacggggataccgatagcggagctggggtttttcccttctttcagcagggcatcagcgcgtttggcgatgtctatcacatcttcccacatcatcaggaacatgcccatattattgggaagatccgggtacagctcctgtgtattgtataacagcccgtccaccaggatggccagttgatctgtttcttctcttaaataacttactagtttcatggtttggtaattgttctggttgtatgaaggatcaaatataagaatggcggttaaaagcattggctatttttttgtgtcctgccagcgaattactttatatttataaacagaaccaccaatatgcgttgctgtttgctgctactcctgatgtatggccaattgttcgttgtgcaggcacaaccccgcacagatacgctgctgaaaaacctgctggaccgtgaagcgcctccggccctccggcatgtgctgcaatatcctgattcgttccgttaccagcttatttatacgcaaatagaccgggatgcccgtaacaggccacatttcaagagctattacctggaagtggacgggaacaagtacttcaatcccgccagtacggtaaagctgcctattgctttgctggcactggaaaaaatgcatgaattgcaggttcccggccttcacaggaatacgcctatgctaaccgacagcgcctgggacggacaggtaaccgtgcacacagatagttctgccagtaacctgttgccatcggtggagcactatatcaaaaaaatattcctcatcagtgataacgatgcctataacaggttgtatgaatttgttggtcagcaaaccattcacgaaaagttatgggcaaaagggtataaagatgtacgtattgtacgccggtttatgccgcttacggaagaagaaaaccggcataccaatcccgtgcgttttgtggataacgggaaggtgatatacgaacaaccggttgcatacgatacccttacctttgattacagccggaaggtaacgctgggacaggggtacctggataaaaatgataagctggttttttcgcctatggacttcacaaagcataacaacctgccgcttacagatttgcagcaaatgctgcaatcggtattgtttcctgcgagtgtgccggcatcacaacggtttgatattacggaagatgattaccgttttttataccgttatatgtcgcagtatccgtctgaaactttgtggccgaaatatgacaccgctgaatattacgacagttttacaaaattcttttttttcaaggccggtaaaaagaacattccgccatatatacgtgtatttaataaagctggctggtcctacggtttccttactgacgtggcctatatcgttgactttaaaaaccaggtggagtttatgctcaccgggaatatttatgtaaacagggatggtattttgaatgatgataaatacgaatatgaggaaaatgggcaccccttctttaaggaagtgggggaaataatttacaggtatgaattacaacgcaggaggaagcataaacccgacctgcaaaattttaagataaactatagagattgacaggagggaataaatattatttatagccttatagagtaatatagtgagcgaaataatacatgaacgttgtatttttgcgttcgatggtggcatccatcttcaaaatgcgcatcatttttgaggcggctgccagggtagataaggaaggttttattcatatcccgtaactgcactctaaaatttgggagttatgaagtttgaaaagattaagaacaaaggacaggcaagattatttgaaagccagtatcttgagatgcttaccaaaacgcatccgttggtgatctgggggctatatttgcccattattggctacatgctttactatagccacaataccttaggctttacacccggttcagtagcaggtatattctttggggccatgttattctggtctttttttgaatatatcatgcaccggtttctgtttcactttgcgagcgacagccccagggtgcagcgttttatttatgtaatgcatggtaaccaccatgagtaccccagagacaaacagcgtttatttatgcctccggtaccaagcctgatactcgcgtccgccatttttggtgtacaatatatcttcctgcgtgaaatcacgtttatgtttttccccggctttatcctgggatacctgatttatgggagtatgcactacgccattcatgcgtggaacccgcctttacggtttatgaagccattgtggcgtaaccatcacctccatcactataaaagtgaggataagggttttggggtaagttcgtccgtatgggatcatgtattcggaaccttctttgacctggaaaaggaaaaggaggacaaggaaaaagtgaaggagctaacattttaaatgtaaacaagaaggggtgatgcttagcatcaccccttcttgtttaccatctttcttcatcatcgggcaaatcgttttgtttataggtggcccgggaaattatcttctgcagttgtctttctataatgagcgcagcaatggatttataagggtcttcccctgtagcggcggcattctccagtattccttctacctttttctccgccacatctgtacgatagagcaggaatataaaccgagagaaattttcgctgatcagttgctgtagtttgcccgccagtatttcttccagcagttcataactaacattcacgggcacacttatttcgaagttgtcctgtgtccaggcagctgtttcctggagatattgcgctggctgtgcggtcattatttcatttgtttgatcttgtaggaggcgttggtaactacttttaccggtactttcaggtcatgttttatacgttttgccttatcggccttgtaggtatagttaccggacatatcggtgttttgtacacagatgctgggtaagccgctgctgcggtttatcaggtaattggaagaagtggtgccgctgatttccgcggtagctttgatcccgtcatccagggtgagcatctgcaccttatcggtattgatttttgaggtaccgccaatttttgctgtttgtgcatcccatgtctgcaggttccagtaaagatctatccggcctaccagtccgccgcgcaggggtacattttcttcccactgggtgccggttttaatgccatgtgctgggtacatgatcagcagttgttctaaccagctctggaacgcttctgttccgaactggtctttcatcagtttcctgtaggcttcctgttcatcctttttaagggtgctgaaagcgccggcggcgttgtccaggatagtttccagcccgtctaccttattgatgataccggtggtttgtatttctacagtaaagggttgatccagcactttttgcagcccggcctggaagggttcttcctgtttggtgacctttgcatctacaaaaatattctgatttttagcgttgaaattgaatttcagatccttgtaccggaaagtgaggatggttttgcctggttctacggaggttacctccatggtaatgatgttgttgtaatcgcgggtggttctttgtacaatttcattcaccgtcatataggtttcgctcctgcttttctgttccagttcaaatagctctcctttattgaaggtatagttgagggctacatattcctgtgctttaacggataaagacagtgttactaccattgcaatcagtcccaggattcttttcattatcatttttattttatcagacatatttttcgatcaccccgaggccaaacaaggcaaaatcatatttggcaggatcatcaggatccagtttcttcagctggtgtgtgagcgcggtggctgttttccaatcggcctttggctcggttataattcccagcctggtggccactctgcttacatgtacatccatcgggcacaccagttgcgaaggtgatatgtgctgccagagcccaaaatccacgccattttcgtcatttctcaccatccagcgtaaatacatattcaatcgcttgcaggcagagttctttgccggtgtggcaatgtgcttaacagttctttccgggtgttccagtgcaaaaaatactttccggaaccccatcagtgctttttccacattttcatcctgcggggtgatgtgggcactgaaggcaaattccagcgatgttacattggtgtaataatgctggagaaactctacaaagtacagcagatctaaaccgttgaaagtacggtgacagaaggaaagtaatttcatacgatcccgcggctggtgatgacggataaagtcatacggcgaatcatccatcattttcatcagttccgtgcatttgttgataatactggtacggtttccccatgccagtacagcagcaaaaaggccggcgatttcgatatcctgcaatacactgaaccggtgcggtatgctaataggatcattagctataaagtccgggtgattatagtatgccgccttggcatctaaaaactcccttaatttctggatcttcataagtttaatcacgtgtattaccacaagcctttttacaccggaatcttcaattcagatataaaaaggcgctggatatggttaggataaatatttacgcttcccggtaaagataatttttaccgcataagaattaaaatctattacttagccgatagcttttgcaagatcttcggtaagatcatctgcatcctcaatacccacgctcagccggatcagggagtctgcgagcccgttcttcactctttctgtacggggaatagaggcgtgtgtcatgctggcgggatggcctatcagcgactctactcctcccagtgattctgccagggcaaataaatgggtgttgctcaggatccggttagccgactctatgctatcatctttcaatgtaaaggacatcatgcccccgaagcccctcatctgctgtttggcaatatcatgattaggatggtctgtaaatccgggccagtatactttatccactctcgggtggttacggaggaaattagcgactattaccccattttcacaatgacgctgcacgcgtacatgtaatgttttgattccgcggagcaccaggaagcagtcctgtggaccgggaacagcaccgctgctgttctggataaaatacagttgtttggcaaggtcttcattttttacgatcacggcgccatgtaccacgtcgctgtggcctccgaggtatttggtagccgaatgcagcacgatatcggcgcccaggtcaagcggattctggagataaggcgatgcgaaggtgttatccacacataagatgacttcacttttgcgggctatggtggcacaggccgcgatatctatgattttaagcagtggattggttggcgtttccagccatatcatccgggtttggggggtaatatgggcttctatgttccgggcatcagacatgtcgatgaaattgaaccggataccataacgttcaaacaccttggtaaagatccggtaggtgccaccgtaaagatcgttggtggcaattacctcgtcgccggggctcaggagcttcatcactgcatctgtagctgccaggccgctgccgaaagaaatgccatgtgtgccgttttcaatggctgccagtgcgttctgaagggcgtcgcgggtaggattctgcgtccgggcgtattcgtagcccttatgcactccgggagcactttgtacgtaggtagatgtttgaaaaattggcgtcataatggcgccggtagacggatcgggagctacacctgcgtgtatgagtttagtacccagcttcatgtctttaatagtttagatgatcaatttctgatggtctccaaatatactccagtttttgcgattggaaattcgccaattgataaagggcaaacttgtccgttttagcttatattaaaatatgatggcataaattccaacggttacgaacatttttatatcgttcaccaattagccactaacggatatgaataaacctgctacattcgttttaggtttttcataggatatggttaaaattcttaaggcggtattcttaccgctttttctttttacaacaacaactgtgtaaacagttttcgtataaacgttaccggggcgggataaaaagcagcagaccactgctttttatcccgccccggcggcattttataatgtacggattacttcttttttgcggtggtgccgccttcggtccatttaatgggaagacttacgcttactttatcccaggcgataatcaggttggcgccgggatcacctttctcaaataccatggtgaaggcttctactgctgtatccagtgataataccgggagggcagttcttaccacatcttttttctgatcgtatttaaaagcaccccatacatcggtgtctttattcaggatgatggtccatgttttttctgttggaatggcatacagggtataacgtcctttcgggatgcttttaccagcgatgatcacgggccggaagaattctatttcagtggcttcgttagcgcccaggcgccatattttgccatattcttccaggttcccgaagatatcccttcctttggtttggggacggctgtaaattactctggctaccagtgttccgggttcgccttttacttttacaacatagggatacatgacagggtaataggccatgtccatcgggctagcatcgagtggaggcagttttttatcctgcgcagcggcgcttaagctgattaggcccgctacaaaggcaaaaaggagaacttttttcatcatcctggaaagctttatttcttttatagattattggcggcaaacctacctttttttaaggaatctgaaaagcgtagttctctcatttaacaagctgttagcggttttcaatttgcaacagtccttccacataagtttgcagctcagggaagaaatcctggtaacattctttcagggcggcataatgttccataaacacggcaaatacaatattgccatcagtttccaggtatttggcccgccgggctacacccctgatagagctggaaattccttctgtagtatgatagttgtagagccagttgtaggcctgcatatattcaaacatctgcaaaaaagctggtggcagctgttctgtgcgctggttaatctggttataaacgtaacgggcaaacgaatacagggaatcgtttgtgaagcgttccggatcagcagccaggaaatgatcatataccaggtcagtgaatacgccgctatataatccgcaggagggacggaaaaactgtttagccctggccgttaccgggtgttggtcagtaaagttgtcgatggcccggtgtatccggatgccctgctggatacctgctgtgtaaactgccatgtttttcctgccctttacaaaatctgcaataaggttaccggtgatcagctccggttcacgaaaagataagtaagcatgggctaggtggttcatcatctcaagatacgtatttatacagcaattggcagggatcggtccatgtcttaaaaccttatccattttaacaatttcttaactctcagccaagcaacattggcaggttggcaccaacaaacaggctatggctggtctgaatagccgtatgtccgccaccggtcaggcggacgttcattaacggatagtccaactaatcatgtgcccccaccagtaaagtatgccttgaccactgggcacttcccggcgtagctttgacttatcgaaacaaaaaaaattacaatcaccataaattttttccgccatgaaaaaacttatcttattagtcagtgcagcgctcctgttgagtgccaatgtgcttctcgcaagcccttatgaaactactgttaacaaaaggatcaacagtacgttcaatgaatctttcaacggtgctaccgatgtaaaatggtacacggatgataatagaacgtttaccgccaagtttaccatgagtaatacaaaggtgactgccttctttaaagaagatggcaccctgctggctacctcccggtacctgcaggcagaacagctgccactgaaagtactcagtaaactgaataaaaaatattccaataccagcgtttattgtgtagtggaatatgcttcttcagacaacgtggtatactttgtaacactggagggtactgatacctggactgttgtcaaaaccgatgcggatgccaatatgaaagtatacagccgtttgaaaaaagcttagttttagtagtgttaaaaatacagggcccggggcatttgctctgggcccttctgttttatccccacgccccttgcccctgcaaaaattatcttaactttgccacctgttaaggctttattagccagactgttaatgtataaatgattaaatgacatgaataagggacctgtttctcaatttatccagcaccattaccgccactttaatgcagctgcattggtggatgctgccaaaggatatgaaacacatttactggaaggtggtaaaatgatggtgacgttggccggtgcgatgagtacggctgaactgggcatttctttcgcggaaatgatccgtcagggtaaagtggatatcatttcctgcacaggcgctaacctggaagaggatatcatgaacctggtagcacatacacactataagagagtacctaactaccgcgatctgagcccgcaggaagaatgggatctgctggagcagggctttaaccgcgttacagatacctgtatcccggaagaagaagcattccgccgtattcagaagcatatctacaaaatatggaaagatgctgaagaggccggtgagcgctatttcccgcacgaattcatgtacaagctcctgctgagtggcgtgatgaaagagcattacgaaattgatccaaagaacagctggatgattgcagctgccgaaagaaatattcctatcatcgttccgggatgggaagacagtaccatgggtaatatctttgcttcctactgcatcaagggcgacctgaaaacgtcaaccatgaaaagcggtattgagtatatgatctacctgtctgagtggtaccgtaacaactctgctggtaaaggcgttggcttcttccagattggcggcggtattgccggcgacttcccgatctgcgtggtgccgatgatgtaccaggatctcgaatggacagatgttcctttctggggttatttctgccagatatccgactccaccacttcttatggttcctactccggtgcggtgcctaatgagaaaattacctggggtaaactggatatccatacacctaagtttatcgtagaatcagatgctactattgtggcgccgctgatgtttgcgtatatcctgggatggtaattgacaaataggatattattatatagaagagcagcggggatattacctccgctgctttttttataagatgaataactcgccggctattccgtctgcgaacaggcgtccggccttcgttaaccgcaaggtttcccctacccgctctatgcggcccatcttaatatacggttcactgtgcgccagtaaatgaatggtatgatcggcgccgaacttctctgccacccattccaggttgcatccggcggaagtccggagggaggtcatgatgtattcgttgaattgcatggccgtagtgagcgactctatttcaaaaggcacggtacctgccgtgatgctttttatgtattgggcattattggcgatgttccattgccgcgaagcgccgttgaacgagtgggctgacggccccaggccaagatagggcttaccctgccagtagctgctgttatgccgggaatgccatcctggtaaggcgaagttggagatttcgtaatgttcatagccggcggctcccagccattccatcagcatttcaaaatgctgcgctgctttgtccggatcggtagcagccatctgctttttctttataaactgatccagcgccgttcccggttctacggtgagcgcatagcacgataaatgcggaacgcccagtgcaatggcctgtttcacattttgttcccagccttcattggtaagcgtggggcctccgtaaataagatcgatggtgatattctgaaacccgagatcctgcgcctgtttgatacaatccagtgcctgccggctgttgtgcgcccggttcatccaggtaaggtcttcttcgtgaaacgactgcacgcctatgctgagccggttgatgccagcggcttgcaactgggcgagtttttcagcggtgaggtcgtcggggttggcttccagggtaatttccgcatcctccgctactgcaaaggtggcgcgcaggtgcgacagcagcgcagcgagttcctcttctttcagcaggctgggtgtgccgccgccaaagtagatggtgtgtaccgggtgctgcgcgagataatccttttgcagcgtgatttcctgcaggatgctattgaccattgcctcctgctgcgacagcgaggtggaaaaatgaaaattgcagtagtaacaggcctgcttgcaaaaaggaatatgtaaataaattccggccatgacgttttatgattgtttacccttattggccgcaaagataccttcttccctttactacactccggtcaactatggactattttaatatctttgcgatatcataattacgtttcctttttgttatgtgggcaggacgttgttaattgccgttgattcctttgtgtgggaaacgggttattgaaaaaccgatttaaagtcattgcaaaatattttcctggtgcgaaactggttactgctgttattcattttaggttatttgcccgttttggcacaaacaacagattccgctgcggtgccgccggcagtaaagaaaaagccggtgataacccgtacagctgcagattcatcgcgcgcgaaggcgcgtaccgctcctgttaaaagagacagcaccagggctgctttaccggcagttgcacgcataaagaaagataccacaaagctcctgaaggatactgcccacctgaaaacagatagcctggcattggcggcagtacctaaggtgaagccggtatcagcatatgatctttacctgaagaagatatcgcaggaaaacgtcttcctgaaacccggcaaaccacggttcgtggataccaacccgataaggccttaccgtaatatggactggcttatttacctgatggcgggagtattgttgatcctgagcgtgatacgcctggcttaccggaaatatttctcggatctgttccgggcattcctgaatcctacgctgagccagcggcagctaaaggaccagttatcgcaatcgccttttcccaatatgttgctgaatattttcttcgctattgtacttgggctgtatttttacctggtattgtaccgtcagcaggtatttccgcaggcggagccctggttgctgataccgggtttaatagtgatggtggctgtggtgtatggatttaagtatgtgatgctgcgtttttgcggctggctgtttgggaattctgagctggcggatgcttatattttcattctttacctgatcaacaagattttgggggtgttgctggtgccgtttttggtgataattgccttctgtacacccgaaatagcgcgcactttcctatatatatccttgttttttattgtattactcattatctacaggtatattagatcttattcattggttaggcagtacctatctttcagtaaattgcatttttttctttacctttgcgcattcgaagtagcgcctgttttaatattaaccaaggtgctgcagaatatctggttaactggtaatccctgattatcgcctattgttaacacaagagcaaaaaacgtatgataaaaggcgggccaaaaaaagatttgcaaggaaaacaaattcagtcaatcctaatttctcaacctaagcctgaaacagaaaagtcaccctactttgatctggccaggaaattcaatataaaattggatttttatccgttcataagggtggaaggtttgccagcgaaggagttcagaaaacagaaaatcgacattctcagctttacggcggtaatttttaccagtcgtaactcggtagaccactttttccggatttgtgaagaaatgaagattaaggtgtcacaggactgcaaatacttttgtattacagaagccgtggcgttgtatctgcagaaattcattctttaccggaaacggaaggtattttacggagcagacggttctaccaaaggagtactggaggtgatgaacaaacaccgggataatgagaaattccttttccccagctctgatagccagaagaaagatattgaagaatggctgaaagcaaacaagtgcgactatgctaccgctacgctttataaaactgtttctacagatgtaaaggaagtattggctgctactgcttatgacatgatcgtgtttttcagtccttccggcgtgaagtcactgtttgagaacatgcctgaatttgtgcagaacgggacgcacatcggcgccttcggtcctactacttccgctgcggtggaagaagcggggttaagactggatgtaaaagcaccgcttccgcaggcgccttctatggcagctgcgctggagcagtacctgactacattaataaagaagtaagcaatttttctgcgataaaattgagcaggggtggcgtagtgccatccctgcttttttttgctgcgatggcaatgcaggggccggtttcaaaatatttctttgtaatcctgaaaaaataaatttctttgtagaagaaataagaagatcaatcattattatcgcgtagggggaatccatgaataagcttatcagtgaaaccagtccatatctgctgcagcatgcgcacaatcctgtaaactggtatccgtggggggaagaagccctgcaacgcgcgttgcaggaggataaacctatattggtaagtatcgggtatgccgcttgtcattggtgccatgtaatggagcgggaaagctttgagcaggaagctacagctgccatcatgaacgaacattttattaatattaagatagaccgggaggaaaggcccgatctggatcatatttatatggatgccgtacaggctatgaccggcgctggtggctggccgctgaatgtttttcttacaccggataaaaagcctttttatggtggcacttatttcccgccggtgaaagcatacagccgtccttcctggacagatgtgctgttatcccttgctgatgcatttcagaataaacgggaggagattgaaacacaggcagataacctggtacagcatatacagcaatcagcccagtttgggcagcagcctgggttgcatcttgatattcccttcgaagaattatttaccaaagcgcaatgtgacaccatttgtgaaaatatactgaagcaggccgatacccggtggggcggttttggccgggcgccaaagttcccgcaaacctttaccattgcttacctgctgaggtatcatcatgcgtatcagcatccggaagcgctgcaacaggcgttgctgtcgctggataaaatgctgcagggaggcctctatgatcagctgggaggcgggtttgcccgctattccaccgatgaaaagtggctggcgccgcattttgaaaagatgttgtatgataatgcgctgctcctggatgtgttgtgcgatgcttatcagctgacacataacgaagtatacgctcaaacggtcagggatacgatggactttatcacccgtgaaatgaccgctcccggagggggcttctatgctgccttggacgctgattctgagggtgtggaaggaaagttttatacctggagcaaggcggagattcatcatatcctgggggaacaggcaaagcctttctgcgagtattatgatgtaagggatcatggcaactgggaggaacagaatattttatgggtgcaacagccgctgctggatttcgcggcagaaaaaggatatgatgcggatattttcggcgccatgttaaaaggctgccgggaaaagctgctggcggtgagggctaaccgtatccggccgggattggacgataagatcctgctgggatggaatgccatgatggtacatgcctgctgtaaagcttatgcggcactgggcgtaccagcttacagggagatggctatccgcaatatggatttctgtttatcgaatttccgccaggaggctgccggtagtgcattttaccatacgtggaaacaggaccaggcgaagtatccggcgttcctggacgattatgcgtgtttggtccgggcgctgatagcgttgcaggaagttaccggcgacacgcggtatttatatgaggcgcgtgatattacggcctttgtgatcgctcatttcagtgatgaagccgggcagttcttttactataccattgagggtcagaatgatgtgattgtgcggaagaaggaaatctacgatggggcagtgcccagtggaaatgcggtgatgatgcagaacctttggtacctttccgttgtttttgatgagaaggaatgggcaaaccgttgtgtgggagccgtttccagcctgtcgcaaacgatagtgagataccctacctcctttggcgtgtgggcgagccagttattacagctggtaaaaggtacccccgaattggccattgtcggaaaaaatttcagggaaagaatggatgaagcgggaaaatggtttatcccgtacaggattcttgtcggcgcagaaaaaaatattccggcgattcccctgctgaccgggcgggagcaggaaaatgacactttagtttatttatgtaaagattatcattgcattaagcccgtacattatatagaagaaattattaatttaatataataattatgtaacttgcctctcgtaagggaggctattgattcaataaatgttattacgtttatataataaaatgttaaaaggtgcgtttaaactagttacagaacggatataaggcgaattgaaaaagttggataaaaagtcactacggattaaaattaattattacatttgctatctttcatataaacaaagcgggtgaaaaaatgagaattgtgttcccttgtatacaggcaaatcacaccaggctggttaatagaaaaaacatattctgatgaaagctacccttatgaagcttaactatgtaaaaggtctgttggcagttttgctggtttccctgctggccagctgtggcggtagtaaaacccctaaaaatgcgcaagggcaattgatcggcgtaagtccgagaccgaagtactctccccctgtaccgtacgggatggtatacgtaccagccggaacttttcacatgggtcccagtgatgaggacgtaaactatgcatacacggcgcgtaacaagtcgatttctatttccggcttctatatggacgctacggaaattacgaataacgagtatcgccagtttgtgaattgggtacaggactctattgcacacattttgctgggtcatgtaaaatctgatgatggtcatgatattattgactggaagcagaagattgtctataaggacaaggctaccatggaaaaactggatgcgatggtgtataccgaagcagaccggttatacggccgcaaggatattgatgtaggtaaactgatttaccaccaggaaacctttaactgggataaagcgaagctgagagaaaatttcggtaagccgcgttctactttcattgtaaagaaagacgtgcccatttatccggatacactgtgctggatcagggatttctcatacgcctataacgagccgatgacacgtatgtacttctggcacccggcgtttgataactatcctgtagtaggtgtaaactggcaccaggcaactgccttctgcgaatggagaagtaaattctgggaagactaccgggccagcaagaagctgtttacggaagataaattccagttaccttctgaagcgcagtgggaatatgccgcccgtggtggaagagagcaaacgccttatccttggggtggttactacatccgtaacaagaaaggatgtttgctggctaacttcaagcccggccgtggtaattatccggaagatggtggtttttacactgttcgtgcagatgcttactggcctaatgattatggtttatataacatgtccggcaacgttgcggaatggacagcagatatcttttacgaaaatgcctattctttcacatcagatatgaacccatatctgagaatggatgtaccggatgatgcaccattaaagatgaagcgtaaagcaatcagaggtggttcatggaaagacgtaggatatttccttcaaaccggaaccagaacatatgagtatcaggacagttcgaaatcttatgttggtttcagatgtaccattgccctgagcagacgagtgaagcacagataggataatcaataaataatagcctgtatttattaacaccaaagaaacctttagtatgtacactattatgagtaaatcagtgagaattaactattccatacagactttaactaacattttaaccagtaaattttaacctatggctatgaatcctaacaaagctaaatggctgaactttttcgtatgtattgcggcttccgtggtaatcgtgggagcattgttcaaattacagcactggcgcggagctgacatcgctttgatcctgggtctgagcgtagaagcgctgatctttttcgtttacgcttttgtacctgattccggcgcacacacggaaggccaggtggtagcagtagcaggaagtccagctgtagccggtttggacaaaatgctccaggaagcagacattacacctgccaacctgcagcgcttaagcgaaaacttccagaaactgggtactaccgttgataaaatgagagatatcagcgatgtagttgcagccaccggagattacacacagaaaacaagagaagctgccagcgctatcggtaatgtagcaaatgcatatactacagccgctgctgccgtatcttctttcaacagtgcatcagaatctactaaagatttccatgtacagatgcagggtatgactaaaaatctggcttccctcaatgctatctacgaactggaactccaggacaccaacaaccacctgaaagcaatgaattcattctacagcaacctgcagaatgcttccagtgcaatgagtggcagcattgaagatgccaagaaaacacaggaacaaatttccctgctcgctaaaaacctcagcaacctgaactcaatttatggtaatatgctgagcgctatgcacggaggaagataaggtaacgctaatagtttctgaattaacacatatcaattaaatctgaaaacaaactatggcactacctaaagatcctaggcagaagatgatcaacatcatgtacctggtcttgacggccatgctggcgttgaacgtctctgctgaaatattgaacgcttttagtatcgtaaataattcaatcaatacttcaaataaatccttagctgacaagaatgacttcatctacaaacaatttgatgcacagatgaaggataatgcggaaaaaacagcacctctcagagcaaaagcccagcaggtgaaacaaatatccgccagcatgtatgattacgtagagtccttaaagaaaaccatcatcacagaaagtggtggcctggacgaacatggtgaaattaaggataaagccggactggacgctcctaccagggtaatggagaatatgaagaaaggtcctgaactggaggctaaattgaaagatttacgtaaccaattactctctttcgttgatcctaaaaagaaagatcaattcacaagaactttaccactgaaaattgaagtaggtaaatcaaatgatgaacatggcggcggtccgaaatcatggactacctaccacttcaacatggttcctactatcgctgcagtaaccatcctgggtaaattccagaatgatatcaaaaactctgagtctgccattatcgatgacctgttccgtcagattgatgcgaacacattcaaattcgataaagtaagaccatttatctccctgaattccaaaaacctgatggaaggacaaaccttaactgccaacatcgcagtaggtgcttacagcactacggttaatccgactattgttgtaaatggttctaccattgaagcacatgaaggtttaggagtatatactgttcctgtttccggcattggtgaaaaaacattaaccgggtctattaccttacctagcccaactggtggcgctcctgaatcctattcctttaccgaaacttataatgtaggtgcttctgctacctccatctccgcagacaaaatgaacgtgctgtatatcggcctccagaatcctatttcgatttctgctgccggcgtacctgccgaacaggtgtctgcttctatatcaggtggtaatatgaccaaacgcggttccggcgaataccttgtaactgttagccagccaggcaaagcagtgattaatgtagtcgctaacatcgatggaaaaaccaaatcactcggccagaaagaattccgtgtgaaacgtgttccggatccggtgttgaaagtgggagttaataaaggcggcagcatgaaagcagctgactttaaagtacagggtggcttacgtgccgacctcgaagattttgaatttgaaggcgtgaaatatgaagtaatcggttaccgcgtaggtatctctgcaaaaggcaaagaataccaggaaggcgatgctacttctgcttatttccccggaaatgtagccgcatccatccgttctctgcgcccaggcgatgaagttttctttgaaaacgtaaaagtgaaaggcccggataatgtggttcgttccatgccgagtactatatttaaattaaactaacggtccattaattactgaattatgcgagcagtaatatttaacagaattggttggtgcactcttttgctggtgatgctggcaacagctgctgatgcgcaacgccgtggcggtacaacccgccgcagaactgctactacagcaacacctgcaccggatagcgtagtaaacccggcaaccgggaatgcggtagcgcctcctcctccatcttctgctcctcctgcttctctgcgtacggatggtatatcagccccgctggtagatactccgcgcaaatcactgcgagtggatggtgtggtggaaagaaaccttgccagggaacgtacacccatcgcctatgactacatccgcgaggatgacaggttctgggaaaaacgtgtatggcaggtaatcgatatcagggaaaagatcaatctccccttccaatacaacgtggaagatgagtctggtaccaatcagctgttcatcaatattttgctcgacgctatcaagaataaagagatagaagccttcaacgctgttgatgatcgcttcactactgtaatgccctactccgaaatacaaactaaactcgcaggcgaagaaagaaccgtacgcagtatagatccggtaaccggcgaagaaaaaatggtgactacccgcgatgacttcgatgcacgtaccattaaacagtacaaaataaaagaggtttgggtattcgacaaagaagcttccgccctcaaagttcgtatactgggtatagctcctatggtatcccgtataaatgaagatggcagcatacgcgcatccatccctttattctgggtgtattatccggattgccgcgctatcctggccaagcacgatgtgtataaccagaataacgatgcatccactatcagctgggaagacctttttgaaatgcgcttctttggcagctacatagtaaaggaaaacaatacctacaaccgcgagatcaaagactatattaaagatggtaccatgcgcctcctggaaggacaaggtattcacgaccgcatctttaataaagagcaggacctctggcagtattaatcaaataatgatcaccgatcaatacggaaaggcaatcagtttatgctgattgcctttctttttttatctttccgtatgtcccttcagcagctacataaaaccgttttccagatcatgcctctcccggatcccgtatgggaggcactggcagcctgctggcatccggtgcagtttaaacgcagggaagtaatgaccgccgccggggaaatagaaaagtatctctacttcgtaacagccggcgtacagcgtgtttttgccctggaaggcgaaaaggaatctacgatcgtattcacttacaccggctccttctctggcgtattggattctttccagcttcagcaaccctcaccctggtacctggaaacccttacacacagtgaattcctgcggatgacgtacgccgattttaaccggcttgccctgcaatatcccgtcattgaaagatgggccaggctgggaaccgctgccgcactggccggggtattggaaagacataaagaattgctgtctttcaccgcagaacaaaaattcaggcaactgctaacccgcagcccgcaggtattacagctgatcccacataaatatctggcctcctatctcggcatcgatcccgctactttcagcaaattactaagtactgtaaagctataaaatgttgatctgcacaaagattttttacaagcaacccacctaattttgtgttaaatcaaaccgaatatgaaccgcgttaacagtgatgagctcctgcaggatttacgaagaaaaaatgcagccatgcaataccaggcagaaagccgtttcggcgggcagcccgatgctgttttacaacatgcacccggtcccggccaatggagtgccgcgcaatgcctggagcacctgaatacttacggccggttttatttgccggcgttggaccaggccattacccgtggggaacaacgtaacagccggcccgctcccttcttccgcagcagctggatcggcgcatggtttacccgcctcatggaacctgccgcagatggcagcttgcgttcccgtatgaaatcccctaaaggacacctgccatccgttcagccggatgtggaagcggtgttgcaggagtttattgatcagcaggaacagatgagagatttattgttgcgcgcagaaaaagtaaatattcaacagctgaaagtaactacttccctgtcgcggtttataaaattatctgccggagatacatttggttttttaacggcgcacattcgccggcatatgttgcaggcggaacgtgctatcggcaccaggcagcaggcaaaaaaggccgtatagccgttaatgttatgcgccttctttatggaagtgttcccagatcagttttgctttggcggcgcccacttcttttacaaggtcctcctgcgtgagcaattttattttggctaccgaacggaatgtttttaatagttgggtagccgtattttcgccgatgcctttaatgctttccagctcatttttaaaggtgcctttgcttcttttctggcggtggaaagtaataccaaagcggtgtacctcatcacgcacccggcggataagtttcaggctttcgctgttatagggtaatttgatactttcggaatctcccgggaaaaatatttcttcttcattttttgcaaggcccactactgtcatgctacctatgaggttcagctcccggatgctttccatagcagagcccagctggcctttaccaccatcgatgattaccagttgaggaagtggttgctgctctgccagcaggcggttataccgcctgaaaacaatttctttcatggaagcaaagtcattgatgccttccaccgttttaatgttgaaatgccggtaatcttttttggaagcaacgccgtctttaaacactacgcaggcggctacggggtaactgccctggaagttggagttatcaaagcattcgatgtgttctggtagcaccggcaattcgaggtcggcctgcaactggtacagcacctgtttccgttccatgtccgacttgccttccaggtgcagaatcttcttccggtataattcttctttaaaataattcacattcttttccgacaattccagcagcttctttttatcgccgcctttaggaacggtaacggtaacactgctttccgggtatactaacgggaatggcactacgatttccgagttgatgcttttaaatacttcccggagataggcaatggcgtaggccagtacttcttcgtcgctttcttccagttgtttttccagcgttacggttttggtatcagcaatagtgccgttgagaatgcgcaggtagtttacataagcgtgatttccttcactgataattgaaaacacatccacattacccatgcgggtatttacgatagtggatttagcggaatagtcttccaggcttgctattttttttcgcatgatttccgctttctcaaactccatcttcgacacatgctccagcatttgttccttgaacaggtttactaccggggtaagattgccttttaatacgttctttacctgctgtaatccttcgcggtagtcttcctgtgtttgcagcccttcacagggccccttgcagtttcccaggtgatattcgagacatactttgaattttcctttacggatattctcttccgataagttgaggttacaggtgcggagaggaatattgtatttgattacatccagtatttcccgtacccgaccaaccgaagtgaatggccccaggtagtcggatccgtctttaataacgttgcgggtgaaaaatacccgtggaaaggactcatgtttgataacaatataagggtaggttttatcatctttcagattgatattatacctgggcttgaattgtttgatgagtgaattttccaggaggaaagcatcctgttcagagtcgacgattgtaaactcaatatgatggatgtgttcaaccagtttgcgggttttatagttgtcgtgattttttacaaaataggaacttactcttttgcgcaaacttttggctttccctacataaagaagggtgccggcttcatcgtagtatttatagataccggcatctcccggtatggtatgtgatatttgctgaaactccgctgctgtcatgtttacatccctgtttttggtgcgatcgttacatttacttcaagttcttttggcgacaggaaagcaattttctgataggtagtcatccgaacctgcctgttttgctggtagtgcagatcctgccggaattcatacaccatgttactggtataggagtggatatttacctgttgtatattgccatgtttatccagttccagggttatttcggaaggattggtttgttttcctttggatttgtagatcagcgatcttcttcctgaaaacggatcatacaaaccggaggtatcgtattcgtcccgaagggagggtttattcagatctgcatctgtgaagggctttaacaggtcgtgtaccgtggcgctgtcgctgccggggatgctcacagtgtctgttttgccgttgagcgttacagacttatgtagtataaagccaccagtgcggatatgagcatcctcctggctgaaatattccggcagttttatgaacttatcgggcgtattattttttgatggtttatttgccaggttacaggccattaagccaatcatggtaaacaaagctgttgcttgcctgtattttttcatgctgcaaaattaatacttaaatacgggtcataaaaaatgcgccgtaaaaacggcgcatcgatgcatgagcaaatctgtcgagagcactaaaaatatgtaaatcagcgtgttgggctgatatttttcgtgggtaacgcttgttaaacggaggtgataaactaaatgttacaggggtgaataaataaatcgccttcggcgatgcggattttgtcttggctcaggattacgctgattatactgattagctggatttttacttttggatttttgtttgattttgagatttaataataattaagggagataaaagcgaatatatccgcttctatctcccttaatcctttataaaatccaaaagtaaaaatccagctaatcagtataatcagcgtaatcctgagccaagacaaaatccgccttataccagcaaattgccggtcatttccttcggaatttccaggcccatgaaatgcaggatggtaggggcaatgtcgcccagtttgccgtcttttaccgggcctctgaaatctttattgataataaagaaagggaccaggttcagtgagtgggcggtattgggcgagccgtcggcgttgatcataaagtcggcgttgccatgatccgcggtcaggaaaacggtgtaatcgcttgcgagcgcagctgttaccacacgttccacgcagtggtctactgtttcaacggctttaattacggcttcaaatacgccggtatggcctaccatgtccgcgttggcgaaattgagcactacgaagtcagcggttttagcctgcagttccggaacaatgaggtctgccagttcattggcgctcatttcgggtttcaggtcgtaggtggcaacttttggagatgccgccatcagcctgcgttctccttcaaattctttttcccgtccgccggagaagaagaaggatacgtgcggatatttttcggtttcagctatacggatctgtgtgcagtggtcttttgccagtacttcacccagggtcatgttcagattatcgttttcgaagatgacatgtacatttttataggtacggtcgtaatctgtcatggtggtgtagtagatatccagtggtttcataccgaaatccgggaaggcttcctgggtaagcacctgcgaaatttcgcggcagcggtctgtccggaagttgaagcaaagcacggcgtcgccgtcctggatagtagctatggctttatgctgatcatcggttacgatgataggcttaatgaattcgtctgtaacaccttctgcataggatgctttcacggcggtaaggagatcctgggttggcgtgccggcgccatttacgagggcatcgtaggccagcttcaccctttcccagcgcttatcgcggtccattgcataatagcgtccggtaacggtggcgattttgccggtagttttttccaggtgggccgacaggtcttcgaggaagcccaatccgcttttaggatcggtgtcgcgtccgtcggtgaatgcgtggatatatactttttcaagcccgtgcgcctgggcgatggtggtgagcgcttttaagtgttcaatatgagagtgaacgccaccgtcgcttaccaaaccaatcaggtggagggctttatcattatttttagcatgtgccagggtgtcgagcaggatctggttttgggccatttcgccatcacggatagctacgttgatcctctgcagttcctggtatacgattctaccggcgccgatattcaggtgacctacttcagagttgcccatttgcccgtcgggaagaccaaccgcttccccgcaggttacaaggtggctatgcgggtattgcttgtataaactgcttacaaaaggggtttttgcgtgtgcaatggcatcggctgtaggaactttaccttcgccccatccgtccataattacgagaatggctcttttcttttccatatcctatctggttatagtttaatataaattcactcgagagggtgaaagtacttataaagggtttaaatattttacaaaaataaagcttccatgaaaaataagcgctgctggcctcttccaatagatttgttattctaattattcaaaatgaaacacatattatcttactgttattgcttacggcttaatagctaccacgataatgtgattttgttgatttgcagggtgtttggcatagttttcgcttttaatttgagttggagaaaaacacatttttaataaaaaaactgacaatgaagaagctattgatggtgctggggattatgttgttggggggtgcttttacaacattaaaattatcagccaggtcaattgaaatcactgttgccggcccgttcgatgatgtggtggcagcacttaagaaaggagatgtaagcggattagccagttacctcgacaataacgtagagatcaatatatccggaaaatcaaattcttacagtaaggcacaggccgaaataattttgaaagatttcttttcaaaaaaccaggttaagtcatttgaactggtgcatcagggcggggataattcccgttttggtatcgggaatatgaccaccggtggcggtaactacagggtttcttttttcctgcagaagaagggtgggacaatggtgttgaacgaacttagatttgagagtaaataaagatgctaacataaattagttgaaaaaccacggtgccccgcaatttattgcggggcactttttatttttgacctatctttcgcgctcagaagcaaagcgccaatctttgcgtgaacaccagataatacaatcaattatgttagatgaagcagcgctgaatgcgtttatcagaagtgcactggcagaagatataggaagcggagaccactccacgatggcttgcattccccccaccgccaaagggaaagcggtgttgaagattaaggaagacggtatcctggccggaatggaagtggcagaagccatttttaaatggctggatatgtttacggtttttacgcctcataaaaaagatggcgactccatgaaggccggcgaaacggcctttgaagtggaagctgccgtacataccctgctgatgggtgaaaggctggtgctgaactgcatgcagcgcatgagtggcatcgctacattaacgcaccggtacgtggaaaaactaaaagggtaccatacccgtgtgctcgatacccgcaaaactactcccaacttcaggatgctggaaaaagaagcggttcgcattggtggcggcgttaaccacaggatgggattgtatgatatggtgatgctgaaagataatcacatcgatttttccggtggcattactgccgccgttaccaataccgttgcatatctgaaagaacgtaatcttccgctcgaaattgaagtggaaacacgcaacctccgggatgtggaagaagtgctggctataggccaggtaaacaggatcatgctggacaactttacccctgcagacattgttaaagcacttgcgctgattaacgggcgtttcgaaacagaagcctccggaggcattacaatagatacccttgaagaatacgctaaaacgggagtagactttatctctgtgggcgcaattatacatcacgcggtgagcctggacctgagcctgaaggccattatattataaaacagtttttttgaagaagattctatttatcatcaaccgcaaagcgggcactgaccgtgaaaaacgattggaaagcgctatcagccggcacttcccttccgatcagtatgaagtgagcactgcttacctggcataccttggccatggggcagacctggccagggaggctgttagtaatggtgtaaataccgtggtggccgtaggcggcgatggctctatcaatgaaatagcacagggccttataggaagcaataccgcaatggccatcctgccgttaggcagtggtaacggcctggcgcgcgcgctgaaaattccgctggatgtaaataaggcgttaagtcttgttgttgccaataaacaacgcgccatcgatgtgggttatgcgaatgaacacctgtttctcagcaatgccggcgtaggttttgatgcgcttattgcagaacagttccggcataataccaaacgtggtttatccggctatgcaaaactggtattgaaaagttttaacagttatgaaccggcagaatacaggatcgatatagatggcgaagtgttgcaaacaaaagcattccttttaactgtagccaatggcaatcagtttggctatgaatttaaactggctcccaaagccagtgtttttgatggacaactcgatctttgcgtaatgccgccggtaggcattctgagcctgttaccggtaagcgttttctccctgatgggtaacattgataaaacaaggtacctgaaacattacaccggcaaagatatcaccatcagcagcagtgcattgcagtatttgcaggtagacggtgatgcagtgcccctcacggaaaacggggtggtacgcatccgtattcaaacagcggccatcaatatagtggtaaacgaataacctttaaatattttagagagatgtcgaaaaagaaaaatacaccaggcaatggaatcgtgtattccaccgatccaaacttctcattggagccggagcaagaggaagcagcagtaacacttgcacctgcagaacaaatcctgagagtaacattggataaaaaacaacgtgccggtaaagtagttaccctcatcaccggttttgttggtaaagaggaagatattgagaagctcggtaaagaacttaaaacgaaatgcggcaccggtggcagcgtgaaagacggtgaaatcctgattcagggcgactacaaggagaaagttgtgaaatggttgctggattggggatataagcgtactaagtaatgcagcgcgaattttgtctttctcaggattacgctgattttactgatttttacttttggatttttttggatttttagatttaataatagtaattaagggagataaaagcgaaatatgtactgccccctaaaagttagacacttttagggggcatttttatggataaacgcagaaaatacagttttgagcaaaaattagccattgtgatggcagttgagaatgattatcaatccgttagt

SEQ ID NO: 3 - DNA, 820459 bp, Chitinophaga pinensis
  source 1..820459: mol_type = genomic DNA
gttttttcaggctggtgatcctcacggtatcataagtagcagcagcacactgtgagtttgaaatctgccagaagaggagcactgagctgtcggccggaacggtaacagtagtagtcgcgctgttgacgttagcaaacttcacagaagcggtagccggtgtgaatgtccaggtgccttttgcgcccagctcagtaggagcggtggcgttgagcgtaaatactgttttgtcacaggcaatctggttagaaccggcatcgcgaacgattggttttttcaggctggtgattcttactgtatcataagtagaagcagcacactgtgagtttgaaatctgccagaagaggagcactgagctgtcagccggaacggtaacagtagtagtcgcgctgttgacatttgcaaacttcacagaagcggtagccggagtgaatgtccaggtgccttttgcgcccagctcagtaggagcggtagcgttaagggtaaacaccgttttatcacaggcaatctggttggaaccggcatcgcgaacgattggttttttcaggctggtgatcctcacggtatcataggtagcagcagcacactgtgagtttgaaatctgccagaacaggagcacggagctgtcagccggaacggtaacagtagtaatcgcgctgttgatgtttgcaaacttcacagaagcagtcgctggtgtgaatgtccaggtgccttttgcgcccagctctgtaggagcggtagcgttaagggtaaacaccgttttatcacaggcaatctggttagaaccggcatcgcgaacgattggttttttcaggctggtgatccttacggtatcgtaagtagcagcagcacactcagaatttgaaatctgccagaagaggagtactgagctgtcggccggaacggtcaccgtagtagtcgcgctgttgatgtttgcaaactttacggaagcagtcgccggtgtgaatgtccaggtgccttttgcgccgagctcagtaggagcggtagcgttgagtgtaaatactgttttatcacaggcaatctggttagaaccggcatcgcgaacgattggttttttcagactggtgattcttacggtatcataagtaggagcagcacactcagaatttgaaatctgccagaaaagaagtactgagctgtcggccggaacggtcaccgtagtagtcgcgctgttgatgtttgcaaacttcacggaagccgtcgccggagtgaatgtccaggtgcctttagcgcccagctctgtaggagtggtggcgttgagcgtaaatactgttttgtcacaggcaatctggttggaaccggcatcgcgaacgattggttttttcaggctggtaatccttacggtatcataagtagcagcagcacactcagaatttgaaatctgccagaagaggagtactgagctgtcagccggaacggtcaccgtagtagtcgcgctgttgacgtttgcaaactttacggaagctgtcgccggagtgaatgtccaggtgccttttgcgccgagctcagtaggagcggtagcgttaagggtaaacaccgttttatcacatgcaatctggttagaaccggcatcgcgaacgattggttttttcagactggtgatccttacggtatcataagtaggagcagcacactgtgagtttgaaatctgccagaagaggagcactgagctgtcggccggaacggtaacagtagtagtcgcgctgttgatgtttgcaaacttcacggaagcagtcgccggagtgaatgtccaggtgccttttgcgccgaactccgtaggagcggtagcgttgagtgtaaatactgttttatcacaggcaatctggttagtaccagcatcccgcatcaacggttttttcagactggtgatccttacggtatcaaagttagcagcagtacattctgtgtttgcaattttccagaaaagtaatacggtactatcggccggaacggtaacagttgtattggctttatttttatccgcgaaagttacagaagctgtagccggtgtaaacgaccaggtaccttgtgcgccaagctccgtaggagcggtagcattgagtgtaaacacggttttgtcacaagcaatctggttggtgccggcatcacgcatcaatggctttttcaagctggtaattcttacggtatcaaagttagcagcggcacattctgtgtttgcaattttccagaaaagtaatacagtactatcagcgggaacggtaacagttgtattagctttatttttatcagcgaaagttacagaagcagtagcaggtgtaaatgaccaggtaccttgtgcgccgagctcagtaggagcagtagcgttgagtgtaaacacagttttatcgcaggcaatctggttggtgccggcatcacgcattaatggcgttttcaaactggtgatcctaacggtatcaaagttagcagcagtacattctgtgtttgcaattttccagaagagtaatacggaactgtcagccggaacggtcaccgtagtggtggcgctgttaatgttggcaaaagttacagaagcagtagctggtgtaaatgaccatgtaccttgagcgcctagctctgtaggagcggtagcattgagtgtaaacactgttttatcgcaggcaatctggttagaacccgcatcccgcatcaacggttttttcaggctggtgatcctcaccgtatcataagtagaagcagcacactcagagtttgaaatctgccagaacaggagcactgtactatcagccggaacggtaacaatagtagtagcgctattgacattagcaaacttcacagaagcggtagctggtgtaaacgaccaggtacctttagcgcccagctccgtaggagcggaagcgttaagtgtaaatacagttttatcacatgcaatctggttagtgcccgcattttgaactgctggttttttcaggctggtgatccttacggtatcataagtagatgcagcacactcagagtttgaaatctgccagaagagtaatacagtactgtcagccggaacggtcaccgtagtagtcgcgctattgacatttgcaaacttcacagaagcggtagctggtgtaaacgaccaggtacctttagcgccaagctcagtaggagcggaagcgttaagtgtaaatacggttttatcacaggcaatctggttagtacccgcattttgaactgctggttttttcagactggtgatccttacggtatcataagtagaagcagcacactcggagtttgaaatctgccagaagagtaatacagaactgtcagccggaacagtcaccgtagtagtagcactgttgatatttgcaaacttcacagaagcggtagctggtgtaaacgaccaggtacctttagcgcccagctccgtaggagcggaagcattaagtgtgaatacggttttatcacaggcaatctggttagtacccgcattttgaactgctggttttttcaggctggtgatccttacggtatcataagtagaagcagcacactcggagtttgaaatctgccagaacaggagcactgtactatcagccggaacggtcacagtagtagtagcactgttgacatttgcaaacttcacagaagcggtagctggtgtaaacgaccaggtacctttagcgccaagctcagtaggagcggaagcgttaagtgtaaatacggttttatcgcaggcaatctggttagtacccgcattttgaaccgctggttttttgaaactggtgatccttacggtatcataagtagaagcagcacactcagagtttgaaatctgccagaacaggagcacagtactatcagccggaacggtcacagtagtagtcgcgctattgacatttgcaaacttcacagaagcggtagctggtgtaaacgaccaggtacctttagcgcccagctccgtaggagcggaagcgttaagtgtaaatacagttttatcacatgcaatctggttagtgcccgcattttgaactgctggttttttcaggctggtgatccttacagtatcataagtagaagcggcacactcggagtttgaaatctgccagaacaggagcactgtactatcagccggaacggtcaccgtagtagtggcgctgttgatgttggcaaaagttacagaagcggtagccggtgtaaatgaccaggtgccttttgcgcccagctcagtaggagcagaggcattaagtgtaaatacagttttatcacaggcaatctggttggaacccgcattttgaaccgctggttttttgaaactggtgatccttacggtatcataagtagaagcggcacactcagagtttgaaatctgccagaacaggagcacagtactatcagccggaacggtcacagtagtggtggcactgttgacatttgcaaacttcacagaagcggtagctggtgtaaacgaccaggtacctttagcgcccagctctgtaggagcggaagcattaagtgtgaatacggttttatcacaggcaatctggttagtaccagcattttgaaccgctggttttttcaggctggtgatcctcacggtatcataagtagaagcagcacactcggagtttgaaatctgccagaacaggagcacagtactatcagccggaacggtaacagtagtagtcgcgctattgacatttgcaaacttcacggaagcggtagctggtgtaaacgaccaggtacctttggcgcccagctcagtaggagcagaggcattaagtgtaaatacagttttatcacaggcaatctggttagtgcctgcattttgaaccgctggttttttgaaactggtgatccttaccgtatcataagtagaagcggcacactcagagtttgaaatctgccagaagaggagcactgaactatcagccggaacagtcaccgtagtagtagcactgttgacatttgcaaacttcacagaagcggtagctggtgtaaacgaccaggtaccttttgcgcccagctctgtaggagcagaggcattaagtgtaaatacagttttatcacaggcaatctggttagtacccgcattttgaactgctggttttttcaggctggtgattcttacggtatcataagtagaagcagcacactcagagtttgaaatctgccagaacaggagcactgtactatcagccggaacggtaacagtagtagtcgcgttattgacatttgcaaacttcacagaagcggtagctggtgtaaacgaccaggtacctttggcgcccagctcagtaggagcggaagcgttaagtgtaaacactgttttgtcgcaggcaatctggttagtacccgcatcccgcatctgcggttttttcagactcgtgattctcaccgtatcataagtaggagcggaacacttcgaatttgaaatctgccagaagaggagcactgtactatcagccggaacggtcaccgtagtagtggcgctgttgatgttggcaaaagttacagaagcggtagccggtgtaaacgaccaggtacctttagcgcccagctcagtaggagcagtggcgttgagggtaaacaccgttttatcacaggcaatctggttggtgccggcgtcacgaacagcaggtgttttataattggtaataaataccgtgtcattggtagtcaaacatggtccgttggaaatagtccataccaatgaagcggtatcaccaacaggtactttcacagtagcattccactgcgttgggttggtgatagtaacccgcgggttaggcgatgtccagaggcccgtagctcctgcaggagccggagtattacctgctaactggaagtcagtagcacggtcacattctgtttgatcggtacttgcattggcaacattaggttttgcaaatactttcaccgttacgcttgcacaggcagtgttaccacaaggaccggtactttctgcccgcacataataagtggttgtggcagttacattattaaatacaacttcagcaccattattaatagaggaagctggagttactgctacgctgcctggtaaaccaggacaagcaccggtataccatttccatttatgtgtagtaccagtagaatcagttcccagggaacctcctatcacttttaaagtaacattaccggtaacgcacagactgtcggagctggcatcaatggaagtaggagcggttgaaggcttttccacagaaacagaaaacggcaccgtaacgctacatccgtgtaacgtatcctcctgtgctgtaatgacgaagtcgtagctaccagcaggtgtgtttgccggcagtttcactttaaagataccagaggtattgttagatggccatgctttggacaccgttacaaaaccaggcatcttcctggtggcggcaacactgagtacatactgcttcaaagtccctggtaccacgttgctgtaggagaccgtaaaggaatccaccgtattacaaaccgcagctgcagcaatattcagcgtaggcttatccttaatggtaaggttaacggtagtcgagttcggaccgggacaaacaccattagagatggtccacgtcagcacaaatgttttaggccgtgcattgctgacaacagaagctatcgcattataagcggtgtcgtagttaatggtgatatctgaagaagtagtacccggcgctaatgtccatttaccggtttcaccaacgcccggcttactggcgttcagctggaaatcacgtaactcgcactgtacctggttcagacctgcaacactcggggtaagaggtttggtattaatgagtgtaacccggttggtatccgtacatgcagccagtgttttgttggtaattatccagaagagacgtaccgtatcacctgccataacacccgtcacgctggtggcggcagtagtagtattggtaataacggctcctttgtttggaccgtcaaatgaccaggtacctttctgatccgaaggaggggtgctccttttaatattaaaggtggatatattacattgtctgtagatggtatccacatccgctaccggcaccgaccgcacatttaccctgaaggtgtcaacgaccgtacaggttttgttggtcacaacaacgttgtaagctttggtaccggtgtctgaaggaacatgcgaaatagcgggcactttacctttaatagaatcaatgccatatttccacatccagttcaaactgtcggcgggcgcgcctgtaatgcctaagttcaggttaatctgtgcaccaagacaaatattcaccggtccgcctgtaatagcggtgaccggttttttatctacaactacccgggcaaatccactgtccttacattgacgcggttcattcttcacagagttccacccataatctgcaatcccgatagcccagtagtctctggtgctgtcgggaaatacggtcattttagggccaaaataaaccgggtccaccttccattcataagtactgtatcctccatcagccgtcagatccacactttgcccgatacagatcctgcccgacgaaatggttactttgggcttcggaagaatagtgatcttggtgtatttcgatggagacgcacagttgctgacgttccccgattcaaggatatttacccggtaatatttatgcactatctggttaggatctcctttcagcgcgccatccgcaaatgtgagcgtgttggtagccgcgcctgatataccgtttccatttacaacaggaaaccagtcggccggattgttttcatccccggtattactgtaaaaccattgatatattggattcttaaaataatcctggttgggatcgtaagtgccattcggcaaatgaccatcaggactatataatgctttaatagtaataggagcgccttcgcaaagtgaatccgctcttaattctgtatcaatctgaccatcgataaatgagtagatgtccgggctgcaataattaaagccgatatcatctatcgcgatatcatttccacaatcaccaagacgatcattgacaatttcaagtgttactgcagttacacctccgggtgttttaaagctgccgccgtattgttgccatgttgaatacgacaggttcatagatacgtcgtaggttttaaaccttgcgagtgtatcccacaatgcagcgttggtgctgccctttttattaatgatgaggaaggtaaccccggcatagtgataaccatccgagttacctgccgcacagttatagttaaatacgttgtagctgtttacgttcaggaaccaggcgctgaaattataagaagagcccgggcatacctgcacattgtttttagtatagaaagattttttattgatagaagagttggcgatgagcataccacccacggagtcgatagtacttccggtatgatctgttgcctttacccactcacttcttatttgagtatgccagaaaatattgtaactatcatcaatgaaattagccccgttcagaggcataggtacatagttatatccggtaaccgctgcattggagcggctgtcggtagcattctttttaaatttaccaaagtcctccaggaaatcgcttttactggtcgtattacccaaacacggttgaattgtacagtcttttacgtaaatggactttgtaaccggataggtattattccccctgaacagcaccactttcaccgtatacttagcggcatcattaaatttaatggtcagggagttcttattaatatttatgccgccggagttataagtgtccctccgctggccaactaattcgtggcctgccctggtatcggtcgtgaagagcacatcataggttccccccgtgattgtccaggtcgcggaatctgcataattactggtgttattccagaagaaggcgttcatactggcgaaacttcccttacatatcgtgtcgggaaggttcataaaggctgtgccgtttgccggcgcagtttgtgctgccacctgtttattaagcagcacaagccccagtatcaggtacaaaaaggttaatagtcgtttcataggtgcaaacagttaagtaagaaaagtatcaggattgagcagcttttgtttgctcaatccatattgtacctcaactctttacatcggttatctttcccggatggttttttccggcagagcgtggagcaagtgtaaaatggtttcataggcgtcaggtgtttatacttggtatggctaaaatatataaatgaattaagattaaaattagatgtaatatagggaaataaaaaaagtgttattaatcgtaatatgataaagcgccagataagttgaccggatgggttagcgaaaaattgattgtcaattgcttaaagggggtaaaaaaatatcagaaaagttatccacattcgcgatgggggctgaattatttagaggagactgtgctttattaaattattttcatacctttgcagaccaaatttgatgtaagatgcccaaagtaaagacacattcccgtgccaagaaaacgttcaaggttggtgggaacggacagattaagcggttcatggccttcaaaagccacttactgaccaaaaaatctacgaaaagaaaacgtagcttaagaggtagtacactggttcacgaagcaaatcttaacctggttaagagaatgctcggaatgcgctagtatctgtcaaaagaatcgaattttataacctgagaaaaaacaaagcaaatgcctcgttcagttaatgccgtagcttcaagagcccggagaaaaaggatcttaaagcaagccaaaggcttctacggtaaaagaaaaaatgtgtacaccgtagcgaagaacgttcttgaaaaaggactcacttatagctatgttggccgtaaattaaagaaaagaaactatcgccagctgtggatcgcccgtatcaacgctgctgttagagcagaagggttgacctattctgtgtttatgaacaaattagccggcaaaagcatcgacctgaacagaaaagttctggctgatctggctatgaatgaaccagaaacatttaaagcactggtagcttctgtaaagtaagacttacctgatagtaaatacccggtagctggcatcccacaggatgtcagctattttgtttttaggatatatcccgaatatcgcggaaccgctgccactcatcgacgcataaagcgccccggacgaatacatttgttcctttatcccctccagcaccgggtgtgcctggaataccggcgcctcgaaatcgtttgacaccatatctttccattcctccaccggtaactggatcatttcccgcagcgggtgaaccggcgcgccgggaacaagctgcctaaatgcccaccccgtatttatatgaatacccggatgcaccagcaaaaacgagtagccggagaggtccagtgtcatcggctccatgatttctccacgccctgtggcgtagcaaggtttattgacaataaagaatgggcagtcactccccagttgagccgcatagtcaaccagcgcagcttccggaagccccagctggtatttctggttcagcagttgcaacatgaaggcggcatctgcggaacctccacccaggccggcgccaatgggtatatttttcaataaatgaatgtttaccggctgcaactgcggaaagtccgactgcaataactgaaaagcccgtatacaaaggttatcggctgcatcaccaggcaccgggacacccgtgctctcaaattgaagttcagtatgcgtaattacctccagcgcatcattaacaggcaggggatagaagatggtttccaggttgtggaagccatcggggcgtttaccggtaacatgtaagcccaggtttattttgcagtttggaaatacaatcatagttgcacggcaaaccaacagctacagtttttacaccgccggctgcagggagtatataaaatgaaaagttatttgcttttgcggctgttgatctcatcgcggatagcgatggcccggatgtagtcttcctgttccagtacttcctgtaacaaggtagttaactcctctacattcagtgcttttaggtcatcttccacacctttctcatgctccgaaatagtaggggtaaccggcttattggtctttttaccggcagggtcgtccagcagtatccctgcgctgttgaggatattctcgaaagtataaatagggcatccgaagcgaactgcgagggccagtgcatccgatgtcctggaatctatctctatggtttcgtcgttgttagaacagataagctttgagtaaaagatgccttcctgcagattactgatgaccacctcctgtaattctacattaaaggcgttcataaagtttttcatcaggtcgtgtgttaaaggccggctgggttgcattttttccagagctactgcaatcgcctgcgcttcaaagccaccaatcacaataggcaaacggcgcaatccgtttacttctcccagtaccacggcatatgaatgagtctgcgtaatgctgtgcgataaagcaactatttccagttctatttttctcatatctgtcttgcgttgtcgctgaatagtttgtaagaccgtgaagttagaaaaatattccttatctaaaaaaaatctataatgataaatctatgatataagaattacggtacaggaattacgaatgaaaaatcaacacgatcttaaaaattgaatacttcattcgtaattcttataccgtaacctggttgcttagctctgtttcagcttgttgacggctgccgtaagcttaggcactatttcaaatgcatcacctattatgccataatctgcggctttgaaaaaaggagcttccggatctttgttaatcaccacaatgaccttgctgccattcacgccagccaggtgctgaatagccccggaaatgcccaccgcgatataaagattggggcgcacggttaaaccagtctgacccacatgttcatggtgcgggcgccagccggcgtcggctaccggacgggaacttgctgttgcagctcccagcgcctttgccaggtcttccaggatgccccagttttccggacccttcataccacggccgccgcttacaattacttctgcctccgttaaaggcacttcaccgctcaccgtttcagttttaaccaccttcactttaaaatcagcatcgctgatagccggagaaaaggcttctactgtagcagtagcagtgctggggttcacagggaaggtattgggtataatggcaatcaccttcttatcagatgtaatattgatatgggcaaatgccttaccggagaacacgtttttctttaccacaaatccattggtagtatccggataggagatggcgcctgccaccagaccagctttcagccgggcagataccctcggcgcaatggctttaccatcaaagttatgagggaagacaagcaccttactgccttctttttcggctgcttcggcaatagctttggtatatacaatgctttctacttcatgtaagcgggcatctgctgcgtgtagtaccttttgtgcgccatagttgcccagtgcggccagttcagcagcgtcaacagggcccagtaccagtgcagtagcagtagtacccagctgttcagccactttagcgccatattgtacggcttccagcgccgctttcttgattttaccctgtgcctggtcggcaaatattaatatagacatgaataatttgattagtagttgagagatagtttacccttagatcacttttgcttcttcgtgcagcaacttcaccagttcttccacgttatcaggactgatcagtttaacgccggcctttgcaggaggcagttcaaagcttactacggaagtgagggcgtctgcagcaacaggttccaccacagtgaggggcttggttctggcggccataataccgcgcatattggggatccgggcttcagccattcccttctggcaggaaacaactactggcagcgatacttcgcacacttcttctccgccttctatttccctgttaacggtagccacggtaccattcaggtcaaatttagcagcaatggatacatagggcaattccagcagttctgccaccataccgcctataccggagccattaaagtcaatggtttctttcccggtaaaaataatatcgtattgtttatcctttgcatgcgcagctatctgcgacgcaatatagtaactgtcagcactatccgcatttatacggaaagcctcgtctccgcccaaagccagtgccttgcggataaccggatcacaatctgcaccacctaccgtaataagatgcacgtcagcccctatggtttctttcagctccagcgcccttaccaatgcataccattcatcgtacggattaataataaactgtacaccagcctcattgaatttcgtgttattgtccgtgaaagctatttttgcagtcgtgtccggagttttgctgatacatactaaaatcttcatggccttaaactgttttgttttaaaatgcggtaatagcaaatatatctaaataatatacgccaaccgcagggagggaagatgattttaatcagtgtgagagattgacatattgtacaattaaataataacaaacgaatggacagaatcgcgcaaataaagcagttcctggtagccacaccaaacgacagcttcctgaaacatgcattggcgctggaatacattaagctcaacgacgatgtaaccgccaggcagttgtttgaagaactgctggcccatgaaccgggctatgtaggttcttattatcacctggggaagttactggaacgtgccggtgataatgccgccgccatcagcacctatgaaaaaggcatggctatggccaaagcaggtaatgaaagacatgcatacaacgaattacagtcggcctacgaagacctgatatactgatattattaatccaacaaacaacgcatgcctcaacatctaataactgatttcactgcttatatctccggccggcaattatttgatcctgcgcaaaaggtgctgctggccgtaagtggcggggtggactccatcgtaatggccgggttgtttaaaaatgccggttaccgcgccggtattgcccactgcaactttcagctgcggggtgaggaatctgagcgggatgaagcttttgtacggaacatggcagcaacactggaactgccgctgcacgtagtaaaattcgataccaatgcttatgtggcccggcatcgtgtaaccatacaggtagccgcacgtgaactgcgttatcaatggctggaagaagtacgcgctgcggaaggatacgcatatattgccaccgcccaccatatgcaggacagtgtggaaacagcattgatgaatttcgccaaaggtaccggtattgccgggctgcatggcattctgcccaaacaggaacgcctgatccgcccgttattgtttacggagaaagaccggctcatagcgtatgccgccatgaataatatttcttttgtagaagatagctccaatataactgacaagtatacacgtaattatttccgtcaccaggtgattccgcgattacaggaagcctttcctggtgttgtgaaaaatatgtcggctactattgaacggatcagggaagcggagatcctttaccaggaagcattggcgaagcaccgtaaacgcctgctgttccagcaggggaacacctggatggtgcccgtattgaagctgcagaaaacgatcccgctgcaaacaattgcctgggagctgttccggacttttggctgttcatccgcacaaacgcaacaggtattatcgttgatggaaagtgaatccggcaggtatgtggatacggccagtcaccgcattgtgcgcaaccgtcagtggttgcttattaccccgctggcaacagatgcgtcgccgctggtagtgattgaacccggacagcagcatattcattttggcggcggacaattacaggtccgtgagcaggagcggggcaacgccggtattccagcgtcgccggaaatagcctggctggatgcggcacaggttagcttcccgttgatcctgagaaagtggaaacaaggcgattacttttacccgctgggcatgcccaaaaagaaaaaggtaagccgtttcctgattgatcagaaattatcaatgccgcaaaaagaaaatgtatgggtgctggaatcaaacaaacgtatcgtgtggctggtaggtatgcgggtggatgaccgcgtgaagattacgcccaaaacgaaagcagtacttagtattacttttgcgaaataagaaatagccggcggagtggaataccaacacagccggcggtttcatttatcgtccgaatcttggatgcttgagcatctccaggaaataggcgcccagttctggatggaaaatcagtggaaatacgataccgaatagcgcgccccacatatgtgcatcatgattgatattatcgccgccttttctcgacatgtacgctgacaaagcgaggaacaaaacgccataaattacggcagggatggggatgaaaaacaaaaagatcgtattccacggatctatcatgatggctgaaaacaccaccgcagaaatagctcccgaagctcccagcgaagaataactggagttgttacggtgttttatgtaagatgggatatttgcaacaatgattcccaatagatagtataaaatataaaccagcttgctgtgaaaaagctgcatgaataaattttcaatggcagggccaaagaaaaataatgtgagcatattgaaaatgagatgctgaaaatcggcatgcacaaaccctgaagtaatgaagcggtaatattgtttgtaacgctttaccatgtacggttgcaggctcatcttgtccagctggtcatagttcttaagggcagtataggaaacaagacaggtaataatgataataatcaaactgatggaaagcgtcatataaccggtttatttaggtggtaaaggtacttattgatgatgatacttttctctgtttaaaactgtataagcacgatacagttgttcagcaaaaataagacgcaccagctgatgcggaaaagtaagcggggataaagacattttcagttgcgccctttgcaacacggcatcatcgataccaaacgcaccgccaattaatatgatcagctgacgtgtacctgcattgttgcgttgctgcaggaagtcggcaaactgcacagtggtcatcatctttcctttctcatccagcgcaagcagaaaatcggtaggctgtaacatatccaggataatttttgcttcctgttttttcaattccggcaccgataaactggcagcctgctttaccgtggggattagttttacttcaaaatccacgtaatgcagcagtcttttctgaaaaacagccatcccatccctgatgtagggatcatgttcttttcctatgctccagagttgaattttcacttcgtttaataattaagcaattggtgtaaaagtaagtgtaaatcagaagattgcagaaatttttttgataactatttgggattttcgaaaaatctcctacctttggcatccattcataaacacatggctccgtagctcaattgaatagagcatctgactacggatcagaaggtttcaggtttgaatcctgacggggtcacaaggcggaattccttaccaataagggattccgcctatttcttttcttgtatagtgatttttcagaacgcgtaacacttccggtaacgttaaaattgccagtgaaacttcttcccaacaactgttcccggttcgaaataacaaatccgcatttatcagtaaacacgaattgatagcttttaaacaatttgcctatgcaaaacaaataataccgcactgattttgctatgacgatgatgttgatattcctgcttataaacgaggcaggaaagtccatcgtcaaatcaagtaaaataagtaataaacattgagtccaacaccgtattacgtatgaactattatacaattccgcctccggtcaaacttgcggaatacattcagttcttttgggtactggaaggttcagctacagctgaaaagccattccatcaccgggtgctggccgagagttcaccggaatggatattttattgcaaaggacaattcgaggcttacggggtgggcgacgaccggcacaaaacttctttctcctgtttatcgggacagctgcagcattttagaaaactatatactttgaacgatttctgcttgttcggtgtatacctttttccttatgcaatccccggtatttttggtttaccagcccatgtgctgagtgatcaaacagtggatacagaaacactgctcggaagagaaggacagttgctcgagcaaaaagtattcgcggcgtctgatcaccggcaacgtgcaacactcatttctcaatttattttgcagcggctggcgaagagcgcggaaacagcgagtcctgtttttacgtcggtaagacagatcctgatgtcttccactgccttgtctattcctgcattggcggatgagtgttatttgtcccgcaggcagtttgaaagaaaatttattcattatgcggggtacagtcctaaacaattccaacggattgcccgtttcaatgcagttataaaagggtttgagaaacggccggtatcgctcacggaaatggcgtacagttgcggatattacgatcagtcccattttatccacgacttccggttattttcagggtataatcccaaagcttttttcacgcatcagaaagatgcggctgattaccgggcgtttgaagaattcaatccctgacgcggaggctgaaacatgtcgcgattttacaattttgttgattgcaccaacagtagctttgtaaaaaaagagccttatgaacttacagcgcaagaccttcataaaaaatcatattccattcattttctttattggattgtttattttgacaacggaaaaagtattttcacaaacaacaccagatggaacttcaccggctgtcagcggcattaccaccgggcgggcccaggccctggctggcgcgatcatcgcactcattagtttaattatgggatggcgggctaaagcccgttcccgttcaacacatcttaccggaaacaggcagaataaaccaacagcagctattattgcgttgtcgctgggagcaatagccattatcctcagtgttgtacatctcagcacttctgccggtgctgtttttggttcaggcagtggaaaagccggagccattgtggcacttgtactggcactgacgggcgctactttaagcggactggcgcttcgtccgaaaggaaagtgaaatagcgtttttcataaatcaaataccgcatgctatggacaagcacaatgaacttgtagctttttatggtgttcgttatatcgtaaaagatgtagccgccactgtaccattttataaagagctgctcggatttacggttgacatgcaggctgcgcagggttttgcaaagctatcaaaaggaaccctccacttgtacctgaatgagccgggctttggaggcgccggacagccgatgcctgatggtaccgcgcctgcaccgggcggatggaaccggatccaactggaagtaattaacctggaggcgttcattgaaacattgaaaacaaaggatgcacgttttcgcaatgggctggtgacaggcgccgggggtaaacaaattctattgcaggatccttcaggaaacctggttgaattatttgaaccaaatgaacaggccaggtccctttaatccctgctatctgttgatggcagacctttacagctacctatacaaatcacgtatacccgttaacggtagtctcggaaaaatagttttaattttttttgtttaatttaaaacaaatcctacatttgcaatcccaaacagggaatggcttcatagctcaactgaatagagcatttgactacgaatcaaaaggtttctggtttgaatccagatgaggtcaccaaaagacagaaaatgctgcattaactgcagcattttctgtcaaaagaaaaaaatctggagaaaagctttcaggtataaaaaattgaaaaataatttgttagaataaaaaattgttctacatttgcaatcccgaaacgggaaaacggcttcatagctcaactgaatagagcatttgactacgaatcaaaaggtttctggtttgaatccagatgaggtcaccaactaaaggacgaatacgagttacatcggttcgtcctttttttatgcccgggtatttacattagttatatttggtatatatttgtaataaccggcacctgttaaaacagtcaaccataccaacacaccacaatgaaatccctatccgcattcgccatcttcctactcatctcctttactagcctggcacagccgcaaaacaaccatacggaagaaaagatctgcttcctcacttacggcttccccgatattgaaagggttcaggtggaacaaaccatcgcccggaaatagggctttgctttttatacagtaggggagtgtaccgttgaccaaacgctcatcgacagcgtagcccgtgtcaataacgtggcgaatagaaagatggaggcaagatatggcagcaactggagcagccgctatcagcaggaggtagacgccgttttcgccacccctgaaagggcgcaggaattggtaaatcagcaactgtatatctggcgcaaggaacaggaattaaaagtgcagaacgacagcctccggtacgcctgggctgctaccggaagaaaaggcgtttataaggtaatcgtttccggatcagcaaaaaatattatcttttacaagctgttggtagactatccaaaatataaagtttccctgctgacagacagataattgttttacccaaacggaaaccgggaattatgatacggatcagaaaagaaggcatactgctgaaacaaaccaatctcgagtttgaaaacgaaggcgtgctgaatcccgccactatcagggcgggaaacgaggtgcttttttactacagggcagtacagaaaggcaatcactccagcatcggtttttgtaaattaagcgacccgcttacggttgaacaacgcctggataaacccattctgtttcctgaacacgactacgaagcaaaagggctggaagacccccgcattgtgtgtatcgatggggtatactatctcacgtacactgcttacgacggtgtgagcgcctgcgccgcgctggccacttcctccgatggtgtaaagtttgaaaaacacgggctgatagtagcgcaaatggattacgcggaatttaaacggcttgcggaaaccaatggcccgctggatgaaaaatatatcctgtacaacgattttaatcctcgtttatgggataaggatgtagtacttttccccagaaaaattaatggccggttttattttctgcaccgcataaaaccacacatacaactggtttcggtaaacgaactatctgatcttacggcggatttctggaaagattattatctccatctccgcgaccatatcatactaacgccaaagtataaacacgaaatgagttatgtgggcgccggttgtccgccggtggaaaccccgcacggctggcttttcatttaccacggcgtgcatgaaaccccgcaaggctacgtatatgtgggctgcgcagccttgttcgatctcaatgatcctgcgaaggaacttgcacggttaccttatcccatattggcgccggagcgggattgggaaatcaggggagatgtggataatgtttgtttccctaccggcacagtcgtattcaacgataccctgtatatttattatggcgccggtgatgaagtgattgccaccggaagcatcagcttaactgagttgttaaatgaactgctggcttatcctgtatagcaggctataaccgcttcaattacgcgtttcgtttcatcagggtcgcgcactttgatgcaggctacgcccgtttcctttgcggggtaatcattgccgcctggaaaaatggcgtctcctgcaaacaacatttcttcaatagtgatccctaaaatatccctgagtttgtggatgccgtaggccttgtcgatgccatgcctcgtgatatccactgaagtagtgccgcccaggcttacagaaaactccgggatgatgccatccagcaaggctttcattttttgcctttttgcaaaatcgggatcccactttttcttttcttccagcggggcttcctgtcctaatgcagagaaggtgatctggctgccacggtcttctatggcaggcccccaaagttttgcagctttatatcccagggtgtttaccacttcattcaaagcgctggtgattttctctttttctgctgcggtgaaatcttccgcatataatttatcccacttaccattgtacgcgtaaaactgtgtgccacaggtagggagaatagatagccgttccagccctttttcgccaggcagttttgccagcacctgctgctcaaactgtggccaggcgccgccggaaataatcgccaccctggccacggttagcaatgaatataatagtccgctcatttcttcatcaatagcagatttactctgcgccaacgttccatccaggtcaaataccaccagcttcttcatttgttgcggttatttttttagtaaggccagtgcgcgttcacaaatattatctgccgtgaatccaaactcacgcagcaatactggtcccggtgcagaggcgccaaagtgatcaatagaaataatctcacccttatcacccgcataacggtgccatccctgtgaaatacctgcttccactactatccggtttgttacatcggggggaagtatctggtcgcggtaagccggagattgcgcttcaaacagctcccaactgggcatggatacggtgcgcacggcgatgttaaatgactgtagtttctcctgcgcagctacaattaagtccacttcggcgccggtggctatcaggatcagctcaggctttgcgtcaggcgcatctgcgaggatgtaaccgccatagcgtaacccattggcagctgcatatttgctgcgatccagggtaggcaccgcctggcgggagaggatcagcgctaccggtttgtccggttcaaggattgctatctgccatgctgcaatcgtttcgttggcatctgccggacggatcactaccaggcggggaatggcgcggagtgcggccagcagttccaccggctggtgggtaggaccgtcttctcccatagcaatactgtcgtgcgtaaacacaaagattactttcagttctgaaagagccgccagccggatcgatggccgcatataatcggaaaaggtgaggaaggtggcgcagtaggggatgatgccgccatgtgctgccaggccgttggaaatagcgcccatagcgtgttcccgcactccatactggatatttctgccatcgtagccccatacaccgccggcagcgccctgcaggtcgccatgttccatcgccggactttcaaaattaccggcgtcctttaattctgtattggtggacgtgttaagatctgctgagccaccgatgaaaccgggaagatgtttgaaaaacgcctgcatcactttccccgacgcggcgcgggtggccagtcctttggcatcagcagcaaacggcgtaatgtccttatcccagtcttccggaatatggtcatgtatcagcgagcgtaattctttggccagctccgggtatttttgtccgtagatgatcatttgctcctcccatttggaagataatgttttgccaacgtctacggctgcacgaaaatgatccagggcttccgccggcactaaaaaatccggttccaccggccagccaagtttctctttcgtgagttttacatcttcagggcccagtggggaaccatgcgcaccggtggtatcctgtttgggagaaccaaaaccaatacgcgtgcgcacgaggatgatggaaggccgctctgtttctgcctgcgccatacggatggcttcatcaattgcttccaggtcgttgccatcggctaccttctgggtatgccatccgtacgattcaaaccgttttgcatgatcttctgtaaaggtaaccggtgtggcagatgccagggtaatccggttatcgtcatacaaatagatcagcttgcccagccgtaaatgaccggcgagggaagcggcttcggatgccacgccttccatcaggtcgccgtcactcaccagcgcataggtgtagtggtctattaccgtatcacccggacggttatactttgctgccaggtaagcttccgccatcgcaaggccaacgccgttggcaaatccctgtccaagcggaccggtagttacctccacgcccggcgccaaacccctttcaggatgccccggtgttttactgccccattgccggaaccgcttcagctcttccaacggcaaatcataccccgtaacatgcagcaaactatataacaaggcagagccatgtccggccgataatacaaaccggtcgcggttaaaccaatgcggatcggaaggattatgacgcaggaaccgggtccatagtacataggccatcggcgcagctcccaatggcagccccggatgcccgctgtctgctttctgtacggcatctaccgataaaaaacgcagcgtattgatacatagttcatccaatgcaacggaattgggaataagagaagtgttgttggtcatggtattccttttttgtaataaaaatgatcatacataggtcaacaaacttcatgcgcagatggttgccgtattattttttaattagtctactaaaattatagacttttcaaaaaatattgtattattgtgcttcgtaggctttccgggtccgctttaggggaaactcatccacctgttgacataccccgtttatctttcaaaataataccgacatggaaacatcattacagttaatgaggaatagttgctgtgtagcatttgcggcaaaccgatgttaggacgcatcaatcagaaataaaaaggccggaactgttgacgcagttccggctggtaatcaaggctgttggagacattttacagtgattgcagttacctgctttcaccggcctcattttttcataccaaagtaaagataatgaaaattgctattgcatgcagctgcgggctgctgctggcggctaccgcatggtcgcaggaattgcgcgcacctcacagcgcagataccaccaaacctgtgcacaggaacattgttcaaaacaacatttcactttcaggacggattatcgacgccaaatcacaacaacctatcgccggcgctattgtgcatatcaaaggcaccacccacgaggtgcaaagcggtgcgaacggggagttcgccttcctcaccggtcagaaagtgccggtcatctaccagatctcttccctgggttataaactcaaagaagtatatgccgataaatccaatgcaggcaatatcgccctggaagagctcagtacacaattgaacgacgtggtggtagtaggttatggtacacagaaaagaagggaccttaccagcgccatctcctccgtaaaaggcagcgacgtggtaacggtgccggtagccagcttcgatgcacagctgcagggcagggccgcaggggtacaaattaattccaataccggtgttcccggcgatggcgtatttgtaagggtacgcggtactacctccatcaacgccgataatgacccgctctatatcatcgacggtgtatttatgaataactccagcctgcaaacggtgaataccggcggccgctcgagttccccgctggcggatatcaatcctgctgatattgaaaatatagaggtattgaaagatgccagcgcaacagccatttatggctcccggggcgccaacggcgtagtgatcgttactacccgccgcggcaactataacagcaaagcaaaagtaacggcagatgtatcggctggtgtagcctgggcgcccaaaatgtgggacctcaccaccggcccggaacatgctacgctggtcaatgagttttaccgcaactccctggctgatgccaccgctctcaacgacaaagcaggcatcaccaaatacagctaccagcccttccgcgcgctgacggacaatccggataaatcgcctgcacccaggggattgccgcaggatcagcaaacctacgaccgcctcggggaaatatttcaaacagccccgcttcagaattataacctgtccctttccggtggtaaccgtgaaaccaagtattatttcggcggcggctattccaaacaggaatctatcctccggcccatctcctttgaaagggccagctttaaactgaacatcgatcaacgggtgaatgacaaggtaaccatcgggtccagcaacagcttctcccgcagcttccgcagccagggccgcgctggtgatggcccgcagggtggcctgttgcaggcagccttgcatacgcccacctatctcccggaaacaaatcccgacggtacaccggcacggtgggcaggctttgataacgtgcaggtactcatcgataactacgacgtacacaccacaagcctccgttatatcggaaacctttacctcgatgccacactgctgccggacctgaagtttcacagcaacatcagcatcgattacaataactataacgaatccgaatactggaataaccttacccagctgggcgccagtcccaccaacggtttggccacttccgccattacacaaaacacctcctggatcaatgaacaaacacttacctggcgcaaacatgcaggagaaaaacatttcttcggcgtactggtaggcaacaccatccagagtaatacggaaacattaacctctgcgcagggaaccggcttccctaacaattcttacaaatatatttctgcggccgcaacccgcaccgctgcgcaaacatggacccgcagcacattgtcgtcgttcttctccaggatcgattacaactatgcaggtaaatattattttgaagcaagcatccgcgcagacggctcctccaaattcggcgacaactataaatggggatacttcccctctgtaagtgcatcctggcggctcaaggaagaaaacttcctgaagtcggtgaacagcatcagcgatctgaaagtacgcgccagctacggcatcacggggaatcaatccggcatcagcaacttcgcggcaaaagggctgtggtccggcggtgcaggctaccccgacaacagtaccggcgatcagccaggcaccgcacccctgcagttgccaaaccccgacctacgctgggagaaaaccagccagttcaatggcggactggatctcggattactcaacggccgtatcaatatcactgcagatgtatactacaaatacaccagcgatgtactgctgcaactgcctaaagcaggcgtttcgggctttacgtcgatctatagcaatgccggtgaaatcagtaataaagggtatgaaatcgggatcaataccactaatatcagcacccgtaatttcacctggacaagcagcctgaatattgccggcaataccaaccgcattgaaaaactgccaacgccgatataccagtataaccgcgactggatcatcatgcaggaaggttcacccatgtactctttctggctgtacaaccagctgggcgtggatccgcaaaccggtaacgcgatctttgaaggtgagaaagatggcaagctgccggtatctgcccgcaaagtaatgggcaacgccatgccgaaattttatgggggcttcagcaataccgtttcctataaaggttttgacctgagtgtattgttatccttccagtatggcaacgacgtatacaacctgaacaaatttttcggagaaggaggaggcacccgcgatgccaaccgcgtgttatttgccgatcagctcaaccgctggcagaaacccggcgacatcaccaatgtaccgcgcctcaccgcttatggtctcaactacaccatcgatcaaaacaaccgcttcctggaagatggttctttcctgcggcttaaatcactcactgtaggatataccattcctaagtctgtcagtgaaaaactgcatatccagctactgcgtgtatacttcatcggtagtaacctctggttgctgaccaaatatacggggctggacccggaatcaaacgtaacgggtatacaaaccgtacagggactggatcttggcacgccgccgcaaccacgcagcgtgcagtttggcttaaacgtaactctttaaacgctcttaattctcctgtatgaaagcatatcggaaatatatatcgctcttctttctttcgctgacagccttgtcatgcaagaaatttctcgacgtggaaccacgggacagtgtgtctgacgaacaaacgatcattgataaaacatccgccactacggctttgcgcggtgtgtacaggaagctgggcagcgacggttactacggcgctttgttccagaccttcggctacctgcccggcgataatgtgcagtggaccggctcccagtcggttatacagcagtttattacccataaaataaatgcggacaatggtaacctgcaaacggtgtgggcggctatttatgctaccataaacggcgccaacaacgtgattgcaaaagtacccggcctgcaggacgctactttttcggatacggaaaagaaccaggcagtaggagaggcgtactttatccgcgccctgagctactttgatcttgcccgcacctggggaaatgtgcaaataacgttaacgcctacactcaatgcttccgataagctggatgtaaaaggcagcacacaggcgcaggtataccagcaggtgctaagcgatctgaatgcggccgactcgctgctgcaaccgccgtctcaaacaggcgcgcctaaccccgtgagggtaaaccagcaaaccgcctgggcgctgaaagcacgctactatctgtaccagtcggactggacccaggcagaagcctatgccaccaaagtaattagcgacacacgaagctatacgctgctcaagccttacagcgccttcttttccccggccagcgccgtggctacaaaagaatctgtatttgagctgtcgtacagcgctacctacctgagcggccaccgcaactactggcaaccgccggccaacggtggtacgcggcaatgggcgccatcagatgcgtttatcacgctggtaaatgatccgaaaacaggcggcaaccgcaacgcactggtagctaaaacctctgccggtctgtggtatggcaacctttactacagaagccccgccaccgatccggcttatgtgatccgcatagctgaactctacctgatccgcgcggaagcacgcgcccaacaggataaaccagatctggcccgcgaagacctcaacgttatccgcgatagggccgggctctcaccagtgaatgaactgattgctaagaatgacctgctgctggccattgaaaacgaacggagaatagaattcgcactggagcctcaccgctggttcgacctggtacgtaccaaacgcgccggcgccgtgttgaatatcacgaatccccagctgtatgtatttccgatcccggccaacgaagtcaccttatcgaacggcaatctgaaacagaatgatggttactgatcttatcaccttataacaaatcaccaatgagtaatgtcacaataggggaaacacccgcctggaaagactatgaaaaaattgggttcagggtaatctttatttacttcgtgttgcaggcgttgccgctcgactggaagttttacagttaccttttttctacccccatttttaaacttcattatgaagatatctttaacctggccaattatgctacgcgcttcagcgcggggcctgctacctatgccgactggggcatactgctgatcattgcagtagcgggcgccgttgtatggacttacgccgatggccaacggacacgcacctacgacgcagccttttactggctgcgcgtgattctccggtaccggctggcactggcactgctggcctatggcttcctgaagctgtacgcattgcaggcgccatatccctcgctgagcagcctgaatacaccgtacggcgattttaaccgctggaagttgttttctctcagtcttggcatcgttccttcctacgaactattcctcggcggtgtggaaatatttttagcggtattgttactgatccgtaaaaccgcatctataggcgctttcatgttcctcatcttttgtggtaatgtctttatgtccaacctggcatacgaaggcggcgaccaggtatacagcctgctgctgatcacctacgcctttgttatcttcagcttcgatctgcagcggattgtccgtctgctcattctccaaaaacctacagcagcagctacgtttaaaccggcgtttgaaggtatccgtaaaaacggcaggtggatcctgaaaacagctttcctgcttttctttgtggtgatttatggtgtgaaaacaggtgtgggcgcaaaatacgatccctatcaatatcccaccaccaaagggttaccggctatcagcgggttatataatgtggccacgtttattgttaatggcgatacgcttgcttattcattaacagattcccttcgctggcgcaacgtggtgtttgaagaatggaacaccatcagcatccgcaccaacaaaccggcattggtagattccaataatcagcacctggtgaaacgtgataacgcggaaaggctatacgaaatagaaggtactagcggcaggcattactacagttacgccgccgatactacgcaacacctgcttaccctgcaaaacaggcaccccaggctgtcggcggaaaccttgtcgctgcactactcgcggccggatagcaacagggtgatactcacgggaaccacctacagcagggattctatctatgtagtactggaaaaagtaaataagaaatacctgttggaagaagtggcaaacggaggaggacgaaacaggaagttaaaactttaaaccaattatcatggctcataacacacaaacattaccagatgaacccgtgatcagggatacgtccccggtggcgttgccggctgtcagtgcacctttgtcgcagctgccggcctggaaagaataccagctggtactattccgcatcgcctttatttttttcattgcgttatcggttcccaatagcgtggagtggtaccagcaactggtgcagcttgactggacgcagttgaactaccgcgacttgtatgatattgcgcgctttggctccgggattaatttccttggcaacgccatcttcggcagctccctgctgggctatgccaactggatcactacggcgttaatagctacagccggcggcctcgtgtggaccggcatcgtaaaagcccgcaagctgccgcgtaaagaatattataccgcgtggtactggctgcgggtggttgtaagataccgtgcgggtatcggtatcatcggctttgggtttaccaagctgttaccggtacaaatgccgtatccatctttcggtattttaaataccaacttcggggatcttactgcacagaaaatttactggttgtctatcggtattgtaccctggtaccaggtgtttgcgggcgtggtggaagtaacggcaggcgcacttttatttttccgtaaaactactacgctgggtgctgttttgttgtttgccgcgttgggagatatcgtgtatgtgaactttgcctacgatggcggcgtgcatgtgtatagtagttatttcgtactgctggcagcgttactgttagtaaatgatgtacctaaaatttatcgtttgctggtgcaggagcgtttcacggtaccggtaaattattatcctgtttttccggagagatggcaacgctatacccgcatagggctgaaatctgctaccatcttccttttcctgggtgtgcttttttatctgcagctgatcaatttcttgtatgatccttacaaacaaccatctgtggcgggcgtaaaggagctacgcggcaactaccaggtaacggaattccggttaaatgaccaggtgatcccgtattcgccgctcgatacggttcgctggcaggaagccacgtttgagaactggtctacttttacttaccgcgttaataagccgcacccgctggatctgtccaatggcggcggcgacccgcagcgcgatgtgaaccgcacctttgaaataaccggtctcgccggcggtcagcgggctttccattattatgcagatgaagtaaataaagtactttacctcgaagataaatataagcccattccggacaggcgtaaccgcaccgccggtgtaggcggcgatggtggcgtggtagtggataaagcggcggaaaaggctgcgcgtgaggaagcggccaaggctgcgaaggactggattccggcagcagcgcgtaaaaatataggtgatgaatcattaaagatagcccccattgcattgtccgcccggagggcaaaagattatgccgccgcacctgcctgggaaaaccggaaacgctttacggtgaaatattccaccagcgatggttcgcatgtggtactcaccggcgtggatgaaaataagaacaacatttacgtggtgctggatcgcatcaacagggagtatacgttgacacccagcaccttgcaggcaggaaaatactaagaagcgctatgttgataaaacgaaccaactgttaccgggtggctgttgtaatggtgttgggtatactggcttgccataccaacacccggccaccggtaccgggttggccggaacattttggatttgggaaaacagccacccgccggcaaatcgattcgctgaacatctccattgctccagatggcaaaggcctgcccgccggtagtggcaatgcagcaacaggcagggttgtctacctggccaaatgcgcttcctgtcatggtgaaaccggcgctgagcccacggccaaccggctggtggctacgctcagcgatacggtgcgcacaaaaaccatcggcaattactggccttatgctaccacggtatttgattatatccgccgcgctatgccctttaatgcaccgggatcgctcacgaatgaagaagtgtatagccttaccgccttcctgctgtatcgcaacgatatcatcgacagcaccctgcaactggatgcaacaaacctgtctcatattgtaatgccggcaaaaaaatattatgtgaacgacgaccgtcgtggtggcaacgaagtaaaatgaatattatgtcaggggaagacaacaagatacctagaaggacaatactgagagcagcggcggtttccgctgctgcggcactaatgggcgcttccagggtgcagcgtggtaccggcagcatcagcgcgggaaaggacacggtttacacggatcctaccaaaatcacgggcacacttccgggcaaactcggaacgcgctcaccatttgagcagccgctgaaaaaaccctccgatatttcttcccgcacgccgctgcaggatttgtatggcattatcactccgtcggacctgcattttgaaagaagtcatgccggcgtgccactcattcatcctgataagtacgaattgctgatccacggtatggtggagcggcctatgatctttactttacgcgatttaaagcgtttcccggccgcatcgcgcatcgcctttatcgagtgctcagggaacttcagatcgggcaaggaaaccatgacgccgcaggaaatttgtggcctcacgagtcagagtgagtggaccggtgtaatgctgtccacccttttccgtgaagtgggcgtgcatccaaaggctacctggttcctggcagaggggtccgatgctgcagtaatgacccgcagcatcccggtggaaaagggctggaaagacgccatgatcgcctacgggcagaatggagaggccattcgtccggaacagggctatcccgcgcgtttattcctgccgggatgggaggggaataccaacgtaaagtggatccggcgtattgaattgtcggaccaaccctttatgacgcgtgaagaaacttccaaatacacggaaaccatccgggatcataagatccggcaattcagcttcgatatggatgcccggtctatcattacctatccgtcgtttccgcagcaggtggaaaagggctggatagaaataagaggcattgcctggagcggccgcggaaaaattgatagcgtggaaatcagcaccgacgcagggaagcattggtcaaaagcagtgttgcaggaaccggtaatggacaaagcacacacctattttcgccatctctggtactgggacgggcaagccacagagatcatgagtctcgctacagacgacacaggctatcgccagccttcattaaagcaactgatacaggcgcgtggaacagacatgggaggatatcatgtgaacccggttaccgcatgggtaataaaaagagatggcaccgtgttgtttaaaccggaaaagtggaagtgagtttattcgaataaggtcagctcatcgcgggtaactgcgtgaaaaagattttgtaactggtgcacatgtacaatggcacggccatatggcaccagtccttctgcggcatctgtaagtggctgaaacacttcgttttcatgcctgatatgcacactatgcagccggttatatttcagggaatatacattttcatcttcgccgtagtcgggatctcctttgataaatccaaatctcagcagcaggtccacatccagcaccatcgggtttacctttgcatagggcagtttactgagcggcagtcctgaattatacacaaagccttgtaagatgccttctactacaaaggctgtttcttccatgttataatcaaagtaagatacatagttgcctatccgtatgtctgattcttctatcatatttttatcttaataaaatataatcagcaacaaggtgatcaacgccggtaacgcctgtacgaaaaagatctttttactggcggtaagcgctccatatataccggcaacagctacacagcttaaaaagaaagtggccacatgcaagctccacaccgggtcggagataaagaaggtccaggccaggccggctgccaggaaaccgttgtacaggccctggttggctgccagtgctttggtagggacaaacaattcccggggcagttgcttgaatattttaggtcccctgctggtccaggcaaacatttcaaaccaaaggatataaagatgttccagcattacaaaagcaaccaatattttgatggcgaccagcatagtgttgaggtttataaataaatataggtcaaattattctttctgcaagccaggcaattgccagcgccagcagggtgcctgcggcataacatacacaatcgctccacaggaatccatgtcccagcaggataccggcaggtgtgttacggaactttactgcccattctgcctggtacagctgctgtatttctatcagcaggcaaaccacgtagttgctgatgccaattttccacaggggagtaaccgggaacaggaaccggatgccaaaaaagatacaggtggcagataacacatctcctccatatatgcgtatgatgtcaggaaaatattgaggtgcccacctggtggcgagtcctaaagggatattcagtaaaataaggaaaaagtaaatccagcgcctttttgctaccataggttcaaaaagcggtaaatatagcaaagaaaaccggaatatgaggatgggtcaggagagagaaaaagggacctgcggccccttatacgatgcaataacccggtggtcgggttattgctgattatcactttcaacgctacttttcttttttccgcggttggttccgcctttacggccaatagcggccatgtgttcacgatttctgctaacggcttcaccgccttttttacctgcagcacgggcttcctcagaagtgaatttgtgggcaacaccttgctggtgtgcagcttttcctccttctcttgaaatggcacgttgctgttcagggtccatagaagcgaatccgcgtttactgtgtttactcttctgatcagagttcttttccgaaacatggttaaccggtgtggcagtttgatatctgatgtcttccataatcctgaggttttttttagtgatagtagttaaacatttacgctaacccggaacaagatatgtgccatcacgggttagccacgatggtagcggatttgaggcacatggggatgtgaaatggggcaatacattccacaatccatagaattttccacacacttttattgtctgttctacagtttttaatcgggaactctctcattttccgtggcttatattttgtttttgcaaccatgtcatttcttttcttaacccatctaaatttttttgttatggcaaaatattcaaaagaatcccagcacaaagtagagaaaagtatgcacgaaatgcatgaaggaaaactgaagagcggaagaagcaaaaagaaagttacgaatcctaagcaagctatcgcaataggcttatccgaagcccgcgaagaaggagcaaaggtgcctaaaaaagcagcggcaaaaaaatccactaccaggaagtccactgcaaaaaaagcagcacccaaaaaagcggcagcgaaaaaatctaccgcaaaaaaatctaccgcaaaaaaagcggcgcctagaaaagcagcagcgaaaaaatctaccggaagaaaaacagctgctaaaaaaacaacggccagaaaatctaccgcaaaaaaagcagcgcctaaaagaaagtcagccgcgcgtaaaaaatcagcagcaaccgcataagtaaagggttttcaggatcgttttatccgtttaatatatacaaaaagaccggtgactggatagcaccggtctttttttatggtatatggcttgcaggattatgaagtatggaaaaacacagcattactgtgatcattagaggtaaaccctacgggttggttattacaatcgacaagggcgctctggaaacagcatttcaagtgattcctgatgtgagcgaacatgtgctcgatgaatttgaaccccacggtacagcctttattgctgatcacgaagatacccttgagggaagcatccgcacggtagaaaccgaacagattgcccgtattatctgggaagatattctggataaaatgaaataaggctttgttgcttcactactacggttgtaccttcgcagcaaagcgagtatgaattgctatgatggtaaccgataaaacctataagaacgctaatcgcagggaaaggatcatattcctcgtaaaactgctggtatatctgggcattgtttattttaaccttgaacaccctgccgtatatgataaatttacatggctgtttaagcttaccaatgcactctcttttttcctgggagccaacctcgttatctccctggcctggctggtaatcctctcgtggtatacccgccgacgcaacaggcagcggcctatcgaaaaagacaatttcattctcggcatcaaccgcatttcctccgtattaaatactatttttctcctgctcgccatcaccttcttttttggcgtaaatccccttaaatttgtcaccagcatcactatcgtggcagcagccattgccctgatcacgaaagattatatcgccaatatgatcaatggactcatcattatgttctccgatcagttgtcgctcggcgaccacatacgcattggcgatatcaaaggaagggtgatggatattaccctcatcaacctggtattgcagaacgacgacgatgatattgttattattcctaattcggtagtgtttacgtcggttgtactgaaccagtccaaacaaaatatccgtaaactcaccatcgagtttgaactggatcataagcatccgtttaccatccgcggcctggaagaccgcctgaagcaagccatcgacgcgtattcccgcagctatacccccgaaagcttttccctgaaaacaatggagatcaaaaaagactttgtacagtttaaagtacaactgctgatgccgcaagccaataaggaagttgaacgcctcatcaggcgggcgctcaacacagaaatcatggccatcgccgaaggtgtgaactaaaccagtaccatcgcttccacaaagctttccacaaactgatctatctgcgccctacttacattaggcatacagatgatatgcgaacagccgctttctgaagccagctgccacttccggcggatgcttccgggaggatccggaaacaccaccgtaatagcatcggggttgcgccatgccggaatgccgttttcgttgaggcgttccactgcgtaagcggctactgttaaactgtgcctggccctttcccgcaaaccttccacacccaggcttttcagtgcataccacaggaacaacggactatggccgtttcttgaaccggtaatggtggtgtccatactgccgatatacgccaccgaccgggcaatcctgtcgcggttggattttctcgcaatcaccaccccgcagggaatcggggcgccaataaatttgtggccgctgatggcaatgctgtctgccccatccgcaaaatcgaatgcaggcctcggctccaggaaagcgctgtagctgccggacaacgccccatcagcatgaatataatgatggcgtatggccaggttcttcaggatatctttgattcgctttacatcatcccgcgcttccgtcatggtagtaccgatgttcgccagcataatcaccggcagatgcctgttcatacggatggtgttttccaggtcgttataatctatttccccgttcggcaatgtgcggataataatccccggcatattgagcaggtgcaggttcttctgcacactgtaatgggtagcctcggaataatacactattcctttgggatataattcccgcgcgagatacaggccgtataaattgccctcggaacccccgttggtaacatacccccaccagtcgtcttccggcgcacggaaaaggccggcaaagaaggaaaccacgaatttctccatctccctggatcccacggcgtaagtggccggcacaaaaggatcacccaggttatttaacggatattgtaaaaagggcaggagtggactataatcaaaatctttggacacaggatatcccaggaaatccctggtacgcgtttgtacctgcgctaacagttcattcagcgttgcagcatctgctgcggccagccggtactctttcataatcgtattttacaggtgtatgatgctgtaaaagtacatattggtaatctgattgaactggaataaatattgaattagaaaatatatactacttttaagtctttgtaagataaatagcactgccgggcaaccgccggacatcttttaaaagaaaaatataactgccatggatacactggataaaacagaccggaaaatactggacgccctccaggcagatgcacgcctgaacaccaaagaaattgcacaccgtatagggctctccgttactcccacctacgaacggctgaagaaaatagaaaaaagcggggtgatcaaaagctatgtaaccctgctgcatggcgataaagcaggcaaaacgctcgcggcatattgtaatgtatcattgcagctgcattcacagccgctgataaagaaatttgaaactgctattgcaaaaatggaagaggtgatggagtgttatcatgtagcgggcacgtacgattacctgctgaaggtagtggtaaacgatatgcgcagctatcagtattttctgacgaataaactggcggcggttgaaaacatcgggcaggtgcacagctcttttgtgatgacggaaatcaagcacaccacagctttccggctgggatagttagcgcctcagcacactcacaccgctgagcggatgatcctgtaccactaccgtataggccagcgggttagtctccggttcttcggacaaagggatggtaaacgagaaactgctgccgttgccgggcatactgttaaaccagatctgtccctggttgcgttctacaaagtctttggaaagatgcagccccagcccgcagcctttttcgttctgcgtaccgctggtagagtagtagatgttggagaaaatgcggtgctggttttccacaggaataccggtaccattgtcttttaccgtaatttccgcctgttcgccgtcatgtgtggcggtaatcattacttcaccgccggaaggggtgaacttaatggcgttattgatcaggttacgcattaccagcctgatcatatctgggtcggcgtataccataatgctcttattcagttcgtgcgacagcttcacttctttctgccgggcaagggtttgcaacagctcaaattcgcggtttaataataaggtgacgtcaaagtcgtcggcttttacaccaatgcctttcatttggttgctggcccattgcagcatattgtccatcatataggccgtattttttacgtccctccataattcgtcggtataaatgcggaactgtgccgcatcaattttctcatctttcagcaaaaagagtagtccttccaggatggccagcggggaacggaggtcgtgcgaaatgaccgaaaatattttatcctttacctggttaagattttccagggtggcgttttgctccaggataatgcggttctgcatggatacttcccggttcttgttattcagttccagatacagttcctgttgccttttataaagccggtacaccattaccgtaatcagcaacaacgccaggaaaagtgccccggccgacagcaccagcacccgctgttgctgaatggtagcgagatgcatgtgttgctctttcttcaataaaatattttcgcgttgcttcttttcagattcatatttttcctgtgagcgggatatcagccggcctttttcagcattgaaaaagtcgatgttacggttgctgtattccttgtaacttgcaaaggcagcggcataatcattccgggcagaatccagctcatagcggatcttgtaataaatcatctcgttttttacattacccagggtatcatttaataactttgctttttccaggtttttggcagcgcctttcagatcgccctgcatagtttgaatttcagccaggttcaggctcgacttcaccacaccgggcaaattgccggcctcctggtagtaggtattggagagctggtgatagcgcagtgcatcgttataccggtgctgaagcatcgcaacaatacccatgttctcataggtataggccaggccgcgctgatcgtgcagttccagctttattttctcggccttctccaggaacagcatagccgaatctggtattttcagggagatataagcagagccgatattattcagggtcttggcgatctccgttttttcgtttcttttcagctttatcgccagggcctttttcaggtaaatgagcgcgtccctgggcgtattcagttctgtgaaaatattccccacatcattattgagtaccccgagtgtgtaagagtcgccgaggacttctgccagtttcagggcgttgagggtcagctgcatctgctgatccaggtgtcctttggtattttccacgagggcaaggttgcgccaggcccatatttttcctttggtataatgaagactgtcgcttaaccggagcgcttcggcgccatacttcgctgcagtaggggcatttatagtaaaataagtcctggctacctggttcagcaggtttacacgggcggtatcgttttgtgaatgggagtgtagtactgccagcaggctgtcgtggataagctgttgcgctgttaccgcaggcgacagcaaaatcagacataatgggattaaaacgctcttcttcaaaggactggccggcagcatatttaatattgttggcagtgacagagtggagcgattcgggggcggtccactttaatataggttaaaattaaagataatgtgccacgattcaaagtaagttgggaaaaaagtgaggaatgggagcatgaatttagtgttatgcccgccataaatcaattaggttgtatctttcccgaaagattaatagcaatgaaaccgctcattaccatagaatactgtccgaaatgcggctggttactccgggccgcctatatggcccaggaactgctgactaccttcacagacgaactgggaggcgttaccctccgccccagcgaaacagggggctcctatattatctggcttggcgaagaaaagatcttcgaccgcaaggaaagcgggcatttccctgaaataaaattcctcaagcagctggtaagggaccatgtgagtcctgaaaagagcctggggcactcggaccgaccgtagcgcacgccttcggcgtgggaaattgtcttggctcaggattacgctgattatactgattttaaggattttgatttttttgatttttttttgatttcgtttgtactgattaggggaaatataatctgtataaaatccaaaaaaatccaaaagtaaaaatcaagctaatcaataaaatcagcgtaatcctgagccaagacaattttcccacgccgaaggcgtgcactccgctaaaatctttacatttgcagcctatgcgtaaaaacctccatatcacggctttatcacttttattagcaataggcgcaaaggctcagcaggatagcactaccacaaccccttcttcttcacgggaagggctatacgatagcgtatggttacgtaaacggagtttctttccgttgccggtgctcggctactcccaggaaaaagggctggaaatcggcgccgccatgttgtattcgttttatacggataataagaatccagacagggctacccgtaactccacgctcaacctgatccccgcgatcaccacggaaagccagtacaagatagacctgaaagcaaatatctggacccgcagcaatacctggcatttcaaaagcaatctccggtatcataactacccgctttacttcttcggtatcggcgataccacccattacgataaccggtcgctggtaaacaacagccgctataaagtacaggtggaaggggaacgccgcatcagcggacacttttatgcaggcgcctccatattataccagcacgatacctacagcagcggcgatagtaaaggcatttataccaccatgccgcttaccgataaagaaggtggatatgttacctttctcggactcacaggtatcttcgataaccgcgataatgaaaattttgcccgccgcggttcatggctgaaactcaacctggcatacgcaccttcttttttaagcaaacacccgctttttaaaatcgaagcacaaggatcacatttcctgtccatctcccgcaaaagcacacttggctttaatggcatcttcaacagtttgcaggggaatgaactgcccttttacctgctgccggaaatggggaacgacctcatcatgcgcggctattacaccgggagataccgcaaccagaactacctggccggacaagcggaatatcgctatctcgttgatcctaaaatgcgcatccatatctggtttgtggatatcaaaccaaaatttgcactggcagcatttgccggcaccggtaccgtgttcgccaatcgtgatttccgtttcggcggatttaaaccaagctatggcgcagggatccgttacttctacgacgaaaatgcaagactcactattcgtatagactacgccgttggagagaagcgcagcggtgaatccaggcaaaaaggattgtatctgtctctggcggaagcgttctaatgtggtgcaatggtgatggttatgtggtaataatttgttaactttcaatagattaaataccatactccaaaaccattgcatatgaaaaatctattcctgctaggagcagttgccgtgcttttgattgttacccacagcacccaggcccaggacaattccagcacccaatcttcttcacattccaaattttatctcaaagttaccggtggatattttttcagcgtatcgccggggcagtttcccaatgttggcccgtatcctccgcaggatctgcacacagagtttaacccggcttccggtatggatacgattagccggaaggtgctcaccggttcttacggagaaggtttcaggggaggactttccgttggctataacatcaataaatattttgcggtagaaggaacctttaattatttccacagcaagaaaaacctgatgacccgtcagcggactaccctggccggttctggcagggaactgggacatgtggagtcgcatggacatgtgaacgcaatagattttgcacccagcctggtggtaagtccgggctttgaaaaagtaaacccctatgtgcgctttggtgtaatcgttccgttatggggccgcctctatattgaaacggatgctacccaggtgtcaagccccgccggtattcctacaggtacgcaggtagttaccaatatcagcaggaaagaagaaatcaaacctaatcctactgtcggtttccagggagcattcggtgtatcatttacagtgtcaccccgctttgatgttttcgtggaaacggaatacaagaatgtgccggtgcgcagtaaagagaaagaaatcactgagtacaatgaaaccaataccctcatcaatggtactaccggcgcggtgatacaatccctgccaggccgtactattaacgatttgtcggtagcggaaaagaatacaaaatacgtaactacgctggatcagggctccaatacgccggtaaaccagcagggcaccaaagtgatttataaagatgataataagccgggcaacgacctgaaatcctatatcaatatcgggggactgggattaaatgtaggattgaaatttaatttgtgatcataaatagcataaaaaaggggaggccatttaacctcccctttttttatgcacttgctttgtcgagtaacgccactgctgctgaatccagctgcagctgcacgccattcatcagttcatgcaattgttctttactggtagcactggcaataggcgccgccactgcagggcgtgtaagcagccatgccagcgccacgccggctggcgtagagtgatactgggccgctacctggtccaatgccgccaggatatgaagccccctttcattaagatagctcaacgctttctggccacgggcggtgcttttgcccgtgtcggcggccgtccggtatttgcccgtcaggaaaccactggccagcgaataataattgatcacgctgagatgctgttcttcacagatctttgcatactgctgctcatattttttgcggtcgtacaggttgtattccggttggaatgtttcgtaccgcggccagccgttttgcttactggcttccaggctttccagcaggcgggcggcactcatattggaagtgccgatagcccttaccttaccggcttttatcaacgtatcataagcggccagcgcttcttccacaggagtggcttcgttatcgaaatgcgtttggtaaaggtctatatagtctgtttgcaggcgcttcagggacgcctctgcggctttgaggatataggccctggtcacatttttgccttcacccatatcaccgccggctttggtggccaccactactttgtcgcggttacctcggtcgcgcatccacttaccgataatagtttcagattcacctcccgaattgcccggtacccagcgcgagtatacgtccgccgtatctataagattgaacccatttgccgtaaattcgtccagtagtgagaaagaagtggattcattggccgaccagccgaatacattgccgccaaaggccagtggggctactaatagcccggattgtcccagtttccgtttttccataataatttttttattgatacctatcgcgggtacatcccgtacgtaatttaattacttttgtctttcaccgactaatttttatgccagaacagatgcctgctatttcacgcgaagattttaactggttaacacaaacctatggaaaggagagtggctactcgcacatagataccaaagaaagtgtggtgcatgaaatttttgtagataaggtgcttatcggtaccgccttcctgaactgtgcttcctatgaactttcttttgatacgccgggactgcacatcaggaaaaacagactcgataattataagttgcacgataaagcagtgctcatccccgatgagatgaatgaggaagatgaagaggagctattgctccgctggtctgatctcatgcacgaactaaagatgctcgaaaaccttcacggtctttcaaatgcccgcgaaccgctggcacagctgtacctggatatctttaatgaagatgatgcggaagaccagatcagtcatttgccggacatcgtgctgccaaatgccacggccatatgggaagaattatatgctgcgctatccgccaccggcaacgtggtggaatttgagtggcagcaatttgcagaaagcggtatcattgcgctgaatgggctcaggccattgcaacaggctggtattatgctgaaagcaccggatgcagatgattttgaagccatcattggcgcagaagattttgccaaaggcgtgctggattttgtaaatgaccagctggatgaacatgaattgaaaatagtggcagccggtaccagtctggatgaatatcaatccttcacctgccttaatatgcaggactttcgcctcgccaatgccctgttgaaaatggaagaactctgcctgatctgttttttttaggacattaaaatccggttaaaaaaatacgaggcgctgtcaaagcaggcacttttaaataccttagtacattcattacagtataccacatgaaattattccggcatttattttatgtattgattacggtgatgttcctgccacaggtgcaggggcagccctggaaaatacaggtaaaaggcacggataatattcacctgaccaccggcatcgcctttaaagcggcggagaaagcaccgcggttccgcactacggttaaccggttcaaacgccgccctgttggtatcaacgacagctacggccacgaaaaggtttgcccccttttattgtccgccgttactacccggtttatttatgtagacaaaaccctcaaaggatattatttcaatccttacctcagcgtacccacaccgctaagaagctggagaggtccgcctgccgcctgataacccgtttatcttttatttatttcattttcttttttagcgatttatgaacttacatatgatcgcgaagaagtggtgttggtggttgctatgtattttccccttcacttctttgttcgcacaatctgcagcggatagcttttcgctgcagcgggccattgcgcttacacttgcacattaccccgctataaaggccaaacaggcccaggtaaacgccggacaggcaaaccttacagatattaagcacaattggtacccggccataaaactgcacgagcaggtagatgccggcacagacaacagcatatacggatcttatttcaccatgggaatgattccctccacttccggggggatccgcccggaaaataacagcgccttaatgagcggcaatatcgcaatggccgctatgcagtgggagatctataactttggcgcctacggcagtgaacagaaagaagcggcacaatcacttaaagtgcagcaaacagatctgaataatacggccaaccagctaacggtatccgttattcaaaattacctggaactgctccggctgtatgccttgcagcaaatagcatcggacaatatccggcgtaatgcagaagtgctgaaggcagtaacggctaccgtgctgcatggcctcaaacccggagtcgacagcgccatagccgccgcagaattgtcgaaagcaagactcaccctgctcgatataaaaaacaactataaccaggtgcgcattcagcttagtgttttcaccggactcgatacggcgctgatcctgcccgataccattaacaacaaacgcctgcggctgttgctgggcagcgaagcgccggacagcctggccgcccatcccatgctggcttattatcatgcggtatacgaacaacaacgcgccgccgctgaggtaatccgcaaagcaaggctgcccaaagtaaacctgatggcagcaggctggatgcgcggctccagcggatcattcaatgatgtatatgataaaaacctgtggagtggcctcgggtacggcaggtacaactatttattcggattgggcatcacatataatcttacagacctgaaacgcacacacgaaaaagttgctgtgcagcaataccgctcggaagcagccgcgcaacaactggctactacccgcactgcgctcagtgggttactgcaacaggcgcagtcggatattcaaacttcgcgcgagaaactacaggaactgcctttgcaactggcagccgcacgggctgcagcccggcaaaaaatggcgttgtataaaggtggtctcaccaatattattgatgtcaccactgctttatttgttttgaaccgcgcggaaacagacctggtacaaacgcaggatgcagcctggaaagcactgttccgtgctgcttatgccggcaatactatttcacaacttttacctgatctgaattaaacgctattcattatgtcatttgtatcttcggcactgaagaagcccattgcggtggtggtaatcaccggcggactactgcttttttcgttgctgtccatcttcaatatacccatcgatatattcccgaaactgaacctgccaactatctacgtgatagagccatacggaggaatgtcgccgcagcaaatggaagggttctttgccacccgcctgcaggatcagttcctgtatgtaaatggcgtaaaaagtatttctaccaaaaacatacaagggttaacgttattaaagctcaccttttatgaaaacacagatatggcggaagcttctgcccaggtggcgttacaggtgaaccgcgccatgaagttttttccgccgggagccttgccgccgcaggtcatgcgtttcgatgcatcgtcgctgccggtgggagagctggtgttcagcagccctaaaaagtcgctgaaggaaatttatgatctggccgctacccgcatccggcctatgtttgcatctgtacccggactgtcggcgccgccaccctttggcgctaactcccggtcggtgatcataaatgttgatccgcaaaagctgcgcagctttaacctcagcgccgatgaagtagtggaagccattgcgaaaaataatgtgatgacgccctcagggaacatccgtatcaacaataccatgtttgtgaccaccatcaattccctcgaaaaagaggtggcggactttggtgatattcccattgttaccaatggcaacaacaacgtgttcgtacgcgacatcgcccgtgtagccgatgctacggatgtaaccgtggattatgcattggttaatggcaaacgctcggtatatatccctgtggtaaaaacagccgatgcctccacctgggacgtagtgaaaacactgaaatccaaaatcccggaaatgcaaagcctgctgccggatgatgtaaaggtatcgtacgaatttgaccagtcggtgttcgtgatcaatgccgtgaaaagcctgatcacagaaggtgcgctgggcgcattgctcaccgggctgatggtactcttgttcctgcgtgacctgcgtagttgtctggtggtagtggttaccatcccggtagcagtgctatgcgctgtaatgggattgaagctggcagggcaaaccatcaacatcatgtcgctgagcggccttgcactggccatcggtattctggtggaccaggccacggtgactatcgaaaatatccatcagcacctggaaatggggaagtccaaacggctggcaatttatgatgcatgcgaagaaattgcattcccgctgttgctcatcctgctttgcatcctggcagtatttgcgccttcatttattatgaccggggtgccacgtgccatgttcctgccactgtcgttgtctatcggctttgctatggtggcttcctatttcgcagcgcaaacattggtgccggttatcgccaactggtggctgaaggctgataaataccaacaccatgcccatgccggcctggcgcttgatgcggaagaaataaacgaagtaaacgatcatctgcagcaggcggtgcagcatccggaaaaagcaaccggcttcgaacgctttaaacagggctttatgcaggttctggaaagcggtatgaataaatcccgtatagtcgtaaccgtttatatcattggttccctgctattggctggtggttgctacgtatggatagggaaggacctcatgccccacatcaacgccgggcagttccagcttcgtttacgcatgcccgatggtacccgcctggagcgcacggaaagcgcactgcatgaagtgctggcggtagtggacagtaccgtggaagggcatgtggccatcagctccgcttacgtgggattaattcccagcagctatggtaccagtaacctatatatttttaacagcggcacccatgaggcggtattgcaggtgaacctggaagaaaattacaaagtaaatatcgagacactgaaagatcagctccggaagaacatcacggcgaaaataccggagatgcggttgtcctttgagccgatagatctcacggaaaaaattatgagccagggagcagccacgccgatagaagtaagggtggcagggaaggatatgaaacagatttccgcgtatgcacaacaactggtagataagctgcgcgacattcctttcctgcgggatgtacaaattgcgcagccactgcatttcccggtgatcagcattcacattgatcgtcttaaactggcacagatgggtttgaacatttaccaggtggcgcgttctgttacagcatccacgtcctccagccgctttacggaaaaaaatcaatggctcgatgaaaaggtggcatatacctaccaggtacaggtgcaggtgccggagtacaacatgacggctttaaacgacctgaaagagatcccgctggtgaaaggccagcccagaccagtactggcagatgtagccactttttcccaaacggaaatgccaggggaatatgaccgctccggtccgcgtagattcgttaccgttagcgccaatatttcgggcaaagatctcggtgctgccacggccgccgtgcaacaggcgattcaggaaaccggcacaccgccaaagggattgatcacagaattgaaaggcgcatcaagcctcctggtggaaacgttgaacagcctgcaaaatgggctgatgatagcggtagcagttatcttcctgttgctggcggccaattatcaatcatttaaattatcactggtggtactcactaccatcccggcagtaatcgccggtgcactgatcgccctgttactcaccggcgctacactcaacctgcaatcttatatgggcatgatcatgtctaccggcgtatcggtggccaatgccatcctgatcgttaccaacgcggaaaaactccgggtggaataccgcgatgcagggaaagcagccatcgtgagcgccggtataaggctacgtcctatcctgatgaccagcctggccatgatcgcagggatgatcccgatggccagcggccttggggaagcaggagatcagacggcaccgctgggacgcgccgtaatcggcggactgatagcttccacacttgccgccctgcttatattaccgcaggtatatgcgctgatgcagcgtaaggcaggttatcagtcgccctccctaatgccggacaatgccaatgtttaaaataaaatctaaaataatgaagtactataaatattacctgttcacggtaagtataatcatggccctggcggcctgtaattcagccgctatgactgataaaaagaaaacaaataaagaagaacgtcattatatgctcgcaacagtggtacagcgaccgctggctggtagtatccgcttgccgggcgcgttagccgccttccagaaggttagcatttatcccaggatcaatggttttgtgaaaagtatttctgtagaccgtggctccaaagtaaaaaaaggacaggtactcctggtgttggaagcgccggaagtaacccagcattattacgctgcacagtccaaatacctgcaggcagcggccatgttcgcctccagtaaggataactacgaacgtaccgtagccaccagtgaagaaccgggcaccatttccccgcacgacctggagctggcaaaagcccgtatgctggccgacagcgcactgatgaacagcgagcaggccaatttccgcgcgcaggaagtaaaccgtggatatttaactgttaccgcgccctttgatggcgtgatcacagaacgtaacattcaccccggtgccctggtggggccggacaccaaagtggatgataagcccatgttgatgctggagcaggaagacaagctaaggctgatgctccaggtccccgaaatatacagcgcccagttatcagaacagtctgtgatcacatttgaggtcaatgccattcccggtgaacatttccagggtaccatcgccaggcaggcgggtacgttgaatgataaataccgctctgaagctgtagaaatagatgtacagaacgcgaaacggttactcaaagcaggaatgtatacagaagtgatgctgccgctgaaaggctctgctcaggcgctgttagtgccggccagcgcaattgttatgtctacggaaagaaagtatgtagtcgccgtaagaaatcactatacaaaatggattgatatagaagaaggtaatcatcacaacgactccacggaagtgttcggccatctgcaggcggatgaccgggtgatcgcaccggcaacagatgaaattaaagaaggtatcatgatcccgtaagcacagttccggcgttttttttgtagccatacgttaaaaccatgacttatgacgatcaaaaaaagcacttccgaaaagcgtgagctgaaagaaacaaagcgtaagaatgaagcactggctccggccaaaggcggcgccaaaaaggaaaggaacgacgaccggaataatgtattggaagggtatgatgaagacgaatacgatcagaaagatatcgcagacagcaaacgcaaaaagaaaaaccaggactaaaaaaaagtgccgtcccgaggagtcgggacggcttttctgctaactgttccgtctatattgattttcttatgttcttattaaaaaaagagaacaaataacatccacctagtaatcaataacggatttacctgttgttcaactaaaaaaactttataaagtggcaatgagattccttcacgtatttttacgcgaaatgttttcgataggttaaaatgtttttggattttatgtttggatgcgcaatgacaatcataacgggttacgctatgcggatgatggctgctatcttcttaaatattctttcccttttgtgttatcttgaaaactcctttagtgcgcatctgaaataataacacgaaacgatttaaaattgttctgggaaaaccgtttttaaaaattaaaaagttcgcggatgccgagcgcaaacatctgaaccccgataacagcgagaataagtcccatcatttttgtgatcaccatcattacattggtgccgattatttttacaatgcgttcacctgcaataaagagcagataggtaatataacatataaatgcataaatggctattacaatagccaggtgtgtaaggtcttttgccgcggaataactcatggaagtggtaatagcgccggggcccgccagcagcggcattgccagtggggtaatggctacgctgatcccctggtcggccttcaccggttgagcgccgagtttgggattttcatttttattttccttttctccgcgtaccatttcatagccaatcacgaatacaaggataccgccggttacacgcaacgcggccaatgtaatgccaaaaacatgaaaaatgagtttacccgccacactgaaaacaagaataatacagaaggcaatgatcactgatttggtggcaatatttcgcttcgcttttttatccatattggatgtcagctccataaaaacagggatggctgaaacaggatttacaattgccagtaatcccatgaatacggtggttgcaaaagcaagataattatcaaataatgccatcatatcagcaatataataaattttatttaccggcaaacatcgctgctaggaacgtaagcggggcaattgccagttatgacgcaggcttagcaaccggatggtcactataacggtaacggctataccctgcgcaatgtctccggaaacgccggtaaagtgccccgcaaccaggtacaggatgccaccggcaatagatgccgcagcatatatttcgcgggtaaaaagaatgggctgctctccggtgataacatcgcgcagtaatccgccgaaagtgccggtaataacgcccagcgctacacatatgggcatgggaagccccgctgccagtcctttattgataccggtaatagtaaacagcccaagaccaatagcatcaaaggtgctgagtaaacgggtgagttttttcacataggaaaaaaataatgcggcaataatagcggcggcaataatggccgtgttggtaagttcgtccgtcatccaggctactggcgtggcgcctgtcagcaggtcgcggatagtaccaccgccaatagcggtgataaaagccagcgccaatagtccgataacatcatacgacttattaatagctgctgtggctccggaaacagcaaacgcaaaagtgcccagtaattccaatacctggataaaggtaagctgcattctccttgtctgatttatgaactaaggtaaggatactttatatgactacgacaggagaacaacaaccaactcaataatcatcctcataggcagattcaccacggagcgtacgctctatctggttgcggagaccatgactgaatccttccacttcaattttaggatggtgatccaggtagatcataaagcgccctgtttccttcgtaacaaggtcatagatatcttccagtaaagcgcaaagtaatctccgggtattttcagcgatctgcgcaagagaggaatcttcaaaatgccggtattcacggtttttataagataaggtaatctgtatcataactgacggtttttctgcaggaattaggattaccggttaaaatatggctaaccggctggttttcattatctaattattaaatctgacataaaaataggcaaaaagaaattgtttttttaatactaaagggtgattttttattaagtgaacactaccgtccctatattgttcattttttttctattataatttggctaccattgcaaattattcttacataatgaagaaacttacgctactcattgtttttatcgcgctgtattatttaccagcacaggcgcagccaggaaagggcatccggtggagcctcgacggcaaatcctattttaaagccacccctgccgggatcgaatcttacccgttgtccggtgaagcatcttccctgaaagtcccggcagtcagctatcacagccttgccataaaggatttttatttttcaggagatgaaaaaaaagtactgctttacaccaattcgaaaaaagtatggcgttatgaaacccgcggtgactactggttactggacatcgccagcggaaaactcctgcagctcgggaaagataaaccggcttcttcccttatgttcgccaaattatcaccagatggcacgaaagccgcgtacgtaagcgggcataacattttcgtggaagacctcgccataggcgccattactcccattaccacggacggtacccgccgttttattaacggtacattcgattgggcctacgaagaagaattcggctgccgcgacggcttccgctggagcccggatagcaagcgcatcgcctactggcagattgacgccacaaagatccgcgacttcctcatgatcgataacactgattccatatattcctttacggtgccggtagaatacccgaaagcaggagaaagcccctctgcctgccgcatcggcgttgcagatatacaaactgctaaaacaacctggatgcaggttccgggcgatcagcaacaacattatattccccgcatggaatgggtgcccggtaaaaataccctcatcatccagcagctgaaccgcaaacaaaacgaaagcaaaataatgctctgcgatgccgccaatggaaatgtacgccctgtttaccaggaaaaggacagcgcctggatcgatgtaaagtcgcgctgggacgatgacaacatcgccggatgggactttatccgcagcagcaaatcctttatctgggtgagtgaacaggacggctggcgccatctctacaatatttctacggatgatggtaaagccactttactcacaccaggaaactatgatgtgatcagcatcgccaaaattgatgaagcgagtaacaccatttatttcctcgcctcaccggacaatcctacccagcagtacctttacaaggtgccgttaaacggaggcaaggcagaacctatcacacccgcgaatgaacccggctcccacgaatataaaatttcaccttacggaaactgggctatccacgacttcagtaacgcatatacttatcctgttagtgaaaacctgcagctgccggcgcacaaaagcaaggacaataccgtactgaatgctattaccaaaggcgctgcagcacccaataaaccggagttcttcagcatcaccaccgttgacggcgttaccatgagcggctggatgagtaaacccgccagttttgatccctccaaaaaatatcccgtggtattttatgtatacggcgaacccgccggcgctacctcgctagacgccattggcgcaggccgcaatttcctctacgacggcgatatggctgccgacggatatgtgtacgtatcaatggataacaggggcaccccgttgcccaaaggccgcaactggcgtaaatgcgtgtaccgcaaagtaggattgatcaatgcacgcgaccaggctatgggcaccaaagcattgttacagaaatatacttttcttgatccgcaacgcaccgctgtatggggctggagcggcggcggctccatgacgctgaatctcctgttccagtatccggagatctataaaacagggatcgccattgctgcggtaggcaaccagcttacttatgataacatttaccaggaacgctatatgggcctgcccgaagaaaaccgggaagattttgtaaaaggttcgcctatcacttatgcaaaaaatctccagggcaatctgctttatatccatggcaccggtgatgacaacgtacattatcagaacgcggaaatgctgctgaatgaactgatcaggtataataagcagttccagtttatggcttatcctaaccgcacacatagcatctctgagggacaaggtacttttgaacacctttctactttatatactaattatttgcgttcgcattgtgaaccgggcgcaaaataagtacctttgcctccctaaattgaaaagtatgtccaggacagctattattggaatactggcagtgttgctggtgattatctgcgcgtttttgccgtggtcggtggtagacgtggaaggcaggcacctggtttttacaggcgtaaacggaacgggttccaattacggagagccgggccggttatgtattatcctttctgtactggcaattggaatattcctggtaaagaataggtgggtgtccagggtgaacctctttattgtagggtttctgctggcctggaccttcaggaatatgttgttgtattcaagatgtgagatgggtgattgtccgcagtcgcaacccggcctttacttgtcattagctggtgcgctggtagcctttgcctgcgtgttgtttacacgtccgcctaaaaacagtaaataaaaaacagcatcgcctccggcgattttaaattgtcttggctcaggatgacgctgattttactgattagtttgatttttactttttggattttataaaggattaagggagatagaagcggatattcgctcttatctcccttaattattatttaaagaaaatctaaaaatccaaaaaaatccaaaagtaaaaatcaaactaatcagtaaaatcagcgtaatcctgagaaagacaaaatccgcttcagaagatggttttatgtaaaatccatgcacccgcaaggataccggctcccatcaaccaataccgtaaaatcaccgggagcggacgttgcgcggttactttcgccttgataaaactgaaaatcgtgagtcccaggaaaaccagcaggatactggtaggggaggccgctgcgaaattttcattggaaagataaggtcccagcgaaaggataccacccagcaaaaagaaaaccccggtcatcagcgcactcttgatagcacgggaacggctaaacgcagattcctttactttctcctgttccagcatcagctcccacgaatgcgcatccttttccatttcctgttctatgtgtgcaatcatacgcgggttgatatccaggcgttgcagcttggaccgttcctggtccgacagcagggcgctgtcgtgctgcaggtcgcctttattagcctggaaagcgctgatcatcaccagtacggcgccaatgatcagtgcgcacaggtgaatggtgtaaaaggtttgtacttcaatggggaatacctgtatcacctgcgtcgcaaagaacaacaggaaaagcccatcgggaaacccgattaaaaaatctgtcttccacccggaactacggatggctttatgggatatagtcatacaaggttcactaactgaaagcctgctccaggcttcttttgatgatctgcacgcaatcgttgatctgtcctgcgttgatagacaggggcggtgcaaaccgtattttatcaccgtgtgttggttttgccagcagaccgttttcttttaaagtaagacaaaggtcccaggcagcttccgggtctttatgttcaataacgatggcgtttagcagtccttttccacggatggtggtgatgtaaggcgaatgcagttccttcaggccgttgcggagcaacagtcccatttcagcggcgttttccgccatcttctcgtctttcagcacctgcagggaagcaatggccactttgcaggccagcgggttgccgccataggtggagccatgttcgcccggtttaatggtgagcatgatctcatcatccgccagtacagcactcaccggtaaggtgccggccgacaaagcctttccaagtatcaggatatccgggcgcacattttcatggtcgcacgccagcattttgccggtacgggccaaacccgtctgtatctcgtctgcaataaataacacattggcatcctggcagtactgccacgctttggataaatacccttcatccggtaccattacacctgcttcaccctgtatgggttctaccaggaatccggctacgtttttatcctgtaaagcctgttccagtgcagttaagctgttgtagggaataacttcataacccggtgtaaacggaccaaaattatcacgtgcagcaggatccgtactgaaagagatcacattgagcgtacgcccgtggaagttattggcgcaaacaatgatctttgctttgtctttcggaatgccttttacaatataggcccaatgacggcaaagcttcagcgctgtttccactgcttccacccccgtattcatgggcaatactttatcatatccgaaataagcagtgatatattgtgcatattctcccagcaaatcattgtgaaatgcacgggaggtaagtgtcagcttttttgcctgctctataagggtggcaataattttagggtgacaatgcccctggtttacagcagaataaccggacagaaaatcataataacgtttgccatccacatcccataaaaaaacaccttcgccccggtccagtacaaccggcagcggatggtagttatgggcaccatattgttcttccagcgccaggtaatgttgtgacttttcacttatcgtgtatgaaggtaccataacccaaaagtaaggaaaaagatgaaagaagctgttagccgtcagctaacagctcccggctaattgccccctttcagtttctttaccaggtccacatattcctgcatcgccgcatccttcgttttacctttcaactccgcccacgcttcgtgcttggctttcgccacaaaatcaaatgggttggaaggaccgtcgttatccacgtcgccggttgttccctgtttgtacaaagcatacaactgcagcaaaatttcattggacggtttctccggcagggttttactggctgctactgcctcttcaaactgactggttagttccatgtgcggtgagttttaaatttaataatacgggttaacaccctcatttttcccttatgtctataaagttgagctttatatattaatatatcaaaaaaagcccgcgccatcctttctatctccttaaaaaccaaataacaaaacataattactaaacgcattaactaatgaactaatttcaatacctttgccggctgaaaaggtccgatgcagtacattgcagcaggacacggaatagcaaaaaaacatatgaagaatattcgcaatttttgtatcattgcccatattgaccacggtaaaagtaccctggcagaccgtttactggagtttacacatactatttccgaccgcgacatgcaggcacaggtgctggacgacatggatcttgaacgtgagaaaggtatcaccatcaagagccacgccattcagatggattacacggcaaaaaatggtgaaaaatatatctttaacctgatcgatacccccggccacgtggacttctcctacgaagtatcccgcgcccttgccgcctgcgaaggagccctcctcctggtagacgccgcacagggtatccaggcgcaaactatctcaaatctttacctggcactggaaaacgacctcgaaatcatccccgttatcaataaaattgatatgcagggcgccatgatcgaagaagtgaaagaccagatcatagaactcatcggtgtaaaaggagaagatatcctgcttgcctccggtaaaaccggtatcggcattgaagaaatcctggaagccatcgtaaaccgtattcccgctcccaaaggcagtaatgaagcgccgttacaggcacttatcttcgatagcgtgtttaactccttccgtggtatcatcgcatatttccgcgtgttcaacggctccatcaaaaaaggagataagatccggttctttaacagcggagaagaatattttgcagatgaagtaggcatcctgaaacttggactcgatccccgcaaggaagtattcaccggggatgtagggtatattattaccggtatcaaaagcgctaaggaagtgaaagtaggggataccatcaccttatccaataacccttgcttagaaggtatcaacggcttccaggaggtaaaaccaatggtattcgccggtatctatcctgtaaatacagaagatttcgaagagctgcgtgagtgcatggacaaactgcagctgaacgatgcttccctcacctatgagctggaaacctcgcaggcactgggttttggcttccgttgcggattcctcggcatgctccacatggaaatcatccaggaacgcctcgaaagggaattcaatcaaaccgttatcaccacggttcccaacgtaagcttcattgcacacactacccgcgatggcgtgatcatcgtaaacaacccgagcgaaatgcccgatcctaccaagctggacaggatcgaggaacctttcatccgcgcacagatcatcaccaagccggaatatattggtaacatcatgaccctgtgtctcggcaaacgcggtaacctcctgaatcaaagctatctgaccaccacccgcgtggaactgatgtttgaaataccattaacggaaatcgtattcgacttttatgataaactgaaaagtcagacacgtggatacgcctccttcgactacacaccaatcggattccgcgacagtgatatcgtgaaaatggatatcctcctgaacaacgaaaaagtggatgcactcagtgccctgatccacagaagccgcgcacaggagtttggccgtaaactcaccgaaaaactgaaagaactgctgccacgtcagcaattcctgatcgccatccaggcagccatcggcgccaagatcgttgcccgcgaaaacatcagcgctatgcgtaaagacgtaaccgcaaaatgttatggcggtgacatctcccgtaaacgtaaattactcgagaaacaaaaagaaggtaagaaacgcatgcgccagataggcaacgtggaaataccacaggaagcgttcctggcggtactcaaactcgatgattaaagcgtaggttgtcttactcaggattacgctgattatattgattaaggggattgatcactttggattttatatgattttgggagatataagcggatatattcgtttatatctccttttaatttttatataaatctgaaaatccaaaaaaaaatccaaaagtaaaaatcaaactaatcagtaaaatcagcgtaatcctgagccaagacaatttccgcatcgccggaggcgatcccgacgcgaaatttattatatttgagaaaaccaatcacccatgcgttctttagtgctctctttaacattcgtattttccgcgctcactttctcggccgtaaaagcgcaacaggcgccacccgccgccgaccaggtagtaaaagatgcctgcgcgcaggcagccaaagccaataaaaaagtgatcgtcatctttcacgcatcctggtgtggctggtgccataaaatggatactgccatgaatgatgccagcgtgaaaaaagcattcgacaacaattacgaaatccgtcatatcaccgtgctggaaaacggcgccaacaaatcgctggaaaaccccggtggcgcagatctgctggcaaaatatcacggcgatcaggaaggcattccgttctggctggtattaaacaccaacggtgaactgctggccgacagccgcatgaaaagccccaccggcaaactgcagaacgtaggctgtcccgcccagaaagaagaagtggattacttcgttggcatcctcgaaaaaacatcaaaaatgaaacgcggagaactcgatgccgtacgcaccagatttggtaaaatagccaacgccgcgcattaagcgaattttgtcttactcaggattacgctgattttattgatttttttgatttgaacattttggattttaaaggatttggggagatataagcggatatgcggattttgtctttcccgctgattacgctgattttactgattatttttttaaaagatttggggagatataagcgaaaatatccgcttacatctccccgaatcatttaaaatccaaagtgttcaaatcccttaatcagtaaaatcagtgtaatcagcgggaaagacaaaatccgcctatatctccccaaatcctttaaaatccaaaatgttcaaatcaaaaaaatcagtaaaatcagcgtaatcctgagtaagacaaaatccgcggaaaaatcgtactttaccactcctttcatacaccagccaatctcccggaaataagtttttatacaacaatctattcatatgcacctgactgcacgggaaaccgagaaattactactgcacctggccggtgaactggccgagaaaagaaaagcacgaggactgcgccttaactacccggaagccatcgcccttatcagcagccgcttaatggaagcggcacgcgacggcaataccgtggcagcgctcatgcactatggcgctaccattcttacccgcgaagatgtgatggaaggcatacccgaaatgatccacgaagttcagatcgaagctacttttcccgacggtaccaaactggtcaccgtacatgatcctatccgttaaccagtactaaatcttacaaccatgatccccggagaatattttttaaagaaggaagatatcattgccaatgccggccggaaaacggtcagggtaagcgtggtgaacaccggtgacagaccggtgcagataggctcccattgccacttttttgaagtaaaccgcatgatgtctttcccaagggaggccgcattcggtatgcggctcaatataccttctggcaatgctgtacgctttgagccgggagaagccaaggaagtggaactggtggagctgggcggcgcccggaaagtgatcggtatcaataaccttgtaaacggcgataccaccgatcctgctgtgaaagccgcagccatagccaaagcagcttccctcaattttaaatccgagcaactatgagcctgtccatcagcaaaacaaaatatgtaaatatgtatggccctaccaccggcgatcgcgtacggctggcagatacagacctcatcatcgaaatagaaaaggattacaatgtatacggcgatgaaagcaaattcggcggcggtaaaagcgtgagagacggtatggcgcaatcggccaccgcactgcgtagcgaaggcgtgctcgattttgtaatcaccaacgtgatgatcatcgatcactggggtattgtgaagggagatatagggattaaagacggtaagatcgttgcagtaggacaggcaggtaatcccgacacgatggacggcgtacatccgcagctcatcatcggcgcatccactgaagtacacaatggcgctaacctcatcgccaccgccggcggtattgatacgcacattcactttatttgtccgcaacaggtggatcatgccctcttcagcggagtaaccaccctgataggcggcggtaccggtccggcggatggcaccagcgccactacggtaacaccgggaaaatggaacatccagcgcatgttgcaggcggcagaagcataccccgtaaacctcggcttctttggtaaagggaattgtgctaccacagagccattggtggaacagatagctgcaggcgcgctggggctgaaaattcatgaagactggggcgctacgccggccgtaatagatgcttccctgaaagtagccgacgaactggacgtgcagatcgccatccacacggatacgctgaatgaagccggcttcctggaagatacactcaacgccatcaacggccgtgtaatacataccttccacacagaaggcgccggcggcggccatgcaccggatatcatccgcgccgcctccttccctaatgtattgcctgcatctaccaatcccacccgcccttatacggtaaataccatcgatgaacatctcgacatgctgatggtatgccatcacctggataaaaaagtaccggaagatgtggccttcgcagattcccgcattcgcccggaaaccatcgctgcagaagatatcctgcacgacatgggcgtattcagcatcatgagctccgactcacaggcaatgggccgtatcggggaagtgatcatccgcacctggcaaaccgccgataaaatgaagaaacaacgcggcgcactggaagaagataagaacaacgggaatgataacttccgcgtgaaaagatacatcgccaaatacaccatcaacccggctatcgcacacggcatctccacgcatatcggttccctggaacccggtaagatggcggatctcgtgctgtggaaacccgccttcttcggcgtgaagccggaaatgatcatcaaaggcggcatgatcaatgccagccgcatgggcgatcccaatgcgtccattccaacaccgcagccggtaatttaccgccacatgtttggcgcacacggaaaagcactgctgcacaccagcgtattattcgtatctgcgttatcgttagagaaaggcattaaagaagaatacggtttacagaaacaattgttgccggtgagcaactgccgtaacatctccaaaaaagatcttattcataacgataaaacaccggatatcaccgtaaatccggaaacatacgaagtacgggtagacggcgaaaaaattacctgcgaaccgttaaaggaactgtcgctcgcacagcgttattttttattttaatccggaagagatatgttggtaagggaaattataggaaatacggatacgcatacacgcagcagtaaagaaaccgacctgctgccgctggaatggtttgaaacctcgcggcgcattcagcgaaaactcactgccggcggccgtgaagtggcattgaagtttacaaaggaagggcagcaactgcaacaaaatgatatcctctaccaggacaacgacctgatgatcgtggtagacatccttccctgtgaagctattgtgatccgcccgcggaacatggccgaaatggcaaaggtgtgctacgaaatcggcaacaaacacctgccgcttttcctcgaagaggagcagctgctgattcccgcagaggagccgctgtatcgctggctccatgcggccgggtacccggtggtaaaagaacggcgcaagttactgcacatcctgcgtactaacgtacaaccacacacgcatggaaacagcggcccttcattttttgagaagatcctggaactggcgtcaaaatagagcatatggaacagcattatctcggcagcttactacacctggcagacagcacattgccaatcggcggctacacacattctgcagggctggaaacctttgtgcaacaggggctggtcaacagcgccgccactgcggctacctttgtgcgcaatatgctgcagaataatatccgctacaacgatgctgcatttatgagcctggcctacaccgcagctacacaaaataatgtgaacgaattgctggagctgcaccacctgtgcactgccgtaaaagcgccgcgcgaactccgggaagccagccagaagctaggcgcaagacttacccgcatttttagccgcaggtacaccagcgacctggtaacgcagtatgaaacagccgcaggtaacagcccgcactactgcctggtgtttggtatatacgcccacctcaccggcattccattgtcgtccgcgttgtatgcgttctattacaacgccgccatgggaatggtgaccaactgcgtaaagctcgtgccccttgggcaaatggacggacaggatatcatctttgacctgcaacatctactaaaagaactgacagcagtaacgatacaacccgacagatcattgctcggcctttgcaacgcggcatttgatatccgcagtatgcagcacgaacgcctgtacagccggttgtatatgtcgtaacaataattattcatacaatgagcagagaatacataaaagtaggagtggccggtccggtaggttccggcaaaacagccctcattgagcggttaacaaggcaaatggcgcaacactaccaggtagccgtcatcaccaacgatatttatacgaaggaagatgcggaattcctcacgaaaaacagcctgctgccggcagagaggatcattggcgtggaaaccggtggctgcccacataccgccatccgtgaagatgccagcatgaacctggaagccgtggaagaaatggtacgccgcttccccgatattgaaatcatctttattgaaagcggcggcgataacctgtccgctaccttcagtcccgacctggcagatgtcaccatttttgtgatagacgtagcggaaggggataagattccccgtaaaggaggtcctggtattacccgctcgaacctgctcgtgattaataaaattgacctcgccccttatgtacacgccgacctcggcgtaatggaaagggatgcccgcaaaatgagagtaggacaacctttcgtgttcactgacctcatgagcggtaccgggctgcaagacgtaattaactggattaaaagatatgcattactggaagacagcgccgtgcccaacctcttaacatgatcagtgaactgaagatattgacaggcaaaagggacagcagcacttacctgaaggaatgctactgcacgcggccttttaaagtggccaacgtgcgggaggaacgcagcgacccggtattgcgcctcatgatgatgagctcttcgccggggatgctggataaagatcattaccagttagatattaccgtaaccgcaggcaccgccctgcacctgcaaacgcaggcctaccagcggctgtttaacatggaaaccggcgctacacaggaaatgtgcgtacgactgcaaacagggagcaccttcacctttttaccgcaccccctggtgccgcatgaaaaggctgcctacaccggcacggcaaacctgcacctggcaaatgactgccgtcttatatggggagaaatcattacctgcggccggaaactaaacggggaaatattcctgtttacaaaactgcacagcatcacacaggtatttttgggggagcagctgttgttaagggataacctcctgatgcaacccggcgttaccagctttgatgcaatgggatggatggaagaatatacccaccaggccaccttcctgttttttgatacccatgaaaaggtactcctgaacgaaactgcggacaggcttcaccgttacctggaagatcaaccccatatcctggccggcgttacccgcactgcgggtaatggcatcatggtaagaatgcttggccatagcggggaacaactatttgaatgtcagcaccaactggcaaagcttttatctctttaaaaatgtagtatgtcatttattgataacagtttattgctaacggcagttactatcagctgtcttcatacggcctccggaccggatcattacgtgcccttcatcgttttttcccgcacccggaaatggtcggtggctaaaactattgggtggacggccctctgcggcctcggacatgtaatgagctcactcgtgatcgggatgattggcgtagtactgggctggcagctgtcgcgttttaccaccatcacagaagtgcgtggcggcattgcgggatgggcattgctgatattggggcttttctacctcatatggggattatataaagccatcgccaacaggccgcacaaacattttgatgtatatgacgacggcgatatgtatgtttatcagcatcggcacaatgaagcctatgtagcgccacagaaaaggatccgcgtaacgccctggatactgttcgtaatattcgtaatgggcccgtcggagcctttgttgccgttattgttttatccggccgcgcaacaatctgtacccggcattgtaatgctgatagctacttttacgttctttaccatcctcaccatgatcatcatggtgctgttgggatactacgggttttccctaatgaaacccgttgccacagaaagatatatggccgccatcagcggcgctgctgttacactctgcggaacaggcatggtttttatgggttggtgaactgtttggcagctcaagctgttatagcaaataaacctttaccacatgaagaaatggctcaggatcatccttattaccggcggtatatttatagcactcctggtgctgttaatcctgggtatgacctggtacatacatgcgaataaagacaatttcctcaaacagatcaccgcccagctaaatgatcacctgagcggaaatatccgcatcgcggatatggaaccttccctctggaagagctttcccagtgtgtctatcgccctgaaaaaagtagtgctggaagacagcctctttcagcagcatcatcacccattgctggatgttgactacattttcgtacgggtaaacacgttatcactgttacgcaaacacataaatgtaaatgaaatcaccctgcaggatggtaccatcttcctgtatacagataccaccggctattccaacacgtatgtacttcaacggaagtcggcaccaaagaaaaacaacggctcaaaagatgccagcattaaaaagctgatgttaacgaacatcagttttataatagataaccggcagaagtttaaactattccacctggatgtacgccagctggacggtaaggtgagcgccaccgacagtagtatccagtttacaatgatatcggatatcctgtctaaaagttttgcttttaacaccgttaaaggaagttatctgaaagataaaaaaatgcagttgaacctctccgtgatcttcaacaaacgcacaaagatcctgcacataccacaacaggaaatccgtatagatgaccacccggtgctcattgccgggcagtttgggtttggagaaaaaccaccaccgttccagttgaaaattaatgccaaccaggtattactgcatgatgccgccacctggctgccgcctgccatcagctccaaattaaacagcattaccctcacaaagccgctggatgcagaagctaacctcaacggttatatgaaatacagggacacccccaaagtgctcattacctggaaaaccaccaacaatgtaatggtaactacaatgggcgaatggaccaactgtaatttcacggggagatttaataacgaagtattaccgggacaaggccacactgatgaaaattctgccgttaatattttccagttgagcgccacgctggcaggtgtaccgctaaaagcagacaccatccgggtggtaaacctgaaacaaccattactgcacggacatttccggtcggattttccgttgaccaacctgaacagcgagacaggggaaagcccgatattgttcaaagacggcaacgccaatgcagatctatactacaccgggcccgtgctgaacagtgataacacgccttcgtccctgcaaggggtagtacaggtaaaacaaggggcatttacctatctgccgcgtaacttatcttttcatgatgccaacgccaccctgcgctttacagggcaggatctgatgctggaaaatgtgcatatacaaacacagaaaagtaacctgcagatggacggcatggtgaagaacttgctgaacctctattttactacgccggataaaattgaactcacctggaatatccgcagccagctggtagacctaaatgagttcaagagcttcctggcgccacggcaaaaagttaaaccaacccgcacccagcagaaagcaaaaatgacccgggtaaaccggcaactggatgtagtactggcttccagtaatgtaaatatgctggtgcagctggataaggttacctatcagcgctttaatgcacaaaatgtaaaagcatctgtacagctaacgaatacggatatactgttaaaacaaattgccctgcaacatgcaggcggaaatatgcagatggccggggtgctccaccagcaagggaataacaacaacttcaacataaacgccacggtgaacaatgtgcacatcagccagctgttttacgcatttgataacttcggcttgtcggccctgaaatcagataacctgagagggaatgtatcggcaaaggtgaacctgaaaggtaatgtgctggataatggaagtcttgctaaaaattcgctctacggtactattaactttaacctgaagaacggtgccctcatcaatttcggcccgcttgcagacattggtaacttcgccttccgcaaacgccgcctcgatagtatcaccatcgataacctgtcaagtaccttccaggtggagggaaataaaatactgattccaccgatgcgcatcgcttccagcgccatcaatattgatgtgaacggggtatacggaataaccggaggtacgaatatcaacctggatattccattgaggaaccccgcaaaagattcggccattaccgataaagcagagaagcgcaaacgcagcaggaaaggaattgtggtgcacctgcatgccgtttcggaaaaggatggcaaagtaaagatcaagctgggcaaaggaaacgatgactagaaagtggcttctgtgaatcatcacaaaagccaccatcactatttctaagccaccgtttggaaggcctgttcaagatctcctttaatatcactgatatgttcaatgcccagcgaaatgcgcagcacgcccggcgctacacccgctttcttttgttcttcctcgcttagctgctgatgagtggtagtagccggatggatgatcagcgttttggaatcgcctacattagcgaggtggtaaattaactttaacgcctgtacgaatttatcagctacttcttttcctcctttgatcttaaagctcaatacaccgccaaagccgttttgcaggtacttcttccccagtgcatggtatttgttgtcgggcaaaccaggatagtttacagattccacctgaggatgcgcttgcagccactgtgccagtgccagtgcattatctaccgttcgctgtacccggagggagagggtttccagcccctgcaggaacaggaaagagttttgtggcgccagtgccggtccccagctgcgcaagccggccacacgtgccctgataatgtaggcaatgttgccaaacgggctgtgggagccgaatacttcccagaatttcatgccatgatacgcctcatcaggctcgctgaactgcacaaacttaccattgccccagttatagttgccaccatcgacaataataccgccaatactggtgccatgcccgccaatccatttggtggctgcttctaccactacattggcgccgtgttccagcggacgggccagataacccgctgcgccaaatgtattatccactaccaacggaatatcgtgcttgcgcgctatggcgctgatcttttcaaaatcaggaatggcaaaccccgggttaccgatggtttccacgtaaagcgcttttgtattggcatcaatcaacgcttcaaaactctccgggttgtcaagatccgcaaaacgcgcctctacgccaatacgcttgaaacttactttaaactggttaaaagtgccgccatacaaataggaagaagttacaaaattatctcccggtaacaggatattatgcagggcaataaactgggctgcctgccccgaagccactgccagcgcgcccacgccgccctccagtgccgccactctcttctcaaatacatccgtggtggggttcataatacgggtgtaaatgttaccaaactgcttcaactgaaacagatccgccgcatgttctgcactctcaaaagtataagacgtggtttggtaaataggcactgcggcagcatgggtagaggattcaggctgataacccgcgtgcacctgtaaagtgtcaaaatgtaatggcttactggacataaccggaaagtttaaaggtttgagtataagtctacaaatatagtagactaattgcaataacaaaatattttaacatgattctcacacaaaaaataatatcttcggcagcataattacaaaatgcatgtttacgtgaagaaacgcagttgaccgatgttattaactattaccaccaaacgttaccccgccacagacctgggctacctgttgcataaacatcctgctaaagtacaaaccgttgaactgaccacagggagtgcacacatcttttacccggaagcaaccgaccatgcctgcaccgccgctttactgctggacattgatcctgtaagactggtacgtggaaacggtaacggccacgactttgcactggaacaatatgtaaacgaccgcccgtacgtggcctcgtcgtttgtgagcgccgccatctctcaagcctttgccaccgccatgaacgggcgttgtaaagataagccacacctggtagatgaagccattccgtttgaaattggcctgtccgtgttaccggtgaaaggcggcgaacctttactccgacaattctttgagccactgggctatgaagtaacggtacaatcgcacctgctggatgaacaatatcccgaatgggggcagagtcgctatttcaatgtaacactccgccacacattgccgctgaaaacaatcctcagacacctgtatatcctggtgccggtttgtgacaacgacaaacattatttcgtgggcggccatgaaattgaaaagctgatggagaaaggagagggctggctggacacacatcctgccaaagaactcattacccgtcgctacctccggaatatcgcaccactcgcaaaacaggcgctggagctgatcatgaaggatgaagtattaccggtagaagaaaaaccggcaaaagataaagtgaaactgcacgatctccgcctgctaacggtaagggatatactcctggaactaaacgtgtccaccgtggcagacatgggctgcggagaaggcaagctgctccgcctcctggtggaaaaaacacagttcaaaaagatcctgggaatggatgtaagctaccggtcactggaaattgcacaggataaactgaaactggaccgcctgcctgaaatgcagcgtaaccgtatacaactcatccagggatcactaacgtacagggataaacgactggaaggttttgatgccggcgtattggtggaagtgatagaacacctggacgaatcccgcctgtcagccctggaaaaagtagtttttgaatatgcacggcctgcccatgtgatcatgaccactgtaaatgcagaatataacatgatgtatgaaaagcttgctgctggctcattccggcacggcgatcaccgttttgaatggacgcgcgcagaatttgaaacatgggccaaccgcgtagccgcacaatttggctatattgtatccttcagaccacttggagaaacagatgaaacactgggaggacccagccagctggcattatttaaacgatcattatgagagacattatattagagaagatagaggaactggaacaacaacaccaggtaaaagtattatatgcctgcgaatccggtagccgcgcatggggctttgaatcgcccgacagcgactacgatgtgcgctatatttacacccggcacagggatagctacctgagtatcacggaaccacgggatgtgattgaattaccggtagatgaagtactggacgtaagcggctgggatatccgcaaaggattacagctgttcctgaaatccaatgctccgctgtacgaatggttacagtcgcccatcatctacaaggaagaaacggactttaagcaaaccctcacaagcctgatggggaagtatttctcgccacgctcaggttgtcatcattacctgtctatggcctttaatgttttctccaacgaattacagggagaagccattaaactgaagaagtacttttatgtattgcgccctatgctggcctgccagtggatccttgccggtaaaggagtgccgccgatggaattggcgccgctgcgtaccttaatcaaagatgatagcatccaggccattatcgacaaactgctggaattaaaagccaccgcagatgagcaagccacggtagcgcctgatgaaacattgcatcagtggatggcatatactttggaagattgcaaaatgcaggctgctgaactgccggctataaaaaacgataccgcggaactggatacgcttttccggaaatatatttcgtatgacttttgaagcactgcaacaacaacgggaatatatcctgctggaatgcatcagcggcagcagggcatataacctccaggtacctacatcagatacagatatcaaaggcgtgttcatattaccgcaacacgaactgtatgggatgacctacacaccgcaggtggccaatcaaagcaacgacgaagtgtattttgaaataaaacgcttcctggaactactggataaaaacaatcccaatatcctggaactgctgagtaccgccaacggcaaccagttgttccggcatccgctgatgaacctcattcagccccgcgacttcctgtcaaagctttgcctggaaacctttgcaggctatgccaaaacacagataaagaaagcccgcggactgaacaaaaagatcaatcagtcgcacggaacagaacggaaaaacatcaccgagttttgttacgtgattgccggcagccggagcattcccttacgggaatggctgcacgaaaatgatcttctgcaaagtgactgcgggctcgcacggatagatcacttccgcgatgtttatgcgttgtaccataccagccagtttgaacccggcgttacctttaaaggtattttctccggtgcagatgcgaacgacgtacaactcagcagcatcccgaaaggaccggatccgttggcgattatgcagtttaacaaagatggctatacggtatattgcaaagactttgcagcctactgggaatgggtggaactccgcaatgaagcccgctatgagcataataaagaactgggggcagactacgacagcaaacacatgatgcataccttccgcctgctcaccatggcagaagaaattgcattatacaaagaagtacgcgtttaccgcaacgaccgcgatttcctgcttcgtatccgcaacggtgaatacacgtatgaggaattgctggatatggctgcccaaaaattaaatgacatggaacagctgtatgctgcctccgatcttccggatcacccggacccggaactggcagcaaagctgttaatcagcataagagacgaattttatgtcccgaagaaatagacaattatcacatatctccctgccggaactttcactggtattattgatcggcccttcaggcgccggcaagtctacctttgcccgccgctttttcaagcccaccgaaattatttcgtcggatgtttgccgcggtttgatcagcgatgatgaaaataaccaggctgttactaccgatgcttttgaagtagtcaggtttatagccgcgaagcgattgaaactggggctgcttaccgtgatcgacgccaccaatgttcagccggaaacccgcaaagaatgggtgcggctggcccgtgagtatcatgtattgccggtagcaatagtgcttaatatggcagagaaagtatgccaggagcgcaaccagctgcggagcgaccgtaacttcggtgcgcatgtgattccgcagcagatcagtcagctccggcgcggtatccgttacctccgggaagaaggtttccggcatatatttgaactgcactcaccggaagaagtggaacagctggaaacagttatccgtaacccgctctacaataataagaaagatgaacacggaccttttgatatcataggagatgtacacggctgctacgatgaactttgcactttgctggatacattgggttacgaagtagataaagaaaactgcagcctgatcagcgcaccgctcactactaacgcagagggatacacgcgtttccgtaaacctgtgtttgtaggcgacctggtagatcgcggcccgaaatccccgcaggtattgcggttggtcatgaacatggtaaacaatggcctcgcgctttgtgtaccgggaaaccacgacgccaaactgctccgctacctgaatggaaaaaatgtgcagctgcggcatggcctcgaagcaacggcggcccaactggctggcgaatcgccggagttcatcgcggcaataaagctgtttttagatggccttgtaagtcattatgtactggacgacggcaaactggtagtagcacacgccggattgaaagaaagcatgcaggggcgcggttccggcgcagtaagggagttttgtttgtatggggaaaccaccggtgaaacagatgaattcggcctgccggtaagatataactgggcgctggaatacaaagggaaggcaatggtggtatatggccacacaccggttcctgaagcgagatttttaaacaataccatcgacatagacacaggttgcgtatttggcactacccttaccgcattgcgctatcccgaaaaaatattggtatcggtaccggcaaaagaacagtatgcagcgccggcccggcctataggctataacacagaaagcgcgctgacactggagcaacaatatgataacgtactggacatagaagattttatcgggaagaaaatactgcaaacaaactatagccatagcattaccatccgggaagagaacaacattgccgcattggaagcaatgagccgctttgccatcaacccgcgttggcttatatacctgccaccgactatgtcgcccgctgaaaccagccgcgaagaaggaatgctggagcaccccgcagagggcctgcagtattatagagaagcaggaatagcaaaagttatttgtgaagagaaacatatgggttcccgcgctgtggtaatagtttgccgcgacgaggccaccgccgtaaaacgtttcggtattgcaggcgaaggtaacggagtagtatatacgagaacaggtcgcagcttcttcagcgataaacaaacagaacaggacttcattgcccgcatcaacacagcgctgatcaacaccggtttttacgaaacctttaacaccgactgggtatgcctggatacagaattgatgccctggagcgcaaaggcgcaggcattgctgcaaaaccagtatgccgccgtaggtactgctgcaggccaggcgttgcccgttgtggtagatgcgttgcagcaagccatttcacagggcgtgccggcacaggcgttgctggaaaaatattcccgccgcctcaagcaaaccagcagctacgtaaaagcataccgccaatattgctggccggtggcgtcattggacgattataagctggcgccgttccatatcatggccacggaaggaaaaacgtatttcgataaagaccatgaatggcatctgtctgccataaaaaatatctgcgccggcgatgaacaattactgctggctactcccttcctggaagtggaaatcgggaatgaagccagtgaaaaagcagcagtcacctggtgggaaaaccttaccgccgccggtggcgaaggcatggtgatcaagccatctgtttttgttgcccgcgatgccaaaggactcattcaacccgccgtaaagatccgcggaaaagaatacctgcgcattatctatggtcctgaatacgatgcgccggaaaacctccaccgtttgcgcagccgcaagctatctggcaaacgttcactggcgctgcgcgaattcgcactgggcctcgaagggctcgaccggtttgtaaataatgcacctttacagtcggtacatcaatgcgtatttggtattttagcgctggagagcgaaccggtcgatccgagactgtaaccatgaaaacatctttctacattaaaaaaacataattatgaaagccgtagccgtatcaaaattcaaagacattcctgaagtgatggacctgccgaaacccgtagtacgaccaggcactgtgctgataaaagtggccgcagcgggaatgaatccgttcgactggaaaatgatcgatggcattatggacgacgggaaaaccaaacaccagtttccgctcatcatgggcgtagacggagccggtaccattgaagaagtgggagagggcgttacccggtttaaagcaggagataaggtatacggacagtttattcattcgcccatcggtgaaggctcctatgctgaatacgccattgtgccggagaaatccgggcttaccaaagcgccatccagcctgtcggccgtggaagcggcagcggtgcctacctccggtatgaccgcccagcaattactggataaactggatctccaggaaggaaatacgctgctgatcaacggcgccaccggcggtgttggctcatttgcagtacaactggccgccgcccagggcttacaggtaattgccaccgtatcggacgatgcgggcgctgaaagaatgaagaaactgggcgccaccatcaccatcaactataaagaagcgccgttaacgcaccaggtaaaggaaaagttcccacagggactcgacggcctgatcgacctggtaagcaacgccgccgcatttgaggcaaacctggatctgctgaaaccaggcagcgcagccctcaccaccatgttcgtagcaaaggaagatgcgctgaaagaccggaacatccgcggaggcaacttcgaaacacaaggcagcgccgcctcacttgataccctgacattagccatcgaccggggtgcactcagcatccccgtagaaaataaaatcaaactggaagacgttccggccgccatagccctgagccgtcaggcgaaaggcaaagggaaaaccgtgatcgttatttgacgacggggaggttgtcttgagcactgattacgctgattatactgattagttggatttttacttttggattttttttgatctcttagattttcttaaataataattaagggagatatgagcggctatattcgcttatatctcccttaatcctttaaaatccaaagtgatcaatccctaaatcagtataatcagcgtaatcagtgctcaagacaacctccgcgatcagatacccgctgttgccttgaacagctccgctccgctgtcagtgctgatctcgtaggtggcgccgtaggcggtaaaagcgcattgccctttttgcagcgccagtgtatcctcacctttaatggtggcgttgcctttcattacaatcagtatttccgcggctttggcggtgtgtttatacacttgtccggcagtgagatcgattttacttacctcaaaatccggcgccggggaaggatatattctctccaggccatcagcgcttacatcgcctttaatgatattgggatgcacgccctcaaaacgggtatgcttcaggagttccggtacgtccacatgtttcggggtaagaccgccgcgcagtacattgtctgaattggccatcagctctacgttctggccttccaggtaagcgtgcgggatgccggcgtcctggaataccgcatcacccggttgcacctgcatgatattaaagaagtaaatagagaagataccacgatccagtttttccctgctgttaggatcgtttaaaaccgcacgggcggcccagaagccaggatcggttttcgacagcttattggctttgtaaggaaggatcaggcggtctgtcagcgggcggagaaggatgttcaccagcgactgcggcatttccattacatttttatacaggccataataaccttctttttcgtatatgcttaccagtgaagtgaattccggaacggttttcagcacttccagcaattgttcatgcggtaagaagccatgaaggagatagaactcactcagggccaccataatttcaggtttatggttatcgtctttgtagttacggttaggggcgctcaatggaatgccttcagcattttctcttgcaaaacctttctccgcttcacttttggtaggatgtacctggatagataacatgtcttttacatccaggatcttaaaaagaaaaggcagctccttaaatcgttcccatactgccggaccggtaatgttggccggatcctggccgatcagttcattcagcggcagttgtccgctggcggtagtaacagtggatggtgcgctgggatgcgcgcccatccagtattctgcactgggctgatttgaaggggctattcccaacagctcaggaatatagttgtgtccgccccatgcgtagtgctgtacttttccttccagtctgaataagttcatatatagtaatctgtttttacttgttaaataccagggaatcgataattttatatgcctgcaaaaataggtgttaagtgtaaataattcccccgcaccgggaagtaaattattcaggcagttgtttgtgataacccaaacccaataacaaatggtcaatcatctgtccctggggcaacagggcgagtcaattgcacaggcttatgttcgccggtattgtgatatcctgcatgtaaactggaaatccggcaggagggaaatcgatatcatcgcccggaaaagtgaacagatttatttcatagaagtaaaaacacgcagcacagatcgtttcggctggcccgaagaagcagtgaacgcccgcaaggaagaacatatccgcagtgtggcaactgattacctgctgcattataacctcaacccgccggccatccggtttgatattattgcgatcacattttccggagaaacgtacgagctggaacacctgaaggacgtgttttaggcaaacgccttttgcgcgaaggttgtcttgagcactgattacgctgattatactgatttagaggattgatcactttggattttaaatgatttggggagatataaggggatattttcgcttatatctccccaaatgattttgaaatcaaaaaatcaaaaaaagcaaaatccagttaatcagtataatcagcgtaatcagtgctcaagacaaaatccgcgttaaccgcttattaacaaaaaaacgcctgtgataattttctcatactatgttattgcctatctttgtaacagcttttagaacctaccccgagttgttatacccccccggtatcccggtagatgacaagcaaacattttctctgaaaagatctggtgcactggtcagcgcgacctatgcaggcagtttatgtacataacaggagagatggataacggcgatacccgtaacaacagaaaggataggagcgtaaaaattaatacacatttgacagcgtttgattaaccgcggctattacgctactaacgcattgatcaccgtaagttgctttcgggagtcagaaagtaaaaaaaagctccgtcttataagacggagcttttatgtttttatgcttaccacaaaccggtgtagttgtgtggtgtgatggctttcagttcttttttgagggcagcgctgatcttcagtccgtccacaaatttatgcatacttttctgcgtgatctgttctccgccgcgggtcagctctttcagggcttcatatggctgcggataattttcacggcgcaatacggtttgaatagcttctgctaccacggcccagttattttccaggtcatctttcagtttagcttcattcaggatcagtttacctaatcctttctggatagatttggtagccagtaaggtgtgaccaaacggaacaccgaggttacgcaatacagtagaatcggtgaggtcgcgctgcaggcgggaaacaggcagcttggcgctcaggtgctcaaacagggcgttagccagtccgaggttaccttctgcgttttcaaaatcaatcgggtttactttatgcggcatcgcggaagaacctacttcatctttcttaatcttctgtttaaagtaatccatggagatataagtccatatatcccggcagaagtccagcaaaatagtgttgatccgtttcagtgcatcaaattgagcggagatgttgtcataatgctcaatttgcgtggtatacttcatacgttgcaggcccagtgtggtgttcacaaacttctccccgaacttttcccagttgatcttcgggaaagccacatgatgcgcgttgaagttgccggtggcgccgccaaactttgcagcgaaaggaatatgtcccagcaggtttacctgtccttcgaggcgttccacgaacaccaggatctctttacccaaaatggtgggcgaggctggctgaccgtgggtacgtgccagcattggcactttcatccaggataagccaagttttttcagctccaggatcatattggccagcgcgggcatgtacacgtgctctatggcatctttccacagcagcggggtagcggtattgtttacatcctgtgaagtaagaccgaaatgcacccactccagtttgtcttccaaacccaggttcttcaattcattctttagaaaatattcaactgcctttacgtcgtggttggtaattttctctgtgtctttgatcagttgtgcgttctcgatggtgaactcctggtaaattttacgcagggcggggaacttggctttcggcagcgtaaacagcttctgctcggagagcgcaataaaatattccacctctaccatcacacggtaacggatcaacgcaaattcagaaaaataattggccagctcgtccagttgtttgcgatagcgcccgtccagcggagaaatggcagttaaaggttgtagttgcataatgtatgtattccagtattactattaacatgtttgaatggctgcaagttctccctaaatcctgatttacaggaccacaattattcatttggaacttgttaaccgggatttaattacttttgcagcttcaaaattactgaaattggaacggaaagtaaaagttgcggctgtaagttatttgaatacgaagcctttattgtatggattcaggaatcatccggtgatggaaatgatggaattatcgatggattatcccgctaaaatagcccagcagctgatagatggagaggtggacgtagcactggtgccggtagccattatccctaaattgaaggaatatcatatcatagcagattattgtatcggagccgaaggacctgtggcatctgtttgtttatacagcgaggtgcccttaaacgaaataaaacgtatttacctcgattaccagagccgtacctccgtagccttactcaaagtactggtacgagaatactggaagcttggtgtggagtttgtagataccaacggggattaccaggacaaaatcaggggaactgacgctggtttggtgatcggcgaccgcgccctggaacaacgcaccgtttcgccatatatatacgacctcgcagaacactgggtgcgctttaccagcctgccatttgtattcgccgcctggatcagtaataaacaactgtccgctgagtttatcaccgcatttaacaacgccaccggcatcggtattcagaacatcccggcagtagtggccgaaaacccttatgcagtctacgatcttaccacttattatattcataatatcagttatccgttaacgcccgcaaagcgacaaggcatgcaaaaattcctcggatacctgctacaggagcgggatacatgatcaagtccacgtcacctccacgttacctccgtatttagcccatggcaaaggcatgtattaagcatgtcctaagcgagtgccaggggagatctaagcgtaggttgtcttactcaggattaacggtgattttattgatttaggggattagatcactttggattttaaaggattttgggagatatgagcggatatatttgcttatatctcccaaaatcataaaagatataatcagttaaatcagcgtaatcctgagaaagacaaaattcgctcacatctccccaaatcctttaaaatccaaagtgatctaatcccctaaatcaataaaatcaccgttaatcctgagtaagacaacctacgcttagttctccccaattttaagtatcttcataattcgcacttaaaattaatctactaatctacgctcatgaaaatcggtatccttggaagcggtcccgttggtttaactcttggtaaagggcttattcaaacaggacatcatgttacaatcggtacccgtaatccctcgagggaatctttgcagcaatggataaagaagcagggtaagcaggctacggcaggcactttcagacaggcagccgaattcggggaactgttgctgatctgcaccagctgggccggcaccaaaaaagccattgaagccgccgggatatggaactttaaatccaaaacagtagtggatgttaccaatccactcgatggcaaaggccccgatgaaaacggacgactcaccttcaccatcggtcacaataactccgcaggggaacaaatacaagcctggctgccgccggatgccaatgtagtcaaggcactcagctgtataggccacgaaaaaatgctgctcccggaactcaaggaaggagcccctaccatgtttattgccggcaataacaacgatgcgaagcgcgaagtcgtcaacctcctgcaccagataggctggctcgatgtggcagatatgggaaggatagaaatgagccgcagcattgaaccgctctctattttatgggcggcctacgggttcctgaatgacagcaccggtcacgccttcaaattactgaaacgataaaataaaaagaggggcctgctatcagcaaacccctctttttattttgcacgcatctttatttcacctgcctggatttaatatagaagtttttatctacttcaaagttcttgaggtcacctaaagtaatattggaactccgccataaagtgcccgggtatatcagcttaaacccgctatcactcagcttcactttcaccggcatattaaagtcttttacatcagacacccagcggtattggatctgctggccattgaagcggtactccagtgtaggaatagtggtatgacgcaggtactggtcaaatactttatccaggttcatacctactgcctggctgatgtattgctctacctcctgcgtggttaccgtttggtgatagaatgttttgttcagcccacgcagcatttggcggaaggcctcgtcgttttccatgatctgccggatattgtgcagcatgttggcgcctttataatacatatcaccgcttccctctgcattaacaccataaggcggaatgatgggcacatcatttaaaatattcttgcggattccctgtacatattcctcagcggccttatgtccgtactggcattcggtaaaaagagtttcggagtagttggtaaaagactcatggatccacatgtctgccaggtctttgctggtgatactgttgccaaaccattcgtggccactttcatggataatgaggaagtcccatttcaatccccagccggtaccggaaagatccctgccggaataccccatgaggtatttgttgccataagccacgccactctggtgctccatacccaggaacggcgcttctatcagcttgtagctgtctttataaaaaggatacttgccaaaccagtattcaaagcatttcagcataggcttcactactttgaaatgttcccttgccttgtcttcattataatccaatacccagaaaccaagatccagtttaccgccttcaccgtgccaggtatctttcatctctatataattacctacgttcactgctacgtcatagttgttgatagggctgcttacataccatacaaaggtccgggtgccatcgggattgtcgatggtcttttttaaacggccattggatacatccgtgaggtcggcaggaacggtaacgctgatggtcatgtcttcgggctcatcactttgtgtgtctttgttgggccaccagatgctggctcccaaaccctggcaggcggtggctatccacggacggcctttgtcgtctgtcgaccatacaacaccgccatcccacggcgctttcaacgccttgcggggtttgccgctgtaatacacggtgatcttttttgatttatcttttacctgtggaattgtcatttttataaaccaggcattgccgtcgcgggtaaaggtgagcggcttcttatcctgcaccacgctgtctatcaccatcggtatctgcagatctatctgcatcactgaatcggttttcagtacctcataggtaatcgtattgaaaccgctgaaggtactgtcgtcctggtttacctgtacatggaggtcgtagctggtaacatcccaccaggcacgctgaggagtaatactgcctctcagcgtgtcagccctgctgaactgttgtgccccggcagttaaagttgccagaagggccatacaaagcatcggtatgccgcgcatatttattcgtatattttagcctgaaagatattaatttactgccaaatgaaaagttgttattgtcaggtggttatatgcagatgggggcttgcaatactatgcagcctcttacttggggcgtgcggtagcccggaaaaacagtcgctgcgcgtattccggtataacagcaccaacggaatagccagcctcgaccctgcttttgccaaaagccaggaagtaatatgggcggtaaagcaattatacaatacgctcgtggaacccgacagcaacctggtgatccgtccctcactcgccaaacagtggcgcgaatcggcggatcaccgcacctatacgtttgatctccggacagacgtatacttccacgacagcgacatcttcccgggaggcaaaggccgccggatgacggccaacgacgtggtgtacagcctgcgtcgtatcatggaccccgccacggcctcgcccggcgcctggatcttcaacggcaaactgtccgccgacagcggtcttcacgccctgaatgactccaccttcgaactaacgctctaccggccgttccacccggtattgggaatactcagcatgcagtattgctccatcgtaccacacgagggcatagagaaatacgggaaagacttccgcaatcatccctgtggtaccgggccgttccgctttttcctctgggatgaaggacaggcgctggtgctgcatcgcaaccccgtttattttgaaaaagatgataccggtcgccgcctcccttacctggatgcagtacaggtaggcttccttgaaagcaaagcttcggaattcctgctgttccgccaggggcaactggactttatgaatgatatcgatgcctcctttaaagatgaagtgctcaccaagcaaggcaagctccggaaggagtgggaggggaaaatggtgctgaacaaacatccttatctgaatacagaatacctcggatttcttactgacagcagcaatccgctcgtcgggaagtcgccgctccgcttgaaaaagatccggcaagctatcaactacggcttcgaccgtacgaaaatgatgacttacctccgcaatggcataggcaccgccgccacagcgggatttgtacccgcgggcctgccttcctttaatgcgcagttggtaaaaggctatccctacaacccggccatgtcgcggcagctgctccgtgaggccggcttcccggatggaaaaggactacctgttatcaaactgctgtctattcccatttacgccgacctcgccaattatgtagcgaatgagctggagaatgttggtatacgtatacaagtggaggtgctgcagaaaagcctgctgctggagcaaaccgctaaatcacaggcattgtttttccgcggcagctggatcgccgactaccccgacgctgaaagctacctggccatgttttacagcaaaaacccggcgccgcccaattatacccgctatcacaacgcggcattcgaccggttgtacgaaacatccttggaggagaacaacgacagcatccggtacatccagtaccgggagatggataatatgatcatggcagacgccgcggtagtgccgctgttctatgacgaagtcgtgcggctggtgcagccaaacgtctccggattcagcggtaacggtatgaatctcttagagttacgttgggtaaagaaaaattaaaatttaaaattattttaacattttcttcaccacctgggaggttaaaactggcttaatatccgcttaattagcttacctttggcgcttatttgtcactttataaagtatagaaatgacggcgatcctgatattcttttgtgtgcattggttcttttccttgttttttcacacattctacttacaccgttatgcatctcaccagatgtatactaccagtaaattctgggaacgattcttttatttcagcacctggtttttccagggttcatcatacctgattccaagagcttatggcgttatgcaccgcatgcaccatgaattcagcgatactgaacatgatccacattctccgcacttcttcaaagacgtatggggcatgatggtacaaacccgcaaaatctataatggttttgtaacacgtaccagtgatgtagatcctaaatttaccaaagacccgttaccagaatgggatgcgatggataaattcggcgacagcaacatcacccgtttcctctggatgggcgcttatgtagcattttacgtagcattcgttcctgcaggtatgtggtatctttatttactgctgcctatccacttcctgatgggacctgtacagggtgctatcgttaactggtgcggacataaatatggttaccagaattttgacaacaacgaccactccagaaatacttctccatggggtatagtactgatgggcgaactgttccagaacaaccaccacaagtttaaagacagtcctaactttgccaaaaaatggtatgagcttgacccaagctaccaggtaatgaagctgctgaacttcgttggcatcatcaagctgaaacccgcaatggtaacagcgcaaatgaagaaagcgaaagctgcctgataatataaacacttcgtacaatcaatctgttacaataatagaaagtgccttgccgtaatggtgaggcattttttatacgcgaagtgcgtaggttgtcttactcaggattacgctgattatattgatttaggggatttgaacactttggattttaaatgatttggggagatataagcggatattttcgcttatatctccccgaatcttttaaaaatataatcagttaaattggtgtaatcagtgagaaagacaaaatccacatatccgcttatatctccccgaatcttttaaaatcaaaaagtgatcaaatcagcgtaatcagtgaaataagtttaatcctgagtaagacaaccttcgctgcaatccccactacctgaatggcttgaacgaaacatgctgcgcaagtgccagcatcggccggtcgccctcactatcgccgtaggcgtatatttcgcggaagttttccaggcggtaggcttcgcggatgcggttcaccttttcttcgccattgcagttgataccttgtattttaccggtgatgactttattttttacttcgagacgcgtagccaggcaaatgatattttctttccggcaccacggcgctacccagtcctgtgcggaagcggatactactaccacatgatgaccctgttgctggtgatttcgtatagccgccagcgcttgcgggcgaattaaagccggcagcttttcccggcagaagctttcacagccagcggaaaaatcgtgggcagacatctccccaaaaaaatattccagcacttgttctttcatctgctgcgccggcatcatttttaatttgaagcgcagcagtggcggcagcaattgaatgatgccggcatacatggcggcgcggcccctgtgatggcggataatttcccatagggtgtcccgggtagtaatggtaccgtcaaagtcgaaaaaagcgatggtcacagggagagttttttgaaaatatcttccggtattaatttgataatgagcataatgtatcgccaatgccactttacatacagcacattctttttgcggttcactgctttgaaaactgcggtagctactgcttccggttgcgccgttagcagtggtgggagcgtcaggtgctgggtcatacgggtgttcacaaagcccggttgcacactcatcacgtgaacgccactacgaaaaagacggttccttaatccgctcaggtaagcggtgaaaccggctttcgcactgccgtagatataattgctctggcgtcctctttcaccggctacagagctgatgcccacaatagttccctgcttcctggccacatagctttccgctacgatgttcaatatagaaacagcgccggtataattgctgttgataatggtggcggcttcctgccagttttgttgcgctttctcctggtcgcccaggtaaccgaaaacgcagatggtgatgtccgggggaacagggaggccgttataaaaagcagcatgcgattggtagccggcagcatcaaacacatgcgtggtggctttaacgccataacgcacctgcagatcctgttgttgaggaatcaatgcggcaatgttcctgccggccagttgaatatcatatttttcagacgcaaacttccgggcaatggcaatggccatgtcggagcctgcgccaagtattaaaagggtaggcatgagtgtacttggttaatcagggtaaactattttgtcaataataaacgctccgattgcagggattcaaaacgcgcgttgttgttatattgttttacaatttcggcaaacctgccggcattaggatagctgttccagaaaatttcctgcttcatccgcgcatccttcgacaggtacaaacgaccgccgtattgcagtacaatttcatccagctcatccaggaattcaaataatcccttgcggatggggaagtccagcgccagggtgtacccctccatcgggaaggaaataaggctgtcttgtttaccgaataccttcagtaccgcgagaaacgaaccccagcctttatcgctgatccgttgcaggatagccaccaggccatctttctgttccagggatactacaaactggtattgtacaaagcctgccttgccgtacccgcggttccagtgaaggatggcgtccagcggataaaagaagggttcataagggattaccttgtgcatcaccttcttataattcttcccgtagtataaccagttaaacgcctttacggtaaaagtgttcagtacaaaggaaggaaggttgaacgggagcgtgagttttcgtttagccggaagggtgaggggggctttctgttgctccgcgctgagttcttccggggtggcatgttcgcctacaatcaggatactccggccaaaagaatcgcctttctggaggcaatcgatccacgccatggagtaagtatagtgcttatattcatcaaacagccggatcacttcttccaggtttttcgccttcagttgtgtttggcgtatataggcagtagccacttttttaaggccgaatttcacccgcgtgattacgccggtaagacccatgccgccacaggtagcccagaaaagatcttcgtgttgggtggcggaacagcaaatggtttcgccattggccgtgagtacatccatatcaataatgtgaccggagaaggcgccgtctacgtggtggttcttcccatgtacatcagaagccactgctccgcctacggtaatatatttagtaccaggggttaccggtaagaaccatcctttgggaacaataatatccagtatctggtccagcgttacgcctgcctgtacatccatgatcccgttggcggtgtcaaaggaaagcatcttatcgtatttcagcatggatatgctgtgccttcccagggaggcatcgccataacagcggccattgccccgcgcaatcatgtggctattagccactacgtatttgcgaagttcatcttcctgggtaaaagcattttcgtcgctgtcaacagcagggaaattcccccagttggctaaccgtttttgcattattcaaaaaaagttttatctgtcggtaaataaattaatacataaaaactcaggacccacaggaggatggttaattgaataaaacggtctttatataggattttggttggagaaccagtactgttctgtacgtaggttatttgcaaatatcgtaataatccgccaattacaaacagggtggtgtaataaagccggtaagtatggaacctggcctgggtttcaggagaaatggtatacatcaggtaggcaacgatgataacagcagaaacaagcgccagcatcacgttcaggaaatccatgttgtaaccccgcaccgccttacgcatgtctttcccggaatcgagtttgatcaggatgtcgtcccgccgtttggcaatggccataaacagcgacaacaggaacaccataatcaccagccactccgacaacgccaccttggcggctacaccgccggatttaacccgcagcacaaatccggttgacacaatgataatatcaaggatagaaatgttctttaagccaaggcaatacaggatgtttagcacaaagtaaatactcagcacaaaaacaaacttttctcccaccataacggccagcgcatacccggcgaaaacgcagatgataaaaagcgctattgcggccgaccggctgatggctcccgacgccagcggacgcatacactttaccggatgcaggcggtcagcctcaatgtcgcggtagtcgttcagtatataaatactgctggcaataaagctgaaggcgaagaaacccaccaggacatcaagcagtttatcagtattaaagatctctcccgcaaagaacaggggaataaacaggaaggcattctttacccagtgtttgggtctcaacagctttaaaaatttcacggaacctggagttgtttggtagttagatggggctaatttacaatttattcaattacttttgcagccattcatattactgaatagtcagcaattacagcgaatcccaatctactatgccaaaattttcactgaacggccgtcgcccggccattgccgaaagcattattattatcgcactcgccctggtgccgttatttgtaacattcccgtaccgcgttaatatttttctatcctgggaaggagcttaccggatatcatccggacaaattcctttcagggatttcggatcgccacttggttacggcttctggatcttcccggccatcttctttaaactattcggacctgaactcatttcccttgtaaaggcgcaggtgctcctgaatatcatggccggctttgctttcaggtccatcatgaaaagcatgggcgtgcaacccggtgtcaggttactgtctgtgctggtatttgtgttgtcctactccttctttaatttctggccctggtataatcatacggtgattgtatttgaactggtgggactgagcttcctgttccggtccttcttttcggatagccgtttacgtagttacctcttgatgttcggtgctgccttctttatcttcctgtccgttttcaccaaacaggacggcggtggaatggcgtttatgttgagcctcctgttcctggcctataatagtttccagacacgccgctggctggacctgcccatctttgccggtatgtttgctttgattgccgccattatgatcctgccgctgatgccgggattcggatactggtttaaccacggacagccgccacacagctcccgactggccttcaacgacttcacagacgaaatattcggcagctccaactggatcaaggcatatgtggtgctggtagtgctgtgccttgtggcgaaagtgaaagcatggggctcctggttacagcagcgccgggaagtactgtttgctttgcttacactgggtatattgggcgaagccgccattttccaggtaacaagctacaccccgccggataacaatatcttcttccacagtttcgcgtttgcctttatcgcttcttatttattggatttagggaagataaatatcaactcgttccgtccgttgttaggggccaccctcctggtgcttttctggtggtctggtacctggtggaaatacataggccgtttcaccgaccgtttatttccggcacaggaaaccgtggcaatgggaacgcccggtcatgagaatgtggtaaaccggcataactttatgctgaataacgataccaccgatgtgccggtgtcgtcctgggttttctcaaatctccgtccgttccgcaaaatatacatgcccgcttccacggtaaagggaatggaaaagattatggcgctgccggtcgtagccgaaaagagaggggatattaaagtactgaacatgtccgagctgactccgctggccgccgcaatgccttataaattggaaaccggtcccgattacccgttatggtatcacctgggagtagggatgttcaacaggcaacttgccaccttcacccaaaaggtaagagaccgtcattacgacctggtaatatatgaatatgctcccaacctgaacaacttttacccctttgcattgaggggagaactgaagcaacattaccaccaggtcgacagtttcctcgcacccagaaggcctactaatgcaattattgaagtatatatcaaataaataatgtaacttataaggtcatccggcaaaaatactgcccgctattaattaccgcatattaaaataccatcattataaagtaaaaagcagcttcagaagaagctgttttttactttataacaaattgataatcattaatatgacactttcgcattaaagcgttgttccaatcagacaaacaccctcattttaccctctttttaattaaccggtaaaataacttttactggttaattataaggtttatcttcgcagtagcatccaaaaaaaaacaaaaaatcagcgtaatcagtttaatcctgggaaagacaaaatccgctcatggcatcctccaaatccattacatcactccggctcgacggtggcgtcctgtgtctcgattttgtgaatacgatcgacaaccgtaagaaaggaatatcgcacgactatctcaacggcatcaaagagttgttgcaatggtacgctcacacccgtgccttatctcccaaaattatccataccctggaacggttggcgaaggattatccgcaaaaggcgaccatggtttttgagaaaagcattgttttaagggagttgctgcaccggttgtttatggcaggtattgccaggaagcaacctgctgcggccgacagtatgcagttcaatacttatatcggggaggcgtacggcaatatagaaatcagttggcaggcaggcgcgggctctttgcagtttaacgcccctgcactggagcaggtatattggtggctggtaaaatcggcagtggaattgtatacctccggcaagccggcggaagtaaaagagtgtcccgcctgcggatggcttttcctggacaaaagccgcaacggctcccgcaaatggtgcagcatgagcacttgcggtgatgtcagtaaagtaacccggaactatcagcgtaccaaaagaaagaaatcatgaacaaaaagacaggcgtattgtcctccaaaatgatcttttgcctgttggcagtatacatcatctggggttccacttacctcgggatgaagatagcgacgaaagtagtgccgccatttctgttgtcgtcgatgcgtttcctggtagcaggagggatcctgctgctggtaggttgcctgcgggagaaaacatggccagggcgcagggagcttgtctctgcctgttttgtaggcgtgctgcttattggtatcgggaacaccacggtagccctggccgtacatcatatgccttccggcattgtggcgctgatagtagctgccatgcccgcctggatcatgggtatggactgggcctttttcagcaaacaacgcccttccgccatgactatgctggggattgtagtagggtttattggcctgttcctgttgtttaacccgtttgttcatcacgaagcacgacagtttcctttatggccggtgattgtaatcgtggcgggcaatattgcctgggcggttggaacgctgctggtacagcggctcccgatgcctacacaaattaccagcaccgctatccagatgctggccggcggcgtattttccctgctgatgagttttgtgctggaacccggcggacttgctaccctgcctctgatgactgcggaagcctggcaggcttatctttacctggtattgatcgggtcactggtggggtatacttcttacagctggttatcgaaaaatgcgccgccgcggctaacggctacttatgcttatattaatcccattgtggccttgttcctgggatgggccattggtaacgaagccattacttcgctggtaggcatttccgctactatcgttatctgcggtgtagtactgatgacactgggccgtaagtcaaaatagggtagtagagatatttctacttccttttccccctgataatgtttatcttgcattttcacacatatacaggtgtagcccttatccgctccggataaaccctgttgatgaaccatagccattgtagcagcattgtatttatttatatatgtaggttccgctcttttgggtgcattttttgttttgttgggtgctattccaattgaatgtaattagataatagattatataaactgactatgcgaaagaccattattgtatcgaacaggctgccagtaaagatttcggaaacagagggggattactcccttcaacccagcgaagggggcctggcaacaggcctgggctccatctaccgcgaaggaaataatatctggataggctggccgggacaggaaatcacagaccagaaggaacaagagaaagtaacaaaaaagttgcgtaagatgaacctgatgccggtatacctgacacaggatgaaatcaacaacttctacgaaggcttttctaatgaaacactgtggccggttttccactatatggctgtttatgcccactatgaacaatcctattgggacgcttattaccaggttaataaaaaattcagggatattattatgaaagtagcagaacccggagacaccatctggattcatgactaccaattgctgctgctgcccggaatgatccgcgcagagatgccggagatctccatcggcttcttccagcacatcccttttccttccttcgaattattccgcctaatcccatggagggccgagatcctggaagggatgctgggcgccgatctgatggggttccatacttttgatgatacccgccacttcctgaatgccgccagccgcatcctgccggtgaccaccaccgccaacgtggtgtcttataacgaccgcgccattgtagtggaaacatttccaatggggatcgattataacaagtatgcagaaatgggcaatgaccccgaagtactgcagcaggtaaaaaacctgaaggaaaactttcacaacgaccggctcgtgctttccatcgaccggctggactacagcaaaggaatcctgcaacggctccaggcttttgaactgctgctgcagctccatcctgaatatatcggcaaggtggtgttgtatatgattgtggtgccttcccgcgaccaggtgccccagtacaaagaactgcgcgatgaaatagataaacaggtaggaaatattaatgcccgtttccgtacgctggcctggcatcctatccaatacttctaccgttcatttccgctggaaacactatctgccctctataattttgcagacatctgtctcgtaacacctatgcgtgatgggatgaacctcgtcagcaaggaatatgtagccagccgtaataacgacgatggtgtattgattctgagcgaaatggcgggggcatctaaagaattaatagatgcgatcatcgtcaatccaaataacattggcgctatcacccgcgctatcgtagacgcgctgaacatgccactcgcggaacagcaacgccgcatgaaacaaatgcgcaccgtggttgccaagttcaatatcagccactgggtaaaactattcatgacccgcctgcaggaagtaaatgagatgcagcagaatatgctggcccgccgcgtaaaccaggaaacagcggtactcatccggcaacaatatttcaacagtaaaaaacggatcatcttcctcgactacgacggcacattggtgggcttccagcccaatatcgacatggcatctcctgatcctgatctgtaccagctactgcgggaactggcagccatacctggcaacgacctggtaatgatcagcggcaggaaccacgatacactgggagagtggttcggtcatctcaacctcgatctcattgcagaacatggcgcctggcaaaaaacgaaagcaggggagtggtaccagctgcccggtctcaccgacaaatggaaaaaggaactgctgcctatcatggaactggctaccgaccgtacacccggttccttcatcgaggaaaaaagtttctccctggtatggcattaccgcaaagtggaatccggcctcggagaattacgcgccaatgaactgatgaataccctgcgctactttacagtggagaaaggattgcaggtattgcccggcgacaaagtaatagaggtaaagaatatcgaaataaataaaggtaaagccgccctgagctggctgaatcataaaaaatacgacttcattatggccatgggcgatgatgtaacagatgaagacatctttaaagcgcttccgaataaagccatcacggtgaaagtaggcagccaggtatctgctgcacagtattacttgcgaagttatcatgaagtacggcatttgctgagaacattacgcaacagggaaagcgtgtaaataataaaaggaggggagcacaaactcccctcctttatttttatgtaaaatcaaactatagaaaaatgggggtatccagtttcatggcaatccggtaggcggcattcatcaatcccacatgactgtaagcctgcgggaaattcccccactggctgccggtggcagattccacatcttcactgaaaagcaacaggtgattagaatattgcagtagcttggcaaattcccgctgcgcatcttccagccggccaacgcaggcaagtgcttccacataccagaacgcacatacgaggaaagtggttttgggtttaccaaaatcatcggagtgacggtaacggtaaaacaatccttccggtgttttcaattccttttccaatgcgatgagatgatcgcgtgcccgttcagaggcaggatccaggtaattcatcatgatcagctgaagggtgctggcgtccaggtgctggcttccagcggcgttggtgtatacttttcttaccgggtcgtaacagctttcaatatgggctgcagcgcggtttttcagttcaatggccttatccagcagggattgattgccaatggtgcgggccattttttcagcagctgcgcagccggcccactggaacaggttcgtgtagcagtgaacgttagccatgttcctgaactcccagatacctgcatctttctcatcaatcgttttttctatcttcttcagcagcagttcaatccaccggtcagaatcctttctttctgaaaaaataaaacggtggtcagtatataatggaagcatggaaataagcacctgtccatatatatcgttctggatgtgctcaaaagcctggttgccgatgcgcaccggtttatttcccatgtagccatcaaggtgtggcaggatggtttccgacagggttttttgtcccgtaattccatacagtggctgataccggaaatcaccggagaaagagatatcggtgatgtaaccgaagtatctttccatttcttcaaaatgaccaatgtggttcaaggcagtgataatataataggtatcgcgcatccagcaatagcgatagtcccaattacgcccgctttcaggaaactcgggtaagctggtggtgctggctgcgatgatggcgccggtatcttcatactggtgtattttcagcgctaaagcagagcggatcacataaggctggaagtaattggcaatggaagaatgcttgatccatgttctccagtaggaaatagtttcccggagaaaccgttccgcggtactggccagtggcgcttcgagcggatggccataagtgagaatcaggtaccgcgtatcattgagtacaaaaaactcatcgtcgataaggtagctgacagcaatattggtagtgagacggatgttttcttcgcagcctgtaaattcaatatgactgctgcctctcatagggcgcaacttcgatgcgccatagtcgcaggtaggctcacaggttacccggatccggggcgagccttccagcggttccactttccggatcagcatgagcggcttaaaaaaacgttcatactgaaggaagcggggcgcaaagtcggtaacgcggtagctaccttctgtagtggtaatttcagtacacagcacattggtgttttccaggtaatactgatgggaagaaaaatctgcctccggtaaaatagagaagcagccacctttcttcgtatcgagcagtccgccgaaaacaaaggagctgtccatgcggggccagcaaagccaatcgatgtttgtatccttatttacgtgcgccagaaatgcacagttgccaataagtcctgtctgataggtgtgtctttccatatgggccttacgtttggtttgaattacatttttctcccggaattgttcacccccctggaacaaaagctgttccaataatatatccgggacaattattaacaaaacatattcctgttgtattcttggtggaaacccttatttttaagtataaagttccacaaagatgcaaacattgaaaaagcagcaataccttcctcattttatagagccggtaagcagtggcgataccaaaacctatctgctggcgggcgacctgggaggcaccaaaactaacctggccttgttcagcagcgtgaatggagaactggagctgatccggcaggaaaaatatgcttcgcgtgattatcagaatttttcagagataattaagcactttctcagtggatgcagtgataccccgccgcagcgtatatgcataggcgtagccgggcctgtggtgaagggaaaagtggaactgaccaacctgagccgggagctgagtgaagaagagatccggcagagcacgggtgtgcatactgtggccctgatcaatgacctggaggctaccgcttacgggttagccacgctggcgccgcagcagcttaccaccctgcacaggggcgcatcggagcataatgggaacatggccattatagcaccgggaacggggcttggtatggcaggattgtattgggatggtcaatatcatcacccgtttcccacagaaggcggccacaccgattttgcacccagaacagacctcgatattttattgctcaggtatctccaggaaaaatatgacgtggtgagttgggaacgccttatcagcggcccgggtataacagatatctatgagttcctgcgggatataaaaggcatggaagaacccgccgaactgcgtgcggcaatggacgccggagacgctgcggctgagatcagcaaggccgctgcagcgggacggattcccgtttgtattaaaacgatggagctgtttgtccgctacctcgccagggaatcatgcaacctggtgttgaaaatgaaggccacaggcggcttgttcctgggcgggggaattcctccaaagatagcggcgctactggaaacaggtgagttttatcatcattatatgcagggcgaccgcatggctgaattgctggccagtgtaccgattcatattgtgaataacgataaatccgccttgtggggcgcggcattttatgccggattattaaaagaataaacttatttttgagagacagataacaggaaatggtgtcttcctgacccaaaccgtcagcccagggctgtctgatggcgcctacaaatattataatggtagcaaagctgccatataacgctgctatttgtaggatatgaaacaaacgaaatctttgctggaacaattgtccgtggctaaccaactgctgcgctggaccgtattggtaacacctgttgccattatagttggatctttagtagccttgtttctctggctgctggatgtagtcaccgatctccgtatggagcatgagtggctgatttttggtcttccgctggcgggtatactgatccactggctctatcgtatcggtggaaatgacgctgagaaaggcaacaacctgatcatggaagagatccaccaacctggtggcggtgtgcctgcacgtatggcgccgctggtattggtcaccacgattatcactcacttattcggtggctctgccgggcgggaaggaacagcggtgcagatcggcggcagtatggccggcctgataggtaaaaaactggggctatcggcgccggatatacgaattttactgatggccgggattgcggctggatttggagcggtgtttggcacgccacttacgggcgccgtgtttgcgctggaagtactggccattggcgtaatgcgttacgaggcattgataccctgcctgattgctgccgttttcgcggatatcgtatgctcctcatggggtattcaacatacccattactatatattttataaggccaatcctttcatgaactggctcccttttgttcaccaggatctgtggttgctggcgaaagtgatcgcaagtggtgtgtgttttggtttgagcagccttttattctccaaactcattcataacatcaggcataacgccaaggcctatattaaaataccctggatgattcctgtggccggcggcgtagtaatcatattactgagttacgtggccggaactaccgactatttgggattaggcgttcacggaaaatctatcagtatactggctgcatttgatcccggcagtggagttaacgactggagttggctctggaagctggttttcacggccattaccctgggaatgggtttcaaagggggagaggtgacccccctgttttttataggcgctaccctgggccatacgctggcgctcctgttcaacgcaccggttgacctgtttgcgggcctgggctttattgctgttttcgcaggcgccaccaatacacccattgcctgtaccttaatgggcgcagaattatttggcaccgaccacattttatactttgccgtggcttgttttacggcctattatttcagtgggcacacgggtatttatggcgcccagcgactggaagtaaaaaagttgcgctaacaattttgttagtaccatcttcttacgtcagcagcttttaaatttgccggatgacgaacatcacaggcatgcaccatgttgccattcaagcgaaagactacaaggctactattaaattttatgagtcgctcggacttagtttgtttcacagctggaccttgccggagttcaatattgaatacggcgcgctgctgctcattcccggaacatcttcctttgtagaaatatttgacaaaggagcgaatatcccaactcagggtcgtcgcggcgtcaacggagaatcaccggtagccggcgccttactccatttcgcatttaccgtgaaaaacgccacagcagcttaccacggagccatcgctgccggagccacgagctgtgtgccgccgtctgtgcttgttttgggcgagccacctatgacggtgtataattctctcgtgtatggattggatggtgaagtaattgagtttattgaaacacttcctggctgatactgttatgctttagatacatagatctgtacctgttttggcgtagctatttccgtttattttgcggggtataaaatgaaaagcatgcgtagatttccacgcaggaatatcccaatagctgctgcagcattggctttaacaggtaccttatttattatcttcaaaagtattgacatggaaaaagaaacaaaaatgccggcgttcattaatcctcccgggctatacgatccggctcccaatgcgtattcacatatcgcggcagtgccggcgggaaatactttggtttttattgccggtcagggcggcgaaaccgctgatggcagcctcgtaaatgattttcgaacacaattgaagcagaccttcagcaacctggatacagcgcttaaatcgcaaggcttgaagttcagtgatgttgtgaagctaaccacgctgattgtggatcacaatgaagagaaactcaaaatcctcacagaagaatccctgcgtatctggcccgacaaaaaattccccgtaaatacgctgattccggttccgcggcttgcactggatggtatgttggtggagatagatgcgactgcggtaaaaagataattccgtagccataacgtctagttgcttcagaatagaaaccgtttgaatgggagtgaactgatcactcgtttattcaaacggttttttgtgcgtgacagtaccggctgtaattgcgaaatcccatcagatatgcagacatgattcttatatgcgattctcagcgccttcatttttagtgaattagcccttaaaatctgcctaataaccaggttgactagaatcttttttttatacttcagcgtattcaaatataacctataatttatattatgttaaatagaataaactgacttaaagaactaataattaatcatcttctctatcctatcgattttgcggccttccttatattcgctgacctatcaacttaatctgatccaaatggataaggcaaacttaagcccgcaagtttgccgattgcttaaagttgccttatccgttgcgcctatcctggataatgaacacctgtagcctcttctgcaaaactccaaagccggttcgccaccatctcatccaagccattcggcgaaatttcagcacgcgctggaaatccccggtatccgccgtcccggtcgggaccatataattcccctcctgttacttcatctgaaaccgcggcatatagcgacggcagagcgccttgccatggttccatcagttcaccaacacgttcttttgcagctgaaaactcagttgcactcatatgacgcgccaactccgttttattcgctcccggttgtaccgctattgaaaccaccttatcgccaacagcgctaattctccgttgcaattctaccgcgaacaatatatctgctaacttgctttgtgaatattctctcaccggatcgtaggaaatctcagatttcagattatcaaaatcgatcactcctctcagatacgccatactgctcacggtaataatacgtgcgcctggcgttgctttgagcaacggatacagatggcctgttaatgcaaaatgtccgatgaagttaacaccaaactgtaactcaaacccctcagctgttttggaggccggcggaatcattacgcccgcgttattaataagcacgtgaagctgcgtgtgatgcttcagaaattcctctgaaaactgtttcaccgctgtgaggttggccagatccagcaaagctgtttccaatgaaccagttcccttatgttcctttatgagtctaagggcacgcgttgcattctcaatacttctacaggccaaaatcacgtgcgctcccgccatgtataaggccaacgctgtttcaaacccgattccggcatttgcacctgttacgatcaccgtcttaccggcttgatctgtcatattatcttttgctgtccacataactttgtttatttgataccacaaagttcctcaaacagcatatgccgatgataccagaatgaaagcaaaaactatgaaaatcaatcagcctcagattgcctgaacttattgggggtgattccggcaagacttttaaagaaagtagaaaaatgattaggctcttcaaatcccaggctccaggcgatttcgttcactgtccagttggtactttttagtaagaccttcgcttcctgcaatatccgctccctgatcagacgggacgtggtttttcccgtgatttctttcaaagctttattaagatggttaacatgaacatttaactgtttggcaaaagccgacggcgtacttaactgaatcacctggttacttaattcaatgggaaactgacgttccagtaactcggcaaacaatcctgtgatcctttccgacgcgttggaacccacgaccgggcctccggttgccggctgcatcttttgcgcctcatgaattacttccatcacaaggcttcgcagcatatcatatttaaaagcataatccccctgcagctcgttaaacatcttcagaaaaagttcactaaaccgggatatactgccagctgataaaggtattacagcgccgtcggcagactgaaataccgggtaatccctgatatttccaaaccggttaaaaaacgcctctgtgaagatgcaaacgtaaccgctttgtttttcgctgatcctctcccaatgatatggaatcatcggattcgtaaataccaatacgctatccagcacttcgatactttgatctgcataatgaattttactatgccctgtaaccagactgattttgaagaagtttcgacggctgtaggtaaccggcttatagtccggtaactgcatatcctcaatcctgaaaatattgaagtggcctgactcctgcagcgcagttgcaatatcccggttaaggatcttataaaaggactgtagttcaacgaatctcatgatagatcaaaggtacaaaaatcaaacaaggctgattccagcattcacccactcatccgaatgtgcttgattttctgcggcaattgcacaatctttaagtgcaatcaagatccaatccatgaatgtaataacaaaacaactatggctgccgctattgctggcaggtactattggcctgcagctacaggcacagcagaagaacaataaagtcaatgcgaccgccaaagaggaaacgccgccgcaatggtccgtcgtcctgaacccggatacggccgttaccacctttcacgatgtaaccgtaaaaggtcagaagatcccttacaaagccatcgcgggcaccctaccagtatgggaccaggatggcaaagtactggcgggtctcttctatacttattatgaaaggactgatgtaaaggaccgcgcagcaagaccgctggtcatttcttttaatggtggtcccggcacgccttctgtatggatgcagattgcctataccggcccaagactactcaatatcgatgacgaaggatatcccgtacaaccctatggcatacacgaaaatccggaaactatcctggatatcgccgatatcatttacatagatcccgccaacaccggcttttccaggcttataggaaaagatgtgccccgtgaaaaattcttcggggtgaatgcagacatccgctacctggcagaatggatcaacactttcgtgtcccggcaaaacaggtgggcctcccccaaatacctgattggggaaagctatggtactacccgtgtttccggcctggcgctggaattgcagaatgcgcagtggatgtatctcaatggtgtgatcctggtatcccccaccgatttgggcatttcccgcaacggccctgtagatgcggcattgcggctcccttactttgcagccaccgcatggtatcataaaatgctgccgccggacctgcaacagaaagatctcaccgccgtgttaccggaagtagaaaacttcaccatccatgaattaataccggccatcagccagggtggattcctggaagaacaacaaagaaaaagcatcgcctcaaaaatggcccgttactccggtttaccggaaaaagtgatcctgcaacataacctcgacgtaccaccgaatttcttctggaaagaattactgcgtgataaagggtttaccgtaggcagactggattcccgctaccgtggcctcgaccgggaagatgcaggcaacggtccggattacaatgcagaacttacttcctggctgcatgcgtttacgccagccattaatatttatctcaggcaagagctgaaattcaatactgatctcaaatacatgatgtttggtcccgtgcatccgtgggataagaacggcgacaacaccggcgaaaacctccgtgaggccatggccgccaacccctacctgcatgtaatgatccaatcaggctactacgacggcgcctgcgattacttcaatgccaaatacagtatgtggcaaatggatcccggcggccggttgaaagaccgcctctcctggcgcggctaccgcagtggccacatgatgtacctccggaaggatgatctggcaacagggaataacgatatccgtgatttcatccgtgcgtcccttcccaaagccgggcaggcggcgaagtactagtgcgcggatgaccgccttcggcggtgcgaaggttgtcttgagcactgattacgctgattatactgatttagggattgatcactttggattttaaaggattaagggagatataagcggatatattcgcttatatctcccttaattattgtttaagaaaatctaagaaatcaaagaaaatccaaaagtaaaaatccaactaatcagtataatcagcgtaatcagtgctcaagacaaccttcgcaccgccgaaggcggtcgcggttttatattttatacgttacgcctaaggtcatgtagatgttgtacaaggggaaatccattcctttaaaatcgtctgggaatatcgggcgcaatccccagttgaggttgccgttgatgctgagttttttacctacgcgataggcagcgccgccttgtaaccccgcatcaaatgaacggacttctgtgccaaaatcgaaggtggcttctgtgatgtttactttctctcctaaggatccgccgttgcggatatatccgtccgaaacattaccgtggaagttggcgctgaacaaccaggccatgtaaccgcccatgttaaaacgccaacggtcattgggagtatatactacgctgatgggaaagaacacatatgcattacgtaccgtggtttcgtttttgccagtaaagtctccttcaaaacggccaccatcactggtggtaatgatagtaggaaaatactgcacttcatctttggtaaacattcctttatagtccagtttcacggctatggcagcgccccatttttttgttttgcggtacgacagctcataacccagcgaaggagagaattcaggccggtaggtttcgattttacggatggtgttgggtaagcctacgggcgccgtgcccccaaagttaacccccgccaggatgcgatgttcaagtaccggtttaaagtggtgcatattcgtttgcccgtgtccgttatcctgcgccaataacggcgaggcagtggcgagcatgcctgatatcagtactggtattcttatatttatcatcatgggtaatcttttgtttatactgcccggttattttatcacttccaggctatcgagtaccagcctgctaccgatagcacctttataggtatcgccatctttgctggaagacgctacaattgccatcatcattttctccgttcctgtatatggctgtacggttttaaacgggatatcaaatcgtgtccatgtgctgtgaggaccgccatccggtatactggcggtggctactatcctgtctgatgtgtggatgttggtggcgtccagcctggtggttcctttgaacagcaccgcgtataaagaacaactgtctttcatgcccgcaataatattcccggccttatcctggtattgttctcccggctgatatttataataacccacgaaacgcagtggcttacctgaatagggctccccgaattgtgtagccgttaacggcgcagtcatggcatttctcgaatcaaatacacctacaaaaagagaccctgcaaatagcttaatgcctaacaaggcggacaaagccgtgcctttgcgggtcaccaattcagcggcagactttccgtggtatgcgtcggaagtggcacgcagcggatattccatcgggtccttctttacgccggataaggctatgcctgggttaccggatgaccagaacgtactactcccatgttcttctacatactggtatttatctttatcctgcagcagccaggtttcgaagtcccatttccatatgcccatcccaccaaattcaatcttgtagatcttcttatttccgttagcggcagtaacaacatactcgcttacctgtgaagaatccaggtgcagtgagtcgccagatgccggcaataccgtagctcccgctgaagtggtaatcgtgggggttacaccgctcttaaacgcagcaggtgtaaggttcagcatgatctttttgtttgcctgatcaataaaaatatctgcagtgagatatttcttttctatgataaatgtttcaatatctgcctccgggttaatgggtgcgtctttaatgcaggcgtgtaacaaaatagtcagcgtggccagataacatagtttccttattttcatgccgttatttggttaaatcactagaacaacttccaactgccaaaagttcaatcatgattgacaaaataagaatcaggcgaacattcatctacgcagccaaatgcgtcaccggcgtgctggtggtgcttggtttgtcgtggttagtcaattacaacgacatcatctgggtgctgatttctgtgatgctggtactgtctcctgacggatcagacgccgtaacgttagcggttacacgcattaaggcaaatgtggtgggtggtatatcgggattcctgttgatattagtgcatccgaatatattgatgatgatgtgtgctgccgtatttgttacggtagtaatctgcaacctgttaaatcttgaagcagctacccgtacggcgctggcggccactattattgtgatgacccatgaggcaggtgaacatgtatgggatactgccgtggcaagagtattgtctgtattggccggttgcctgcttgggctgctgattactttcatcttccataaccgttataccaaacaaaccgctgaaatgatccttcccaaacccgaccggggcggggaataagatgatacagaattacttcagaatcggctcctatttttgatgtaacaaggagtgacgcatgaagaaaatgatattatcgacaggtttggcgttgggcgccctcacctgctcttatggtgctaatgcacaggaaacagattccctgcctgccggaaatgattccatccgttttacctatcctgtacaaaagagccagctgcctgcctggcaaacaaaacaatttcataccactattgcgggtgttgctgttccggtggcaatgatcagctacggggtgtttgcgcttaataatccaacgctgagggacctgaactccactaccaaagcggaaatcaaagaagatcaccctcaattccgcacacatattgacaactacctgcagtatgctcccgttgctgcagtctatatcctgaatgccgccggcatccagggaaaacacaacctgcgcgaccgctccatcatcctgggaatatctgccgtaattaccgctggtaccgtggaaattgtaaaaaatcgtacccatgaagagcggccggatcactccgactatctttctttcccctcgggccatacagctacagctttcgctgctgcagaatttctccggcaggaatacaaagacgtatccccctggtatggcgtggcgggctatttagctgccaccaccaccggcgctttgaggatgtataataataaacactggctcagtgatgtggtggccggcgcgggtataggcatactgggcaccaaaactgcatattggatgtatccctggattcagcggcagctctttaaagatccggcgcacccggcgactaaaatgatcatgccttactataacccgcaatttcacagtgccggtcttagctttatcttcttcccccgctaagtaacatgataagtaaatagtaagtcataacgcctatagggcgctatgacgctgcatccgtcccggatgtaaaaaatacatatattaaaatattaattggagtgttaactaaagaatacatgggggttaacccctaaagctgacctggttacaaacacctgttttttggcaatacggtaaagttgcaggtttatcctgagaaattttgtgatttaattgttaacgtgcaaaaaaaatgttcatttttgcagaagtacctgtggaaacccatcgatctgtgtaaaaatatcatgctttcattaacatagaatttacatttacctgtgcaagaccgcttattttagcattatcaatatgataaaataaaaaccctgtgacctccaagcgactcaaaataagactgatgccctgtttaataatcccctcctcaaaagctgttaattatgtacgttccggtaatcattttcttttttttcctgttgtggtacattcatttccgtacccaaagcttccgcggcgcggccttcaaggaaaagaggccaaagcctgtcgcaggtgaagatgccatccatgccgtcaggatagtaggcgtttccaatagtgtattcagcgtatccaaatacctccgcagcgtgaagaacctgtcggacagccggtttatgactgtggcaattgaccaggtgatcactaccactatgggtaccacgcaccaggcccgcctcattgaaaatcttgctcccggagaggaacggcggctgggacatacggatcatgtcagggatggtaagcaccagatttacatcggatatgaaatactgtgggcacggtacacccctgcccctgtgtggcacaaagaaaaaaatactgataccacatctcccgcaaaattatataatgaaatgctcaggcagcaccaggactcgctgatacaggaaatggaagacaaaaaagatttattgtcctgacagttgtgctgttttgcccctgaagatgcttaaccataccatagaaaagaaaacgccaagcgtagcgccggcggtcacatcttccaggaaatgctggctcatatacatccgggaatatcccaccagcatggccagcgccaggtataacagcgaccagtacttattctttgcataataggaaagcacggtggcagcagtgaatgcacatacgctgtgccctgaaggaaagcttctgaaattatcaagtaccgatacgcctggtacaaaataaatttcctgtaaacggctggcaaaataacggtgagggcggggaaagccaatcaatgctttcagtgtaaaactgatagcggcggtaaacaggtacgcggtagccagcataacgcctgcccgcctgttaatgaccagcagcaataatgaaatgagaaccgctgcggcaacgcttcccagctctgttatccggggaaataggaagtcgcccgccggcgtatgcagtttattaatgaaaaaataagcatcctggcgacttactaccagccgcattaccagcacagtaacgactaacaagacaaatggccataccagccatttcagttgctggtatactttaatgaaattattcaggaaggcattcatgggatcacgactgggttaatcggcggtgataatttatttgtccgagatgataattaagatgtgtactcagatgtacgaggaaatgcccggtagacatcgttcctgaaaaaaccttttccggatatgttttttcaagttcttctgctgttaaacctgctataacggtaaggattacacgacgcgtggaactgatcagcaccagcagatcttccgtgggtacgttcctgtcgctgaactccaggtccctgttgcggacatagtccgtcttacccaataccgcgcctatataatgctgcaggttaccgcagagatgcagacaaagattcccggcgggatttgttataccgggaggaacctgccagatgccggcagctgtttcatatgcggcaatctcctcctcgagtttgctgagatcccgctcaaataaatttattaaaattccggttagcatatgttaaagataggaaaagccgctaatcatcttttgatattattataaaagttttcactaaacataaactaacctgcttttgttttaagtacataactcaacaggatgactaacgatagcaggcgcgaacttactcccttccaggagaaatggcataacattatttttgaggcgagcacaccggccggccgggcgttcgatattatcctccttgttgctattctgatcagtgttgttattgtaatgatggaaagcgtggcgcctttgcaggagaaattcggacacctgtttcatatattggaatgggtattcactattattttcacgctggaatatctcttccgggtttggtgcagttaccgtccgaaggcatatattacgagcttctacgggcttgttgacctgctctgcatcctgcctacctatgtggaagctttttatggtggtgcgcacttcctgctcaccatccggatactacggctcatgcggatcttcaggatatttaaactggtccccttcctgaacgaaagcaaacaactgtcgctggcgctacaacaaagccagcgtaaaatatttgttttccttttttttattggattgttgaccgttgtattaggcgctattatgtatgtgatagagtctgaccataattcagggttcaccagcataccggtaagtgtgtactgggcggtggttacgctcaccacggtgggttacggggacattgcgcctgtaacgccaatggggcaagcgttttcagcgctcatcatgataatgggttatgcaattatagcggtacctacagggatagtgacggtggagatgagcaggatacgcagtcgcgatgatgtagatcgcagagtttgtccgcattgcatgcgtgaagaacacgatgccaatgcggacttctgcaaatactgcggtaataaactctgaattattttacactgaataaaggctgtacgtctatcattgctttctggtaagcagcatcaaaaagttcccatttaccggaaatgccgatgcgtatattgcggccatctatcagatcgaactcggcaactcttttgttaaagccctgtttacctcttctgaaatctgttatatcagataacggaaattccagggtaatttttttacgggaaagcaaccaaccaatgacaccaaataacaaaatcatcaccattggtttggcttcaagaacaattctctcgtttgtaatatacagtgtaccttgttttgcattgaacctggtcttcatgtacactgcatcaattttgaataatatggtttcctgtgggttaaggggccatttaactttaatctgcttcatggtaagtgagaatatgattaaatgcaaaaatataattttattgtgaatctaaacgccaaatatgatccttacttcgcttcttgataacgatttctataaatttaccatgcagcatggcgttgtcaaattattcccgaaggcccgtgcccgttatacgttcattaaccggggacagcatgcctttccgccaggctttgccgaagccctccgtgaagcggtgaataacatgcagctgctgcagcttacccctgaggaaaaggattacctggctgttacctgtccttacctcgaccctacctaccttgatttcctgcagggctaccgctatgatccggccgaaattcatattgcacaacagggcgaacacctggaagtacatgccgatggctactggtaccgcactatcctttgggaagtgccgctgatgtcgctcatctgcgaactctattaccagctgaccggccagcagcgggtagctgatgaagaagtgatccgcattacccgcgaaaaaattgaaaaatataaagagatggatatcaccatcgcggattttggcacccggcgccggcattccctcgccgttcataagctggtggtgaaaacgctgggtgaatatggaacaggttgttttattggcaccagcaatgtacacctggccatgcgcaacggggtaaagcctgtaggcacccacgcccatgaatggtttatgtttcatgcggccaaatacggctttaaaatggccaacatgcttggattggagaactgggtacaggtataccgcggggatctgggaattgcgctttcagatacctacaccactcctgttttttttgagcagttcgacaagaaattcgcccggctgtttgatggggtgcggcacgacagcggcgatccactcttgtttgcagaccgcactattgcgcattataaaggtaaaaacgtggatccgctcagcaaaaccatcattttctcagatggcctcaattatgagaaagtagcggatatcgccgcttactgccggggaaagatcgggatgtcgtttggcattggtaccaattttaccaacgacgtagggttaacggccctgaatattgtaataaaaatgtatgaagccctgcccgaagatgctacccggtggtcgcctgtagtgaagttgtctgatataaacgggaaatataccggtgatccaaggatgatcgaactggcaaaggaaatgctgaatatttaacgatgcaccatttccggatttgtattactcctggtacaggtatacaaatccggaaacccctcgcctaccagttacccaggccgatgcccgtgtcaccgtcggccacattcccggattcaaagcctttcttaaaccagaacatcctttgttcggacgttccgtgcgtaaaggcatccggcactacctggccagtgctggcctgctgcaggcggtcgtcgcctaccgcgctggcggcattcaacccggattctacatctcccggatccaggaaaggtttgattttattggcacggttagcccatacgcccgcaaggaaatctgcctgcagctccagcatcaccgataatttattgtattctttttcgcttagccgggaacgcatggattgtaatttatcgctgatgcccaaaaggttctgtacgtgatgccctacttcatgtgcaatcacataagcctttgagaaatcgccctttacgccaaattgttgctccagttcattaaagaaagaaacgtccaggtatactttacggtcggccgggcaataaaatgggcccatagctgattccgcaaagccgcagccggaattggtacctttttcaaaagacaccataccgggtacttcataggttttgttgcgctcctggaatccctgcttccataccctttcggtactgcggagaactttagaagacatgacctcaaaaggacttgcattttccttcgtaagtttttcagatgttcccgcctgctcctggcctggggctacctgttgaacagcctgcattacctgctgcgggtcctgtttaaagatcaatgccagcactataatgacaagggtgccaatgccgccgccaaccccgatcttgcgcatgccgccaccggaccgtttctcgacgttttcgctcatttcttcatcatcaagacgcatagtagattttaaatttaaggggtgaaaattcttacccgaatgtacatttttcattgataattccactcttttctccccgggtaaacaaaagcattttttacctgttaaataatcattgccattcctcacttctataaacacccgcgcatatgaaaataaagcagatcctgctcgccgccagaccaaaaggattacctgtagccggcaactttgaaatagtagatgccatcttaccggaactacaggaagatgaagtaatggtaaaaccactgtacttttctgtagatccgtatatgcgtggccgtatgaacgacgccaggtcctatattcccccattccaggtaggcgaacccattgaaagcggcggcgtggcggaagtaacacacagcaaaagcgccctgtttaaagccggtgataaagtaatgagcagcggcccccgccccttcctgccctgggcaacggcggctatattccccgcagggcacctgcgtaaaattgacgacagcatcccgcttacttattatctcggtctccttggcgtgccggggttaaccgcctactttggcatgacagatatcggcaagcccaaacccggggaaaccgtggtggtgtccggcgccgctggtgctgtgggcatcattgtagggcaaattgcaaaaataatgggctgccgcgcggtaggtattgcaggcggcgctgaaaaggtaaaactgctgacagatacctttaatttcgatgccgccatcgattacaaaggtaacaccaacatagaagccgcagtggcggcggcctgccccaacggcgtggatatctatttcgacaacgtaggtggcgatatttccgatgcggtgatcaaacagctcaacttctttgcccgggtgccgctatgcgggcagattgccttatataattccacagaagtgcctatgggcccacgtatccagcctattatggtaacccggagcattctcatgcagggcttcattatcggtaactacgccagcaggtttggcgaaggtttcaaacagctgtccgaatgggtgaaggcaggaaaaataaaatataccgaaaccgtggaagaaggatttgatcatctgccggcagcattactcggattattttcaggaagaaacagcggtaagatggtagtgaaagtgtaattttgagtatgacaaatgctgttgttcatacccgtgtaaaaaaagtagccgccggaagtattacagatgccagtgatacactcgctacagaagatccactcgaaataagactggtgcatgggccttcccataaccgccggcaacagaatatttccgttaccatgcgtacgcccggtgaagatatggaactggctgccggcttcctctttaccgaaggggtgatccgtgaccaggctgctatccaggaaattattttgtcggaagataataacggcagcgttgccaccgttcacctaaaaccatccatagtggcgcaacttggcggtacccagcggaattttgccgccacgggcgcctgcggggtatgtggcaaaacggatatagcatccattcatacaggcgtttccgttagcaacggtaccctttgcctctccgccgggaatttattcggactgcccgccatactaagaaatgaacaggcgctgtttgcatctaccggcggactacatgctgctgcacttttcaacagcaatatggaattactcctgctgcgggaagatatcggccgccacaatgcggtggataagcttattggcgcagctcttcagcaaccattaatgccgctggaccaatgtgtcctgctactcagcggacgtgcaggatttgaactgatacagaaagccgctatggcgggaatacctgttattgcagccataggcgcaccttccagcatggcggtaaaaatggccgtcgaatggaatatcacactgctcggctttctgaaagatcaacgttttaatatttacagcggagcagaaagaattgacgtaatataaattcacctttatggatagtgcagaaaacccggtgcggttcaccggtatcagactgggacctcccaaacaagtagccgcaggcatccctgcggtagtgtccagtatgcgacacatcctggaggaaatgaatgccttccgcggaatgaaagccctgctggagcttaaccagaaagatggattcgactgcccgggctgcgcatggcctgatccggatgacgaaagatccggcatcgcagaatattgcgagaacggcgccaaagctgttgccgaagaagctactaccaaaaagctgctgccggacttctttgcacagcacagcatcgcggaactcggtgaattaacggattacgaaataggcaaaaaaggaaggatagcccaacccatgtacctcgcgcccggcgccacacattatacacccatcgcctgggcagacgcctacaaaatcattgccggtcatcttcataaattaccctcaccggatgaagccgtattttatacctcggggagaaccagtaacgaagcggctttcctgtaccagttgatggtccgggaatacggcaccaacaacctccccgactgttccaatatgtgccacgaatccagtggcgtagcgctgagtgatgcagtagggataggcaaaggatctgttaccctggaagacatacatgaggcagaagtgcttattatactgggacaaaatcccggaactaaccatccgcgcatgctcacggctttacaaaaggcaaaagccaacggcgctaccatcatatctgtaaaccctttacccgaaaccggcctgctgaattttctgaatccacaaaccgttaagggaatattaaacattaaaacacatctcacggacatttttctgcaggtaaagatcaatggagatatggccctgctgaaagccttgtcgctgctgctgttgcaggaagaagaacgtgtacccggcagcgtatttgaccgggaatttatagccgcaaacaccctgggccacgatggttatatcgaccatctgaaaacgcagtcgctcccgcaactgatcgccgacagcggcgcagcgccggaattgatacaccaggccgcacaagctctgttccataaaaagaagatcatcgcctgctgggcaatgggacttacccaacataaaaacgcagtagacactatccgcgaagtggtgaacctcctcctgctgaaaggcagtatcggtaaaccaggagcaggcacctgcccggtacgcgggcacagtaacgtgcagggcgaccggaccatgggcatttacgagcaaccatccgccgccttcctcgacaaaattggcgctgtatatggatttcagccgccaagagcacacggctatgatgtggtgaatgccatcaacgccatgcaccgcggggatgccaaagtgtttatggcgatgggcggcaactttctttcggctacaccagataccctgtataccgcgcaggcactgcgtaactgcgaccttaccgttcacgtatctacgaaattaaaccgcagtcatgttgtgcacggcaaagaagccctgatactgccctgtctcggtcgcagcgataaagacctccaatacggcgagcagcaatttgtgacctgcgaaaattctatgggcgtcattcagatgtccaaaggcaacctgcaaccggtatccacccatctgaaaagtgaacctgttattatctgcgaactggctatggccttgctgggcgaaaaatcgcgcgtaccctgggcagactatacgcggcactatgaccatatccgcaacgatatagaaaaagtaattccgggcttcgataattacaataaaagggtaaggcatccgggaggattctacctgcccaacggcgcacgcgacggacagttcaatacctacagcggcaaagctaatttcaatattgcagaagtactcaccacgccgctggccatcgacgagtatatgatgatgaccatccgcagccacgatcagttcaataccactatatacgggctggacgaccgttaccgtggcgtatatcatgagcggcgcgtaatattcatgcatcctgctgatattgccgccgccggatttcacccgggcgatgtggtggatctctataattatcacggtggtaaagagcgcgtagcatatggcttcattattgtatcttatcacatacctgaaaaatgcactgctacctatttcccggaaaccaatgtgctggtgccggtagacagcgtagcagataaaagcaatacgccaacatcaaaactggtgatcattaaaataaaatcatcgactataaaaaactaacgcatgcaacccattatatggcaggcactattatggccggcaactgaatattttacattgcaggaaaatggaacggggaggctcgccactggttgtatcaacggagtaagggatcagcaaccattttgtattcattataaaatagagatcaccgcatcctggcaggtgtcttcctttcatattaaacaggaagggcttacgccaacagaactaaagcttacctccgacctgcatgggcattggtttgataaagataataaccatatagatgcatttgataactgtatcgacattgatatttcactgactcctttcacgaataccctgccggtgaaacgcctgcagtttgagttgcaggaaagtaaactgctggatatgctgtatatcaacctgccggaatttgaattgcagaaagtgcagcaacgttatacccgcacaggccagcaggaatacctgtatgataatgtatccacagattttacagcagcattaccgtttgatgaaaacgatattgtaacagattatcccggtattttccaacgcatcacttactaaagatcaaggctgtttcacggaccagctctgcgaaaatatctgccgtgctccaggcacgcgcctttccggctgcctgtccggcccacatatttacaaacgcagggttatccagttccttcgctactctacggatgggctgcgttaacgcatcctggtaaggatattcattaatgggtaacccggatgcttctatttctgtgatcaatgtattacgaacgccccttgcccaacgaccggagactgcccgcgtaagtagtgtgtccgtatccgttatatcggccaatgcggctttatgtgcaggtgtagcaaggctttcgtgggctctgaggaacaggctgcccaattgaacgccagcggcgcccagcatttttgcagcggctactcccctgccgtccattattccgccggctgctataacgggcacgtgcacacgatcagcaatctgcggcaccagcgcgaatgtgcccgtttgcggcaggtttcccggcaggaaagagccgcggtggccgccggcttcaatgccttgtgcgatcaccacatcggtacctgccgaagcgagtacagtcgcttcttccaccgaggtggccgttcccatcagcagcacatgatgctccttcagcagcctgaatccggcttcatcaggcatgccaaatgtaaagctcacatgttttatgcctgctgccaggataacgggaagctggtctctccaggaataaaaaggtacttcatcgaaattcaccggcgcagcggcaagcctgttggcaccatacaggaattgcaggaactcctgcatatcatcaaatattttccggtcgtaatgcgctgcaggctcataaacaaagaggtttacggcaaacggttgttgtgttaatccctttacctcccggatcagcgctgttatcttttccggaggcaaccctcctaccggtagggaacccattccgccgctgttgctcacagcagctaccatggcgggtgtagtgatccccagcatgggcgcctgtatcaacggataagtgatccccagcatacgggtgagttcattcttccattccatgacacaaaggtttagtactataaatttacggaatgaaggggtttcctccacatgattttaacggaagttcagcaccgtaggcgcgcgcagtgcagatacgtcaaaacgaaaatcaacgatggtagtaatttccagcatcagctttttcatgggggccggcgcattgggataataatagccggaaactttgatggtgttcaaagagaggttttcattgcgtacccggaagccgcctcccagtccgaggtaaaccggattgcggaacaggtcatcacttttattggtgatcatagatgcctggagcgctgtaaagaaattaaatttgaagcccaggaatttcagggggctgtagtacacggtttccgatcccaggttcaggcgctgatagccgttgatcatggtattcttatacccccagatgccgtattccatattaatgttgagcggcttattaaaaaacgggttggggctgttgaggtagtcggcgttcagaaactgccggaaccgtgatttccggatattcagcaacttgctgtaatattcaagacgggcatgtattacgccgtcttcccaggcattattaagccagaaagtactcagcccgatggtagagttaaagaggccctggttcctggtggtccagaatttctgcgcttcaataccggtgtagatcctccgacgatccttccagctttcccagccgctggtggcgctgatgttatatcccaggggaatatcctctgtgcggccaaagccgaaaaagtagtgggctttaaaataatcaatgcggtaagcctgtagttctgccaggtaaaggcggtggttattataaacgggatcgtctttataccgcaactgatccggctttcgctgaaaggataaattatagtgcctggccagcaccgcgaaattgggcttcttcccgatggtcccgtcgtgtttataattattgataaagttatacccgatccaaccatctattactgcgtaaacatagtcgcggtaaatgctgtcgccgttttcgggcagtgaaccccggatattaatggaccagttcttcgacagggcaaaaccgcccaccagtttggcggaattgcggtacaacggtttattgagattaataaataccgctccttcaaaggcgttggtatccagctgggcatagttattcagggtagtatagcccaggctcacatctataaaagatcccaggaggttatatttcgtgtaccttacttccgtgttccaggtgggagaataatcggagcgccactgcattccaacccggagtccctgcccggcgccaaacaggtcgttgttggatacgctggccctgatgtcttttgcactgaactgcgagatgtctacgccatattcaaagagatctttcgtaactacttccacatcgattgaatcgccgtcgttattttttacatataaacgggcatcctgtataaaaggccggttacgcaggtaacgttcgttatcggccatttcaaaggggtccaggggctgattctcccggaagaacaacgactgccggatcacccattccctggaatcgtagtgcatccggttggccaggtggatcagcttcatgctggtggtgaaagtggtatcattgatgttgcgcggaccgaaaacctttactttcctatagtagatatttctgatcactttgcccgcaaagggggtaaaatacgcctcacttttgatgatggtgctgtcgttatcattggaatgtgcctgaacatcctgtttggtaatgcgttttatgagcgattgccggtactctttgttacgcatggaatcgcggtattccccgatttttttgaagaggccactacttttatgggggacagtatccgctgcgagcggtgactgttggccttctgcgtataaacagacaggactatgcaggccaatcagccagcataagacagttagtgtaggccatattttgaaataattcctcaattctagcagcaggtaacaagtatatcgaaaaaaaatgaaatagcagcaactgcaattattgtacttaccggaatgataattgtgtaaaattgaacggattacctggaaaagtgttacagatattattgttcaccttaaagttttagttatgttacgctgggcactcatcttttttatcgtcgctattatcgcagcagtatttggtttcggaggcattgccgccggagcagcatctatcgccaagattctgttttacattttcctggtgttatttgctatttctttactgacaggactgctgcggaaataggagttgaaccgccttcggcggttgtaaattgtcttggagccggattacgttgattatgctgattttattgatttgatcaacttcgatttggaagataaggaggatactgcctccactcttttaaaatcagttataaaatccaaaagtaaaaatcaaactaatcagtataatcagcgtaatcctgagtcagacaacatccgcaactacttcatgatgctggtttcccagccatcgtattctgcatttacctgctgggccagttcccaaaggctcattaccacactatcgatggtggcttcactggctttgtccaagcgggaaatacataatttataagggaattccggattatctgttttctcttcccgggccagcgcaaagccattttccttgatgtgttcccagtaagcaattttatcttcttctgttctgaagtgaatccaatgctcaatgatacgttccttttctgaagcatctccatgctggcgcaacatacgaagcacctttctgttttgaatgcgctgaaactcgtacacatcaggaaagagaaaatcaaaatatagttcccagttattatcttcctttacgccgtagtcgtaacggtaatcaggaaaattaatcattgcatccgcaatgaatttatcatgcagcaaagtggtgcctgaataaaagtaaaaatcacgtacgccatttgaaaaagtgcggcctacaaaatgcgcatccagtttggtttgcagttgctctaccaaactatcctcaatttcacccatgacggcaaattcatcgttctgcgggaatccgtcctcacgtggattgttaagatacactgttatatatatggcattcggcttttcctttaatggcgcaaatcgtctcagatcaaggtcaaggcctattactgctggactttcttcaatatggcacgtataaatatcccagtccggtcggtaatccttatgcatataaaaaaattaaaataacgcaacagctggctgtaaagatacgttgctctgtaatacaatggaaacgataaacttgtattgacctcttttttatccacaaaatttagcgtatgctatgcgttggcctccactcaattacaccggttacaaaccaggcttaacactaattaacacttgtggtattttctctgcatattttctgtaaccggctaccacaagggatcctgtgcaattctgtagttgaaacagcggactgtaaagggttccaaccaacctttcatcctaaaaacagtcaattcttcattcataaaaggtaattttacagggctataaattgttggaagctattatgagaaaaattgtatcgttaattacaggctggctgttattgttttgtattactgctgtggcgcaacaaccgggtggaaaggccgcccccgccagtacgggcgttatctacggcaaactgctggacgcacaaaccggcaaacctattgagtacgcatctgtagcgttgctgcgtcccgactcctccgtgcagacaggtatgctctccaaaaccaacggggacttcagtttcgaaaacattgcactgaataaatatatcctgaagattaatttcatcggttacgaaaccatatataaatcagcggtgctgtcggctaaaaccaacagtgtagacatcggtaacatcaagctgaaggcgaatgtaaaatcacttgccgccgtgaatgtagtaggcgagaaaccggcctttacaatggccattgataaaagagtatttaatgtagaaaagaacctggccagtatcggcggtactgccaccgatgtactgaaacaggtgccctccgtgaatgtagacatcgacggaaatgtaaccgtgcgcaacggcgctcctaccatctttattgacggacgcccctctaccctcacattggaccagatcccggccgatgccatccagaacatcgaagtggtaaccaacccttctgccaagtacgacgcagaaggaatgagcggtatcctcaacattgtattgaagaaaaataagaaagcagggatcaatggcgccgtaaatgccggtgtgacctccctcggcagcaccaatggcggcatcgacttcaacctgcgccaggagaagttcaacttcttcataaattataatttccgtaaccgcaaatctcccatgaccagccgccttttccgtaagaacctgggcgctgatagcacctcgtatacagagcaactggaagatggtgacttctaccggaaattccagaccggccgcatcgggttcgattggtttatcgataaccgcaacaccatcaccgtatctgaaaacattaccggcggtaatttcaaccggtacaataatcaaatactgaatgaactggacgataagcaacaaaaagtacgctatggtacaggtatcaacaataccttaaacggattccgtaactacactacacagctgggttacaagcatacgtttgccaaagaaggtgaagagctgaccgcagatttcacctataactacgccaccggcgataatagtgccaattactccctgcagtattttgatctttccgggcaaccgatctatgatcctaaaaagcctgaattgcgctatggcagcggagaaggaactactaaatatgttactgcgcaggtggattatgtaaaaccgctgacagaaaaatccaagatagaaatggggctgcgcagcaacacccgcaagtttgataatttcaccaatacctatggacaaaattatccttccggcgatttctcactggatactgcgctctctaatagctatcattaccaggaacagatcaatgcgggctatgtaagctacaccggcgccaaagataatttcggctaccaggttggcttaagggcggaacaatcgaactacgacggagaaacaagactgggagagaaatcttcctataagatcaattatccgatcagcctgttccctagcattttcctgtcgcagaaatttaaaggcgatcatgagctgcaactgaactatagccgccggatccgccggccgtggttccgtgatctcctgccaaccatcgactacagcgggcaaagcgccaataccggtaatccgcagctgaaaccggagttcacgaactcctttgaattgtcttatctgaaagatattgcgcataaacacaacctgctggtatctttatactaccgcaataccaacaacgctatcactgatttttatgtagatactaccctgaacctgaatgggcagaaccagcacgtattactctcctatcctattaatgccagcacccggaattcatatggtgcggaatttacattgagaagccagctcacagaaatatgggacctgaccaccaacgtaaacctggcgcagacaaagatcgacgccaccagcaatggcagcaatctctccaaccagggccttacctggtttggtaaattgaacagcaacaccaagctgccgtggaatcttacgctccaggtaagcgccgaatatgaatccaaacaaatcctgccacagggcgaaagagaacctaaatggtcggccgatgccgccattaaaaaggacctgcttaaaaacaaagcgttgtctatttccctggggattgcagatatattcaataccgatcgcaatcttacctataccacgaccagcttttccgagcaggaaaattaccgcaaacgcgccacccgggagctgaggctcaatgctacctggcgctttggtaaaatggacacgcatctttttaaaagaaagaataacaagtccaaagaaaacaacaacggagaaatggggggaggtgataatttttaattcgtattttgtcgttgcaaacaacacttatggattctatttatcacactatcaccctgcggttccttgcggagccgtcagacgtaaacttcggcgggaaagtacatggcggttctgttatgaagtggattgaccaggcaggttatacctgtgctgccaactggagcgggcaatacgccgttacggtatatgtagggggtatccgtttttttaaacccatcgccatcggcgacctggtggaaatagatgcaaagatcatttataccggcaataccagcatgcatatttctattgatgtatttgcaggcaatccccgccagcaacagaaatccaaaaccacgcactgcgtcatggtttttgctgcagtggatgatcacggcaaaaccgtacccgtacccaagtggacgccacaaactgccaacgaaatcagcatggaaggctatgccaaaaagctaatggacctgcgtaaagacatcgacgaagaaatgagaccctacatgtagcgggaatcgtcgcggattttgtcttggctcaggattacgctgattatactgattaactggatttttacttttggatttttttagatttttagatttttcttaaataataattaagggagataagagcgaatatatccgcttctatctcccttaatcctttataaaatccaaaagtaaaaatccagttaatcagtataatcagcgtaatcctgagccaagacaaaatccgcgcgcgttagctcgcaaactgcatatcgctcagtgtccggtataggccgtccaggcctattaattcgctgtgggtgccttcttctacgatatggcctttgtcaagcacgattattttgtcggcctggcgtacggtggcgaggcggtgcgcgattacgattgatgtgcggccttccatcagcttgtccagcgcgtcctgcaccagtttttccgattcggagtccaatgcggaagtggcttcatccagtatcaggatgcgggggtttttcaataccgccctagcaatagcaatacgttggcgctgtccgccggagagttgaatgcctctttcccctactaccgtttgaagacctaacgggaaccgctgtatgaattcccaggcattagcctttttcgcggcttcctccatttcttcgggtgtggcgccgggcttgccgtaggcaatattttctgcgatggtgccaccaaaaaggaacacgtcctggggcactactgccatttgcgaacggagctgcgacagcggaaaggcagtgctttccttgccgtcaaacaggatgctgccgtttaccggatcgtacaggcgtaacagcaaggacacgatggtgcttttccccgcaccgctggggcctaccaacgcaactttctgatcggcatacacatcaaacgatacatcgttcataatggtaaggtccgggcgggaaggataatgaaaagacacattgcggaagctgatctgtccgtccagctggttttccggcgcaatggccgtcacctggctgatatcttctgccggttcatccagtatttccagcaggtgttcggtagcgccaatgctcttctgcagattggtatatacttccgctaaacccgcgatggaaccgccgataaacagggaatacaacacaaatgacagaaggtcggaagtaggcatcccgatggaaacgcccctccagatcactgctaccagtgcgccaaaaatacccatgataataaaggaagaaaaagcgccgcggaattttccgcttttcatacccagcctggcggcttcattggtgcgttggcggtagcgggcaatttcaaaaaattcattcgcaaaagccttcacgttcaaaacaccctgcagtgtttcctccactactgtgttggaagctgctacctgttcctgcacctgtttggaaaagcggcggataaatttcccgaaaaccacggcgactaccatcatcagcggcaatatggccagcataaagatggtcagatgaggcgaggtgaccagtaaaataaccacacctccaatgatgatgatgatctgccggataaattccgccagggtggtcgtaaaagtttcctgtaataaagaaatatctgaggaaatacggctgctaagctctcccacccttctttccaggaaaaatttcatcggcaggcgaatcaggtgactataaatagtttgacgaagcgtggccaacgttttttctgttacattaacgaataatacaacgcgaaaaaaagagaagatagcctgtgctatcagtacgccaatcagcaatacgccagctttgttcataccgttaaacaggtattcattacttttcggatctaccaggttgcccagcaatttcggaaaggccaggccggctaaactggaaaccaggaggaaaataaaacctaacgaaaactcaggccagtagggttttacataacggaacaggcggaatgtttttttcagagcggctacctttatgggttgctttggtgccgggggtgtggtgtcgttttgcattcggatatagtctttattaatagaggtagacgaaacgtatccaaatatattgcaaaaagcgggataaaatttataatgcctccggggattgcctttcccttgccggaaaaacaaataccagaggcattataagtgcggctaaggccgtggtctgttcttggatgaatctgcggcaccggtcccaaaacgggaagaatcttcccctgggttaatagctccgggaggcatttgtgccgcaggcacggtgtcctgctgtatcataccggctgtatccattgtatttaccgttgaatcggttccggatttattgccgtttccgcatgcagcgagcattacaaccgatatacctgccagcatgagcatgtgtgttactttcataaactgaatgtttaagggtgaggtaattcatttatcagttaacaaagcgttgtccctaaacaagcgttacagcttaccgctgggttgaatccggtttggttttagtagtgtctacgggtataacactggtactgtctaccgcaggcatagataccgcagcggaatcggcttcacgactggcttctttggaactgttacaggcaaacaggaaaaggctcagcatcccggttaaacagaggactacacatgatttatagaaaaaggcttccatgttgatcttttttatggtgataaatttcattcgtaacaggcattaaagcaaacagttcaatatgctgttacaattgataaaggaaagaattgtgccaacacgtacatttgtaagtatatattttgagacgatgaaagatgtattgcatatcatagaagaagaccagatactgaaagtgttgatagcgttggtgatgggtgcattgctgggtcttgaaagagagtataaacgaaaggctgctggtatgcgtaccatgaccctcatatgcatgagcagcactgtattcaccatcctatctgcagagttgggatatcctcattcagcagatcgcgtagcctccaatatccttaccggcgtgggtttcattggtgcaggcgttatttttaaaggcgattatacgatagatggaattactactgcggcatctatatggattgctgccgctattggtatggccgttggtatgagccagtactggctggccgcttcagctcttgccggtgcgctgattgtattggttacactggaatttgtagaaagaaaaattgcggatataaatgttaaacgttattacacaattttttttcatgaagaaaaatttccacatatggatgttgaaaatatcctacatgattttaaactgaagcataaaagaatgatgatcgtgagaaaggaacatattgtggaagtgaactacgcggtacggggcagcaaagaaagtatggagcagtttgataacttcctgctgacgaacccatttatctcccaatacgagatacaggcaaacccatcgtaagatttttaattgattattatgccatcatatgcagatctgcctttacattacggccaggttccgccctggctggccaagcggatgagccttctgggcggcgctattgtagaggctattgtaaccgattacggtaaaggagaagtgattaaacggctcagtgatccctgctggttccaggcgctgggctgtgtgctgggcatggactggcattcatcaggaattaccaccagcgtaatgggcgcgctgaaaaaagcgatcaatccccgttctgctgaactgggtatctatatctgcggtggcaaaggccgctacagtaaacaaacacctgctgaactcaccgccattgccaacaaaaccggcttacccggcgaccagctcgtgtacagcagcaagctcaccgctaaagtagataataccgctgttcaggatggcttccagctatatctgcattccttcattttatcagatgacggcgaatgggcggtagtgcaacagggaatgaatgatgccagcagcatggcccgtcgttaccactggcattcgtccgcctttcagtcgtatacagaagcgccgcatacttttatttatgggcgcaaccagggcaggatactcaatctcaccgacttacaggccggtgctaccaaaagcggcatccttcagcttacaaaagaaaaaccggtgcacctgctgcccgaaatacgtaatcttgtgatgccctcccatcatgatgtgagagcggaaaacgtgaacctgaaaaggctgggaagcgtgctcgccctggcgcatgataccaaccctgcggattttgaaaccctcctgatgctcgaaggcgtaggcccaagaacgctgcaatcgcttacactggtgagtgaagtgattcatggcaccccttcccggtttgaagatcccgcccgcttttcgtttgcacacggcggaaaggatggtcaccctttccctgtgcccactcgcatttatgatgaaactattcataccctgaaagaagcgctgcacaaagctaagatcggggaatcggataagaaggatgccatcaaaaagctgtcggcgctttccctgcagattgaaaaagattttgaaccgaacagcaattttgagaacgtgatagaacaggaacgccgcgattcgtggaaatatggtggcagaaccgttttcgggaaagctgtaaaacctcctgcacccaaaggcggcgaccagttaacccttttctgagcagatcaaataacggaatccatgatcaattacaatgaactcaccgttccggaagccactgttatacaaaaggaattacgtgactccgtaaaaataacaccgtacaacggccctataaactatgtggccggagcagatatttctttcaataaattcagtactactgtatacgctggtattgtaatgatggaatttccatcgctaaaaccggttggctacagtcttataaaaaaagaagtattgttcccttatgttcccggtttcctcgccttccgggaagttcccgccctgctggatgcctgggcgcaactgcccgtaaaaccggatatattggtggtggatggtcatggtattgcgcatccgcgccgtatgggtatcgccagtcattttggagtgcttacacaacagcccaccattggcagcgccaagaaaaagctgtttggtgtttatgaagaacctggtatggagaggggcagccggaccccgttaacggataaacagggacaacaactgggctatgtactgcggagtaaaaccaatgtggcgcctattttcgtgtcacccggccatctgacagatattccgggcagtgcggagacccttatgcagtgcataaaaggctaccgtttacctgagccaacaaggttggcgcacaacgcggttaaccaattccggacgggagtcattcctgaaggatggaccagtctttgaacaaacctaaagactacaactaaaactttatccacgcaatatttgcttttttctccaggcccttgcgcgaaatcagtactgtagcatatgtgcgtgtttgtgcattataatctgctgcgcccatcatacaggcatatccttttgttacttccggcgcaccgaaaagaaacaaccggtccatctttcctttataaaaacggtagcagacaaaattcgcgtctgccgcgtatttcaggggtttacgaactttgtcctgtccgccggtgtcgaggtattggagatagtcattgaaaagtacaaacgatacatccggcgaagggatatagtcgtacgacaaccaggtgttggtattcaatgcggcgattttattgcggaacacccactcacttttactgcggcgctgcaactggaaaggctcacaaacaccggtgatcacctggtattttgaaacggccagtgtggaattttcccttcccgccgtatccagtaaagcaatcccgatatctcccagattcgtgtgtaatttattcagctgtgagttaccttgtttaaaaaacgagaaactttccatcagcaacgtgctgcttccgtcttcgttcaggtgtatccgttgtggtgtgcctttgtattcttctttgtagttgagattctgctgcacattacgggagagctccggaaacgacagctgcacatgtttcttcagcttaccggtagattcccggaaagtattcatgatgatgccggaatacccgtctttttgttggggagacacatacagcagcatccgcagctgtgaagcagccacctgaatttctccaccaacatttccaaagccggcagtataatccagcacctcgtgcgcaaacgcagccgaatcaggcgataacatggagaagagcacctttgctcctgcgtcgccgtcttttcgtttggcgttaaagcccactgtgcccatgtacactttttcctttcctttcactgccatatcgatataactgaaatagctatacgaagagtcgggcatgtaaaacaagccactgttaattagttcatgccccggtgaaaaatgcatgacccggatacgttcgcgaacactgtcatttttctgaaccggcgcccctgaaaacaaagccacagcatagtaatcgctgttgacatctttctctacatacatatcatgagaagcgagattatcatctacaaatacgctgcggtgctgtacgctgggcagctctcccagtttatcctcccggagcagtttccctgtttcaccatccagtatcagacggtacatcacgggattgtattttacgagttgttgtaaaaaaagtaccggctgaccgtttatttcaaagatgccatctatttcagtagactccaggtctgccgcattccattgactggcatgtactgtatcagctactttcagggcccgggcgctgtcgtaaatatttaccagtagcccgtcctttttggagaaatgcaggtacaccgtgttaccattccttaactgcagcagtttatcccagccatctcccggctcggcgaagtccggtcccagtgttacgaccggtacctgggctatggcgaaactgctgatcagtaaagcccctaaaagaacggaccatctcaaatagttcattttcttatcaattaataatttcaaatatatgaaattatttaaattaataagacagatcactgcctaatgcccttcatgttctccgctgtttttcaacttagccagcagatcataggcgcctgttatcaccacatccccgtccggcgcctcttccgggaaaactacttcggtatagcccagttcactgtttccttttttaacctccagcatattgaaatgcaaagtgctgtctgttcccggtttttttacgaacacgtacgctttgttgtcgaaatccacaagggcggcatcaggcaccgcctttacggcagcggcgccggtttcaatcatggcctggagataagtacctggcagcaactgtgtatcttcttcctccaggtggcaatgcacccttaccgtacgttggggactgatttcacggccaatcaggtgaacagtagcggtacgcggcttagtttcattagccagcgtgaaacgtaccagctgaccgatctttaaccggggcacatctttttcaaacaccgtcagctccgcatgcagatgttcggtattcacaatgcggaaaaggatatccgcaggcgttacaaactggcccaggttaacgttcacctgtgttacatagccactgataggcgcatatatattaaccgtacgctgaatggttcctttttgcagggcagggaggttaatattcagcacggacagtttttgcctgattccattctctttggcctgcagggtttgccagctggctttggcttgctgcagcgttttcagggcgttcacattttctctggccagttcctgctggcgatcgtgttcttttgttgcatattccagctggctgcttacttccaggtaatcctgttgtaactggatgtagtcgaggttttccagtactgcaattacctgcccctgcttcactggcattccctgtaataaactggtttgctttataaatccacccattggtaccgagatgcttacctgttgctgcggcggtacatccaacaggccatttactttcacggcgccactgatctgccggttctctggtttaccataagtaatacctgctgttttaaattgtgcgggagtcagctctacaacaccaggttcctcttcatgatcatgcacatctgcagtagcaggtgtttgtttattgccgcaggaaacaagtaaaatgctgctgataacggtaaaggctatatgttttttgaataatcgcataatgatattttttttgttgatgaccggcggaacacagcttactgctggccggccagatatgccatgtataattctgcctgttttacttcattgcgcgccagcaggtatccctgccgtgccgtaagcccatgttccaggttaagaaaatattcagcgtagccaatgtctccgctgctgtaggatttttcagattgcttcagcagcagttctacgtttggcagtgaagtactttcataaaactccaggctgttcctgtttttgataaactcctgtactgcctgctcatattgggattgcagttgtataaggttattatcaaactgtaaactggccgcctgctgctgcttttcctccgcccgtacttttgctttgagaggtcctatccaaatgggcagcgccagtcctacctggaacccctggaagcggttactgttggtagccagtggcgcgccggaagcattcaacggagtgccgataaacgactggttaaaataacccaccatgatatccggcagtatcgcggctttcaacagcttcttttgcttttcggcaacggttacctgctgcttcaggtattgcagctgcggattggccactatggcagcggaatcactcacaagggaaaatgctgcatccggtatagccgtttccgttattgtaacgggcttgttggtacccaataatgcctgtaacctggcggtataaattttaagatcagcctcgttttgacgcagggcgttctttacttcgttgagccgtccttcggcagcgattttttccagcatccggctttcaccggtacggtaccgcaggtctgcgctgcgggcaaacctggtgaagatactatcctgccggagtatcagggctttcacctcctgcaggtacagcagctgtatgtacacctgtttcacctggtacaccagttcattctgcgtaaccgctttctgccaaactgctttgtccacctgcgcatgattcagttccttcctggcgctgaatacggttgggaaaggaatggtttgcgtaacactgtagttgttatcattggaaacataactgtttgtttgaccgtactgcaggttcacatctgttttcgggatttccccgctggtgcctgtcattttacggtagtaaccaatggaagcatcggcagatttcaaccctttgttttgctgcaaggccagctgtacagctgtttccagcgtgagtacctgcgactgtgcagtaaccattgcaggcaacagcaggcctgctaatatccagatcttcataatgtatgttttgaaaaacctttctccaaatagatgtataaacacggtaacaccaggagggtcagtaaggtagaagtaatcaaccctcctattaccacggtagccagcgggcgttgcacttccgctcctgcgctggtggccagggccatcggcaaaaagccgagagatgccacaaaggcggtcatcagtaccggccgtaatcgggtagccgttccatttagtactacgctgttgaggtcctgcaaaccggattcctttagccggttgaactcccctatcagcacaataccatttaataccgccacaccaaaaagcgcgatgaatcctacgccggcggaaatactgaagggcaaaccgcgcaacaggagcgcaaaaacgcctcctatggccgacatggggatagcggtaaatatgagcagcgattgttttacagagtgaaaagtaaaatagagcaacccaaaaatcagcagcaatgctacaggtacggcaacggctaaacgccggttggcttctttcagattttcaaactgtccgccgtaccggataaaataacccgcgggaagttttacttctttgccaatggcggattcaatatcggctaccacgcttgaaatatcgcggccccggacattaaagccaacgatagtgcgtcttttagcatcttctctttgcacctggttggggcccgtcgtcatttttacttccgccacttcctgtagcggcacctggtttccggatggcgtggtgatgtacaggttttgcacatctgccagctgctgccggctttgctggtccagccgcagtaccaggtcgaaacgcttctccccctcatataccaatccggcgctctggccggcgaaagcagtgttgatggtttgattgatggtggcaatgtcaagtccgtagcgggctattttgtccctgttggctgttaccacaatctgtggcagcccgccggtttgctccacgtacagatctttggcgccgggagtgcggcttacaatacggcctatcttgtcggccagtgaagccagcgtagcgagatcttctccaaagatcttgatccctacgtcctggcgcacacctgaaatcagttcattgaaccgtaactggataggctgtgaaaaaccaaaactcacgcctggtaccgcttccagggcttcctgcattttattggccagttcttcccggttgcgggcgctggtccattccttcctgggcttcagtaaaatggtgagatcacaggcctccatcggcattgggtcggtaggaatttcagctgcgcctattttgccgatcacttctttcacttcagggaattgtttcattaatatccctgaggccaggcttaccttgtcgatggtttcggacagggaactaccggtgagcagtcttgtttccacggcaaaatccccctcttccagggtaggaataaattctcctcccatcttaccaaataaaaataatgcgatcacaaaaagcagtatagccgctcccgtgaccaccgcctttgcgcgtaatgcgccgcgtataatgggatcgtatatacgctgaaagaagcgcataagccggtcggctaccgtgactttgttatcgagatttttactcagcatcagcgcggacatcatcggcacataggtgagcgacaggatgaaagcgccgagaatggcaaaggaaacagtttgcgccatcggccggaacatcttgccctcgatgccggttaaagcgagtatgggcaggtatacaatgagaataatgatttcaccaaaagcagcagtactgcggatcttgctggcagcatcaaatacttcagtatccatttcctgctgtgataaacgtaccagctgaccggttttattcctgccggcaaggtggtgtaaggtcgcctccactataatcactgcaccgtctacaatcagtccgaagtcgatagcgccgaggctcatcaggttacctgataccccgaagaggtacatcagggaaacggcaaacaacatcgataacgggatcacagaggctacaatcagccctgcacggaggtttccgaggaatagtaccagtacgaatatgacaatgagcgccccttctaccaggttcttttgtacagtgcctacggctctgcctacaaattcgctgcgatccaggaacggttctattaccacgccgggcggcagcgttttctgtatctgttcaatccttgctttcactgttttcactacctcgctggagttcttccccttcagcatcatcacaatgcctccaacggcctccccatttgcattgcgggtaagcgcaccataacgtacggcatctcccaattgcacggtggcgatatccctgatcaatatgggcaatccgtcaggcgtattcttcaccactatcttttctatatccgccaaactgctgatcagcccttcgcttcggataaagtaagcattgggtttcttgtcgatataagcgccgccggtgttctggttgttcctttccatagcgttgaacacgtcggcgatgctcaggtgatagctgcggagttggtcggggttgagcgtaacctggtattgcttcagcaatccgccaaaactgtttacttcggctacgccgggtgttcccagcagttgtcgccttacataccagtcttgtatagtacgcaattcacgcgcatcaaacttttcttcataccctttccggggatgcagtacatattggtatacttcccccaatccgctggaaatgggcgacatttccggggtgccaatgcccggaggaatactggttctcgcctcgcccagcttttcatttacctgttggcgggcccagtaaatatctacattatcatgaaatacaatggttacaaccgacagtccaaacctggatatagagcgtatttccgccagttccggtattaccgccatcgtttgttcaacgggaaaggtaataagcctttccacttcctgggctgcgagggaaggcgattgtgtgatcacctgcacctggttattggtgatatccggtaccgcatctaccggtaaacgtaacagggaatatacgccaaatgccgccagggcacacgtaaatatccctatcattaatttgttcctcacagagaaacgaatgatcttatccagcatgattgattcaataagtaataaaatgacgtaccatagccatatctacgccggtaaaggcatggatatgctcatagcaaaaacatctgtaaacggattaaaccagctgtgggggctgccagatattatctgataaagaaggaagcgggttaacgggcaacacggggtaatctatactgatccgttgcgccataaaataaaccgtgacggccacaccgggagtagcctgtatattacagcaactgcatacgcacaatggcgagcagtagtccggttgtgtttcatggtcgtgggaagtggcgagttgtacaactgcgctatggtttcccggctggtagtcgttgcagggaatgcacgacagcagcaggatataacagcttagtatgtaaagtaaccacttcatctttacaaatgtaaaaattaaacttaaaacgccattggaaaaaactgcatcgcagttgcggctgagatgattttatattacgatttgtacttaaattagccgcatgaattgcctgatcgtagacgataataagctggcgcgtaccgccatgaagcaattagccagtcatgtggaacaattgcatgtggcaggtgagtgcagcagtgctatggaagcatataattttttacagaaagaaaagatagatctcctgttactggatatagaaatgcccggtatgagtggactggagcttacccgcaacctgggaaagaaacgcccggtgatcatctttaccacggtaaaaaaggactatgcagtagaagcgtttgagctgaatgtggccgactacctgattaagcccgtacagcctgcccgctttatccaggccattgaaaaggcccgtgaaatcaccgacagcgatcaccgcgaactacaggtatccgataccgagtttgtgtttatacgtgataatggcatcctgaagagaataaaaacagaagatatccttttcctggaagcaatgggcgactacgtaaagttaaataccccgcagaaattccacgccatccatactacgctgaaagcactggaggaaaaactgccggctgctaaattcatgcgtgtgcaccgctcctatatcgtggcgctcgacaaaattgaatctattgaagatggcaccatcattattaataaaaacgcgattcctgtagcggatgcctaccgttctgcattgaataataaactgaacctcctgtaactcaacgacactttcccctttttgaccgacagctgctgcctgttgggccattagtattaccatcacttttctggcggatgtacctttaggtcgtcaaacaattgatcactaaataaaatatacagccatgaaaaagtttggtattgtaatcgccgcagctatgttgtttatgagtgcatcatcttttgcacagaccactgcatctaaaaaagaaacaaaaaaagaagcgactgcaaaggcgcctgctcacaaaacacatgcgaagcatcatcatacagcaaaacctgttgctgctccggctgcaccaaaagcgaaataatcatagtcctttgtcaacataattagcctcagcgaattattacgctgaggctaattatctgaaggaaggagcaataaaattgctacttttattgaaccggctttcctatatcagcgttttatatgtactaaactgtcatgcagcctaaaagaatcaaatattacctcctcggcctgttcattaccggaatgatattatttgttgtgctgcaattcaactccgcaaacaatatccataagctgatcaaaggcaatgagcagctgttacaggagcttaatgtaaagaacgaactccagaagctgcaaaccaatatggccaaaaccgacagcaaggtacgcggcgcagtgatttcccaggataccattcatattaccggcatcgaagccgaaatagccattattaaggcagatctcaaagagatcaataaaattatcagaaacgacagcacagaaaagttactcacccagctcaactacctggtagatgaaaagaatgcctttaacctcatggtactggatactttttacagtcagggtaaatgggcggctgaaaaattaattaacaaccagaaaggaaggcggctgggcgaggccatcaacggcattttgcggcaactggacaccacccggcaatcggaggtgaaccgcaccacccacctgatagacagcagcgggcaaaaagcgcagcgctggggtaccgtgctggtattttttgcctgtttaatgagcctgctggcattcttatatatcaccagccggatccaccggcaggagcaactcattgaagcgctggatgaatcccagcgacaggagaaaaaactggcgaccataaaagaccagttcctggccaatatgagccatgaaatacgaacgcccatgaatgcagtgctgggcttcaccaacctgctcaaagcccagccgctcaacgataaatccaaagaatatgtaggcgccatagacagcgccggccagagtttactggaaatcatcaacgacatcctggatatctccaaaatagaatccggtatgatgcgcatagaagccacctcttttagcctgcgcagcgtgctccatggtgtaaataccatgttcagacccaaagccgaagaaaaacaacttcagctggctgtgaccattgaggaagatgtaccggatatcttatatggagatgtaatgcggctgacacaggtgctggtgaacctcaccagcaacgcggttaaatttaccggtgagggcgaagtacgcatacatgtggcaaaagtatgggcagaagaaaatgcggttcgtatattattcaccgttagtgataccggtataggtattgacccttccatgcaacaaagtatcttcgaccgctttcaccaggcggaagctgctaccacccgcaagtttggcggaacggggttgggactggccatcgtaaaacaactgatagaattacagaatggctttatttcagtggagagcaaacccggtgaaggcgctacatttaaagtagaactcccttacacattgggggaatcattatcagaagaggggcatcattattttacagagaacgaccaactgccccttcatccagatgtacggctgctggtggcagaagacaataagatgaaccagaacctgcttcgtcatttgctgggcagctggcagttgcagtataaaattgtaaacaatggcagggaagtgttgcaggcgttggaccggcagcactacgacctggtgctgatggatattcaaatgcctgaaatggatggctacaccgccgtacaggccatccggcacgagctgcactccactatccccgtaatagccatgacagcccatgctatgaccggagagcgcgaaaaatgcctgcagatgggtatgaacgagtatatctccaagcctattattgaagaggacctctacagaatgatccaggtatacattggtaaactgccgccccgtgaactgccggctgtttatcacctgtcaaatgaaaatggcgcccagcatctcatcaacctgaattatctccatgatctttccaagggtaatactgaatttgaaaaaacaatgctggagcaattcattgcacagttgccggaagaactatcgttgctgaaacaggcagtgatagctgaagacattgcagctatacgcgctaccgcgcataacctgaaaacaaccgtttcctttatcggtttgcaggatcacctctatcctatcctggaaccactggaaaaactacaggaaaacaactaccatcccggtacggttgccagccagttcaataccctgaaacacctgtgtatacaggctgtacaggaggccatccacatcctgttataactccctgttgtatattaccgtacattttcccctgttcaacgacagtaattccctgttcaccgaaacatcccgtcaacaccgcctttgctgatgtaattttactacagaaactataacaaaacattcttcatctaatcattttaaaaagacaatatcatgaaaaaaagcctgatcgccgctgtagtagtaatgagcatttctgctgcatctttcgcacaagcaccagctgctaaacctgcaaagaaagctgctaaaactgaagcaaaagctgaagcaaaaccagctgctgacactactaagaaagccgctaaacacgaacatgcaaagaaagctgctcctgctgctaaaaaagcataacgagtacatacagcgtttgagttaattgtcccgcaagtctttcggcttgcgggatttttcgcggaggttgtcttggctcaggattacgctgattatactgattagctggatttttacttttggatttataaaggattaagggagatagaagcggatatattcgcttttatctcccttaattattattataagaaatctaaaaaatcaaagaaaaatccaaaagtaaatccaggtaatcagtataatcagcgtaatcctgagccaagacaacatccgcgaaaaaaaaagagtccgctgtcaggcggactctttccaataatatcaatacgcggtttattgtttagcacctaaaccgtccagtttctttttcacttcttctacttttgcagtgttgtttttgatcgcatagatcttctgcagtgcatagaggcagctttcgtaagtttgtttgtcacttgcatcgaggctgctggctttagcggtgaagccggcgtcagctttctcgaagaaaggcagtgcctgacccatcagtccttctacttttccctgtaattcttttgctttaggagaagtttgctgtttgctgtccaggccattcagttctttgttgaaaacaactgcgcggttaaagtacagggcacccagctggaagttagcggtagcatcggcaggattcatttcgatcgctttcttataggctgtttctgctttacctatcagttcttcgtagttagctggtttaggagcatcaccgcctttatcatcgcggggattagccaggttatctacgcggatagcgtaatccagtacagctgcctggtcggttggattgtcggcgattttcttttccagcatcgtcagtaattcgttggttttacctgttttgctgtagaaagccatttccatatcgttaaagcgtttatccttagggaataaagctttagcctgttcgattgttttcagccagtttgcctggtcgcctttttcttcatacagctgacccaggattacatagagagcaggttcgcctttgaactgcagatcggctgcttttttcaggtaggtaaaagcatcatcttttttaccggcctggttggcagcgtaaccaacgtagaaagtgagggcagtatctgcaggaatagagccaccaaggtttttactgttgtagaagtcagctacttcaaaagcctgtttgaagttatacagggaggagtcccatttctgctcattcaggttagcataaccggcgttggcaatagtagcgtatacattgaacaacggctggttcatttccagcaccgcttctttcattttaggatctatctccaatgcttttttgaaggcggcaaaagcttctgttgccagtgcagcgcttttctgcttggtgcccatagcttccaggatcttaccatctaccagccatgttttagcgtcgttcttggtcttttcattctgtaatgctgcgtcaatatccgctttggctttttccagatcttgcttcttcaggttctcatccgcactgctaacttttgcccgttgtgccataaccgatacaccggccgtgcaaaagagaagagataccaataattttttcatgcttttgtttttttagttgctgattacaataagagtatggtgctccaataaatagtaatacaaccagtagtatagttaccactaaaagctggctgtattttttttatcagaaaccggtaacagaccgggttaaggacctgttaccggttataattttatttattcttctgtagtgtcagtagcttcaccgtcggttccttccggtgtattgtcattttcacctgcgtcaggtgtttcatcacttgctacagcgggcgtttcgctaccttcttcgccttcttccagtagtattacttcttcttcctgttcatccagtcgtgctacagctgcaatttcgtcgttgtcatccaggcggatcaggcgtacaccctgtgtggcgcggccggcttcgcggatatctgcaacggccatgcggatggtgataccggacttacaggtgatcatcaggtcatgtttctctgtaacatcaagtacagctatcaggttaccggttttttctgtgatgttaatggttttcacacctttaccaccacggttggtaatacggtattcctcgatgttggtacgtttaccgaatcctttctcagaaaccaccaggatggttttctgttcatcttccttattaacacaaaccataccaaccacctcgtcgttgtcgctgtctacctcaattcctcttacgccgatggcgccacgaccggtgtcgcgtaccgtagcttcagggaacctgatagcgcgaccgctctggatggccatcatgatctggctgtcaccggtagtcagtttggcttccagcagttcatcgccttcattgatggtaatggcattcacaccgttctgacgcggacgggaaaactcttccaccatcgtcttcttgatgatacccttcttggtacaaagtacaatataatggttattgataaaatctttatcactcaggtctttaatatcgatgatagcgcggatcttatcatcaaccggaagctggatcatgttctggatggcacgtcctttaccactcttttccccgtccggaatttcatagaccttcagccagtagcagcggcctttttccgtgaaaaacagcatggtatggtgtgtagaagccacaaacaggtgctcgatataatcttcatcacgggttttaccgccgatggcgccacggcctccgcgtttctgctgccggtaatcgtaggcagaagtacgcttgatatatcccaggtgggaaatggtgatcaccacatcttcttctgcgatgatatcttctatcctcatttcgctggcgagatactggatttctgtcttacgttcatcaccgaatttcttcttcacttcttccagttcttcgcggatgatcttcatacgtaaagattcatcagccaatacctctttcaggtaagtgatcagtttcatgatgtcgtcgtattcagcgcggatcttatcgcgttccataccagtcagacgttgtaaacgcagttccagtatagctttcgactgtaattcagacaatccgaattctgtcatcagcccttccctcgcaatatcaggcgtagcggcggcgcggatcagtgcaatcacctggtccaggtgatccagtgcgatcaggtaaccggcgaggatatgcgctttttcttctgccttacgcaggtcgaagcgggttcttctcactactacttcatgacggaagtcgatgaattccccgatcatatctttcaggttcaggatacgcggacggccttttaccagcgccacgttattgataccgtaagatgtttgcagttcggaatatttaaataactggttgatgatcacattggagattgcttctcttttcagatcaattaccaggcgcataccttcacggtcactttcgtcacgtacatcggagatgccttcaataatcttatcatttaccagctgtgcaattttctggtgcagtactgctttgttgatctggtaaggcagttcatagatcaccagcttttcacggccgtttttagcggtttcggaggtaattttacctcttaccactactctgcccctgccggtttcaaaaccttgtttaacgccttcaaaaccataaataacaccccctgttgggaaatccggtgctttaatgtgtttgatcagctcttctatagtgatctctctgttttcaatgtaagcgatagcgccatccactacttcgctgaggttgtggggcataatgttggtagccatccctaccgcgataccggaagcgccattcaccagcaggttgggaatgcgggtaggcagtaccgtaggttcttcgagcgtgtcatcgaagttgttggtaaagtccaccgtttccttttcaatgtcttccagcatggcttctgcgatcttctgcaggcggatctcggtgtaacgcatggcagccggcatatcgccatctaccgaaccaaagttaccctgtccgtccaccatgggataacgcatgctccagggttgcgccagtcgtacgatggtgtcataaatggaagcatcaccatgtgggtgatatttacccattacttcacccacaatacgcgctgatttcttgtaggccttgttactgtggttgccgagttcattcattccgaataaaacgcgccggtgcacaggcttcagaccatctctcacatcgggcaaggcacggcccacgatcacggacatagaataatctatgtaggccgttttcatttgctcctcgatatttatctggacaattctcccttcctgatgattttccgtatgctctgtcattttgtgtgttgatttacagttttttctgcgtaaaacagataaaggcaaatatagccatttcagcccttattccggcctaaaaatcaaagaatgtgaataaaaaacgccatagggattaacgcttatattgcaatatcgatatatgattgatttacacaatgaatgacaaccatttatatagcatttgtgttatagtaaaacaaccctgattttgatttaattgcaatatgttaagacacattaatatattagaatataaatattggcaaagtatttgtttctaagaggctgataatcaattgttcgaatcaacggaaaacatatatataataagaacaaatccgaatttgcttaaaaattcgaacattagtataaaaagtgctgttattcccctgattcttaatcacttttctaaagaagactatgaagaacatactgttgtttggagccggtaaatcggccaccagtttgatcgactatctgttggcaaatgcaccgaggcaaaaatggcatatcactgtagccgatcatgatctttcgctcatcaaatccaaaacaggaaaatcatattatgctacccccgctgcactcgatattaaagacagcgcggccagacaacaactcatccgggataccgatctcgtcatctccctgttacccgccaccctgcacattttggtggccaaagattgtcttactgaaaaaaagaacctcctcaccgcctcctatatcgacgaagaagtacggcaactgcaacccgaaattgaaaaagccgggttactcttcatgtatgaaatgggattagacccgggtatcgatcacatgtcggccatgaaactcattcattccatcgaaaagaaaggcggacagatcttctcttttaaatcctactgcgggggccttatctccccggacagcaacgataatccctggcagtacaaagtatcctggaatgcccggaacattgtaatggcaggcgtttccggcgctacctacaaagaaaaaggaaaggtaaaggaacttagctacgaacaactgtttgatcatacaaaaacgatccaggtacctggcttcggtaaactggccttctatcccaaccgtgactcactgggatatatgcaggcgtataagctggaagaactggccacttttatgcgcgccaccctccggtatcccgacttctgcgaaggctggaacgccctgatgaagctgggcctgacagacgacggtcataagattgccacggataagcttacgtatactgagtgggccaccaaatccgttaaagaaggaacaggcaccccggaagagaatatggcccagttcctgggcgttagcaccaagtccaaagtgatccgccagttaaaattcctgggattattaaatacagaagtcataaatttaggggagcaaaccaacgcaggcgttctccagttcctggtggaaaacaaacttaaaatggagcctgccgacaaggacatgatcgtaatgatgcacgagattgagtttgaacgccgcaacatggccaccaggatgcacagttacatgattgttcagggcgaagacagcatacataccgcaatggctaaaacagtgggacttccgctcggcatcatggccaaaatgattctccaggataaggtaacgttaacaggactacaaataccggtaatgccggaaatatataaccccgttctaaaagaattagaggagtatgatatcagatttgaagaaagctttgaataagcgcaaagttatttttttcctatgatggactctaaccgggcacaaggacttgtgatacctcccctgaagtggggaggttttttattttacaggatacttaataattccagcacgccttctgtagcaggcttttcaatcaggtgcaggttatccgcttttcctacttcgggaattttccggtcgatgatatacaccggcacgtccggttttacatactgcaacaagctggcggcaggatatacctgcagggatgttcccaccaccacaaacacatcggcctcccatacttcccgtgcggccttttcaatcataggcaccgcctcgccaaaccaaacgatgtgcgggcgcagctgtccaccgtcttctgcgaggtcacccatcttaatatcctcccggatatcatagatcagcgcttcattattcacgctgcgcatcttgaaaatttccccgtgcaggtgcagtactgtagtggaacctcctctttcatggaggtcgtcaatattctgagtgatgatccgcacatcatacttttcttccagctttgccaggcctgtgtgtgcagcattgggaagcgccgccttcacgtcctgccggcggccgttgtaaaagtcctgtaccagggcaggattcttctcccagccttgcggagaagccacttcatacacatcatagccctcccataatccatccgtgtctctgaaagtccggaggccactttctgcgctgatgccggctccggtcagcaccaccaatcttggtttcatgtgaattcgtttataggtttacgttagctggggttttacgggatttccatctccctactcctctttttataaaaataaaaataaaaacaataccaacaatcaaaggccatgcactcaatatgcccaatgcaaaagataaaagcccgttccagccatctttaaacgacaaccacgagcgttgcaggaatcccggcgactgcggatctgtattggcaaacgtctggtaatactccaggctgatattgctgtaggccacatgatgatccatgtactgcaaccggccctttgcggattctatttcttcacggatgcctttcagctgtgcctccacttccagtatttcttttacattcttcgcctgctgcaggatctgcacataacgctgttctactgccagccgtgctttcatacgggcgtcgaggtctacatattcttctgttacatcagtggaggtaatacttttttcatctacccgggaggcgccgccggtgaggctttccacgcattgttcaaaagcggccgccggcacttttatggctacctcattccgccattgcatactggtattttcctgtttttcactggcaatgtagccgccgtactttttaactgtatcggctatacgttttttacaggcttcaaagtcggaagtggaaaatcggagcaccgcattttttattattttttgagagatgggtaaggcaggcgcctgatcagcttcgctttcagacaggggaagctcgtcgctggctactacaggcgtggtcatccggatatctttctgtttgaattcagttgcaaccggggcactgttattgcggcaggccggcaataaggccactgctgtgcaaaaggctaatatgaaggaatgtttcatgagctggaattttctctatgatgaacatctttcacgaattccataaacggcgaaggttatcttccataagaaagataaccttcgccgtttatatctctggtaaagtacctacttcttcataccacccatttccatgatcgcctcaaattcttccggcttcacatcacacacggataagcggccctggcggataagcgacaggttggccaatcgtttttcagttttcatctgtaccagcgtcacggcctttttaaatggctttaatggtttaagatctaccaccacccagtttggatcgggtgtagtgggatcctggtaagcttctttggcaacggtggccaggcctactatttccatcccttcattgctgtgatagaacagtacctggtcgccttttttcatgccccggaggttgttgcgcgcctggtagttgcgcacaccatcccaaaaggtgatcttatcttttacaaactgatcccaggaatatttaaatggctcagatttcaccaaccaataattcatatagcaattaattttcgtaatcagatagttggaattaccaaccgctggccaatacatctgcaatgtgcatcactttgatgttggtaccgtgcttacggatatagccatccaggtgcatgaggcaggaaaggtcggtggagatcaggtaatcggcgccgctggcaacggcattgtttactttctgttcgcccattcccatggaaataggttcaaacttaacggagaaagtaccgccaaatccgcagcatacttcggcatcgttcatctctttcaactccagtccttttactttttccagcagtttacgggggccttctttgatatggcattcccgcagtgcgccgcatgcatcatgataggtggctacgccgttgagggtagctcccaggtctgttacatgcaatacgtcggtgagaaattcggtaaattcgaagaggtttttcttcagcagtttcacatcattatgtgcggctgaattatcgaacaatttgccatagtagtttcttacaaaaccggtacaggaaccgctgggagcaacaatgtagtcgaaggttttaaagtcctttacaaacttggtagctacggtacggcattcatcctggtacccggcattgtaggccggctgaccacaacaggtttgttccgtgttatacattacattacatcccagtttctcgagtaccttcaccatattgaaggcggtttcaggaaacagctgatctacaaaacacggtataaataactgtacattcatctctatagcttttagcgattagcccttagctcttagctaactttctttgcaatgcaatcatcttcagtgcagtaatggcagcttcttcccctttatggccgtgggccccgccgagtctgtcctgcgcctgctgttcgttatctaccgtcagaattccaaatataacaggaacgggtaactgaaggttcagttgaaggataccttctgttacggctttacacacataatcgaaatgaggtgtttcgccacggatcacgcaaccgaaagcaataatagcgccaggctgtttgccggtgcctttggtggtttcccagtattgcttacaggcgtaaggtaattcgaaagcgccaggtacaattattttttctgatttggtgatgttatactgtttgagggctttttcacagccgcttaccagttcattcacgatggcatcattccattcggtatacaccataacaacactggcatcctccaggttgagaatgccagcgtcatttaataagctcttattgtgctcggacatattttatagctttgggctgttggcagttagctgtcagctaaaaactaacagctaactgctaatagctagttctttacatctcccagtcttgccaggtatttatccatttcacgaccttcgttggtggtagggaaattctttttaatttcctgatagatagcgattgcttcctgcgccttaccagctctttccagggcctggcctgcacggaacaggtatacgggggcagtcagttcattatcgttatagtgacctgctttcttgtaggattcaataccttcttcagctttattcagctccatgtaagcgtcgccgatcaaaccgtaggcagtgggttgcagcagcagatcatttgaactaaaagatttcagcatgtcgatacccttctggtattcgcccaaacggatgtagcaaacgcctgcgctgtatttagcgaggttaccggctttggtgctgccgtatttatctgctacctggatgaaaccgtagttattaccatcgccgttcagtgccagtttgaatgaatctaccgcgaagtagttttgcgcatggaaaatcatttcctgtgctttattttcattaggctgttttacaaaacggttataagcgaagaaaccgcctaccactactactacagccaatacggctatagaaataacatttttgtttttatagaagaaatcttccgccttgtgcatggatttctccaggtcaaaatcttttgtaggttgaggcacggtggctttatctttagtttctgccattgtaaggtgtaattgtgattgcttggttattaaatatagggtttagctttaggctttaagcctttagcagatgcagctttgctacatttactaaaggcttaaggcagatagctaaatacattagtcaacgatgaatggataatcttcctgaacgtaaacgtctttcagcaattcatcatcggctggccacggagattcttctgcgaatgttacacactcttcaacttccacttttacgcgttcgttgattgcttcaatttctgcttcggtagcccatttatttttctgaataactctcagtacttcgttgatcggatctttctccttgtattcttcgagttcttcttttgtgcggtatttagcgggatcactcatggagtgaccacggtaacggtatgttttgatttccagcagggttggaccgccgttttcacgaccgcgtttcaccgctctttcgataccatcatgtacagcttcgcagctcataccatcgatagaatcggccggcatttcgtaagcatccgccaacttatagatatccaatacgttggaggtacgttctacagaagtacccatggcgtacatgttattttcacaaatgaaaatcacagggagcttccaggtcatggccatgttaaaggtttcatggaggataccctgacgggcagcgccatcaccaaagaaacacaacacgacgttgtctgttcctttgtattgctctgcaagcgccagtccggcacctgtacctatctgagctccaacaataccgtggccaccgaagaagccatgttctttagagaaaaagtgcatgctgcctccctttcctttcgaacaaccggttgctttaccatacagttcagccatacaagctttagcggaaattccttttgcaattgccagcgcatggtcgcggtaggccgtgatgaatttatcctcgggcttggtagcagtcatcgcaccagcagcaattgcttcctgtcctatgtacaaatgacaaaagccacggattttttgcatcccgtacaattggcctgtcttttcttcaaagcggcgcagcaaaagcatcaattcataccagtacagatatgtctctttggtgaatttcgtcttcacgtctgttttagtttgcactctttctaaatttgttcgcaaatataacaggaaaatcgtaaaatataaatatcaattctaattcccattaaattatgcaatttcatcaatttcaaacagttttgcatttatttgcacgggaatcacagggaagttcccattagagcggttttttatcacttatacaattgataattttcgcatattattatttacgaataatctttttctttgctttatataaataaaatattactcgttcagttcaaaaattacagccaggcgaccttttccttcgggcacaggatcgtgggcatcaccggccgcaacggtgccggcaaaacaaacctgctggacgccatctactacctttgcttcacccgcagctattttaccagcagcgaaagtcagaatacccagtacctgaccaacggcttccggctggagggctatcttgaaaaaaataaccaggaagaaaaaattgtctgtaccctcaaagagggccggaaagaaataagccttaacgacgaccggtacgaccgcttttcccggcacatcgggcagtttcccgccgtaatgatagccccggacgatgcggacatcatcctgggaggcagcgaggaaaggcgtaaatggctggatagtctcctctcccagctgtatcccgagtacctcgaccacctcatcatctatcagaaaatattattacagcggaacacgctcctgaaaaacatggccgctaccgggcagaaccaggatagcctgctggatgtattcgacctgcagctggtgatgcatggcgtaccggtgtacgaaacccggaaagcctttctccaaacctttattccgcaggtacagcgcctgtacgattatattgccggcacccacgaagtggtaaatatccagtaccagtgcaccctgcaggaagaagattacgcggtacagctgcaccagtccagataccgcgacatgcagttacagcgcaccactaccggtattcaccgcgatgacctcctttttttgctgaacggccacctgatgaaaagcagcgcttcacagggacagcgcaaaagctttttgtttgcacttaagctggcacagtttgaagtgatccgtcagcataaaaaatttcctccgctcctgttgctggatgatatattcgaaaagcttgaccaggaaagggtgagccgcctcattgccctggttgccagcgataattacggccaggtgttcattacagatacgcacgcagagcgcctgcaagaggcatttgcaggcaccggcgaggccatacagctgataacaatatagcttttagctttcctccgtaaagttgatcaccaaaagctaaaagcccatcacagagaaccaaaaaatcactagcttcgcaccatgcgtcatggaaccaccagtatcggagatgcgctccgggaatttatgaataagagcaggatgaaaccccgtctcacggaagtacgcatccaggaaaactgggagaaactgatgggtaaaactattgcccgctacacacagagtatccagctgatcgatcatacactgatcgttacaactacggtggcgccgctaaaacaggaactaacttattcgaaagataagatcatcaagctggtgaatgaaatgctcggggagaacattgtaaaggaagtgatgatccggtaagtatcagttggaggcaaactggtgaatcagttcgttgatatcgctcattttcagggtagtttgcaggttgacgatcaaaaagtcattttcgtcctgcaccagcatcaccacattacccaattcatcgtcttttcctttgttgagtatatggatcaggcttcccttttccctcacttccatcagcaaatcaaaattttcattccgttgcaggttacttttcagatcggcgatatcgtcgttgctcactgtgccgcctttcacgttagagatggtgtacatctttactttgcgcacatttttaagcgcatgtttcattgtctgggcatctgcatcttcactatcaaacgacaagcataaacttccaagccgcatagcaaagttgccaaagctgatggtatgtgtttcggcgcttcccctgtacttgttgcggaactcccgcaggcatttatcctgggcctttacagcggtggcagacaaaacgatacaactggcggcaatgagtaatgatttcatgggggtggtttttaaaagttatttcttcttcacattttttagtttatccattccctggatattcacgccgttggcgatctgtgatatttcattgaggtccatggtgcccacgaggctcatggccaggaactgatcggaactgcctaccagcatgaccagttcattgatatttcctttcgcatcttctttgacgaggaacttcaggtcgctgtctttgtcgcgtaccgtcatcagctcttcaaaatcgctgccaaggaaggcggcggcctctttgtacaaccggggaccatctttggtggtttcctttgtaaggatacggagtcctttcagtttctggatcaccttcatcatgtttttggcatccgcgtcgccggcatctactttggcgaacatgctgaacattttgggggtaatggtgatcaccgtgaaactgcgatcgttctcgtacttctggaaaaaccgttctataacgcttccctgttgcgcgaagaggtgaaaactggcaaagactgccaatagtaataacaagaatcgtttcatctttctaaatttatatcaggttttaaaatggccgttagtcttccttgccttctaccacagcagtagcttcattgaaataagacagctgctgcatctttgaggtgcctttgtgcaggtttttagccagcagctgtaaagccctttttgtttcgtccagcgctttctgcggatcgttcagttcctgctgctccagggctaccaatacctgttgttcacgctgctggtgctgtttgagcgcataaccgatgcctactgccaccatgatcacagctgcatacttcatccaatgccgccagggcgaaagcttcaccacttttaccggcggcgcttcccatactttttccgcctcccggtgaaaatagccgaacaggggcgctgcttcctgcaatacttccggcagggctgaatgtggcgtactgaaaaaatcccgcaacaccgcttcctcttcgagggaagtttctccttcccagtacttttccaccaatacagtgatttctttataatccatatacctgcaggttttgtagtttctcgcgtaccgttttacgggcacggtgcaaattcactttaacgtcgttcatgtctatatcgagtatgtcggcgatctcctggtaggaatgcccgtcgatatccctcagttgaaggatggtgcggtacttttccggcagggcgttgatagccacatgcactttttccattacatcgttctgttctgttaccgcatggggacttttctgctgcgttgccggcagctctcctgccctatccagttcatcagacatccggtatttcctggctttgattttatccagggccaggttgcgggtgatgcgcatgcaccaggcctccatgttttgcagttccgccatcttctcctgcatgccccaaactttcatcagggcatcctgggtgatatcctgcgcgtcttcctcgttgcccagcaggcggaacgcaaagcggtaaagctttggcctgactggaactacctgggtaaggaatcgatctaatgacatgcagaatagtgcgttttgaaagaagacgactgtaaaaagaagatgttacaaagatgccgatatttttttgcggattttgtcttggctcaggattacactgattatactgattttctggattttgtttttttgattttataaaggattaaggggatgtaagtgtatatattcgcttttataatctaaaaaatcaaaaaaaatcaaaaagataaaatccagaaaatcagtataatcagtgtaatcctgagccaagacaaaatccgcgttagtccagtttgatccgcgggtcgatgagcgtatagagcaggtcggccagcaggttgacgatcacgaagatgccggccgtaaagaggatggctcccattaccacggggaagtcgaatttatccagcgcctccacggttactttgccgatgcctttccagccgaagatgtattccacgaagaaggcgcctgccagcagttcggcgaaccagccggtgatggcggtgatcaccgggttgagggcgttgggcaatgcgtgccgccagatcactgcggagcgggaaaggcccttggcgtaggccgtgcggatataatcctggtgcagtacatccagcatggcgctgcgcgtgagctgcacgatgatggccagcgggcggataccaagagtaatagccggcagcaccaggttgcgcaggttaagtaccctgcctttgaacggatccacatcaaacaggttgccggacatatgcaggccggtataatcgctgagtacaaagccaaaaagataagccagcacgatgccggcaaaaaatgaaggggcggaaatacccgccacactggcgaatactgcaccagtatccatccaggtattttgctttaccgccgataatacgcccagggcaatgccgttgatggtggcaaacaccatcgcagctatggccagcagcaacgtacccggcaatgcctccattaaaatatcccacacctgttttttgccctggtaagagcggcggagatagggtgctttcagcaccaggagtttgtcctttgatatatgcgccaccgttagatagcggagattttcatccgcttcctgttgggtgtggactccaaccggcagcaggtcgttcaggtaatacaggaactgcgtccccaccggctggtcgagatgcagttcccggcgcacgttttccagggaggccacatcggcccgctgccccaatgtaagccgcgccggatcgccaggcagcacattgaacaggaagaacaccagcaccactacgccgagcagtaccagcaatccgtatccggttttacgaagcagaaaacgaagcatatattattatggtatatcgttatagtgccatttccctttaatggtgcctttgttcagcaggatcagggcaggattacttctgccggcggttttaatggctacgccatccatctgcacaaatggaaactccaggccatgttgttgtttgaaggcagcaatttcttctttggtggaagcggttactccatatataactacctgctggtttttccattgctgttgcagggcttttattttttcgtcccatccgctgccggccttttgagtattcaataccaggaagagatataccggtttggtttcagacaggatggcttccgtttggttcaccccatcgagatcagtgagaatgaaatccttgatggccggttccgcgtttcctttcttcaccagtttatctttacggtccacaaacttccaggtactgtcggaccacgggtaattgtcggcagtaaattctttcttctgcccatccttttcataaatgaagatcatctcatacacgtctggcgtagcgcccggcggcagtttcatcttctcgggaatattattacctactttatacggcaggcaatcgaagagcggaaggtgttttaaagtataccgctggataccgaaggcgaataaggccgagagcaacagtaccgcgccggctcctttaaagagtggctgtatggtgttccggtaaaagaagatcacgaggatcatcaccagcaggatcacatctttccagaaggtttcctcggcggtgagtttgatacagtcgccgaagcagccgcattcacggatggtaccgctgaataatgcgtacccggtaaggaaggtaaagaatataatgagcagcaacagcagtacggaaaaggccctcatgcggtagccgatgagcactgctacaccggcaataatttcgaaggcattcatgataatagaaaatgccagggaatagggagacaggaaggtaaggtgcaatacctcgaaaaactcctccattttatagctgagtcctaacggatcattagctttaatcagacctgagaaaatgaataacaccccaacgattatacgtaacaggttaaggataatcttcataaaatagtttaatggttaagtgatccgtgaagataagaacaatcagggtttaccttcccgggaaattgatgagcgtatctgaaagtgagttgacgacgcgccaaatctatttctgaaattgaactgctaaattcctaaattcggcaatgattgattttccttcttagatttgcaggcaaaataaagaatttcgggtaaaaggccggaactatgtgaaaattcaggagcaagagcctgcatgctaacttcttaacgcattcaaatgaaaccagaccatatccccgtaacaacaatgtcttcaccggtaataaattgcagggggcaattgttatccctggccacccctgctgtaatgggtattattaatgttaccaccgattctttttatgaaggcaaccgcatgcatgagctgcaccaggtgatggagaaagcgaagcaacacctggaggaaggggctgccatactggatctgggcgcacagagtacccgccccggtgcggagatggtgggacgggaagaagagattcaccggctgctcccggcgatacatgccattttgaataagtatccttccgcaattatatctgtagatacctggtatgctgcggtggcagagaaagcggtacatgccggcgcggctattatcaatgatgtgagcgccggggatatggatgcggagatgattccggttgttggtcagctgcaggtaccttatattgcgatgcacatgcagggcaagcctgccaccatgcaaaaaaatccgcagtacaacgatgtggtgtccgaagtgctcgattacctgaaagaaaagctggcggcctgccgtgccgccggtataaaggactttattgctgacccgggatttggttttggaaagacaattgatcataactatgccctgctgaaacacctgcgcctgttttatgatgtacttggagtacctgtgctgacgggcatttcccgtaagtcgatgatctataaactactgaacataaccccggccgatgccttgaacggcactactgtattaaacaccatagccttgcaacagggcatccatatattaagggtacacgatgtaaaagccgctgtggaagcggtaaggattacggagaaaatgaacggataatttaatcttgctatttttacaactatgaaggaagtaatagaattttatggagttgagtttcgatggctggatctgctggacctgctgattgtaatttttttgatcattcagttgtatcgtttattaaaggggagtcttgcttttaatattttcgtaggcctgttaatggtatatgccgcatatttcctggtgagggcgttaaagatgcctattctcaccattatcctgcaaaactttatcaatgttggtatcattgccatcatcatcattttccagccggagatcaggaagttcctgctggtgctgggtaagaaaacgccgctgagcaaggacagttttttaaccaaattgttcctgcctgataagtttaagagttataaagaagaagaaaacattattaatgaaattattgtggcggtgagccggatgcagagcacctttaccggggctttgatggtaattgccaccacctaccgtttgaaatttgattccgcatccagtattcctattgatggaaacgtgagtgcgaaactcattgaaagcatttttgagaaacacagtcccctgcatgatggggcgctgatcattgtgggcaataagatcctggcggccaaagtgatcctgccggtatctgagaatcctaaccttcctacccgtatagggctgcgtcaccggtcggcggtgggcattacggagcatagcgataacctggcgatcattgtttctgaagaaagggggacggtgtcttatgcgatcgacggggtactcacccaggatgtgtcgctggaagacctgaaagtaaagctatatgaagtattgatagatggatatgcctgatccgggaataagccacatagcataaaaggaaagccccctgccatttggcagggggctttccttttatgcggttataatcaattacttaccgggagtagcgaattgagaaggagccggagcgcctgctttaatatctactaactctacgttaaatacgaggacagagtttccaggaattaccggaggacttccctgtaagccataagccagtacagaaggaattaccagggtagctttggaaccttttttcaggccgcttaaaccagcatcccagcctttgatcacgaagccgcgaccgatagggaacttaatgggttctaaaggcatgcccgggcgcatagttgaatcctggctggaatcaaatactttaccggtggtgagcttacctgtgtagtgtacataaacggtgtcacctggattaggtgtactgcctgtaccttcctgggttactgctacgtaaacgccttcagcgtttttagtggcattgatcttgttcttatccaggtattctttaataactttttcgtctttttctttctgggcagcagcagagtatttgttttctactgcgaaagtgattttcagtttatcaccttttttaccaaatggaggacgctcctgggctggtaatgaatcccatggaatgataaaggttgcgctatcaccttcgtggaggagggcaataccttccatcagatcgtacttattctgtggttttgccaccagcaccggaattgcagcacctaccattttgcgggaatcgcccagcagggagtcattgatacgctgggtaacattcaccagggcagtatcgcctaatttcagttgtgctccgctgccggatttgtgaacgatatactcaataccgcccggtgtttttttaacacctgtaccgcaactggctaaaagaaagcctaaagccgcagttgcaactaaaaactgattgttttttttcatttgattgtattagtaggttgaaatactttatttacagtttattgtaacaggtcttcgttctcttccacggctttgataaagcggtccactgttttttccagcggatcggtgctgcggcctccggaagcgttgaaatgccctcccccgtcgaaatatttgcgggcgaaggtatttacgtcgaagtcgccttttgagcggaacgacagcttcacttctgagttacggtcaatgatcaaagcggccatcttgatgccctgtatagacaacaggaagttcacgagtccttcggtgtctcctgtctggaggtcgaaccgtttaagatcggagtacgggatggccagcatggcggtattatattcatagaacacttccatgcggttcagcagactatgtccgaggaagcgcaggcggttttccaggaagttatcatagatcgcctggtggatcacctcatgtttcagtcccctttccatcaggtcggctaccatacggtgtacggctgcggaagtagatgcaaaacggaaagaacctgtatctgttacagtgccggcataaatacactgtgcaatttcgaggttaatatactgctcatctcccaatttatatatagtttcataaactaattgggcggtggagctggctttggtatcgcttatgccatactcaaagctgggctgtggctccaggtggtggtctatcagaattttgatacagtccagtttttccaggtgcggcgccaggtttttagtgcggtaaagcgcgttgaaatccaggcaaaacaggagatcgatgccttccagcgcctgaatggcccggtccatagaggattcgtagtcaatcacgtcgtcggctcctggcatccatttcaggaaatccggaaaatttgtaggtgagattacagttacctgatgccctttctgtactaagtagtgatacattgctaaggaagatcccatggcatccgcgtctggcttctggtgcattgtaatcaccactttcttagggctctccagcaaaggcttaatttcctcgatcggcttcattaaaaaactgtaatgttaagagttgatttccaatcacaacaagtggttgaaacagaaaacgaagtgcgaagatctttatttgagccagaatttcaaaattttttaccactaaagaaaatgtaattacttttgcggcctaatctgtaattcggaattaaacattatatgagcaacagaacatttactatgatcaagcctgatgcagtagcaaacgggcacattggcggcattttaaacatgatcaacgctgcaggtttccgcatcgtagccatgaaaatgacgcagttatctattgctaaagcaggtgagttttatgcagtacatgcggaaagacctttttacggtgaactggtagaattcatgagcagcggccatatcgtagcagctatcctggagaaagacaacgccgtagaagattttcgcaaactgatcggtgctaccaatcctgccaacgcagaagaaggtaccatccgtaaaaaatacgcagagtctatcggccgcaatgcggttcatggttccgactctgatgagaacgctgctatagaaggtaacttcttcttcagcggtctggagaaattctagtcctgacgggcaaaatcattacaaaaaggtcagcttcgaaaaagctggccttttttatttgccttcaatgttttgcttcatgataacacattcatttagattaatttacacaatctataagaagtaacactttagatataatgcaaaagctgacaaaaaggcgtaatcacatgatttttaatgaaaatatgagccccgaaaatcagcaaaaatgaacgttttaaagaggaaaacagacccgttttacatccttatatacatttcattatcaaataattacaacaaaactccatcatcttactttaagtaaaaccactctcctctttttcactccagaaacacctgtttttcctgatattattttacccctgaaaggatatttcccggatagccgtgaccgtagttttgtaaaaagcttttaacttgccggcatatgtgggaatcattccggaaactgtttaaagggtatttaagattagagcggtctatgtctgaccactccgtggaagcatatgtaagggacgtggaaaaactggagcagtacctcctcgctcatggaaaagaaaagctccggccccaggatgtaacatttgaggacctgcaggattgtgtgcaatggatcgccaaactgggaatgactgccagctcccaggccagaactatttccggcctcaaagccttttacaagttcctcctgctggaagacatggcccacgaggaccccacccaactgctggaagctccgaagattttacgcaagctgcccgatgtactcaccttcgaagagattgaaaagatcattgcgcagatccccctggataccgcggaaggtcaccgtaataaagccatccttgaaaccatgtacagctgcggcctgcgggtaagcgaggtcattaacctccagatcagccagctccacatggacgtaggatttatccgggtaatcgggaaaggcgacaaagagcggatggtccccatcggcaaagatgccatgcgccagatagatatttaccggagaaatgtccgtatagagctgcccgttaagcacggccaggaagacacccttttcctcaaccgccgcggcggcgcattgagcagggtgatgatcttccttattataaaggagttgacccaaaaagccggtattcataaaaatgtgtcgccccacactttccggcactccttcgccacccacctggtggaaggcggcgccgatctccgcgccgtacaggaaatgctgggacatgagagcattactactacggagatctatactcacctggaccgggaatatttaagagataccctcctgcgtttccatccccggttttgataccgtaaacaaaaaacagctaccggggaaaggtagctgtttcatttctgctgttagaaggtcacaaacaatcgggtagtttttgccatgataaggaaggtgtattcaaacaatcttattacaataagctatgggttagcaagcggtatttatcctgcttgttcttctttgggttagtaagggtgatcacatcactgaaccagttgccaatctggtctgaggcgcgtttcacccgggacggacggtaaattatattcacattgctgcagggacccaggtcctgccggtggggcatccgggccatcttctcatcttccgcccacagcaattcgttattcctgtaaactttaaagtacacatcgggccccaggttcttgcgtccgggtataatggagtgcaggatgccatttgcaagatgctgccttgaaaagtgcagggtgtagcgtccagcttcgttggtgtgcgcctgcccaatcagtttgccggtgagcgcattatacgcttccactttcagatgaggctgtcctgacgccgccatgtggggttttactacgccggtaattacccaggcgcccgcgttggcgtatatattatgccaggtggcggcggggataacataagcatatgcgcctacgtagccgccgctgttacgtttccagtgcaacaccagtttactcaggtggaagttacgggactgctttgtaccgttctttcccggcagctgatccaggcacagatccagttccaatgcttcggtgaacaggtgtacttcattccaggagaggttgaagttgcctttttcatccagggtggtttccgccagcaaccggtcggccttcatcagtacttcccgggccgacaacggtttcatgtcgttaaaaattccgtggggctgatctgccgcctgcaatacagcagggaggtaaacccggatccgcgcgtttgccaggggctctacgcaatcgttacaaataagtgcagagatgtttccgattaataggtaactcataattttattttttttaaagaaaaaaaaaggggttaacgagcatcacctgatgaattgattctgcatattactaaccgaaaaaaacaaacatggtagaaaggccaattactatgaacttttctgaggacaatagatttaaagccggttgacaatacaaagattaagaactttaaaggagtagtcaagcgtttaacaactgaaaaaaagctttacgtataactacgcaaattgaatatgggaactacgctattcaccttttggttgttttccggcaggtaaaaagtaatgcgtataaatacgcattctgaagtgaagcctacggaatccgctccctttacttaagaggataaaaccgctcaaatgcaatagcacattcaattccacctgcgtaaaaacacagtttcgggttacattaccggttggtggccggattgtatatgcgattatttgtaataattttactgcaaactaaaacttacccacaatgaatgattttccaaaaaggccgatcccttcggataccggcgctttcatttcacttgaagaaatgaccacccttacaaaaaatcacgatgaggatcatgtaaatcagaagtcctttggtacccatgttaaggcgatgtgttttggtaaagacaaaattattgaattgctggaccaacccggggcaacagctctgagaatctattatggtattaaggtagatactgacggagatggaataaaggaaaagaaaatgatcctggtagccgttgatgaagaaggtaatgacatccttcctgcagaaaccaccaatgcaggccccggtggcgtggtatccaaaggcgctatggcgaaaatacttgattcaggattaccttgccccgaatattgtacaaaacccggaggaaaaggataagtgataaataatatcatcaacaaagccatctcgtgaatgtaactttattttttactattttttacagcatggtggggatcgaagcactggtcttgatccccttccttttaaattataagtccctggacttctcgtccaggtgcatatttttttacattttgagctgtattttttttgcaggagggtctgttctggtagaacggtatatcgggaacaacatgtggttcttcagcctcatgcactttatccagtttgtgatcctctctgtatttttttaccggagcatctctaaccccactatgaaaaacattgtgaagtatatgcctttactactactggcaatatttatatttgacctgtttttcatagagggggtacgcgcctttaattccatttcatcgggcgttaagcagctggtagtacttacctatggtctatatctctttttacaactgctgagggacaggaatctcatagaaaaatcgatatacattgattctttgccgatattctggtataattcagggatctttatctttgcctgtactgaatttctattttgcatcagctataaccacttacaggcgcttttcaccaccggtgttgccagaatgggtatgaccatcgcaatactgagtatcaattatattgttggaatgatatcaatgattcttctttatattgggttctctaagatcaaaaaactaagacatgcgaattattgatgttattgtaattggtactacagtaatgttaatgctgggagtcattgtgatattgctggtaatgctccaacaaaaaatggttatccaacataaacttgatatacgtgacaaagaccttcagctccaacgggaacgcctcatcgcagtactccagggccaggaacaggaacgtaaaaggattgcggaagacctgcacgacgaagtgggcgcacaactgtctgtgctgaaactcaacctcggaggccttcagcccctgctgaaaaccggcaacggtgaaacagaacggcttaaggaaaccaaagactttaccgatactattatacaacaactgcggttcatctcccaaagcctgcacccccaggcattggaaaacctgggcctggcacatgcgctggactccttctgcaacctgatgaacaaaaacaaacaggtaaaaatagcatttaaaacagccggcaacgggcaaacggtagaccgcgaaaaagctttaaacgtttaccgtgtggtgcaggaactgatcaataacatcctgaaacatgcgcaggcaacggatgtactcatcacctatcaaaccactccgtcccttcttaccgttaccgtggaagacaatggtaatggcgctttgctaacctctctgcccgcttcccgtgccaaaacaggcagcctgggacttaaaaatattgaaagccgcctcaatattatcggtggaaatattaacttcactcccggaacaccacaaggtaccattgctacgataagtgtagagaattatcagacacctgcacagaatagttgatacttatgttgttttattgctaaattgccatccggttgtgttgaacccgcttgtaacgacatgactcatagtaatttattctgaataaaataatagcaaatcttctaactgtccacctatggcacacataaaagtggccattgctgatgatcacaagatcttccgcagtggagtcataaacacactgattccttatgaaaatatcagcttcgtttttgaagccgacgatggcctgcatctgctgcagaacatggaaacacaacagccggatgttatcctgatggatctgaaaatgcccaatatggacggcattgaagccaccattaaggtaaaggaaaagtatcccgacgtaaaggtcattatactcaccatgtatgaggacgacaacttcattgtccacctggtggaaaacggcgccaacgcctacctgttgaaaaatgcggaaccggaagagatctatgaagccatctgtactacctttgaaaaaggattttattttaatgataacgtaaacctggcactgcttaaaaaggtattacacaaaaacaaacaacaatttaagccaacactaaaaaatgaaatccagctcaatgaccgggagcaggaagtactgaagctaatctgcaatgaactgactacccaggaaatttccgaacagattttcctaagcccccgtactgtagaggggatccgtcaaaaattactggaaaaaatcaacgttaaaaacagcgttggtctggtactgtatgcattccgtaacggattaatagaatagttttaaatacccaccaaatatgagtactatcagaacctttgccgctacagcgggcgctatgctgctgttgtatgccggcactaccctggcccagggcattaaaatgcctgcgccaagtcctacgcagaccattaaacaggacttcgctttatccaatatagagctgagctactcccgtccgctgaaaaacggccgcgttatcatgggcgacctggtcccttatggtaaagtatggagaaccggcgccaacagcgctaccaccgttactttcggtgaagacgtaattttcggcggcgtacccgtgaaagctggtaaatacggtttgctttctattccaggcgctcagtcatggaccgttatcctgaccagcagcctcgatgtaaccagccctgctgcttacaaaccagaaaacgatgtggcccgtgtaaacgtaaaaccggtagctacccctttcagccaggaaagctttaccatcggattcgaaaatgtacgttccaactccgtggtactggccctcagctgggataaaaccaaagtacccgtagtgataaaagcggatatcgacgataaaatcaccgcccagatcaacgatgccatgcagaacgccgaaaagaaaccttacttccaggcagctgtatattactatgaaagtggtaaagacatcaacaaggcggtagaatggatcaacgaggcagctacacaaagccccgacgccttctggatatggtaccagaaagcccgcatcaatgcgaaagctaaaaacgtgaaagtggcgaaagaagcagcgcagaagtcaatagaactggctactactgctaaaaacgacgattatgtaacgttgaacaagaagttactggctacgttaaaatagcgcgcggaggttgtctgactcaggattacactgattttattgattacctggatttgactacttttgattttaaaagatttggggagatataagcggatattttcgcttttatctccccgattcctttataaatcctttataaatcctttataaatcctttataaaatcaaaaaagtaaaatccagctaatcaataaaatcagtgtaatcctgagtcagacaaccttcgcgtatttacaaaatactggaagatccaacccagtaatactaccagcaagcagccgatcgcattcaaccagaggaaggacaccgtgccggtccagtaaattaccaataccacaatttctccaatgatggccgcccagaaagtagcggtgcctcctacccgcttcaggtaaaaagctaccatgaaaataccgaggatcaccccgtaaaaccaggagccaagcacgttcaccacttctatcaaactgcccaggctgccggcaaactgcgctaccacgatacagaatacaccccagatcaatgtccatagcttggatattttcagataatgatcttctgaagcatgttcgttgtacaatcgtttgtacacgtctatcaccgtggtggacgccagcgaattcagcgccgcagcaatactgccccaggctgccaggaagatgatggcaatcagcaatcccaccagtcctttcggtaaactgttcactacaaaatgaaggaatatatagttggtatcattggtgtctgcagtaggatcggatgccttgatgagtgataatgcctgggttcttaccagctgcgaccgatcatcggtttgctgcaacgctttttttgcagaggcaatctgtgtgtggttatctgtttcgagtgcagcagccagttgctttacctgctgctgttttaaggttcccagctcattgtactggtcttccagtttcagcatcgccgggccctgttcggttttatgcacccttgccagctgtgcttcattgaagaaaatcggcgcacggaaatacaggtaaaaaacaaataccagggcgcctatcagcaggatcaggaattgcatgggcacctttacaagaccattcatcaggaggcccatacggctttctttgattgattttgcagtaaggtaacgacctacctgcgactggtccgtaccaaagtacgacagcgccaggaagaaccctcctatcaccccgctccagatgttgtatttatccttccagtcaaatttcgtaacaatcacattcagcttgtccatttttcccgacacctgcaacgcctgcttaaaaccaatatcggccggcaacaggtgaacgaccatccagcccgcgaggaacatacctccgaaaatgatggccagctggaatgtttgtgtgtaggccacagctcgggtaccgcctgccaccgtataaatgatcagcaatccgcccatgatcatatttgtccagtacaggttccagcccagtaaagaagacaaaataatagaaggtgcacagatactgataccggtagataaaccgcgttggatcaggaacagggaggacgcgagggtacgggttttcaggtcgaaccgttgttccaggaattcataagccgtatatactttcagtttatggaagatgggtacaaacgtgatacaaagcactaccatcgccaggggcaaaccaaagtaatattgcacaaagcgcatcccatccgtatatgcctggccgggcgctgatataaaggtgatagcgctggcctgggtaccaatgatcgacagcaaaatgatataccagggcatggactggttatccaggaaataactttccatgtttcgctggccacggcttttccagacaccatagcatatgattacagtgagggtaccgatcagtaccatccaatctaaaggactcatgaaaacgttttggtgaataagtagaagaacgctaccagtaacagcaaccaggctgttaccaatacgtaccaccacgtccatgacgggaacaatggcggcttttcttcctgcaggttatctgctgccataatttaatcgtttgagttgcttttagtccacatgctgctggtcaacaatcccaacgcaataccgatgatcaatcccacctgcacgcgcttgatggtaaatccgatcagcaaaccgaggataatacaaaagccagcggcgatcttcagcctgggacgattttcttgatgcttcttactcattgtctttcatccctattttacagaaatcaggtttacaaataaacgataggcgccaggtacgcctgcaggcagctgcctgaaaaatgataagccggtgtacacataggctcctttaccgtaatgagcaacgagggttgatccatcgagcggtccttcccctttgtcgttcatgctgaaaggcttatcataagctttgtctgcattagcggtgtaatacaaacctctttcctgtacccaaccgttaaaatcggcggcagtaatttcatttggataatgcagcaccggatctttcgggttgttaaatgttacagcggcattttcatccgttaccctgtcgcgcgacaatccaaacggatacggtcccaggttgcctgttaccagcggaccattcacattgtactggatcaccagtttgccgccgttgtttacgtattccatcagcttcggctgccagtatttcatacgtgcgtttacgttataagcgcgcactccggtgatgatggcatcgtattgctgcaggttaccgcccataatatctttttcacccagttcggttacatcgtatccaacctggcggagcgatgctgccaccatgtcgcctgcaccgggaatatacccgaggcggttgccgttatgtttcaggttaacggataccagcctggcctgcgctggtggaaacagggtgatcagcggaatatgatcatagcggatctgctgtaagctctgcgtatattctttaccgttacaggtcattacaaccgtgagggtatctgcatgattttccgctacgcctttaacgggtttgatatcaaaccggaattccacctcatctcctttctgttttaagctaaagggctggctgttgccatcggtgaagccggcgggcaattgcagacgtacagttccctgtacgttatcagccatcgcgcggagcttcacaggtaccgactgcgctttggtatctgtaaaaatatatacctggttgctgagatcggctactaccggcggcgctatcaccagcggctgatacagctctccctttacagggtcggtatatttatattgtaaaggccgtgcaatggtaaatggttgtccgccgatagtcaggtggatttgcgcctgcagtgcaggaatattttcaggattgcccaccagcagcggatcattgatgatgtaagtacctaccgggtgcgcgtctgccagccaataaggctgcgactccggcgtgccggcgggtacctgcattgttttggagatgctggtgaatttattaaaggccagtggttgctgatcgcctgcattggtattgccgggcagatcaatcttatccagcgttatttttaccggtcccctgttgatcagttgcacggtggcttccatattggttccgggcactacggtaggtgaagtgctgtaggcttctgcccacaggcctgcgcatgcgtagatcagttgctcggtttctttcagcttcagatcacgccagtacccttccggtaatgagcggatggcgctgcgtatttccagcagggcgggcacggaggccgcaggatcttccatattgtaggccgcgagggcggcgtctaccagggcgcctactttgttgccgccgggaatccttgtccagctggtattgatatcgtcgagtaaactgtttttgggtgtgttgcctttaatcgtcaggaaatattcctgcgagctgcccctggctgccgcaacgccaaatccctggcttttgtgctgggagcggctttcggcggcaatctcaccaaagccttttccaagcaatggattataggcgcctacatctattttaaactgatcgtcggaggtagtgttgacattaccgaagctaaaggtattccagaggatccgtttggcctgccagggttttacccgtgtcagctgttcgggaaagcgtttgggatcggctgcggcgctataggcttcctccgccagcatggccgaagcggtatgatgtccgtgtccggcgcgactgtcggccgggaagcggcaaatgatcacatccggttgaaatttgcggatcatatatactacatctcccaggatctgttccctgttccagatggtaaatgtttcctgtggatttttggagaagccgaagtcctgtgcacgggtaaaaaattgttctgcaccatcgatgcggcgtgccgccagcagttcctgtgtacggatcaggcccagtaactcggactgttcattgccgaccaggttttgcccgccatcaccgcgggtgagcgacaggtagccggtgcgatatagtttttcctttgccaggtaaccgagcaaacgggtgttttcgtcgtcaggatgggcggcaatgtacaatacgcttccaagcgtatctaactttttcaattgcagttttatgtcggctgcgttccatacaggcgaaggctgtgccaatgcgggtaaacccaatgctgccaataaaattataaccagtgcggtagatcgtcttataaacatttgttggtacgtgaatttacagatggccaaaagtaataattaattagtgggacgggaagataaatatgatgaacgtagcagaacgcaggatcgcagtatcttcaatacatatacgaacagtagctgtatcaaaaccgaacaatttaaatatattctaaatatacattcttttggtttatagtggtcccggtcagtggcatctcctttgggcaacacgaaccacatattctctgctatgataaaaaactacctgaaggttgcctggcgtaatctgatcaaagaccgccggtttgcttatctcaatttaattggtttatctacggggcttgcatgtgcgctcctgatctatgtttgggtacaggatgaactgagtatcgacaaatttcataaaaacgacgccacccttttccaggtattggaaaacagagtacaggcgagcggtatctggacggcgaaatcctctcctgtaccaatgcccgaagcgctgaaaaaagacatgcccgaagtggagtatgccgcctatgtctctcccgtgagacaatccacactttctgtaaaagatgatgttggcataaagaccaagggtaaatatgcggacaaggattttttcaatatgttctcttttgatctgatggaaggaaatccaaaccaggtgctggctgatccaacagctattgtgctatctgatgttatcgccacaaaattgtttggtaccaccgaaaatgtgatcggcaaaacggtcgacttccagcatgagcaaaaatttgttgtttctggtgtgtttaaagcacctgatcaacattcatcggaacagtttgattttgttttacctgtccgcatgctgaagatgataaaggaaaacgctgatgaatggggcaatacaggatactacacgtttataacgctaaaaccaggcaccaacatcaacaagttcaatgctaaaatcgccaactacattaagcttaaaacgaacaatgagattacctaccgcacgccattcattcagcgttattcagagaattatttgtatggccgctttgagaacggtatccaggtgggaggccggatagattatgtacggctgttttccattatcgccatttttatactggtaattgcctgcatcaattttatgaacctctctactgcaaaggcagccggaagggcaaaggaagtaggcatcaaaaaagcgatgggcgccggccggggtgtacttatgctgcaatacctcggggaatctatggtaatggcttttgcatcgctgctgatggccattttacttgtgttcctgttgctgccggttttcaacaatcttacagggaaacaactctcgttgttccattttgataccgcactgatattatcaggactcggcattacattctttaccggtttagtggcaggtagctatcctgcgtttcatctttcagggtttaagcctgctgccgtgctgaaaggaaagatcaatggttctgtgggggaactgctgatcaggaaaggattggtggtgtttcaattttccctctccattgtactgatcgttgcggtgttggtggtgtaccggcagatcagctttatccagacaaaaaatctgggttacgacagggaccatgtaattacgttcgcgaaagagggaaaactgtcacggaatgaggtaagtgaacgttttcttgcagaggtgaaagatataccgggagtaaaaattgcttctggtatggggcatggattaaccggtcatagcagcggtacctccgatgtagtatgggaaggaaaggatctgaaagatgaaaccgaatttgaagtggtggatgtaaattatgacctgctgaaaacgctggacattaagataaaagaaggccgggatttttcacgcgactttggcgctgacacctccatgatcatctttaatgaagccgccataaaattcatggggatgaaagaccctgttggaaaatccgttaaactgtggggtaaggatatgcggattggaggagttgtgaaggattttcattttgaatccctgcacgaagaggtaaagcccttgttttttgagctgtctccggaaaatgccaaccggtttatgattaaagtagagacaggccgggagaaagcagtgattgccagattacaggaaatgtacctgcaaatgaacccggggttctcttttgattacaagttcctggatgaaagataccagaccttatatgccgcagaaaaccagatctcccggttgtccaggtactttgccggtcttgctattctcatttcctgtcttggtttattcggactggccgcctttacagcgcagcggagaaataaagaaatcggcatccggaaagtactgggcgccactgtaggtactattgtgatgatgttgtcgaaagatttcctgcgacttgtattgatcgctatgctgattgctttcccggtggcctggtgggctaccacgcagtggctgaaagggtttgcctatagtatccgtatagacgcggggatatttgtagtagcgggtatttccattatcctgctcaccttcctgaccatcagttttcaatcggtaaaggctgcattggctaaccccgtgaagagtttgaagtcagaataaatagaaaagtcccggtgagaaccaccgggactttatttcttcataagcaaaaatccaaccagctcgtaagcaaaaaccaattattaacaaaggcggtttagatttaattgtaaccttcgttctgctggttgcgtatgttggggttagcatccagttctctttgtggtatgggcaatattactttcgtactaggccacgctaccggtatcgttttgtcactcgccaggtatttggtgaatgaacgttttgttctgattaagtcaaacagccggtgtccctcaaaggccagttcctttcttctttccaacaggattgcgtccaggagtgcaggtccggtaacggttaccggcggtgcattatggtcggcgcgttgagccaccagttgcaggtcagcctgtgcttccgcggtgcttccaaggtgtgcagcggcttctgcacggatcaggtataattctgccagccgcatcactttaatactttctgtgaatgtgctcacatctttgtatttggtgatgatgtttgccgggtcttcgccaccgttgccggcgcgtttgcctttcagcagaaagtcccttcttacatctgttgcctggtagatattgtagatgttattcgttgcgagtacatcaccatatccatcctggctgaacatataacttaaaccatctgtgttccggttatctaccggggtattgatgatttcaaaaacggtttcattgttattggtgatcttaaaatcgctcaccagttcttcgttgggcagcagtgcgtatttgttggaccggatcactgcatccgcataagttgcagcgccctgccagtcttctttatacaacaatatcctcgacaacagcgccctggcggaatacacattaatacgtccggaagagaaagccgtgcttttgctttcttcaaacctgctgatcgccgtggtaaggtcgcggatgatctgcgcatacgtatctttcatactactgcgtgaaggcgactgcacggaatccacgttggtgatggtcacaatgggaatccccatgtgcgtggccccgggcgtatagttataaggctgcgcaaacatgcgcgatatatcaaagaacacctgtgcccgcaatgcgtaagcttccgctacaatctgttttgcctctgcgctgtctgccgccgatggtaacagggagatgttgggtcccttcataattaccatattggcattggctactacggcgtataactggttccatgaatcggtggtatactggtcgttggcagtaacaatgtactggtcctggttacgataccggttgctgttgatgacgctgataaatccattgtcggaccggagatcaggcagcagcggcatggtgcgtccgtaataattttcattctgcatcagcgaatacacgccgttgatggctgcccgcagtccgggcagatcggtaatagcgcgaccggtttctgttgactgatccggcttctgatcaaggaaatccttgctgcaggcgccgagtaagccagccagtaacaggagtacgccgtatgtatatttcttttgcatgaataccttaaaaatttacatccaaccctaccaggaaggttttaaataccggcggacgctgatcataatctcctgttaccggtacttccgggtccattgtgagatacttatcttttacatacgtccataaattattgccgcgtacatatattttcacttcgttgatattggctttcttcaaccagtcttgcggcaggttgtaagcgagcatcacgtccctcagccggataaagctgccgtcgtacaggaaccgggatgagctctggttgcttaaaccggattgtgtgccaccgaatactaccttgggtacgttggtgatatcgccgggtttctgccagcggttttcatagatgaggcgcgacatttttgcgcctccgccaaatccaccactgccatctgattctgtgaatgttccccagttgtcgtatactttgtttccccagttataaaagaactggaagctgaaatcaaatcctttgtagctgaaataattggtaaggccgccataaaattttggcagggcgcttccctggttaaacctttgtgcttcgccgtaagatttggtggtagcggttttagacgcatctttataccacagtgcttcaccggtttgcggatccgcccctgcgaatcctgcgagaaaaaactggtagaaatctgttcccacttctcgtttatacgggatgccggtaattggattatccagccgggtaattttattattcagcgttgagatgttggcatctgtacgccatgagaattcattttcattttttgcgatgatgttgcgggaagaaagggatatttcccagccgctgtttttcatctctccattatttctgaaaacagtagtaataccatttgcagaagataccggtacattgagcagtaaccttgaagtggttctgttatagtattccaccgaaccggacaacctgtttttaagcagggcaaaatccagtcctatattaaatggcctgttctgttcccatgtaaggaaaggattgggatattgcgtgagcacataccccggtttcccatcataatcatttgccggactatacagcgacaatgaagcataattatcaatagcctggtttccgttgctgccgtagctggctcttatctttaattcgttaatgacgtttacattccggaggaatggttcccggtagatattccacgcggttccaatggaccagaatgcggcacttcttttctgacggccgaacctggaagaggcgtctctccggatggaggcggtcagataatatttctgctggtaatcgtagctgttattcagaaacaatcctgttaatgaatttgcgttggatacagaggatacactttccggtttggaagcatcggccagcagctgcaggtcgggcagcaggttggaggctgctgaggagttaccgctgttggttgttttctgtgcttcgtatcctacaaaagtattgattccgtggtaaccccatctcctgttgaaccgcaggatatttgtagatacccagttgttccacaggttgttgtttaccgatacccagccattggtatttcttccgtcgccaaatcccggtgcaaaaaatgaattgctgcgggcgtagttcaggtcgaggctgatcttcgtttcaaaggaaagaaaatcagtgaatgcgtatttggcgccggccccgccgagcaggccatagatggtacctgtgcgggtatcgccattcagtactgccaccgggttaaaggtgttgttgtagctgaagtcgtagctgccatcggcgttataaattttcagccagggttgcaggcggacgagtgagcgtaccgggttagccatcagtcctacatctcctactgcgtttgcacgctggtaggataacgacaggttaacgtcgaatgataggcggttggtggcctggttgctcaggttgagcttacccgtcatacgtttatagtccactcctttcagggctgatttggaatcatataagccgccggaaacataaaattttgttttattacttccgcctgcggcagatagattggcttgtgtatagcctccatggcgggttagcacatcgatccagttggtattaacggttgtatccacgccacgtgcgcggagttcccgttgaaaaccggcttcccctgtgccatctgctttgtgcgcccatccttcgcggaggagttccatcatctcgttggtattgagcggatagttggcctgcggaatggtgagctggttgctgcctctttgtatggttgcgccgatctttgttctgccctggctgccggttttcgtcgtaatcagtattacgccgttggcagcgcgggagccatagatcgacgcagaagctgcatctttcaaaacagagatagaagcgatatctgcgctgttaattcctgccagggaattaacattataatcggtgaggttgtctgttaccacaggcgtgccgtctaccacgtaaagtggcgagctgcctgcggtaatagagcctataccacgtatgtgaatactgggtatggatccgggctggccggaaccattggtagattgtaagccgggtacattgccttgtaagctttcctggaagctgctacggggcgctttatcatacaatgaagcacttaccatagtagctgaacctgtcaaagaactttttgtttgcacgctataagctactaccactacttcgttcaatcctttggaatcgtctttcagcatgatgttgagatgagccgtgttgtttaccgtcacccgctgttcttcataaccaatgaaagaacagatcaacgttgctgaggaaggcgcttccatgtggaatgctccgttctcatctgtagtagttcccttattaagacctgcaatacgcaaactcacacctggcaacggatgtccgaaaacatctgttaccgttccgttgatactgacattcctgatctctttgttttccggtgcaatagccaccagggtggcagaaagctgtttaaacgtgaggccggtgtttttcagtatcttctttaagatatcttctgtcaaagcattggtttcattcaccgacacttttttgcctgcgggaataagatcgttgcggtaaacaaaacggtaaccgcttttcttttcgatcatcttcagcagccgtgtcaatggcaatgaatctgctttgatggaaatgcgccggtcctgttgaccgaagacattcccagttatttgcaaacaggtaataagaataataaaggacaccagtttcattatcagtacaacttttccctatgtttttagacgcaaaaggattacataatgtatgatttttttccatacatttaggttgtaaaaggtcataaaactacgacaggactacattgccaagtgaagctaactgccgtttgatctcaacaaaaggggtaaatgtttgcagcatttgcccttttttttatatgagaggtatcgattttctgttgacttccacccctttactgggtaataaatacttcattgcttactattctgcaatgaaatgatgttgtaaccttcagcgcttccagtacttctgaaaacgattcatttttaaaagtagcggtgaaatggtattgttttaatttgttaccgttgagatggattttgataccataccaacgttccattttcagcgcaatatcttcgaagttatcattgtcgaatacgaggtagttgtcgcaccaggcggtttccgccaccatgctgtcctgcgtgttactatgaatattttccaccttgtagcctgccaccaggttgggttgtgtcaatttatctgccggtgcgtgttgtaagatgatcttttggttaggcgttagtttcacattcctttccatgccgtcattcaagattacttctacggcgccggtgatcagtgtagcttctgtggtttgatcccctgtatatgcttttacattaaaagaggtgcccagtactttgatatccatcctggaagtgtggatagaaaagggtttggctgcattcttcgctacatcaaaaaacgcttctccttctaaagtaacctcccggttttccaggttgttcatatcaggattataggttaaacggctgccaccattgagccatacttctgttccgtccggcagctgtgccctggagcgggaaccatcgcgggtataaatggccgccatagctgctttaccggctttttgcggatattttattgataagagatagatacaatagcctcccagcatcactaccagtacagaaagcacggccacccatttgcggaagttccttttgactttcttaacgggtaattcctcctgcggaaactcctcttccattctcacgaggtgtttttccaatgcaagcccggtcctggtttcccattccttattgccggccggttggggccagttgcttaatacagataatttatatctcagatccggatctttctgcaatgatgcttccagttcacgcaactcctccatcgtggcctcgcccgatactttccttcccatcaaaagccatattctttcctgttccatgtgtatgatacaaaagcatgattatatagaaggacaagtaaattgcaagaatctactactccacctaaaaaaaaaattaaattattttgttttgataaaggagaggttaattacctcgctgatttttttgagtgcctgggccatgtgaacatcaatggtgttcacagaaatatcgaggatctgggctacctctttatatttaaggccatcttcgcggatcagtttaaagatcatcttccttttgggtgggagtgcgtttacggcggcttctatcctttttaccatttccccggaaatgaagatctgttccggcgtggcgtaactgacgctgatatccactgccacttcatcgagactgaaatgttgcgtgcgggcttccttatttaagtagttgagggcaatatttttggtagatacatagaggtatacccggaggttatctacctggagcagacgttcgcgctgcttccagacgttcataaacacatctgacgcaatttcttccgcagactcccaggatttcacaatagaaaaggcaaactgactcaatggtttgtaaaacaacctgaacaatgctttataagcctgttcatccccaagagatgccacccgttccaccagtagctgtatattagcttcttccctcaatgatttggtttttggttgaaagttgatccctaaagataatacagattttttcttaatttgatcttgtctaacatctttttttatataatatgaattgatcctaaagcatataagcccgctgctttaataccgcgctactttttaaacataaaatacacggcgccgatgagaaagaaaaacgaaaccaggtagttccatctcaggggttccttgagaaaagtgacggcaaaaatgctgaaaacggtgagggtaatgacttcctggatggttttaagctggaagccgctgaacccctcctgtgcgccgtagcggttggctggcaccataaaacaatactcaaagaaggcaatgccccagctgataaggattactttccagagggcaacatcctggtgtttgaggtggccgtaccaggcgaaagtcatgaaggtattggagatggtgagcaaaataatagtgcgcatgcgtgattcaaagtttgtccaaatctataattttgtaaaataatatcccgattatttgttcacctgtattggtatctcagggcgggacctgtaaaccttaaacaggattatctgacaaaagtgtaaacctatttcaggacgatgccaccggcatagtgtattgggagtgtatgggaagtgtatcatgagtgtatcatgagtgtatagggagtgtatgggaagtgtatggggactatatggggagtacgacacatacgctactcctaagtatccgagaagtattggagatgtatcggagaagtatcccagaagtaacagctgtatcataccggcgcccggatccggactgcttctgttcagaagcggacagtaaaggatctttatcgatttgataatcaaatcaatataaaaaggcatgtttttgggcgatagttacccgcaaaaagccaattggtcagtatgttcaaaaattatctgaaagttgcctgtcgaaatctgctaagaaacaggaccttctcctttatcaacctcactggtctggccgtgggattgggttgctttttgttgattgcactgtatgtgctggacgaattgagctacgaccgttactacaataaagcaggagatatttaccgtatcaacgcggatgttcgttggggtggccaggagcttcgggtggctgagacttcagatatgatgggccctattctcaaagaggattatgcgcagatacaggaatacacccggatttactcccacagtggcgacacgaagctgatcaggaaagggagcgaatacatcaccgaaacacgtacggcttatgtcgattcaaccttcttcaacgtctttgcattcccggcgctggaaggcgatacccggactgcgttgaatgtcccctatgctgtggtgatgacggcatcggccgcggcccgctatttcggatcggccaacaatgccatcgggaaaacgatcgaagtccaggacggcggtaaagacgttccctataaagtgactgccgtgatcgcgaatataccgggcaatacccacttccattttgacctgttgttctccatgcaaagcctcgattacaaatggggacagataggcaatgtcaattttcacacttacctcctcctcaaacctggcaccgattacaaggcttttgaaaaaaagtttcccgcttatattaagaaacatcttattccggccatgaaggattttcagatctacagtatggcagacctggaaaaatcggggaacggattccgcttttcactcattcctgtaacacaaatacatctgtattccgacagacagggcggtgaagaattgagcccgcccggcagtgttcaatatgtcgccattttttctgccgtagcgttgttcatcctgcttattgccgtcgtcaactttatgaacctgacaacggcgcgatccgccggcagggcgcgggaagtgggcgtccgtaaggcattaggaaccgcacgcggggagctggtgatgcagttcctgacggaatccaccctgatggtgttcctgtcgttattgattggtatcgggatcgccttcctggcgctgccccttttcaattcattgtctggcaaaacaatgaccctggccagtcttttttcgccggtgattctcccattgctgattgcattgccttttgcggtgagtttgctggcaggaagctatcccgcttttttcctgtctggctttaaacctatcgaagtattaaaaggtcagttgaaggcgggtacaaaaagtggatggctccggagcaccctggttgtcgtgcagtttaccatttcaattgtgctgatcattgctacaatcgtcgtgttcaggcagctgcgttatattcagacacgcgaccttggatttaataaggagcaggtattgattattgatggtgttgatgcgctgggcaataatgcggatgtttttaagagggaagtgacgcaattgtccggcgtgaaagcaggaacactgagtgcctttttaccggtttccaaatcggcccgcaatgtatataatgtcttcaaagaccctgttcaaaccgcatcaaatagtttcaatgtagaaacctgggcgatcgatgacggatacttttctaccataggcatcaaggtcttaaagggaaggaacttttcccccggtttcaccactgattcgtcggctgttatcatcaacgaggcggctgcgcggattttaggctacgccgatccggttggaaagaatatatataccttcaacgatgccggaaagccaaccacttacccggtcataggtgtagtaaagaattttaattttgaaacattacaccatgaggtccgcccgctcatgttcaccttgcaaagaagcacaggcctcgcctcttttaaagtaaatacttcgcttattgccccgctgatcggagaggtccgggacaaatgggctgcactggcgcctggcataccttttagcttccggttcctggatgattcttttaacgagatgtaccaatccgaacaacaggtcgggaagattgccactatcttttcggtattggctatattgatctcctgcctcggtatgttcgggctggcgacttttgtggctgaacaaagaacaaaggagatgggaatccgcaaggtattgggggcaagcatacagggaattgtccgtttgctttcggcagattttataaagctggtggccatcgccttcgttattgccactcctttctcctggtggatcatgcgtaaatggctgcaggactttgtttaccgggtaaacttcagttggtggattttcctggcagcgggtttggccgccttgctgattgcattggttacggtgagttttcaggcgatccgggcagcgctggcgaatcctgtcaggagcctcagaatggactgaattttattgtgaaggaggtcagatctgttaaaatcaggaatgtttctttgtactaaccaatagctcccgtacgtctacatctaatgcagcggcgatttcaaataaggtttctatccctggttgaacagtattagtacaccatttggacacgcttccaatagaaacacccagttgttctgccaaccaattattagtttttccctgttctactattactattttaatccggttaaatatttttttagacataaataggtgctttcagaactataaatagcaaaatagcaattatttattaactgaataacaacattatagatatgagcacagcataaattagcaatattataaccaatataagttataatattactaatttaagtatctttattaaaacatttaaccatgcaatcttcttcagccatctttgtttttaaccaaaacccatttcgcctttccgaagaagaataccattctccggaaatggtgttgaaaaactactttgagctatttggcccgggtgaaaccaacgacatcctcgcttctgttcaaacagaagcgcttacaaaccctggcagtccctatagcgctgtgagtgagcgaatgaaagtgttgtcctgttttacagaactaaaccggttaatagaggccgcgtttgtcatctcccagaaaaaataaaagaccacctgcagctaacccaacaatactatcccccaaaacaaatcccaaaatccaaaagtaaaaatcagtcaaatcagcgtaatcctgagaaagacaaaatccgcgcataaaaaaaagagggaccgtaagaggcccccctgcatcaaaccaaaatgggttttccatcatggactgattttgtgttgttggttgctatttcattattaaagactattgttctaatttgatttcgcccaggtcggtagctttaccgtcttctacttttacatctttaactacggcatttttgtaagggcttttaccgagaatagtaatagtgtaagatcctgctttagcagcggggatagtgaatgcaccctgtgagatagcgcctttcagcttatctgtaccattgtctgcttctacttctgtagcactgtcagccggagtaattttaccggtgatagaaccaccttctactactaatactttcagagaatctttaccttgtaaagaatctactctctgtaaagagtcgattccggttaaagaatctacctgtaaagagtccattccgctcagggaatcaacctgcaaagaatccattctgctcagggaatctacctgtaaagaatccattccactcagggaatccacctgtaaagagtccattctctgcaatgagtctattccgctcagggaatcaactttctggagagaatcgattcccatcagagaatctactgtcattaaggaatcaaatccttttaaagagtccaggcgctgtaatgaatcaacactgaaaacttttactgaatcgaggctaacaagggaatctgttgcaattgaatccaccattgcggcggtgctgtctacagattttactgcttttacatcagcacttttgaaagcagacattccgattaccattgttgctaaagcgagcgttcctacaattgattttttcatggcatcaattttttgtatggttaatatttatgatgattatccccggtccggatgaatgtgcatggtttttgttatatgccctcatcgttggctaccgtatataaacaatacatccgacaattcacttaccattagtcaaagaaatgttaaagtgaaaaaaagaattatgaatcagtatactggctgctttcgtaattagtaattttaaaaattatcttcgcactacggaaacaagacaaaagatcaaaagcatgttgcaattgagtaacgacgaaatagtaaaaggcatccggagcagaaacaaagatgtattcgaagctgtttttaaacagttcgccccttctatgtataatatagcggtccggtatgtaaaagatgaagatgacgcgaacgatatggtacaggatgttttcctcaacttgtggaaaggtgcggaaaacctggatgagagagccccggttaatcattatctcgcaagagcgaccgttaacacctgtttaaaccgcataaaaaaagaacaacggaaagaagtatacgccaaggaacaaatgcaaactgccagtccttcggaaaataatcattccctgctggaacataaggagctggaagccaaataccgctctgccctggagaaattaccggaacaatgccgccgtgtttttgaaatgagccgcctgaaaggcttgtcgccagccgaaatcgctgaacaactgaatatctctatcaatacagtatacgcccatttgaccacagctttaaaacgattacgggtagaccttattaataagtcgtaggatacgcctgaaattttttttattatcgcttaatggtataacgttccctggttgtattactaataagaagccatgaataatcaaacagacatagatatagtgatccgttacctggaagatccggacaatgagcagcacaaaatgcagctcaacgaatggattcaacaggatgctggtaacctggacatcttcctggatatgaaaggcatgtggcacggcgatccgcttcctgctgcctctgctttcgacacccagggacaatggcaggcactggataccatgctggataaggttcccgcagtcactgccgcgcttcctgcacaagagcaaaacacccgtgtgatcaggatgaaccgcaggtactggtgggctgccgccgctgtgctgctgatagccggcacatggacctggctcggccccggtggatataaaacctatgccactgcacagcaacaggatagtttgcgtctgccggacggctctatgatgtacctcaacgcgcatacacaggtacgctatgcccgtggatttggaaaagataacagacaggttaaaatagataaaggagaagccttttttgatgttaccaaaaacgatgccctccccttcattgtaaatgcccccgaagtagaagtacaggtactcggtactgccttcaacgtgaaagccgccaacagcggtgttaaagtattcgtgcagtcaggaaaggtaagcgccgcctacaaaggcaaagagaaaaaggtaattctcacccccggtgtggaagcctctctgaagcataatggcagcgaaatagatacccgtatccataaaaagaacaacaatattctggcctggaaaacccggaccttaacttttgacgataccccgctcacagaagtggcggacgcccttgaagatttttataatgtagagattaaaatcagcaatcaacaactggctgataagaaactgctggctaccttccccaacatgtcgctggatgaggtactggacattatgagaaaaacccttcaaattaacatttcgcataaaaacgacctggtagacatctactaatgcgcgcctgaccttttatttatgcagcaattattgctacaggcgcgtatctccaattccaggtttggacgcgtgcctgattttattttcgttgttatcctggtattggccaatgctgtagctatggcccaaaatcctgatgcccctccaagaaaagtttcccttcagtttaccaatgccagcctgaaaaccgtgatccgggaaatagaaaaacaaacaaagtatacctttgctatttcttccggagaactggaaacccgccagggcgttagcttacatgttcacaacagccctctcctggaagtattgccgaagatcttccctcctgccaaatataaagtagagataaaagacggccagatcatcgttatcccgctcaacgccactgcggcagatctcacacctcctcccagcaccagctccaatcctgataaatggacccttaccggcgccgtttccgacggtatgcagcctttaagcggtgtatctatcagggaaaaaggcaccactaacggtaccgccactacggaaaatggtactttcaaagtggacctggccaatgggcaggctatcatccaggtgtcccttatcgggtttgaaaccaaagaaattgccgtgagggaaagaaggagtatatcggtgttgctgcaacctgatctgcggaagctcaacgagctggtagtattgggttatggcctgcagaaacgcgctaatatcacaggcgccattgcgcaggtggatggcgtacggctcagaagccgcccggtagccaacgtgatggccgccttacagggtaccgccaccggcctggtggtgacccgcagcaacggacagcccggccgcgaaggatttaatatacaggtacggggcgtaggctcttcttccggcagtaatacgcctgtggtcatcgatggcgtgcccggttccctggccgtcattaaccccgacgacattgaatccgtatccatcctgaaagatgcagctgctgcctctatttatggcgcacgcggcgcaggcggtgtggtgctggtaactacccgcaccgggaaacctggtaagctgaaagtggatttcaacacccttggcggatttgaaacacccatccggttgcccaaccggctgccctcctggcaatcggccgccatgcagaacaccgccgcggaaaatgccggtcaaaccgccccctgggaccccatggagatagatttaatgaaaacagggaaccactatgcgatcgactatcaaaaccctgacttctacaaatactattataactacaatcctttgccggtgcttaccaaaagcagaaccggcattgaaaactataacctgtcggtaaaaggcggcgacagctccaaccagttctctgcatcgctgggttacttcgggcggcagggactatttgccgttggcccggaccgtacccaccgagtgaatgcccgcgtgaacctgaacaaccgctttagtaaacacttcagcctggaaacgcggttgtcgtacgcccaaaccaataccttctccccttcccagccggtagagggccccaatggcttgctggcaggcattttccggggaccgggtaatgtgccggtgtatgtgcccaataccggcaactatgcctatggcggcgcaccgggatatgctgttttggaagatggcggggaacgcgatgaaaaaaataattatatcgatgcggtatttaccctgcgggccgacagcctcgcaaagggtcttacgctccggcttatttacagtccgcaaaaacacaccctgcgggacgatatgggccgcaataccattgccttatggaaccgggtggataccgccacgctggtacagccgcataatatgctgcagaaaagcaagctggaagcaaaaggcggcaacctgcaactgctggccgactacgacatcaaagaaaataaaaataacattcacctgctcggcggcgccacgcaggaaacatacaacaccacgcaaaacacggcggcatcgtacgatatcagccaggctgaaatcaattccaatcactttaataacgcgcctgcatacacgcagttactggcggccagcggttctttattgtcgatattcggaaagatcagttacaactacgacaaccgctacctgctggaagcaaacctcatagcatcgcgcttatcacagtacagcacctcttttgttggcggcgaacagtggcaggcattcccgtcgttttccgccggctggcgcctgaataacgaaacatggtttaaccgcgcgttgccatttttcaatgagttcaaactgaggtggtcatggggcagattggggaatatcaacagctggaacagtattcctaacgacgaacggttgcagactttcagctttaacaccttgccccgttttcagccttttgtttacaagaaccccatcatccaggcacagggatgggaaaacattgctaccaataattacggctgggatgctactttgttcaggggccggttgaccattgcagcagattattttattaagcataaccgcgacatgcagatcccggtactgacagcctccacagacggggcctggccattggattttcaccggggtgaaatgaaatcctggggctgggaaatcaacctgggctggagagacgaccggggcccctttacctggtatattaacgggaatctcttttataaccgcaataaagtactgaaaaatgataatgtggcgccacaggctggctggaaccagggcatcgcaggatatccttactcttccctgtttggctatgagtctgatggctacttccaatcggccggtgaagtgacgcagcatgccttccagcacgaaaataccggtccgggcgaccttcgctataaagacatcgacggcgataacaaaatagacaatgccgacctcgtatacctgggcagcaccgatccgcagttctcctacgggatcgacgcgggttttgcctggaaaggatttgatgtctccgttttcttccagggagtggccagacgcaaggtgatgcctgatccgcgctataatcttccttttaccggtaactggcagcagccctgggacattaaccaggactactggacgccggaaaatcccaacgcattatttccacggctgtatctgaacgaccagcagaataccgccccatcctcccactgggcaatgaatggcgcctacatccggttgaaaaacctgcaggtaggttataccctgccgccgaactggctgaagaaaatatggatcactaatctgcgtatttatttctccggacaggatctgtgggaaactactaaaatgaaaattaaatattatgatcctgaacaggcgggaggttataacggaaacgtatatccgtttttcagatcatatactttggggctgactgttggcttctgatccggccttatgcactgccattaaaatcagctagtgtgcaatcctgtagcgactcagcacctggggcgctattttcaaatcgggtcgaaagcgcatgataccttttacaaaatgcgccagcaggtcattcccattgggtaccaggaaaattctaaactccaccgcctgcaaccgcaccgctccggattcgtttttgacaaacacatacaaacccggattcgtttcgtcgtaaccccaatcggtccaaagcacgtcgtacgcatcgccgctgctatttgtactcagcgcctcataacacaacgacagcgcaggtacaccttcgccgtattggtgcagcccttccctgtctacccgggcccgcgtataccggggcttgcctgaccggtaagtggcgactgccatccatatcaaagcacataaaaccggcgctgcgacgcctatcgtaagcatccgtgcacctgtttcttttatccaaaaggaaaataccacacctgccagtagcgccgccaggaccaatgcaaaaaaggtcagcaggcatactttcagcacaacggttagccgtcttgcggattttgaattcaacggaggaaaatcgtcttcattgggcaacatagcaggtagtaagtatgtttctactccgttttctttcctgcgagcaggtacaatgccgccatacgtatggccacaccgttttccacctgttcgaggatgatggactgacctgagtctgccacatcagaatttatttccaccccgcggttaatgggtccggggtgcatgatcacaatttctttatttaaactatcgagcaattggcggtttacaccgtatgcgagggaatattcccggagggaagaaaacagcggggtgttttgtctttccagctgaatacgcaacacattggccacatcgcaccattgcagggcttcgcggatattgtagctcacatttacgccgagagcagctgccatgtatttcgggatcagtgtgggcgggcctaccactgttacttctgcgcccagttttttgaggcagtagatattggaaagggctaccctggagtgcatgatatcgccacagatggctaccttcttaccttccacactaccgagcctttcccggatggagaaggcatctagcaatgcctgggtgggatgttcattgatgccgtcgcccgcattgaggatgggcacgttgatgtgctttgccaggaaatgcggcgcaccgctggcagagtggcgcatcaccaccatatccactttcatggataagatgttgttcaccgtatctatcagcgtttcccctttggaaacggaagatccggaggcagaaaagttaaccgtatctgcacccaggcgcttttccgctagctcaaaagagatgcgtgtgcgggtagagttctcaaaaaataaatttacaattgttgtatcgcgaagcgtaggaacctttttaataggcctttgtaaaacctccttaaactggtcggctgtttgaaaaataagctctatatcctggcgctgcagatcgcgaattccgagtaagtgttttacagaaagtgacattaatgtgcaaatataaagggtgaaatctgaattctgaaatccggattcattttagtcaatcagaactacttcgtctttaccatctctttcgttccacaacacccttactttctgggaaatgagggcatcaatggtacgtccggtatagtcgggctgaataggcaactgcctgctgaagcgacggtcgatcagcgtgagcagctctacagccgcgggccggccaaagtccagcattgcgtccagcgccgaacggattgtacggccggtatacaacacatcatctatcaacactacctttttattttctatggaaaaatcaatattcgtttcgttgggtacatgcagggttttgctctggttaaaatcgtcccggtaaaaagtaatatccagtttaccgtaatcgatacgcgctccgggtactaatttcagcaaggtttgatgaatccttccggataaataaattccccggggctgcaatccaatcagcacggtttgctcaaactgtaagttattttctatcaactgatgacaaagcctgtctatcgtaatagccatttgcttgccgtttagtatggttttcaaaacacaacgttttaggggccaaaaataatgattaaatgctacagataaaaagctgaatattagaaaagattgataaacaagggaatcttttctaaaacagggctgttttaaaacaggcttgctgccttatagttacacaaaaaaatcaatatgacccgttgctcctctactcttcgtactttagcagtatcaataaacggggtatgaaacttttaaagatcattttagctatgaccgcctttctgcaattatggggatgtaaatcccagggacaattaaaaacaggggataaaattccagccttttcgctacaggaccagaatggaaaaacttttgatatcaataccgtattaggcaaacagccattggtcatttacttctatccgaaagatgaaaccagtgtatgcaccaaagaagcatgttcattccgtgattcgtaccaggactttcagaagtacggcgcactggtaatcggcatcagtgccgataacgtggcttcgcatcgcagttttgccacgcatcacaatcttcctttcaccctgctcagtgatccgaaaaatgaagtacgcaaattatttggtgtgcctaatacttttgtgataccgggtcgtgtgacttatatcgtagataagaacggcgtgattgtgcatgaattcaattcgctgcgcgatggagagaaacatgtaacagagtcgctggcagcgttgcagaagttgcagtgagtgatgcctcaaggcatcactatttcatttacctgtacagaaagatgtgctgccagttccccgtcatcattatccagtggataggcggttaaatactttagacggcctgtttccccattaggattaaagaaaaatcttccgggattactataggttgtcaatacctttgctgtaagtgatgaattagagaggttaatcagaagtccgaaggtgatctggctgaacttacctaccgcttgtaagttattacctgtaataacaaggtaatcagcattattactatggaatgtgtatacgctattcaacgtaagatctgatgctgcctggttttcattggatgactcccataaccatctgtctatttttctatcgttaatgattagcttaacagcagttggttccgtataacctgaaaaatattcataatgaatattgtactgctcattttgcaaatcgacccgctttaatagtttttctcccatcacttcttccgtctccttcattttaacttccagttctttttcgaaggaacgctgtaaatgatatttctcccgcaggaaattatcgagatccttgacgggaatctcagtgggttctccggttactttgctgaatacaatttgtggggatttgataacctgttttacaggagcaggctgaatgattttatctgcaggttctttgtggtgtatactacaacctgccagggataaagaaatgaagataaaaagctgtctcatgggtatcttaagatactacaactttctcatatccttaaatgtggaaatctcttccttaagcgcaaacagctgcatgccccatatgatccctagcaccaacgcaaaagctaccagcgccagggacaaagacacctgcataaagctgccttcttcgcggttggtaagggtaataacgcggataagggcaatgaggcccacgccaaagaagatagccgctttagttccttttttacgcagctgtttcttaaaatactcatcaaaagcgccggcggcagcgatgctggcttcaggctgcggcgttccgtcggcgagcagtaattgttcaaggtctgctacgcggtaatgctcatgaggtgctgagaagtatttttgtaagatatctgcctgcataattcctggatactgaatgaggatgcaaggtacaaaaaaggcgatggatatagatccaccgcccgcatataaatcatgaacatttactaagcttctttcaggaacgggtaccggtaatcagtagccggtacaaaagtttctttgatgctcctggcgcttaaccagcgatagaggttcagcatagagcctgctttatcgttggtaccagaagcgcgggcgccgccaaatggctgctgtcctactactgcgccggttggcttgtcgttgatgtagaagttaccggcgctgtttaccagggtgcgggtagccagttccactgcataacggtcctgcgcaatgatggcaccggttaaagcatactcggaggtactgtctaccacctgcatgatttcttcaaatttctctgcgtcgtacacgtggatcgttaatacgggtccgaaaatttcctcacacatagtgatgtatttcggatcggtagtttcgataacggtaggctcaataaagtaaccttcagctttgttgtaattaccgccggcaatgatctttaccgccggatctttctttgcattgtcgatgtattgggcgatcttatcgaaagagcgttcatcgatcactgcgttgatgaagttgctgaaatcttcggtgctgcccattttcatagttttcagctccgcaactaattttgattttatatcgtcagcaagattgtttggtatgtatgcacgggaggccgcagaacatttctgtccctggtattcaaaagcgccgcgggccaaagcggtaacggcgatgtcaacatccgctgatttgtggatcagtacaaagtctttaccacctgtttcaccaacgatgcgcgggtaagttttgtatttgtggatgttttcaccgatggttttccacatggtctggaatacgccagtagagccggtgaagtgaatacctgcaaagtgaggatctgcgaagcaaacgtcgccgacaacgggaccgttggcatacacgaggttgataacaccatcgggcaggcctgcttcgatcagtaccttcatgatcacctgtgcagcaaacacctgtgtattggcgggtttccatactactacgttaccgcacatagcggcagacgtgggcaggttaccggcaatagcggtgaagttgaacggtgtaacggccagtacaaacccttccagcgggcggtattctaccctgttatggataccgggggcgcaaaccggctgctggcggtatatttcgctcaggaagtgtacgttgtagcggaggaagtcgatcagttcacatgcgctgtcaatttcagcctggtaaggattcttactctggcccagcatggtagcggcattgatgtgatagcggtatttggtggccaggagttcggcagcgcgcaggaagatgccggcgcgttgttcccagtccatattggcccatttttcacgtgcctccagcgctgctgcgatggcggttttcacatgagacgcatcgcccatatggaagtgacctaatttgtgtttgatttcgtggggagggcgcagatcaacggtatttccggtgcggatttctttaccaccgatatacatgggtatatctgctacttcgcttttgaaggcggctaattgtttctttaatgcaattctctcagcagaaccgggtgcataagacaacacaggctcattagcaggcgctgcgtactcaaagtatcctgtattcattgtatcctaatttttatatttgtttatttgatcatttgtaaacctggaggcgcacaaacaatcaaataaacaaatgactacgagtattgtttccgcagcaaaattaagttatacaacgcctacgcgcttattaataattagtcgatacttattaattattgtcctcttccttctgcatcatcaggtatgctttcacaaagccgttcaggtcgccgtccattacaggtcctacgttgcctacttcaaagtcggtgcgatggtccttgatcattttatacggatggaatacgtatgatctgatctgtgatccccactcaattttgcgtttgttggcgttggctgcatttttcagttcttcccttttgcgaatctcttcttcatacaagcgtgatttcagcatggtgagcgctttttcacggttctctccctgcgtacgtgcctgctggcattcgatgatgataccggatgggatgtgcttcaaacgtacggctgtttccaccttgtttacgttctgtccgcccttaccacctgaacggtaaaattcccattccaggtctgccgggttcactgcaatctcgatagtattgtctactaacggatatacatatacggaggcgaaagaagtatgtctgcgtgcattggaatcgaaaggtgaaatacggacgaggcggtgtacaccactttccgctttcaggtggccatatgcaaagtcgccatcaaattccagcgtagcggatttgataccggcgccatctccatactgtgtatcaatttctgatactttccatccctgcttttcgccatacatgcggtacatgcgcagcagcatttcggcccaatcctggctttccgtgccgcctgcaccggagttaatggttaatactgcgggcatttcatcttccggctggttgagggtggatttaaattccaggtcgtccagcgctgctactgcagcattgtaggcctgttccacctcttcttccgttgcttccccttctttgaaaaaatcgttcagtacagcgctgtcgtcaattgcagcgttcacctgatcgtaaaggtctacccaatatttgttaacctttatttccttcagaatcgaagtggctctgacgttgtcgtcccagaaaccgggcgccaggcttagttgtttgtcgttttctatttttgctaatcggtcaggtacgttaaagaaaacctcccaggacatataaacggtccctcatagctttaagttgctctgctgtcatagctggcaaatgtatggaaaaaatggagatatatactaacggctttcaaactttgttgtgattgtttactttagcataatttttgtgttgtaacacggtaaccatgtcactaatattataaaaagcacccatccgttatggtgagccatgaaaccctccactttaaaaaccggtccatcttcaacacgctaggttttattatcatgatagccgcaaacgcactggcagtgctgcttcccatcaatggtaaaacaaccgcacagatttcggaagaataccctaacctttttataccggcgggaattacgttctctatctggagtgttatctatctttctttaacggcatttatcatatatcaattatggttatctttctctaataaacaaccggcaacgctggcatatgtgatgcagcgtatgaaagactggttcctcatttcctgtgtggccaatgcctgctggctgtttgcctggcattatcacctgatacctgtgagcgtggctatcatggtgatcctcctgatttcactgatcatcgtacatctcaactttggtatcggcatcgctcctgctacgctgacggagaaattatttattcatattcctttcagcatctaccttggatggatttctattgccaccatcgctaatatcacggcgctgctggtatacaccgggtgggaaggcagccgccattcccaggtgctgtgggctattgccatgatcagcgtgggtaccctgctgagtatagccatggtgctgcttcgcaacaatatcacctatgcccttgttattgtgtgggccttctatggtatcctgctgaagagaagggctgccgacaccatggatgagaaccccatcatccatacctgcattattgccattggcgtgattgccataacaatttcctggcaattgtacaggaaacagaaatcatgaatctaaaagattatttttgatgcgcatttaatatatacacgactatgtttccatctaccaatccaacaaccaccaaatcgtgggacgccttaaagaagcacgctgaagaaatgaaaaaggtacatatgcgtgccttgtttatggaaaacaaagaacgcttcagtgagttttccctgaaatttgaagacatccttttcgactactccaagaatattattacggaagatacccgcagcctgttattaggactggcagcagaatgcggcgtaccggatgcgatcaaagcgatgtttggcgcagaaaaaataaacgtgacagaaaaccgtgctgtactgcataccgctttacgcaacacgtcagataaacctgttttactggatggccgcgatgtgatgcctgatgtaaaagcagtgctgaacaaaatggatcacatctgccggcagatacactccggcgaatggaaaggatacacgggtaagcctatacgttatatcgtaaatatcggtatcggtggttccgacctcggcccggtgatggttacggaagcgctgaaaccctactggaaacctaacatacaaacctattttgtatctaacgtagatggcacacacatcgccgaaaccctgaaaaaagttacaccggacgaaaccctgttcctcatcgcctccaaaacatttaccacccaggaaaccatgaccaacgcccacactgcgcgcaactggttcctggaacacgcggaagatgagaaatttgtagccaaacattttgccgctttatctaccaacgaaaaagcagtaacagcctttggcatcgatccaaaaaatatgtttgaattctgggattgggttggcggccgctattccctgtggtccgctatcggcttatctattgcactcaccatcgggtacgacaacttcacgcagctacttgatggcgcacatgcagtggacaggcacttcgccgatacaccaccggaacagaatatacctattatcatggcgctgattggcctgtggtatggtaatttcttcggcagcgccacagaagccatattgccatacgaccagtacatgcaccgctttgctgcttatttccagcaaggcaatatggaaagcaatggtaaatccaccgatcgtacaggccacaccgttagttatgaaaccggccctatcgtttggggcgaaccaggcaccaacggtcaacatgctttctaccagctcatccaccagggcacccgcctgattccctgcgactttatcgcaccggctatcagccacaatcccatcggtgatcatcatgtgaaactattgtcgaacttttttgcacaaacagaagcgctgatgaatggtaaaacggaagcagaggtacgtgctgaactggagaagtccggcgcttcggcagaagaaatggcgaatatcctgccatcgaaaattttccctggcaaccgccccaccaattccttcctggtaaaggaaataaccccccgctccctgggttcactgatcgccctctacgaacacaagatctttgttcagggcgtgatctggaacatttacagcttcgaccaatggggcgtggaactcggcaaacaattagccagcaaaatattacccgaactggaaaacaacgacatcatacttaaccacgatgcgagcaccaatggcctgatcaacgcgtggaagcatatgcgcacggcgtaattgttcgcctccggcgaacgcggatgttgtcttggctcaggattacgctgattttactgattagctggatttttactttttgattttataaaggattaagggagatagaagcgaatatatcgcttttatctcccttaattattaatctaaaaatccaaaaaaatccaaaagtaaaaatccagctaatcagtaaaatcaacgtaatcctgagtaagacaaaatccgcgtaataaaaaacccccggagaaatccgggggttgcctattattttttgtaaaaatctttaagtaaaaatcttaccatttgtctacctcgtctgagctatgtgaagccggggcggctactgacgcctcaacaggtacttctacctcaacaggggcggctattgaagcgctaacttcaactccttctgtttctgtttcgtcctgttcttcctgcacataatcatggttgtaggcatcaaagtcgaaatcgggcatcaactccgttttaacatagttgatggtttcggttagtgcgttcaggaacttgttgaagtcctccttgtacaggaatactttgtgcctgtcataaccgttgtcattaaaacgcttcttactttctgttatagtaagaaaatagtcgtttccccgagtggtctttacatcaaagaagtacgttcttcttttgcccgctttcaatcgtttagaaaagatgctatcattgtttctttcctgttgattgttgttttcgtacgccacagttgatagatttaagtgttaacgaatcaaatcctgttacaataagagacaaatatactattgttttacaaatatcaaaatatttttaaatgattttgaaaaatcataaaagccgcgtgtaacgggctgcggcagggaatatacaagcacgtgattgctactcacttacactttcttcgtcgccggattgctgacgcgcgtacagctctgcgtagtatccgttcaatgacaataaatcattatgtgttccctgctctacaatttttccttcatcgagtacgattatgctatcgaactcaaacaaggcaaatatccggtgagtgatgataatggctgtcttatttttcagataggcatacaggttacctataatctctttttcggtacgggcatcaacggcggagaggcagtcgtcgaaaatgaggatgtccgggtccttgatcagcgccctcgcaatggagatccgctgtttctggccaccgctcagcgttacgcccctctccccgatggcggtatcaaagccttcattgaaacccaggatgtctttctccacggaagcctgcctggcagcggtttgcaccgcctggatactggcgctaggatcgccaaaacggatgttattggcgatgctgtcggaaaacaggaacacatcctgcggcacataactgatctggctacgcaaatcggccagccgcaggtgacggatatcctggtcgtctaccatcaccttcccctcctgcggatcgtacatccggataagcagttgcgccagcgtacttttgccggacccggttctgccaataacggccaccttctgccccggtttgatatccaggttaaaatcgctgatggcggtaatccccgtatgcggataagtgaaagtcacattttccagccgcacccctccttccagtttcaccgtttttgcatccggttcgtcctttaccgtaggcgctatctgcaaaaattcgtttatacgttgctgtgaggccgcagcacgttgtatcatggacgccaccatcccgatagaaaagaacgggaacatcagcatgtttacatagatcacaaattccgccaggttgcccacagtaatatttcccttgattacctgaataccacctatgaaaatagtgaggatcacgctcaggccaatcatcagcgccatagtgggctgaaacagggcgtctgttttagccaggctgatagagctgtctttatacgcttcgctcgcttcttcaaaatggcgcgcgctggcatcttcctggatatatgattttattacgcggataccggaataagattcctgcgcaatggaagtaatattggataactgcgactggatcttttcgcttttgcggtgaatgatcctgttcacataataaatggttaaggcaaggaaaggcaatggcgacaaggtatacagcgtcagcaaaggattcacctccagcatcaggtatacaatgatcacgatgagaaatacagtccgcgatgcgtacatgatagcaggacctacatacatgcgtacccgtgatacatcttctgtaatacggctcatcaggtcgccggtacgatgcatcttaaaaaagttaagatccagcttctgataatgctggtaaatttcattcttcagatcgtactcgatatgacggctcattacaatcagcgtttgccgttgcaggaataaaaagaatccgctcagcaatgcaaacagcaggatactcaccccgtaaaacgccagtacatgcgtgaaatccgcacggaaggccaccttcagcgcagtattgtccagcagccggtattcatctatattatgcgccagcaggtcaaagatctggcgtaccatgataggctggaaaacactgaatacaatggatatagcggtaaacaacagtccaaggatcagcagccatttattggtaagaaagtatttattaagcgcggcaaggtgtttcaacggtcgtcaatttgcaaacaaaaataaggcattcgacgcgaattttgtcttggctcaggattacgctgattatactgattacctggatttttacttttggatttttttagatttttagattaataagtaagggagatgaaagcgaatagatccgcttctatctcccttaatcctttataaaatccaaaagtaaaaatccaggtaatcagtataatcagcgtaatcctgagccaagacaaaatccgcatattttactttgcggtaaaagaccccaggatctcttccagcgctggttcatattttgccaggtcgtcggccagtgtggtgagggtaatggcgtaggcgatattattttttaccaggatggttacctctccgttgagcagggtaccgctttcgcggtgggcatactggcatttcatccatttggcttttacgccggtgaccgtgcgttcgccggtatcgatctttttataatcaacgaagaaactttccatttctttttgggtactttccatcaccttatccagcgtaaatcctttcttcagttcctgcgtaacaatatttacattggcctgaaaggtactatcatcggttaccggcgccatcataaacgtatattctatccggctcatcacggtatctatcttcgtccagccggcgggggtatttacggtaaaggttcctctgccggcattcatgcccggcgattttcctgccagttccagtacttcctcgctgcttaattctttaggggatttggaggtgttgttgcaggcggcaaagcttaacaaacaaactaccgcggggatcaataattgtaatttcatcgtgcacaaagggataaaaaccgctccggcattgcaccggagcgatcgaatgattataaacttttaagtgcagctattatcctggattctgcatccgcagccgctacttcttctttcacaaatttctgaccggtaatattttcaaacagttcaatgtagcgctcgcttacgctcgttacaaattcgtctgtcatttccggtacctgctgaccgtctttaccctggaaaccgtttgccatcagccactcacgcacgaattccttgctgagctgtttctgctgggcaccgttcttctggttctcttcataaccttccgcgtagaaatagcgggaagagtcgggcgtatgaatttcgtcgattacataaatggtatcgccgatcttaccgaattcatattttgtatccaccaggatcagtccgcgtttggcggccatttccttacctctttcaaataaagcgagggtgtacttttcgagttgctcgtagtcttccttgcttaccagtccctgcgcaatgatctcatcacgggaaatatcctcatcatgaccttcatgtgctttggtggttggagtaatgatgggcgacgggaagaagtcgttttccttcagtccttccggcatggttacaccacacagtacacgctcaccggatttgtaagttctccaggcgtgaccggtgaggttaccgcgtaccaccatttccaccgggaaagtttcacatttcagcccgatagttacattaggcagcggagaagattttacccagttaggaacgatatccttggtcgcttccagcataatggccgcaacctggttcagtacctgtcctttgaaggggatcgggcgtggcagtaccacatcaaatgcagagatgcgatcgcttactaccattaccatcagcctgtcttcaatggtgtaaacatcgcgtacttttcctttgtaaaaggcagtttgacctggtaatttgaaacttgactctaacatgaataaaaaaatattaataattaaaaatgaaaatcacttttacgagatgcaaaagtaatcatgaatcaggtgatttataacgatcgtgtattttttttcttagcggaggttgtcttcctcaggattacgctgattatactgattaatttgattttactttttggattttataaggattttaaatgattttgggagatataagcgaatacccgattatatctcccaaaatcatttaaaatccaaagtgatcaaatccctaaatcagtataatcagcgtaatcctgagccaagacaaccttcgcatcaccggctgttgccggcataaggccggagcaggctgataatcacttcgttttcggcgtaaggggtcaggtagtcgcggacgtgggcggcttcggcagtgttcacttctgcagggatatagcccattccataaaagcggcccttttccatcaggatacagcttttctcgctgctgttgcggcctttgtctacgatgatgacggaaggctgttgctcctgtaaaaatgcaattgccgctttcatgcgctcattatagctttccggcttttccaccttatcgcaggcgccattacaggtgccggcggtaatgcccgcacaggtgccattgcccttttgcaggaagcagagtttgggacacagttggaactcctttatgagggagcgcagcagccggtgaccgtctatcagcaggttaaagctgtgtacagggtgcgaatacttccgcttcttttctataaccagtcgcaggtatccctgctggtcttcaaacaggtaaaatccatacctgaactccacccgcttctgggcatagttaaaaattggccacaggcgctttatctccaccgactccaggatgcaggccattaattcggtagccgtttcctggtaggaaatgcggtgaatagtacgcaggaaattctgccgctggcggctggcgctatgcccggtaaaatggctgtttacccgtttacccaggtcctttgccttgcctacgtatactactttgtctttgtggtcatggaaataataaacacccgggttggccggcaatcctttcacatggtccggtggcaggttaggcggcaggaactgttcctttgatcccaccttcagcatggaagcaattaccttttctttatcgttggccagcagcatcccgaaaagcacggtggtggcttccgcatcgccgccggcccggtgccggccattaaccggtatgctgaaatggcggcagatattacccaggctatatgatttcagccccgggaagatcttgcgtcccagccgtaccgtgcacagcttcttacattgcaggtcgaagcccgcattggccagctggtgctttataaatgagtaatcgaagtttacattatgggctacaaagatccggtctttcaacaggtcgtataataacggggcgatagcctcaaagggaggtgcatccgccaccatactgttgctgatgcccgttagcgactctatgtaataaggaatggggattccggggtttaccagggtttggtaatgctgcgtcacttcgttcccgttgtacaggaaaacggcgatctccgttataccattggcgctggcatgcccgcctgtcgtttcaatatctacaattgcatacatccgttacaaagatatggattgttgccgcttattcaaacgccttaatccaagtaatgccagcagggtataaaaccccgatagcgccagcaaatgtaatacggaagaagcattatccgccagggcgccgcccatttgcacaatggactggtacactttcaggaacggtgtggtaggcaccatggacgataaccactgcagtggtaccggcagggattcatatggccatgcataacccgcaatgaggaataccgggtaggtggaaaacaccatcatctgcgccgccatcagctgactgcggaacatagtgcccagccatattcccagggggatgagtgtgaaaaagaaaaggaagaacaccaccgccacatccagcacccgtccgcggaaagggatgttcagggtggtatagttgaccgtcataaagaaaaacgcatagcagcaaaaaagcaccatataaaaaagtcctttcccccagagggtggccgataagccgccaccaccggttttcaccagttcaggcacgcgccctttttccttgtcgagcgccatgctttcggaaagacctatcagcagcgtttgctgtaatatcagcgccagcagtcccggtaaaaggaacgcgccataactggagcgtgcattgtacatcggccggtagtcgaggttcaccggctgggtttcccgcatggccatctgggcattcaacccctgcatttcgttatacttcaaccttacccctgcccctacggtaagcgccagcgtggtgatgccacccgccagttcgctggaaggcaggaaccgcgcagcgttcacggccagcacaatatcggcctgttgcagggccagcacttttttctctacgccgtggggaatgtacaggtagccctggcactcgccgtaatacattttctcctgtgcatcctgcaggtccctggcgcctgttacggctgcaatctgcattttgcttagttgctgcaggaaggcgcgggataattcacttttgtcgtcgtccgccaccgccagtaatactttctcttctaccttataactataaatgctgccatagaaaaaagcatacaggagcggcgctatcagcagggtaagcaacaaactgtggtcggtggctaccatcctcacttcccgcaggaacaaccgggttatatgacgaaaaaaattacgcatgctgtaaggaaagtttatccagtttccgttgcaggaataccaatgccaccgggaatgtaactgctatataaatcagcagttggcccgcttccttatatacatactgcatgggcaactccataaaatatactttgaagaatccatccaggaaaggcgtaaacggcatgagccaggcgtagtattggtcgtaccacggcatggcccagcggggaaaagtaaaaccgctgaatacaaaggccggggaagtatagaacagtccgaggtcgcaggccaccattacatcgcttacaatggccgataccatcaatcctatgctgatacatccgatgatcagcaaggtaaaaagcaggaaaagcggccaggagccgcccattcgtccgtgcgcaaaaagcgggaacacaatacatgttaccaggatataatgcagccatcctacactcaggtgcgccaaacctttgcccagcaatacattggaggctgatccattggccattgcattcagttccgcgaaggtgcctcttttttcttccaggtttaaagcaagcactgttaccatgatgatcatcatctgtagtgccactgcaattagccccggcaccaggtattgctggtagttgtattgcggattgtataacatataagaggtgagccggatgggctgcaccagcgccatcgccttgccggcaggcataccggtttttacaaacttctgtaacgtaactcccgagcccgccgtaattaatactttcgcagcatctttatagatcagctttgctgttactaccgctgcggtattggtgtacacggtgatatataccggttgacggcttttgatatgatcatccattttctccgggaaatggatagcgccctggatcacgccttgttccatcatcttttgcagggtaacttcattatctacctgctgtgtgatatggatactctccgtttgctccagcataaatgcaaacttgcgcgataaaggcgaatgtgattcatcccagatggccaccgggaggtcacgggcaaactggttattatagatatagccatagagcaggcataccagtggcggcaacaccagcagtacgatgtagtgttccgggagggtaagtatgcgtttccactccctgattgtaatatggaggatggaacgcatcatggcaggttcatggaggcggtcataccagggcgcagacctttcacagccgcctggttaacaggtttcaggtctaccgtaaaagtgcgcagttcaaacctgccctgttcttttaccggtacccagttggcgaatgtgagagaaggcgctaccttatgtacctcggcctcaaaattctccggatcgcatcccggcacccgcacctgtacgcgggctcccagcgggaaacgttgcatatcatcctggcgcacgttataggtaatatgatacgtggctggtttctggatcgtcatcagcgggtagccaatagccacgatctccccttcttctatgaccatggaagtgataacgccgtctgacggtgcatgtatataagtgttatcagataatgctttggtgagttcatagccttgttcagcctgccgtacaatggcggatgcggtggtgatgagttccggcctgctgccctgttgcagcatatccatgttcagcttggccgtttccatttcttttttggcggcttgcagtttgaagtataccaggtctttttcctgtcctgaaatcacttcatcgttaaagaggttctgcatacgctgataggttttctgcatcagctcatactgttgctgggtgatattatagaggttatccgctgctttgatggcttcgggccgggcgcctttctgcaacagggtgagctgtccttttgccgcatctatggccgcctgcgcctggttgcggatagcattgatttcggtggagcggagcacccccagcaactgccccttacggacggtatcgccctgtttcaccaggaggctgtccagccggccggggaattctgccgccacatccacgtagtcggcgtccaccatgcctatcatggattcatctgcagctgccggcttcttcacaaagaagatcagcgcaatcaccaggatagcgatggggatcagcagggcccaataatttttaagtacagctctcatgaaaaaatctgtttatctgtcaacatattctgcaaattgttccggtgtgcctattacattccagtactgcgccagggcgaggtagtagcccattacggcggtatagtagatcttatgcatttcctcttcctgcaggagtgcatcattaacatcttttacagacgacagctggttttgcatacggtcggtgaccaatgtggtggtgaggtgcgcctgttgccgtgcgctgtcgagcgaggccacatcattttgcagggctttcattttattgatcgacaccctcagttgcagttccagcgaggttttagtgttcagggccgccatctgcgcttcttccaccagcattttactggctttggtacgtttatatttctggaagccgtcgaagaggttccactgcatttccaccccgatgagccatggcggtatggttaccggtaaatctttctggtacaggttcaggctgccgatggcaaaaatattgggcagggcgagcgaccgcgacgcctttacagctacattggccaggtccgttttgttttccaccaggcggtaagtggggttattgcggagcaattccagttggcccgtttccgttaccggtttcagttcgtattccagggtgtcgttgatttcaataggtgtttcaatcggctgcccgagcaagtcgtttaattccagcagtgcattttctttctccagctcgaggttgttgtaccggttggtggcctgtacaaaagatacccttgcccagttgagcaggtaaggcggcaggatctggttatcttttaaagaggcggcataatcgcggttcttcctgaaagattcaacgattacggcttcatgggcaagaatggtattcaggtagaggatgcggaggtactgtgcactgatggcaaagaacaaccctttttccaccacctgctgattgaactgcccggctgttacctgtgttttggccagctgttgtgcggttgcaattttgccgccgaggtatattggctgccgcagcgccagggctgccgtgaaataagattgctttgtaagctccgggttataatcggggtaaaaggtagtgatgatgcccttcgtagcgttatagataacgtcctgcacattttgcggaagcggctgaccggtaatttgctggtaaacggtattggcggtattcacgctttgggaagaagacccgttaaccaccccgtctttcacctgttgcaggtttatctccaatggtttgccgaggtaattgtaacccgccagcagatccactttaggataatacgccccgttttctgcctgcaggttatactcccgggctttcagggatcgctgcgcctgctgcaccaatgtatttccctgtttcgcaagccggtaacattcctttaaagtcagctgtggtccgttttgctgaccgtgtacaaacaatgctggcagtaacggaattaaaaacaagtaatatctcatacggttttctttacatcaggaaggcttgcggttgaaccctaacacctcaaaacaatctttcatgaataatgtttgaagtatttgaaaaaaattatacatcatttgataataaagggcttatcgttatatttcttacctttaagcgcatacacaaaaagtacatcattatgtgtatttgatccatttgaacccacctgttttcacccgatatttgtgatacaaaagattgaacaataggttcctgatcttgttaaaatataatcctgcagcggtttacgcagcattgcaattttattgattcattataaaactacatttacttatggcaaaacaacaatgggtagccgacgcgagtcacagtgaacttggatttaaaatccgtcacctgatgatcaccaacatcaatggtaagttcaacaacttcacggtggacgcagaaacggaagaagaagattttatgactgctaaagtgagagtagcggtagatatagactctatttcaaccggcagcgccgacagggacaaacaccttcgttctcccgacttctttgatgtaaacacctacaaggatatcattttcgaaacgaccaaatatgagagcgttgataacgatggctcctatgaattatacggagatctgaccatccgcgggatcactaaaaacatcaaactcgctgtagaattcggtggtgtggtaaaagatccctggggcaataccagggcaggttttactatcaacggaaaaattaaccgcaaagattttggccttacctggaatgcagctaccgaagctggtggcgtaatggtaggcgacgatgtaaaaatctacggagaagtgcagttgatcaagaagcagtaagattatcagctgttagtctttgtcttgtacaaagactaacagccaacttttaaaaggaggaattatgaatgaaataacaggcctgcatcatatcacggccatttcaggcaatgcgaagaagaactttgatttttatacccgtgtgatgggattgcgttttgtgaagaaaacggtgaactttgatgatccccacacttatcacttttattatggagatgaaaccggcacacccggtactatcctcactttcttcccatgggaagatattatggccggccgcagaggtacccacatggctaccgaggtaggctacagcattccggaaggcagcattgacttctggttaaaaagatttgaaaaagagaacatcatctataataaaccatcttccaaattcggggaaatatacctgaccttcattgatcccgatggattgaaggtggaactgaccgtaccggaaaagccggacaaccgcacaccatgggtaaccaatgaagtgagggaagaaaatgccacccggggttttcatcatgttacccttacgctggaagatgtgcagcctactgccgacctgctggtatctgtgtttggttacaaacttgataaacatcataccaaccgttaccgctttgtaagcccggccggcgataccgccaattatatcgacctggtagaagccaagggagaaccccgcgggcatgttgccggcggaagtgtgcaccacattgctttccggatgaaagacgacgatatgcaactgcattaccgccagttgctggaagaccgtggtttaaacgttacgtcgcagctggaccgtaaatatttccggtctgtttacttccgggagccgggcggtgttttatttgaactggccaccgacgttcccggtttcacggtagacgagccggcagccgaactgggcacgcacctgatgctgccgccgcaatatgaaccgcagcgggaagagattgtgaaaaaactgattaaactggactgatatggattttaaaccgatgcagtatgtatacgaagcggtgggtaaccccgccgcctatacgttactgctgttgcatggcacaggaggagacgaaagggatttattaccgctggcaggatcactgggtaaagggtttaatatactcagcctgaggggcaatgtacaggaacatggcatgccccgcttcttccgtcgtttaggcatgggcgtatttgacgaagaagatgtacatttcaggacgcatgaaatggtgcatttcctgaaagaattagccgctacagaaggcttcgatatcaataaactgattgctgttggatattccaacggcgccaatattgcaggcgccgtgcttattttatacccggaattgctggccggcgctgtattgttccgtcctatgcaaccgctgagcggtatagaagacagctttgaaacgcagcgacagcagcccgtatttatgagctccggcgtgcaggacggcaccgtagatcctgcggccacggcggcttatgccaccctgctggaaggcaatggctttaaaataagtaccttcgatattcctgccggtcataacctggtacaacaagatattactttggcagcagcatggatgaaagatcattttcagtaaaaaaaatatatggaccaggaagttagagtaagtttatccggccgtccttaccaggtgtcgatagatacgagggatcaccgctggctggcagatgaaccgatagaagccggcggcgacgataccggcccgcagcccggggaattattactgagcagcctgggttcctgcactgctatcacgcttaaaatgtacgccgacaggaaaaagtggcacgtggaaaatattgaaattgagctgcgctttaacaacgccgcgaagccggatccacttactaccgttatcgatatcgacatgcactttaccgggaaccttagtgaagaacagatcgccagactggagcagatagcgcgctcctgccctattcataaagtattgagccatccgattattatgaacactaaagccgtataaaaatgaaagacatcaccaaacactactccaacggagaggtaaccattgtttggaagccaggtgtatgtatccattcggagaagtgttttcacggccttccgtccgtattcaatccaaacgaaaaaccctggatcaatgcacagggggctactaccgaacaaattatatcgcagatcaaacaatgcccttccggggcgctgagcttctttatgaatgcagacgcgacgaaagaagacggcaatttaccagacaaattataatctcctttttatatggaacttaccatcaggaataacatcgcaaagaaacagtttgaaaccgaagtggaaggacataccgcgctggttgcctataccctgtaccccggcggcattgcctttatgcatacagaagtgccgcctgcactggaaggccgcggcattgcagggcagctggctaaatacgtgctggaatacgcccgggaaaatcatcttaaagtaaaaccttactgtccttacataaatgcctatatgaaaagacatctggagtataatgatctcctgtaacagatttatcacttcctaaattcctttccatgcaacttatgaaattcattcagcaaccctggcactggtcggtatccgggttgctgattggtcttacggtaccggtgctgttgctgctgggcaataaggcctttggtatctcctcttcgctgcggcatatctgtgcagcatgtttcccggcgaatatttccttctttaaatacgactggaaaaaagaggcctggaacctcttctttgtagctggtattgtattgggtggttttattgcggggcactacctgcaggatggcaacgatatccaggtggctgccgccacacaggcaaggctggccacttatggcgtgcatgattactcagcgctgttgccgccggaaatattcagctggtcgaatgtctttacctggaaaggactggtattctttgtgctgggtggcttgctggtgggctttggtacccgctatgccggaggttgtacatcggggcattccatcatggggttgtctaatttacaatggccatcgctggtggctacgtgttgctttatggccggtggctttatcagtgccaacctgctcattccttacctttttaaatggctgaactaacatgaaaaatatcaggtacctggtagcaggaactttctttggtattgtgctggtaaaggcgcaggtgatcagctggttccgtatccaggaaatgtttcagcttacctcctttcacatgtacggtgtaattggcaccgcggtaattaccgggattatttccctgcaactgatcaaacggcttaatattaaaactatccagggtgaaccgatttcggtggctcctaaaactttcaataaaggacagatcttcggcggattgctctttggcctgggatgggccatcaccggggcttgtccgggtccgctgtttgcgcagataggtaccggtttcacggtagtaggcattactttgctgagcgccattgcaggcacgtggatctatggtgcattaaaaccgaagctgcctcattaaaaaaagcttcaaggaacaggcccttgaagctatggttgcaattctctggattcacagataattattttttcaaagcatctttaattgctttcgcggaatcctggtgtgccttcagcgttggcagtgtattcctggcccaggttttcaggtcttcatctgttacattatcgcctgctttctcaaatttgttcacgtctttatcgtggtcgtctaccatcatgctcatgtattccttgtcgaaatccttaccggttttcttaccaagatcgtcgatgtgtttctttgtttcggtagacaattctgccggcaaagtgatgccttttgttccggccagtgcttttaattcatcccctgctttggagtgatcgttcaccatcatggtggcaaaggcctttactcttggattctgtgctttttcctgtgcaagcttacccatctcaacttccatcataccgccgtttgcagcctccacagcaaattcagatgatttttcatctaccggtttaacagtttcgttgacatcctttgcactgtcgaccggtgtttccgattgtggattcttcgcattgttgttacacgattgcgtcatccacacggctaaaaatgttgctgataaaataactagcttcttcattgtatattgttttgggtttgtaataggtgtgcccgtttacatagctctactttgcaaaaacggtaccctgaaaacaaataacgatcaaacgcaatacagcaaaggattttaaaggaagagtcaaagcggactgacgcaagaaaaatgtagattgttttccccggaacgcgcaaaaaaaatggttattgtaaaaattacaataaccatttctctttaatagcgcctgctcttattgagattgagcgaactggtaaataataatgatggcggcaatgatacctaggataaggcctacaattttcatccagctgtagggacggtcgcccgttacttccccggtgcaggcatttaccacaaaatgatagagtttgttattataccggtaggcgctgatccaaacgggcagcagcaaatacttcaggccaagctggttgtattccacgtcgtagtcgtcgatgcgttgttcgtcgccgccgatatcatcacagatctcattacggattaccgggtccattcttttttttgcgattgccagtgcctgttcggcattcgtttggtaaagttccgcccggaaaccgctgaggtaccgtccgtcgtattttttcagttgttcgaggtgccagggttccaggatctgcgccattttcaggggcaaagaaggactggcagataccaacacgtcacggaagttattgttcacactgccggaagccgggtaccacgcggtatgccgtacctgccgggtgcgggtttccgtccggccgtttacttccactgtatagctttctgtggtgtaataatattcaccgcgggagccggagtattcagtataagtgtccgtatcgtagctccagtgtggaatgtacacgcctttcaattgttgagaggagctgtcttttactttcttcaccaggtcggacggtgcaaaccaaagtttcttcatccaggtttgaaagtggtccaccgcggttttgtcgctcactacaaagggcaatacataatgcggttgcaggatggaagtcgtttgcgcggtatccaccaccagcggcgacgcgcagaaggggcatgaatcggcggttacattgggcagcatggtagtagacgcgccgcaactgacacatttcactactactgcctgttgggtagcttccgtatgattttgctgtgaagcaataaaagcgtcgtaatcgatgggctgtatagcgtccggctgcgtatcatcctcaatctggttcacggtaccgcagtattcacatttcaggctgttagtgcctggtgcataatgcaggatagcgccacagttctggcatttcaacgagttaactgtttcgcttgttttttcctcaaaagacataggaacgtatggatctaataccgtccggcaccacgtgatgccggacggcctgctttagttaaggtaatggtggtggtacggtggctaataccggcgccagttccggcactgtgttggcggcggcccatgccgccatgccgtttttccacaccagggtttgcgcattcaggctgcccgcggcggccagctgacggagttgatcggcatcgaaggggccggattgtttgccgtctaccgctacaaaaaacgatgcagcgccgggtaacggaggtggtgctccaccgcctgtattggcctgctggttattattctggaagatgttacctacctgtcccatcatggctgcgcccatgccggcgcctaagccggccgctgcgagtccgccgccggaagggttttccgctgccttttccatggcgttggctgcctggaattgcgcatacgcgcccaggttcccaacgatgcccatgctgctgcgtttatcgagtgcagcttccacttccggtggcagggaaatattttctatcaggaacttggtcagttccagtccgagttcattaaattcagtaccaattctaccggtgatctgggtggatacttcttcataattagccgccaggtccagtaccgggatctttgcttctgccacggcttccataccacgggatactgcgagattacgcagttgctcgttgataccttccacggtgaattccggattagtagctgctacttccttcaggaattgtccggcatcctttacgcggaaagcgtaactgccgaaagcccggagccgcaccggtccaaactccgcatcacggagcataaccggattcttggttccccatttctggttggtaaactgccgcatgctcacgaagaacacgtctgctttaaaagggctgttgaagccgtatttccatccctgcaaggtgctcaggataggcatattctgtgtagtaagcgtatacatgccgggttgaaaaacatcggcaatcttaccttcattcataaaaacggccacctgtgattcgcgcacagtaagcttggcgttcatttttatttcattctggtagcggggaaacttccacacaatggtatcggcggacgggtcggtccattcaataatgtcaataaattcattcctgagtttatcaaaaattcccatggtaacaggttttagagtggaccaaatttagccatttattcactcgaaaagctacttcctgaaagttataatttatgtaaacttacttcacggttgttttcagccatttttccatcagtaagggccaggcttctcccgcgggattgccattccgtaagccgtatccgtggcctccttttgcataaaaatgcagctccaccggcactttggcgtcgcggagggcgccggccattaccagggcactattgccataggtatcatctgcggtagcaaaaaggaacatggaaggcgtttcactcgttaacttcaactcaggggtgagtgacctgttttctcctttatcaagataagccgggtaaatgagtgcactaaaagcgggacgtgcagacaaagagtcggccttgtcgattggcgtataggtatgcacgttatattgcactgatgccctggcggtaagacttccacctgccgaaaagcccatcattcctatcttgtcgggctgcagcttccattcggatgccatgctgcgtaccaggcggatggcacgttgtgcatcctgcagggcgccggcttcttttttgggtacccggtattgtaatacgaaagcagtgtaacccagtttgttgagccaggcggctacttcgtatccttccaggttaatggccaggatattataaccaccgccagggcagatgatcacgcctacgccgttgttattggccgcatcggccggaaacacttccaataccgggtcggtaacatcggtgagccgtgttacatgattgctgccatccggggttacctttgcggtttgtttgacggctgtttcaccgggtacggcagcgggccagagatggatctgctgctgttgtgcggatatcgttgtatttactcctaacatcattaataagataactatttgtttcataaccggattttcagatttcatgtaatgaaacaaatgtaataaaagaaaggagcagataaaaccggttttattttacacattgtaaccaggcttccgccatcagctgggcgccggctacgctgggatgtacaccatcgccggtccaataggacgccggtgccgacttctgtgctttatcaaaaatggattgataaggaataaaagtggcctggtacttatctgccagttcccgggcagctgcgcgatactcatcgaacgtagggtaccatttatcatctacggccttcacgccttttaccgcaaagggttcgccgataatcagctgaacatccggcagctcctgtttggtgcgtgccagcagtttatcgtagtcgtcgcggtatgttttggcggtgcctttatagttattactcaacgtatgccagtaatcatttacacctaccaggatactcagcacatccggcttaatcagcaggcaatcggtgtcccagcggtcggccagttgaaatactttatttccgctgatgcctttattatacacttttaaatttttatctgcacttttcagcagcatggaagatgccgccatcagcgcgtaaccaccgcccaatgcgccacctgcattaggttggtcgttgtcgcgtttacggcctgcatcggtgatggaatcgccctggaacaataccacgctctcttttttgagtactatctttttagatttctctgctaccgttgcggcggcaacaatatctggaatgctgatggcagcaagggctcccagggaaacgttcctgaggaaatgacgtctgtttgatgaattcataacgatacggattaaatgctggttgcggcatagtccacaatccggcatttaaactataaaaaagatttgatattttatacaaatgcgctgaagccggtaatggcgcggcccacgatgagggaattgatttcctttgtgccttcgtaggagtaaatagcttctgcatcggccacaaagcgcgctacattgtattccagcaaaatgccgttgcctcccatcacttcgcgggcacggcttaccacatcgcgggtacgcaatgtacaaaacactttggccagcgaggcatgctcgtcttttaacccgccggcatcctgtatttccgataagcggaataccattgtttgcatggcagtaagattggacagcatttccaccaggtggccctggatcagctgaaaagcggcgataggttttccgaactgcttacgggtttgcgtatacgccagcgcgttttcataggcgccacgggcgcagcccaccgcttcccaggccacaccggcgcgggtcatgcgaagtacacgggcagtatctttaaaggaagcagcatgttgtaagcggtcggattccgctatgcggcaatctttcagggtgatcaatccattttggacaatacgcagcgccattttatcatggatcttttccacgctgaaaccgggcgtatcttttctcagcaggaatcctttcacctggttatcgtccacatcccttgcccagatcacaattacatcagcaaaggtggcgttgccaatccatttcttctggccattcagtatccaggtatcgccttcccgtttagccgttgtggttagtccgccggcggtgccggaacctacttccggttcggtaagtccgaaagcgccgataatattcagctgttgcattcccggcagccattcctgtttctgtgcttcagagcccagcatataaatagatcccatggccaatccgctctgaacgccaaagaaagtagctacagaagcatctatacgcgccatttccatggcaatgatcccttccatcaggaacgaccggttaggacatccgtatccttcataagtaaccccgcagatattcagctccctgaatttcgggatgatttcaaaagggaattccgctttcagccagtattcattaacgataggcttgatttccttttccataaatgcccgcaccttcagctgcagtgccctgtcttccgcattgagctttgccccgagatcatagaaatcgccttcaataggcggcagttctttcttcttactgccactggtgagcattttcattaagccgttcagctgcgtatcatccattttccctaccgactccatcaccttcgggagatctactttttcggatagtttagccagcatggcgaaatcaatgctcttcaacaggtggtacgcattctttagtttcgtgagaggtccggacatcttacatggttttacttaaaaatacgtaatccgcgggatttacgcggatgttgcctttctcaggattaacggtgattttaaggatttgggggatttgaacatttgggattttaaaagattcggggagatataagcgaattttgtctttctcaggattaacggtgattttaaggattaaaaggatttgaacatttgggattttaaaggattcggggagatataagcgaattttgtctttctcaggattaacggtgattttaaggattaaaaggatttgaacatttgggattttaaaagattcggggagatataagcgagtagcaatccatctttttaaatttaaaaaaagaattcagtacaatcagcttaatcagcttaatcctgagaaagacaaaattcgcttatatctccccgaatcttttaaaatcccaaatgttcaaatccttttaatccttaaaatcaccgttaatcctgagaaagacaacatccgcgcgggggaaattaaaatagggttgcatagaaccatatgcaaccccgtttaaaaacacaactaaaaaaaactaacttctaacaaacataataggcatagctgttatattgctgacgcagagaatccggtatccctctattggcctctccacttttttttaatcttttctaccaaataaaaatataatctgtaatgtgtaaactgtaattgttttcaaaaagatagttactttcgcagcgatcatttcatatactaaaacttcctgaaggttaaatgattacatcaccttcttaccaggcgtataaagaattatttcattcacaatacaatgacttatgtaactatgcctatagtttcctgaaagacgatgcagcagcggaagatgtggtgcaggaaacctttattaagctctgggagaaacaccggcagctgatagacatacctaatataaaagcatacctttttcgtgcggtgaggaataattctatttctgtgttacgcaagcaaagtaccgaggaagctggcaacaaaggctttgaatggctggcagaaacggcagaagatcccggtgctaaagagattgaaaatgcaaagccttactatgaacagctggtatatgaggctattgccaaccttcccccgcaatgccgggaagtattcacctgctgcagattgcagggaatgacacatcaacagacggcaaccaaactcggcctttctgctaaaacagttgaaaactatatgggacgggcattgaagctgctgcggaaatatttacagcaatatgggctgcccgttagtatcttgtttttactaaaaatattcatgcccctgtagagggttgttatattaatgagcgttatttaagtagagcacactgtattatggagcattttgatacctacctgcatgagctgattgctaaaaatctgtctggtcaatgtacagaagcggaatccgctgccctgcaacgttggctggaagcctctcccgaaaaccgggcagaatatgaaatactggtaaaactatggggggacagtcccgctgcagtggcgcccaaacgggaatacaacacggccgctgcctgggataaaacggaccaggcaatacagctggcgccgtcccgtgtaaaagcactttataccaaatatgctgctgcggcagccatcctgatattacttacagcaggcgcatggtggctggaaacacgctcctcgcttaaaaaacatgagctggccgcgaatgacggcaaaataaaaagcctggagttacctgataaatcaatggtaaccctccggcagggcgcaatgatccggtatatcaatggctatcaccacaaccagcgtattgtggaactggaaggagaagccttttttgaaatagccagtgatccggaccatccttttttggtgaaaacgcccaatcaatccgtgattgaagttttgggaacctcctttaccgtgcaaacaggaaaagacactacagccgttaccgttgcttccggcagcgtaaaactaagtctggaaggcgataccaccgccatagtactgaatagtggccaacggggtgtatggggcaacggacagttatctgccaataataatcacaacctgaatttcatcgcctggaaaacaggtattttgcaatttaatgaccagacactgcttgaaatattgccacaattagccgacttttacgcaaaagatatcagggttgatgaaaaatacagggaaaccgcatcgcagcaaaaagctacgattacattccgaaatcagtcctgcgatgacgttttgcatgaattacaactattgcttgggttccactatcaacaggacggcgactctatcgtcatcacccagtagaacaaaaaacccgcttttccttatttatggaatgctgttgttactgttcccgtttcaattcctgcaggcacagcacaatggaaaggacattctccatgaaagctatacccctgctgcccggcaggggaccattttattttatatccaggatctccagaaagttaccggtatcaacgtttcttatagctccagctttttacacctgaataaaaaagtacagctcagcggaacagaacacactaccggcgacgtactgaaggttattctccagggtaccggtatccaggtggctgccctcaacgggaaaatattcctgctccgcgaaacctcccaggtacaatattataccatcagcggatttgtaaaagaaataaacagtaatgagctgatcatcggcgcttctgtatacgatcccattacacggaaaggcactgaaaccaatgcctatggcttctatagcctgcaagtgccggacacctgcctgggcgtggtgttttcacatatcgggtacaaacccgtgtttcaacatcttccaccgccggacgacgggcagctggatatacacatggaagcccgcagcatgctgcaaacagtagtggtaaacggcgaaaatgaaaccgttaattcccaacccggctacatcaatatgcccgttggctatgtatccaacttcccggcactactgggcgaaaaggatgtgctgaaatcactgcaactgtatcccggtaccggcagctccctcgaaagcagcagcaacctgctggtcagaggcggaggcgcagaccagaacctgtacctcctggatggggtaccactttatcataccggtcacctgttcgggcttttctccatcttcaacggagatgcggtaaaagatgtgtcgctttataaagatgccttcccggcgcgctatggtggccgcctttcctcagtagtggatatccgtacaaaagacgggaatatgaaagagtggcatggcagcgctaccgtgagccccgtttccggcagcttcctcctggaaggtcccgttgtaaaagaccgcagctctgtttctttgtctgtaagaagatccctggtagatgccctttatggaagggcttatctgaaagattatggtaaatattatctctatgatgtaaactttaaactcaatcaggtcatcgataacaaaaacaggatctatgtcagcttctataaaggacaggataaaatgtttatcaggagcgagaacccggttatccagctgtttgatgattacaattttgactggagcaatgttactgctgccgttaaatggaccaaagtagtgaatccaaaaatattctccagcaccactgctacctacagccgtttttataacgtttttacgcagaattcgatcatccccctctccttctacgactccctgtttgtgcgggggaaaggcgtttcccggatcagggacgtggccatcaggaacgaaacggaatatgcagtgagcaacagtcatcatatttctttcggcggtgcttatacctatcacaactttgcacctacggcttatcataataacatctccgcgggagaagctacgcagcggaaagcgcctatttattatatgtcggagttctccgcatacgcagaggatgaactccgcttattgaacgaccggctgatcgtgcggcccggactgcatttcggggcactggcgcagcgtacctctttttaccccagtttacagccccgacttatgctgcggtggaaactgccccattcacagtatttacaggcatcatttgctgaaatgacacagtttgtgcaccagttaaccacgccggttatcaacctccccaccgatctgtgggtaccgagtaccgagaatattaaaccggagcatgcatactcctacagcatcgcctatcagcggcagtggagcaaccaatggcgcttcaatgtgaacctctattataaacaactgaaaaatattgttaccaccaacaccgtactgaatatcttcgataactcggatctctgggagaaaaaagtgatcgccggcaacggctataactatggcagcgaagtgctgctggaaaaaacacaaggcaagctgacaggcatcttctcttataccctgtcgtgggcctggcggcagttcgaccggttgaatgccgggaagatgttcccttataaagaagaccgccgccacaatatttccctggcgctcaaataccggtttaatccgaaatggagtctatccgcttcctggaaattcgcctccggtgcacctttcaccctgccggtgcagatattcccggatttcgactggagccgcaatatcaaaggctacctggacgaacgttattccccgttctctactttccaggtaaactatttgccttatatttcccggttaaataactaccggctaaaccctgtacatcacctggatctcggggccaccttaaacctgggtaacgaaaaacgttttcatcatgtgattaccgcgggcgtttataatatttataaccgcacgaatccttttatcgtgagctttgaccagttctcttacctggattacagcgacgtgtacccgttacagttatatcagtatagtttattcagaacattgccgtatctgacttatacgttcaaattttaatcatgaaatacctgtttatattaataccggttttaaatattttgctgctaacgggctgtgagcaggaactgccgcttcctcccaacaatgccgttcccagggaggtagtatacagcgagctggtggccaacgatataccggaagtgcgggtaggcaaaagcaaaccggtaggtccaggtatcaacaccggctttgacctggtagaaaatgcggatgtacagctgatggacaaaaacggacaaccgctggaagcacttacgtatgtgaaagattccagcaatgccatgagcgtataccgtggtaaaattacactggatgcaggcaaaaattataaaatacgggtgacagtgcctggcttgaaaaccgttaacgccatggcttccatccctccgccttttaaagtggaactgctggacacgctccgtaccttgcttaacggacgcccggtgttacgctttcattttaccgtgaatcccattcccggtgtgaaacaatacctggtaatggaggccctgaagcaaagcgttatcacggatactaccttttcgtataggggtatgcgatataagaagagtgagcacgattctctctaccagcgtgtaaagcatatgcctggttgcaatcctaaaaaagacagcagcttcctcaatgattacctgcgcattccctgctatacacaggatgaaaatgctgacaataaccagatcggcggtttgaatgaaaactataacagcattttgtttacgcaagccggtaagccgcttaccacttatttttatattaatgccacggccctcagctccaatcctgctgaagccattgcgcccgtaggaagggtgctggtatatgtaaaatctgtctcaaaagaatattatgatttcctgcttacctatgagaaggtgaagcgcaatcccgggctgaacagccttatacaggccattcagctcaaaagcaatacacagggcgggcttggtattgttggaggcagttaccagaaattgtactatctctattacgataaactatagccggttattttatttcgtaggtgttatcccgtttgttgatgtctgctgtccaggtgcttcccagtgttacttttttaatttttttgagagataaaaagggaagcgtcgttgttttgttgcccttctcccataccgcgatgctccggtgtaacttcatggtgctgttgtcgtcaaaaaagagggtaacatcaaccggaaccggtttatttccgatggaagtaatttcaattgttccttgtttccctttttgcgtaacccgtgtgatacccaggtcggggaagccattgtcgaagaaccagcttttccagaaccagtccatattcctgccggcgccagtgttcatacagtagaagaagtcgtatggctgggggtgtttcccattccactgcgacatataataatgcagcgctttcaggaaaagggtatcccccagcatgtcttttatatagagataacccagggctggtttaggataggaattggtcatataggcgtccgtagtttgattggagggcgtcatgatgggcaggtccgcctctttgcccgcgatgaagttatagggcgacatgccgtagtcatccacgatggagctgtcgatcaatggagagatgatccattcgccgatcgtggcccatccttcatccatccaggcgtattgtgtttcattggtgcccatgtagaagggaaagagcgtatgaaaaatttcatggtcagttaactctatggtctgggctttgtcggccagcgggttatcgtttaccatcatggggtattccatctggtccagtccgtcgaacaccgtttcgtgcgaatacgggaacggccacttaggaaagtggtggcttatcttattcacggtggcgcgggcgtaatgtatcacatcaaagaaatccgcatgctgtgggttaaaggctacatccacacgggtgcgtcttttggtggtagcgtctacttccacgctggtggcgttccagcaatagtggttgctgacggcgaaagcaaagtcggtgacgttggctgcttcatactgccaggtattggcgttccgctgccgcgtgatattcccctcccgcacatcgttgctgtcgatcaccgcgatgatgtcgttactcttttcagcagcagcgatgcgttgtacatatttatcgttgtatacggctgcggtatttttgaggtcgccggtcgcccatacttcgtagttgccgggcaccgtaatggctacacgaaaatcgctgaagtcgttatagaactcctgcgtacccgtgtaagggatctggtcccacccgttgatatcgtcgtataccgcaatacgcggaaagaagtaggcgatgaaactggcgccggagtccacggcgccggttctgatgtgtgtattttcgttcagggtataggaaaagtcgagatcaaactgcaccgactgccctgggtaaagatccctgatatacaccggcatattggtgccgcggatgatagctggtaccggcttcgcttcaccatttaccttcatattctttattacaacgccgttggtcaggtcttccggggaaaccgccatatttctcacggctcctttctggaagagattgggaaacagtttgaagttaatgacctttaaggtatccgggctgttgttggtatagcggatctgttccgagccggatataccgtttgttgccgggtcaaaggccaccttaatatcgtacccggctttgttctgccagtacctggcgcccggggcgccactatagctgcgggtttgattgtcatatgcctttttgatggtcaggggcatatataaaggggtttgcgcggttgcctgctgaaatgctgccagcagcagccataaaataccatattttctcataagtgatataaaagcggtggcttcaaaagtagggaataacccggaaacggcatggcagaaagaagcgctatgggatatgagtggtatctaccggcactttaagagaatcggcagggatacgtaaactgtcagctgcgttggtatgcaggctgtcggtggctgaattcgtactgtctttaccgttggctcctttcccgggcagcgggatagtaggtgcagtattgcggcgtttgggggagtaagacgttgcagtgccctgcttctgcatatcgttcattgtttttttatcaaagagatacttggggtgtttctccggccggagcccccggtcaaactgggcctccgctcccactgcgggcgcctggtacaccttctgcgaagaatgacaggcccacaaacagataccggcagccaatacgaggtatttcatacaaatgaaaataagagtgaatacaggcaaagggggacatcttctaaacgataaagccgggttgtttattatcagcagggaacgctttaccggcggcgatgcattttgaaatgtaacatcgctgtattaaatttagcataaattcactggttgtcacccccttattctaatattttatatctttaaccgctatttcaatcccgatgaaaaccctccttcacggagagtcacggctacattcgttattataacaaagcactatgaaagtatcaacaaccagcttcccaagcgtttttgaaaccgcattcggaaacacagaaaattcaagtaaggatcttctcaacggattaaaaattaaaaaggatgaagcctggtacctggtaggcaacctggcaaaacgaggtgggatcaatcccggcagagttaccaatgcgtcgcccacagaagaggattatgaaatactgtttaaagctgctttgctgaacaccattgataaagtacaacaacccattgcccttaccgtagggttccccttctctacttacaatatttacaaaaacgctgcggaacagtttttaagtaaacggcatttcctgattgactacgatacgcaaacttacaataccaaaggttcttttaagaaggccatgtttgatattgagaagtatgaagtgatccctgaaatcgtgggtggtatcataggattgaagaaaagtatcaatgaaccccagctcgacaacttcattgccatcagttttgggtttggtactattgaaggcggcatggccaccggcgacggattggttcaccgtacctgcttcagttcccatggtatccgttatgccattaacaaccttacccgtgagctgaaccagaaacactacctggaaatgaaaaacgaacaccaggtggatgatgctttcatgaaggggtctattttcaccaaccgcaagcggatcgatctgcgtgatatgcgtaaaggtgtgctcacacagtattacagggaagtagtttccccgctgatgcgcagttattttacagatctggattttgaaacctgtgaaaagatttacctgatgggcggtggcgcttactatcgtgaactcacagatgcctttgtagaagaattccgtgactttattccggtagaagttgctcctgaacctgaaaagctcatgagtatcggttatctttataattcattgagaatttcagataataaacctcaaagaagcgtggggcttgacctgggtaattccagttctattgtgtctacttttgaagatgtaacacagcatactcctgctacacctaatcccatcaccctctaatttatacttgtgatcaatgtcagacatattttccgaaatataattgttcccggagcctttcgtattcctgcaacagtgtccgtgaacggtagtatagatgcttcagtttccggccggattgatgggaatgtaagaggcgatgtaaaaaccagtggtaagctggtggttagtgaaacagcgagcatccgtgggcatatatatgctgccgacctggtggtgcatgggaaagtgtatggcgatgtatatatcaccaacaaagcccatatcagcaataaagcgctggtaaaaggcgatgtgaatgcgatggtgctggaaatagaagaaggagctgtggtggaaggcgctatccgtaaaaacgtgcagcccgttctgaaagccgatcttagtcacaccccggtagctgaagaaatcaaagtgtcggctgcggtggatgctgaaaccggtggccaggaagaagaagaaaagaacaccagctggttctgatgagtatcactgccaatattatacctcgttcaggcggttgtttccattgatggcaacaaccgctttttatttccgcctgcgcaggcattaaggatatcgcttctttttcaggggatcgagcaattgggtaagaccgttcatttttattaccagcatcgtttcgaggagcattcccagcttgcctttcgggaagcccttccgctggaaccactccaggtaactcaccggcaggtcacaaagcaccacatctttatactttccaaacggcattttcatcactaccagctgttgcaacatttccggatcgggtgctgacatctccataaaaaactgatttataattaagtcggcaaattaaaattataaattcattttcccgcgcttcttcgtaatttgtaatatctcaaaagtgatcatgcatgaaaatttccctgatactgttaatggcgctttcttttgcaggatgtgtacaacccggagccaagatcagcctggccaattccaatacccttgttgtaaaggatctctttgaggctttcaatgaacacgactggaaaaagctggcagcctgttataaggataccgccactttccttgatccatcctttggaccggatcccgtgcaacgcacccgcgaacaaaccgcccaaaaatacaaagaactgcaacagcaattccccgatattcatgatgaagtggtgaatgtatatggagataaaaatcatattaccgtagaattcatttcatcagccaccggccctgatggcaaaaagtggcgactgcccatctgcaccgtattcaccatagatgatgggaaaattgaaaaagacaatacttattacgataacagtcactgatcatcttttcaataaccctccattttccagcgcatcagacacctgggtagcaaaggctttggcaaatgactcgaggctattcggattataggtttccgactgacccgaccataccagctttccgtcctgtttcaggtcatacaggttactttccaggaaatatcttttatcggtggtgtaatagcccggagaatacaccgagccgtacatatagccataatatccccagaagcggccataccagccgtatgcaggataaggagcataggaaacggtgcctggcacatatctcgtttgggattccttattaaccaatgaggtggttaatacggcggtgtaccctgcatcctgcattttctgcgtagcagcgcttttatctttttctgttagcggattgaatttaggaggaaacaggtccagtcctttcccggctacagcaccccgtttctgaagggctgccgccatctgggtttccaccacctgctgcgctcccacattggaagtaagtgaggccaccagtatattatgatacccttctgcaggggcttccggggctttccaggttcctgtcatatgcacggtggtaccacacgcgccccataatagcactatgcccaccagcatggatttgataattgctttcataaaatttgttttatgtatctacaggcttcattagaacaacaagacacccaataaaaagtttagctcaaaaaatgacaatcctcttttaacaatcggctgtctgtaagtgtaataagatgtacatttatatgccagctaccatgaatatgaacgcaaatagtaaacggggattaacgacgctgttgatggtggacgatgatcaggacgaccaggagttttttaaactggcgcttggcaccatcagggacgaaatcacccttaccaccgccggtaacggccaggaagcgtttgacctgctccgcaacggtgcatttacgccggaccttatattcgtggatatgaatatgccattaatgaatggctttgctttccttgaaaaaataaaagctactccttacctgaaggatatcccggtgatcatgttttccaccagtgatgaaaagcatgaaatagccaaagcaaaatcgctgggtgcagcggattttgttaccaaaccagcgcggttcaatgagctgtgccggctgctgcaggaaaagctgaattcctacacaaaggtataaacgcttaatcttctatgcgttccgcacaggcaaccctgtaaaactcatatcctttttccgaacggccgggtaagtaatgtttccggtattcgctggcgccgaggtcttccagcaggcgaaagttatattggcgaaggtatgcgggtaatgctgccggttcaaaaccaaatgtccatcgttcttccagctctgctacgtctttgagcagtttttcgccaccataaaatgccgaagggttatccagtacggcctggtgtacataggtaaaaataaccctggaaccgggttcgaaccgctgcaggaatgcaaaggtgctgtcgatcgcttccttgttcaggtaattggttacgccctcccagataatggcggtaggcaccgtaaaatcaaagttattcagtgcgctcagctggtcgaggctttgccggttaaaatctatctggtaatagtatactttggctggcagtttatgtgcgcgtaattttgccagcttataggcggccgtattgggatgatcgatttccaccactttcagctggcgcagaaaaggaagccgcagtccgcgtgtatcaaaaccagcgcctagaatatacacctgctgggcgccgttatccaccgcctgcagcaggaggtcgtcgatatactttgtacgggcgatgccggaggataaagcgccggggatcttcttccggataatccattcggcgaaggaccgccagcctggtatgcggcaaagccatacgcctattttcagcctgctgtccaggaaccaggatgcgaatttatcggtgaacaaccgctggtcccgcgagcgggtggtttccagcgcccggaatagggccatatattgcgcggttctactcgtgacgtcttccttcatggatagtgttttatgaactcctccattaatttaatcaaaaaaagcgaatatcgttttgctcctgcccgggccgtgaatttattgaggatcagcaccgggataatttttgcgattatttcaaaaaaatacctatttttagaaaatattctaaatcgcatcaccaaaatgagtcaaccattaaatattgacaaattagacttacagatcatttcggaaatgtccactgacgccggtatctcctatgcagagttgggtaagaagctctttgtgtccggcggcactatccacgtccgcatcaagaaactgcatgaaatgggtgtgatcaaaggcacccgtttacaggttaacctgcgtgctatcgggtatgatgtactggcgtttattggtatttacctggagaaaagttcattgtatgaaaacgtcgctaagcagctgttaaaaattccgcagatcgtgagactgaactataccaccggttcttacagcatgtttgcagaaatcatttgcaaagacagcggggagctgcgtaaaatattgcaggacgatctgcagcatataaagggaatagaaagaacggaaacgattatttcactggaagagagtttctcaagaccgattaacgtgagtgaggtagtataagtataaaacgctttattttatgaacgctgctttataggcagcgtttttttttatgtctttcgttaacggataaacgaaaagctggcagggctttaataccctgccggcgctatcatttagagtttacgcgcgtcgcgggtaccggcatacagctcgtattccagcaggcgacaatcgatcgtactgttgtaaaactctatcctgcgtttggctttaagacctatcttcttagccagttccaggttcccggtgaacacgtatccaaagtaaccaccgcattgctgcttcataaaatcaccgatacggccatatgtttcctccagcgcttcaatttctccaaggcgcaatccgtattcggggttcatgtataccacgccggcagcgccttccggcacttctgtgctggcgaaatcgcatacgcggaattcaatcatatcttccacgcccgcagcctttgcatttttacgggcgtttacaatcgccatttcactcagatcggtagcgataatgcgcagctccggtacttccacgatctgtttttccagcagtcctctttcatcgaggtacacattttcatcaaagccacggaggtgcataaaggcatagttatcgcggaaaagaccgggacggctgttggtagcgattaatgcggcttcaatggcaacggtgccggaaccacacatcgggttgatgaaaggcgctttacggtcccagcgggaagccaggatggtagatgccgccaatgcttccagcatcggagcgcggccaggtattttacggtatccatgccgtgcgagcgagtcgccggtagtatctacaaatatttcagcattttcatttttccagaacaggtggattactgcaccggtaagctccgcaccagtggatggacgcttgcctgttttttcccgcatacggtccactactgcatcctttacccttaagttggcaaacatgctgttgttgatcgtttcattctgcacattgctggtgatggagaagtaaccatcttccggaaggatcgtttcccagggataggatttcagctgattgtatatttcgtcgccgtcgattgcttcaaattgtttcaggctgtacagcacctggctgccgcaacgcaggttcaggttaaggcggatacactcattgagagaggcattcaaccgcacaccggtaacgaatgtttcgtctacagtaaaacccagatcttttacttcctgctccaggtaaggtgtcaggcgtttgttacaggtgatggtaacggttccctttgttgtatataatgacataaggcggcaaatttaccaatctttatgataatccccgtgcattccttattttaacaacttaaacatacctcagcacctatgcgtttttatctttctttgttattgccggcagtcctgtatttcccggccaaagcacaaaccaaagcagtgcctgtgcgtaatgagctcattatgccggtgccggttacgccatccagtcatgcgtctaccattgcggcgttgtcttccggggatttgctcagcgcctggtttggcggcgatgaggaaggaagtaaaaatgtggagatctggtcgtcgcgctttaccgccggcaaatggcaggcgcccgtaaagctggcagatggtattattaacgacacgcttcgctatccctgctggaacccggtactgttccgtacccgggccggtttactttgcctgttttataaagtgggtccaaatccacgggagtggtggggcatggcccgctacagcagtgatgacggcagcagttggtcatctcccgaaaaattaccggagggcatgttaggccctattaaaaacaaatgtatacaactcccggatggacggctgctgcacccttccagcacagaaagtgtaaagggcaaccactgggtatcgcatatggaaatcagcgacagcacgggacatcaatggcaaaaggtggttatagattgcgacacgttcggcgttattcagccgactatacttacccaccgcgatggacggctccagttgctgttccgcagccggcagcatgtaattgccacgagctggtcgaacgaccagggcgccagctggacacccgttaccgcactgaaactgcccaatcccaattcaggcattgatgcggtaacccttcccaacggcgcgatggcgttggtatataaccctacgaaaggcggaagcgactggtctgacggccgcaatgagctgcgactggccgtttcaaaagacggtattacctggaaagatgtgtatcagctggagaaacgtgcaggcggcgaatacagctatccagccattatcgccaccgcagatggtttggtgcatatcacgtataccgacgaccggaaaaatatccgcgcggtaacattacaactgaaataagcttagttccatatttcattggcagcggtaaggatcaccggttcgcggtcagtaaccacgatggtgtgttcgtgctgcgctacaaaaccgcctttgtttccaaccagtgtccagccatcgttactttgattggcgaaggatgaaacggtggagataaaggtttctatcgctactacggaattccttttaaaacgggtgcggttaaaacggacataacagttaaggatatcatccggcgattcgtggaggcttctgccaacgccatgtccggcgaggttgcggatcacggtgtagccagatttccttgcttctgtttctatcagtttgcctacgtctgccacgcgtgtgccacctttgatatactggatggctttataaagaatagcctttgatgcgcttaccagtgcctggtgctgatgaatatcttcgccgaacacaaatgaaccgccattgtctgaccagtagccattcagctccgcagatacatcgatgtttaccaggtcgccttcctgcagtatttttttatcggatggaatgccatgtgcaatttcattgttcacgctgatacaggtccagcccgggaagccataggtcagcttcggcgccgatttagcacctaatgcatttaatatctctcctccatattcatctatttctttggcggtcatacccggcctggcataattcctcatttccttcagcgtaacggctactgcttcactcactcttttcatgccatcgagttctgcttctgtagtgatagacataatgattattttttcaaaaatactgataaaaaaacaaagcccgcacaacgggcgggcttcgtcagattgtttttaacaattacatgaggatgccccactcttcatcccgttcaggataatctttaaaacgctcagtgcctcccctgtctttccagtcggaatctatcaccagcttggaactgataccccccctgggattgcagatgagcgtgatacgcaggcgatcagcttcatacacttccatcatatgatcataaatgatattgatgagtcgctcgtacgatactatgatatcacgcaaatgatatacataaagtttcagcgacttcagttctatgatcttattttttggataaaaagtgatgtagagcttcgcaaaatcgggttgctcctgcacgccgaggaaagtgaactccggcacctttatcttcatctcatatttttcctttgaaggatttggtaatcctttaaggattgttttatcaatgtgttgatagagctttttagacatataggtttgtaattattggcgtgctgcaaagtaatatttctccagatcaattcacctgacatcttcacaagataacatttattggatatactttacaggcacttcatccgtaagccatacaccgttatcggagaggtagaacagtatgccgtctctatgcatatcgccgctgcggatggtgaggatatgcggtatccctctcctgctgcctactttctctgcggtggccctgtcgttggtaagatgtacatgctgccggctcattttctgtaacccggttgtacgtatctgttccaaaaaccttgctacggtgccatggtaaagaaattccggcggtgtagctggtggcaggttcagcgatacttccagggaatgtccctggttggcacggatcattgttttgctttcattgaaggaaaaacgctgcttgtcattttccgccacaacgctttccagttcttccatcgtgaaatgatgaccgtttgctttgcattgctgcaggagcgtgttcacatttgcccagccgtgggcatcgagcgtaagttgtatggtatccggactatgccggagaataaagctcagtagtttactgatagatttgttgttcatgttatttaagttggtcccgtactaccatgagcgcgtaaccgagcaggttatgaccgcgccattgcaggggattttccacatgttcattggaggcagccataccaatgccccatacacggtccattgggctggcttctaccaggatacgttcatgtgtattgagtaaaaaagtttttaatgccgggtgttgtgaaaatttatgatgatttccattcacgaccaggtcaaatttatgtgcgtcccagttagcggcgtcgaagctcttcacttgtcggcctagctttttagcttcatccggtgtgttcaccagcaggatccgctgcagggttacatcatcgttgaacaacctggctttacccgccatcatccagtgttctgccgttttataggtgatgccatccactgtgaaaggagcgtgccaccactgactgaaacagctttgggtaacgctgccatccgcagatgggcgatgcccccagaagaataggaattttattttttctttggcctgatactttgcgatcagccagttgttatcgtacttcatgatgagcgaatttgttttagtatttcaccggggcgcaggaatgttggcggggttaacagttccattgcacaagtgcagggtataaattttgtttacgtcattatgacgcaaagtaaaggaatatttttttaacgtgtataatttttttcgggagatgggaaacggggtggtggaatgtgatggggagaactgggcgaaggtgttaaaaagtagattcgttactcttccccaaaataaatttggattttaattgtacacaatctaattttacacaataaatataaaatactcatgggaaagatcgaaaaattatacacggcacacgctaccgccaccggcggaagaaacggacatgtaacctcatcagacggcgtactggacctggaagtaagaatgccaaaggaactcggcggcagcggcggtgcgtataccaaccctgaacaactgtttgcagcgggctatgctgcgtgtttcgacagcgccctcaacctggtgatcaggacccagaaggtaactgcaggcaccacacaggtaaatgcagaagttagcctgggcaagaacaataacggtggttatgggttatcagtaaagctactggtagcgattccggatgtggaaccaaaactggcacaggaactgctggaaaaagcccatcacgtatgtccttactcaaatgctacccgtggtaatattgaagtagaattagcattgatctaaactccatctcatgaaagtattaatcgtactgacatcccacagcgaactgggtaataccggccataaaaccggtttctgggtagaagaatttgctgccccctattatgtgctggcggatgcaggagctgaagttacactggcttctcccaaaggcggacagccgcctattgatccgaaaagtgagctgcccgaattccagacggaagctaccacccgcttcaaacgcgatgaggcgttacagcaaaagctcgctgctacccttaagctaaacgaagcagatgcatccgactatgatgcagtattctatcccggcggccacggccccatgtgggatcttcacaatgatcccagctccattgcactgattgaaacattctaccgtcagcataaacctgttgcatttgtatgccacgctcctgctgccctgctcaaagtaaaggaccaggatggtgcgccaatggtgaaaggaaaagaagtaacgggtttcagtaatacggaagaagaagcagtacagctaaccaatgtagtgccgttcctgttagaagatgagttaaagaaactgggaggtatttacagcaaaggtcaggactggcactcttatgcgctgaaggacggattgctcatcaccggccagaatccaggctcctctgaagccgtagcccggattttaatggaaacattggcgtaattttgtgttgctaaataagctactttgaaacaactgaaattatcaaatcaactttgcttctcattttatgccctgtcaaggctggtaacttcacattaccagcctttgcttggcgcattggatctcacttacccgcagtacctcgttatgctcgcgctgtgggaacatgatatcttgtctgtaaaagcgctggggcagcagctgatgctggattccggcacattaacgcccttactgaaacggctggaaataaaaaagcttatcaaacgtgtacgcagcaaggaagatgaacgtatcgtgaatattcatttaaccaccgccggccggcagctgcaacaggaagcagcggacatccctgaaaagatcagttgcagcatgggttttaccacagaagaatacaacacccttaaaccgatgatcgacaacattctaaaaagacacgcagatgaatagcctgtttatttcaccgccaccatataccctggatcttcaataatatttacttcaatcacacccgctgcatctttcagcaactgccggcaatccgggctcaggtgccgtaaatgcagcgttttaccggcctgttgatagcgcgctgttaatttattcaatgcttcaataccgctcatatctgcaatacggctgtctttaaaatcaatcaccacttccgccgggtcattaatcacatcaaacttttcattaaacgctgccaccgatccaaaaaacaaagggccgtaaatttcatagtgtttaacgccctgttcatctgtatacttccgcgcacggatgcgtttggcgctttcccacgcaaacaccagcgctgaaataatgacgcctatcagcactgccagcgccaggttgtgcaaccataccgtaattgccgccaccagtattcccacaaaaatatctgcctttggcattttattaataatccggaagctggcccactcaaaagtagagatcgccaccatcaacatcacaccggttaacgccgccattggcaaacgctcaatcaccggcgcgccgaaaagcaccaccgccaggattgtcaacgatgctataatccccgacagtcgtagttttgcgcccgcagaaagatttacaaatgtttgtgcaatcatggcgcaaccacccatgccaaagaaaaccccgttgagcatattggcactgccctgcgccatcgcttcccggttgctgttccccctcgtgccggtcatttcatccaccaggtttaaggtcagcaaactctctgtaagccccactcctgccatgatcaacgcatagggaaatattacctgtaacgtatcaaaagtaaagggtacctgcgggaagtggaatggcgggaaaccaccactcaccgcggcaatatctttcaccgtcctggttgaaatgcccaatgccagcactaccgcaaacactacaataattgccaccagggaggcgggtattttttttgttatttttggaaagaagaggactacggcgatagtcaatgctaccagcccgatcatggtccacagcggatttccgctcatccataccagttccccgcccaccatcgttttaaattgccggaactgcgatataaaaatgatcactgccagtccgttcacaaatccgtacatcaccggctgtggcaccagcctgataaatttgcccagtttaaatatgcccaccagcaactgcaatccacctgccagcagcaccgccgcgaatacatattccaatccgtgcgactgcatcagcgcaatcagcaccaccgccgtagcccccgcgccaccggataccatgcctggccggccgccaaaaacagcggtgatcaatcccatgataaaagccgcgtacaaccccaccaacggcggaaaccccgccagtatggcaaaggacagggattcggggatcatggtcatggctacggtgagcccggccaatatctccgatttataatcgggctgctgcgagaaatcaaataaacctgcaaaaggcttcatcagagaaaattaaaggtgtccggtttaaagaggcgcaaaaatacgcattaacccgtagctttcagctgtgtccaatatattaggcacaggctataatttcttcggctgaattcttatctttctctcctatagttctgtaaaccttatttaattattccacgctatggagaatttcaacattaaccgtcgccgtttcctgaagggggccacggcttcgctcgcgctttctgccatcggcgccagtgcgcttgattttattaacccggcaaaacctttgcgggtagcgctgataggcacaggatggtatggtaaaagcgatttattccggcttatccaggtagcgcccgtaaaagtagtggcgctttgcgatgtagataaaaatatgctgcaagccgctgcagagatggtgcgcaaacggcaggcctccggtgaaacaccgcgtctgtatgccgactaccgtaaactgttatccgaaaatgaactcgacatcgtattgataggcacccctgaccactggcatgccctgcaaaccattgatgcactcaaagccggcgccaatgtgtatgtacaaaaacctatcagcgtggatgtaatagaaggtgaagccatggtggccgccgcccgcaaatataaccgggtggtgcaggtgggtacccagcggaaaagcacgccacaccttattgatgctaaaaagaatattgttgatgccgggttgctcggcaaaatatcgcatgtggaaatgtgctgctactatcacatgcgcaacaatggcaatccgcccgtgcaggcggtgccggaatacttcgactatgaaatgtggaccggccccgctcccctgcggccatacgacggattgcctcatgtacgctggtggcgcacctttatggaatatggcaatggcatcatgggcgatatgtgcgtgcatatgttcgacaccgtgcgctggatgctgcaactcggttggcctaaacgcatcagctccaccggcgggatctacgtacagaaagaaggcaagtcgaatatatcagatacccaatcggcgatttttgaatacgacggactaaactgtgtgtggcaacaccgcacctggggaacagctgctgatcccaaatacccctggtcttttaaattgtatggagagaaaggtacccttgccgccagcactatgtcgtacgactttatccctgaaggcaacggcactcctatccataaagatgtagtatttgaaaaggaaaagtacccggaagacctggcggaacccgctattgaactaaatgcggcaccggccacccgcctgcatatgctggacttcctgggcgccatcaaaaatggcagcaggccggttgctgatatagaagaagggcatatttccaccgccagttgtatcctcgccaacatatccatgcaaacaggacgccctgtagtttatgatccgcaaaaacggattatcaccggcgatccggcggctacggccttgttagaaagaccgtacagaagcccctggatacatccggtagtgtaaatacattcagcactatacataaaaaagaacggcctgctatgagcgccgttcttttttttcttcagtaaaaaaacaaacttattccctgatcactcttacctgcgcaggcgcgttaatcgttgatttaatcttcccgttcgccaggcgtgtatgcttcaccgttacaataccataaggcgtgggaaaagttccctctgcaaattgcagatccccaagatggggcgctactttaatcaccttacaccccggctctatcacggagataccaagtacgtgttccgtcagccatggagttggcccggaggcccatccatgacataaactatgacggaaacctttataacaataagcgccataatcgccgtgaatatctttttgcccggcaggcattatctcatcaatgcgggaagcattgggaagccagtccatgttaaagtcctcccagaacgtagtggcgcccagcttcagcatagcgccccagtaggtccggatatcgtttagccctccctggtaatcgcccgctttggcctttgcctgtagcatatagtatccatagaaagtggaataatcctttacgccaccaacgccgataatttcatcgttcatcttttttgcgggcgccaaacctgacaatgccattaaggcggcggcctgtttggagccattggcatcgggtacattttgcttcagccgggcaatagcggcttcgcacttcttcacggtagcgtcatccttcagtactttgctcaatgcagcgccggcatccagggtcatgatcatcattgcctgtagtcctgcatggatgccaggcttgttttcgctggagggccagtcgaggaaacgtgtgccgtcgtgcaggtcttcactgttattggcatctattttctttgagagatgatccagtaatcctttcaggtacccggcctgctgttgcagataagtaaggttaccggtgtgctggtaccagtcgcgctgaataagtatccaccacatggaatacgacaccatgccattcatatactgcggcagcggcgttatatcgcgtgaaaggtccaggctctttggcaccacgtcgttatacccgaaaactgcactgatagcagaggtttcggggtgcatatcgccgatccatacgaggcggtcgcgtttaatgccatcccataaatagtcctgcatgttcagatgaacggtgtatgcgcccgtcatccagatctggttcagtaacgtatcactgcatttaaaagagcccaggtagggcagatcgcggtatatgaagatggcccttacctctttgagttgcagctccgtattatcatccaacagatcaatacgcacaaaacggaaaccggtattgcctacttccagcttgcccagccacggcacttccactatcatatcgcgcatggcgtgatcattggtggcattctttcccggttcaatatcgctcatcgcttcactcacggattcaccaaagcgtatccgcaactttaccggcttaccggttttatacatcccggtaaccagttgcaagccgccatgcaactctttcccaaaatcgaacagcaaggcaggatgcacggtggttgtgcttttcagcacacacatgttttgatttgccaggtcggcttgtccgttgcctgccagcagaaagcgttgtgcattgataatatttgtacctgcattaggtgtttgccatataattttttcgggagataaatagcgccgtacggtagctgttgcatggactgtagccatacggctgctgtcgaataccggtggcaactgggcccgggaagaaacggcacatagcattatgatggctacctctaagatccggttatatattttcatgtgatcaggttcctttgaatgtaattaatattttactgcgatgagttttacaggacccatcaggccggaagtctgataagcatctttcggcgtatatgggttcacgttactccatgttttcctttcggcagcaggtagtttgctatctcctatgaggcggtttacccaggtatttactaccgttactgttagtttattctctcctttcttcagtgcctgttttacatttacccggtaaggcgctgtccatacgttgcccagcggcaccccgttcagggttacatccgccattacactcacggcgccaagatccaggtatggtgtggattccgccggtagttcatctgccttaaaagtaatttcataaacagcggtaccggaataattacggatctgttcattggtgtgggtactccaatctgtcagctggtcaaaaatcaccggttgagcggggccacgctttgccgcatcaaaactcactttccatggcccctgtaattgggttaaggtgattgccccggggaaattaactcctttgcctgttgccgccgccttcttacggaatactacaaaaccgctttggtaaggggctaacgttaacggcactacggtatgtgccggctgtggtgtaaactccttcaggtcgcgggtttcgccggtcacagcatcccaccattccggttgtttaccctgcacacggaagacaggcgataatgtgatgttttggtccgactggttggtaacaaaatatatttgtccatctgcagtactgcgatgggtatacaacacctgttccggcagttgtgccacatccgcgggcaactgcaggatgttcaatgcctgcggcatgtccatcccgctgagcacctgtcctttgccatatttcctttggcgctcctggccatggccccacagctccgtggccagctgctgtactttggtatctgccgctgggtattgctgtaagctcggagagcgtttgggcgcgggtcccaggatggtggcgccttcctttaccagctgcgcaattttctccagcagctccggccgcatggtttcgagttgcggcagtaccagcaaacgatagctcataccgtccggtaataccagcctgccatcctttacacgcaggcgctccaggattacttccgcattgatgtagtcataggagtatcctttcggcagttcaggatttcttacaccagtcattttaggcgcatcttccccgatgaagtaagcaatatcatttactgttttgccttgttgtaagaggaaattacatctcctgatataatctataaatgctttcccctggtaaaaccaggtattcttcctgttaaactctgtcccaaaacctgcgtttacaccgggttcgcgatcatcatagggctgttcaataaatacatgcaggaggctgtgattgatcccttcggtgaaggaccagtcgccacggcgcttcagcaacgcgggatagcggccgtatgtattaccaccggcggtaaaagactcggcagccactcttgttttaccataaatatgcgccgcggaagaagcagcccggcactcgatattgcccagtgttccttcgttccagaattcaccgcctatttcatccgactggccaccgtacttcagaaactctgatgggaagccccagtggccatagttttccagccatagcttcaaaccatctttatgactggctttgcgcaaaccggctacatatttataagccacgcggtcggcaaccaggcggcgcaggtcccagaggaagcggtccgactgatcaggcgagctcactacccttccggataataccggcagccatggtaacggatcgtagccatattgtttttggaaatcatccgccatatcatcggtccagttttgcgaaccggtttcgtagctgtctgccactacccacttcaatgaagtacgctctgcttcggggatgcttttgcggatcttacctacaaaggcatcgtagtggtactgcgaccatttatcgctgatcttatctatttccaacccggttccttccggtgaagcaggaccattggtgacgccggtgggcagcatgccatagcgcaccaccagccagtcgcccgcaggcaccttccatgtaagcgtaccgttggcggataaatttttagtgagattaattgctttggtgggatcgatgatcaaaccggcgccggatatttccggctcgggtggccactgatattcgttccatagcggcagtggcgtctggaacattttggccagctgcttttcttcaaagcgttcgatgcgtggcgccgaaagcagctttacttctgccagcgaaggattgccttcgctgatcaacagccggaactgcctgccggtggtggcattaaaggaaacggcgactggtgcatacggtttaaagcctacattattttgcggattactgcggtccaactcaaagctcttcactgttcgccagatgtccccttctttcacctgcagttcaaattgtgctttgaaaggtttttgggccgggtaaatgatgaggcttcgtgcagtgaagtcgccggttacctccagatcgatgtgcgcgggtgttgggcgggcaacaggcgtggtaacaattacttcttcggtagtatttccgtctgtcagtttttcaatatcccggaacgcgatgttagaagtgatgtgtggcgtatgtttcccaatatcatctccatcgccgcctggcaccgggaaagccattacagccaccgtctgaaaatcagcaggtcctggcggcagttgctggttatattcctgtggaccatgaacagtaatttcttcgccggcgaggtagcgcatcgattgtgatggctttatccaggggccgccactttggctccagccggggctgttgaacaagccgatatccagtcctttttcagtggcagtgcgtatagccgttcgtgttaccttccaccattcatcggaaaacagctttacttttccgtaaggaacctcttctttcggataacctatattaccgataaaagcccggccaatgcctactttcgccatagcttccacatcctgccttaccccatcctgtgaaatattatcactcatccaataccagtatacacttagctttgtactgtctggtggcgttataaaaccacgctgcaaaggcgtttgttgtccgctggcagttaatgcagcggttaacagcaacacagcggcagcatattttcttatcatagtatttgaaaattcgtttaaccgtaaaagttatagcgacaggcacccggttgccggactgttatccgccaacgaacccattgcagtatttcccaaagtaaaaaacgttatcagtataactgtcctgtacctccctgtagtaaaggattaccggggttgagcatgcccattctaccaagccacttcatggtgatctgcatccatacatctaccggcagcttcaacacaaagccgtggttgccttcggggtaaatatgcatttccgctggcacgtgctgatggcgcagggcctggtaaaacaccaggctgttatctacatctactacagtatcatcgccggtatgaaagaggatagttggcggtgtttgaggcgttacctgccggtcgttcgagtaattccttatagcttcttctcccggttgactgccgagcagccgcaaacgggaaccgggatgtgcgaggttcttttccatgctgatcaccgggtataccaggatcataaaatcggggcgcagattgatgccggcattggcggccagcaccggtttattgaagtgcgtacctgttgtggaagcgaggtgcccgccggcagagaaacccataatgcctacacgattattatcgatgttccattcagcggcatgcgcccggatcattttcatcgcttcctgcgcatcctgcaaagggccggtacttttatcctgcatgatcttatcatctggcaggcggtatttgagtacaaaggcagcgatgccctgctttacaaagtattcggcgatattgagaccttcccgctgcagcactactgcgcggtagccaccaccggggcaaatcagcaccgcagtgccggtagctttgtctttgggcggcaggtaagccgttaaagtaggtacactggtatttgtacggttattgtccttgtcggttacttcctcatccggtgcggcaattccgccgggaggaaggccattatataaaggcattatggtttgcgcgttggcaacaatggtaacgaagctgaagagcaggataaagagggcacgcataagtttatttattggcagtaatgataatcaaaacttcataaagtagcatcatgtgtcaccgaataatatttcagttctatcaggtcgttgggcatgggcttgctgttccaggcggaatggatggccagtgcggctcccatcgcagtagcctgggccatggaggcggcaaagatttcaatatcaggaaacagtgcagccagcagattcatatagatggcatttttactgaatccaccgtcaacgaatatacgttttacacgggctcctttcagtaccctgctggtagcgatatattgctgattggcgatatccagcatcagctgatgataggcttctgtatccgaagaaaaactatccagatcccgctgcccgaatacagatgcctgcatccgttgcttgtcggcttccagctgcggcgcatcctgtttatttctttccttcagcttgcggatgatgtttccatcgtactctactccacgatacctgccggtatgctgatcaaaatgtgttgcaatacgctttacctgttgttcgtgctcgtaaccggcaaacagccgggaagcctttaccggcttgccctggaaagacatataacataaacaatccgcttccagttcttccggtgtaagcggcgtatcattaaatggatttaagctgatacaccaggtgccggtagatatcagtacaaaaggttcatgaaaatttaccaggtatggaatcagtgcggcggagctgtcgtgcagaccagtacctactgcatagctgttgcccggaaaggccgcgggcattacttctcccgaagaaaaaagaggcgccagcttttccagcaccccttcctttattaaccacgaatgataattgttttgtttaaaatcccacaggttggtatgacagccaatgctggtgatatctgagcaggcaacacccgacagcaggaagctcatgtattgcggcaggtgcaatgcatacttcatgcggctgaatacttcgggttgctcatatttcaaccggtacaactgcatgccggagttgagacttcccaataccggcgacgccgtttgcacggagaaagcggttttgccaccgtaattgccgtagaactgctgacttaaagtctccggatattctttcaggtagttgtacaatggagttaatgggcgcccttcttcatcgatgtatacgaggcttgcgccatacgttgaaaaattgatggctttgatcgttacatcttttctgctgaatacttcccgcagggaatcaaatacggaaagccggaggctttccaggttttcacagggcgcgccatcttcatccacggtttccgtaaaacgggcggtgcgctcaaagatgatcctgtactgttcatcaaagagaaacagttttttgttggtttttccaacatcaaaaatagcaataacgggaatttcgctcataaacacatttaaattacaaaccagtcgccattgttttagcgcctctttcacggatcaggtgatccctcactttttcagcacggtacaacgccagcggattcaatgcgccgccggcctgtatcctggcggcagctaccaaagagcgtacatctgtacggaacgcctgttgcagtatttcctgtgcggtaaccacatcgttgtgctgttgtgcagccagcaattttttacggtctaccagcaacgcctgtgcgtaggtgatcatgattgcttccacagattgcagcagatcttccagcgggtctttcacgttgtgcgaggcgtctatcatccatcccagatctgtagtatgattcatgccgcgggcatccattccttccaccagttcgttgaagatcaggaacagctggtagggcttgatgctgcctacggtgaggtcatcgtcgccgtactttgaatcgttgaaatggaagccgccgagtttaccttccatcagcagcagggctacaatctgctcaatgttggcattaggcagatgatgcccgagatctaccaacgtataggctttagggcccagtttattggcgtacaggagcgactgcccccagtcgcccaccgtagtggaataaaaatttggttccgcggctttatattccacaaacattttccagttatccggcagcgctgcataaatttcctgcaaaccttccagtgtgttctgaaaagcatggcggaaattcagctggccggggaagcaggaaccatcggacagccacacggtgagtgcatcagagcccagttctataccatgacggatcacttctatgttgtgctcgatagcctgtttgcggatgtctttgttgacatgctgcagcgagccgaatttatagctcagctgctgcccgggctgatcctggaaagtattggaattcatcgcatcaaagcggaggccgtgttgcgccgccatggctttaatatgcgcgggattggacggaatatcccagggtatgtgcagggaaatggcgccgctggattggttcagctgatgaatcaacccgatgtcttcgatcttttcttccaggttcctgggttcaccgccgccggggaaacgcccaaagcgggtaccgccggttcccagcgcccagctgggaatgcccacctggaaagatatcagctgctgcaatatttcaggaacatttttaatttcccccgagagatattcaaatgcccgctgctgcgccgccattcctgcctggttatgctcttctatcctgtatttttcgattctcatgataatctttttttacgtagataaaataacatacttatctcacaaaagccattgctactccaccatctacattcagtacattgccggttgccttgttaagtaagccgcctacaaaagcatagcaggcgttggcaatatcttcgggtacaatgatttcgtttaacagcgtacgtttcgcataaaatgcgggcagttcttccacctttacgccatatgctttggcccggccttcagcccaggcgcctgcccatattttactatcggaaattaccgcatccggatttacaacgtttacgcgtatacgatcttttcccagctcggcggcattgagcctgctcaggtgtagctgcgctgccttggcagatccgtaacctgcattgttaggaccggaaaccaacgcatttttgctgacgatgttcagcacatccccgccggtgtcctgcttgcgcatgatgtccacgccggcttgcgtaacgaggaactgtcctttcaccagtacgtcgtacagcaggtcccagtctttttctgtatgatcttccagtggtttggagatcgataacccggcgcagtttacgatgatatcgatgccgccaaaggccagcacggccgtgtcgtaggttttacggatggatgcggaatcggttacatcgagcaggtcagcggcaaacacatctttcccgtacaatttattaaactcttcggtagcagaggccagtcgctgcgcatcgttatcgttgatgaccaccaccgcgccttcctccgcaaactttttagcgatcgctttaccgataccgccggcactgccggttaccagtgctattctgccggtaagcgctttaggcttgggcatgcgttgcagcttggcttcttccagcaaccagtattcaatattaaatgcttcctgccgtggcagggaagtatattcagagatggcttccgcgcctttcattacattgatggcgttgatataaaattcagcggccaccctggcggtttgtttatcttttgcgaacgtgaacatgcccacgccgggatacaggatcaccacggggttaggatcgcgcatagccgggctgttcggatgtttacaggtatcgtagtattctttatacatttcccggtaggcggtaaataacggcgccagggatgttttaatggcggctatatctttcaggtccgcatccggcagcaggttcagtactaacggactgatcttcgtgcgcaggaagtgatcggggcagctggtgcccaggggcgcgagcctgtcaagatcattggaattaataaattcaagcactctcgcgtcatctgtaaaatggcccaccattttctgttgggaagagcagtatccgcgtaaaaccggcgccagcgcagcggcctgggttttacggtcgtcaggcgataatgactgtatttttgcgccgccaaacaccggtttatggcggccggtgttttcttccaggtattctgcgcagcgttcaattacttccagggtattgatataactttcgtaggcggtatcgccccaggtgaacaggccatgagagcccagcatgataccgcggataccgggattttcgtcgaggcactgctttaattgcaatccaaggtcaaatccgggcttctgccagggtacccagccgatagtgccgttaaagagctcctgtgtgattttccggccatcttttgccgctgcaatagcaatggcagcatccggatggaggtgatcgatatgtttgaaagggagaaaaccatgcagaggggtatcaatggaaggcgcttttgaggcgagatcataaatacagtggttaaacaattccaccatttcatcttcatgcgctattccccggtaaatatgctggaggctgcgaagacgatctacatacaaagcggcgaggccactttttttgagcgtgcccaggtccccgccggagccctttacccacatcacttctacgggctctcccgttaaaggatcttttgcggtggctttgcaggaggtgttgccaccaccgtagttggtcaaccggaggtctgcgccgagtaaattggaacgatagatcagcaaggctacttcatcaccagccatagcggccgctgttgcttcatcccataaatagctgacatgcctgaattgcgtggtagttccatctaaagacatactctataatttttacgtttttaattgcgataatgcggagggttaattttctaaagaattaccatatccgaccaggactacagaaagaataatggtgaatatacccagggaaatagtaatgaatgtttttttactggcatttttccattccttcagcacaaaaccccacataccggaaatcaggataataaaagccatgtgcaggatccaggagctggcgtcgttacccagtttactttctcccattccataaaaaaagaattgcaggaaccacgtagtacccgcgatcgccgcaaacaggtagtttttcaccagcggggtgtttttattcgtatagtcgttgaacgagcggttacgcctgttgagcagcatgcaccagataaaattggtggtgagccctcccagcataatcactacaaaaataacattgttccggaacaaagggttggcattattcgctactgcggctttgcccatgctgttgccggcagtaatggcaaaactcatacaggcgctcaggatgccggaaacaatggctacggccagtcctttgcggaggtcaaattcgcggatgctttcggttttctgttcaccggtgagttccttttctttcaacataccggctttcccgcaaatggcaatccccaccaggcataccgccacgcctgataacacgtacaatcccctgctgctgtgaaacatggcccccagtgtattagcgtcatctgtaaacagtccacggtaaataggtggtatcagtgcaccaaaggcggaacaaaagcccagtgccacagccattcccagcgacataccgaggtaacgcatggataaaccgaacgttaaaccgccaataccccacagcacccccaggaaataagtccagaaaagaacagtgccttctgtattacggataatatccataaaccccggaacggttaaccaggcagccagcagcggaactaccagccaggagaagatcccgcccacaatccagtagctttcccagctccacccctttacctttttgtaagggatatagaaacttcccgatgcgaacccacctatgaaatgaaataaaactcccagtaaagcctgcataatgatgtagtaatttgtaacgtggaaacgaatgttccataaaaataaaacatgtaacttttaaaactgtcatggactgtcatggttccggcaggagatagtaattgtagaattaaatcactatcattgtcgtgaaaacagccatgtcagcacctgatagctaattccgcggattaatacctgatgagccatgaaacaacatccgatctttaaatacctttttattgatgatttttctgccacgcctaaatattaccagctggccaactctatcatcaaagctattgtggacaaaaaagtgcagcaggatgatatactgccgtccatcaatgaagtcagctacgcttttgaaatttcgagggataccgcagagaaagcatacaaatacctgaaaggactgggtatcctggggtccgttcccggaaaaggctactatgtgtcgcaaaccaatcttgaccaacaatttaagatactgctgctgttcaacaaactgagcgagcacaaaaaaatcatctatgattcgtttgcagacaagctgggagaacaggccaatatcgacttctatatttataacagcgatttcagtctctttaaaaaactgttatcccagaatattaatgaatatacacatattgtgatacttccgcacttccgggaaagatgggagcacgtagatgaagtgatcaataccatcccgaaagaaaaactcatcttgctggataaaaagctaaaaggcgtaaccggcgaatacggcgcagtatacgagaatttccaggaagatatttacggcgccctggaacaggccagggacaagctgcagcaataccacactataaaaatcatttaccccgataatacctattacccggaagaaatttacgaaggatttatgcaattctgtcagaactatgccttcaacagcaagaaggtggaagagataggagaagaagatattcagccgggagatgtatatattaacctgcgggaaaatgacctggtattattgatagagaggatcatctccttaaacctgaagataggcaaggatgtagggatcatttcctataatgaaacaccgttgaaaaaatttattctcaacggcatcaccactatttccaccgactttaagtgtatgggagaaatggctgcacagctgatactggataactccagggcacagatagaggtacccttttatgtgaccatgcgggcatctttgtaattaccttacctttggctatcaaaaacggaacaacatggaaacaccaggcgcatccaaagacccgctgcacggactaacactggaaaaaatagtgacacatctttacgaaagctatggctgggaagaactgggctaccaggtaaggatcaactgcttcatcagcaatccttctgtgcagagcagtttaaaattcctccgtaaaacaccatgggcgcgtaaaaaggtggaggatttttatgtatattctttacggaagaagttattaaagtagtgtccggaaccggacacgcaccttttcaaaaccggacatccctcctcttttaatctttctttacatactgaaaaccagcattttaatatgatggcatttacttcgcagcaagttagctccatcctataaattgcatttgcatgttcagcagttacattaaaacagctttcaggacgatcacgcggaatctcagctatacatttctgaatgtatttggcttaacgcttagcattgctgcctgcctgatcatttttctcattgtaaaaaatgagttgagttacgacagcttccacaaaaaagcggaccggatttaccgggtaacattcaatgccctcgattataaccccagcacctcgctggcggtagtacctgcgctgcgcaacgattttccggaactggaacaggtatcgcaatactggtaccagggtaccgggctggtaaaagccggtgatgcacgatacaatgaaaaaggatttgcttttgcagatgctgccttcctgcagatatttgattaccactggctggcaggagatgcacgtactgcgttgtcggagccgaaccaggtgatactgacgcaaagtatggcccgaaaatactttggcactaaagacccgctgggccaggtgatcaacctcaacaaccagtttaatcttaaagtaaccggtgttattgaagatgtgccgggcaataccagtcagcctttcgtattcctggtttcctacgaaaccatccggaaggaagcgctggcacaggcctcgttttacagcatcaatggaggcaatgcatttgtattgctgccggaacactataacgtggcgaagttgcaggccaggatgcccgcctttattaccaaaaactggggcgcagatgttgccgccggaacaaaactgttgctgcaaccgttgaaagaaatccattttgaccagcgttaccagagtagtcctgacagtcctaccaccagccgggaaacctattggggccttgctatggtggcattgtttatcattattaccgcctgtattaacttcatcaacatggcaaccgcacaggcgatacgccgtgctaaagaggtaggcgtacgtaaagtgctgggggcttaccgtggacaactcatccgccagttcctgtctgaaaccgcattactggtgttgattgccgttgtgctgggaacaatagctgcaggcattttgctgccttttgtggccacctggatgaacgtgaagatcggggtatcacaattgatggagccggtcattgcagcgttgctggcagcaataacggtaacggttatacttttagcgggcctgtaccccgcctttgtacagtctgcttttcagccggcagcctcccttaaaagcaatacgggtattaccttccggggattgggtttaagaaagatcctggtatccacccaatttggtatttcacagatcctgattgcaggtacgctgatcgttggctaccagatggacttcctccagaaccgggacctgggttttaataaagatgccgtggtttctttccgggttcctgacaaagaaaaacgcgatattttgcgggagcaattattatccaatccaggtgtaaagcagctgagctttgcttccggaccgccggtaggtggcagtaattatgccgcctttacctgccctgaagccggtgtcatcaaggatgatgtaacagagatgaaagccattgatgaacaatacctggatatgttttccatcaaactgctggcaggtgaaaacctccgtaaattaacagatgcagataccgtgcgccgggtgctggtcaatgaaaccctgctacacaaaattggcatacaaacaccggaaaaagccattggtaaacgtttctacatcaatggcagcccctcccagattatgggtgtggtacagaactttcaaagcgaatcacgttataaaaaaggaagaccctgtgtgctggaatacagctccaatggttttagaaccgcctgcgtaaagatacaaccggcaaatatgcgcaataccctttctggtattgataaaacctggtctgcgctctttacggagaacctgtttgaatacgactttctggacgaccggattgccaatttatataaccaggagcaaaaattatataccgccttcaagcttttttcgtctcttgccatactgatcggttgccttggattatacggcctggtggcctttgcagcggttcagcgcaccaaagaagtgggtatccgtaaagtattgggcgcttccctcctgaacatcgttgggctatttgcaaaagaatttattgtgctgatcatcgtgtccttcgtcattgctgcacctgtggcctggtttgtaatggcgcgctggttagacaatttcgcttatcagacccatatcggcggcggcattttcattattgccatcctggtatctgtattgatagcaggagctaccatcgcttaccagtcggtgaaagccgggctggcgaacccggttaaaagtttacggatgtagctacagtttaattttcagccccatttcgcgtttcatggtaagcagggcttcggcattgcctttcgcgtcatctaccgggtgatgtgtatgggttgttttgcgcaggtgtttgaaagtctggaaagtatcttttgtaatgcctttgtacaaactgccgagattttgggagctaaatccaaatggattttcaccggtaaagtgatgaaaataccagcagataaacatccagtcgaacccgttgttatcgctgataaaaatgggccggtccttactaacggagataatccattgtttaaaatcctgcatcacctgtgcgggatcattgaagcccagggtttcctcccgcgtatgattagaaactgccagtgcttcgggaataaatttatcggaaatgggtttcagctgaccgtaaaaagtttggtccagttgttcatttaccagcacggcgccaaaagaaatcatagagtaatcgccgggaatgggaccgtctgtttcaacgtccaccataataaaagccatgtgttatagtttgttaccttggggtcaccaacgcgttatacatctcctaaaaatataaaaaatattatataacaaagaaaaaggcatcccggctatgccaggatgcctttaacgccaaagcgttaacagattctttaatggagccgcccgggttaaactaaattaaccttaggtgtccatgaatattctgtagatagcatgaatacctccttttctttggtgaataatgaaactacaacaaaatatctaaattagaaaacgttacaacaaaaaaataacatatcgttgcagcggagttatgtaaataattgttagccattgccagaacgctggtaagaataaatgaacggcttttcaatttattgcttctttaatgcggtggcaattgctttttccgccagtggccccatcacgaggtagccggctttgttagggtgtacaccatcgtaggtgagctcggctttcaggccttttctttcatcagccatcgccgtataataatccaggtatacgcaattatttttagcagcgtagtttttaaggcgctgattcaggtcggcgatctttccaaccggctccagtcccttgcgccatggataatcaaatgccggtattacggaagacaacaccactttgataccgtttgctttggccagttccgccatcgatacaatgttcccgaaaattgtttccaccggggtaaagccggtattgcccgcgatatcgttggtacctgccaggatcactactactttgggtttcaggttaatcacatcaggacggaagcggatcagcatctgtggcgtggtttgtccgctgataccccggttgatgtagggcttgccttcaaaaaactccgggttcagcttcccccatccgatggtaatggaattacccataaataccacccgttgttcgcctggtttgggcggggttacctgggcattcgcttcttcaaaacactttaaacaggcccagtcctgcttcatcagttcctcacgctgcttcttttcctttgcggcggcatcagcgtccgtggtattctgtgcaaaagccgtagtgcccaatatggcaaacagggctaccagtgtcaggctctttctgttcatgatcatacatcaggtttttaactatctgcattttaataaatgcaacggaaagtaacaatattttcccggcttttacaaacgcctctttgataaccgttaacatgccctgatacaggacagtacaggacagtacaggacgcaacaggacaggaatgtattattcttccgctaaatttatttccgttaagtaatgccgtttcatcaaaccaaattccactcgttatgatcagaacttccaccctttatcaaaaaggatctttctttcacgcacgttttggcatcacttgctccgctctgttattcatcagcactttcacctatgcacagaagaataacgttggcggtcaggtaacagatgcaggaacgggttccccgcttccaagtgtaaccgttggcgttaaaggtaccagccagggtgcattcagtgatgccaacggcagatacacgatttccgccagtccgtcagactcccttgttttcagcatcatcggttatgccagcaaaacttatgctgtgggcaaccgtacccgcatcagcgtacaactggagccaagtaataaagtactcaaccaggtagtggttgtaggatatggtacccagcagaaaaaagatgtaacgggatctgtgggtattgttaccatgagaaatattaaagacatgccggtggctggtcccgaccaggcattagccggccagattgccggtatccaggtgagtacttccaatggtattcctggtggcggtccgcaggtacaggtacgcggcatcggcgcagtgggtgcaggcagccagcccctctacgtagtggacggttatccgctggcatcttcttccgaccaggtatctgatccgatgaacgctattaacccgcaggatatcgaatccatggcggtgttgaaagatgcttctgcaacagctatttatggttcaagaggcgccaacggcgtagtgctgatcactaccaaacgaggcagctccggtattccccgggtgcagctttcagccaattacggcgttcagaccatccctgataaaggacgtccgaacctgatgaacggacaggaatttgcgcagttcagaaaagaagcgattgaagataatatccgtttcaccgaacaccgcgaacctactgatgctgacatacccgaagtttaccgcaatccgtcactgatcggtaaaggcaccgactggtttgatgccattacgcgaacagcacccatgcaggatattaacctgagcgtgagtggtggtaccgataaaatcaggacctatgtctccgctggttattacaaccaggatggggtgatcatcaactccggctacagacgtttcacagtaagagccaatgtagatgccaatctctccgacaggttcaaggttggctttaacgtagccccttcttataccacgcgcaagggtaataccaacggggaaggccgtgaaggcgtttttggtattgcgagtcctatagagcctatctataaagcagatggcagttataatgaatacatccagagcccgggcacttttggtctcccgaacccggtaatgatgctcaatgaagtgaccaacaaatccaagagcacccgtatccttttcaacacttacggagaatatgaaattataaagaacctgaaatttaaatccactttcaacgtagattaccaggaaggaagcgctgagttcttccggccttccactattggtaacaccaatgcagcgccgccaagtattccttccggaggttacatcaccggaaattacctgaactggctgaatgaaaatacgctcacttaccagtacaccagcggcagcgggcatgcctttaccgggttgctgggttacagtgtacaatcacagaaggaacaaaatgtgggcatcaatgcggccaacttcccggacgatgatattaaaaccatcaacggtgcagctaccctcaccaataatcctaatgtaacagataaaacagagtgggcattattatcttacctggcaagggtaaactatgcttataaagataaatacctggtaaccgctactgtgagaagtgatggttcttcccgctttggccccaacaaccgctggggtaccttcccttccgtggcattgggatggcgtgtttcacaggaagatttcatgaagtcctcccgtgtgttcagcgacctgaagataagggcatcctatggcttctccgggaacttcaatatcggtaactacacctacatgagcagcatcggcaccagtgattatgtactgggtggtgcgctgaatggtggccgtgtaatgaacacactcggcaatccgaatcttggctgggaaaaaatgcgtgaattaaatataggcgttgacgttggtttgctgaaagaccgcatctacctgaccatcgatgcttataaaagaaatacacaggacctgctgttaaacgtggaagtaccgcagtccagcggctttaccaccgtaacagaaaacagtggcgacatggaaaacaagggactggaaattggtatctcctcccgtaatatagaatccaaatctttcacctggaccaccaactttaacattgccttcaaccgcaacaaagtgctggcattaggaaaagacaatgcccctatctattccggtaacagcagtgaaggcaatcctaccaacgtaagtattgtaggccagccactcgccatgctgtatggatatgtatttgacggcatttaccagaaccaggcggaagtagataaaggccctgctttccccggcgctattccgggtaatatccgctttaaagatatcagcggcaatggtgtgattaatccgcgggaagatttcgcgatcatcggtaatccatatcccgactttaactggggtttaaccaatatcctgaactacaaaaaatttgacctgcgtgtattggtggttggttctatgggcgccgatcgcttacatgccactaatgactacaacggcaatatcgatggcgtatttaatgtacgtaaagatgtagccaacaggtggagatcagaatccaaccccggcaacggcaaagtacctactaccaatggttccggccgcggcagggtaatgtaccgcgacgtaagttcattgactgtagagaaaaataattatgcctgggtgaagaatattacactaggctacagccttcctaagatgggatttgtggaaagtgccagggtatatgtaagtgtgcagaatgccatcctgtttaccaactacagcggtaaccctgaagtaaccaactacatgggcaaaggtggaagcggcgcactggtacctggaatcgactactccagttacccggttccaagaatttattcactgggcgccaatctctccttttaattcagtcaaaaaaagaatagcaacatgaaaactaagataccttttatcgcgctgcttgcgatcgcactgaatggatgtactaacatgctggatgtaaagccaaattctttttccagcggatccaactattatactaccgaagcacaggtactccgtgcggtgaatggctgctacggcgtactacaggaattttataccggcgactactgggcgatggcggaaatgagagctgataataccaactaccagtatgatgaaagtgaccgtggggctcagcaacgcgaagaaatcgacgagttcctgatcactcctaccaataactatgtgaacaatgtatggacgcagatataccgaaacatacagcagtccaacgtaatcattacccgtattgatggcgtaaaattttccaacgacgcaactaaaaagcagtatctcggtgaagctaaattcctccgggccctgtactactttcacctggtgcgcctttttggcggcgtgccgttgctggtgaaggaagtagcaagcccggatgaggcttccactccgaaaaaagccaccgtggaagaagtatatgcccagatcattgcggatgccacagaagccgctgccaacctgcctgccagctactccggcggcgacatcggccgggctaccaaaggtgctgcacttactttactgggtgaggtttacctgaccatgaaagattatccaaaggcagtaaccaccttacaacaggtaaccacactgaactattcactggtagataactacgcagataattttgatccggcgaagaagaacaattcagaatccattttttcagttcagtacaactccggcatcgaaacagaaagcagcaattatattttcaacttcggtccacgcaacggtaaaaaagacctgaccggcttcaatggcaacctgggcggcgtaaacatgcccactcccagtattgtgaatgcgtacgatgcaaaggacaaaagaaaggatgcatctatttttatgtactccagtccgaccaatgctgctttcgcagaatcagttgcctttggtggcaaactgccgctgatccggaagttctatcatccgccttatgcgcttgatggccgtgcgaatgaaaactggccggtgtaccgttactcccaggtgttgctgatgcttgcagaagccatcaatgaaaccggtaccggcaatccgctgcagtatatcaatcccgtgcgtcaacgggctgggctggatcctttaccggctttaagtcagagcgctttccgcgatactgtttttcacgaggtgcgtgtagaactcgcctttgaagacaatcgctggtatcagttgcttcgcaccggtaaagccgtttccgtaatgactgcccacggaatagaagaaaagaaaaggctgaccaggctcagcccggcatcatataacatacagccgttccagttattatttccaattcctgaaagagaaatcaggttgaatggatttgaacaaaataccggctggtaaaaaaagttggaaaaacgggaaaacgtttactatattactacagctatagtaaacgttttcccatatcaatagcatcaactcaggaacctattcaagattatattatgaccacgttacgtaaaagagctttcccgctgctgttgttggtttccaccgttctgatgaccggtgtggcctgcaataacggaaacgactcaacgtcagagaccaagctaaccggcaatccgaaaatcgatgccctgaaattacctgataattttaaggcagagcggttgtacagtccgggcgacaacaaccagggctcctgggtgtcaatggcctttgatgacaaagggcgcatgatcgtgtccgatcagtatggttttctttaccggttgcagctccctgccgtaggggaagattctgccaagctgaaaatagaacagctaaggattggcaatgatacttccacacagaaagtatctatgggttatgcacaggggctgctgtatgccttcaacagcttgtatgtaatggtgaatcacaacagtgacgaccgtttcgacaaaggcagcggattgtatcgtttacaggataccaacggcgacgaccagtttgataagatcaccctgctgaaagcactggaaggcgaaggagaacacggcccgcacagcattgtattatctccggataaaaaatccatctatgtgattgccggtaattttaccaaaattccggagatgaataactataaagtgccgccatcctggaacatcgacaacgtgttaccatttatcaaagatcctaacggtcatgataatacggtgaatacacatggcggatggatagcgcacatcgattctaccggcagcaactgggaactcatcagctccggctaccgtaatccctttgatcttacttttaatgatgccggtgatatgttcacctatgactcagatatggaatgggattttggtaccccctggtaccgtcctacccgtatatgccaggtaaccagcggcagcgaatacggatggcgtccgggtacggagaaatggtctcccgcctatcccgataacttaccaccgctgctcaacattggtcagggctcccctaccaacctgatctatggcggcaatgcacggttcccggagaaataccgcaaatcattatttgcattcgactggagctttggtatcatctatgccatcagcttacaaccggatggcgcttcttacagggcaggtgcagaagaattcctgtcgggttctccactgccattaacggatggtatgatcggccctgacggtgcattgtatttcctgaccggtggccgcagactggagtctgatctctaccgcgtatactataaagacaataaggaagataacgcacctttggctgcagcagcgcctacagagggcgctaagatccgcaaacagctggaagcctaccacggcggtgcaaaagaaggggcagttgagtttgcatggccttacctgaaaaacagtgaccgctttatccggttcgctgcaaggatagccatcgaaaatcaaccggtaagtcagtggcagaataaagtattacaggaaaaagatcctgaaacactgatccagggagcgatagcgctcgcacgccagggcaaggaagatgtaaagaagctcctgctgccgcaactgatgactatcaactatgggcagttgtcgccttcccagcagattgacctgctgcgtgcttttgaactcgtatttgtacgcatgggtaaaccagatgcagaacaatctgcgcaaatagccgcctaccttgatccgcagtatcctgccactaccaacgatctgaacaggtcgctgagtaaagtactggtatatatcaatgcacccaatgcggtagaaaagacaatggccttgctggccagcgccaaagatgataccgctgccgccaaaactgccatgaaatcagccgacctgatcatgcgtaatccgcagtatggactggacattgccggtatgttatctaaaatgccacccttacaacaaacctggtatgcaacggtattaagccaggctaaaagcggctggacacctgaattacaggaacaatatttccattggttttataatgccttcacttttaaaggcgggcatagttttatcggcttcatcaacaacgccaggaaaaacgcgttagccaatgtgccgaaaaaagagtttgcacacttcaaccagatttccggcgattcgctgttaaacagcggcggtaacctggccgcaggctttgcgcagccgaaaggtccgggcagaagatggacagtagacgaagcacttaaaatagtggacagcactaccggcaaacgtgactttgaacagggccgggcaatgtttgccactgccttgtgcagctcctgtcatggtatgcgtggcgaaggcggcgtagccggaccggatctaacgcagctgggtacacgtttttccaataaagatattctcgaagcaattattgaacccagcaaaaccatctccgaccagtacgaagccaccgtattttctttaaagaacggcagctccgtagtaggacggctggtaagccaggacaaggataagtatgtgatttcacagaatccatttgccacacaggatcagcgcgaactgctgaagaaagatgtaaccggaacaaaagcatccaaagtttcagtgatgctgccggggttaattaaccgtttgaatgaagaagagctgagggacttaatggcttatctgaaatccggcggcaacaaacaggattctgttttccttgctcccaagcagctgggtcgtaaataattttttttggaagataaataacgcgcggatggcattgaataatcagtcgtggcaacataaactctcgaatcattttcaactgggaggtatagaaacggcggtgctggacaacggccccggaaggggcacccgcattgcctggatcaataccggtaccgggctgcgttataaggtagtcatcgaccgggccatggatattgcagatgcgttttatcatcagcatagcctggcctggttaagtcatggcggtattactgcacctacccgcggggcgaacaaaggtttggactggctccaaacctttggcggtggattgattaccacctgcggactaatgcatgttggcggtccggaaaccgatgaatacggagaacgtggtttgcatggacctatcagcaatacgcctgctgaaattgtttccatcatacaacccgacccggtggccgggcagatggacatgagcattaccgggatcatgctgcaaaccagcgtcctcggcgcaaagctgatgctgaaacgtactatttccggcacactcggtaaagcggagatccgggtacatgatgaagtgacgaacaggggcaatatcacggcgccgcatatgttattgtatcatttcaatttcggctggccgctggtagacgaaggggcggacatttgctggaaggggaactgggtttcccgggaaggcaatccggatcacatttttaatgcggatcacaactataaaaaatgcctcgcgccgctggatagtcatgccggcagcggtgaagaagccgcgatcattgaccccgtggcggatgccggcggatggtgcacctgtggtgtacacaacgcggcgctccaactggctttttcactgcggtttaaaaaagcgcagttaccggtgcttaccaactggcagcactggggcaagggcgaatatgtgatggggctggaacccggcacccatccgcctaccgggcaggcaaaggcccgcagggaaggtacgctgctattcatggaaccgggcgaacgccgtgaatatgaattgcagatagacctgttgcataccaacgaagacatcaaatcatttctcactgatcttttataatcattttaaagctcatggaaaaaacaagcttagcagaaaaagcactcgaacagggacaagggattctccggctggcaccaaactgggtacccagatcattttgcgtgccaggacggcggatcaaattacacccggacgattattacgtcctgggaggcgaacgtggcggcatcgatgaacgttggttgtcgtctaccactccggcaaagaacggccctttaacaggcgaaaatgaaggtctaagcatggtggtagtaagcgatagtagtggtacgcagcaatttttactgaaagatgccattagtgcgttaaaagataaactgatcgggaaacgtttatgggatacttatggcgcgtggccgatgtattccaagttctttgataacatgggaccgctcccccaccatattcatcacaatgatgaaaaggcagcgctgatcggacaggccggcaagcccgaggcttactactttccgccacagctgaataatcatggcggtgatttcccttatactttcatgggtattgctcccggcaccacccgcgaacagatcaaggaatgcctgttgaattttaccaagggagataataagatcacgaactactcacaggcttatcgcctggaaccgggcaccggatgggatgttccgccgggactgctgcatgcgccgggtagcttgtgtacttacgaaccacaaaaagcttccgatgtatttgcgatgtatcagtcgctcgtaaacgaagccatcgttcccgaagtattgctctggaacggcacgcccaaagagagcatcggcgattatgatgcattgatggacgtgattgactgggaattgaacgtggatcccaaccagttccagaaccggttcatgccgcctgtaacagcagctaacggggatggttatacggagaactgggtatgctataaatcggatgctttcagcgccaaagagctaaccgtagcgcccggcgccacggtagtcattaaagacagcgccgcctatggcatcatcctcatgcagggacacggcaaaatgggcgtatgggatattgatacgccggcgctgatccgctacggacagttaaccaacgatgagttttttatcagtgaagcagcggctgttgcaggagtgaaaatcgtcaaccactccgctactgatccgattgtgatgctgaaacattttggtccgggtaaccccgacctcgtgttataatcttttaaaaacgacgttatgaaagataataattatccaaagctgcacaatgccacctggccgggcattgtaggaaaaggagatggcgcggagcccatcatttcgtttgatacgttgctggaaatgacagccaacgcagcagtcaatggcgttaagtttgacggtatcgatatcgggttgtttgacccgcacgtatccgcagacagctccgacgatgacctgaaaagactggtagaaaaagtttcctcttataacctggagataggcagcctggtggcgccgatctggcctcccagcggcggttccgcaatgggcagcaaagaagacagggctaaatttgtagaacaggtgcggaagtcgtgccatgtgggcaaacgcctccgtgacctcggcatccggccgagcggtgtggtacgcatcgactctgcctgcagcccggaagactgggccaaagatcccgcaggcaacacaaagctgattgcgcaaaccttccgggaagcatgtgatgttgctgccgattatggcgagagactcgccgcagaaggtgagatctgctggggtggtatgcacagctggaaagcaatgctggatacccttgaagcagtagaccggcccaacatcggtttccaggcagatatgtcgcatacgtttttgtacctgctgggttataacagtccggaagacaggatactgccggccgactttgaatggagcgaccgcgaggcgatcaaagccgggctccggaagctcacacaggcccttcgtccatggatgatcgatttccacgtagcacagaatgacggtaccgtgcatggcaccggctcccacgataaaaccggccgccactgcctcgccactgatcccaacgggaaattgaatattgcagaagatgcaggcttctggctccgcgacgacaagggagaactcacgaaggcagtgaaacatatctgctgggatggttgtatgttccctaacgccgtgatgacccaggcgaaaacctggaacgatatcctcgccgccatgatcgctgtaaggcaacagcacggctggcaggaatagttttttaattataacccgtgacaactatgacaacaaagaaagaactgaggataggattaataggatgtggctttatgggcagaacccactccaatggctacctgcgcgtgaaaaacttcttcccggacctggcatatcagccggtactgaaagcagtatgttcccgcacggaaagcaaggccaaagcgttcgccgcccaatggggatatgaatccgtggaaacggactggaaagccctgattgcacgcgatgatatagatgctgtggacatttgtacgccgaacgacaaacacgctgaaatagccatcgccgcagctgctgccggcaaaatgatcctctgcgaaaaaccactggcacgtacactggaagaatcggccggcatggtagatgcaattgaaaaagcaggcgtgcccaataccgtgtggtacaactaccgccggctgccggctgttaccctcgccaagcagatcattgactccggcaagctgggtcgtatattccactaccgcgccaacttcctgcaggactggaccattaacgccaacctgccgcagggcggcgaaggcctctggcgcatggatgcagacgtagccggttccggtgttgtgggcgatctcctctcccattgcattgataccgcattgtggctgaatggcagtattaccaacgtaactgccatgaccgaaacatttgtaaaagaacgtatgcatcagctcaccggtaaagtggaaaaagtaaacatcgacgatgcctgttccttcctgtgccgcttcagcaacggatcgctcggcctctttgaatcaacccgttatgcacgcggacataaagcattatatacgtttgaaatcaacggcgaaaatgcctccatccgctgggacctgcacgacctgaaccggctggaatactttgataacgccgacgcctctacggtgcgcggatggcgctccatccatgtaacagatggcgatcagccttatatggataaatggtgggtacccgggctgggtatcggttatgagcattcctttgtacaccaggtagctgattttctgaaaagcctggaaaccggcacaccctgttctcctacttttaaagaagcgctggaaacgcaaaaagtgtgtgaggccgtactcgattctgccgcttccggtacctggaaagataccaatgctgcctaactaccggtaacggttatacgcatcattctttctatctccccaggatatacgaaaaaatacaaaacacaataaaatattaattatgctgaaaaaaaccagtgcaatgcttatcccgctggccgcagccagcctgctgtttacgacagccagttgccagaatggcgcgggcaaaacaggcgacagccataccggcgacagcacaggtaacgataaaggcttcgtacagatttttgatggcaaaaccctcaatggatgggtaggcgattctattcactggcgggcagaaaacggtcatattgttggtcaggtaactcccgaaacgttacttaaaaccaacaccttcctcatctggcagggcgatcagccggctgatttcgaactcacctgtgaattcaaaatcaccagcggcggcaacagcggcatcaactaccgcagcgtaatggtggagaatgtgccgcatgcgctgaaaggctaccaggccgatattgatggcgccaaccgctacaccggtcagaattacgaagaaagaggacgtactaccctcgcctaccgcggacagaaaaccaccattccggaagcaacagactcgctgaagaacggcgtaaaaaacaacgcctggagcgccgccgtggtgaccggttcgctcggtagctctgactcgctgcaaacattgattaaaagcgaagactggaataaatgccggctcgttgtaaaaggcaaccatctccaacactatatcaacggtgtactgatgagtgatgtaaccgacaacgacactgtaaacgggaagtccaaaggattgctgggcgtgcaggtgcatgtgggcccgcctatgacagtggaataccgcgatattatgctgaagcggctttagacgcggaggttgtctttctcaggattacgctgattatgttgatttgggggattttgttttttaggattttatttgatttttcttttaggattttattttttaggattttatttttttgattaaacggttgcggcgatggtatgttgatgccattactacagccgttttttcttttatgacagtgacttaccggatacctccgttttcactgcctttttattattatattagccccacaaaaacaggaaacaatgcaattatcgctcgccatagacatggacgaaaccattgccgacccgattaaaaaagccagggcatggtactacagggacttcggcaaaacatttaccacggaagagctgcacggcaaaacactatcagatattttgccggaagaacataaagcgaagattaaggaatacctgaatacacccggctttttccgtgacctggaaatattcccgaacgcagtggaagtaatcagagagctgaataagaaatataaattgtatatcgtttctgctgcaatggagtttcctacctccctgaaagacaaatacgactggttgcaggaacattttcctttcctggaatggcggcagtactgcctgtgcggcgataaatccattgttcaaacagacatcatgatagatgacctgatccgcaatttcagcaatttcaaaggcaggccgttgctgtatcatggacaccacaatgtacatgtagaaggttatgagcggatcatggattgggaagatgcagcgaaaaaactgctgtagttaaatgttcgtacctttaacgtccacttaaatgccgcttatatgggaaagttttttgacgatattaagcccgtacaccaggactttattgctgcgcagaaattgttttttgtagcctccgcaccgctgagtgatcagggccatgtgaacctttcaccgaaggggctggacagcttccgggtgctttccccgagtaaggtcgcctatctcgatattgttggaagtgggaatgaaacctcagcacatctccgtgaaaacggccgcatcacctttatgttctgtgccttcgatggaccgcctaatattttgcgcttatacggtaaaggctatacggtgttgcccggtgatgcggaatggccggaattatcagccctgtttacgatgttgcctgccacccgccagattattgtggcggatatccataaagtacaaacctcctgtggctttggcgttcccttgtatgaatacaccggggagcgggatcatgccgccaaatgggcggaaaagaaaggtcccgaaggcctggaagcctataaagccgagaagaacctggtgagtatggatggcttgcctaccgaactgggtgcataatcattaaacaatattcaccagcgggatgatgtatttgccgatcaattcaatggacttcagcaatttttcatgggataatcctgcgttgtccatttgaaatgtaatcctggagatgcctcccagcgcttcactgtggcgaaggatcttttccgctacttcttccgggccgcctaccagcaacgcgccggtgggacctacctgggcatcgaactgcgctcgtgtaaccggcggccatccccgctcctttccaatccttgtaaaagtttcggcgtagcctgggaaataatcgctgacagcctgttgcctgttttccgcaacataccccaacgaatgcacgcctaccgttaatttatcgggcgaatgcccggcttttctgccggcttcccggtagaggtcaaccaacgggcggaaacggtgggtttcccctcctataatagcgaccatgagcggtagtcccaacgtaccggcacgggcaaatgattgcggcgtaccgcctacacccagccaaataggcaacgggtcttgtacaggtcgcggataaatagcaatattattcagcgctggccggaaacggcccttccaggtaactacttcattatcgcggatattcagaagcagatccagtttttcgatgaagagcgcatcgtaatcctggagactataaccaaaaagcgggtatgcttctataaaggaaccacggcctaccaccatttctgcgcggccacgcgaaataatatccagtgtggcgaaattctggaatacccttaccgggtcggcggcactgagcacagttaccgcgctggacaggcggatatgttttgtacgggctgcggcagccgccaggataacggtgggcgcggaatccaggaattccttccggtgatgctcgccgatgccaaatatatccagcccggcatgatcggccatcactatcctctccagcagatctgccatttcatccatattactttctgcagccgacttgttatttaaaccattcgtagcggcaaagctatctattcctacttccatgacctgtccttttagaaatggtaaatataaacaataaaaaagccaccaatggtggcttcgatgtattaaacacttcaataaaaaattagttcagcacgtaatgcgccagtactttctgtacctcgtacacatccaccgatttgctgaattgctttttgatgctgggcagctcttcaccggagatccagatcttcagttctgcatccagttcaaaagtaccggctgtttccacgctgaacctggaaatgcttctgtaagagatactgcggtattctgttttgctgccggtaagtccctgcttatcgatcaggatgaggcgtttgttggtaaatataaaagtatccctgatcagtttaaaccccagttctacccgctctgaatcgagcagcagtttgccgtaatctttcgttaactgctcctggctaacggtggctgcattgccaataaggcccgaaaaaaatcccatattcaatgacgtttgttgtggtgatgggttacaagatattacaaatattgtaaataacagagcacaatggcgataaattcagcaattgccaccaccctttaagtacgctttaaccatgctttaagtgcgcttcatctacgcttcatccttggtatttctcacaaggccaatacccgatatgaagaagacaattcctataacagcagccaccagcagctgtcgccattgcatactttgctggataaaaccataaccggcataaatgatacccactattcccaggatagtcaggatggttccgaagagtcgttttacattcatggcttatgatatttgactgttaatcaacaatatctatgccgtgcacgaagctatgtcagccgtttggggttattgccccacatctgtccggaacgaagaagcaggcaacccctctgcgttataaagatctcccttcacccaattcttaaatgcgtatctcacagccaccggcgctgctactgcgtcacactgaactttcacctggttgctgtgaacgatcaccgctttagccggataaaaaatatgatcattgcccgctatttcaaaatgttccagcggcttattgttagcggttaatccgtgtttggcgaaattgaaataaagataagcctggcttcctttgatcttcatctttctaaaaaccggcgaagcacaggcaatgcttttctgatgatatgtttttgccagcgcccagtacgaaaggcgttgactcaccacggttttatccggcggatggatgtatctttcttcacctgcatcaagtatcacggccatacctgcgttgagaatatcgttcagcgccagcaattgtgattcccgcaatacggccggcagttgctcatgacgcggatcagcatatccgtagggtgctatctgcacataataaaacggcaaacggctccctccccacagcgctctccattccttcaccatcgccggcaacagtctgcggtaaagcaacggatgctccctgtttgattctccctggtaccagataaatccttttacggtataatctgaaaccggcaggatcattgaattgaaaagaacagatggtgcgcgctcaggatctttctccggatctttgatcgtatccggccggctggtagaccatgcctccgggaaaaccgacagtgttttttcactcatccaggattgtatggcggttcctccccaataagtggcaataatgcctatgggtacgtgcagcttgtcatgcagtatttttgcatactgatacgcaactgcgctgaaatccttcgcggtagcggtatctgtggccttccagctgccgttgcaatcggataaaggtactggtgatactactttgggtacccggaaaacatgtatatccggatgattggccgcatcagcaataatagccgctgcgtttaaaaccggttgtttattgtatcctttcaacggcatctccatattggattgccctgagcatacccatacttccccgatcaatacatctttcacgctgatatgtgttgcttcgctgttaaattcaacggtgtacggtccgccggcacgtggtgtaggaatatgcagtttccatttcctggtgctgtctgcaacagcggtatatttcctggaagtccagccgggtgcgatgttcacctggctgcccttgtccgcccatccccatagcacggcctttgagcgttgttgtaataccatatggtcacttatcactgcaggcagtgataagtgaccggcatgcgactgcggcaaggttctcaacggaaaaatgagcagtgctaaaatgtttaaaagaccagttcttcctgacattgtatttctttcttcttcataaatttaaactccacattctttcccagtaaatcagcagctaccttattatccttgatgcggacgttcctgcaccctgataggaaaaaggccgccttgcgggcatgataaggcttataatcgtagctcctgatgagatcattgttaacaaactgcaacccatttaccgattgtgcaaatagtataggatagtcaaacgcataaaaactatttccttctatctgtatatttttatggtaaagcggtgtgctatcgttcatcaccggaatttccgggtaaatactgatcacggcttctgtaaactggtagtcggaggtgttacacggcgcgagaaatttatttccttttatcagcaaatcggtgatagcgccggattcgtaccaggaatttacatcgccggctatcaggatggccgaaccgctggaggcaaagctgttgttttcaatgatcacctttttaggagtggttaccagcagccctcttgcacggcagctttcaaaagaagtattccttaccgttaccgccggcgtccagctcatattttcgaggccatctccttcattcacatgtgcaggtacttcgcccgccagggtgagttcaaaatcagtggtacttttcttcctgaacgctgttacctttcctttgccgatggtagccagtgaatgatgatctatgaatgcaatattatcgcctgcttccgaccactccatccctacgctcatcggctccataaagcggcatagcagcttatttccggccagcttgctgataatgcgcacataggtgccatgcacgttaatgggatcatccatcaggccgccaaagcgacagctgtcaacattgatattaccacggcaattggaaaagtgcagtccatcatcatgaccgctgaaatatcttccctttgctatatttggaacaatggagatgtttttaaaagtaagatccgctgtgtactgcgatagtatccctaaccctgcacaatggtaaccggtcaccttttccattaagatgttatcgctgtgcgttacaaaaatcatggcatgatcgcggctgttatgccgtaataccaggatgtttccgggtgaaggcttccgccggaagggataatgcaaccgcaccacgccgttgtccattacggtggctttatatccccgccagcccggccccagggcgctgggatcatcgccggttctgtaagcaataagatgcgtgtccttttcgtactccatgatgccggtgattttaccactccagccttcggcggcaaacagcagctgcccgtttacaatggtgtagggatattgcgccgtatctatacgtacattgatatacgcagcggtagtatctgttacaaccgcctgcgctgttaagggaaactcccagtcgatggaaaaatgacggagcgtaatatggctgctccgttcaatggtgaacggctgaatgcggccatgatacacaaattccgatccggcgccttctatcaccagcttcttaaatcccgctatcatgatagcgttatatttcgggttgatatccgatgtattggattcatagtatactttctttaccgcgtgctgcggccagaaatcgtaacggcctgccgggaaaaaaagcagcgggttttctttttgccggcaggcttccagcgcggcctgcactgcggttacggcgtcggcgcgactgcccggccgtgcgccgaagctggttacgtacacggtgtcataggcagcagcgccatacgtgtattgagacaacaatatcacggccagtaaaagatatatcctgtttaaatagctatgcatgatgcggaatattagtagccgggattttgtttcagtttcggattcagatcaatttctccctgtggaaccggccagagataaagggcatccacgaaatgacggacatccagttgctgccccgtcatcgttttaattacggcgccatccatcagctctttggcaataccccagcggcggatatcagaatagtaaataccttcaaaggccagttctatccttctttcgtgtcggataatatcacgcatttgttcctttgttttaccggcggggatggcaggcatgtctacaccttttcttgccctcgcctggttgatggcatcatacacagcggcatccggaccgtttgtttcattctctgcctctgcatacagcagcagcaaatcggcataccggaacacgatatagttcaacggggaatcgccccaattgtagccatctaccgttaatacatgtttccttggcaggtagccgatgaaggttgattttgcgccgcccactttgatattatcataggcaatccctttccatacggagcctggacggataatagtataatccagccgcgggtccctgtctttaaacggattggcaggatcaaatcccgaagcaggatcagtgatcatcttcccgttcttcatctcataactgtttacaagatcctgtgtgggatatgcctggtcccagccttttccgaaagagctctgtggtgccataaatccatcgagcggactgccttctcctaaccccggcgcagcatactgcacatcaaatattacttccgcattgttttccgccgccacatcggtaaacatggcttcgtagttatcatacaggcggtactgacctttgtcgatgatctgcttggctactgcagctacctgttgatattgttttgccagcaacagcgctttggctttgagcatcagcgcagcgccctgtgtggcccggccggtattggctttatcataaacggccggcagcgatttcacggcttcatcgcattgtgcttctacaaaggtcagcacttcttcgcgggtatttctgccgggaagcgctgcacctagttgaagggtatgttcaatcaaaggcacgcctccgtaatagtcggccaggttgtaataaaacagtgcgcgtaaaaactgcgcctctgccagcagtcgtcccttcagggcttcatccatttttatacccggtattttttccagtgccaggttcgatttatagatgccattgtacagctgcacccacttatcatttaccggtgtaatgagtgtaggcagcaggttgcctttggagataccgccatatccttcgaggtagtcgctccagatccaggcgttgggtgtcattccatccgtcatggggttgtagccataaatctggtagttgtgctgcatctgctcatagatagcggtgatgccggaaagcgcgtctgcatccgactgccagaagttagtatctgaaagctgatccgagggctttgaattcaggaaatcttttgtgcatcctgccagcaggattatataaagcgcaagtgctaattttttcatggtacactagtttagaatgaggcatttattcccaaagagaacgtgcgcacatttggattctcaatctggtaatcggtgtaattacctgtttccgggtccagtccattatattttgtccaggtaaaagggttctgcgcatccgcgtacacctgtatccctgaaataaatgatttcttcagccagccagccgggaaattataggagagctgcatattttttactctcaggaaagaaccgttttgtacccagaaggaagatgcctgcgtattgtcgctgttgctgtctgttgtcagccgcgggatatcgctgttggggttatctgttgaccatgcgttaaggaaataggaattgatttcccggccataacgtaccgcgctggtgtaccacaggttctggtaataccttttcacgccggcgatgccctggaataaaacagaaaaggaaacacctttgtatccagcctggagggtgagaccatacgtgtattcaggaattacgcttcccaggtaggtccggtcgctgccattgataacgccatcctgttttacgtccgcgtatttaagatcgccaggtttattgctacccgatagtttttgtttggcccagttatcaatatcatgttgatttttgaaagtgccctgcgcctggtagccgtacaatgcgccaataggcagtccttgtttaatgatagagttattgccgatactttgtattacatcgggattaccctggaaacgcagcaccttattggagttatggctgaagttaccgctaacggcgtattggaaagaccctacagtatttttatatccgagtgccgcttcccatcccctgttctgcactactgccacgttctggtaaggtggggtaagcgcgccgtataaagacgacagtggcaactgtaccaggatgttgctggtgcggcggttgtaccagtcgaacgtaatatcaaaatgctccctgaacaggctgatgtctgccccgatgtctgtagtagcggtactttcccaggtgatatccgggttaggtaatgcctttggcgctaaacctgccgacaggctattgccgaaaatatagttctgtccggcggcatacaagcccatgtactgatacagcccgatgttctggttacccagttttccccatgatcccctgatcttgatatcatctacaaaagacaggtctgcgttacggaaaaagttttccctgctcagccgccatgcgcctgaaaacgacgggaatattccccagcggttaccggcggcaaatcgtgaagatccgtcgtagcgcaggtttgcttccagcaggtatttttctttgtagttgtagttcacgcgtccgaagtaagaagacaacgcataagaagacgaggtacctccgacaatgggttgcgacaggcccgcgctcagctcccaggtatcattggaagggaagccctgtacactacccgagaaccaggcattccggctggtttccctgctggcgcccagcaacacggacaggtgatgatcttctgcaaatgttttatcgtagttgagcgttgtataaaaagtaagtgccaggctgttatcatttctttgatacaatgtagaaggaacagaggcattgcttacggttacttcatccttctggaagttccatagattctgcacagcgccggaatatttgtattgcttgctttccttgttatatatttccgcgctgccgtttacctgccatttcaggtctttcataatttcccattcgccgtataacttggcgaaagagtattggcccacctgcggataaaaccaggtatccatgtactgctgcgggttaatggcattgggactttcatcatctgtgttcctgccgccatatcttgttacaccgtctttcgtcatggtgggcgttacacccggtacggagttggcgctgtagtataacaaggtggtcacatcaaagggttcgttcaccttattccagtaagaattcaggttggcgccaatttttatcttatcacttattttgtggtccaggttcaggcgcagggtatacttggtagcgtctgtggactccatgatccctttgttatagagatatcccatggagagataatagtctgttttctcgtttccgccgctcacagacaggttatgccgggtgataatgccctggccgaagatcacatccatccagttggtattgggaaacaataccggatcggtggcatttttccaggcgtcgatagtagcgggtttgaacaggtccgtattatccgggttatccgctttctggatgcggttcatgagccgcatgtaggtaacgtagtcggtaaccggttcaaagagatgcgtggctttttgtacgccggcagatccgttgtagttgatcaccgttttcccttttttgcctctttttgtggtaacgaggataaccccgtttgccgcgcgcgagccgtagatggcagcggaggccgcatccttcaggatggagatgctggccacatcgttggggttcaggttattcagcgaacctacgataccatcaatgagtaccaggggatctgaattattgagcgtacctacgccacggatgcgcagcacggcgccatcgcggcccggctgacctgaagtttgcgacacagagataccggcagcaagtccggacaatgcctgtgacacatctgtaatggcgcggttttgcagctgctgatcgtagttaatggaagatacagaaccggacagatcttctttacgttgtgtaccatagcctaccactactacttcactgaggccggtattggaaggtgaaagcacaatattcaccgttgtttgcccggccagcggtacttctttctttatataacccaggtatgaaaataccagcacggcattgtccggtgcgctcaggctgtagtgccctttttcatccgtagcaatgcctgtggaagtcccttttacctggatggtaacacccggtagcggtttcccggtgacggcgtcggtaactgttccggtaacattggctgcaacgggcaataccggcgcctttggctttacgataatgattttctcctgtatggcataatcgagcggctgatgtgcgaagcagatatccagtacatcgcggagtgccgcgttctttacatcgagcgttacaggcaccacctgttgcaggtcttcgctggtataaataaaattgtagccggtctgactccggatttcagtaaagatttcctttaaagagatgttcctgccggatatggttaccttttgagcgcgggcggtagcacatacctgcagacatgcagcgagcaatacaatagctgtgagttgcataacctttgcagttaaggaattgagaaggcacaggattccccagcctttgaaatgagcattcaaatacatacatttgatttgggataaaagattacggttaccagaaagaattgttttcttttgccttacagaccgggagcattaggccgcttccggtttttttggctgttgttacagtcagctgttcataactagtgttttaaggtgtgacgattatttttccattgttcattgtaaagtgtactccgcctgttttctcgagtacttccaaaacggttgatacattcacgtcgcgtgggatggagccggtaaaatgacgttggatattacctctgatctccacagctatattatattctcttgacaattgccgcattacggtatggatatcatcctgttcaaaccagaagaggcggtttttccaggccatcactgcattcaggtcggcgtttttcatcacgcggatattcccctggcggcgcagctgcgcctgttccccgggttgcagcaatgcggtggaattgcctccgcttacctttacagcgccttccagcagggtggtattgataactgcttcatcttcatacgccatgatattgaaatgagttccaagcaccgttacctgcaggttattcacggtgactaaaaaaggtttgtctgcgtttttcgctacctcaaagtaggcttccccggttagtgttacctgccgttgcgcccctgtgaaggctgccgggaaacgtaaggtagacgcggcattcagccataccttggtaccatccgacaaggttactttgtattgcccgccgcgcggcgtgatgatggaattatacagtggttcagcagacgcccctgctgcagaactgtacacaaggcttccaccggcagactggatgatttgtgtttgcccctggtgggtaagcaagccgctggaaacgctgtctaatgtaacagacgcaccatttgccaggatgaggatggcttttttctttcccggtgcggcatcattccgggggggatgcgcaacagcgttgtgcgccaccggccttgtgacaggagaacgggaataccagcgccagacgcctcctgccaataacaggaaaactactgcggcagccacctggtaaggcagccatctccatgcttttactttgtgcattggcagcggtggcgtgatgcgggtacttaccgcatcgatcacgtccttgtgcatagcatacagcccttcttcctccgggtggtcatcggtggccacctggttgatcatctccgaaaatatttccctgtatgcatccttctccacatagtccatcaacaggatgatttcatcttcactgcagcggttttccagaaatctggcaaataattcttttacaaaagattcatcaggatcttggttcatatcagctaatacgaacgggcgaagatttacatttacccggaaggaaaaaaaatttatcagcgcaggatcaggtacgccagcagtatgccggcaacatcgcggttggccatcaacttcttttgtatggtgctggtagcctttacgatctggctgttgaccgtggcgggggaaatgcccagcaactcgcttacttctttataggttctgttttccagtttgcaaagcgtaaagatgattttacgctggggaggaagatcgtttatagcagcctgtatgaggtgcatggtttccttttcgtgcagccattcttctgtgtgcaggtaatactcctgcgcagctgccagcaacttatccatgagcagcttgtcccgcttcactttccggtagaagtcgatcaccaggttgttggcggtggtaaacaggtaggaacggaaagatttttcgggatcaatggtatcgtgccggagccagatgtttacaaacacctgttgcaacagctcctgcgcaaggtcagccgatttgaccagtttcaataaattgccgtaaatacgtggactgtaatgataataaagggcatgaaatgccttttcatcccccagggaaacgctggcaaggagctctttttcattgtataactgaacgaatgacaaacgtaccggtttgattacagagcataaatttaatgaaaaaccggtacgggatgtattaattttaggtttcgttattccacatgaaatacttcttccatacccgaccaggtttctcctttagcggctgcatccggtaaaggaagctgacagggagccgttactttccaccattgttgtgttgtactgtcctgtttcattttctccatatctcctttaaaatctgtaccggtatattcaaaatagctgaacaaaaaccagtggtcatttatatttttcaggtagatggaatagttgtggagatgacatgcttcaatcatcttcagcacatccggccatactttggcgtgcagtgatttgtattcggctattttctccggccggagaccggtaaccattccataacggctgttgtgacggggagcgtctttacaggaaaataaggatagtgacgccaacagcagcaagtgatgaattttcataatcgtggtttggttacgaagatagcgggcatcggggaatgataaggtggtttctttgacttatttcagcacgatattgactattgttattaattcgttaagctgatgtgatgctgaggaatgagggaaatgagtcttcttttagtatttacttgcggtatcattactggtttgtatcaagcctttattaaaacagtagttattttatgggttctttctacgatttggattacataattgaaataaatgaaaaaagactggaacagtattcaaacgcttatcaaaaaaacatagacaagtttactaatattctggttatatattccgcgtttgctatctttcttattcctatcgtacaatcccttttctttacagaaacaaaatgcctgtggctacatcatgcttctttttatattttcatatccctattctccatttcactggcaaacactgttcgcctgctaatacctgttgaagtggcctatttacaagaacctaaactctactatgaggaataccggataggttacgaggaagaaaacagggagagaattgaggtagatacgttaataaaagcttcctatataaatgagcttgaagaagctgtaagagtgaataatgagatatttaagcgaaagggattattttactacagagcttttacttttgcaattttagcaagtgttccatatttgttatgcattggttttcagattgctattaaggaggacaaggtgcaaaaagtaaaaattgtgaataatttcagtacctttaacaaaactcaatacatggcaaaagattccaataaaacacaccaaagcagcaccaccacaacaaaattaccgggtgttgataatagccaggtaagaccatccaaaccacaattaattaaggagaactttcaaattgattccgtaaaagctaaaacaactaaaaggtagctcaaagagcactcttattctcctcaaatatctccttaaaactcttattcttctgtttttgaataactgcggaaaacctcgcgtctacaggacgaagcaactgcaaacacaactgcttatcatcttccgttaaatcctgcgtaagcatagccactactttcaatatctgctgctttgcctttttcagcgtttcatcaccggatgcggtgagcttaagtcgctttacccgtttgtcttccttatctgtatactcattgatcaatccacgttcctttagcctgccgaggatattggtgccactggacaaatccaggatattgctgaaaatcacttccgatttgatagggttcttctggttgaaaatagtgaccagcatgccaaattcctcgatctgatcaaggccggttccttccagtgccttattggtatacaccatatgaaatttcccgatcctgctgatcagcttcaccagcgctccgtttaaatccggctgcagctgccctttgaacacaaccgttttcttctttttgatagctgttgccaactgactacgacaaaaatcttcaatagaagcatcgggatgccgctgctcatattctccccatagtcttaccaattcaacggttttattcatagaattacttccttttggaagcaaaaataaatatttaatcccaaataattgtattttacaaccaaatggcattattttacacaataaaacaaccaaataatagtaatgaaactatatctcattctccgcatactgttggccctgcatattaccgggttggtaaccatggcaggcaccacgatagtggattatatcaccttcaataccttctggaaatttgcagacgaaggcgacaaccggtcgctggggctgctccctttaatggccagatatggggcgttggtcagaacaggcgccgctatgttggtgataacgggcatcaccatgctgatacttgtaaaaggcgcatggtggggacagttatggttcaaaataaaaatggcgctcgttattttactggtgctgaacggcatgctcataggcaataaacaggggacgaaattcaggcaaatcgtatcagacaacaccagtggtttcatgcagcaaactgcagatgtaagaatcacgcttcatcgcttttatcttattcaactgggaatcttctttattattattcttataagcgcggttaaatttgactgccattaatacaccggaaaatgagcacagctaaggttatagcactattggcaaccggattgctttccggtgcatttatgtctggttttctgaatgtggttcctgctttctatgaagtacctgtaaatgtacatctcgtttaccgtacacaattaatgacacacaatggcattaccatgcagtcgttgatggccctttccattataacgccgttatggtatgcacgtttacgcaggcgtttaaccccggtaaggaacctcgctattctttctgctgttttagcactcactacattactgataacaagattgggcaacgtaccaattaacggcatcatcaaattatggccgccgcaacatccgcccgttggctggaaagctttactgcatacgtgggacatctataacgcgtggcgtacttttaccgcattgggatgttttatagcctttattgctgcctcccacttaaaaaaagaagagacgctgaccggcagcgtctcttcttcatcataaattaattcatttatcagagcttaatcaccttgaacgtgatcgccttaaattgattttcaagtttaagcaggtaagtccctgccggcagtgaactgatgttctgactgatgcgtgtttgtcctttgctgatacgccagtatttaaccacagcaccgtgcatgtcaagcacagaaagcatggtatacaccggttccttcaattccagggtcagctgccccgttgttggattgggatagaagatcaccttttgggcatctgctgctgccggttccggcgtgtattttacatcgctgtaagccatacgtgcagaagaagaatcggcggatgccaccgggcagttatcaatgctgaaccagttgaacttaaaggtaccggatgtgatatgaataccagtatagctcagtgccggcaacgtgatggtatcgctgatggttttccagactcctccggttgatggcaggttaatgctgccgaaattatagccgctgtgcccaatccatatcaccgacggcaccgtagaggagatccggaagctgatggtatactttccggccgacggtacaatcagtgtgttgtaagtgaaccagtcgcctacatacatataggcaaaattctgtccgccgccaatatcagtgcaggtctgcagaattggcctggtagtacggttggaagcactttctgcctcgtacttattattaactgaacagaaatcgccgacactcgctacggctgtcgcgctgatagaatcacgggatgcagtaacggtgaaagtacctgttgtattaccagccgtgaaaacgcccgttgcgctgatcgtattgccggcgccggtagtggtccacacaggcgtaaaggcaaagaggctgtcgcgctgatcatagcctttagcagtaaactgttgtgatgcgccaaacggtacagcagccgtatccggtgtaagtgtaatacgcgttaaccggggcgcagcaattacatgcgcgctggcggtatcgctgatggttcctgcagtagccgtaatcgtataatcgcccaccacgtttgcctggaacaagccggatgcactgatgctgttgccggtgccggaaacagaccaaaccgggtttatggcaaatacgctgctgtcttgtccgtagcctgaaacagtatactgctttgtggtgccggtaatcattgttgccgtatccggtttaacagtgagccgtgccaatgaaatggaatcagcccgtatgaaacgcagccagttgaagttccagccatctttaccggcctggatcctgatcgttttctggccgggtagtaaacgtataggcgccgacgttactgttatccatttttgccagccgccgcttggaggcaggcttaccgtttgcagggtcgctgtgtccagcatcaccttcaggctggaaagcgaattaacagccacgcggaactggatccggtattcgctgctgtccggtacactgatatcatattccagccagctactggctccaatgtagcttacattcagcccgccaccggtatctgatgtggactcggtgcagcatacattgctgttgccaaaattctctgcctctatttttgcgggtatcggtgtatagttggcggatcgccggttagcaatagccacgcccgttttggtgacgctgtctactgttatggtagcggtaattttagccgtatcgtttagtgtggcaagcccgcctgttgtaatgctgttaccgctgccggtaacactccacaccggcgtaaccgacatcacacgcccgttctggtccagcgctttggcaacgtattgctgcgttttgccgggaaggaatgtcagcgtggcgggtgttaccaccacggagtccagtatgggtgtgcctaatcctttctgggaaatacgcacataatccaccatcatactatccggccaatctgcatccactatattaccacccataccgccgccgacggcaacgttcagtatcaggaaaaatttctgatcaaagggccagtctttccagtcggtatgcggattcgggtatgtcaacactttaacgctgtcgtacagaaaccggatggaatccgcgccccattccatactatacacatgatacgtagtatctgcatcgggtaaaattttggtagcagatacctggccgccgttcgtccagttatggttttgtgtatgtacggtagacagtaccgtgccaaaattattacctacatgttccattacatccagctcgccgcttttgggccagccgccataaacgctgctggtgggcatcagccagatagccggccaggagccgcgtgcacggggcaaccgggcgcgtacatccaccctgccataaaggaaatccattttgccttgtgtaataagacgggcagatgaccagggttcagtagtgtttccgttggggaaatcctttttccctttgatgatcaacttaccgtttttcacacgcgcattgtcgtgtgtggtatctgtatacacctgctgttcgccgttaatccagcctttgggctgcggatctactttccatttggtaacatccggtacgccatcaacattaaattcatcgttgaagatcaccgtccagttagggtttccttcaaatactacattgccttttacattgtacgcagtggtattggcgtttaccagttcctgcccggaaacggtcagttttaaaatagcccgggaataattagctgctgaattgccgctgagcgtaacccgtgcaatggaatcatttacccgttgcacattaccgatagtaacgccgggaggcaggttggtggcggtccagttggcggcagtgagtacagaatcgaatacccctccccgcagggtggcggtgagtactgcaccattttcctgccccattaaaatactggtatcttttacggtgatgccagtgggattaggaccttgtaccaggtcgaagtacaggataccattggctttcttgccatcgatataatgtacttcgatgcggttaaaatctgtccgttgttttacgctctggaaattaaatgttgcttcttcccattgattgatctgggttaccttgtaagtaaagtacaccgctttggaatagttgtcgccaggttgcagcttaaacatgatctcatctttcgtactggcatacaccagcatcttaaaggtgctgttggtggagagatcgaatgaatcagtaagactgctccctgcactcatgtattcaaagcaagaagtatcctttatgaacttggctaccagcggactggtattcagcccggatacactcgggttaggcacgccgaactgcactttccccgtagtggtattgccggcgtagtaggtccacctgccagagcaggggccactaccttccatgttatctaaaagcaggtattgcgcctggagcgggccacacaggaacacgccaagcagcaacactaaaagtgttgagatgtttttcataacgcttcatttaggatgagtaaccgtggatttataaattcgggtttaccaatgcatctacacctggtataggcagccagtaatctgcctgggtgatggccgcagcaggctgcaggtcaccgggatctttaccggcgttggcagcagctacctggtccagccgcacaaggtcgaaccagcggctccactcacctgcaaattcccaggccctttcatttacaaccgcagcagcaaagtcggcgcccgacaggtttgccgccagcggcgccaatccagccctgtcacgtaccgcattgatggctgcataagcttcgctgttgggcgtgcctgttgcgcgtgcctgcgcctctgcatagatgagcaacacatgcgcataacggatcatgatcacggggttgttcgacatgtacactgccttatccccgtcctgctggattgtgaattttttatagtaaggatgtttggtggtggtttgctgccaggggatggtattgccgcctactacaaactccgtggaaaaagtagcgtctttccgtttaccagcagggaagttattgaagaacttcagctcaggaaagaaatcactccagccaccttcattttccggcatagtagaaagaccgtaaaaggaattgtaggtagaccattgcccgcgggtgaaaagcgtgaacacgtcttcctttgtaccgcccacgaagatctttaaaaaaccatcctggaaaagatcgaagccataggctgctttattgtctattacttcttttgctttggccgctgccagagcatatttcgactgatccttcagcggccatccggcttctgtaaggtatacatctgccagcagcgctttcacagaacctttgttgggtcttcccggatcgcgttttttgttgggcacccattgttctgctctcgccaggtcttcttcaatcaacttatatacatcggcaggtttactttttttgagggtaagaaattcaggagaataaatttcagacgggatgatcggaacttctccccagaagcgggtaagccagtagtaacacagggcccgcaggaagctggcttctcccacaatggtttgcgtttttgttgcatcgccatccgttacccgtgagtagttgttgatgatgttggtggtagactggatggttttataacagcccagccagatgggtgtcatccggccgttcagcgaggtaacattgaaacggtcaaattcgcggaactcttctttattggaaccgggatgtgtggtgagatcatcggcgcccatcgtcatagcgatctgggacacgctggtgaatccgctggtccatggcaccattaagctgccatatgcaccggtaagcgcagattcaagtcctgcctggctgctcaatgcctccgctcctcctaccaaacccctcggatcttctgtgagctctttgctgcaacccgctgcgaataacagcgtggctgcgagaaatatctttttcatgtggaatcgtttagtcatgtacgttattttttaaaaactgagcgtaacgcctccggtaaaagttttaacattgggataagaaccgaaatctatcccctggcggatatcaccatcggcggaattggcttccggatctataccgctgtaatcagtgatggtgaacaggttggtagcattcacaaacaccttgataccgagggcatttttcagttttgattttggtatgtcgtaagacaggcctacatttttaagacgcaggaaatctgctttttccaggaagcgggtactttgtgtgaagttcctgttcgtggtactgaaggcaggaatatctgatgtttcattcacgcccggaatatacctgtctttaatttgagccagtgtggcttccctggcatctccgccatagtacatggctgcagcgttattatagttcaatttatcaaatccaaagagtccctggaaaaacaggtttaatgtaaatgctttgtaggtaaccgtattattccagccgatggaagtttttggaatccctgtaccaatcacgccatagtcattggcatctatctttccgtcgctgttaatatcgaggtattttgaatcgcctggtttagcgccaaaatccgcggcctttgcatcgcctggtttccaggtgcccaggtaagtgaggccccagatagcacccagcggctgtcccggcattacaacgaattcgggttgctgtgacataccacccccaattttgcgggtgttcggatcaaagatcatcgttttaccagcgccgatatagattaccttatttttgataaaagaaacattcgctgagctggtccagtttacggcgcctttgtcaattacaacggcttctacagataactcccaacctttattctgtacggtaccaacgttccgggtaatggtgttattacccaggtaaagcggtaacgtttcatttagcaacaggtcgcgggtatcttttataaagtagtctgccgtcaggctaatcctgttgtttaagaatccaacatccaggcccacatttttttgctctgtagtttcccacttcagatcagggtttccaatattacccatgacgataccggtcaggaaagtggagttggtaaatgaggccaccctgttggaataagccgaataagtaacgtaaggagctacgccctggttacctgtaagtccccagctgccacgcagcttcaggttactgagcgctggcatctccttcataaatggttcattcgaaatcacccaacctgcagacacggaagggaaataagcgaacctgttatcaccacggaacttggaagaaccatcacgacgcagcgcggccgaaacaaggtatttatctttataaccatagttaacacggcctacgagggaaaacaaggcccatttggaatagccggaaccaggatttcccggagtaccctgcgtaagattattccactggaagttttcgtaagtaagattggaggcgccggcagatacataattataagtagactgctggtattccattaccgcggttacatcaagactatgcacctcattaaataacttccggtagtttaatgtgttggtattctggagtgtgatctctttgttggaccggatactgctggttgctgagcctgagttggtgatctttccgccgaaacttttgttctcgtatcccaggtagtttgcgccatattgcaggtgatagctcagccctggcaggatctcaaagcggaaacctcctatcaggttagccagcatcctttccgttactgcgagccggtcgacagttaatgccaccgggttgaaaaagagggaacccaccgggtcgttgggtgtgtaggtaccgtcggcttttcttaccggcacggtaggcgaccaggtgatggcctgcgccagtgggctgctggggccatcggcggggatatctacattctgcgcggtactgtaggagccggtgatgttaagcgtggcagataccctttctgaaagacgcgaattgatgttggatcttaccgtataacgtttgtaagaagagttattgatcacgccatcctggttcaggtagttgccggaaataaaataaccggatttgtcgttgccgccggcgaggctcaataaatattcctggctgggcgccgccctgaaaatttcgtcctgccagttggtgccgccattggtgcggtaacctgccacctgctcatctgtaaatggcttcgtggtgcctaccgccgtagcgtgtgcgttggctgtttccgcaaaatcaccggcattcaggaggtccagttttttaataacggtagaagaagaaaaacggctggtgagattcacttttaatgcgcctttgctgcctttcttcgtggtcacaataataacgccattagaaccgcggctaccgtaaatagcggtagcagatgcgtctttcaacacctggatggattcaatatcatccgggttgatcgaaaaaaattcagctcctacaaaaccgtccactacgtatatggggccattgttgctggtaatggagttggcgccgcggatacggatcctgacagcaccgccgggagaaccagccgcattggttacctgtacgccggcagccctgccctgtaatacctggtccaggcgattcactggctggtctttaaacgattccgcggtaaccgtggtaattgcattggtaagctccacccgcctttgtacgccataacccactactaccagctcattcatgctggaagcgctggattggagtataaccggcagttcgcttttagcgcccaccggtacctcctctttaatataaccaatggatgaaacgattaatatggcgttttcggtggatacggtaatggcgtactcgccgttttcatttgttaccacacctttgttggtccctttcacctgcactgttacgccgggcaggggttctcctttcgcgttggtgatacgtccctttatttccttatccggcggcgcgtttgtgggtgtcaccggcgcgtctttccgtttaataacaatcaccttaccgctgatggtgtaagcaagcggctgatccataaaacaggcatccagtgcttctttcagggaagcatctttcagttgcaggctcactttactgatgtgaagcagttgttcatcggtatacaaaaaagtataccccgtttgcttcctgatctctttaaaggctttgtccagggatatgttacgttgcgatagggtaactgtttgtgaatacccggctgcgtgtacctccagtagggtaatggtcatcaaaagcaccgttaatttcataatcaggaacgtttttactgataatcgtggaaattttttgacccacgcagggcttggttgcccgctttgggaaaaaagcgtcaatagcatacatttgtgtagtttgggttgataatgataattgtcgaaagcgattttaattacaagcccggatgttaccgggggcgcagcgaacgctcccggtttttttgggcacttcataactggtaacggaataaacattaaggactcatgacgtcaatgtttttttaacgtggaaaaagaattcagggcgatacgatcagttgttttccctttatttcaaagtgtacttcaccggttagttccatcattttcaacacctgcgacaccggcacattcctgggtataattccccggaagtgggcggatacaggcgctttgtatattatttccacatcataccagcgtgaaatcaaacgcatggcagaagcgatgtcgttaccttccagctggataaatccatttttccaggccactgcttcttctgtatttacatttgccggggcagataacgtgttgttgtttttattaagattcacaccttcgcccggctccaggcgtttactgctgccatggctgcttacgcgcacggccccttccagcagcgtggttttaatctgctgttcatcattatatgccatcacgttgaaatgagtgcccagcacggcgatttccaggctgtcctttccattattggcatgcgtgggcaccattacccggaaaggttgctgcgcgttggcagctacttcaaaataggcttccccgttcagttctacctgcctgttgcggccggtaaaggaaacaggatattttaatgtgctctctgcattgagccatacgtgggtaccatccggcagcgttacctcaaactgtccgccacgcggggtgcgcagcgtattatattgcatcgtcaaggcatcatgtgatgctgcattataagtgtaggtgagttttcctgcgccctggcgggaaatttttgtattgccttgttgcgccaatgcgccgtgtatggcgctgtccagcggtacctgtgtaccatctgccagtgtgagcactgctttgttggtaccgggagccacatcgttggccggcgcaggagtaaccgttgccattggtacgggagccggcttttgccataaccagtacgcggcgccagataacagcaacagtccggaaacaatggctgctgccagccatgcgcgccggtatggcgtacgcacaggcgccagcatttccggcgaacggtcggcggccagtatattgctggctacctggttccagtaagtttcatcgtaatccacggcttcgccggaaaggtcctttcgcagcagcatttccgccagttgagcggtatgcccggtttgatcagcctggatcaggtctgatagttcctggagttcggcagcagtagcagtatggctcacagcctgttgcaggaggtatgctaaacggtcttgtatcgacaatttatgatctgttttgattgttattcagtgaacgtggttgcttcattaaaacgtgtactatgcatacagacgcgcaggtaaatgtttaggacctatggaaaagaaaaaaaatttaacgggtcagcagccataccaccacggcgggaaagaggtgcccggatagctccagttgcttccggataaactgcagggacctgaccagggagttcttgacggtattaggggaaagggatagctcgtctgcgatctccggtattttaagccctttttcgcggcttaaaagatagatccgctttgcctgcggaggcaactgtgccacggcggcgcttacctgtttcatcatggcattgtataccatggtttcttccgtggagctggcagacgcatctgcactataggctgatgtaataatatcgatggccttatgatgtaccacctgtttacggagataagaaaacgacaggtgaaaaacaatccgcaacagccaggaccggggattctctatttcggggagcttatcgcggctgatccataaccgcaaaaatgtttcctggacaatatcatcggtcaccgcttcggttttggtcaaatgcagtatcagcggacgcagctccggaacatacctgcgaaagagcatgcggaaagcggtttcatcgccttccgaaatcagccggaatagttctttatcgttatatagctgcgcatgcatatagactgccccctcgctaatgtaggaaaatttaattgcgaattaatattttcctggaagcggcaatacgaagaagccccggggaaatgaattctccggggctgttatcattcatctaaattcacaatcttatttcatccaccaaacttttacggtattggagttaccgcccatctggtcggattgtgttttattatttacagtattgttgatcgcttcctgttcaggatattgcagcctgttaaaattcacgtaggtagccgggttaccgtcacgtggtgtgcggccggtccttctccataaattataagcaagccagggctggcggaaaaaagataaccactcctgtgcataaatcttatccagcttctgagcgtcggtaccggtaaaggctactttcggattggccaggaatgcggccatctgcacaggcgtaggactcgcaggcgctacactcgaccaggcatcattggttacattggtattatgcgcaataaagtaccagaaattcactgcagaagtaatcccagcagtatattccgtacctgcggttaccatgttcttggctacaccaaggccacgggcgtatgcctctgctttcaggaaatgtacttcggcagcagtgaggaataattccggctgataataaatatctcttacgatataataattaaagggagaaaatttgcagttgtctttgttggcgaaattggcatccctggtatcctggtaaggattgttattatcacctaccgtgctgcccggctgaagtggcgcccagttgccggcctggttggtttcaaagaatagtactgcgcgcggatcaaagatctgtgcggtgtttgtgccatctgccatcatgttccagcaggtagtgcttaaacgcacaaatttatgtgaggtgaaagaccagaagcggctgtcgttgagcacatagccacccagcttgccgggccacataccagcgtcttcaccctccccgatcagcggaataccacccagcgcatattggaggtaaggcgtggcggtagctgcatctttttccactatttgcatagcataacgcagcagtaacgaattaccaaacttctgccacatgctgatgttattggcaaataaagtttctgaagcgcccagcgactggtaaggctttcctcccggcgtgttggcagcggtagttaggtgctgtgacgcccacttcaactgctccagcaggcttttgtaaatgctttcctgtgaatcgtacttcggacggtaattggcggtattataagtatatgcaagccctgcttctgagtaaggaatatccccaaactgatcagtgatgcgcagcgttttataggcacgcaaaatgtaagtgatggcctgcacattatccatttctgctttatccccggcatacgcatttatcttatcctgtatctggttcaggttctgcagcgcgccataataatcattccagatatccagcgcaccgttttgcaccaggtaaccggaactgccgctgatagtagccagttgggtaaccgggtagtagtattcgttatgaatggctgcctgttcctgtcctttcaggaacagggtgctgatcacaccgtttatcattggcggtatggtagtactggttggcaatcccggcgtggtgttgatctcctggaaatctttggtacaagcgccaagcgtcatggaaacaccggctatataaaggaatattttctttgtgttcttcatgttttgcacattttaatcggtgagtagatctgttcctttagaaggaaacccttacctggaaacctaaggagcggaagctcggcatagacataaattccagtccctgcgcattgcctgcaccgtttacaccttccgggttgatatgatcgggcaatgaagtgtagaggtaaaaaagatcccttcctacgagcgacagggaagctgcctggaatacttttgttttcctgacaaagctttgtggtacctggtagttaacagaaatctctctcatcttcacccaggtattttccagcacagcgcttttgttgatccagtcgcttcctttcacaccggagccgagatcggtactgctccatacgccgtaaggcatgtatttataatagtaatgcactacgttatcgttcacctttccatcggggaacacacctggcaataccacgccccagttggtttgtgtgccattaggtgtggtatatggcagcccgccgccattcctttctttcagtgtttccggcgcctggccctgttgcataatggtagcataggtaccggaccagatgtctccaccgatttttgcatcaatgagtgcgcttacagaaatcccccctttgaatgtaaaggtattggtgataccgccggttaatttaggtgtagcattacccaaaggcaccaggccgtcggttgcctggtacatggtaccgttcatggctgcatttccgaagggattctgcaccatcagcggcaaaccggttttggggtcgtagataaaatcatgaccgtaaatggtgccgaactggtcgcctacccttgcagaaataaccgggccgtgtgagccgccatcattccaggcactggccatatccacacgatccgtaccatcagacaatgacaacagcttgttattgctgtgcgccaggttcagcgctacatcccatccaaattctttgcggtcaattactttagcgcgcaggatcagttccatgcctgaattttcaagcacaccggtgttcaccacaatggtgttcaccccggagctcattggcaatggagagctgagaatctggttcctggattttcctttgtaatacctgaagtcggcattcaaacggttatgcagaaagcctaacactacgccgaagtcggcagtggtgttaatagccggcttgaagtccttcgccggcagggagcttggcaacaggttagccgcctggcctgcgaatgttaagctggaataattatagttgatctggtaaggtgcaggatctactgctgcctgcgcccacgctacccttattttaccaaagctcaggaaagccggatctgtcttcagcagatcagaaaatacaaagctacctgcaaaagaagggaagaaataagaccactggcctttgggcagggcagatgaccagtcgttacgaccggttacatccaggtagagaaaattcttgtatgacaggttaatgaaactgtaaacagaattcatgcgcttgcgcaactggctttctgttaccgggtgcgggttaccgagataagtaccggtgttcagtgaatatacattggggatcgcccagttgtcgttgtagttaaacatgccgtacatgtcgcgctggtaaatagttccacccagtgagaactttgcattaagcacaccattcagcaggttttccttatgcagcgttccgatgaaatccatgttggaagcgttgtcctgttctgtaccatgaccataataccctttggtgatgcctattacatccgtcggtctgttcttgatggtcagctcgttggtattattatccaatcctcccctgaaaacaaagtccaggaaatcggtggcttcataattcagctgtacgccggccagcaatttacgcctgttctgaacggtattattttccatgatgttccatacggtagcgccgccgttacccacccatggaaaaccggagagggtattttgtgaaccatcttcatttttatagataccaatatcttctccccggtagttccggcctgcattgtataccaggcgcttcatccaggaattggcatcgtcgttacccagttgcggagggttatgatactggttaacgatataggaagaagttacctgcacgcttacccttttcgtgagcttcatgttggcgcccaggttgaaggtattgcggtaataatcactgttaggcaataccgcctcgttatccaggcgggaataggatgcccggatagagccccattcgttaccaccggaaagggatacattatgtgtggactgtgtaccgttgcggaacagcagtttaatattatcgggttggggcacatctgcctgttgggaaccatcccaccaggtaattgatttgccttccatttttggaccccaggaaagaccggaaccggcccatcccacctggttgtaggtattcacgccatacgggcctgaccctgttttaggatccacgtacatgcctgtccagccttctgttaacttagggttgccgttggcatccgttaaatattgcggtggatctaacgacaccataccgcctgcgccatattggttctgcagttcgaggaaacggtatggatcaatatttttataaccgtaggtatagtctacaccaagaccgttgcgtttagcgcctttttttgtggtgatcaggattacgccgttagcgcctttaccgccatacaaagcagcagcggtggggcctttcagtacactgatcgtttcaatatcttcgggattgatcatgttgatagggctgccgaaatctttcggggaactggtgctggcagcgtttgcgttgtttccggcgtacatggcgctaccggtaggtgcattacgcacatcgtaaggctgcgcgaggtcgttggccatcggcataccatctacaatgatcagcggctggttatcgccctggatggtgttgttaccgccaatcacgatgcgggtggtaccaccgtccacaccattgggactggtaacattcacgcctgccatttttccggccagtgcattcacaatattgggcgcattggatttggccacttctccgccttttacttcttcctgtgaatagcccaatgttcttacgcttcttttaatacccaatgctgttacggctaccgcatccagcgaggtggcggaagtagccattacaatattcagcacggggttggcgcccacggttacacgttgctgggcaaaaccaatagaggaaaaaacgagcacatcgccttcctttgcctctacttcaaagtgcccgtccacattggtaacggtacccctgttggtacctgccaccattacattcacacctggcaacgggctgccgtcgctggatttcacgactccattgatcttctgaaaaagcacattgaagccctctatattcatggaggcttccttcttcagcacaatctgctcattgatcacttcaaaagtgatgtgcaaaggagtgagtaaacgctgcaacacttcgcccagctgctcatcgctggccttcacggcaacacgctgtttggctggtaatgtgctgttgttgtaggtaaagtttacagctgttttttctgtgatagctttgaggatattacgcaggtcggtgggcggcatgtttaatgacaccttctttgtgagcacctcctgggcatgcacatcccgggcgaatgtacaagtgatcaggcagaacaataagcctatttgtaatagtgtaaccctcataaaaaatatgacagtccggttggagtttgcaaatttgtgcataacttcaagtgttttgttgtgattaatgaaaacgttaatacgacaaatcctttcctgcggcagttgtccagacgttacaggaaaaaattacagggtggcggtgttagtgcatcgcccctttttttggttgataatcaagtgaattcagggatcattttagcggaattacaagtgaacaatacttttaactacacggcttcccggtgatatatacctggcccccgctgattttatagctggcattgatagcagcacaaataattttcagtttgttttcaaatgattcattggtaatggtagtggtgatcatgcacttaccaaatacttcctcgctcgcgttaatttttatactgtaggccgtttccattgcgtggaatatgtcggttacggcggtattatcaaatacgaaaggcggcggttccacggcaggcaatagcgctgccacatcgctggtattcagcgaatcggctacaaatgccgccgtgcggatattaaaacggattttgtgattaggcgttaccacgtaactgcgctgttctttatcggccaggttgtacacggctattttaccggttttaacggttactgttaaacttccgttttctgcggatacccggaaactcgttcccaacaccttgatgcccacttcaggcgtgtatacaaagaatggcctgccggcatctttggcgatatcaaaaaacgcatcgcctttcaggaatacttctcttttggactgtaataaaaaggcatcgtgccggatagaggcgcctgcttttagtactacggtggaaccatctgttaaccaggctacctggttggcatcggtggtattaatgcgggtgagctgctcatcttccatatggcttttcagcttagcggctaccggtgttttgttgtcttttttcaggtagatggataccaatgtaatccctgccagtactgcggccgctgccccccaccatctgtagcgggaaatcgttctcacgcgggttggcgcccattccgtagcaggacgttcttctgcaatatgttcttccagggcggcgtacacttcctgcagcagcgattcctctactgcgggttgcggtacgtttcccaatgtcagcaccatactcctggccttttcgagatccgcggcccgttcagggtgcgctgccacccactgctcccaccgggcggtattggccgcatccgggcgtaacacccattgaacaaagctatcgtcccggataaactcccaggtatcctctccaaaatgcttcatgcagctgttttttctgagacaattaactgcccctttatcacaaatgacaaagacgccgattttatactcaaaaaaattaaagtttttttaacaaaggctgaaatgccctgccatggcggagataaaataatcagataaagaagtaaaaggtttccagcaggcgcctggcaaacggagtggtttccagtgtttctttaatgcgccccagggcgttgtaaaggaggttgctgacagactggtacttcatgtgcatcaattctgcaatctgggcattggtgaagcccatataaaaacggagggtgataatttcctgttgccgccgcgataatttccggatcgcattgtcgagcaatatactgcgggaatcactgatttctgcgtcaatgatcctttcttctacggtagattctattgggttatgctggtgaaggaatttatcctgtttatcggaggcagaccggtattggtaattggccctgatcagtttgtacttcaggctgcggcataaataaaaccggatggccacgtcgtcactgatagtctccctgctgttccatatctctataaaaagatcctggatcatgtctttcaacttctcccggtcggtacaaaatcggaaaccatattgaaacaagtgcctggtatattcgcggtaaatcagcgtaaaagcggttttatcaccggctttaaatcgcttccataaagcagcttcctcaaaacaaacgtcttttcttgcaggcatgcgtggctcttttacagcaaaactgattactgattctggtattattggctggctaaaattttggatgtaaccgaaatgtaaatattttttgtcaatcggtcaaatatcattcaaataccacaaaggaaaaacataaaaatatcagtaaccctgtatctccctcattcagtcagcccttaaaatcatacagattttttagtatatttatcttaacggtatacacaccttaattttcacgtatgaacaatctttcgaagagacgactttttgatgctgtcgcctggcagctggcccaattccctaaacctgatatgctggcggctaaaatcaacggacaatggaaaacatatgacaccgctaccgtcagcgaaattgtaaaccgtttcagtgcagggttgttacaactgggtgttgggggaaacgactttacgcctgaaggcgccgataaaattgccattatcagcaataaccgcccggaatggatattcaccgatctggcggtacagcaaacaggcgcggtgctggtgcccatctaccctactaccaaccccgccgaattacagttcattctgaaagatgctgccgtaaaatatatgtttgtgagcagcccggaattgctggataaagtaaacagtatccgggaaggggttccttctttacaacacatttacacctttgacgagatacccggcgctacgcactggtccactatttcaacacaggctactcccggtttgctggagcaggtggaaagtattaaagcgggcatcgacccgcatcacctggccaccattatttatacgtccggtactaccggcacgcccaaaggcgtgatgctttcgcacaacaatattgtttcgaatgttttattgtccaaagaaagttttccttttgaagactcaccgcagcccagtaaggtattgagttttttaccgctgaatcacatttttgaaaagtgcgttacctatatctacctgtacagcggcatcagtatttattatgcagaaagcatggataccctcagtgccaacctgaaagagattagccccgatggctttactactgttccacgtctgctggaaaaagtatttgaaaaaataatggccacaggcagcgggttaacaggcatcaaacgtaaactgtttttctgggccgtatcgcttgccggtaaatacgataataatatcagtggaggcgcgtggtacaatttccaactggctattgccaataaactggtgttcagtaaatggcgggcagcactgggtggtaagatccggtttatcgtaaccggtggcgctgcctgccaggaaaagttgctgcgcatttttaacgccgcgcagatcccggtttatgaaggatacgggcctaccgaaaacagcccggtaatttgtgtgaaccggaaaacgcgcggcgatacgaagtttggtactgtaggccctcctatcaacggtattgaagttaggctggcagaggacagtgaaatttgtgtaaagggtccgtctgtgatgatgggatattataaaagacctgacctcactgccgaaacagttattgatggctggctgcacaccggtgatgtaggattatgggtagatgataaatttctgaaaataacagaccgtaagaaagagttgtttaaaaccagtggcggaaaatatgtggctccccagcccattgaaaataaatttaaggaaagtccttttattgaacagatcatggtagtaggcgccggtgagaaattcacgggggctttaattgttcctgcctttacctacctgaagtactggatgaaccagcagaatattccttataccaccaatgaagccgccgttaaaataccgaaggtattggaaatgtaccaggaggtagtgaacaactacaaccagcattttaatcacgtggagcaaattaaaaagtttgaactgctcaccgacgaatggagtatttccggcggggaaatgacgccaaaactcagcctgaaaagaaaggtggtaacggagaaatataaagatgcgatagcaaaaatatatagttaggaagatgatttccggaactccttcacgatccgtatcaccacgggaatggtaaccgtaaccacaataacaacgataaaatatttgagataaggtttcaggaaaggcatgctgccaatgagatatccggccagtacaaagctgaagccataggctatggagccaatggcagcaaacaaaaggaaacggcggaaatcgagcccgatcatcccggcaacaataggcgcaaatgtgcggatgagcggaagaaagatacctgctgttagtgtggtagcgccgtactttttataaaatgcttctgctgatacgaggtactgccggcgaaagatgccggagtcttctttgttctttaataaatgtcctgttttccggccaatccaatacccggttacatttcctgcaatagcggcaatggcgcacagcgcgcaaaccaccagtatattgtaattaaaattcccgttggcggttagtacgccggcggtaaacatcaggccgccgctgggcaggaagaagcagaaaaacaatcctgtttgcccgaatacagaaaggaatacgatgagtaaccctccatagctgattaatgattcagcatccatgttatagttagttttaaggattggtattcgctgataaaatttcttttattaagatagttgctgtgagcagatcctgcgcatcactgctactcaatttacaatttaaacttttattcattttaaaaagcatacactacgctaattggctgcgtggtccttgattaatttagtcgggtaattgtttgtatctaaccacttttatgttaaccttaaaaagaaagaaaaaatgaagtctaattgtttgttatcccgttgtgcgggactttttttccttgtcagtatgatagcgtgtaaaaagaatgacgcgcttattcagccggttcccgatgcagccaaagagatggtagccggtacattggtaaccacaggcgatgtggcggtccctgtttcctggtatacgctggagttgaagctgataaaagaaacgccggggtttagtcctcctgtggcagccagggctattgcctacaccggcgttacgctccgcgaggcagtactggggggcatgtatggagcgccttcactgggcggacagctgaatgggcttggccgtcttcctgcgccggaaagatggaaacgttataactggaccatagcggccaacagtgccatggcgcagattattaaaaaccttttcggcaatgccagcgtggagaacctcaacctgatcaaccagatggaaagtgataacctgcaggcacattcggatacctgttcacaggaagtgatcaaccgctccatcagttttggcagagccatcgccactgccatttaccagtggtctgcttcagacggcggaaaggatggctacctgaacaactttcccaccgactatacgccaccggttggaccaggctactgggtaccaacaccaccgcagctgcaacgggccatgttgccttactggggaaagaaccgtcctatggtgaagcctacagcagctgattcggcagtgatccagccgcctgcttatgctacagacacgctcagcaccttctacaaagccgcgcgctttgtttacctgaaaggaaaaacacttaccccggaagaaaacctcattgcccggtactgggcagatggcggcggcaccttcactcctcccggtcacctgattgcactcaccatgcaactggtcactgaacaacacctgagcctcggccaggcagctacactttttgcgcaggtaggaataggattgaatgatgcaggtatcctttgctggaaatataaatacaagtataacgtgcttcgccctattacgtatatccgttcgcatatcgacagcacctggtcgccgctgataggcaccccgcctttcccgtcgtacacgtccgggcatgctacctttaccagtgcagcaggcaacatcctggctgcccgtttcggcaacagcttcacgtttacggataaacaaaaagtgccggaaggtttttcgccacgttctttcagcagcttcaccgctatgatcaatgaggcctccatttcaagagtgtatggtggtattcactacgatttcgacagtgaaaccggcagtctcaacggaaagggcctggcccagcggatcctgttgctgaattattaaagaaaaaatgattgtatgttccgatcaggtgccagatgagaaaaggctgtatcaaaatatgatacagcctttcttttctttggagtgttacaaaaaaatatctttaaaactcaatatcatccgctacgttgcctccctgcttttcagcaaacaattgctggtactttgcctggtaagccgcctgccgttgattatacccggcataatcagcctggatatcgcggtggatctggtcattccataaggacgcggcaatctggaaatccccgatgggaataccgtaattgtcaacgatccattgggcgccatccaggccataatcatacgctacctgcctggcaacttccagttcctggtagaagtctttatcctgcttgattttttcgatattgcctgcaccctgcggtgaaggagccgcctttacgccgctgaatttcggatgctgatcagcctggccaaagtattggccgaagagggtaacaatgtgaaaggtggcgtcctgtttcatccgctcgggccaaagcaggttagcttcctgccaaacgggtaactccacccctaaagcctttgctacatcgtcttcacttagcccgctgccgagtcttgcgcaggcagcgccgtaatcttctaaagtaattccgtgaatgggttctaataatggattgccagacataatgtttctatttaaagatgatgattaatcgtgtattcattcattaaacgctcgtaaaatttctcattctctgtcaccatatcgggtactatcttattccattcatcaaacatggcacgcaggtagcgacggtacagatctggattctttggcgtagctgcctcatagctccggagcaaatgggctgttcgctgttctgccaggctgcgggcctgatgcaataccatacgagccccggtggatgggctaaaggtattctgcgactggcaaaacgggcaggtgatataagtatcgataaagaacatcctgggaatagtgatattgccaccacattgcctgcagctgaacttatcacgtatccgttcaaatgctgccagttcttcctggtaagctgattccaggtcctgttctccggcagcgccctgcagcaggctaatagcataatttattttctcttcaaaaacaaaatgccggttcaggcaagccattctgaaagtatgcagcttagcacggtattcactcccggccctggaaataatggaaggcagcgatgcttccgcttcatatacaaaagcaacaatattatcttcccggatctcattcgccttattccgcatctggttaatttgtccgatcagcccggaaagcatatgaatatgcgcacgcttataaggatcggtatcctgttggaaaactttccggagttccggcactgcggcgttgttcatctccaccatgcgggcttccagtttatccaggaaaacaaaccatctctcctgccgggtctttatttcatcgagcagggcagcgttctcatatttcttattgaataaattgaacatgatttatgaattattttccttcctgatattcacgccatccgttagtttggtatccatgaatataaaaccacaataagcgcaggcagtgagtcccttctgatacgcgcgaccggccccgcattccgggcaatcacgaatatccagtttagctgcttcgtttgttatttccccgccataattttcctgggtctctaccttctttttgagctgttccaggtaggcttgtatccgtttcttttcctctcccataatacctgtaagttgaaggttagagtaatttcaggagttcttcttttttagcagcatattcctgttcggtaatcagctgtgcatcgaagagcgttttcagttgtttaagtctttcggtaatatctgttgccggggcgggcttaggctgcatcgctccctgggtaatcatattggtgatcatgcccatggttaccgcctgcctggcgccatctcctatatccgaatgatctttgtccatcgcattggcgatgctatactgtgaaaatttgttcatgtccgttaccatattcataccggtaactttgtcgtattgtttaaggacttcttccggcaatgtgatactggtaatggtgaagcgggtaatttccaggccgaagtccgtaaaatacggctgaatgaggggctgaattttttcatttaaaccggagatattacctgcagcatctaccactgaaatttgtgccagcgcaagtacctcggcaaatttgggggcaataaaatcacgcagctgcaactccagctctgtgatgcccagtcgcggccaggtaccggcgtattctttaaagaacctggatacatctgtaatacgaatattgtacgtaccaaaagctcttacacgcacctggccaaaggtggcatccttcatcaatacaggtgcaggggtaccccatttgaggttaacaaactgatgggtgttaaaaaaataaatgtctgctttaatgggactttcaaaaccgtatttccagccccggagccttgtaagtatagggatattttcggttttcaggatgtgctttccggcaggaaatacatctgccagttgtccttcattcaggaaaagggcatgttgactttcccttacggtgagtactgcaccatccttaatttccttatcggcatctgcaaacttccacattaatgcattaggatccggcgttacagactcaatgatttcaataaaaggtaatcccatcctgaaaggtttttaatataggcgccagggccgtaaataacatggtttcaattcctcaaccggtgactctctttgattgagttaccgtacaaaattaatgcgatcaaccaaaacaataaaggggccaacaaacaatagaaaatgttaatgcaggctaattgataaaagaaaatttgttctcgaatactttaccaattaccggaacaggtttttctgcctggttggctgcattgataattcccaatacccagaatataaggatcacatacccgatcaggccgaggaaagataaagccggcaccaggtgcgccacaatggtcaacgtgatattgagcaggatgctcacaatggcgagtcctaacgactgcttcaggtggtacctgagcaggctgtcggttttctctttaccggagaagtaagcaatcagccaaccgatcagggttacatatgataaaatagataatgttttgctgttcatgggttcaaggtttttttgttggcgttattgcctgtgcaaatgtgtggtgaatgtttattaatcaggcatcccggtatcctacaaaacgactacccatgtaaaaagggcgtctacaatatgtctacaacattttcaaatcatttactctgaacatcttacaaatacagatattcataactttaatgatcttttcataatgactattaccgatttatagtaatttaaccccatgaagttattaccatatctgccatttgtttgcgtgttgatctgtatttgcggatggtcatcttttgtatctgcacaggcgccgttgccggatagtttacaagctctaaccgctgatcccacattcaatgaaaaggaaaagcccccttcacttaaccagctggctgagatataccgggccaataaaaactattccctggccatggctacagccaggcaaagcgttgttctttcactccggcatcaaaattatcttgaggccaccaaagcttacgcgatgctggcaaatattaagttcaatacacaacagtatggtgatctgaaacaaaccgttgattctgtattcaccagcgcgcaacaggccaaccacccggtggcgatggcgtatgccttttatatccgtgcgctgttgtataaaacattggataaatcagacgaggtggtgaagtattgccagctgggcctccggcaattggataagacgcctgacccttatatggccgccaaaatatattaccagctttacgtggttaattcaggctggaacaacgaagaaaaggtaagtacctatgcccgcctggctactgataatgcgctcaaagcaaatgatttcaacctgctgagcaattgctatactgccctttcggtagcccatgaatacaaattcaatactaccaaaaaccgccaggagctcgacagtgtgctgtattacctgggtaaaacggaaacgctctaccaacaataccctggcagggtggccgctaatccctatgccattgcctgtataaatattgccaacagctacctgaaatacttccctgtggaggatgcgagggccaaagcacaagccgttcattatgcgggcgttgcccggacggtgctaaaagatgccgccaacagtgaagaggtggtcgccagcagcctgggcatactcagcgaatatgcccggcgggaaggcaatgaggcccaggccgaaaactacctgctggaagcctaccaggtcatgaaaacggctaacagccattcctattataccatgatcaatgtggtgcaatcgctgtctgatttttatgaacaaaagggcaactaccgcaaagccctggagtttcagaaagaggccacgttatataacaataaagtgttcaatcagcaacaggcactcaatacccaaaagctggaaatacaatatgaaacggaaaagaagaataacgaaatgcagatcctgaaagaacgggagaagagccgcaccatgcaaaattatctgtatgcctgcattgcgctcgcctccctgcttggactggtgttcatgttccgctcatatcatttcaggttacgttactccatgcagcgggaaaaacagctgcaattggaaaaacacgagtcggaaatgcaggtgaagctggaaaaagaagaacacgccaggctcagggccgagcagcagctactggcaacccggcaacagcaactcaaaaaagaagtaatggccaatgtgctgcacctcgaacataagcatcaaacgttactgaacatcaaagacaaattaacggaaggcgatgccgtaaacatgcagaaaatcctcaaggaagaaatggtaatcgataacgattttgaacacgcaaaagtccagatccaacagatacaccccgatttctttcacctgatcaatgaaaaagcacaaaagaaactcaccctgcttgatctgaaactttgcgcctacctttatcttaaaatggatacccggcaaattgcccagctaatgaatattgaagccaaaagcgttagaatgagccgctacaggatcaaacaaaagctgggactggacagagaagatgacctgaatgcttttctgcaggcgttggaaagttaatattgtaaactttaaacaggatatctgacaaaagtgtaaacctatttcaggacgtgaccctatgtcaggacgagtcatagtgtattgggagtgtatgggaagtgtatcatgagtgtatcatgagtgtatcatgagtgtatgggaagtgtatcatgagtgtatgggaagtgtatggggaatgtatagggactatatggggagtatatggggagtacgacacatacgctactcctaagtaactgagaagtatcagagaagtatcagagaagtaactgagaagtatcccatcagttaaataaaaaacagaatatgacagcttccggttattactcagttaaaagaccgcctgaattcaagcggcgacagtttggttttggttttaaacagcttactgaacgactgcggatgttcgaaacccagggcataagcaacttcactcaccgataaagtagtcgtagaaagtttttccttcgccttttcaatcagtttatcatggatgcgctgctgcgcgttttggcctgtgagtgcacgcagcatatcgcttaaatagctgggggacaaatgcaggttatcggcaagatactgcacagtggggataccattgcttaaagaatgctcattaccaaagtaatctgtcagcaggtcgtccagtcgttgcagcagatcatgactgaccgccttccgcgtaataaactggcgcttatagaaacggttggcgtaattcagcaacaactcaatctgggagatcaccacatcctggctgaagtcatctatccggctgttcagttcttcttccatgatcccgaaaatggaaatgatcgtgtctttctcactttcagaaaggtgcagcgtttcgttggctgtataagagaagaacccatactggccgatctttttggctattggataacccaaaaagaaatccggatggatgagcaacgtatattcagaacatacgggtccgtcattttccccgccccccaacacctggccgggcgaagcgaacagcaagcctccttcatcgaaatcataatatccctggccatattttaatttgccggcaagtttgggcttgtaggaaattttataaaatcccagtacatggtgctgcgctggctgcggcagttccgaccaggacggcgccccgttgatcaaactgatcaatggatgctttggctgaggcatgccaaaggcccggtgggcatctgccaatgtctcaaatttatgtacgcttttttcttctttcttcatctccctacaaatataatcataaccggtaaccattttgattaccggttatgaccggttattatttagctattccctgggctgaactggaaatgggatcccagttttcccaaagcgccaggcgttcctcataagccgaacgtacccacggcaggttgtgactgcccaggtggaaccgcaatggcgggttttcagtatccaccacctgaaagagcgcttgtggcgtggcattcggatcccctctttccaggtctcttaattttccgaaaaactggtttttaaagtccgcatagatgtccatgccggcagcgaatttcagcgactcctggctgccaaattctgtagcataagcgcctggttcaataatggtcactttgatcccaaaatccttgacttcagcagcaagactttcatggatggcctcaaaggcccattttgttgagcagtagtatccgattaccggcagtaccacatgccccaggttgctggaagtaccaaggatatgtccgccaccttgctgccggagcagcggtaatgccgcctggataactgcaacggccccaaaaacgttggtttcatacatcgccttgatatcttccgcactcgcttcttcaatagtgcctaccagcgaataaccggcattattcagcacaatatccaatctcccgaaatatgcatgcgcctcgtctatggctgatttggcctgaccaggcttcgtcacgtccaatgcaagggttaatacctgttcgccatatttttctttgagtccggctaggctgtcgatgttacgtgccgttgcagccactttatcgccacgctccagtgctgcttctgcccaaatgcgtccaaaaccacgcgaagcaccggtgatgaaccaaactttactattcatgtcgtttctcatttttattgatctttaaatttttgatgaagcaaagttcaggtgatgccgctggccgtacgtagcctaattgaggacttttgtagtctaattgcggatttgatatgattacccttaaggtgcagctacacgtcccgtttacacaccggataaaaaatatttttatttatgtagtcaactacgtagttttgtactataaattaatacaaatgagtacagcacctgttataagaccaattcacaacaaatattgccaggaaataattgacatcatcctgcctatccagcaaaaggagttcaatgtgcctgttacgctggaagaccagccggacctgcaggacattgacacgaactaccaccgcaccggcggcggattctggggaggatttatacaggaagaactggccggcactattgccctgataagcatcgggcaccgcgcaggggccatccggaaaatgtttgtaaaaaaggagttccgcgggaaggaatatggcattgcacagcaactgctggaggaactggttgcctatagtaagtccgtgcagataacggatctgtacctgggcacggtcgacaaactcgctgcggcccgccgcttctatgaacgcaatcactttaaagaaataaaaaaaacggatttaccatcgtattttcccctgatgaatgcagacaatgtattttatcacttacacattaatgacggagcagcatgacaaatgtaattgatgaatcagggatactggctatttctaccaggttacagcgactcagtgatcagttgcggaaagacgggctacagatttataaggccaacgggatcgactttgagcccaagtggttccccgttatctatacgctgcacctgaaaccggtgctcagcgtggtagaaatagccgtggaaatcgggtactcccacccttctactatcagcctgttaaaggaactggaaaagcaaaagctgatccgctcaaaaaaagacaaaacagatgaacggaagcggcttatcctgcttacggaaaaaggaaaagcgcttattactgatatgcaacccgtatggaataagatggtggtggcccttactgcgctgacagatacaaaaaataacctgatgaaggccattgaggaggtagagcaacaaatgaaatcgtttagtttttttgacagggtacagcaactgtaaagcttacgccagtaagccgttcaccagggctttccactgcaactttgatataccaatggcgccggtggcgcctaccactgcattacggagcttatcgcccaggtcattggtttgtgtattcggcacctcattacgtccgtaaacagtggcagttatttccgcaccgttacgtaccaacacaaaggaactgctggcttccttgcgcagaaaatgcgcaatgcccgcacttttctggatagggtgctccgacggacgggccctgataaaaaacacttcctggtgctcattaagcaccacatgctccttctgctcaatctttacccagtcgaaccccttccctgcattggtgcctggtccgggaatatcaatccgtatatacatccctgtttccgcactgccctccgccggtttcccggccagatccgtcaactggaaccccgacgacatactgccgctcagtgtagcccaatgatttacatccagcagccgcgcaaccgccgttttaaagaactcctgcgcggccgcttcatgaaccagtgtttttacctcagcagttgtggtagcctcgcccgtatactgcgccggaataaatggcgccgcaatgttatctgccataaccttaaaatttactgtaaaataataatgtaagtattcgggtaaaaaacttgtgccaattttatattacactacctttgaggtgtaaaagtacggacaatgcatttcgggccttcaaaacgatgctacagagaagcgcctcttttgaccatatttactcttcattaagagcacgaatcccacaactgtcaacaccttagtaattgtaaacaccgccattgccgtagagcgatctatacgcatggggaacaatttgttgatatttaaagatacggaatatgaatagtatatactcgcttatagtgagctgttttctctccatggcctgcagcaatgcaaagcccaaccaaacaaacgggaaaatcaccggccgctggcaacccgtaaaatcggtgatgagctgcgtagaagacggcaaaaaaacttttgataaaacagattccagtttcagtcctaacgacgtaatggtttttaaagataacggcatgctggaagacggcggccagcgatacgaggcctatacgcttgaccgtcgcaccaaagaactcacgctccaggaaggcggcggctatggcatcacctttaaaatccggaccatgaaccccgaggaactggtcatcttccgggaagatgaagaaatctttaaaaataaaaaacggcagatgaaacttgaaatctacttccgccgcatatagtcatttcagcaccggcaatataatgccggaaggatgcgcctcatcatgataaatacggatggtttcctttataaaatccttttctgttgcttcataaatattgatgaactgctgcggattacggtcggctaaaggaaaccagctgctttgcacctggatcatcagccggtggcctttctgaaaagtatgcgctacatccggcagctggaacttcacctgcgttactttgcccggaataaaaggcacgggcttctcaaaactctcccggaaacggccgcggaatatatccccccgtaccagcatctggtaaccacccagcggataaggcccgccggcatcacgggttttatttggcggcggcgtatccgcatagcggaaatcatccgggaacacatctatcacttttaccacaaaatccgcatcactaccggttatgcttacacgaagatcaacggttacaggacctccaatagtcaggttgtccgtaagcgtatcggtttcaaaagtcagcacgtccgcacggcgcgacgcaaaacgctggtcatcggtcatataatcccttgtacggatgtaatgcacgtcctgcgtatagggtaccggatgcgccggatcactcacatactcgctaaagccggtaccacctttatcccacgacagcccaccactctgccgtaaaaaaatctccttttccgttgccaccggcggccatttgctgaactgatgccatttgttttccccgctgaaaaagatattcgcttctgcgagatctgacagatttccttttcctttgagataataattaaagaaaggcacttctatctgctcctggtaccaggttgccgtattacttccaaactgaacatgccccaggcgcgtaccatcattgccggcccactgcccatgataccagggtcccatcaccagcttattgaaatgggtggccgggttttgttgctctatcgccttatataaattccaggcgccataacaatcttctgcatcaaataatccgcctaccaccagcactgccggctttatctgcgctacataattccgcgggtcgcgttccttccaccacccgtcgtattgcgggtgcgcgatgagttctttccagaaagcaagactatcgccggttagccgggtaaaattcctgatggtccctatcttcagaaaagtgctgtagttatcagcgcagggcagcttcaacgcctgcacaggcgctgtagatacgggcgacggatgcggatagccaaagcctttggtataaaaaccaaagcaatccatcaggaaaaaagcgccgttgtgatgaaaatcatcgccgtggaaccagtcggtcaccggcgcctgcggactcaccgccttcaatgccgggtgcccgctcaatgccgccatagtagtataaaagccgggatacgaaatacccagggcgcctaccttgccattgttgcccggtacattttccagcagccagtcgatggtatcgtatgtatcgctggcttcatcaatttcgcgccccttcttccccgggataaaagggcggatatctttaaactgtccttcactcatccagcggccgcgtacatcctggatcacgatgatatacttttcttccgcatagcttttccagtaagtattccagagattaggcgtaaacgccactccataaggcgcggcagaataaggtgtacgcgtgatcaaaacaggatgcttttcactgctgtcttttggaatataaatagcggtgaaaagatgtacgccatcgcgcatgcggatctgccgctcttctttataataatgttcctttacccatacggagtctccggcatgctgagccccggccgggagcacggcaaatgctcccagcaacataaaaacaaatcgcttcatcctgctctttttaattcaaaccatctaccgtcaaggattctgagggaaattggctggatcgttatgtatatctatttcgctttgtggtataggaaataatagcctggctggcgtaagcgccggcgtagtaagattatactcgtttttcaggtgtgcctgcataatggccagtccttttgaataacggaccaggtcaaaccagcggttattctcaaaggccagttctacccttctctcagcaaaaaccgcatcccggaaactggcctggttgggcaggtctgcgggtgttttatcgcccagtccggcgcggcgccttacctggttaagaaagccaaaagcgctgttggcgccggtagcagcgctatacccctgttcgttcaatgcctctgcctggagcaacaggatatcggcatatcgcaataccgggaaactgctgccgccatcaccggtagcaccgggagcatctaaatatttctttacataattaccgggttgcgtagtagtggcattcttatatgaaacggtatccagtgaggcgatcagccttttgtcgccggcttcataagccgacacaatatcatgtgtggggcggttgttgttagatcccccataggcgacaccgttataatagaaagaaaacggcaccatgtcggtgaagtagtagttgccttcagagggattcaatccttttttaaaacggatggtaaacaacacttccgcgttgataccggcagccgggttatacaaggctgcgtaatccggcaacagcgtatatccgttcacgtttttaagcacggtggtggcatcattccatttcttctccgtaacatatactttccccagcaaaccattggcactaccggcggttactctcccatagtcgttcacgttagtatacacggcaggaagcagggtggcggcggattgcaggtctttctcaatttgcgcatacacttccgcaacgtcattccgcttatcattcagcgactcggtagtggtttccacccttgttacgagcggtactttgccatacaaacgcaccaggtcgaagtacacaaatgcccgcaggaaaagggcttcgcccctgaattgttttttggccgaatccgggatagcggcagcatctatctggtccagtactgcgttagcacgggatatcgtgagataggcgcctgcgtatacatcggtcagaaatggattggtagtggtttcggtgaacaggtcgatctgtgaagccacgccgcctaatgcgccgcggtcaaggatatcggtgttatcgcttcttacttccatcaggtagtaggccgacttaccatagctgcgcgtgttctgcaatccatcatagatagcgtttacaccctgctggaaatcgccggtggttttaaagaaggtagccgtggtttgattggataccggcggcaggttgatgaaatttttactgcaggaagtgatgaccgttaccagcgacaagcctgctattgcttttataatatttaactgcataagttcctgtttttaaaatgaaagattaatacctgcggtgaatgttctgggcaacggataggtaccgtagtcctccccttgcgacaaaggcgcatcgggccgtgcattcacttcggggttataaccggtgtagtccgtccaggtataaatgttttgccccgacaggtacacccgcaggccctggatcttattattaaacagtcgctggttgaacgtataaccaatcgttaaattacgtaaacgcacatacgaaccatcttccacgaagaaggaactcggctgcgtgctgttgccggtggtaaccctgttgggccgcatggaattgccatcaccgggatctgtgggtgattcccagtaaccggtttcttcgatcatctggttggcatttccttcactgttatacaggaaacgacgttgcaggttcatcactttattaccctgtgaagcctgtaatgatacggtgagatcaaaacctttatagcggaattcgttggtgagtccccatataaatttcggaaagtagctaccaatatctgttctgtcggacgcatcaattttcttatcgtctgttacgtcaacaaacctgcgatcgccgggtttggtgcttgcataatgcggataagcgtctatttccgcctggtttttgaatacgccgccatttacataaccataaaaactgccaatgggcgcacccactttggtgatgtacaactgtgagatggtaccgttaccaccgtcggagatgatgggtgcattattagcgccgagttgcagtacttcatttttatttgccgcaatattaaagctggtgttccaggtaaaagcaccggtgaagttgcgggtagtgagactgaattccacaccggagttgcgcaccttaccaatgttcttcaacgctttaccaaatccggaactcagtggtaccggtacttccagcagcaggttggaagttgtggcgcgatagtaatcggcgctcaggtaaattctgttggaaagcaaaccgatatccaggccggcgttgagctgcaccgttttttcccaggtgaggtcggggttggctggttgcgccagtcccacgccatttaccgcggtgccgcttccgttgcctaatacataaccgttggaagccagcagatcgtatgctgcgtagttggcaatctggaagttaccggaagtaccatagcttaccctggccttcagttcggagatggcttttattttaaagaaagattcgttgctgatgagccaaccgcctgatactgcggggaagtagccccacttgttgttggcgccgaaacgggaagatccgtcgctgcggatgctggccgacacaaagtatttatcgtcgtagttatagttaacccttcccaggtaggaaagcaacgaccactgcgattccgtggaggtaccgctggtgatggtggcggcatttaacgtttgtacggcgtcgttaggaaagccggtaccataggtttcgttggctttggtggtattcttctgggaagtatatcctgccagcacatcaaaccggtgtttgccgttgatattgaactggtagttcaatgtattttcccagagccagtttacagataacgccgtttgtgccgatcctttggggatggtaggcgccgcctgttgaataggccggtagcttcccagtacggaaggccggaaataattcctgctaaagtgattgatatctgttccgaagaaggttttaaacttcagtcctttgatgatttcatattctccccaggcgctgcccaggttacgcacgtgatccagtttatctttgatctttgttgccagcgctaccgggttttcaccaccggagtagccataagcccacacgttctgccggttggtggccagtgatccatcgggattatacacggggaataccggcgaggctttgagcgcgttgctgaggataccgtcaaaggtccaggggccttcgctgttgatgaggtcataatgatcaaaggtagggttaacggtaacgcctatctttaaacgggaagtaagttccgcagtgagattggctctcagtccataccgtttatagccggagcccaggatgatcccctgctgatcgaggtagttgccggaaatgtaatactggaatttatcgttgccgccggaggccgacagggtatggttttgaatgggcgctgttctgaacagggcatcctgccagtcggtgttggtgaggccggggttacctgcgaggtaaggcagtatttccggtgcgatctggtaattggaaccgccccttgtggcgttatcatccgtgatgctgccggaaggtttaaaatccaggtaagcgttgttcttggcatcgaagctgaacctggaccactgataggcatccatcagctttatttttttactcacctgttgaaaaccggcgtacatgctgtatccaaaggaaggaggaccatttgtttttccttttttggtggtgatgagcactacgccgttggaagcgcgggagccgtaaatggcggcggaggaggcatctttgagaatgtctatagacgcaatatcatcgctgtttaaagtgctgagcggatcaggggatttttgaaaagatgcctgcccggtgatgtttaccatgtccgtagctccctgtaagtttttcaggtcgttcgacaatggaataccatcgatcacatacagcgggtcgatgcctgcggagatggagttcagtccgcggatacgtacgctgatgctgcctcccggcgcgccggtattctgtaatacctgtacccctgctactttaccggcaatggcctgttcaaagctggttaccggctggtccttcagatcggcagcccgcacagaggctacggcgcccgtgatttccctccggcgttgcacgccgtatcctactactaccacctggttaagcgaggaactggattctttcaggacaactgccaccggctggttctcccgcaaagtaatgctgcccagctgcgcaggctcataaccgatagaggtaaaccggaagctgtaaggggcgccaaccaccaggtcaggaaaacgaaaggtaccgccggcattggtttgcgtggataccgtagcacctgaggcttcatttttggcggtgacagatacgcccggcagcgcttcgtgcttttcattttgcacggtaccggtaacgcctgtacgcttttcctgtgcagccaggtataagggagttaataacgtgagcagcagaagtgtgcttctccatttttcttttaaagaacgaaagtaaaaagagtccataggtgatttttgaggccctgtgcaggttgttgccatgcctgcagccatacaggcaccgtttcagatacctgttgatttaccagggccggtttataaaacagcggaccattcattggccggtgatgcgatattagattttcagtttacagcgttaaaagtaacaacaagtttttagtctaccaaatcaatagactaatatccctgcagttattttgcggtagataaatttatcgtgttgcggattgcccttatcaatttaactcatttaacccggggaaaagggaaaacattgcctgtccggaaatgaacacttctcccgtaaaaacggacaacgtaatggtagttgttattacattacgtgttgataaccaataaccagaagattggcattttcttagcgcggaaatagcctcaacattcttctatgttcggcaaccaatttaaaatcgcgtggcggaatttccgcaagcatctcacacatggcctgttaaacctcaccggtctcacgctggggcttaccggttgtttctttattacgttgtatgtaactgatgaatacagctacgaccgctggataccggggcacgaacaggtgtaccgcgccggcatggaagtaaaaacccaaaccaatgatgtgattgcctttgcccaaacatcaggtttcctgcgacaggcactgctggtatatccgcaggtaacaaccgccacaaggatctttgaatacggcagcaatacagcggtgagcagcaacagcggtgcgcagaaaaaattcaatgagaaaggcatctactttgccgacagtaccctgctggaagtgctcccctatcctttgctggcaggtgatgcccgcaccgcgatgaacaatgcggatggtattatgctcacggaggaaaaagcggaaaaatatttcgggaaagaaaataatgtcagtacctatctcaataaaatattaaccatcaacgaaaagaactaccgggtaacgggtgtgctaaaaaatgtgcccaccaatacttatttccggccggattttgttatttccacggtaagtgtccgcaacgaacaatggttccggcgtaacatggaaaactggcacggcaccatgacgcataccttctttaaattaagacccggcgtgcaatgggaagcctttgaaaagcagatcaggaacatcgcctaccagtatgtgggcgatgaaataaaggctaacaaccaggtatatacgcatttcatccagccgcttactactattcacctgcattcaaacctccggtatgagctcagtaaaaacagcgatgtattatatgtgcgggtattgtctttcgtagcgttattcatcctgctgatcgccggcatcaatttcattaacctggctactgccaccgccagcagcagggctaaggaagtgggcgtaagaaaggtgattggcgccaaccgctcccagctgatgctgcagtttatgattgaagcgctgatgatgagcgtaatggcatttgtgcttacggctgttttaatagtcgtgctgctgccttctttcaatcatattgcagataaaacttttacggtgtcacagttgttccggccatcgctcattggcgcgggtcttggcatcagtgtgggcatcggcatactggccggcatctatccggctattatactttcaggatttaaccccatgcgtattatacaacggtatggtgcgcaaaagaaaacgcattcgctgcgcaatgtgctggtggtaacccagtttgctatttccatcctgctcattgtggccaccatcgtggtgcaccggcagctgcaatttatgaagagcttcgatctgggcattgaccagtcgcaggtactggtgattcccgttaccgggaaagatgccactgccaatattaaaacgctcctcgaaaaattccggggacaggcagacgtgatttcagtaagcgcctccggtaatgtgcccggccaggagtttggcaataaccttttccggctgaaaggcgaccagacaaagcaaaccgacaccaggctgctgtcggccgacaatgaatttttccgtacatataatatccggttgctggcaggcaggttagttaacatgacgccggacaccagccagaaaagcggcgatatcatgatcaatgaagcggccctccccttctttggctggaagaaacccgaagatgcactggggcatgaatttgattacggatggggtactgtatgcggcgtatataaagattttcattttacttcgcttcaacgcggggtaacgccgctggccattttttatgatccttactggctgaattatatcagtgtgaagatgaatacccgtaatgcggctgctactgtagggagactggaaaagacgtggcagtcggtggttccttcgctttctttcaattactttttccaggatgaagcatttaaccggcaatacctggcggaacaacgactgggatcactgtttatggtctttgctttgtttgctattgccattgcatgtcttgggctatttggccttgcttctttcacggctgcgcagcggaccaaagaaattggtatccggaaagtgttgggggccagcgtaacgggcattgtaaaactgttgtcgaaagatttcctggcattggtggtaatggccgccgttattgcatttccggtggcgtggtgggccatgagcagctggttacagcacttcgcttatcgcgtgccgctgaatgcgtgggtatttatcgtcgccggcggaggcgccttgctgattgccttgatcacggttagtttccaggcggtaaaagcagcgctggccaatccagtgaacagcctgcaggcagaataattgcggcaaaggcctgtactgtctaagtacgggcctttgctgtctattttgtataaaacacgatatcgtctccatccggttcactgtctgccagctgttcttcccagcctgcgggcaatttaaagatggtatgtaagccgcccagcagttccagccagccgctcatttcatcggacacttccagggtttcgccctccattgttttaaacaccaggaaggctgcttctcccgggtacgcatatactttgtatccggcaatataggttacatcatcccagaagatagtgttatcaatatcttcatcatatttcacataaagtgtccgttcatcaaattgtatatccatagtggtaagattatttagtttgcagtaatggtaaaacttactttaaacaaccggctggcgccggcatcattatcggataccaggtgaagcgtgaggatgttatcctgtatgctttccaggcaaataccttctatcttctctcctttgaaagcgggatctgctgctgttaaattgagcatgccatccggcgtaagggtagtttgtgataatttccgggagatattactgatccagccaatatagctgtcgccgatggcgccatcgtcgtaagcattggcagtggcttcggaagaaaaggtacacagtaacaggtccttttccgccacgtaacaaagttccgatatgccggtaaatacaggcgttggcgttagtaacgtaaacggtactacgttaaccgccggtgatgcctgttcccagaagccggggaccgttagcaccagctggttctgcggccaggtgtcgttaccgcggttactcagcagcaacatattgtttaccacggcggccccttctatattcagttcattgatcccgctgttgagcagttgcgtggtaaaatccggcggatagggaataaactgcatagcagcggagtcgtcatccggcagcggcagcagcatcagctgacggcgcttttccgttgccagggagccggaggccatgaggtaggttttaccatgcaggttaatcagtgcggaagcttcatagtcggccttttccgcttttgcaatgcgcttgccgctgatgccgggaatgggaatacttttaacgacctggtactccttatccagcacctggatacaggtggcatcatctcctatgagatacaacctgccgtcatgaaattccactgcggaggcagaaggaaaatcgggcagcagcaatgtgcagatgagtgtgatgacccctttcatgctatatgtgattactttaaactgctcactactttcttaatagcctgtgcccagaaggttcccagcacttccgcgccttttgcattgggatgcagctggaaaacgcctgcttttccctgctcctggataaacagttccgggtgcttcttaaaatagttaaacccgtcgcgataaccggtgaatacctggtgtggatggctggtgcggtagctggcaacaatagcgtccagcaccgggaaataagactgcaaacgggcctgtccttctgcgaggtaacgggaactgttttgtgtgttggcactataccaggtgggatgatgcaaaatgatgatacagccgggatagttggtgaacagctggtccagtatggcttttacatttaaccggtactgctccggcgacaccggtgacccgttggggccttctatggcgctgtcgttggtacctagcaccatagagaacaggaggatcgcgtgctgatcgtttttaaatgcatctgccgcggctaccacgttattgaataaacgaccggtagctggtaggaagtcgaccgtagtagaaccgcttacgccctggttgctgtattggatctcccggtccggcatcgcatgtttcagccattcccaggcctttaccgggggcgcttcctgcaacgggtgttgcaagccgccgccttgtgtaatgctgttgccgataaacacgatatccagctttttcttttgcgctgccgcgccggcagcggtgagtaccaggaagcaaagggcgacagataatattctcatcatgatataaaaactttcaaacttgtaaaataacaccttcacctgagaataaaacatttttcctgaaacacttttcccggaaataaatttttgcgtaaccaaatggttacttatatttgtaaccgaaaggttacataacttaaaaacaattaccgtgagaagagatgtatttcaggcaatagcagatcctacccggcggcagatcatcgggttactggccaacagttccctgaacctcaacgccattgctgacaacttcgatatcagcaggccggcgatttccaaacatatccggatactaacggaatgcgggctggtcaccatccggcaggaaggccgcgagcgcttttgcagcgcagatctcaggcagttaaaaaccgtggccgactggacagcccagtaccatgaattctggacacagaaactggatgcattggaaaactacctggccaaatcacctaagccccgcaggaaaaaacaatagtcatgtcaatcgttcatcaataaaaaaattcaccatgagtaacaaaccactggtattcgaacgtaccctggacgcccccgttaatgcagtatgggaagctattacagacaaagacaaaatgaagcaatggtattttgatctcgcggcttttaagccggaaaagggatttgagttcagcttcacagtagaaaaagataacaaacaatatgttcatctttgtaaaatcacagacgtgataccgggtaaaaaactcagttacacctggaagtacaaaggcgaacccggcgaatcggaagtaacgtgggagctgtttccccaaggtgggaaaaccaaactggtgctaacgcataccggcattcacagcttcgcagcagcgaatgatcctgcctttgccgccagcaactttaatgaaggctggacttatattcttggtacctctttacctgcattcctggaaaaagaacaggtaacaaattaagtacaacgcctgatggaacgatgtttcatcaggcgtttcctttattctgccacggtcacgagcaatggggattcaaacatgcttaccggcgaaataattttctccgacaacgggatattgtttccgtagatctctttcatttgctgctttaccgccgcactgcccaggtcaaaatctttcagctgctgcagcttgcctacttcgaggccggttccttctttataaattttccagaccagttcggaacaatagatccgttcatcggaccagccaaaatagaagtcgtagtccttgccattgtattgctcccctgctaccttcattttagccaccacttccggtgtgagcacggtaccagcatctttcagccgttttattacaaaatgccggccctttcccctgttaatccattgcatcagcggagtatatcttactggttgtaaggcctcatatacaaaccactgatcatctctcttaaaaattattccgcaatgactatatttggaatgtgttgcctgttgaatagctgtgctcagatctgactgggatacctggaaaatgatatccccttcccggacagccggaaatgtagctgttaattttttggagagatgtttgcccgtgaaaatataagacgccgccagtaaggtacccgttacaatggtgagcgccagtactgtaagtataatttttttgagacctggcataaacccgaatttaagtaaaaatagatcctattattatataacccatagaaaatgaacgacatacttatcgtgccggctattacagctgaagtggaactgttacagcagatagcccgggaaaccttccaggagagctttgcagccgacaatacaccggaaaacatgaaacaatacctgcaggagaatttcagtattgccaaattatctgcagagctgagtgagccggattcggaattttatttcgccatgctcaaaaatcagccgatcgggtatatgaaagtgaacttcagatctgcacaatctgagttgtacaacagccgggcggtagaactggaacgcatatacgttttaaagtcgcaccaggggaaaaaagtgggtcagcagctgttcaaccaggctatgacccttgccatggaagcccgcgctcctttcctgtggctgggtgtatgggagcacaataccaaagccattgagttttaccgtaaaaacggctttaccgattttaccacgcatccgtttcagctggggactgagatgcaaacggatcttattatgcggttaaacctgccgctgcataagctgcaataaatttatttcagaaggatatggcaaggcgcgtcactggtaaatccataacagcaccggccgggaagaggtatctatataaggttgcagcgaagtgaaataagcagggttcaatgtaggacagccatcgctgcggcaaataccctgatcctgtgcagctgcgggcacacaggcgtggctgtgcaatactacaaaccggtcgaacgcacgactgttgctgctatccagcccatataatttatacgctgtgccaaaccggccactatacttgccgcctatacgatatttcccaagtgaagaacagcggctgccgggtacattggaaaacaccaccttttccgctctgaaatccggtccctggccatgcgccaccaggccgctgctttttattttatgatgcagcagatcgtaacagataaatcttttgccaccggaaaacacgctaaaatctaccaggaaagcgtaacgggtattataaccatgtttcacggcatactgttgcaacgcttttgccttttcgtgcagccgtgcttcatcaggcgccattacaagctcctgcggagcaggcagcaatgatggtattgaatgtgtagtggtatttttttctttacaggcggcaaataaaagtgctgccaacagcaaaacgctccatgctttgaaccgtatcatgcttgtcagatgcagcaccacacattttccataagcatccgtaaaaattgcgataatccgcttttatctcccttaattattaaatcaaaaaaaatccagcagtaaaaatccggctaatcagtataatcagcgtaatcctgagccaagacaaaatccgcgttattcccagatatctttgacatgaatgaggatcgagtaacggccggtgggaggataatgaccgatgtgcaactgcgtttcatcaaagggctgcggcagtttatctgcatattgcccgtataattcctgcactactgcaatggcttccgccttattttccactacccatgatttggcggtcctgttattatcaaactgctggttaaaggctttccgggcagattcagtttgttcaaacggcactactttcagcgtccacacctctcctatcttctccgattgtgcgggtgtatccaggttgatcttaaacctttccaatcccgcaggatccagggcacgcatgatatccatcgcaactgacataattataattttttctgaccgcaatattacaacttccgggtgttattcagcgccttttacgttcatacggatcgtataaatgcctttaccggcggtgatgaacaggatgttgttatctttcccgccaaaacaggcgttggcggtccattctgccggcacgtggatctgcccgatctgttgaccgtttttgttaacgacggtaacgccgtttccacagagataaaggttgccttgttcatcgagtgcaatgccatccgttgttttctccgccaggaggtattgaccggttaaacggccatctgcctgtacgttatagcggtaaactttgccgccgccgatatctgctatgtataccagctttccatcgggcgtaccgataataccattaggcttcttaatatctgccgcggctaccaccgcttcttttgcgccgggcgccaggtagtaaacattttcttctttcatatcgggtttcctgcgcaaccagtaatcacgctgataataaggatccgtgaaatacataccaccgccaggggccacccaaacatcattgggaccattgaacttatgaccgccgaaattatttaccagcacttttatttttccactgggagagatggaccacaactcgtattgctcatctgcacacgctaccaggttgcctttcccatcaaaatacatcccgttggcccggcctgcttccttcaggaaaacagacagcttccctttggtatcatatttccagatcttattgttgggctgatctgtaaaatagatattcccttttttatcggccgcagggccttctgtaaagtcgaattgttttgaaaccagcttcagccgggcatctttagccactgtgggcggaagggtatcttttgtaaccgcacctgcaccgaggtagcaacaggtagccagtagtaacgtggaataaaattttaaccgcatagtgctccgtcaatttttacaattgtaatcaatcctgcggagaattttttcaaaaaatgatggagagaggggctggtggaggagatcatatttatttacagagccggctatgtaaatagcccgcctataggtaaacatgatattgattttttggggtaaccaacgctggatgacattttacccgattttagaatggcgttctattccggtatggggatgctactcctatggagaaaggtcgtacgttgatggagcgaaattatcgtgcttaatggcagggacatagtacaaaagcgacatcttttgctttattccattattttatggagccgtatggtgttggtgagttcctgttcatgcataaaggaaggggttatgcccgcaaattttttgaagtcgcggataaagtgcatctggtcataataaccacttttgtaagcaatttcggtccaggttttctcgggaaacagttctttcagttgataggctttacagaagcggataagccgggcatattgcttgggcggcatgcccagccgttcggtacatttccgttcaaactgccgcaggctgaggcaggcaagcgacgccagggcttctatcgttccgttaccgccggtgctcaccagggcagccattgctttgtccaacggcaggattggctttacctgggatatttttttaagcagataaaactcaacgatacttatcatgtgcccccaatcgtcggcttctttcaaccgttcggtgatttcatcaatttcattacccatcaacaggcgggtgtcaaaatcctggtcatatatttcagacatgggaatcctcagcaggcggtgcaggccaccgggttgaaagcctatgcacagcgccaggtggcggcgtcccatatccagggttaccggctgctcctgcggcccgatggttacacaaatggttttggttacatagtcgctgtgaccggccttcaatactttgataggatcttccaggtaaaaaataataaaccgctgataggcgggcacaaacctgtaaatgtttgacagcgccttgttttggctaaaatctatttcgtagatgccaaaataactcacgagatccctcagggccggatgtggtttgtaactttttgatttcatggatgtgtgcggctataggtgctcagtactgtgatccgctgaaacaaatatatacaaatattaaaaaagacaaccaatgctacctataagcgttatcttatacgggttaattttattttatatttaaagatgaaaattgcgatgaccggagcttccggctatataggcagtgtgctggtgccgctgcttttatccgaagggcataccctgcggttgcttacccggaaaccgttgccggaaaccaccccggagggcataactttcgtacagggggagctgttagccgaagcggctatccgccagctcgtagcaggtgcggatgctgtgatacacctggcggcagtcatttcggtagatgaccggcccgataaaaacctttttcacatcaatacggagggcacgcggctgctggccgccgccgcacaacaagccggcgttaaaagattcattcacctcagttccgttactgcttacaaccaggcgccctatgatgaaccgatgaatgaaagccgcagcgtggtaaataccacgcggcacggttacgactattccaaagcggtatcgcaggccattgtgctggaatataacggcagcggcatggaagtggtggtgctggcgccaacagccgtaatggggccgttcgaccggcaaccatcgctgataggtaaagccatcattaatatgtataaaggaaaaataccggctctttttcccggtggtgttgatttcgttgatgtaagggatgtggccggggccattgcaagcgcattaacgcggggaaccgccggcgctgtataccttctgagcggcgaatgggtatcacttgtgagcctgaacagggaagttggccggataaaagcacggccggtaacgctgcgggtagtacctttatggcttgtattcagcatgctgccatttgtgagaatgctggcagtgatcagcggcggaccgccgttttatacgcggcagtcggtgtacaacctgatttacagcagcaaaaaaattgatcattcaaaagccgccgccgaactcaatttcaggccgcggccctttacggaaacccttcgggataccattgattggttcaaacaaacaggcgctatcaaatgattgactatttaccatcaccaggttatgttgtttttgtttgttgctgggcgcttaccggtattggcgcgggcatttacctgttacgcagggaggcgccttacggtcgctacagcagcgataaatgggggcctatgatctcgaacaaactggcctggctgctgatggaagccaccgtattggttaccttccttatatggatcccgctccgtacttttccatggcgttcccccgccggcgttatggtgttgcttttcctgctgcattatgtacaccgcagtttcgtatatccgtttatgatacgtaccaaaggcaaaaaaatgccggtggtgattatgttgtcggccatgctatttaataccgtgaatggttccctgctgggcatctggtttaccgcttttgaccactatcccgatcatacattttttacaccgtcgtttatcaccggcctgttgttgttcctggcgggtatgttcatcaactggtggtcggattaccagctgatacacctgaggaaaagaaatgaaaccggttataagataccacaggcggggcttttcaaatacatctcctctcctaacctggcgggggaaattattgaatggggaggctttgcactgcttacctggagcctgccggcgctggccttttttatctggacctgcgccaacctggtgccccgtgcaatggccaaccaccgctggtatcagcaacaattcccggaatacccggccaaccggaaagcattacttccttttatctggtaacaacccgcttatggcaaagaagtacagtcagtttaaagcagcattggtgatggcaaaagccagtcttattgctacgctccgaagccctacttccgttgtatttgccctcctgttccccgttattttcgttacggtttttggcgccatggtagacaacaccgccgtaaaagtaaaggtccggctatcaccgcacagcgacagcgccaacccgatgtatgcggccattaaagccatccctatcttcgacctttcttatggcagcgattctgctgcgatgctgtcggatctgaaaaaaggaaggatcgccgccgtgctttatcttcatgcgcccaccgtggtaaacggcctgccgcaattccggacggatctgctgggaagcagcgctgtagcggataaaatgccgctgatccaggcagcgctgcaggaagcggccagcaaagtaaaccaacgcatcctgccggatcagccggcgccggcatccatacaggtggtgaatatacccggacgggtataccgccagatagattttattttaccggggcaactgggcttttctttactcatggcaggcgtattcagctctgcgttcctcctgtttaacctccggcatacgctggtactgaaacgcatatacgtaacgccggtgagccgcgcggccatcttgttgggtgaaatgctcagccgcttattattccaggtcatctgctttattatcattactgcgctgggatactttgcattccagtttacgttggtaaacgggctcctcacctttatggaaatgctgctgctctctgtttttggattggtgatttttatgggcatcggttttattatcagcggcattatccgcaatgaaagctccattgcgccggtggctaatacgcttaccgtgccacagatattactttgcggattatttttcccgatagataattacccggtgtggttgcgcactttttgtgaattgctgccactaactttttttgtagacgggttacgcaaaattgcctttgaaggtttgcatatctggcagataccgctgcaactcgcgggcctgatcgtatggggtatacttattgccgggttatcgatccggtcgttcaaatgggaataacaaattggcgcaactgccccttttattgtcgtatccggccacctctttctttacagcagcaacttaactttatggtatcttattaaacacaaataaaaaataaaaacatggcagcagttaatccttacctgaatttcaacggcaattgtgaagaggcttttaatttttacaaagctgtttttggcaaagaattccagacattcacccgctttggagagatggcgcattgcgcggaaggcgaagaaaataaggtgatgcacgtggcgctcccactcggtaaagattctttcctgtttggcagcgacaggcccggcgcatatggcaaaggcaccctgggcgaccttttctttgtggctattgcggcagaaagtgaagcggaagcagacaaattgtttaaaggtttgtcggaaggcggccagcccaccatgccaatgaacaaggctccctggaatgcctattttggcatgttaaccgatcagtatggcgtgtcctggctgatcaattacgactatgcccagaaaggctgattcccgtttaaaagaaataaagcagccggttcactccactgaaccggctgttgcattgtgacaggtataggacagcatttcttttatttgttgacaattagtcccgtcagttgtttatccaattgctcgccacggaggttttttgcaataattttaccgtccggcgcaatcaggtaattggtaggtacaccccgaacaccatactggcgcgctaccgcgttatcccagtatttaagatcggatacatgcacaaagtcctgcaaaccgtctttttcaatggcgcccagccaggcagccttcttccccggctgatccagcgatacgctcagcaccacgaagtttttatcatggaacttcttataggcagccactacattaggattttctgcacggcagggtccacaccaggaagcccagaagtccagtaacacatatttacccttgaagtcggataacttcacgggcttgtcgttgatatcattctgggtgaagtccggcgcaggcgctccaatgcctaatgccttttcagtttccatcgattggtaaaactcctggccggcggggcttttcttcagcgcagccgtgagaccattgtacatcggcgttaactccttcaggttcatattattcatcaccgccagctctttcagcgctacaatgctgaaaaaggaattaggattttcgctgataaacctgcgctgtaaagctttcttttcagcaatggcagcatggaagcgggtattcagtttattggtgaaagcggtatcatttctttgcgcttcggtagccgctccaaaatccttgttgatacctgccatagcagtatcataggccgcaataaacaatttgtaacggtcgtgttctttatttaccggggaaccggtgatcaccgcatcgctgatattatcgctgccggcaatggtaaaagtggtattatccaggtaaagcaggcggcggtccatgtccggcccgtggttaccggtgcctttatgatccaccatcagcatcgccaggtagggcgatttcagcgtgcctttaaattcaaacatgccatttttgataacagccgagtcgaggaaggtttccccgttcacgcgccggtcgagataagctttggcgccgggttccacctgccccactttacctttcagtgtgtatgcctgctgtgcaaaggtcatggccggcaatgccagtgctcctattaacatccctattttcataaattaactttagatagttggtatatgaagacataaagcaggaaagcaccggaatcttagcgttattcctgttttttttattccacacagtggcgcctgcgcggctttaacagtagttaacattgtcataataaactaattagccttaccaccgtctaataccccgtagccagctaccggataattatcgccgttttttgaacaatacaattgaacggatagttactcatagtacctgattgctgtctgtattatttaaatgaactgtaaaatgctatgagtagatctaccattgcgctcctgctgttgctgttatgtgcctgtaaaaacaagaaacaagggaacacacaaaccgctgtaaagccttaccctgtgattgtactgcaacctaaaaacgccactatcaatgccgactatcccgctaccatacagggtatccagaatattgagatccggccaaagatagatggatatgtggatgccatctacatcgacgaaggcgctactgttaaaaagggacagctgttgttccgtatcagcgccccgcaatacgagcagaatgtaaacactgcccaggccaatatcaaaatagcggtggcagatgtaaatgccgcacagatgcagcttaacaaggtaaagcccctggtggaaaaggatatcatcagcgcctatgaactggaagctgcggcgtataacctgcagtccaagcaggcagcgctggcacaggcccaggcggcgtttaacaacgccaaaaccaatttaagctacaccactatttacagtccggcagacggcgtggtaggcatcctgccttataaaataggcagcctggtgagcagcaccaccgccaacccgctgaccaccgtttccaatattacccagatctacgcctatttttcgattaacgaaagacagggactggatttcttcctcgcctcaaaaggcgccaccatgcaggaaaagctggctaccctgccaccggtaacattggtgctggccaatggcattgtgctgccccgcaaagggcgcgtggaaactgccagcggtttaatcaacccctccaccggtgcgctcaatatgagggccaccttttccaatccggatgggttggtacgcagcggcagcagcgccattgtaaggatcccccagctgatagataccgcactgctggtaccgcaaaaggccaccttccagatccagggtaaactgttcgtgtatgtactggatgcagataacaaagtaaaatcagtagacataggctccaatgccagcgctgccggtcagtcgtttgtagtgcagcatggcgtgaaagcgggcgataaaatagtggtagacgggatcagtaacctccgggaagacctggtgatcaagccacgcctggtaaacgcagacagtgtttacaacagtctctgatccatttaaaacaatatcatgttaaaaagatttatagaacggccggtattatcaacagtagtgtctatcattattgtcacactgggcatactggggttggtgtcactgcctatctcccagtatcctgacattgccccgcccactatacaggtgcaaacgtcctacagcggcgccaatgcagacgtggtgctgaaaagtgtggtagtaccgctggaacaacagatcaatggcgtggagaacatggactatattacctctacagcaggtaatgacggttcagcgaatattaccgttagctttaaaattggcagcgaccccaatatggccgccgtgaatgtgcagaatgccgtggcccgtgccacaccactgctgccgcaggaagtaacccgctccggcgttactgtgcaaaagaaacagaccagtaacctgctcatcttttctgtttacagtaccaatccatctttcgatcaaaccttcctgcaaaattatactgatattaatatcaccccggtgatcaaacgtatccccggtgtgggcgatgcctccgcctccggtaacatggattactccatgcggatctggctcaatacgcaggcgatggcttcctacgggctcatacccgctgatatcactgccgcgctggctgaacagaatatacaggccgctcccggccagtttggggaaagcggcggacaatcgttccagtatgtgatcaggtatccgggcacgctcatagataccacccagtttggcaacattgtattgcgctccaacctgcgcagccgtttgctgcggatgagggatgtggcccgcattgagctgggcgccctcagctatttcaacagtacccgtaccaacggctatcccgctgtttccgtaagcgtagcacaggtggccggctccaatgcccgcgatgtgatccgcgaaaccttgaaggtaatggaagaagcttccaaaacatttcccaaaggtgtgaaatatgtggtgctgcaaaatgtggacgacttcctcaccgcctctatcgataaagtattgcatacgctggtggaagcatttatactggtgtttgtggtggtgtttattttcctgcaggacttccgctctacgctgataccggcgatatcggttccggtagccattataggaacttttttctttctcaagctgtttggattcaccattaacctgcttactttatttgcccttatcctggccataggtatagtggtggatgatgccatcgtaattgtagaggctgtgcatgcccgcctggataccggctataaatccgcccgcaaagcgagtattgatgcactggatgaaatatccggcgcaattgtgtccattacactggtcatgtcagccgtatttatcccggttagttttatcggcggatcttccggcattttctacaaacaattcgggctcacactggccattgccattgtgctttcagcgattaacgcacttacgctcagtcctgcgctctgtgctattttcctgaaacctcacgggaaggaacatacgaaaatgaacttcctgcagcgtttctatcatgcgttcaatgtggcttttgaacggttaacaaaacgttataccaataccttgcgctttttcagcaaacggaaatggataccggtgatggtgctgcttagcttctgtgcggggctggtaatccttgccaggatgacgcctacggcttttgtgccggaagaagatctgggtacgattaactgtaacatcagtttgccaccggatgcctcgctggagcgcaccgatattgtgacgcgcaaaatcgaaaagatcgcagccacgataccggaaatcaataacgtgctggcggttacaggacgcgggcaattgtccggtaccggcagtaactatgcaatggtggtgatgcggctcactccctgggatcagcgcaagcggaatatccagcaaattattaaggaactgaataagaaaacggcggacatgaccgaagcggagattaagttttttgcgcccggtaccatccagggttttggcgcatccaacgggtttgcttttcagttgcaggataaaaccggcggcgacattgcgcacttttataaagtaagcaaagacttcctctctgtattaacccaacggccggaaatacagtttgccaccacttctttcaatcctaatttcccgcaatatttaatgaacgtgaatgtgccgaaaataaaagatgcggggctgaatgtaacagatatcaccaacgccatgcagggatattttggcggtatttatgcttccaacttcaaccagtttggtcagcagtaccgcgtaatggtgcaggcttcgccggaattcaggctcacggaagaaagcctgaacgctgtgtttgtacgtaccggcgagggggtaatggtgccgatcacggagtttgtgagtctctcgcaaacctacggtccgcaagctattacacggtttaacctgttcaactccatcagtgttaatggaacacctaatgccgggttcagctccggccaatctattgccgctatcagggagtcggcagcggaaacgttgccaacgggctttgggtttgagttttcgggcctgagcagggaagagttggcagggagcagtcaaactattttcattttcctgctctgtctcattttcgtatacctgttgctcagtgcgcagtatgaaagttacctcttgccttttgcgatcctgctggccataccggtgggtattttcggggccttcctttttgcgcagctatttggtgtgagcaacaacatttatgtacagatcacgctgatcatgctgataggattgctcgcaaaaaatgcgatcctgattgtagaatatgcagcagaaaggcggcgcagcgggatgagtattgcggaagcggcggtgagcggcgcgcaggccaggctgcggcccatcctgatgacatccttcgcctttatccttggccttatcccgttgatgctggccaccggcgcgggcgccaatggaaaccggtctatcggaacaggcgctgtgggcgggatgctggtgggaactgtattcggtatatttattacgcctacgttgtttatcatcttccagactttacaggaaaaaataaaacgtgcaccggaggaagatgatgaggaagaagcgcagccgccggtaacagcaccggcatcttaaaaaaatcctgccgcaggcagatctcaaaacaggtcatatgaatggtcgtaacagtatatatatttttctttttgtagtcctggcaggattcgtaactgcctgtggcatcacgaagccataccaatcgcccggcattacagacaataacctgtaccgggatattcatacaacggataccaacagtctcgctaccgttcactggaaagaaattttcacggactcgctgttgcagcagcttattgacacgggtattcagcacaacctcgatctccaggtggcatggtcgcgcatgcggcaggcagaagccagttactcgcaaagcaggcaggcattgtatcctgccgttaatggtgatgtgagcgccggttatgcaggcgcctctaatcaacagcgtacaggcaggaccgttataccgcagcaatataatgccgggctcgcagccacctgggaagctgatatctggggtaagctgcggagcagcaggcgcgcgggtttagcggcattcctgcaggcatccgccaatgcaagggccgtgcaaaccgggttgattgccagtattgccaccaactactacaaccttaccgcactggatcagcaactgaaaataacgcaacaaaccgttgtgaactggcaggcgaccgtggaggtgatgaaggaactgaaaaaaggtgatgtggttaccggggcagccgtggtgcaaagtgaagccagcagatacgccgcagaagtaacgatccccgatttaaaacagtcgatccgcgaaacagagaaccagctgaacctcttgctgggccggcctcccggtcccatcagccgcagcggcatggacgaccagcaaccagtcatgctgctgaaaaccggtgtacctgcacagctgctggccaaccggccggatgtgcaggcagcggaatataacctgcgttactattatgaattgaccaatgtagcgcgtacttatttttacccggcgctcaccatctccgcttctggtgggtataccagttatttgtctctcaccggtcccggctcgtggatcagcaacctgacggcgggtttaacacaacctatttttaaccagggcataaataaaacccggctgaaggtggcgaaagagcagcagcaacaggcggcgctggaattccatacggccgtattaacggccgggcaggaagtatcgaatgcattatattcttaccagactgccatggaaaaaggaaactcccggcggctgcaattacagaacctgcaattgtctgttgactatacacaggagctggtgcgttatggatttgccaactacacggaagtattgaatgcacaacagagccttttagcagcgcaactcaacaggatcaacgatcacctgcagcagttacaggcagtggtattcttataccgcgcgctcggcggcggatggcaatagttcctgccggaatgccagcgcaggcagtgcggcagcactgttcaacacttcgtctaccagcccgaaatcacgggcttcttctgcggccatgaaatgatcattgcgaaaggcatgctccacctcttgcacggagcggccggattgcatggcgatgatctggaaaagtttttgctgcaacctgccctgttcattaaaagcaatacgcacatcttccgtatatcctttggcgccgccgcttgccggatgcatgtggatggtagcattgggcaaggcataccgttgaccggtagcgccggccgtaagaatgatggtgcccatgctgccggtgaaacccattgccatagtggataccggcgatttcagcattttcatggtatcataaatagccatgcctgcgtaaacaacgccacccggactattgatgtacatatttatgggccggtgattttcactgtcgaggtacagcaactgcgccactatcaggttagccacctggtcgtcgatggcagtgccgagaaaaataatcctttctttcagcaacaggctgtaaatatcaaacgcaccgcggctgtcgccgtcgattacggtaggaaccaggaatgccatattatttaaaaatagaggtgatagaattgttgaaggccgtatcctgcatgagacgcaggaagagctgatccagctcctgccgtttttcttcgcgtgcgagccagcgcacgagctgcattgttttccgctggtacttcaccttttcgcgtaatgccggcgccaccagcatcctggcctggaataccagccgggaggaaacaggcatttcccgcagcaggtattgttcaatttcccgtgcttcagctaactgtttccgcataatctgattgtttaatttgttcccttactttttccaggcatttgtatttctgtacgctggcagaatgttccgttttaaaattaaagcctgctgttatttcgggtatggaaagatggtcgtaataaaatgcgtgcagcagctgcaaacattttttcccggcggcttttacatattccagtaccggtttcgccacgggaggcggcgcataataatctgctggtacgccaatatcacccgctatgtcatcaagtggaatatgcggaccggattgtttcagtttccgcacagcgagaatcctggcgatccctgtaatgtatgcttccgcaggtaccccggcaggtagtttgttttgctgttgtttttcaagatagataataacagcatcctggaagatatctttggccatttccaggtggccgcccatccggtatatcatgcctgctacccgtggcagtgtattccggtatatttcttccagccattgatcttcatgagtacgcatatgagcctggttttatatactagtgtcagaaaccactgatatatcacctaaaatttaagaatttttttttacctttgctcaaccatgtgatcaatactctacatacaatagcaggctgatacctgtatacatgccgttctggcgtgtttcatttcccatttatatattttttaccgtcatacagtgatgctcctgcatacgctgatttattcaactaaattttactgccatgaaaatgcgtactgtcatttcccgacccgctaacccgacgcctgccgtcgccattgttcatttcaaaacgattttacatgcttatcagcgcacaacaactcagttaccagcttccatcggggcagtatttattccaggatgtcagtttcacgcttcataaaggctaccgggcagcgatagcgggtcctaacggcgcgggcaaatctactttgctgaagatcattgccggccaggaaaccgcgtcttccggtaccgtccgcactaccgcgccctgttattatgtaccgcagcatttcgggcactttaacacgcttaccgtggcgcaggccgccggcaccgcgcaaaaggtccaggcccttgaattaatcctgcagggcgacaccagtccgcacctttacgatatactcggggacgactgggacattgtcgcgcgcagtgaagctgcctttgaaaaatggggccttcgtgcattgcaaccggatcagcccttgtccaccctcagcggcggcgaaaaaacaaggctgttcctggccggcatcgatatctttgagccatccattgtgttgctggacgagcccaccaaccacctcgattacgacgcacgggaacagctatacgaatggatggccgctacctcgtgcacgttgctgatggtgagccacgaccggcagctgctacgcctctgcgaacccatctgggagctgcaatccaatggcataaagacttatggcggcaactacgatttctatgccgcacaaaaaacactggaagcggatgccttacaacagcgggtggctcaccaggagaaaacactgaaagaagccaaaaagcaacgccaggaggccatagagcgcaagcagcatgccgatgcacaggcacggaaacataccaaaagtgcagggttgcctaaaatattattgaatgcgaggaagaataatgcggaagtatctacctcaaaattaaaacaggtacatactgaaaaagtagaagaactgcgtgcaggctggcaggaactttctgccatgatacagctccagcgcatgatgaagggctattttgagcaatctacccttcatacagggaaagtgctggtgcaggcaaacgatataaacttcggatggcctgctgcacaaccggaacccgcggcgccggatcccccgccatcaaatgaaccggcaaaatcatcatctccggaaaatatgctctggaaaacaccgctcacctttacaatccgcagcggccagcggctggccattacagggcccaacggcagcggcaagtccaccttgctgcaactgatactgggcaggctgttgccgtcaacaggcgagctgtataccgccgatacgcgcagtttgctgctggaccaggactatacgctgatagaccggagtaaaacggtattgcagcaggcattgtcttacaacagcaacctgctggaagtatcgatggtaaaaacggtgctggtgaatttcctttttggccccgatacctgggataagtcgtgcgcagtgctgagtggcggtgaaatgctgcgactggccctctgcagcatgaccttacaggacaaagcgcctgacatgatcctgctcgatgaacccaccaacaacctggatctgcaaaacattaagatactgacgcagatcttcggggagtataaaggtacgttgctggtcatttcccatgatcccgactttattgcggaagtgggtgtggatgatgtactggcgttaaacacctagtgttatcttttcccggaaaggcttcgtgaaagcctttccgggatccttgttatagttcgggaatgccatccaggctgtacgcgctgaaggcaacgatgccggtaactttaacaggcaggaaactgcccgtagcggtgagatactgatacgtatcgcctgttctgcaaagcaacgggaagctgtacagcacttccgcggagccatagcggggtacttcttccagcgctatatcatcaaaaagctgtttgcttaccggttgtccggcttcattcaacacggtaaatttaccgcctgtttgcgccaggaatccccgtccgttcttttccacgagcaggcgatcgtatatgggcggcactattactttgccggtgctattggcataaccataaagcggatatcctccgttagccgtttccttttccagcagccgcgactttttttccgggacaatgggcactttaggtgcgggcatctttacgccgttatgattaaagaaaagttctttgtagctgccttccggggtgctttgggatgccaggaataaactgctgtctgccgatgatacgctgatgctgttatatactgcggggatcagcatcttcttcttcctgatatcatacacacctgtgccggtttctttctttaccgccaccagcccgggtaccaggtcatccagttttttatacgccacgggcaacacctgctcccctgctgcatcatacaagccatacatctcctggtaacttacttccagtaattctatgccgggggcagtaactgtggtcctgtcaatatcaaagaaggcaggttccactactttcctgttaaccgggttataaaaaccatagagtgctttttgcttcagcttaacgagaggggcggaaaaacgtttatccatgaaggttatttcggtataatcttttgccagtaacttcttaccggtggtatctgtcaggttatagttgccatccacccggataataaaatagtcaccggatcctgtaatatcaccttcgtatacaggagcaatcattactttcccatcttcccgcaggatgcctgttttaccattttttgtgacctgaagataggggcctctttctgtttcgccataagcatcggtgatatcgtcataaataaaatcggctatggtaacgccgtcttcgttaatcagtccgtacttcccgttcttttgcgctttcagcaaactgttacctgttatcgtcatatctgtatactccggtgcggtatattctttttttgttttcaggttgatggttacttcgtgcccctgctttttgaaacattgtacccagttgtcgctgcgcataaaagcgtgtgcatgttcgtattcaaaaggcatcaggacattattgttaaaatcgatgataccccatttaccattcttctgcgcaaacaggtaatctcctttcctgccgcatccgccgcagtagtcgaatgattcatacatggccggtatcagcaaccggttttctgcggtgctgtagattccccatttaccgccggttttcacatcaaagtgtgtatcgtccaatatgccagcgtcttcaaactgtagcggcagcaacagcttcccgtcggtatctgcataagtcattttaccttgctgacgtaataccaggtaagttttccatttcagttcgatggtatcatatgcaggcggcagcagccactttccattaccggcaataatgcctgttttgccggcgctgcttaccaggagcatggtttcctgtgcttcaggcagtgcttcttcatctgcagctgtggcggcagcggggtgatacagggcaacgatctggtcaaatgcttttttgccggtggaatctatataccagcttttgccggattcttccatacgggcaaacccattatgaaacgcggatccctgctgtgcggataagctatgagccgccagcaaaaaactacctgccagtaaaaaacgtatattcctgcctgttatacccttaatcatcatatccttttttcttcagtgatttgtaggggaatgctttcccttgcgcatcgagataaaaataccatttgccttcctgtaccagtattggaaagatatttttgtcatatccctggttgacatccatattatcatagatagcgggaatgatcattttgccggaggcatctgcgataccgtacttgccggcgcgcgttacctggaacaggcgctcatctttccggtagctgatatcatcaaattctaccggtaaaattattttacccaggctatctgttacaccatatttattattgcgtgacaccttgaaaaaaggcgcgtcatagatatcgtcgatttcctcatactccaccgggagcaatgttttaccttcttttgtgatcagtcctttgcggtctcctttttttaccacgagcaggttgttcattgcataaatatcgtcggctgtaaccgggtaaataatttctttcctgcggttgatgatgccgtataaggtatgttgcggggtgctgtcgattcctgccagcgccaggtcgttccagaaatctcccacaaagctgtagccttcaaaaaccacttcttttccgttaggatctaaaaagacattgttgcgggcgttgctccataatttcaataggccgttattgaatcttgcattgcttcccttttcgctttccggcatcagcagccgcgacacctggttttctttaaactcccagcgctggctggtatagagcgtattgcctgcgagatcggtgagcaggctggtagtggagccatcgtcgttgtattgtgtttctacaatcctgttggtgtccaccgcagtaaaaaatccataccgttttccgccacggagaatctttcccgttacatctgccagggaagtggtatcgcctttgcgcagcagcagtatccggctgttttgccactgcagccattcgtactgggcggggataatttctttcccggtcgtaatattaaccaatcctatcttctctccttttacaatgggcaggtaatcttttttgctttcccctgcgttatcatcaacatatgaaaatccgctgccgaagccatttaccaaaccatcatagactactggcagaattattttcccatccattccgaggacgcctgttttaccatttttctccgctgccaggtaaggagtgtcctgccaggagaacggtgttatgcggctgtatgtaaggggcagaaggttcttcccgtttgcatcaaacaggccggtgccagtggcatcgcttaccaggaaaactaccggcacgggcgacacccggtctgttgcctgcccgggcgccgatattacgccaccgtcaaacacttcctgtcccgctgcattaatcgctttaatgtcgctgtaccgcggcgggatgatctctctgccttcggtatttaccaccccgtatttatcgcctatgctcactttcatgacattgcccgtcaaaccggttcccgtgtattgaaacgggagcagtgttttaccgcccgcgtctacgaggccggttttaccgtttttttctacggcaaacagcgtggtggccggtccgggcttgcatttatcatagacagccggaataatcacctttccgttttgatccatgatgcctgttttaccgttggcagtaaaaccaaaataagtgctgttgccgccgaggtaatcaaacgattcgtaccctgccggaacgatgatggtgccgtcttccgctgccagtccgactttacctgctttggtaatttctatagcgttttttagtgcatagcttttacctgcttcttcgtatatgggttcctgtaataccttaccggttttaatctctatccatccccagcgtccatccttctttattttcaatacatggggtgtgagcgcgcttacctcggcgtatataggcggacagatgatattgccgagtgtatctgcggcgccatattttccattgagccgggtaattacaaagcaataattttttgtggagtcgttgttgtcctgctcatcggccagggtgacctcatcatatttgaaaggggcaatgattttaccggcattgttgatagcgccataggcgttgtgcttcacggctactacggtattgtagtaacccgtgttttccgttttatctaccaatactgcaccggaaacatgcagccattgtttttgctggttaatcaacacgggggcaaactgtccttcgaatcttccgaggtagcccgctaccacgggctcttgtgcatgcagggatatgctgtttaaaaggagtcctgccagtaaatatctttttatcatctgtcttgctacattatgaaatagtattcttctcatggaagatatgcaaagatgcggatctttcagaaaacgcaaataaatatctcttgttaaaaagataccggctacttttccgggaagcgatccatccttttccgttcaacgaaaaggtgcagggtttttataatttttttattacgtttgtcgattcccaattggggtgtgaacctaagaaatgaaaaaaatctgcattatgaatggaatgactaaatctgttgccactgcattcctgggcgcgttcgcagcgctacaggggctcaccgcagtagctcaatcgaatgaaaagccgaagttgatagtaggcattgtggtagaccagatgcgctgggattacttataccgttactacgaccgttacgaagcgggtggtttcaaacgtatgctgggcgacggcttttcctgtgagaacacttttatcagccaccttccctcctttaccgccgtgggacacagcaccatttatacaggcagtgtgccggctattcatggtatcaccggcaacgactggcccgatcagcttaccggcagaaaatggtattgcacagaagacactaccgtacaagccgttggcagcaacagtgctgcgggcaaaatgtcgccacgcaacctgttggcctccactattacagatgaattaaaactgtctaccaacttccgctccaaagtagtaggcgtatcactgaaagaccgcgcctctattcttcctgccggacatacgcccaatggcgccttctggctggacgacagcaacggcagctttattaccagcacctggtacatgaaagaactgccggagtgggtaaagcgttttaacgaccgcaaagagccccaacagttaatgtctaaaccctgggaaactttatatcctatcaatacttatgtgcagagcagtgaagacaacgtagactgggaaggtactttcccgggtgaaaaagcccctgtttttccgcatgcactaaaagatgcttataaaaaagatccgggcaacctgagatccactcccggtggcaatacgctcacactggattttgcgaaagccgccattgaagggtatgacctcggcaataataccgtgaccgacttccttactattaactgcgcttccaccgattatgtaggccataaatatggtcctaattccattgaagtggaagatacttacctgcgactggataaagacctgtcggccttttttacttacctggaccagcgtgtaggaaaaggtaattacctcgtgttccttactgccgaccacggcgccgcgcatgccattaaattcatggaagagcataagctgccttccgggctgacagaaagcaggaaactggtagctggcctggatagcacgctgaatgcacgttttggcgtaagcaaactggtgtcttcctttatgaactaccacgtaagcttcgacaaaggtaaaattgcggcagctaaactggactatgatgcggtgaagaaagaaacggtgaagtattttgaggcacaaccgggtatccagtttgccgccgacctggataatatcggcgcaaatcctttaccggagccgctgaacaccatggcgatcaatggctacaaccgtaaacgtaccggttccgtgattgtgattcctgagccaggatggtttgaaggttcgctgaagggcactacccacggtaactggaatcctttcgatatccatatcccactggtatttatgggatggcatgtaaagcatggcgcttccaatgaaaccgtacatatgacagatatcgccgctacccttgctgcaatgctgcatatacaaatgccaagcggttgtgtaggcaagcctgtaaaggaaatactgcaataatatattccgggaggacttacacatcctgtaaatcctcccggattctttttatactcttcccataaacggatctgttatcccttcttctcctgtttccactcttcctgcataccgttgactaaaagtatcaaagccagcagcctgtacactgaaatcgtaccagccatgacttttttgcaatggcaatacaagttccaaagtggcgccggcggcaacattccgctggattacttttccgccgtaggcattgtctgtgatactgaaatcgcgtgcactgctaccggtattggctacacgtaaaacaagattgccggttgctttctttttcagcttgccatttatttcataacccagctccaggtccagctgcggatgttttgcggagccttcaaatgcgcggtagaatccgttggggccgtgcaggtgcagctgataacggttatccgcaaaggctttggcgggccactcataggtgatcgtgtctccggctgccactgcaaacgaccaggttcttcctgtttctgtttcaccggtttgttcgtctttgtaagggaggttggtgtatacagtaaaaggcgcgccatgtgcccggtcgccgaacaattgtttgtcggctttcattttcagcgtcagcaactgctcaccggctttccactgaccatccgccagcagttcataaggcaatgcgcaggaagggcgggtacctttttcctgttgtaagatcgtagtgccgttgccgttagcaaaggcttttatctcttcaccggtaacctttttaaagcctgcgggtgctgatttaaagcgggcgttattaatattttccactacacggcgctggtccaggaaaatctgtttggctggtgtggtggtattaaacggactgaaggctgcggtaagatcaccgctgatggtgcgtctccactgactgatattatccaggtgtacctgtttgtttagcttcttactaaaaaatgtttccaggaattgtaaagtagaagtatgctcaaatacctgtgagcatacctttcctcccctgctccagggcgatgcaatcatcataggcaccctgaatcccagtcctaccggggcttcccgggcctgcttttcacttatgccctgtttcagttcatgcgccagtctcacctgttctatctccgtatctattccggcggagcatttaccagtaccgggtttattgttatcgcagatagagaaaggcaccacatgatcgaagtaaccatcattttcatcataggtaacaatgaaaatagttttcttccagacgtccggtttttgtgtgaggatatcgagtatttcggatacgtaccaggcgccataccagggggcgctggggtggtcggagaagttctgcgggcctgccagccacgatacctgaggcaatgcgccttcgttcacatcttttcggaactggtggagtacatcgccggcgggcactgtgatggtgcgttcctttgagccgtctttataatttacggctgttacgctccggtaggcgggatcgtttttattcactacaaaagcgcgttggtacagcgatttctgttgatccgttaatttctcatagctttctttattccattgcaggagttcctgggtagcattgtccagcaccgcttgttttttggagatatcggtgcggatcttttcggcggcggcatccgaagaagggctggcttcctggagtttattgatttcgtccggcagggtttccacctgtttcaataatccgtttacataccgttcagagaacttcacgttataggccgcaaaaaattccagcaggttacagccaaaatttgcgagccatgccctttcctctcctttccatccgccaccgcagctgatttcattctggtaaaatttccaggcgatattattttcctccagtaattccgggaatgttttccacggtagtttcccgtagctgaagtcatcgttccggatatgtgcttttggcagtccgtctacttcatgtacaattttgcccgtccagaaaaaggagcggttgggcgtggtgctggtcatagccgagcagaagttctggtcgcataccgtgaaagcatctgccattgcgtagttgaaaggaagatcttcacgggtatagtaccccattgttaaaggcatggccgcatattccttgttgccgggtgtttttgcgatgagccatttatcgtagcggcctttgttgtaggcatctacctggctgggcctggagtggggcaatgctcccatccacgtggctttggtatctttgatattcagccggaaaggtgcgtaggtatcaccctgggcgttggtttgaaaccataccggttttgcgtccggcaagcatacggcgcgcggatcattaaaaccccggacgccctgtaaagaaccaaagcagtgatcgaacgaacgattctcctgcatgaggatcacaatatgttccgcatcgtggaaagtgctgccgggagcaggatctatggccagtgcccgttgaatggatgcgggcatcatggttgacaagcctgctgcaccggatagtaataaagatttttttagaaattctctgcgtgagtccatttatattccgattgagtgggttttacattgttcgaaaaacaaaataaaaaacattctcaaggaatgcaatggcgcctcccgttatgtgtttattatccggtatgtacggctatggttgaggacaaccggtaagggtatgccattcgtgttcggttcgggtcatgagcagggcattgtcaaatgcaaccgttcctttcttaaacaccgttgtattttcaaaaaaactggaagctacgtgcagcagttgcaacgggcttactttccattgataggtttgtaactttagcccgtcgagcgactgctgactattcggagaataaccaacagcgccaccttcaaaaaatgcagaggcgttttccagcgtttcaaaaacagaggtcgcgggaaactcgctggtgctgcgtgcgtcgatggagatagaggttttatctgagctggtaaaatcaatatgaaaatgcccgccggcctcttttacgtgaaaatccgccaggtgatgtttcccgggaaacagtcgtccgccggcaagggcgtttagcttcgatgaggtatccctgcgtgggatataaacgccttctttcgtaataccgttctcctcccactctactgcaatgcgatgggcgccattttccgaggaaatgcccataaaatcaggcaagcctttaggcttaatatgtttcagtctgatcaggcagataccggcaatggctttgcctttgtaaattttagggcggaaaggtgcgggcaacagcgactgaacggcttccgggtccacggtaaaattcaccaggatgcggcggtcaatataaccatgtataacgggtagcttcatataggtaaggatctgattaaaggtactgcaaaacaacttcagaaatgactatttcataaaattgaacaaatgttttgaaaagttgttcaatttactatctttgtaaaatattaaactcaaaaccagactatggcggtaagtgaaaagaagggaaatatggatgcttccaccgaagagcggattaaagccgcggccagaactgtatttaccaagaaaggctaccaggctaccaaagtaagggatattgcagcagaggctgatatcaacctgtcgcttgtcaattattatttccgcagcaaggaaaagttgttccagtttgtgatggcagagatcgtggagaaattgattaccacggtaacgctgatccttaataacgaacagttaagcgtgcagcagaaagtggaacaggtagctaatcactatattaacctgttgctggtgaatccggacttcccgttatttatggtgaatgagatttttgccggcacggatgagttgttgaaagacaaccgcaaaaatgccatcttccagtctcatttctttaaacaattagcggcgctgcataaagaaggtaagctgagcatccagccgatacagttaatgatgaacctgataggctttgtggtaatgcctttcctggccaggcccttactggaaaggaacaaggtggtgaaaccgggagaattcaccgcgctgatggaagaacggagaaagctgatacccatctggattaaaggcatgctgaaatagctgcttttttttgcccggaaattgaacaacttttcaaaacaataattcaaactgaatattgcactatgaacttatttaaagctttgtgctgtttcatattattggggcctgcggtgggcagggcatggagccaggcgcctgccacccttaccattgaagagtgctataccctggcccgccagaattatccgctgatcaggcagtatgacctgatcgcacgcagcagcaggtattcggtggaaaatgcagggaagttgtatttaccacaactcaccgtaagcggacaggcaacgtaccagtcggagaccatcaactttggcgaggcaatcccttcattgcccggcgtgacattcccttcgttgagcaaagaccaatataaaatacaggcggagatctcccagcagatctatgatggcggcgtaagcaaactgcaaaaggaaagcagccgtgccaacgaagccatacagcaacagcaactggaagtaaacctttacgccatccgcgaccggattacgcaactctatttcggaatattactgatggaggcacagctggagcaaaacgggctcaggaaagctgacctgcaaagcgccacggataagatgcaggcggcgctcaacaacggtgtggcctaccgtagcaatgtggatgaactgaaagcggaaattatgaataccgagatggccgccactgaattcagcgctaacaggaaggcctatatgaaaatgctgtcggctttcatccatcagccgctgaacgatagcacccgcctggcatggcctgcaccagtgacgccacaacaaggtatacatcgaccggaaattacttactatgatattcagaaaaaagccttcgacgtacaggaaaaacaattgcagtccggttaccttcccaaactgagcgcttttatccagggcgcctatggacggcccacactgaatattatcgacaataaattcggcacctggtggctgggtggcgtacgcctgaactggtctttaggcagcctctactcgctgaaaaacaaccggcagctgctggacatcaaccggcaaaacctggatgtaagcaaggaaactttcctgttcaataccagcatgaacctccagcaacaaaaccaggatattgataagtttgccaccctgatagaacaggatgacagcgccattacgctccgctcctctgtcaggaaatccgcgcaggcacagctggacaacggcgttatcaccgtacatgattacatctcccagctgaatgcggagaacctggcgaaacaatcacgtatcctccacagcatacaattattacaggctcaatacaattataaaaacacctccgggaactgattaattattgcatatgaaatacaacatgatacttggtatagccgttgtgatgatgatcaatgcctgcggaagcggcaaaaacgatttcgatgcgtccggcaactttgaagcagatgaagtgatcgtatctgccgaacaaaccggtgaaatacagtccttcgttataaaagaaggcgacaagctcactgccgggcaaaccgttggacaaattgacgtaaccatccccacccttcaaagggaacaggtgcaggcatctatcaatgcgctgaaagaaaaaacccaggacccggtgccgcaaacagaactggtgcgcaggcagctgctggtgcaggaagcacagctgcaacaacaataccgggaaagaacacgcacggagaacctggtaaaaagcgacgccgccacacagaaacaactggatgatatcaatgccctcattgtgcagctggaacggcaaatcagcgtgacccggcaacaactgaagctcaacaactccaatacgtctacccagaaccgcagcatactcagtgaaaaagcaccgctggaaaaatcactggcccaatatgcagaacagatccataaaggacagatcattaacccggtgagtggtgtagtactgctgaaatatgcgctgcagggggaaatggccaccgtcggtaaaccgctgtacaaagtcgccaatatcgataccctttacctgaaagcttatgtaaccggcgttacgcttcctcaaattaaactgggtcaacaggtagaggcgcgcattgaccagggccaaaagaactataaatcatacaccggtgaaattacctggatctccgataaatctgaatttacccctaaaaccattcaaacaaaaaatgaacgggctaacctggtgtatgccatcaaggtaagggtaaaaaatgacggctatctgaaaataggtatgtatggtgaaatgctgataaataaagcatccaaatgagcgcagtaacactggaccatatcaccaaaacttacgacaagggtaaggtgctggcagtggatgatatttcactgcaggtggaggaaggtgaactgtttggcctgatagggcctgatggcgccggcaaaacatccgtcttccgcatcctcactaccttgttgctgcccgacaaaggtacggccaccgtgcgcggctatgattgcgtaaaagactatagagaaatacgtaacaggatcgggtatatgccggggaaattttccctgtaccaggacctgaccgtaaaagagaatctcgatttctttgccaccctcttcgggagcacgattgaagataactacgaactcattaaggatatctacgaacagataaaacccttcagcgatcgcagggccggaaagctcagcggaggtatgaaacaaaagctggcattgtgttgcgcgctgatccacaaaccggaagtattattccttgatgaacctaccaccggcgtggatgtagtatcccggaaagagttctgggacatgctgaagtacctgaagcaacaaggtatcaccatcgtggtgtctactccttacatggacgaagccgtgctttgtgaaaggattgcactgatacaaaatggtaagatcatgtcggtagatacgcccgataatatcatgtccaggttcccggtgaaactctatgccatcaaggcggacaatatctatcacttgctgacggacctgcgcagcatgccggaagtggacagcagctttgcttttggggaatacattcatattacgctgaaagacgccggcgctgatatagaggcattgcagcgtaacatcacccaacggggacatacacacgtagccataaaattaattcatccgggcattgaggatagctttatccggttaatgaaccaggcctaaaacagggtatcatggaagaaaaagtgattgtatgcaaggaccttacgaagcggtttggcgacttttatgccgtcaataagatttcttttgaagtaaacaaaggagagatcttcgggttcctgggcgccaacggagcaggcaagactactgccatgaggattctctgcgggctctcccaccctacttccggcgaggctaccgtagccggttttgacgtatataagcaaacagaatccatcaaaaagaatatcggttacatgagccagaaattttccttgtatgaaaacctgacggtagtggaaaacattgaattctttggcggcgtgtatggggtttcctccaccgaaatccgtaaaagaagcgataacctgatccaaaagctggggctcaccgctgaagcaaaaaaactcgtaggggcgctcccgttaggctggaaacaaaagctggcgttttcagtagccatctttcatcagccgcggattgtgttcctggatgaacccaccggtggcgtggatcctgttaccaggcgacagttctgggacatgatctatgaagcggcggcaagtggcattactatttttgtaaccacccactatatggatgaagcggagtattgtaaccgtgttaccattatggtggatggaaagatagaggcattggattctcctgttaacctgaaagcgcagtttaaggcagaaaatatggacgaagtattttaccggttggcccgtggggccaaaaggtcgggcgactaaaacatttttatgaaacagcttcttgtttttatccggaaggaatttttccatgtattccgtgacaaacggaccttactgatcatgtttggcttgccggtagcgcagattatgctgtttggttttgcactgaccagtgaggtgaaagatattacgctgatggtgattgatcattcccgggatgctaattcacaacagctaatccataaaataaaatcatcttcctactttatcgtcagtgaatcatctgtcgattataacgatatagaagattcctttaaaaaaggtaccacaaaatgcgcgctcattttccctgccggttttggcaacgacctccggcacggtggcaaagcgcagctgcaaattattgcagatgggtccgatcccaataccgcaaaaaccgtggtaaactatatcactgctatcaccacagcttaccagcaggagatcagtccctcgcaacaactgccttatgtcattgttccggaatcgagaatgctgtataacgaagaaggcaatggctccctgaattttattcccggcgtaatggccctggtgctcatgattgtatgtactgccctcacctctgtgtctgtagtgcgtgaaaaagaactgggtaccatggaaatattgctggtatctccctttaaaccactgatggtgcttattgccaaagccattccgtacctggtgctgtcgctgctcaattttaccctgatcctggtgctggcggtgtttgtgctggatgtgggcattaaaggcagtatcctgctgctgtttatggaaagcatgttgtttatcattacctgtttatcgttcggattgatgatttccaatacgaccaactcgcagcaaacggctttgcttttatccatgatggggctgatgattcccaccatgatctttacgggctttatgttcccgatagaaaatatgccaaaggttttccagctcatctccaatattattccgtcccggtggtatttcctgattattaaatcggtgatgctgaaaggacttgggtttgaatatgtctggaaagaaacactggtgctgttgggtatgaccattgcgctgctcactattgcgcttaaaaattttaaaacgcggttatcatgaaagtgctgggttatttattaaaaaaggagttcaggcagatcttccgggacaaaacgatcctggcgatgatgtttgcgatgcctgtcatacaactgatcattcttcccctggcgatgaactttgatgtgaagagcgtaaaccttgcggtggtggacaatgatcacagttcctattcccggcagctgattgccaagataggcgcctccggttactttaaaatagtggctgccgagccttcctttcagcgcgccatcacctatattgaaagggaaaaagccgatgtagtgctggagatcccaccaaattttgaaagcaacctgataagggaagggaaacagcgtgtaggggtatccgtagatgcgattaacggcaccaaagcggctattggcggtaattacctcatgacggtgattaccgacttcaataagaatatcccggttaatattggcgggaacatgatgccggcggctggtatcatcgatattacctactccaactggtttaatcccctggcggaataccggttttatattgtaccggcgatcctggtgctgttgcttacgctgatcggcggctttatgtcggccctcaatattgtacgggagaaagaagtgggcacgatagagcagatcaatgtaacgccgattcagaagtggcagtttattctgggaaaactgattcccttctgggtagtgggcatgattgtgtttacgcttggcttgctggtggcctggggaatatacggcatctggccggtggggagttttgtaacattgtatgtatttgccgcggtgtacctggtagcattgctgggcttcgggctgctggtatctacctataccaataaccagttgcaggcgatgtttgtggcattcttttttatgatgatctttatgctgatgagcgggctattcacggcggtagacagtatgccgccctgggcaaaggtgatcgccaatttaaccccggtgacacatttcatcaaggtaatccggatgattgtactgaaaggcagtggttttgccgatgtgcagatggagctgttgtatcttatcctgtttgcagtgctgttaaacggatgggcgatctttaattaccggaaaacgagttgaatcattctaccggacacattatgtttttccacagtatatatctccttcacatattactaaccgtacgcatttacccaaaataaggtggtttccaagtcccacctcaaaaaattacaaataactgactatcaacccaatacattgtaaaacaggctcaaacgcccgtcctacctgctgtttcgccctcttttcctgcttattgttagaaaaaatattgaaataaaatagattttatgaataaatttgaacaatcaagtagctacttttaaaattttaaaaaatgagcaataaacccgctaccttatttgacaaagtatgggattcacatgttgtgaggaaaattgaagatggtccggatgtattttttatcgaccgccactttattcatgaagtaaccagccctgtggcttttcttggaatggaaaacaggggtttaaaggtaatgtttcctgaaaagacctttgccacagctgatcacaatacgccaacgattaaccagcatttaccggtacaggacccgctttccgccaaccagttgaaagccctggaaaccaattccaacaagtatggcatttcccactggggattaggcaatccaaaaaatggtattgtgcatgtggtaggtccggagaatggtattaccctgccgggtatgaccattgtatgtggagattcccacacctccacccatggcgcttttggagctattgcatttggtataggtacttctgaagtagagatggtactcacctcccagtgcattatgcagccgaagccaaagaaaatgcgcatcaacgtaacgggtaaactggggaaaggtattacgccgaaagacgtaaccctctacattatatccaaactcacggcagccggtgctacgggctactttgtggaatatgccggtgatgtttttgaaaacatgagcatggaaggtcgtatgaccgtttgtaatatgagtattgagatgggtgcgcgcggtggcattattgccccggacgaaaccacctacaattacatcaatggacgtgagaaagcgccaaaaggagccgcatgggacactgcgctggcttactggaaaacgctgcgtaccgacgaaggcgccacgtttgacaaggagtatacttttgatgcagcggatattgagccgatgatcacctacggtaccaatccaggtatgggcatgggcattaccaaacatattccttctgcgctggccggcgacagcaaaaccagctacgaaaaatcattgcagtacatgggtttccacgaggaagaagccatgctgggtaaaaaagtagattatgtatttattggcagctgcaccaacggtcgtattgaagacttccgtgcatttgcttctattgtaaaaggaagaaagaaagcagaccatgtaactgcctggatcgttccgggatcgcacatcgtagaacagcagatcaaagaagaaggtatcctggatatcctgacagaagccggtttccagctgcgtcagcccggatgttctgcctgcctggcgatgaacgatgataaagtgcccgccggcaaatacgccgtgagcaccagcaacaggaactttgaaggcagacagggaccaggttccaggaccatgctggccagtccgctggtagccgccgctgcagctgtaacaggtgtggtaaccgatccgagagaactgattgcttaatcattccccttcttacaaaattttataaacgatcaacaaaaaatggcttacgataaattcacgatattaaggagtacagcagtacccatgcccatcgaaaatgtggacactgaccagatcattcctgcacgattcctcaaagcgacagagcgcaccggctttggcgacaacctgttccgcgactggcgctatgaaacagacggcacacccaaaaaagatttcgttttaaacaacccgatctattccggtaaaatactggtagcgggtaaaaactttgggagcggcagcagccgtgaacatgcggcgtgggccatctacgactatgggttccgttgcgtagtgtccagcttctttgccgacatcttcaaaaacaactctttaaatatcggcatcttacccgtacaggtaagtcctgaattcctcgacaaaatattcacagcgatagaatccgatcccaaagcggaattggaaatcaacctggacgcgcaaaccatcaccatcccggctaccggggaaagcgagtcctttgccatcaacagctataagaagcacaacatgatgaatggctatgatgatattgactacctgcaggccatgaaagacgaaatcaccacattcgccggcaagagcctgtactaaaaacattccataagtattatgccagtgacccagcgccacgttgaaataatggacaccaccctccgtgatggtgaacaaaccagcggagtatctttttcgccatcagaaaaattaaccattgcacagcttttactgacagaagtaaaagtggacaggattgaaattgcctccgcccgtgtttcagagggtgaatttactgcggtaaaggcaattaccaaatgggccaaagcgaacggctttctggataaagtggaagtactcacctttgtggatggcgacgtttccgtagaatggatgctgaaagccggcgccaaagtaatgaacctgctcactaaaggctcgctcaatcatttaacccaccagttaaagaaaaagcctgctgaacattttgcagaagtagccgctgttgttgcactggctaataaaaaaggactggaatgcaatgtgtacctggaagactggagcaatggtatgcgccattccagggagtatgtgttccagtacctcgacttcctgcaaaatgtgcctgtaaaaaggatcatgctgccggatacgctcggtgtgctcacgcccgatgaagtgaaagcatttgtttccgacatcgtgcaacgctacccgaaaagtcattttgattttcatgcgcataacgattacgatcttggtaccgccaacgtactggaaggcgtaaaagcaggcgcgcacggcattcaccttaccatcaacggtatgggcgaacgggccggtaacgcttcgctggccagcgccatcgccgtactgaacgattttttgccggaggtaaaaaccgccgtggcagaaacctcgttgtataccgtgagcaaactggtggaaaccttttccgggttccgcatcccggtgaataaaccgattgtaggggaaaatgtatttacccaaacagccggtatccatgccgacggcgacaaaaagaataaactgtacttcagtgacctgatgccggaacgatttggccgtacccgcaaatatgcactgggcaaaaccagcggtaaagccaatattgaaaacaacctgcaacagctgggcattaaactgtcggatcctgatctgaagaaagtaacgcagcggatcattgaactgggcgaccggaaagaagtgctcacgcaggcggatctgccttatatcatttctgatgtgctggacagcaaccggatcgaggaaaaggtgaccgtagaaaactatgtgcttacccactccaaaaacctgaacccttctgttaccgtgaagatctccattgatggggaagtattcgaggaacattcacagggggatggccagtacgacgcctttatgaatgcactgaagaaggtatacaaaaagctgaagcgcgagctccctaccctgacggattacgcagtgcgtattcctcccggcggtaaaagcgatgcgttgtgcgaaacgatcattacctggaggctgaacaacaaagagtttaagacccggggactggacagcgaccagaccgtatctgccattaaggccacacaaaaaatgctgaacctaatctaaactatcaataacaactgaatggctaccaaacatattttaatagttccgggtgatggaatcggacaggaagtaactgcagtaggtaaaaaagtattggacaggattgctgaaaaattcggtcacacctttacttacgacgaagcgctgataggccacgtagccattgaagctaccggtaacccgttgccggatgagtcgctggaaaagatgcgtaaatcagacgccgtgctgtttggcgcggtgggtcatcctaaatatgataacgacccttctgccaaagtaagacctgaacagggcctgctgaagatgcgcaaagagctgggcctgtatgccaacctccgtcctatcaaattatttgatgaattactgggcgcatccagcattaaacctgaaatattaaaaggcgcagatatcctcttcttccgtgagctgaccggcgatatttactttggtgaaaaaggcagaaagaataacggcgatactgcctacgacatagcggaatacagtcgctacgaagtagaacgcattgcccgcaaagcttttgacgcggcgagaaccaggagaaaaaaactctgctccgtagataaagccaacgtgattgaaacttcacgtctctggcgggaggtagtgcagaaggtagccctggaatatcctgacgtggaagtggagcaccagtttgtagatgccactgctatgttgctgatcaaggacccgcgccgtttcgatgtggtggtaactgccaacctgtttggcgatatccttaccgatgaagcttcgcagatagccggatcaatggggatgctggcctccgcctctattggcgatggtaccggcgtgtacgaacccattcatggctccgcgcatgatattaccggtaaaggcatcgctaatccgctggcctctatcttatccgccgcgttgttactggatatctcctttggtatgaaggccgagtcagaagccgtgatcaacgctgttgatggtgtattgaaagcaggcttccgcaccgcggatattgccgacaagcaaacgccagccgataaaatactgaataccaatgctatgggagaagaagtgctgaaattactttaggcaatactgacaatctataaacaaatgcctccctccgggaggctttgttgttttatgccttaagcaggcttcatgtacacctttgaggtggacttgatccgcaaatgccctgacggaatctcccccataaatgtcagaattgcaccacatccgtattcgatttccgcggtatgtttgtgatgtacttaaaaacatatcattatgagaagaatagtttccttcatgcatgtttccctggatggttttgtagccggacctgccggagaaatggactggatcagtgttggcgatgaaatatttgatttcgccgcacaacgtaccaacgaggcagatactgccttgtatggcagggttacctacgaattgatggacggctactggcccactgccgccgaccatcctaatccaagcaagcatgacattgaacactcccggtggtataacaacgtagataaaattgtgctgtccaatacgctgaagggattaaagaaagacaaaaccacggtgatcagtgatgacatcgccggtaaaataagtgcattaaaacagctgcccggcaaggaaatcatcatgtttggcagccccggcgccacgcagtcgctgatgcaacaccagctggtagatgaattctggctgtttgtaaacccggtattgataggcgaaggcattccactgtttaaaaatatcagggaacgggtagggctgaaattactggcaagtacctccttcccggattcaggcgtggtgtgtttgcactatgaaaaaaaataaatcttcctgaatgtgagcggccggcagtatctgccggccgttttttatttaccactcatcatctcctaaaacatcccgtaagtacatacctatatttcctgtaataggtttccttttatagtgcttaaatactgcttaatatctacattagcagtaaataaaccccttcagatgaaaaagaaaacagtcttttttattgcctttataatttccgtcactacttacataaatccctgctttccgcaggtaaagtctcctggttttaatatcagcggcgttctccgtgcggatgatcctgcgttgctgaaagaggtggtgatacaactgctgaacgccacggataagaagatggtaaaaattgaatacgccgacagtaccggcagatttacgtttgaacagatccctgccggcagttatgtgattgccacgcagagtatggttttcgggagacatgaatctgctccgttccggcatgaaaaaaatacggcggccggtactatcacattgcaggtaaagacaaccgcattaaaagaagcgtcggttacagcggtaaagccttttatccagcagcaatacgataaaacagttttgaacgtggagggttccatttccgctgccggcagcacagcgctggaagtactggaaaaagcaccgggtattaccattgatcagaacgataacattgccatgcgtggcaggcagggcgtgctcgtgatgatcgacggcaaacaggtgcccatgtcggggcaggacctggccaatatgctgcggaatatgtcggccagccagattgaaacgatcgaccttatcaccaatccttctgccaggtacgatgccgccggcaatgccggtattatagatatccggctgaagaaaggaaagaaatccggcactaacgggaacgcgtctctcagcctgagccagggcaggtaccccaaagttaatccatctctcaacttcaatagcaaacaacaacatctcaatattttcggttcttataattataattaccggcaagatatgaatgaccttaccatttaccggcagttttatgatgaaaacaacgcctataccggtggtaacaattaccagaacttttttaaataccggaacaataaccataatgtgcgtgtgggagctgattacaacattaataagaatgtggtcgtaggttttgccgccaatgggatgtttaatgccagcaacattacgatcaacagtgtggcgcaatctgttgatgcgcaccaggcaaatacaggttcctttattacgctgggtgataactatcccggcaggaagaacgggagcctcaacctgaattacaaacacaccctggataccggcgggcgggaactcactgccgacctggactatgcccgtttcaattcttccgaagaacaaaattataatacccgttattatgatctgtaccaggcggaaaccaaaacaccttatgcactctttggtgatttaaacggcgaacttagtatccggtcggtgaaagtggattacacgcaacccctgaagctgataggcgccaaactggacgcgggtattaaaagcagctgggtgaaatcagataatgatgtgcagtttttcgacaggagtaacggcggcaatgttttagacaaaggaaaaagtaaccgttttatttacaaagaaaacatcaatgcggcctatgtaaacgcttcccggaaatggaaacgtttaagcgtgcagctgggcctccgggtagaaaatacgctggccgacggattccaggtaaccaatgctgaaaagtttaaccggaactatacacagttgttccccagcggctatgcaggctatgaattcaatgcaaaacacgacctcggtttttccgtgagccgcagaatagaccggccctcctaccggcagctgaatccatttaaagtatttctggacccgctgacctcttctgcgggaaatccattcctgctgccggagatcaccaactcgtttgagcttacgcataccttccggcaacagtacaccactaagttagggtatagccgtacccgtgataacatccttattgtactatcgccggatgaagcgccgggagcagtcatccaaaccggcaggaacctggctaagtatgattattacaatctcagctttggcttcccggtaaatatccgtaaatggcttagcagcaccaacacagcgctggtgtattacgggcactacagcggcaacctggtgaataccgatctcaatgtgaacagggtatctttcaatttcaattcggtgaataccattaccgtaaacgcattgactaccattgaagtgaccggcagttatgaaagccgggcgtattacggtttccttgatatcaggggcttctggtttgttaatgccggcgcacagcggcagttatggaaccggaaggcatctgtaaaactgaatgtgggcgatattttctttaccaaccaaacgaatgcagtgacccggcttacgggctatggcgaaacgtttaagcagaaaagggatacgcgggtagcgacggtgaccttcaattataaatttggcggaactggagccggtggcgtcaaaaggaagaccggcggcgctgaagacgaaaagcgcagggcaggataaaaatttatacatttattgcatgaacttagttaccgaactggaagaactggccctggccacccgtttaaaacggctggcagagcgcctgtcgcaggacgtgagccagatatacaaagaatcggatctggactttgaagcaaaatggtacctgatcctggaactactgagccgtgaaaaagtaatggcggttacagagatctcttcttcgctgcagctgagccatgctgctgtagtacagtttacggagcagatgcatacgcatggtcttattaaaacggcgcctgactccaaagacgcaaggaggagactgatttccctgacgcttgccggtaagcaaatgcataaaaagatcggtcctgttttgcaggtgatcaaagaagaaaaccggaaatggctggccgaggccagcgcagaccttttgcagctcctgtctgaactggagaaatcgctggatgaaagaagtatgtataagcgtattaaagtgagcctggtagagcaatctgccaggtgaaccggttatttgataccgagtttatccaatacatggttaaccactctgtcgcagcggataagatggaatggaaacaccaggtcgtttttatagtaatcggaaatctttccacgcagcatgagccgggccctgatataccggacctttacgtttaccgcggagatattcaatgcagctgcggtggctgccacgtttaagccctctacttcccgcattacaaataccaggcggtatttctcagggatttcgagcagggcaagttccattacccttcccaattctttatcaataacttttgccacgggcgattcttttaccccggcactatttgccgggtgatgatcatctaaaacagatagatcctcactgcccaaccggtttttctttttcagcaactgactgcactcattaatcatgatcctggtcagccaggtcccgaaggcggattccatcctaaacttatccagattctgataagcattgatataggtggtttgcatcatgtcttccacatccatatcattatccagcatggtcatgcctatccggaacaggcgggcattgtggcggcgcatcagttgctcatagaggcgctcttcaccggccagtactttagtgattaattcgtagtcaatttcggtgtcggttttcggcagtgtggtcattcttcttttattagatgataaatcgactgagaagttacaaaaaacttttatgggattttgtaaccatttgaattttttatactctaattaaaggagggccggttaacggcccctgatttttgacataacctaacttgtgaagcagctgctatgaaaccagataacatttttcatctgcccggcataaaaatgccggagctaacccatcagaagatccaggagctgaagaaaacagcgaagggaaaactcattaccggtactcccatggaggctttccaggcattggtgagctcaatggaaattgcgctgcaggagcaactggcgcaatatgattatatccagcaaaccgtaatggacagcgccaaacggaaaatgctgctcctggaaatgctggacgatcatctctacctcgaatttgcctatcatattatgtttattaaatggcgggagcaacaaatcagtaaagcatcctgagagggatgccggtgacggatgctgctaatctcattaaaactatacatttgcacacaaacaaatgctatggagaattacagcatcgtcatttttatactggccatcatgattatgctgtctgcggtggcagacaagataaagttaccttaccctgtgctgctgatctccgcgggaataggcatcggatttattccggccctgccaaatatcacgctgaacccggatatcgtgttcctgatatttctcccgccattgctatatgacgctgcgtttaacatctccccacaggaatttaaaaccaacttcaacaccattggtacattggcgatagggttggtgtttctgacagcgggggccgtagcggtgattgcgcattatcttattcccgggatgagctggccgctggcttttgtgctgggcgctatcctgtcggccacagatgcggtggcagccatgagcattaccaaaggactgggactttcacataaaacggtgaccattcttgaaggggaaagcctgatcaacgatgcttcggcactggtaacttatcattttgccattgcggcggccaccggtaccgcctttgttttctggaaggcctccctggaatttgttatgctgatggcaggtggcgtgctggcgggtatagtagtaggcaggatattggcgatgatcctgaaaagggtgcatcaaaacgacctggtgaccatcagctttatgctgctgatgccatttgttacctacctgatggcagaagagctgcatgtttccggcgtgattgcagtagtagtgcttgggctgatgattgcgcggatcagcgggaaagttttcccggagaaattaaagcaacagtccaggtccatctgggatattatcatcttcctgctgaacgggcttatctttattatcatcgggctgcagtttccttatatcattaaaagtattcccagtcaccagatcctgccgtatatcggttatggatttatcattaccctcgccgctttgttattgcgcatgggcagggtattcctgcaacagatcaatttagaccaggctttcaaaaagggcaaaggcaggatcactgaaaacgcgttgctggatttcaagaacagcctgatcatcagctggtccggtatgcgcggtattgtatcactggccattgccattgggctaccgatgacactgaaagatgaagccccctttccggagcggaatgccatcatttttatttctgtggtagtggtgttgtttacccttatcgggcagggtatctctttaccgtggattgtgaaagccgtaaaactctccccggcagataaaaaaacgccgcattaacttatcacaacagccggaaatatactatcttactactaaaggatgcgtggatgaaaaaatcactgttgcttttcaactgccttattttattgttccttcctgctattgcccggcaggagccgccagatacggttaaaacaggaatatacattaccagcattcatgacatcgacttcaaacaaagtgagtttactgtcaacctctggttgtggcttacctataaaaacaagcagttcgattttatacagaacctggaaatcccccaggcaaaaacctttaccaaatcctactccactatcgactcttccaatggccggatctatttgctgatgaagctgcaatgcgtgatgaaggactcctggaggatcaacaactttccttttgaccggcagcgtttgcggttttccattgagaactcacagtttgatgccaaatcacttgtgttttcagtggactcactaggcaaacattttgacccgcgctttacgctgagaggctgggtgatcgacagcttccggatcaataccggtataaaagcctatgaaaccgcgtttggcgacgaaaatatcggcaggccacatacagagtacagtaattttacagtgagaataggcatcaacagggatgctacccagttgttctggaagatgtttctcggcatgtacgtttctttcctgattgcttacatctgtttttatattcaccctgataatattgattcgcggtttggacttggtgttggatcgctgtttgccgccattggtaacaaatatattattgattcctctctccccgactctactacttttacgctggtagataccctccatggcattaccctgttctttatttttgtggtgatcacttcttctgcatggtcgttgcagcttattaaagcaggtaagtttaagcagagccgccggctggatatcggtttatcgataggtgtgctgctggtatatgtgctgctgaatatttattttattacacaggcggtgtacggaaattagcaagctaaaaaaataaacatagtaatagtagttcccatgtaaaaaatattaatttgcgggaacttatacctattacaagctatgaaattgaagtttctatgttgtgcatacccgctgtatgccttcgccgccatgttcctgttaaccggcaaagcccattcacaggacatctacaccccggcgaccgttaacacctcctttctgcataatgcttccagtaagctggaaaaggaacacaaggatgtaatcagtcatcttccaaaagaaaaccgcgacatgtataaggaaatatatggcaagcggtgggaaaatatcaagtccaagtttgaagagaaggaagtgtatactgctcctgctgcgcagaaatatatcgacagcatgctgacggcgattgtgcaaaccaatcctttgctacaaggccgtgaaatacatgcatacttttcaaggtcggccgtacccaatgccagttatataggccagggcgttattctgttcaatatgggcctgttccggcagttgaaaaccgaaagccaggcggcatttgtgctgtgtcatgaactggcgcattactacctgcatcacaacgagaactccattaagaaatatgtgacagacatcaactcaaaaagtgtgcagcaacagttaaagaaaatcaagaaagagaaataccggaagcaggagcatcttgaagaactgaataccctgctgaaattcgacagccgccggcacagccgcgatcatgagtcagaagcagattcgctgggactggaattcctgcataacagtcactttaatactgccgatgctcttaccgcgctggcgttactggataccattgataacgactccctggatatcaaaccctgtcttgaaaagatgttccggtcgaaaagctatcctttccaatcgcgttggttagcgaaaagcgatctgctactgggtggccatgcgcaattattaaacgatcacgcggtggaggattcattaaaaacgcatcccgactgtaaagtacggatcaacgtactggcgccggcggtagctgaatacagcagggaaacaaacaacaacagcattaatcccgcaatgtttgaaaaactgaagaaggaattctcctatgaaactattgagtatgcgtataccaataacaactatacgtccagcctgtatcaaaccattacgctgttgcaggaacaaccggaagatgcctacctgatttgccagacaggcaaaatactcaacagctgttaccaggcacagaagcagcatcatatcggcgataaaatagcgatgccggcgccgggcaacccggactcttataacctgctggcacaatttatcaggaacctgtacctggaggattatgcccggatcagcaacagcttcctggaacagtacaacgccaggctcaacagctacccggtattccagaaagaaatggcaagaagtatttcttacgtacagccttaaccgttaacaacatctatccctattaactaaaatatatgatacggaaaatactgatttcccttttttgtacgatgatgttcgtcactatggtatatgcgcagagaagactaaacctcggcgatgtatccaacataagagtggccaacagcggcaatattatgcggaataaaaaaattaccggctacttcctgctggtaatcaaggatcagctgagcaaagataccatccggtacagcctgcagatcctggatgagaacatgcacaaggtaagggaatatgaatacctggatgcaaaggacgtatacgtatgcgaagcggcttccaacgacagcaccaccgcattcctcctgagtaattcccatacaggcgacatggaattaaagatcctggatgcagatgggcagcttaaattctcttacaaaagaccttatgtaaagggacagggaaagccaaacatttattacagtgcttatcatgatatcagggatgccaaccattccctttttgatgcaggcacacatggctatatggccatactggatgtacgtcatcgcattcacaccgctgtatttgaagtgaattattttgatgctgctaagaaaaagcactggaaatatacgcagccaaaagaagcacacaaagaatgggtagccgaattcatggctaaaacggataacctgatgctgctggaagttacccgcagcaggaagaataataagtgtacttcttccctcaccgcatttagcattgagtcgaagaaaaaagtttttgaactgaaagaaaaaaaagaagcttatcacctggtaccttctttcgtaatgccgaagcccggcactgataccatcaccgtggcaggtgaatatttcaagggggccaataaggtgagaggccgcgccagtaaaggaatcggtttttatgatatcgactcaaaaggcaacatcctcaccagcacctacaacgcctggaataaggaactgtccggcactttaacggctaacaaaaaagggaaataccaggggttggggtatctttatctccataatatgattcccggacctgatggtaaattatttgtggtaggagaaggttataaaagggtcctgagctcgcagggcgtgatgtttaataacaccaaactgatctctacaaacctggtgatgctggaatttgacggtaagtaccacctcaaacgcaccaacgtttatgagaagcaacgcatcaccctccgggatatggccgatttcaggaatatccataaaatgggttatgccagtaaacgatacaacagcttcgactataaactcacgaccattacggaagactataaaaacttttccatttgctataccgatatgcgcagggtctccaaaaaagaaaggggcgcttatcatattatacgctacaatggcctgaagttccgcaatgatgatttgccgatacagaaagataagaccaatatcagtatatacccggctaaagcggggaacctgctgatatttgaaacgaatgagaaaggtagttcgatgcggatggagaaggtgagttgattttcccttacttcttcacccggtagaaactaatgtcccttctttgctcaaagcccatgtgctcatataaacgcacagcccgttcattggtgcgggttacatgtaaaaaggaggtgatgcccgcgccggcgtgctgatagcatagctgtgtaatcagcttttgcgcatatccgcggccggtgtgatcggggtgcgtacaaatggcgctcaattcggtgaacccggtgagctgcatgcgttcgccggccatagcgatgagctggccattgtgccggatgccatagtagttgcccatcaggcgtgtaccgtgattaaaaaatcctggttgaatgctgttgatcagttcatacatatcgccggcgtcttctggccccagcaggtgcaccatggccgcgtccttttcagacaagggggctggcatcgttgtcagtatcatctgggcgcagggcagttcattttctacggtccaggtacccggtaacacaggcaattcaccgacgatataaaatgtttccccggcatcaatcaaagtatcgagtgcggcaatgctgtcgttatcggtttgcctggcggcaacaaagggtgcaatttcccgctggtatcttttcgcctggtctgttccttgtgcaaagtacgcatgcgtagtggttaacgcgccccaggcggggttgtctaagatggcttccttcatgcatcgaaattatacatttatcagaaaaaataaccggggaagaatatttttttcaggaagttcatcccataaaaaagcggtttcctttgcaggaaaccgcttttctttttatacctgttagtgttccaggtttaatatttctatccttctgaaatcaacgggttgcccttcgctttgcagggcaataaagcctttggagaggagcctgccatctattttaatggtggagtcgtagttgtttaccacaccaccgccaatctgtggcttggaatattgcaatacggtatcgccgttgatgatatgcgtgatcagggaatcgcccagtacaatcagttcgcccctcacccattgctcgccttcataagttttggaggtggattcaatacaatgcgtttcatccagttttcctttgtaaaccacattggtgcccggcgagcacatgttaccggttgggcgtggcttaccatcacctaagccagccagcagctgcatttccacggagatgggccagtcctgctccttaggcatggtgcgcgggtcctgggagtgaaacattacgccgctgttcagcaatgtatattccggtgcggacggataccattttcctacaaaccggtattcaaatttgagatgataatgtgagaagggttgcttataataaagatgcccgaactggtcgttaaagtcgccgtactgatcatagcgtatcttgatgatgctgtcttctacccggaaagtatttccaaagttctctcctggttcgtggtgatggattttcacgatccagtcgttgatatccttaccattaaacagggacacccattcctgttttttttcggattgttttacttcattacaggaaacactgcctgccagcagtgctatcatcaatagtttacgcgagatacggactttgctcatatagataattaaagattttttcattttattgttttctgctgcctggttttggaaatacctggtgtgtttgcgcccattggtaccaaagggtttgcagctgttgtaccttttcgggatactgtgccgccaggttatttgtttccgttttatcggcagcgagattaaataattgccaggtggtatcattgctgagcgacaccagtttccagttgcccgagcgtgcataccgtgcaccgaagtgttcattgaacagctgatcgtgcccggttgtttttttatttttgaaagatggcaacaggctcatacctgtagtggccgggatcttatgaccatggtatacttgtggatattgcgcatgggcgagtgcggtaaacgtagacataaagtccattacatgtcccgcatgatcactgaagcctcctttgttagtggtaattcctttgggccaataagcgatcaatggtgtgtggatgccgccttcatatgattctgctttccagtattgataaggtgtattggctacgttggcccatgtttgcccgatggaagcatacgtggtttgcgggcccggcattgcctgttttttggtggcataaacgatcttgcggccatcgcgggtttcatcggggcggtcgaaaccagggccgtagttggcgcaattttccgggctggcgccattatcagacaggaacaggatgagggtgttgtccaactgccctgttgctttcagcgcttccataatgcgaccaatgccctggtccatccggtcgatcatggcggcgtgcactgccatggccatggcatcccaggcggtatcagggttttgcgcccaggtctgatcctgattccaacgtttaggcaacggcgtagtggcctgatcaaccagtcccattttcaccattttgttatagcgggcggtgcggatagcttcccagcctgccttgtaggtgtctttatactttgcaatatcttctggcaatgccatcagcggccagtgtggcgcattgtgggccacatacagaaagaaaggcttttctgtttccgcgtagcctttgatataagccacagccgtatcgttgatagcatcggtgtgataatagtgatcaggcactgctgtgatgggtgttgttccgcttaccaggctgaagggatcaaagaaatccactactccccagatggtgccgaagaacttatcaaagcccctgctggtgggatactgcgctatgggggaaaagtcgccgaatgtttgatggtgattaagccaggccatttgttcagccggggttttctgtccgactgtattagatacatgccacttgcctgacatggcggtctggtagccggctgttttcagtacttccgccagagttactgcgttagtggaaatatgtccctggtacccgggctcatcctctgcctcggtcatcttaccgatgccagcctgctggttatataaaccggtgagcagcgaagcgcgggtagggcagcaacgggaagtattataaaactgcgtataccggataccgttagcagcgaggaaatcgagattgggtgtatggatttcaccaccatagcagccggcatcggaaaaacccatgtcatccgcgaggatgacgataatattgggccgcgcgtctttcctcagcggctgtttactttttttaaaccctgtgagcagcagactgctcaacaggaatggaacaatataaactgactttggttttacattcatgggttctcaccgttttattactattgctgcggctataccggattcccgttaaaataaaataaaacggacagaaaagtaaataaaccggatgattgggaagaattattttggcaaccggttaaattttccccggaccagttatttcttccagggcagcagccagctcaccggcttcggaggtaatgttccggataacgccttttttatccacgatcaaatgcgtgggataaagatttacctggagactgtcgctgatataacgctccggcacagggatcacggcatagtcaaatattgtttttttcataaagctgcgcagttgctcccggtcgtcgaatgccaggcttaaaaaaagcacgtcgtcccggttacggtattgctgcaccagctggtttaaccggggcatttctttcacgcaggccacgcaatgaataaaccagcatttcacgacaagtatcttgccactggttgactccttcgtgtatgcctggccgttaatatcttccaaagaaataaaaggaaaaggttttccttctctcttatagtatccataataagttttcccgtagtactgcagtgcacttctgacaccggcgggtgttgaatccggcagcgggtagagtttatacttcactgatgaatctgccgtaacaagcttcagcggaagatagttgccgctcgcaaatgcctccaggaatgcttcccggctgatttcatgcgatgcggtatccaatgctgtatacttcaccgtgagcatcatctcacctgttttgtagtaataaagggaagcgtaatcacgaagaatggcgtcgggcgctatcgcgggttccccgggttcaggtccggttgatttatccgccggctgtgagcaggcgcagaaaagaataataataagcgtcagtgtacgggcaggcagcatatggtatccatttacaggtatgcataagttacaaattatttccttaccctgttactctcttctgccgccccgctgcgctgcttccgctgcagctggttcccgaaagtttttgcccatgtcagctttatgatctgcattttgcctgattccggctggaaggtaactttacttttcaggttaaacgcctcttccgccagcgtcccgaaataactgctgatgtgcaccgtgcgtagtatatccgttaccgttagctggagacttcccccgtttttattcagttcttttttaagaccggcattcagcgcaccgaacggatctacctttttggaaccatcgtacgacgcactgttataccagccggagatttcgaggtagaaacgggcaggcaatgtaaaggccgtggagaagttagtattaaagccaaaatattgtttctctactggtgtggcggtatagtccagtttaaattgccgccatccacccgtaaacccgaagttcatattccaccagtcgctcaccttccagggcagcagcgcctgaaaggaaacattatcctggaacaacaggttttgcggagatacccatatcacttcccctgcgggattgggtgtaagctggtagcgggctatgggtgcatcatccctgctgtaaagcagggaaaacgagtagccgtgatagttataaccaacctttacattgttggtgatcgttggcttcagcatagggttgccggtttccaccgaagtgggtcccgagtaaatgacaaatgaggccaggtcgttgtaagcaggacggctgatcctttttgtataggacagttgccattccgcttccttttttttccatgtcaggaaaatgcccggaaagaacttaccggaggttcgtttggtgatctgttgcttattttccggatcatccatttgtgtttgtacatattcatatctcaaaccggctgccagccgtagcgcaggatgcagttgcgcttccagtgagccataggcggcccctatgacttctttcataatgatattattgatagcggcggtactgcttacccaggcctcatccaggaagctttctatcctggagttactgttgttttttgtataggttcctttcagccctgtttcaatttttattttgggagatagctgcctgctgtaatccattttcaatacgccgatccgcatcgaggacacagaaaaggttcgttgcaccggggcaaaaagagtatcgttggtacccggtgtatggccggcgctatccacgaaagcgctgataccggcagagggccggttgtttttataatacaggtaatccaggtcgatgttcagctgctctccttcgcgcatttttctttctgcatacacagatgcgcccaggttatcccagttgttgttaaccctgatatccgcatccatgttataggcggtggttttattcaccaggtattccccgtggttcaacgtatgatctgtaacccggctgatgttgccattgatgctgccgccgatgatggtacgcggggtcaggttcacatctgctcccagtatgatattatgactattccccacggacttcgtcacgctgaggaaatcggaggagctggggcctcccagcaattgcatatcatctgttgcgcgggcaaaccagtcgtaataggatttgtcgtgcgagaaagaataacttccgtacaaggtcgtattgcggagcgtgcggccgaaattaaggctggcggcggccttctctccatagccatatccgccggtaagggagaaatttccctggttcctgtttttcctgatgacaatattgatcatcccggcattgccggcagcatcgtactttgcaggtggtgtattgagcagttcaattttttccacgtcggcggcggtcatgccctgcaggtagatcatcagctgatcggcagacatgcgcagcaacttgccgttcagcatcaccatcaccccacttttgccattgagtgcaattccgttggttctccggtcgatatttacgcccggtgagcgttccagtacttccaggaccgagctcccttttgtaagcacactgctttgtacattcaccaccgtgccatacgcctgctgctgcaacaggggcttgtttgcccgcaccatcacttctttcagctgtttcagcgccggcaggctgtccggcgtggcggatttcccggatgcctgtgcccgggtatccagggccggggacaacagtaataaggtaaggagtacatagttcataagagatcacttctgctgcaaataaatgcgtatccgcaacgccggaaaaacccgaatgaccacgggcggcaggagattgaccacctgcacaaaaggcatcgtttcccggctaaatccctgaaaagccgggaatacggccgttcagcagctgcggtatgcgggtcatcatttatttgctgccattgacatagtaccgggagagaatcagcaaaatgtggttatctttagtaacaggtaattttttatatgctgaacactaatacaagccggaactggctgctgaaatataaactttaccacatccccttctggtgtctttaccattacctgtggtgggtagtggcaatagggaatcctgtgaaagctgccaactccattatcttattccctttctatatcaagtttgcgttttatgtgatattccaggcagccgcggtatatttcaatctctattacctgattccaaaatacctggaaaagggcaggtataccgcctatattacgttgctggtgcttaccatcgcggcaactgcctgcgctattgttggcgggtattatctttgttcagcagtatcaggaaaaagctttgccgtacttttcgggccgggagattactgcttcctgcacttctttggcaatgccctgccctctacccttgccagcatgacactggccatgagcataaagctgaccaaaagctggctgcaaaccaaaaggagacagcaactgctggaaacagaaaaactggaaacagaacttaacttcctgaagaaccagtttaatcctcattttctttttaatactattaactccatcttcttcctgatccataaaaacccggatgtggcctctgcttccctggcgaagttttcagagttgctgaggtaccagctatatgaatgcaatgataaacagattgccctcagcaaagagatcggctacctggaaaattctatcgaactggaaaaactgcggcttaacaataacgtggaagtttcgtttgcgtatcaccggcagcctgtatcacacctgagcatcgccccgtttatactcatgacctttgtggaaaatgcgtttaagcatgtatccaaacaggccgatgggcctaactggatcaggatacagctgcacctcgacggaccgcagctggcattcactgtttccaacagctgtgcggcagacgaatacagcgcacccattattgattatggcggtatcggtttaaaaaatgtgcagcggcggctggacctggtatatcccggtcaatatgaactggacatactccgcgaagccggcagctttgaaatacggctgcagctggaactggccgaactcacggtaccacaattactatctacctaaaatgcctttattatgatcaactgcgtgattacagacgacgaaccactggccagggaaggcatcgccagttatgtaaaggaaatagatttcctcacgctgaccggcatctgtgaaaatcctgtggagttggtaaacctgttaaagcggcaaccagccgatcttatcttcctggatatacaaatgcctaaactcagcgggctggattttctgaagatggtacaaaatccgccgatggtgattatcaccacagcgttccccgaatatgcgctggaaggtttccagttaaatgtgctggactatttattgaagcccattacgttcgaccggttcttcagatcggccaccaaagcgagggactatcaccagttggtaaacccgcccgccaaaaacaactccacgcccgtggaagccggcgcggatcacttttttattaaatgtggcagccggtatgaaaagatccaggtggaagatattctttttgtggaaggcatgcagaactatgtaagcatctatacccgcaagggaaaatatataaccctgttatatctcaaaaacctggagcagcaattacccgcccaggcatttatccgggtgcataaatcttatattgtagcagtgaataaaatagacagtatccaggggaatgaaatttgtatacaatcgcaccagatccctatcagccgcaattaccgcgaggcagtgatccaacaggtggtcatgaacaggttatgggataaagtttcgcggccccccttgccgtaaggtcaaaacattgtatttttggcgccctaaaaaaagcctctgaatccttgcgatccaaaggctgctaactcaaagtaaatctgattatgtaaatgtagtcctgcctggcggtagataccggccggcatcatttcgtatcctttttcagtcaggttcctttaacaggtgcctcgcaaaaacggggtaaccctgaaaaaaagaatggcggcttttaagaaacaaaactgctggtattccttttttcaatatgatgatcaaaaacgtttccaggtataccccaaatataacatggacgcggagtttccacaataccggcatactatgatttatttatacctgttttcaggtatttttgccggcaacgatcatgtatacccaattgttttatattttggctttatgagaagactatctttcctgattttcctggttacagcaacttcctggtgcagtggacaggcgcctccgctgaatgaaaaggcgcttacagacagcctggaaaatgtattgcaacggactacatccgacagtatccgtgcccgggcacactattccctgtcggaatactgggctgtcaacgattcgctgaagtcatcacaacacctggaaaaaggaaagcaatacagtggaaagaattccttcctgcaggcgctttactattactatgaagcgaatatgctgaagaaatccgcgcctgacagaagccagtccgccttcctgaaagcagataccttactcagcaggtttaacacttccgaagcctattctttccggtctaaagcctggtacgactatggcgctattgcccaacggaaagacgattataaagcatttgcagatgtcttactaaataaggcgattccgctggcacaacaggccggcgatcaaacggtagtggggaaagattacctggcggtgggaatcgtttttaaaaatgcgggacagttcgacaaagcagaaacctactgcctgaaggcgatagaaactttcaaaaacgcgcactcccctacgcatgaactggtaactgcctatcataccatcgcagaaaattattcgctgtcggcccagaatgccaaagcaaagcctgcgctggacagcgcctggaagctattggcgcctttcccggaatctgagtacctgttggatcattatgccgccgaagggatgtattatacccttgaagggaaattcaaagaggcgcttgccagcctggacaaaggaatacaactggcccggaagaaaggtttgcgttatgaagagcaacggttacaaatgcagcagttttacgcttatttcaatgataataactttgtaaaagcgaaagagatggccacgctgctgatgcagcagaatgaaacaatgaagctggtaactaaccgcctccagttgttttacgggatggcacttacctgcgaaaacctccggcagatggcgcccgcctatacatggatgaagcgttacagtgagcttagcgacagtcttaccaaagcacagcttaccaacgatgttcatgccctggaaataaaattccggaacgcagagaagcagaaagaaatagatgcgctgaaagccaaaagcatccaggatgcgctgcataccaaaaatgcccggctggtaaactcattgctgggcgccgctattgtcattttactggtggtattgctgtttgccgttttcgtttaccgcagcaagcagaaactggcggcgcaaaaagagctaagctaccggcaacacctgcacgaaatagaacaacaacaacaattacagttcagccaggccgtgttacagggcgaagagcaggaacgccgccggcttgccagggacctgcatgacggcctgggcggcatgcttgccggcgccaagataaacctctctgcacaaattgaagatacctactcgcaggaccaacgggccgaactggaaaagatcacgcttcagctggatcattctgttacagaactccggcgcatcgcacataatatgatgcccgttaacctgctgaaatttggtttgaagacagcgctcaaagatctctgcgaatcactcatgaatgacgctacccgtattgacttccaggacctgggaattgaagataccctccgggaagaagtacagatccacatctaccgcattgtacaggagctgttgtccaatgctatccgccatgcgcaggcgaccaatatcatactgcaatgcagccagaacgaccatatcttttttattacccaggaagataatggcaaaggttttgacacgcaggcggcgggtaaggagaaaggcattggcttaagcaacatccgtaaccgggtgggattcctgaaaggaaaaattgatattgactctgccgcgaacgaaggcaccaccataaatattgaattacatgttgattaatcccgctacactcgctattgtagacgaccatccgattgtacttgagggactgcagaagttgctcacgaatgtgaagagcatacagattaccgggtgcttcacttccggaatggcttttatgtctttcctgaaagaaaataaagtagatgtactactgctggatatcacgctgccggatgccaacgggatagagctatgccgggaaattaaggcgctgtcgcccgacacacacgtactggcactaagcaatcattctgaacgcagcatgatcctccagatgatccagaacggcgctacggggtacctgttgaaaaatatttcttccgaagaactggtggcctgtatccaggaagcactcagcggaatgatcactttcagcaaaggcgccaaagaaattatggcacgcccttccatcagcgaactaaaaggtattccgcagctcactaaacgggaaaaggaaatactgcacctgatagcagatggtaaaaccacccccgacattgcgcagcagcttaaccttagcccgttaaccgtagaaacgcaccggaaaaacctgatacagaagttccaggtaagaaatgtggccgcgctgattaaaatggctgctcaacaagggctgttataagagctgtttatttatgcagtcctttcctgcgcagataagccaatagcttttcaggataatctgtctggatcacattggcaaaggccgcgtctttacgcagctgatcaaaaccggcatcgtctttttctgattccagtttatcatactttcccaaagcgttcatccatacccgtgtgccgccggtggtaatgcttttcaccagggaatcggagtaaaaagaagcgtctccgtgaataaccgggaacttgccctgcttcgcggccatttgttgtatttctgctatttccgccacactgtgcgcgcggggcattaccgggatctccggattccagctgtacagggtgggcgctgtatgatgatcatagataaagaacaggacctgttcttccattccatgtgccgcaatctgggcaaaggcctgcctggctgccggctcgctctcttccttaaaatctacatctacaataattcttcctttggtgatctttaatacctgttcaaaagaagggatagtctccgtggtgggttttcctttaaaaagtaagggaaactgctgcagttcgtggtaggtataatcccttaccttgccgggtttcccggtggtgcgggtaatggtttcatcgtgcataagcacgaggatatgatcttttgtttcatgcagatctatttccacgatatcaataccctgttcaacagcttccttcacagcagcgagtgagttctccgggtatttgttatgcgaagcacggtgtgccgccaccatgatatgttccgggtgatgtttaaactcgtcgaggatagcgtctgcaggcgttttttgctgtgcggttaccggcaggctgatggcacataaggttgctaataataaacggttcatcaggtatttatttttttacagcgatagacaggatgttcctgtgaaagtatattatttcacagaagatccctaccggcttaataaaaaaataatcttagtaatcataggtgtcggttgccggaaaaaatagttacattatagtgtattaacacccatcaaacaatagccatgaatattaccacgcagcggttaactacgcatcacctcgccgaatttattgaattgctccaggtatatgaagcggtatttgacatgcaggacttccaaatgcccgataagagttatctcaaaaacctgttgagcggggactatctgattatgtataccgccatgcatgaaaatgccgttataggcggacttaccgcctatgtactgccctcctgttacgcacgcgctgctgatatatatgtgtatgactttgcggtgcataccgaatttcaaagaaagggtgttggcaaacatttactatctgccttcgcggaatactgccgggagaataactacgccacgttctttgtacaggcagtagccacggatgtacatgccgtggaattttaccgtgctaccggcggtgcgccggaaaatgtagtgcagttcacttacaccgatattaaacaataaacgaccgtccttctttgttcatttccttccggatgccatttaccacatcttccagggcaaccgatgttgatttccgttccagcgctttcaggcaggcgtattgtactacattgataatatttccgccggtgatttcatactttttcacttttccgggaatatcttcttcatccaggaactttacgtttggcgggaaggttttctgccagatagccgcccgctcccgttctccgggtacctggaattgtatgatggcattgaagcgacggataaaggcgtcgtcaatattatttttcatattggtagccagtattaccaggccattaaaatcctcgatccgctgcaacaggtaagatacttcctggttggcgtatttatcatgtgcatcccgtacgctggtgcgttttccaaacagcgcatctgcttcgtcaaagaaaatgatccagcccttatctgctgcctttgcaaacaatgtttccaggtttttttctgtttccccgatgtacttggaaacgaccatcgacaggtcaattttatatacatccctgccggtatatttaccgagtaggctggccgtaaaagttttgccggtaccgggaggtccatagaacaatgcgcggtagcctttcttcagcttatgtttcatgccccattcattcatcagctgatcgttgtgatgcagccatgtttccagctcccggatctgcaccataatggattcatccagcaccaggtcgttccagctaagctccgtggcgatgagcctggcggggaagctcatgctgaaatgcggcctgccgggttttccttttataaagagatttacatagtcgatgtccatcataatacgggcgctcatcagaggttctcctgcctgcacatcttccagccataatattcttttgagcgcaaattcatgatcgggttcaaacagctcctgtacctccaggcgttttttccagttggtgcctgccagcaagaaaagcgctgtttctccggtgggcaggaagccccggaattgtttaccgcgtacaccgcccagttgcgggaattcgcccgcctgtggcaggaattgctggatagccgtgtcgtaaaattccggcaggatatgcggcaccaatgctatcagcagcagggtgagttcttcgtcgctccatttgttttgctgcatggcttccggccgtacaatttgccaggtagtcctgtcgggtatagcaggcggtttggaaggcgtgccttcttttttaaagtagacacccagctgatagttgatcaatgcctgcaaataggccagttccggcgccgtggcggtggtttcggcgatgggtaccgcggttattggctgtttcgcggttgttttttttggagataccttgttgttaatcttactcatatgtttgtccctcccggttgtgtagcggatttttctttagcagcgccctgttgtaccacatgtgtaagttcatgtgccagcaggtgtttgccgttactggtgtcaggattatattttcctgcattgaaaaaaacatcattcctgtgggtaaatgcctgcgcgcccagttctttgctcatttgtatggcggaggtgcccgtatgaatatttacgtggctgaaatctaccccgaatttatgctgcatttcgtgtgttgtttgccggctcatgggattgcctttaccggcagcactttcaatctgcgcagagagctgcggtgtggcggaactgctgccactaccgcctccggtagcttcggatttttgcacctggccttcttcctcgtgttcacaggcagcacatttgcgttgcagttcgggcttggtttgaatatctttatcgcggcgcatgcgggcatcgttggtgcccagcttttcttctgcttcggaagtagccagccgctgtactgagctgatatcttttttctgtactaccgggccggcgccgctgccaccgctcaccaccttatctgctaccgaatcggcttcccgctcaaatgcgtctccgggtgtgttgacggataattttgtctggaagaaagtactttctttcttctgttgcacgccgctgaaaaagggttctttcgcggaagcggcggcgggtaaagactgtttactatcaaacataaccaactattttattctgcttagaaaatcttctcccagcctgcgataatcttttgcgccatgcgacacgggatcaaagctgaaaatatccattcctgcttcctgtgctttggccagctgtatattggaacggatataggtatccattactttgccgttgtactctgtttccagttgtttcaacacctgccggttcatggatttccggtcgtcgtacttggttaaaacaataccgagcacttcaaggttggtgttcagcttcttttttatattctcaaaatgatacataaaactgcgaacgcctttcagcggaagaaattctgcctgtagtggcaacagtacgtaatcgctggctaccagcgcatttacggtaagcatgccaatggcgggcgggcagtcgatcaggataaaatcaaactgtggcagcaacggtttcagcatccagctgaatacctgttcacgtccgtacatacccaccagttccagttctgcacctgccaggtccagcgacgagggtatgagcatcagtccgcaggacgatgtgagtatcacctgcgacaacaatgcctcttcacctgcgatctcttttttcagtgcggtgtacaggtgctggggcgggtcttctgcatatcctagtgcctgcgtgagattcgcctggggatcggcatccacgagcagcacctttttacctgcctgctgcaaggcggcagccaggttaatagcggtggtggttttgccggagcctcctttctgaatagccaacgatattaccgtcataagaaatcagttaatcataatgttccgttgaaaaaatactttgctttttcccatacgatcctgcctactttttgcccgagatattgcccttcctggttgctgcgcggaaaatggattccaccgtataaccgcgacagtccagcttgcgcggctgcttccgaaaatgtattccagcttaatgaaatatcgcgtgaaggcgtataaccgggttctatcagcgaaccacctttgctgcataatacggtggcgcccagtttatcgccaccggtaaactgcgccatgatataggccgcggcgctgctaaaggtgctatgaccggaaacatattctgcaaagggcggcgtaatagcggccggtggctgaaatggcagccactcctctccttttatttccttagtaccttgccccggaccgccccaggcttttattatgcgtcctttgtatacatagcgcacggctgaaaccgggcgtacggcatcatgatgtcgtttactttcccagcaggcaatactggcatccagcattgcattgctgagggcaaaaaatagtttcaggtcctggtgattacaatgctgatcccggttagatacatactgtgcgatctggcaccaatgacctggcggcgttacggtgccgggaccatcccaccaatattccgcgattactttttgcaggtcggtgaggccggcactgatcgctatcacctggtctacctgctgctgaaactcggtactaccgggcaggtaaggcaccggcggacgaaactgtgccgcgtgctgcaacgcaaaaggatgcaccagcgaccaatgtgacgtgaggaactgttgtgatttaaaatgaccattgccgtccggaacaagcagtggttgccagcggcccggttccttcagctgctccggtgtgttcactggtttatatcctgtataatccgaccaggcaggcatttgcagggtgccataagcgttggcaccatctcccgcaaaggcttccagtatacaacgtcctgcgaggttaccaatgcccgctgcattggaaatatccagcgtggtgatggcggggtcatagtcgaggtgcagcatcatatcatgaaacatgtttttattttccgcgggtaaaatcagccggaatagttccgtgagcacgcggaaagcggcgtagctgtatgctttgcgtttataggcagctttgtgttcttctttgggccgtttaatataagcgccggtggcggtactgatggcacaggggttgtaggccgtccacgcattgtacatggcggtgtgtaccatagccagtgcgcgtgcggccaatgatggtggaagtgacgagcagcggatcgcttccactgccagttggttccattgcactacgagtgttgtcggggttgacatatcatcttttcattttataataatgtagtaattctgacgactgcaccgtgcataaaaaacgccagcaaccggttgttgtctgctgccacggagaagatagcgcccggggcttctacctgctgctgttcatggggtgcggcggtattgataagaaacgttttaccttcaaaatccaccgctatgatgtatttgccgtccggtgtgatggtggcatcattccagtttcctttccagtggtttatttcttttcctgccgtagtatcccaaaggccgatgtgattgtattgtaacagcagcagttgtttttcatctgctgtcatttcaattctcacggcgggcaattgttccgggatgatggtggctttaaaagttgccttatcgaacacgcggaactgcggcgtgcctgccagtatccatttatcgctgatatacaacgctgccaccggcaggttgctgtcttcccaaagagtttgcagcaggtggccttccttgtccagcaacagcacctttgcgggtggcgggcctggtatgcctatccattgtactgatacagccacggcactgccatcgggcgcccaggcaaacacgcttggcgtatattcgttgccgtgagacacctgatattgtccgcctgccgttctgatagcttcctgcatgcccgggatttcgtgccgtacgttggccgccaggtcgaggacaccggcgccccaatacagctgatcgccgatgagcgttggaaagcccggctgtggcgtatccgtatgatgttgcagcaacggcttgtcttctttccataccgttacctggtgcagggaggcagctatcgaatagttgtctttgagcaccagtttgttgccaccgttacctgtcaatgttttccagttcttcatctttctttttatcattttgtttccgggagatgtgcaactgctgcactacttcctataacaacatttattcacggggtgtttgtattggtttattgctatggtggtgtaatctgcgttttatccacataccccagtttgccgttgaaatcaaatgcagcccatgcaccggtgaagccggctacctgtaaaagatcacccggctttacccagccaatacctttgtgttttggaccgggacctctgaacacggggagttttttcagtgccgttactgttgcgatatatgctttctgatcaatgagtaagttattaaatccacgtccggggatgcgtgcattggccagtggccggtcgtcgcccggcttatcggatcttggcgccaggcgacccagtggcccgagaatttcatccggctggcggccggccagttctgctgtaacgagtgccgacagcttgggaccggttgctgtatttgaaatctcatttctgaagaatgcttttacaaaggcatttgccggttcgttgtgcagccatgccagtgcaagcctgatccttccggacgtgtgcggagctgccggagcaaacagtgtagcatctgacggtttaataattgctacgtcgagatgtacttccatatgccgcacaaaatcggatggtacgccttccaggaaagttacgaatgctcctgctcttgcaggatcaaagttgagccatgcctgttccatcaaaaatctgccaatccgtttctccgtatctgctgccgccatcattgacggcgttttgagcatttcgtcgtagatctctgccgcaaatgcaaggcggtcgttgatccagcctttgaagtgcgcaactgatataccatattttgttccgaaaccggcaaggaacgggaactgcgctacctgggcaagttccagcaatttggcgaggcttaccgggttggggcccagtcccttcaatgctacctttacaaaggctactacgcattcatcccaccatgatgtagtggctattcccattctgttattcaacagcacggtggctgttgcagcatttgcagccgctacttccactgccgccctcatgacaccttccggctcacggcctacagccaggtaagctgcagcggtaccaaaagcctgcggatcaaaaggataatcgatatgaagatcattgctgacaggatctctcaaggtggttgctgagagtcctacggatgcacgggctccttccacctgcaccggttttccaagggctgccgccctttgctgtgtatactccacaacatttggattagcggctaaatacggcgctacattggccgcggcggtgcctgtaggaaccgggtgtgccccaacaagacaacccgcaaatacgatgcgggcagtggcaggatcaagattattgatcagcacatccagcagcgcctttgtttttaacttttccagaggtttgctgatatcaagactttcagagttgtagtcaacacggcctttcacaacgtttggtaaacttgtacccgccagttcaagactatgcggcgaaccatgccctgcgatgatcacctgtgcaatctgagagcccttgccgtatgtagcagcaattttaggtacctctttaataatatcagcgatcgaattttgaccttccagcatcagcaccaggttcggtgagttgatgatcacgtcttcaaatttcggcgccgcatcctggaatgcgctggcatcgataccggtgtgaatgatgaggtgcaacggaaataacttcagcctgttgccgtaattagccaccagtttattgagcgccaatgtgctgaagcgatgcaggttccgtattcggcctttcaggtcggaataaacggatggcgaaagagctgtgaacatattgatcatcttctggaattccgctcccctggcacctgcgccgggagaataccctctttgcaggtgaggctgaaagtctttccagtaatctttcaggttcgtcagtaaaacgggtcttgcctccacatctatcaattgcagttcagacactgtttcgtgcagcactttgccgccaatcagtttttccagttccagcatggttttgcccaatgccattcgccgcgctaccggtggcgtagtgtttagtattattaccgtgtcgccctggttacagccgttaccaaaggcgcccagctttgtccattcatccggcgtcagcggaatcaggtcctttagcttcagatccgaggcgccagccagtatatgaggcccctcgtctattttagcgatcatcttccacaatgctttccggtcggcttctattagtgtactctcggcaaaccaatcggcccggcggcgtatgtagctgttgaattcatccagcgacatacccgtgttggcggctgtaccgtcaccgagaagttccactttattcgccagtttaaatttggaatacgcataggccaaaggcgcgcgggaaatcatctgcgccggactttgctgcactatatgggtcagctcatgcgccagcaggtgttttccttcagcgctgtcgttatgctgattggcgccaaaataaatatccgttccatgtgtaaaggcttttgcctgcaattgccggctcatatccgcagcgcctgcatcttcatgaatacgcacgccgctgaggtctgtaccaaaggcgcggctcatttcttcattacggcgcgatggcagcggcgctccgttacctttactttgcgacagctgttgttctaccgctggtgttacatccggtgttgcattagcagtagcttcgcgttgcagggtgccgtcttcttctccatgctgctctttccgctgaaagaaaggatctttcacgggggtggggccaaagaaagggccttcccgctgctgcggtgcagaggattttagtccgggtggttgtatctgtgtatttgctgctgccacttataaaaacttttattcaatcgtttcattgggtttgcatacgttttccctggcggaaaactgttctgatcttcttacatatctgcaggtaggaccggcataaatagcttccaggttcattcccggcgccatgcccggctgccagtcacttaccacagaaataggcgccatcccgcttacagacttctgtttaatattcacgtcttccgatccggccacactccagaaggcgtggtttaatggaatgaaagcccccatctccctaacaccaagtattacggtaaaatccatcagccagaaataattggtgagatgaaaaggacccgtttttgagtcggggtaatgcagtgggaacgctgcgcccggccggtccctgatggctacttttccctgagtggtgccggggccggagttaaacatactgaggccatcaatggcaaaatgactggtagcattttccagatccttacagggcaacaggttacagttgccataatccagcaacaatgtgcggcctgcattatcgctgtactgcgccatgagcgtatctcttgtgagcacctgcgaaaagccgacgccggtacctcccagcgaagtaagtgtgatatctgccgatgccttcatggaaaaatggttccgggcaaaaaagttatccttttcgttaaaggtgggcttaggtgtaggcactccctgctgaccaatgaacaggttttgtacctgcacatctacccagggtggtaatttattgactacgggggtggagcggaacagaaagagttctactctcctgttgcgggcctggttttccggcgatgtttccggcgccatactccttggagtggatgtattatctatcacgatccggctgtcgggaatttttttagcgatgagaaagtcccggatgatgccagcccgttctgccgccagggctttgttactgtctacattgccggaggtgctggcagctccctgcagttttactttcagtgcgccgtcttttttcaatatctctacccagcgatcggctacttcgtttagccgttcacggtgggcggcgcgcatagctgcttctcccacacaataattccagaaaataagctcattactttctgatttgccggcggatgtgtcttctacgccaaatacctgtcccgggttatcattggcccatttggattcaggtgtgctgctggctttacacgcatccgccacggctgcagcgggcgcagtgtctttggcttttgcatccgccggttgtaattgcagtgtattatctccaggtttactaaaaaaagattccccgttttcagctttgctgaaaaaaggtttatcattttctgcctgtttgtttttaacgtttttcggagattttttcatgcaattactatttaagtcgtcttcatcagggtgttgtacacgggtatccgtaaggtgcgggattcagcgaagtgcgttgtcttacgggttcccatacgtaatcaaatgaaggtgttgtaaatggtacgttacaggtggcggggcaatttggtttgttgccaccggacgccacgcctgatggcccgccgttataagtagcgcttgcccaggcgataggatccatcggattttcatgatcgtatagcttataggcggtgatcagcgccaccatagaagcataagagaaggcgccgctcagcaggccgaatggcggcggtaaaaatccgataggagaaataaagccgttgcacaaccgcatcatgatgccgtaggtaccgtaatttacggtaccggatttccagcagctgctgcctgtttgcacggtgttggaacatacgtcgtctgcttcatgcagcggatcacggctccagcagggatccccggctgatcccggcacaccgcatggcggatgataaggtccttgctgtgtccaaccggcagtattcaggaataagccgaacgtatcaaatgcgtctttattaagttgcggtccgccgctgcccataatcacaggctgtaccagataacggcaggcattcaatttatccgtgaatccccagctgttgaaattactttgtacctgcgcccatacccgtgctatttctgaagtaacattgggaccgcactttctttcaggaacaacgggaggcgttggacctggcggtggcggcggtggtacgggcactaccgaactgataacggctaccctgttggccaccggatcggtacgggagaagtgattggtttcaccatgtgcaaaaatggaaataaacccggcgccaataccggggctgccatcagttggagtaatcatctcgtcccttactgcctgggcacggtggcacgacagcccccagttgaacgcatcagtgccatccacactggcaaagccatctatccgtacggtagcactggccccgaggcgatgccagttggccgcaaatccgctgatcagccgctggttagcaggcgataaaccggaagaagataccgtgaacggatagctgtcttccacccttggtgcactggtatctacgggacaggccaatcctgcaggcacctgcgacaggtccccgtgttctttcacgggagctacctgccgtgctatgcctgttgttccctgtccttgttgtaaagtatgtgtaagctcatgcgccagcaggtgcttaccggtgctgctgcccggagcatattttccttcgttaaaataaatatcattgccggtggtaaatgcctgtgcattcaattggcggttaagtcccgctgcgttgctgccagtatggatttttacgctgctgaaatcagccccgaaagcgccgttcatttcctgcagggtatctcctttcaatccttctccctgtcctttggtactgttgatattactttctactgttgttggggagatggcggccggagaagtttccttccgctgcacgttgttcttcttttcttcttcttcgcagtgagcacatttacgctgaataaccggctggaaaaacggttgcgccgcgggctttccccagaaaggggttactgccggctgtttaaggccggaggcgggggctcgttgtatatttgcgggtgataatgtttttgtactcatgcggatgttgtctttcccaggattacgctgattatattgattagcttgattttatcttttggatttttattgatttaagaagcttatcgccattgtacgtgtagtggtattttcatccattttagttttatgatgctgatgttccagggcaggcgatccaaaaggatgtcgatggtgtctgattccatttgtaactgatgcttatctgtgccggtgatcaatcttccggggcgttgcaggaacccttcccgtagcccgtctgcagaaatactttttaatgccttccagtggctgatgacattttccatcagtccgtcggcttcttccatggcttctgttgttggggccagcttggtatccagtggccttttcagcggccagccacataataattttggcaacaccacttcaaattcatcggcttcggtttgcccggttgccatgtagtgtaacagcatagtggcctgctgcttgcaggcggcgttgaggaactgtttaccatccgtccattccaactgacggaacaatggctgcaaccagtgatgcaacaggatgatccccgcatttaccacgtaaaaagttttggcgccgatagtagtcgctgatatttcttcttcaggcatatcagtttccggtttggataatggttcgttggttaatggtacagcgaccggttcttttggcagcgctgccgcttgttgtatgttgacggaggtagccgcggctaatactttatcccagccattattgcggcataccgttatcagttcctgtagctgcgtaacaaataccggctgttggattaacagctgattcatttgtgcagattcacttaccgttgggtcctgtgccgccagtaataacaatgaatgccagcatgcctgttcgaaggcacggcggttcattccatcgctgtgcgcgagttgtaacaggcggtaggcatcataaagctggtgcattacgggcggccagctcgtttgttttctggcggtgatgatggccagcagctgcgtaataaattccggtgaatgctgcatcaggatgcgcgggagataatcccggttgttcaacaattgctggcgcagcgaggtaattgcctggtgactggtagccagcacctgtaatacctgctggtaccatatctcatcgggccgtgacgcattccagggaagcgtgccatgttccatgtagtagcaccactgatcaaaagcgtgttccggcaaggatttacgcggtgtttcttttacatggagcgtggctagtgcagcggtcattttctccagcagcagggccacgtaatgatcattattaagatcggccgccttgatttttccgaggtcaatttcaaggcgatctatataaataaccgtgtcgccgctgctatagctatcgaacagcttttccagtgcaggaatgatcttgttccaatacagcgctgttacctggtgttgccaggtaaaaacagtgtctttgttatgcactgtcagcaggaatgtttgtttacggatcttatgcaacatgattatttatttcatccatcgcaggcattgtgctacgaggtcttcattttcatcagagaccaggtcttccggtttccagtcttttgccagcgccgccaggttgattcctttgtctttcattttgcgcagtgtttgctgcagctgtttcttttcgtgggcggcaatgcttaccggcacacgcagcagcagctgatccaggcaaagccaggtggcgttgcgcagcagcaatgcctgttcacttgcagcggcttttttcccggcaggcatattttttagtaagaagtcggccagcgtactgtacttatgcatattcagcgggcctgcttccataaatttgccggtgcggtcgtatgcttccgtgtctacaatattatcggcatccaccggcaggatctgttgtttgtattttgaaatacgctgacggcctttccggtcgcgtagcagcacatcttccggggaattgcttctgtgcgtggcagcagccggcgacgcagggtcttccaccagttgaggcgacgttggcgctgctaactgcggcgatgttgttgccggcgcgctaccccgtttgtttgccaggatgcgtccgggtggcggcgtggtttcattggaaagacaatcaatctcctgcatgtcgcagtttttacggaacaggcgattgatccagacgccgaagtcagattcaggtagcttattttgcctgttatcatcaaagcaggatggggtgatctgctggcaatcgggatctgtttcagtatcaggcaccgcatccatgatgccggtttgcccgaagaggtaacagataaggcagcattggatatgcgcgtcatcaccacaaacaggtttgcaggcaaggtgctgcaaccagcggcggtaaagggtttcaaactcgcagaagctgcgtggccgcagccataatatattcagcagcacatgcgcgggcgcttctttccggagcaggttttccatcatcgcacgggtgctggtattgcggaaacgcacgggccatccgggcaacacaatggtggctacaaaagaatagggatctgtaaaaggaactacggtcgttttaaataccgcatcttccggatccacatcatagcctaccacttcttcttcccagggcagcctgcaaagcggttcaggcttcaccggcaataaacactggcaatcatcttctacgcgtggccggagcaggatgtgttccaccacatgcatgccttcgtcattaatggccgcagccgtgcggtcaatggcatcctccatcgcaggcagtgtggcataacactgcgggttggcggcgagcacataactgctgtctaccagttcaataccgaacgggccgcaaccttctcccagagagggtttgtaattaccggggatcgacaatgcggcacagaaccggtaaaatccacggatagccgcattcaggcactcatatagttctgcgctttcccagatgatggcgccgggtttacgcaccggtggcggcgcatcacaggcgcatccgttgttttcatccggcaggggctcttcggggatgaaatcatcgtggtacaaacggaaagaataagtaaagccgaaggccgtttttacacgacgtaccgggtaataaagcgcgctttgctgcatttttgctttccattctttcaggtcatccgccgacagcacagcgtcgcctgatggtttgaaatagccgctcacggcgctgccgttcaacagctcaaaccggttggcagtggtgttcagggaatagttgccgtctttccacaataacgataatacttcaaacagccaatcgtcctgtgccctttcagcattgacagccgacgtatattgctgcccggatattaagatcacttctccgcctgccatcaactgtagttggaaatagttaccggcgtaataaggttttacttccaacgatacctggcagtttttaccgagtttcaacccgatcatttgtaattgctccaggtattttgccctgatttcttctgtgttgtattcatagggatgtactgccagccggtagcctttcttcacggcgttaaaactatagcagccatcatcttttacatatccataatacgcgctgttgccatggcgggtagcatcgagcaatagttccagcccggtgtacacgtaatctccattggcgtttttcgtagcgctgccccaggcatcttccaaagaattatactgttgtacactttccagcagcacttcattcatgaccacctggtagcggcaactggtttcattgagccgtacgccgctgttaccggcgtaccgggccaatgccaggaataatttcagcgcttcgctggcggcggccatatctgcaaagccattgcagagtttccagatcttttcccttttggtaatatcgtacaggcttacccgtagttgctgcacattgctcagccaatgataagggaagcttcgcatgatatgcggtacaacgtccagcagcggcccttttccgccgaattgtgcaatcgtatctgtgggcacaatagccaatggaattgtatccgttaccgggtctccttccaggataatgctggtaccccaggctgcggggttgcctgccagatgtaccagttgcaggtattgctgccggaaggcggttaatgcttccgcagcagatttgtaagccttgtaactgcgaaagtattccgtttctgtttttggatagatgggtgaatgatagttcttttcaatgccgcggatcacataatagtagttaactgcctgtgtttgcggatttttcacgcaggtaaccacttcttctccccccatacatatttccaggtaatcgattccctgctggttgcggctgcgcgaggcggccaggcggtcggttgccggggctttggcagcaaaggttttagggaacctggcaaagcaaccggttttattgattacgcggtatacaaaggcgccttccgcgctggctgttgtactatgaatataggaatcgatatcggccggggcggcgccggttctcagctgcgcgagtgacaaagcatgctgcagtttaccggctgctgttgccgtgggcaggatgatcttcttattcaggccggcatgcagtaaaacgggtttggcgcccttttctgctttcagttccagctggtccagcgatgcagtgaaagtatccatctctgtttttgccagctcttctgtggcatattcttcttcgctgttgaacaggtacggctttccttccatgccctgcaactgcactttgtatttccatgcagcgggctgcctggaataagatacctggtataactgcgcctgtataagctgttgtatatgcaatacggtattatctgcctgcagctcttcatcaaataaggccgggtgcatggcttttacgttgctgcgttctaccaacactacttcatacctgccatcggtggtttgccgcaccaggtaacctgcgggagtggccgccagttgcaggagcaggtgaaattcttcggttgcctgctgttcatttttcaccgccgatgccgaagtaaacataataaacgcatcttcttcgatgctgatctgcacttgtaattttccgcctttctgctggatattatctgcctggaaggcagcaagattgataaaggtagtgtgggtggcatttacgggtaacaactgcaatgccggcaaatcttctgttggtggaatgctccagtcgtcttcctgtactgctgccagtaaatcgtcggtagctgcaatggccttctgctgatcggggaatgcctggtttgaatgtagcagcggtttcccgtcggggctggtcacttcaataaaatgatcataccggctgatttccacggtaccattcagtggctgttgcgtaaaatgttcctgtaactgtaacaggcgtgcctcccgctcttccggcgttgtggccggagatgccaggtatgcgttgcctgccagcaaaggcacctgcaagccaaattttccctgcacgggatcatctgtccggataagaagttccgggtgttttaattgttgcgcaagatgcaccaatgcagcagatgcatcttcctttgtaacgtagttacttgttctgaacaacacctggctatctgcatcttttatttctgcataaaaaaaagtttcataaggtcctacaataaaggggcacaggtaatgacggtcacttttttctatgccagctaatgcacttacccgttgttcgtagccggaagtattggccgtattccatttattaacgcggtagtcgtaagccttaccgcggttcctgcttaatttatcataggaagaaagaaattttgctttggcgcgcaaacccttctctgcagccttctgccggtcgctgatgccatataacaccaatgcataatcggtaaaagtttctgcgaagcggctgagcaggtgattgagcatggtttcgcggcgctgctgatacagggctttgtcttccacaatcttttgcaggtagccctggtagtcggcgaggctgaataccacgtcgaaggcgtactgctctttgttagccgcatttttaaatccgaacgaccggagattttccgggtatgctgccaggaagatggcggattgcgcagcttcctttgctttttgccgggagggataatagcggcagccgagcaatacatattcccttccgggagtggctatcacaaagcaccagcacccatcgccataaagataagtggtaatgttagtggtattatcctggtggctcatatccagcagcagctgttccaccgcggtattccgtgcagaaagataatcgaagctgtagtatttgttacgccagcgctggatcacatctttcttaacggtaacgcctgtatgcagttcattgagcagttcttttccaaccggcagcatgagcgtatcatgctgtttccagcccaggtcagcataaaagccgccctgctgaaaacgcaggagtttgtcgaggtccggaacgtcggtaacagcgccgctgaaatacgtttgtgccggcgcatccggcgacatagagaacaggtcgcgcaggtgttgcagttgcgccaggtaattagataacagctgatcaaagaacagcaggaagcctttcagctgccatgcctgcactttgcgctgcggcgacgcatcgttacccaactccccgttgccaatgccgtatacccgtggaaaatcacgttgcagggaatagtagttgcccaggtcttcccggtaaaaaccagaaggcaccgcatgatcaagatatgcggatgactggtcgtaccacactttggtgccgttgagcagggaagcgtttaaatattgctgcaggttggtgccatcaaaagtaaaggtggcgctgccgcgtttaaacacaaagcggctgtataccagcgacagcagcggcaggtggccatccagcaaaggcagtatccaggcggtgccgtttgtgctggcaacgggcgtatggtcgcctgtaacatagccggctatactaagaccggaaatggtggatactcccggcacttcgaacattacgtgatatacatctgatacgcggatttcgcggaggggtttgatcgcttccagttcggcggtgtcaatgaaaccatggctcccggctgaataggcccttcccgcaaaaatttcttccatcgttaccttcttttcttccagcatctgttgcagggtataaaaagtaacgcggggagaaaaaaggtgataaagctgaagtaccagttcgttgagcacagtggttacatctgcattttcctcgagctggatttctgtgcatacgccaatttcttcatggcacagaatggtgatcttataaaagtcttcacacaaattgcggtgcgccattaatgccttgcgaatgcgttctttcaggtcggccagcgcttttgctctttcctggctgtcgtccggcagcgtttccggttcaatgaaaatattataaagcccattcagttccagcagggaaatatcttcattggtagccgccagctgcgggttgcggctgcggcactccaggccttcatcgccaaaccagtgtacttccggcggaatgttggcagcaatttccagccatgcgttccttacgccatcgatatcggtaagcagtttgcggtagtcggtaatggtgagcgggttaaccgtgagaatctttgccggtgtaaagaaattatcttctttcccggttcccgcagggttcatggtgagcaggtcttccaacggcaaactggtacggtagcccatatccagcagggagtagcacaacacttccaggatggtgatgccaggatcgtgcgcgttgtggtcggtccatattttgccggagagttttcccaggtagtcgatgccttcactccgcaacttttcgaaatccagttccggtggaaaagcaggatcatttttaatgatcacgttcttggtatttgtgtcctcagccataacgatgtagttaattaatgatagggtcctgcggcgttgacggcggttcctgccgtgtattattacatggcgggatcaggggttccggaatattacagtctgtttcccgttcagggatgcgtgttaccacatcggggcaaaccactgcgttcttttgtgtactcacggtaatgttaccgcttaccaggatggaacgcggcgtatgcggttccatatgctgcgatggcgctgtttccagctcatgctgcatggtaaggcactctacatagtccacataatccagttgctccacaaaccgtacaacgtctgcctggtgcacgatttgtccgaacgacagtttatccagttttcctatcgcccagggggcgaaaaattcctgcaggtctgttttcagtttttcggtataatatttttcatctttccctttatataattgaatggagatgtcgaccatcactctttcatatcttggattggtgactttcagccgtacaaaaggagatgaacgttgtttgaggaaggtgtgaatcttttccagcaggcttaacggcgctttgggttccatgagattgcctgctgccagctggcgcagatccggaattaccgccactaccacataaccgccggcggctaccaggtcttgctggtacactttggcgccgaggcccagcgtatggtttacgcatttcactttatacagctgcggaaactcttcgagtaccagtctttcataatcaaacgactggatagcgcgtcctttgtgccgcagctgttcgctcacgcgtacatagaaatgccctgcggcttccggtaaccgtccgttgaaagcgtcatacagctgggtcacggttttgatatgtgcatctgcttccgccagtttggtaatgctgccggcttttaatacatctcccaggcgcatcggatcattttccggcagcacggtgaatgtggccagtgcggcctgtgtatgcacgccaatggtttcacacacagcggccacgttttcggggatggcggctttcagccagtaggtaccggcgggcataacggtattgactatattaatatcgccgggcacggctattttaatgatgccggagcgggttaatccgtcggtatcgtcattgagcacttcaaatcctttgcgaagcggcttccagacattgctgcacaggtaaaaccattccacttccgctttctttgactccgagtcggccgtagcttctgccagctggaacaggaggttcagattgccgtatggctgcaaacggtcaagccctacaaacaaagtgccttcgtcgcagaataccggtaacagcgagggttccaggtccagcacttcttccttaaaagtattttcaaaaggatacaggtgcagcagctgcacatcttcctttatagcagtagcgctatagtcgatagagatctggctgatcaccggcgtccagggttcattggggatgatggccgacagggtgttggtgtctaccacggatacctggatatcctccaatttttccttgatatcttttgccagctcggtgagtccttcaaatccctggaaaaaaccgccgcgtgtggggaagtccggtggattggggcctcttgaaatgtagcggatcgttaatgcttccgccggggtgggcgtccatgcccagggcggcgacatgctgtcggatggaatcctgccatcgaggccactgggcccctggatatatttgttaagatttaaggcatctgcataagtatcctgtaccagttgttttaattcttttaaattgaacactaccggggaccctactgaattgtagtaagcggcggtatcaatcctgttcttaggatctttcggatcgtccagcaggcggttaaacgccgtcatttgacgggcgagtacgaacgcataatccttatgcatgaagtcctggcgggcgagggttattttggcgaagtaattacgggtatcggcattgtaccgggctaccttttcgctggtaagactgaactgatccttgaaccctaaagctgttggctgatcgaatgcaatggaataatcgtatatcttctgcggatcgcagggaacatccacatttttagtgaacagttcttctgccgaagcattctccttaaaccattttccatcctgcaaaacatacttattaatcttgaagtcggtttccgctaacccgccctggacgtagcctgcatagtatccttcaaagctggccggtttgtctttccagttcatattcacatataccttatcccattttttcccgaagatctctgtggagccgatataaaaactggggcctttggcggtgttggaaaattcctttttacctttcagtatttcgaagtcaatcagcgcaggccgggtgccaaagggataaacaggcgagttaacatcctgcacggtttcatcattctgcacgattacatttttaaccccgcaaacatctactttaatagatacattccggatgcggaagtcgcgcagaaaatgatacaatgcaatagccgtcaccgtattctttggctggcgttccagttggcactggccgcaatcgccgcctactttctcgatcagtatatcatccaggcttagcttcacctgctgatccacctccacgcgcaataccggcaacgtggtattgtagttgccattgagcactttcttatcataaaaagtaaccgcaggcacttccggcggaagccctatctgaagtgttaatttatagccgctgccggaaggaacaattgtaatatctgcaagctttggcggtgcaatccattcttctgcaccgctgaaaaacaactgcaatacgctgcgaggtttgaacagttcttttactgccgccggtaatgtgttgatgtttgccaaaggcgcatcaggggttacgccgttgtctgttaacaccgcatgtgtgccatctgaggcatatcttacatccgtaagcgcatcccgcagtatgttgatggtagcggcatccacacccatttcttctgctttcgcaatgaggtcgtccgacaggtagatgtatttatttttcaggattattttcaatgcatcgaagtaatcggtatcctgcagcaaaacattatcgtcgcagttttcagaaagcacgcactcaatatctaccgtgatattccgggtaccttcctgcagcaataataccggcgaagccagcataaatccgagacgggcgtaaggatgctgcaccggttgtactttgcccggcgcaataaatttactgtagcgggaaccggcggtaaaccagttctttggcatattttcctggaagggtttgtctaccccatccgccatattggctttggtggcgatatacaatccttcgatgaaatttcttttgtaacaaagctggttgccatctgccagcgttcttttgaaggcagttaccgggtttacatacagggtaagtaaactggagattgcagcattatctaccactatttcatcttcaagccggaagataacatctgttttcaggctgtcctttccatcgcgcagcgcggttcctttagaaagcaggtattgttgaaagggttgctgtacttcaaacaccacgtgcgccttatccggcgtgaggggttttggtactaattttaatacctgttgaaagaagaaatcgagatgtttttgcgtgaatccgttcagctgttgctgtacgtgtgagaagaggtacaggaatgcaaagagcagacccaggtgcggcgtatgattctttttataggcttcattcagtggttgcaggctttctgagatactgtccggcgccagtgtggcaacagcggcaatagcatccaggaatggctgaaagatggactggtaggcctgcaacagcagtagtgctttttcgcgggaggtggctgcgtaatgaaaactttcgttccattccaggtaagcgaacagcggatcgatgccccatatttcttcatttgtaatttgtgaaagatcgaggggacgaacacaaaaccacttcacggcgccgttggtgaactggataaaccgtgacagcggtgtacggagcttttgctgaataatggcttctatactacgttccattagcagcccggtaccctgaaaagctacctgccactgtgcaatgggaacgattacatcatcatataaaaaattgatcaggagttgaagcgtatcttttgcgggtcgttcatgtacctgttttacatatccttcaaaattatctttcagctggctggtatttgttttagtcagctgcgccagcaggaaagggaggctgttccggaagaaaggctgccagtcgttgatcaggtacgcgtctttatattgatagtaattgatctgcggcgccatttgtacgaaataatggagcaggtccgcgagctttctcccgtctattggtgcggaggcagcatccagggccggtagtagccggttgcgctgactgatgcctggttcatattgaaaaggatgtacgatcatgatttaactgattaattgatgaccctgcagcggaggcgcctgtcagggtttttgcgctgcttccagcaaatagaaatcatacacataattgtaccttgaattagtacttgcaatcgtatagtcgatagagatagtaaaccttccttctatcaggtcggggctatccatgggcaccacgcctatttcttctactttgatgcggggttcatagaagagaatggcattttccacgaggtctcgcaggaagccgatcatagtagcattgagcggttcaaaaatatagtcctgcaggtcgcatccgtagcggggttgcatcactctttctcccaaactggtagacagcaatatgtcgaggctttctttgatatcggcttcgttgcttaccagttccactgctccgctctgcagatcaaatgttggcgggaatttccagccggtgccgaggaatgaacggggatcattttgtaacatgtttctgaatattttttaaccgccaataatcactgtgggagctcccattacaattacgccgccatgtgctgtgaggtcgcccattcttgcggcgggccgccctcctatcatcaccgtggcagatcctttcacgatcgcatccggcgggcccacgcaggtgcagatatcgccggtaacggctgccgggataccggcaatcatcaccgtggctacgcctggtcctaccaccggaccgcccacatgaggtaccggtcccgaaaacagggggcaggtgtgaaagtcgctgatgcgtgctgcaggaggcatgagattaacaatttaagtgaccggcaatcgttgttcattttggggtttgccggttaatttatttttactaaagaacctgttatttctgtgataccctgggaagataattttgcgatcgctcctttcaattccactgcgccatctgctgctgcggaaatgctggcgcctcctatcgataaggccgcgccggccgacagcaccaggtttacgcctgctttcaactccacgttcatggggctttccagtttgataccggaagtatccatcgtgaccgtgttgctgttctggtctttcaatttgatgctggtactcgcttcatcgatcgtaatgctgtttcctgcgggggtatctatagtgattgttttcgtactgtcgttgaagtgaatacgcatgccgcttcttgtcacaaatcctttttcatcattggcgtcctgcgcggtgatgggtgccggttttgcactgctgttaagcattcccagcacaatagcgtcacggggatcatcgttgataaagcccacgatcacttcatcgtcaatttccgggcggaagaaagcgccgcggttattccctgcatcgaggctggcgactcttacccagatgccgcgggcggcgttgtctatcaccggtatctttaccaggatgcggtgttcgccgtcgggatcattctgaagctgtaccactttcccgatctggaggccgtggatagcgggcagcattcctgctgcgggaatatctgaaatatctttataagcttccgcgagccagtcgggttccagtccgaactggatatgagtgtcccagctgccgtgtgctacttcatgccgcacaccggttacaaaagcgttgccgttataccggttgccgatgccctggagcgtaaccatatcgccgggggccacgccggagaagccgaggaactttgccctgccgcggatctttgccagcctgcttttcagcatggcggcattggtgagctgctgcagttcttccgctgcacggcggccgctgtgtgccagttcatagtgttgcaacccgatcacatctgccagtgtgctgccggaaacattgccctgctctgtataatcggccgaagaggtttctgcctcgtataactgctggccggtgtagtcccaggcgctggcgtgtacggagctccattgatagcgggcatccatttctgcttccagttccatcagggaggcgccgtaggtgagctgtaatacagccgatgcagtggtatccggtttctttacctttacttttccctggtcggcgatcaccagtttgccattggcttctgcgcgaagcaggaggaagtcccagtcggtgctgtggtgctgtaccagttctttgtgctgaacagttgttgcctccacgtctgcgcttaaactgctgtatcccctgatgagctgttctatcacctcgctgtcctttactttttcatagtaccggctatgcctgccgatggccattttcacggtttcatcgcggcattccaccgtgagcacggggttgccatcctggcggaatttgatgccctgatgtacgatgacgcctttgaataatactttattggagccatcgcggccgattttgatggtgagtttggtaccgggcagcaggtcgccggtgttgctgatagcaaagtcctggtcggcggcggcgccatctcgtaacacgatctttgccatcggaattttattcaccacctgtgtaagtgtgagcgaaagtacctcgtacacgggattcagcggtgtagtaccgttcaacaggatgttgtaactcgctacatcatgtgcagaagtattgggtattcctgtttcgttcatgatacttcgcttttatcgaatggagggaaatagatctctttgccaaccggtactcttttgaaagaggtgaggttattttgccgggctacctgtaacatgtacttaggttcctggtagattttaaaactgaaaagatccagccggtcgccctgtttaaaaacgcggtggtgtgtaaggtcaggcgaagctttgctttgctccctttcattagcttcccttgcgcggtagttgagaaaggtagcgctgacttttacccggagcggacttccgtctgcattaaacaacacgtagttcaggtcgaggttggacataacgcagggaaatgcgatctgtttgccccagaacactttcaggaaacgcggccggtgtgtttccccatccatgtagtacacggtatccagcagcagctttacctgcgcctgtacatccataccgggataaccgtatccttctatggtgttggtaccgtcgagtacaaagtcgagcttcagttcttccgggatggtagaaataaaacgcgcttccgttttctggctgcctggctcacggcggatgtcatagtctaccttcagcgaccgggtataagtttccgcatttaccggaacggtaaatttgtggttgttatccagttgctgctgcaacctgtcggaatacgtgaggatgtagatcttttccacttttgcgtctgtcatcgttcatttttttctttcagtgcctgtaatactttttccacgcacaacgcgatcatggcttctgttgcatggctgccatcgcccgctgcggtagtattgctgcctgccgatccgccggaggcgttatccggcgctacttcagccttgatgatcagttcacggatttctatgggcatgactcagctgtttttaaattcaaaccggttatagttcagttccagtgtttctatcagcacttcgctgcgttctgcatgtaactctcccagcttccagctgcggggccatacccaggcgaggttccagtacatgaggatgttgtgttcctcatccagcagcgccacctttaccagttgcaaaggcttgatctgctggtcttccagcgccctgcggcaccaggccgacaaggaagaatcatccggccggagcagtccccttttcagtatcagcggcgaataggtgcgccgtacggggatgttgtgctcaaacctgttctccccgccttcctttacctgttcggtaccgatgctggcttccaggccggtgacgctctgaaagcggatatcgagatccgaaccggaatctttgccaccgctgtttttgggtaatccaaaaaaggtgacagagaaatggaagcctaccgtttgccagaagttatcgggctttatcactgcttgtgccatgttagtctacgttcatgatctccagcccttcgtgcaccagctccattgtttcaatggctacttcgttggcgtcggctttcagatcagtggaagttattttagaaggccatgcgttcagtactttccaggtgatcaccggctcatggctttcattgagcagtttgatggttacatcgcggcggtatttgctaccggctttgttgccttcctggaaatagtaggtttcgcgccaggctttgtagaagtcgtagtcgccttcaaatatgccgcgtttcaggctgatattggcatacttggtaagccctggctgtttgcttttattgtatttcttgctgttaccttcccggtattcgatcacttctgtttcaaagtcgaggccggaaacttcagtgaatccaaggcgtacgtcttttccccattctaccaggaaatgaaatttgggtaacgggtatgttccttttgcgggcatatctttaaatttaaaaagatgataaaaaattgaacagtgcttattggtcaggcgccgttatttacaggctttggcttcctgggcctgtttgatagctttggtaagactatccgtacatgcctgcaggcggtttgcttcctggcttactttatcgtattccggtttaatggccgccagccgggtatccgcattggtaagatgcttttcagtaagcgtatagtaatgatcatttttgagcgggaatacggggcataccagtttgtcggtgcagcatatttccatgctgtcatcttccccggctttgataccaccgttgcctgaattaccgttggcgggaggattaaagatgcaaccgataccagcgatggccgacttgatcccgtagtccttttcgcagatagtttcatccaggatggtagccgctttcagggcaatcacgatattattgaaaatatcattgccgatggtgatcacgtcctggagttttttgccatagtctacccaggcgtcggtgataccgccttttttcaatacctggtcgttggagcagtcgatggctttggaaatattattgtagcaggctgctacttcatccacttttgtatataactctttggtcatacagaagaagatttcgatggcggttacagagaagccggtgcttttgcagagtttctccaggatgtccagcactactttcactttgctggtgatggcgtctgctttctcggcacttttctgtacgttatcgaagtagagctttactttattgcgccagtcgagtgcgcgggccagctcttcttttttcttggcggcttcggctgctttctgctgatacaggctgccttttgctttcagttcttttttccagtcatccacacagccgcactccgtttcgttgctgccggggatggtagcgcaacaggagtcttcactttctataaaggggtcatacactttatcgcaattcatggtgaatatttttttgtgatcaggaatatttattttctgcgggatgggaatcagtcatcacagtgtcctccattgccgttgctgttgcagtaattcccctgtgcctgttcgcagatggatttgatagtgggtaaatcgccgcagggcagtgtgcaaaggaattcgcggatatcgtcgattccctgtgtctgggttctggccgaccagagtgtttcgcggatcgttactttctggatctttgcatcgcccagttcgccgtaggttttcttctgatcttcctctcctgttttgatattctgcagtacatcatcccggaaggttttgattgcatctgcgagatctttgtgcagggcgatcacgttttccaggctggtaaacgactgtatgccggaaacgtcgccgatggcgcagtgcagcttgttgatgctaacggtttcgccgtcgccgcaaccgccttcagaggcgtacatttcctgtgaaccgtctacgatgttatcgaagcaggttttgaaatccttgctgccggctttcagtttacccagtgccgcacgctgtgctttgttgcagttgtcttctgctttgttgttcagcttatgggctgcttcactcagcagggcaaacttttgcttggcatcctggatatttttggcaacaatggcgagagcggcggcaatggctttattcacgtcatttgctttgctcagtttttcttttatcaggtctgcatctttctgggcgggtaatgtggcgcacaggtcgatggagcggtaaaagcgccaggtttcttctgctttgataaagaaacactgtttgtatttgtacaccggcttattgcctttgtactcgccctcccgcatacgcaatacattcagcgaatctgagaaggcgctgcagatcccgcgtttgttgttatcgatgtattgctgggttttattggtggagtcaccgcagccattgctggccgttgatgtcgtggggttcattgtgttcatacagtattcagtttatttggtctgaatgtaaaaggattaagattcctgcagcattttgtggctgaagcgcaggatgatgaattctgcagggcgtaccactgccattcctatctcaacgatcatacgtccttcccatacatccagctctgtcatggtttcaccaagtccaacctttacaaaataggcttccctggtggtggtgcccattaatgcgccggccttccattgctgtgtgaggtagttttctatcatagatttcacgcgtacccaggtgttcaggtcgtttggttcaaacacaaactgctgggtggcatttttcacagattcttctaccatgttaaagaagcggcggacggagatgtagcgccattcgttgtcgttacctgccagcgtgcgggcgccccagatgatcgcaggaccacggccggggaagaaccggatcacgttaacggatttaccgtcgcgtacatccacgttcaggtcgtcctgttcgcgtttcgtaacaatcacttcagggcttacggcgtaatcaatgccgatgttggcgggggctttccatacgccgcggctgttgtctgtttcagcgtatttacctactactgcagcagatgatggcagcagcattcttatctgtgtaatggcatttaatgcctggtagtaataagcattgttgatgcctttcaatgccgcgagggtaccgttgagagagccatcgccgccggtttgcaccacctgtaccgtagcttcgtcgtatgcgtaggacagctgggtattcacgcgcggaaaataaacggcgccatattttttggtttctatctcaccaaaaccggcgtccctgaacagggtaacgttatgatcgatgatgctctcagcagggcctatggcggggtccatccatatatcaaaaacggtgaagcggtctttcagcaggctgcactgatccaatgccgacttatgcagcgtgtaataggaagccgcatctgtgaggttgatggcatcggggaagaggatgagcgttacttcatcaatcttttccacggcattcagtccgtcggtgagcgtggtaagggaaatcacgccaccggtgctgtaatcgcctgtggaaacgatgtagcaagggccgccgccgttgttgaaaaacatctgcagctggtaagccatcaggtatttggatgcttttaacggatctatcactgctttgatcactgcctgtggctgagagctgtcgatgttcaccgtaatactttcttcttcctgctgcgggccaccgaagatacggttgtagtcgagcatggaagtgatacgtgtaggaaccatcaccagatcgcctggcactttgttctgagcagattccgtatagccgatgaaagccggaatagctgtttcaacagaggctatggagggggggaattttacgatctcctcgatgtagacgccgggagttttatattctgccatatgtttggggttttaactgtttttaattgttgtttgaatagatcatacgctgaacttaaggcccttgcggaaatatttttgagagcagcactaccacatccgcgtacagccgctgatcggcatcactggtgatggaaagtccccttggattgggtaacagttgttcgtagttagtaatattgttttctgtaacggggaacaaccggttattgaatgaaaacggccagggctccttggtggtgcgtgcgccgttgtcgtctgctacggagagcagtgtgttggcatggttactgaacaccagcgtttgcccgtattggggggaatagcgccaataggaattcctgcttttaaagcgcaattcgtaaatcgtatggggaatttttgtaccgttctgttgcagttttgttttgagggtaccatcggcgtccagcatggcaaagtcgccaccggtggtatttacgagaagatccaccaccccgatattgcctgccctgtacaggtcatttctactcacatataccaggtgctgcgcggcgaagttattgctgccggttactttgagattataccagccatcagggagcagggttttatccggcagcagcccggagaaatcgagtttcacctgtgataaaatactggtggaagtaaaggattgctgcaaagaaggattacctgtaatgctctccagcacggcggttccggcggtcacgggtgcggcgggcggaaagaaatactggaaggagaaaggcaataacagccggtcgccttcatgtacaaatccgctgcctttaattttgcgccattgcgaaggatcattgacgggtgtacccggtttgttgagatactcggatatatcggcgcctaccctggcgagttctccctgttcatattgccgggtattatcatttaccggaaccggaacagagagcgatggaaatgttttagtgttatcggtgttatcgttggagaaatagtattgcgccggcagcgcacggcgcatccgcatgctggtaaaggccagtgcgcctgcactccggggcaccaacgcaaaccggaaggccgtatccggggggattggcacaaagggcgtgtatgcgagtgtggttccctgcatcaccttcttcacttctatggctcctttgaaacctgtagcagtaggcagtaaccggaggtgatagtttttcatcagtacggcggtagccggcaggggctgaatgtcccagtcgcgcagtaaccggtactggtcctgccgcagcttttccatcaggaaatctgcacgttgctgatcggtggcctgctcaaaaaaggaaattcctttactgttttgcagatagtattcgtgcagcaactgcacttcaaacaatatcttgtaaataacagacataaaactttaagaagtagggtgttgtgtgtcttctatttcctctatcagcggtactactctgagtacagcattttccgtgatagcaacgagtcttaccttatacatcacaaaggggacctggcgtccgccgagcgatgcccagagatggttaatctgttcgaatgttagtgtgtacaattccagggtgaggtccagcgagccatcagcattcttgaaagtcttctgtgcctggaaaaaactgattactgccgacaaccggtgcagtgcttcttcgtagtagtcgtgcgtggcgtctccaaaaagcacggcggtgaacagcacgtacaggttgaggtacaccggcgggtgctggtaccgggcgcggttatccggccatgtggtatacgccttgctgtttttaagggtactctcctcttctacatttacaagggagataataacgttaccattgaagttattggcatgcgttgtttccagcaaaccaatgttttcaacgatcacactattggcagggaatcctctgagcgcaaagaatgcctgcaaatgatcacgtatcaatgtaagcgcgttacttatcacgaatgacgaggggatttggggttcagtaaatttggggtttcaattacctgtctcttctatgtctttcaaaacgttcttgttaactaagttaaagaacattttttaattgggaaataaatatttttttaagatgtaattttcacgcaactgtattttgcggcaacacaccacagaacacaataccagcaagcatcttcaatcatctccctaaattattcttttttaaaatatccccctgcgggaaatacgcttccaggttgccggtaaactacatttaccattcatattaaacaagccaccacaaagcattacaggaaaattattccggcacttcaacttcagttaagttatgattcctatctaccataccctacgtataaatacgtaattttcacataacacaaattccggcctcaaaaaaaggcaggtgcttatacatattcctgtttcatttacctttatttctgattacaaccggtaataagttcccggaaagatacttgcggtagcttcggatacaaagtgttttataaatcttaattaaaatgaataccgatatactttatacacatatctgctcctatgtcaaaatatccagggaggagtatgaacactttctccagctgtttaaaccggttcatttaaaaaagggtgagctccattatgttgcaggtaaagttcctaagtattggtcatttattttaaaaggctgcctgcgtgaatacctggttgatacctggggcaatgagcagatctttcaattttatgaggaaaacacctgggtgggccaggtggaaagcatgattacgcggaagccgacggaaatgagcctgcaggcgctggaggattgcgagttattgtgtataacaggcgaagatatgtgtgaggcggtaaaaacgccctggatccagcactacaccattcagaaaagttttgctgataatgcagctttaatatcggaaaatttcaaccggatcaaatccacatcacctgaagtgttgtatttagaaatacttaaagaaagaccctccctattactgcgtgtcccccagcattacattgctaattttcttagcatgcggaaagaaacgctgagcagggttagaaaaagagtgtcccgcttatgatttgttgattcaagtcaacaagatccgatttcccttccggtaattttacagcgaaaaacaatcacaatgataatctcgatgtttctacgcttttagcacggcatcaggacaactgtgatttgtgcattcttttaagaacaatattaaatctatgaaaaagataatttacgatcaatacggtagtgttgatgttttacattccgtggaagtaaataagccggtacccggtaaggaacaaatactggttaaagtaaaggctgttggtattaatccgctcgactggaagatcattatgggtgaagttaaagtggtgaccgggaaaaagttcccgaagtctgtgggctgcgacttctccggaacaattgaaagtacgggtcaggacattcaaaaatttaagataggagacgatgtgtttggcgtagtaaatccttttaaagaaggtgttctcggagaatacatcctggtgactgaaaacgaaatcgccccgaagcctgctgacctgtcatttgagcaggctgccgcgataccaacagccggccagtcggctttacagatgctcattaaaaacgtaagcaatcttagtggaaaagaagtactgataaatggagcatctgccggagtgggcatgtttgccatacagtttgctaaaagccagggcgccattgtaaccgctgtttcgagcgccaaaggacattcgctgttaaaaaaatggggcagtgattatgtgattgactacaacaaagaaaaggtgacagatttaaagcaaaagtttgatgttatcattgaactctccgcaaaactatctttcgggaaagctaaaaaactgatgaaggccaattcaacttatatcagtgtaacgccgtcgctctggaattttgtacactcattttcaaacaacctgttatcccgaaaaaaatataagatccttttaatgaaatcaggcacccaaagtttgagccggctggcacacgaggtaataaaagggatggatgtttacattagtaaaacttatccaatggcagattataaggaagcttataaaacggtcatcaaagagggcgctttgggtaaagttgttttccatgttgcgtcctaagcggaagcgcattgcacctaccttgtcacttcaacgaactgcggtattcattgggggaatgcccgacatgctgtttaaagaaacgggtgaaatgtgaaggatacttgaagccaagcatataagccacctcgcttacagatttgcttacatcaagtatccgttctttcgcagcctcaatcagcttgagctgtatgtactccagtgctgatttaccggtttcttttttcaccaggtcaccgaaatattttggcgacaggttgagctggtcagcacagtacgaaacggacggcagtcccagggtttgcagcttttccgattggaagtaatcgttcagcaatccttcaaatccggtcaatacgtctttatgaatatgttctcttgtaagaaactgccggtcataaaaccggacgcaatagttcaggaacatttcgatgttactcacgatcaacgtcctgctgtgtttatcaatagggtgcgctaattcataccggatcttgttaaaacactccaacacaatttcccgttctgcatccgacacgtgcagcgcttcattgacgttgtaggagaaaaaactgtattcgttaatacatttaccgaggtgggtgccgcggattaaatcgggatgaaagattaatgcccaccctgatggctgtatcatgttttcgctgtcattaaatccgaatacctggcccggggcgataaaaagaagtgttccttcttcataatcataatgattgcgaccgtattttaattctccgcacttttcgtcttttaaaaagatcaggtatacatcggtaatataacgtgtttcttttacaggcgtggacaacgactggtcaagcacacttaccaaaggatgcagggtcttttgtccccggtcgttattgacctgcgccacactttcaattctaagaggtttgcccatggcttcggtttttaattaaaaataaatgaagtatcctgaaaattcgtgctgaagcatgcctgaacagatatagtggtaagagaaacaggaatctgtataacatgctgatgcaaaagtatgaagaactttgcaccgttccatgaactattgaatcattcgatgcagttctgcaaaaaatcaggaaaaatgaatataaaaaaagttcaaagatgcaacagtagaaaactcactatctgatcattgactaaaacaaagcaccaatgaaattatcaaacaataaaattctgatcaccggcggagctaccggcatcggccgggggttgacggaaagatttatccgggaaaataaccaggttattatttgtggtagaaggaaagaagcgttgaaagaagtgtccgacaaattcccggcagtcatcacaaaggtgtgcgacctatctgaagaatccgggcgtacagaactttatcactggattgccgaacagcatcctgacctgaacgtattggtaaacaatgcaggtattcaaaactggatggatatttcagacaaggacttttatgataaagcaaagaatgaaattcaaataaatgtgctggcgccgttacatctggttgctctctttgccgggctccaatcgttggataccgttatcaatgtaacttccgggctggcatttgtaccactcaccaaagtgcctgtttactgcgctaccaaagctttcttccactcgtttactatttcactgaggcatttgctgaaagcacgcaatatagagatcattgaactgatccctcctgcgctcaacactgacctgggtggtaaagggttgcacagcgagcatccttctgtagctgattttattaaggcaatatttcaacaactggaagaaggcaaaaatgaactgacgtttggatatagtgaaatgctgtcgaaagcaacaccggttgagatacaggggatgttcaaaagaatgaacccgtaagctgagttagcatattggaaataaaacggccggcagatgagatcacttccggccgcttttttgttttattgttttcagacaaccacactctcctgtcctttttgtaaggcagtttcgcgcagcgtcggcgaactcacgccttccacacggaaggtggtgacatcatgcactccaataaatccaaagatccatttgagatacggttctgcaaaatccatcgccttcatcggcccttctgagtacactccaccggatgcgatggccaggtatacctttttattttttaacagtccttcaggttgcccgttaccataactgaatgttttgcctgcgcgcacaacgtgatcaatccaggctttcagcgcagaagggatgtgaaaattatagataggcactcctatcacgatgatatctgctgcttccaactctgcaatggcttcattagaatgctgtatggccgttttatatgcttcgctttcgttttccggaggagcgaaaaatgcagtgaggtgcgactcttccaggtgcggatactttttctgtacaagatcccgttgggttaccatgctgccgggatactgcgcttttaatttttcaatgatggtgttggtcagttgggtgctgttggaagcactaccccgtgcgctcgaaattatttccagtatctttttcatgtcgttattttttgctgatattgatattgcaaaactatccatctttacattcgctttacccggagtatgctaaaggttaccactaacctttgggttactggtaaagcgggggcttacccatttaccacgaattaaaaaatacctggttccgggtatataaacataaacaggtgtagggtaattttgcggtggaaccatcttcttaattatgaaacgtacacttattttcagctttctgatttccattgttttgttttcctgcagtaaagacgataaagcaaaaggccccagcaatgaagaaatcctgacaaagaaaattgcggacatcattccgcagaaatatcttgacactttaaaactgatgggactggatattcaccagggcgtgaaccctcccaatgtagaaggcagctacaagattgcaccgcataaactggataccagtaatattgcgggcgaccgtcccggaacatatttcagagatgggctggtatctctttcagaacaaagtacaacagattacagcattaagctgatcggtaaaaatttcatcagctacgccgacaccagtattgccactgctgtttccggctccggtaacaactttacagtatatggcaaagtgaaagccaccattggtacttactccgctgtattcgcccttattttcacgggcaccaaagaaggccaggacctgaaaaacgtgcgggtagcgattatcaatgtagataacagtcttggcggaaccggtatttttattcccgaaggctccggccgtatcggttatgatgaagatggcacttcgccgaaagtggcggagaaagcgcttcctgaaagtggcggacgcagtacattcctgcatacactagggcatttctgacaacaataaaataaacacaactaaaaaatggaaggtggctggtaaagccacctttttttgtgcccctacccctctcccaaaaaaaaatatttgctaaaccaaatggttatatatacttttactaaaccaaatggtttagtattttaattataaggaatgaaagcgagaagagacgtgttccaggcgatcgcagaccctacaaggcgcgccatcataggcctgctggcacagcaaacgctcaccctcaacacggtggcagacaactttaacatgagccagccggccatatcaaagcacatgcgcatcctcacggaatgcggactggtgatcattgtaaaacagggaagagaaaggcattgcacggcgagctttgaagcattggaagaagtagcacagtgggcggaacaataccgccgtttctggacaagccggctcgacacgctggagcaactattaaacgaaccaggatcctagctgtttattcatcataaaaaacgatacacgatggcaagcaatgaaacgccctgggtagaagcccagatgctgatacgcaaaccggtatcaacggtatttaatgcctttattgaccctgatgttacgaagcacttctggtttacaaaaggcagcgacaaattagcggtggggaaaacggtgacctgggaatgggagatgtaccaggtatcttccaaagtaaacgtaaaagagatcatacccaacaaaaagataacggtaacctggaatgagccggcaaccacgatcgacttcaactttcaggcggtagatgatcattcgacttacgttgtgattaagaattatggctttgataaaaccggcgatgagctgctgcgtgaaatcaatggcagcaccggtggcttcaccaccgtgctcgatggcctgaaagcctacctcgaacacaatattaacctgaacctcatagcagacaaatttccaaaaggtgtggcagcacactaaaataactatcaaccttttaaactaaaggacatggaaaaaacaggacagatcctctctcccggcaccattcgctttgagcgcaatttgcccggtcccattgaaaaagtatgggcctatctcaccgaatccgaaaaacgcggcaaatggcttgccagcggcgaaatggagttatttgaaggaggcaaagttcatttgcatttcctccaccaggaacttagtccgcttccggataatattcctgaaaaataccgcgacatgaaagatggtcatcatttcacaggcacggtattaaaggtagaatcgccacgcctgctggcgtttacatgggaaggcggatcggaagtgacgatggagttagcggagaaagatgaccgcgtattattaacccttacacaccgcaaactggccgacgacgttaaaacccgcagcagcgtaggcggtggatggcatacacacctggatattttaatcgccaacctcgaaggcgtaacacctcccccattctggagcacacataccaggctggccgcattatatgcagatatggcgtaaatttgatggtaatccatcaatacctgtcagcatatatggaggactttatctcaaaaaaaacagaccggaaaacgggcatacccaacttagtacaattgctgcgcggacaaatcagcagctcagagctgtcgtccctgctgctggaagtgtatcagcagaagtcggaagacatacagccggcggcgttgctgcaacaataccggcaaaacatctacgtgcaaccggccgacaccgacatgattgatatgctggaaaaggaattgcagctccttcgctttttaaggcaacagcaatatgaacctgtagagttgtcgccggtagcgcagtttggcagttgcgcggcagtgggcaccgttagccagaaaaagatcatcaccgcactccggcacacggaagtgctcgcagatgctaccaattcacttgcccttcatattgcagatctgaagcagcgtggcatagccacggctcccggtgaacggctgcgtttttgtaccgttcaccggcatataagggccatgcagcttcctcccggcaaaggctatacgccgcacttcaaaattgcctgtatggtagccgcaggaaaggataccggaaattttgattttgaactaaccacctgtgcagagcagatgaaacatatttattacctgctgcataccctgttcaacataactgatatctactttaaaatacaaccccggtccggttacaaaaacggccgcgcactgacggatgctttaatgaactatctttcttcccatctcccgtacaaaattatttcagacgatgcccccgcggaaaataattattataaaggcatacaatttaaagcggtagtacaactggatgataacgaaatagaaattgcagatggcggctttgtcgactggacacaacaactgcttggaaacaataaagagcggtgcttcatttcaggcatcgggctaagcctgctgatgaagctctcctgattgcatttactccagcaccagccggatttcgttattcctcttcatatcggtactaaggttcagcgtttttgattcctttccaaaccgtatacgcagctccgcggtattaggcggaatagatccaaggttgtcggcggtaaacaataatatattctctcccggctgcagccggatagcaatttgctgtatggctttcttcaccgggaagccggtaaccacccactggccgtttaaccgcagcgaaatgctgtcgccgtcctccatccgggtatctttcagttccaaaataatatcagccgtgcgaaccggtatagtagctaccggcaccgctgttcttttgatcacattactggtaatggtatccacattattatcagcagaagaacggtagatgtttgccaccaggaaagttgcccaggcattggagcggtcgctgaaatcaaatccgtagggtctaccgttaatggtagtacgaatacggccggtgttgggcggaagcccgccatagttatctgcaaaaagaacaaagtagttccggccggtgtccagccgcgctttcaggtgacggttatgatcattgatctgttccctggcgaaaataacgtttccattgtgaagcagcgttatggtatcttgatcatacttttcctggtcttctatttcgaggggaatttcgctgtctttcgccacaatgctgtcgtagatgccgaaatagatctggctggtttccgggtgcatgatccgttgcagactggaatcaggcaatggcttattcccggctttagtcagtttaaaatcgccgcggtagaggaagtcgcgcagcgccactttggattgttcataaatctcatcgccttcatctaatccccgcatccagaaactggctttgttgatccacatgcggctcagcgaaatactgttgtccttgtaatccaaagtgccattgagataccacatccagatgccgagcttatacggcgtttcctttaatggatatttattgcggcctattcccaactgtccgtcgtttttctttgccagcagcagttcataaataccggtaaactccccgtattgtaaagtgattaccgccggatacagcacgccttgctgtgcctcgccaatatgcagctgcatggtgatgggtgttcgcagtccccagggatgaagggccgctttccagatgccggtccacttatcggtttgcgcattggcagcatggatgatggtagttaacagcgcaatggtgataaagcatttcaatttcaatatggtcatcattatttaggattcacaatttaatactattttgggcgggcaacagcgcgttgaatgcacagttgtaaaataactaaatttaaacagataatggaatacacaaaggaatacgtcgcaaaagaagagcatatagatgttcagaatattatggatgggttatattatcctttctatatggagtattgccggcacgactacatcagggaaatactgggctttgattttgaggaacaggccaggaatggtgtttatatggttttatctggttacaagatccagtttttaagatccctgaaaaaaggagatcagttcacggttacctgtactttatttgccgatccgtcgggcgggccgcgactgcatttcaaacaatccatcctcctgaatgggaaggtgatgacgaaagcggtttttacaggcacctgtattccggcttccggaggccgtccgtatttaccgccatcggtgatggagaagatagccggcgccccggtgatcgacagctcggaagtgtaaacttatcatctgcagctataactagcaaagcggctttcgggaagaaggtcactttgcttttttagtttaaagtattaaattgtttgtgctatagcattctattattaaacagaacagatgaacaaactctttgcggcactgtcgctttccctgctggcattgaccagcgcgggccaatcttcccaacacgatctgcaatttaatcagctggctacccgctgggatgaagccatccccttgggcaatggttggctgggcgcgcttgtctggcaaaaagacgatcacctgagaatatcgctggacagggccgacctctgggatatgcggcccatgaaagggtttcatcgcaaagagttcagctaccagtgggtgatagaccaggtcaataaaaaagactacaaacccgtacaggaatacctggatgcaccctacgaccgggaagccgcgccttcaaaaatacccggcggcgcactggaatttgatacgcggaactggggcgccgtgcaatctgttcatcttacactgtctacagcgctatgcgaagtaacctgggctggtggcgtgcgcatgaaaacttttgtagacgctgtaaagccggtgggatggtttcgttttgaaaatgtaagcgctgatttcgtgccacagctgctggcgccgcaataccagggtgcagtgaaaaatgcaggtgatccggtgggcggcgatgacctgtcccggctcggctacaaacaaggcagcatccggcaaaccggcaacagcattacctatcagcaggaaggctggggtggatttacctatgaaatcaatgtgcgctggaaaaaaataaacgctactacgatagaaggcgtatggagtatttcctcgcaatatcccggcaaagcggttaatgaaccggcttcaaaagtaacggccaaagccgccggcaacaacttcaacggggaactggcagcgcataccggctggtggcaacacttctggcagcaatctgctattcatgtgccggacaccttactcgaaaaacaatggtacctcgaacaatataagtttggctccgccgcaagaaaaaatgcgccgcccatttccctgcaggccgtatggactgccgacaacggccgcattgctccctggaaaggcgactaccaccacgatctcaacacccaactcagttactggccttcttacagcgccaaccacctcgacgaagcaatgggatatattaatcaccttgaagccaacaaagcgaattataaacgctacacaaaaatgtacttcaatgcagatggtttagccgtgccaggcgttaccacgctggatggtactgaaatgggcggatggatccagtactcgctgtcccccaccgtgtcgtcgtggctggcccagcactattacctgcaatggcgttacagcatggataagcaattcctgaaaacgaaagcgtatccctggataaaaagtacggccgccttcctggaaaatattacaatcaaagacagcaacggacatcgctcactgaaaattagctcaagccccgaaataaatgataatagcctggatgcctggttcctgcaaaataccaactacgacctcgccctgatgaaattcactttcagcaaagccgcggaactggctacggtgctgggattgagcaacgaggccgcgcactggaacaaaatactttcccaatttggggacttcgccctctctcccggcaaagaactgatgtttgcccccagcatggcgtataaccagtcgcaccgccacttctcccacatgatggccattcacccgctggggctgatcaaatgggaagatggcgcgaacgcacaggcgatcatcaacaacaccattcacctggcggacagtatcgggccggattactggtgcggctactcctatgcctggatgggcaatcttaaagcacgcgcaaaaaatggcgcaggagcagcaaaagacctccagacctttgcccaggccttctgttctgtgaacagcttccacctgaacggcgaccagacaaaatcggggctgtcgaaattccagtaccggccgtttacgctggaaggtaattttgcctttgccgcaggattacaggagatgctgctgcaaagctatgcaggctttatagagatcatgcccgccataccagccgcatggacgaacgtatcatttgagcaattgcgcgcagaaggggctttcctggtaagtgccagaaaagatggcggccaggtggacgaagtaaagattgtagcggaaaaaggcggaaaaacccgcttaaagttgccgtttaaaactttctttgctgccagcaataaaggatttgtaataaataatccgggagatggattcctttccctgacggcaactcccggagcggtgttggtgctgaagaatggatatgaataagatacttacagggcgataactaacggtgttagttgtcgcccgtcattgaaaaagaatattattcctgcggctcttgttagccggatgtgttatttcccatttctcggaaaaatatttaccgcactctttgaggtacttgtaatacaggtaatctgtttcaaaactcagcagcagttcatagctgggtctgtattccaccataaaaacctccagtgccggtgattccagcccggtaatcttctttaccagtgttttattaaagcggtgatcgatgtacttctcccgttcttcccgttccaggaaacgccggaagttctccatgcgcttaatcttcttcatgctgaaaagcgcatccaggttaatgccggcgcccattccattgccgccactggtaagataatccggtgagtaatcgaacactttgcggtattcattgcggaactccgccgaatcctgcccgtaactgcgcggccgtgcggcagatacttccacttcccgtaatgaatgaatacttacatgcaggctcatatcgaaagtgcggttaacagggatctctttcacagcaaacttcatggttgctttcccctggtaggaaaagctgatggaatcattggccgccaatataatactataatgaccagcggaatcagtcaccgtgccggctcccgagttgctcatcacacttacgcccgccataccgaaacgggccgtacgatcgtatacagtgccacggacccgcacctgcccggcagacaccaggtgaagcgagaccaatactatcaatataaatatcctttgtaaaaatttactcatttccatctcaatctaagacaggatagaaacataagcaagggtggcctcaattattaacaattttctatgttttgattatgccggtgtcaaacccctttgctattaccaatcctatcgtatatttggcaggaaaattgacccaaaggacccaaaaaaaagtaaaccaggcttatgtacgaagtaaacccactgacagacgcactgaaaagaggcaacctgtcagcagcaaaagaacggatcgaccaaggtgaaaaattacccaaagacctttcatcctatgacaaaaaacaaatctatgataccctgatcagggcaaaagcttttgagctgatcgacacactggtaaaagaccgtatcattgaaacggatatttacgagtacgaaaaatttgatgagacgatcttcccgagcctgttcaggtacctgggcactgagccggcagacctggattttcttacttccttcaccgggaagctggataatatcaacgatgcgctccaggataaaaccttattgagcattgccttcgacaactccgctcccattgagcacattaaaatactggtagcagcaggctgtgatattcattacaaagataattacgatcaaaactacctgtataaaattgtacgggagtatacaatcaaagaagataaaggcgtggtttacctcgagtacctgattggagaaggattggatcccaatgcaggaaatatcgtgaaagaaacgccgctgcacctggctattagtaaatggcaggaaaagtatatcgacctactactgcaaaacggggctgacctgaaccagccgggaaaagacgatgaaacggctttctatgcagccatcgtacaccaggtatgcagtgtggaaaagtatgaaaagctggccgcatatgcccccgtggatttcgatattgtcaacaaaaacggggaaaccgtttttagtggcgctatgcgtatgcgccggcagggttctccatctgaagtgcagctgttaaaagcgctgatccgtgatggcgcagatatttaccagacttctccttattacgccaaagacaaagccgcactggactgggtggcggaacgccccgcagatattttagaggccatactggaaacaggtgtggtagaactggaccggcgggatgatgaaggcaacacgctccttcataaagtgtgcgcctataacgtaaactatgagcaggaagcagccaggcaactttaccgcaaagtaaaactgctgatagaacatggagcagatgtaaatgccaccaatgatcttgatcagcgacctattgacctggccagccaggacaacctgaaatcaaaaacagtagagttacttttaaaaaataaagcgtagtactatgtccatgtcttttataattgcctgtgaaagtggcaaacgtaaaatagccgaaattttacttgccaataacgaagtagatgttgcctataccgatgagaaaggaaggaccgcgctgcattacgctgcacatcacggatacctggatattgcaaaactattgctcgatgccggggcagatctcgactacgaagaccataacggggaaacgcctttttacttctcctgtctgcaaaaacaaaaacaaaccgcgctgttcctgctggaaaaaggcgcgcgtacagatatcaacgacctccagggaaacagcctgttacatctgactgctaaaaccggtcagaaggaactgatagaaaaattgctcgaaaaaggcgttacagtggacctggaaaacaacgaggccgaaacgcctttactcattgcttccgcctggcgcaataaagaagtggtgcaaaccctcattgatcatggtgcggatgtgaacaccaccaataaagccggcgatagcccccttatagtggcagtgcgctccaaaaacctggcgatggccgattgcctgattcaaaataatgccaacgtaaatcataccaatcatgcgggggaatcggcgctgctgattgcctgttatgataccaaccgggcactcaccaacctgctggtacagcacggcgcggatgtgctgatcacgtctaaaaatggtttgtccccgatatggtacgcctgcgccaataatcagaaagagatcgtcaccctgttcctcgataagggcattgatgttaatttcagtcagccgctttccgcagacaccgccagtatgaacacctacctggattgggtggaaagtgcttccagtctttctatggacagtgcctttaccctcaatcacacctatagctacggtggagaaagcctgctacatgtggccgctaagaacggccatctcagcatggtgaagctgttgctggaacgcggcgcccatgtaaatatccaggatgaatcgggaaatacagcgctgcattacgccgcctccaatggtaaaaaggatatcgtaaaatacctgctggaacagcaggcagatgtatcagtagttaataccaaagaacaaaaggccattgactatgcatccatcaagggatacaacgaaattgccgcgctgctgctcagttataattcgccccaggcaaaagaagtgaaaaacgaagtacctgtagcggaagcgcctgcaggaaaaagcatggcagataaaaaacaagctttgctcgatctcaaagaactgctggacgccggcattctttctgccacagaatttgatgaggagaaagcgaagatattaaaaggataattccattccggcgctcctggtgaaggagcgccgatttatttccgcaccatcgccccataaagcgggctcataaaaaataactatctttagcccgtaaccatatgaggttgttgggtataatattctttctcctatacaggacaatgggggattgcgcatatagataataacctctatatatccggaatgctatgcgcaatgctatcgtaaaaaaaacagctatcaagacattgaaaattatttcaatatcaattgctgccatctttcttttattgtttttgctgcccgttcttttcccaacggctatttccaataagataaaaacctggaccaataacagtattaccggggatctgaacttctcccgggcacggctgtcgtttttcaatcacttcccctcgctgacgctcacgctctacgatttcagcctgaagggcgccgctccttttaaacaggacacgctgatagctgcgaacgaagtggcccttggtgtaaacctggccagcatcttttccagcgccatcaacatcgatgaaatttacctgacccgtggcgatattcatgtgttgacagatgcggaagggcatcccaactataatgtttacaaatcggcgccagccagcgctgccagccaggcagacagcggcagtgcgtcccttaaaatagaacgcatacaactggaaaactgcaacatcatttatgatgaccggtcgctgcccatgtacatccaggccaaagatgtgaactataccggtaaaggcgatctgagcaaagcgcagttcgacctgcactcacgggtacgtatcggggcctttgatcttacctatgccggcacttcctatatcctgtcgaagaaattaaacggggaactgatcaccaagatcaacaccaattccctggacctgatttttgaaaagaatgacctgaaactgaatgagctgccggtacggttgaatggctctttcggattcctgaagaacggctaccggatggacttccgtttgagttcgatggaatccagcctgcacgctattttcagcgcattacccgcggaatatgttacctggatggataaaacagacatacagggaacggccgatgtaaatgccagcctgatcgggcaatacatcgccgaaactaacaccatgcccgatgtaaccttcaacatgaaagtacgggaaggcgtcattacaaacgacaaagccccagcacccataaagaacctcttcctcaatttccagtcgaggttgccacagctcaacctggacagcctttatatcaatgtggattctatcttctttaacattgataaagattatttcagctctgtgatccgtgtacaagggcttgccactcccgacattcacataaagctgaataccgacattgacctggaaaaatggaacaaagccacaggcggccagtcctttgatatgaaaggacggctgcaggcacacctgcaggcctacggcaaatatgccaaaggcgttgtataccacggcctccggaagcaggcagataccgtgattaccagcatcccggcattcagcctgaagtccaacctgcggaatggctacttcaaatttacgtccatgccgcaggcgcttaataatatcagctttaatgtagacgccggctgcccggataacgactacgcacatacgtacctcaacatttccgacatcaacgcggagatgctgagtaattatatcaaaggcttcttccggcttcacaatgcacaggaaccggtagtggatgcacagcttgcatccgtattgcacctcggcgatatcaaacaattctataaaatggacagcctggacgtaaccggtgatctgaatgtcaacatcgttaccaaaggcagctatgtacccgcaaaacgactgttcccggttactaccgccaaactggccatgaataacggcaccgtacaaacgaagtactatcctcacccggtggagaaaataaatgtggatgccaccatcaccaataccaccggcaccatgcgttccctggaggtagatcttaaaccggtggcctttgagtttgaaggacaacccttcatgctgaaagcggatctcaataacttcgatgatctccggtataacattacgtccaatgggattatcgaccttggtaaaatatacaaggtgtttgcactgcagggctacgacgtgcagggttttataaaaacggacctctcgcttcgtggcacacaaagcgacgccaccgccggcagatacggcaaattgaataataaaggctcactggtagtgaagaatattattctcacagctgaactgttcccgctgccattccatattaaaaacggcgttttccgtttcgaccaggataaaatgtggttcgatcaattcgatgccagctatggcaaatcggctattacgctgaacggattcctcagcaatgtaataggctatgccacattgaaaaatcaaacgctgcacggcacgttcgatctgaaaagcaattacatcctggtggatgaactgatggtgaacggcgacaccaaaaccagcgctagtcccaccaccactacttccaccggcgttatcatggtgcccggcaacctatcgctggcgctgaatgcagccgtgaataaaataaacttccagggcattgccatcgacagcttccgcggacaacttaatgtagacagtaacaaagtacgcctcagtaaaaccggcttctctgttattggtgcacccgttgaaatggaagccacctatgtaagtattcagccaaagaaagccacgttcgattatcacatcagcgcaaaagagtttgatataaaacgggcctataacgaaataaagatctttcatgacatcgcctcctctgcttccagcgccagcggcatggtgggactcgactaccagcttagcggtaagcttgatgaaaacatgcacccggtatacccttccctgaaaggagaaggcgtgctgtctgtaaagaaaataaagatgaaaggctttaaattattcaatgccgtgagcagctctaccggcaaggatgaggtgaaagatcctgatctctctaaagtagatattaagtcgtctatcaaaaataatatcatcaccattgccaggacaaaaatgcgggtagccggcttccgcccgcgtttcgagggacaggttagtcttgatggaaaactgaacctgaaaggccgcctggggctgccgccatttggcatttttggtatacccttcaacgttacgggtacacagagtaatccaaaagtacagctgcgcaggggttccgaaaaagataacctggacgaaacggcggatcctgatgaggtacagaattgattttccggtacctgcttatttctctttaaagatttttgccaattcttcctggagatgctcttcccggagattttgtgcgatgattttaccgttgggatcaatgaggaaattagcggggataccgcggatcccatattgctgcgccacttcgttatcccagcctttgaggtccgatacctgtggccaggttagctgatcattgtcaatggctttcagccaggcgtccttctggccgggcatatcgagcgatacgcccaatacggtgaaacctttctctttatatttattgtaggccttcagcacgttggggttttctttccggcagggaccacaccagctggcccagaaatcgagcagtacatagctgcccctgaatgaagaaagctttaccgctttgccatcgggggattgttgtgtaaagtcgggcgccaccttgcccatttccgtgtttgcccttgaggcaattaaaaccggtatcctttttcccagcggtgaatttttcagatgggcgggcaaacgttcatacgccttccctgctgccgctgccattcccggatgggcggctgcctggacgagactcaccacactgagataagaggtgggatacttttgggcaaactccaggtatacctcatacgactctttaagcagctggctttcccgtgccatgaaagcatcgtatacttttttatccttctgctgtgcttcgggcatcgctgtaaattccttctgcaaagcggaaaactgctcatcattctttttcaacatcgaccggagcacggcttgctgatcgtttacaggtgagtttttgatcacgatgtttttcagtgaatcccttgcttccacgttaaaggcagcgggctccaggtataatcgaacatagtctatttgctcacctcttcccatttgttccacatagggatttttgcggaggaataacccggagtaaacggggtattccagttttcccctgaaaacaaaccggccatctgttaccatggcggaatccgttatccgctggtcttctatctggtaaacaagataaattttatcgccattatgcaaactatctacctttcctttcagttcaaagtgatcctgggccaggagtgacagcggaaataaaaaagtaagcaataataatgtacgcataggattcattttaacgtttatgggtaaccggtagtaatgttatccggttggaaaatgtagttgccaatcgctgttatccgagcaactgcctgatccctgcaagatgatgatcatcatgctctgccacaaaataggccaggtcaatgatccgcataggcgttttcaggcgtgggtgcagcgctgtttttgccaggtgctcatcctccaggctccaaagcctgctgacgagctgttgccgctgctcgtggaactgttgcagcaacacgctggcgggtgttgcattatgattggcagcatgtgttttctggttggttaaatccgctaccctcagctcagtggcgccgttgataagatcttccaggcggcccagccacagcggttccatatccgaaagatgccctgcttcctccttgatgctccatttctcccctggttttataatgagtaattcaggagctgtggtgcggatgatttcttctatgcgggcgggcgttccgctaagccgttctataatagcgggcagcaggccgttgtcttcaataacagggaatgttctgttgaaccattcagttcttttcattactatctgattacttaacttaaaaataatgataataagtgatttctatcaaaaaaataaacacatgtaaacatgaattttttgttaggaatactaataatattttttattactaaacattcttcttaagttggtatccgaccggcattcattgctggtatgatgatcctcaaatatttattattcaccctcaaaatttatcaaatgggtatgatcgcattttatgaaggcaacaatggcacggagagccttgtacaaacagtaaatgacaaccccggacaagacttccagccggtaaaggctgagatccgctccctgcggctatttgatgtcaggggccgttgccgcatcaggatatttgattcagcggatggcgctttatcgaatgaattttgcattgttgatgtaaaaaacccaatgccggagtatacagtgaacatttttgtaccaagctatgaagatgactatgtagtggtaacctttataccggtcaagggtcttgtgggtaaagtattacgcataaaaatagactaaggaatgaaaacagccggcgccataaattgggccggctgctttttaatatgtttcccccgtatactcccccgctttttccgccggcggatgaaattctttttcgctttttgcaattactatcgtagcaacaccgtttcctataatattcgtaatggcacgtgcttcactcataaacttgtctacccccaacaggaaagcaagaccttctaccggaattttatgaatagcggtgagtgttgaagccagtacaataaagccgctgccggttacgcctgcggcgcctttcgaggtgatcatcaatattccgataatagtgaggatttccccgatagtcaggtgcacatcatacagctgcgcgataaaaataacggacatcgacaggtaaatagaggtcccgtccaggttaaaggaatagccggttggcactaccagtcctactacggatttactgcagcccatcttctccagcttcagcatgatggaaggcagggcagattctgaggaggaagtacccagtaccaataacagctcttctttgatatacttcagaaatctccagatgctcattttatagtacttcaggataccaccgagtaccaggaaaataaaaacagccatcgtgaggtatacggtgcccattaatttggccagcggcaccagcgtatgtaaaccgaacctgccaatggtgtaggccattcccccgaaagcgcccagcggagccaggtacatcacgtatttcaatgctgtgaaaaccagtttggaaagtttgctcagagctttaataatcacctgccggtattttgagtaattgagcaataccccgatgatgatggcggctaccaatacctgcagcgtcatgttattcaggaagaaggtgagccagtcgaaactctttgctgcaccggaagtgtatttggaagcattttcgatttgcagggacgacttgtcaatttttcccggccggatcaataaggccatcaaaacgccggcggccagggatatggtggaaactacctcaaagtaaagcagtgatttaacaccaatacgacccacttttttcaggttctccattccactgatccctaaaacaatggtaaggaatataatgggtgcaataaacagcttgataatatcgataaaggtttttcctataatttccatcttcacaccggtggccggcgccagggtgcctaataatatgccggcgataatggcaatgagcacccagaaggtgagattggtaaagatcctgatgtgcaaactccggttcacggctacttccggttgatacgacgcaatgtcttcgtgcatgggttctatcggttttcgttgaaattccccgtcaagtaacgaaattttagccgcttatttcagcaagggtcatatatttattttatgggatcggttgcagctttacaatccaccggtttcaataacggaaataatttgctgacgtgcctgcctggattcaggtaagttaatgagcatccagtcgtgtaccatccctgggtattccacatacgtaaactgcaacacttccggggccatcatctttttcagtttacgggcatcggctaccagtatttccctggatcctgcaaaaacagtgatgttttccaatcccttaaatgagccatagatcgggctaagcaggtaatggtccagcggtgcgttacccgcatagatcctgccggcctgcagaagtccatccagtcccataaagggatcctgcgtaacgatttcgtgtatctccgggttactcaaactgatatccagccagggcgaaagcaggatcagttgtcccggctgcggcagctgttcctttaccaataactggcatagcgccagtgccagccctcctcctgaagaatcgcccatgatgatcaggtcctctttggctactttttcaagtaattccctgtaaagggctaacaccatcttaaaagtatcttcaaaagtaaagtcaggcgccagcgggtaatccggcgctgagatagtgcaatgcgtggccgctaccaattcggccataaaagaccagtggtgcgatgtaaaattttgtacataagcgcctccatgcaaatacagtatatgcttccgccctttcccggtgcgggactgcagggtgaaaacaggctggccgtttagctgccgtttggctaccacgcaaaatttgtggaccttagccgtgggctccggactactgtaaaaattctgcttgcctgcggccagcagtgtttttagaaagtgcttcttcccgattaaccggagaaaaagggcaaataatttgctgtgtatactggccaaattgatctgttttaaatataacaacggtgctgcctcgcatcataatatttacaaccagtaaggtatgcctaatattcagacaaacgatttctggctccgcctggataatgcagcaaaaatttatccggctattaaggataacgagcttacctccgttttccgcgtagcggtggtgttaaaagaccggataaaggcaaaggctatgctggaagccgttcacgaaattgaaaaccggttcccttattacaaagtaaggcttaaaacagggttcttctggtattacctcgaacagcaacagggcccggttcccgtagaagcagatctgcaaacaccctgccgcgccttccggaaaaaggaactgatgtttcgcatactgtaaagaaaaacaggatcagcgttgaattttcgcatattctgacagacggcaccggcgcgtttgaatttctgaaaacattattactcgtgtattttgaaaaatgctgtattccacttgcagataaaccggcgttttacaatcccgatcaaccaccggcgccggaagaatacgaagatgcctatagcaggtattttaaaaaaatagacgcgccgcatataaaaactcccggcgcctttcatgttcccttctctttaaaaagaaaacccaggttcagtgtgcttaccgccatcatgcctgtagcccaggttactaaaaaggcaaaggcgctgggagtgagcctcacggtatatctcaccgctgtttatcttcacgcactacagcaaattcatgaacaacaaccccgtttaaaaaagaatatcaacaggaaaatattacgtatcgaagttccgctgaacctacgtaagttgtaccccacgcggtcgatgaggaacttctcattgtatgtacttccgcaaatcgatctcaggctgggacattatacatttgaggagatcgttaaaaccgtatatcaccagatgcaactggaaaccgaccagaagctgatcaataaaatgatttcccgcaatgtgggtggtgaacgcaatacgctggtgaaaaatatcccgcttttcctgaaatcgcttttcctttccaggctgtatattgttggtacaaaacaatacagtggcgtagtcaccaacctgggaaagatagacctcggaccagacgccaatcacctgattgagcagtttgtatttattgcccctccgcccaataaagtattgaaggtaaattgcggtgttgccgggttcggcgacaacctcgtattaagttttggcaatatcaccacctcaaaagaactggaaagacatttcctgacatttatggcgcagcagaatatcgctgttaaaataataaactcatgaagtattgtaataactgtggcgtaatactggaagacgatatgctgatatgcccgctatgcggcgccggagcaggtaccaacagcgaaaagcaggaaacagttgacaacggcaggaaaataatagcagccccggctgaaacgctgacaaagcaacaaaagaaactggtgtgggaaattgtatccctggtgctgatttcctctattgtagctgcgttgctgattaatcttattatcaacaaaaccgtttcctggtcggaatacccggtggctgtttgtcttactattttcgcctatgtttccttctttgccttttggtcaggcagcagcacggcccgtatgctgggaggatttatcacctcgtctgtgcttatgttattattggatgcgctaaccggtggactcagctgggcggcccccatagcgattcctgttttattgacagccagtggtattaccgccgttttgctaagcatcatccggcattcggtttccaaaggcgttaacctgatcgcctatacgtttattggcggcgcggtattatgtatagctatagaggccatactatccctgtaccacaccgggaatattcacctggaatggagcctcattgtttgtttatgcgtgctgttggtggctattgccttattatttctgcacttcaggttaaagaaaggcagaagccttgaaaaaacttttcaccggtaatcacagtttgtaaacttcactacccgctaacaggaaacagcctaatccataatcttcgaagtcgggtactttatcaaaggtaacgggctgtccgtctttaggttccttaccggtgccctgcacatagcctaatcgtccatctttatcgatacagttttccaggagggcattccatgctttccggactataggcagataggttttcttatcgaccaggtgatgattgatgccccaggccattccgtatacgaatagcgaggtgccggtcaattccattccgccgtagttatccgcatcatgcaaacttacattccagaagccatccgggcgttggatggggaccagggcttttaacatatcctggtagtcctgcaggtattccttgtaatgcggatcgctggtgggaagcaaatccagcgtgcgcaccagtgcagctaccacccagccattgcccctgctccagtagcagtcttccccattcggtgcagtatagggaggcacaaaatctttgtctctccaccacaggtgatctgccgggttatacaaacccttaccgccgtgattatatttcgtgtaggcgtacatggtatacatccggttaaaatagctggtatctttgtagatcacgcctagcctggcgaacacgggcatggccatctgcagcgcatcgatccaccaccagtcgtccacttccggggaggctttcatattatccatggcggctttaatatccctgatgcgttcttcttttttatcgatgaggtacaggtctatgtaggtttgtccgcagcattgattatccgcattccgtacttgtgtgccgccccaaagtccccactgatgactattgccccaggctacggcataatcatagtaagcggcttgcttgtcgatattgtagagcgccatgagtccttcataataaaccgcccgggtccacaaattagagggacgttctttattggtaaaagtaggcttgcccggatctggccatttctgcataaaatattgattggtgaggcgcattgccgccagggtctctttttttgccggcagcttttgtgcaaaggccagctggctgataaaacatagcgtaataaacaggcttttcatacgtggtaatttatttcagattcttctgatgggttactgtatataactgtcaatttaacaattataaacaataccccatagttttacgggtacttttttgcggtccggtatgggtattgttgtaagtttggaaaccaacaatttttcaccgtatgaaacaaagcgccggtattttactcatccgtgctgccaggagcggacctgagtttttcctggtacaccccggtggcccgtttttcgcgaagaaagacgctggctggtggacggttcccaaaggagaaattatgccgggagaggatccgctgaatacggctatccgggagtttgcagaagaaacggggtatacgccggccgctcctttcacccggctgactaccattacccaaaagggtggcaagcaggtacattgctgggctgcatccggtaacctggatccggcgaaaatagtgagcaatacgtttgaaatagaatggccgccgagaagcgggaaatataaaacctatcctgaaatagacaaagccggttggtttaccctgcaggaggcggcaaagctgatcaatgaaagacaggtagcgtttttggaagaagtattgcaactgggcttaacagctttataaaagccgggccggatggcgcatccggcccggctaatactacacaatggtattgagcacacctccatctgcgcggagcgcagctccgttggtggctaccgacaaaggactggaaagataagccaccaggctggcgatttcggaaggctcaatgaaccgctgtaataaggaggttggattcattgttttaataatacctgttttcactgcttccacgcccaggttttgcgcacctgcaatttgttccactgcgttcgccacaccttcggaataggtgggcccgccaagaatagcgtttatcgtaaccccggtgtttttagttaacgctgcaagtccacggctcaccgacagcatggcagttttagtggtaccgtagtggatcatatttcccgggatatgaataccggattcgctgctgataaaaacaatcctgccccagttacgctccagcattttgggaagcagctgccgcgatagccggataccactcaatacatttatctcaaaaattttctgccagtcttcgtccgtgatatccgtaaactcctttagttcaaatattcctacgttgttaattaaaatatcaatacctggaagcgtatccaataaccggttcacctccgcggcgctggcaaagtcagctgctatgccggataccttagcttccggtatttcttccttcagtctgttcactgccccagctgtcttttcaggcgttcttccgttgataatgaccgtcgctccttcgagcagtaataacctggcaatggcaaagccgatgccctgtgttgatccactgataaaagccgtttttgatgttaattgtaaatccatgagcgtcctgttatattattttaatagcgaaagattttgttctgtgttgatcactacaaatatcagcaaaaaaaatcagcggaggatttccagctgcatttcaatctgtttgaggaggattttattatcgggatacatccgcctggtaacgttcaacccgttccagagtgtaaccaggtagcggcccaggatcacgggatcggtttggtttttcatagtgccattcttttgcgcgcggcggatggctttggtgtatagttgttctacttctttcagaatggttacggcttcctcttccagttctttgtcaagagacgccatttccaccacggtgttaacgatgatgcagccctgcagatgcgtttcccggtcggcccgggccatgctgcggaagaagtctttgatcagctccattggcgcatcactttgattaagcgctgtttcaaactccttaaatgcttccctgcgctgttggatggctttttggaacagctctttctttcctcctttaaatgcattataaaagcttccgctgcctattcccatagccgtgagtatatcttccagagatgtagcggtatatccctttgtccaaaacactttctgtgccttctctacaacatccttattatcatatatggctggccgtcccctcatacaatacaaattttgtgttaatcactacaaaaatagatattttttaggaacagtcttaattatctttaaaagattagtgtttgaaatacttccacaggtaggcggaaacgttcttgatcagcacctgtgcttcgttatcgtctgtccagcgctgatctttattatttttggtgcccacataaaacacatactccccccgcggttcatttaccaggatcacttctgacctggactcatccagtgaaccggttttatgggcggcctgtacatacggcggaatagccgacaacccggtttcatcataatacccgtgggtcattaaccggtacatgcgttcggaagcggccttgctgatcacctcaccattacggatcttcaccagcagggtggccatttcgcggggggtagtcatgccccagccgtatactttccagatctctgcacggccgggggtacgcgaatttacccgcgtaacagcaagtccgtactgctccatcagctcattaatgcgttgcccccctcctgccagcgactggttccagatggatgcggtattatcgctgtaagacatcatcagcgccagcaatacactcacctccgttgaggtgctgtctttaaagaactgcatcaggcccgatccgccatacttaatggaatcgcggtaaaccagcggctgatgatatttcagttcgcctttttcgattttgtcaaacatgcccaccaggataggaattttcacaatgctggccgtggggaaaatagtgtcggcattgatagcggcataacggccggttctcaggttctttacgtaaattcccacatcgccgtgaaacccggtgataatatttctcaatcctttttcaagtttacggtcctcctgcgaaaaagctagtacaggagtcaacagcagtagcagcaaccatttgtgcatatataaggaatgtttgctttaagttataatacgggagccggtattcataggaggtattattctgaatcctcttttggttcccaaagttcaataatattgccttccggatcgagcacatgaacgaatttgccataatcatattccgcaatctcatcaacaatagtcacgttttcctttttcagttccgctaccagcgcaacgagattttccacgcggtaattgatcataaacggcttgtccgatggcttaaaatatgccgtatcctgtggaaacgcacaccaggaggtagatcctttcttcgacggattatcggcctcccgccactcaaacgtagtcccgtattcgctggtagtcaatccgaggtttttagcataccattcgttcatttcctgcggattagcgcatttaaaaaaaacgcccccaaggcccgttacttttttcatatgtacgattaaaaaagtgaaagaagaagtcgatagtcaatatactaaagaatatgtaacctccatccgggacttttaaaaaaaatgtatttcctgttgacatagggttgtcatatctcccttttatttttgttaaaacaaaccaactcactatggccgggaaaatgattgaaaaaggcgctatgacccaacaggggcaacaagcgatcgaccatgcaaaaaaaaccggcaggtgggagatcgtgtagtgctcaccacttcactaacggatttcgccaccagtcgtcctgcccgttttcgctggagtagagtccgaagttcagcgatggatcgtccgctttttttgcgggatgcaatagttttaaaatataattccctttgcgcagtggcagtatcaccgtttgccgtacatggccatccgccgggttgtactgaatccacaatgaatcactaagatagagttgtgtgccttccgaaggcgttagttgaaatacatagtagccatcacgcggaatagcgacgaccccggtcagctgaccattcacaggcttcgattgcagatcgagctttggcaattgccgggtagcacgcaacatcttttccggcgtcagatagtcacctgtccgcaggttcattggcagctcatgatcgtatcgcccgcccggcgaaaacgatattgcccggatacctgaaggatcatctgtgatcaaatgatcatctaccagcgcactgttgcggttgggcaatgaaccatcctgcgtatagcggatctcagcgttatcagttggcaaaaacaggcggatcggccggcccttcaccacaatgccgccggtcggttgataacgggcgttgcggacgtaataccccaggtaagcatatttaagtccatcatagttcgatttgaacacactcgatccatgcgtttcattgtcgtagagcgccgagtgccagtgcagccctgaaggtgcattcgctttcagcatgctgtccattgcatcacgcgccatgtcgccgtaggaaaaaccactgcggccaccgatattcagcacggtgttgcggaattgaaccgactttagtttttgcgctgccatccgcacgaggtgccggtcgccgaactggaaagccgggtcgccgagcgtatagaaacggaacaagtccggccgctgaagcagggtgtaaaaagcaaataccccacccaatgatgtaccgaacaacccgctctcgctactcacgcgatacttgcgattaatatagggcatcagctctttttcaaagaaggcaagaaatttgtccgcaccacccgagctgtccacatctttcgattggataggggtgaaatcgcggtcgcgcaggttgaaaccgttgacataacggttggggacattcacaatgatcgcctgcggagcgaactttatcgccaccaggaaattgaagatattcgtaaacgtatgcgtattccactccccatcaatcacgtaccacacatcataatgagtagtgtctgctgcgtaattgtccggtaaaataatctcaattttacgtagttcacccaggctattcgagtaaatcgaatcctttgttgatgtggtatgctgggcttcaacgctaattgtaacaagaaataagaaacaaaaaaataaacgcatcgtcctgttttttgtgcttaaagttgtcactgatactttgctataattccgtaatttcaagtacttctttgctatattttaaataggaaacgagcacttttgtgcctattgggtaatgatagtagtccgctttcttaaccggcaggctgaatttctcgcctttatgccgccctgcaaaggtcacaatatattcatcattttctgttttgtgacggctgataattacactcgacaatttgtttttcccgtttataatatctttcttccaatcgtttttaaaactcctgaacgttagccaaacaaataaataaaaaagaccgaacattgctattcctgcaaaaacaaacaaaatgtaatggtaatattgtagattaatttcgtgttgtataaagtaataagcgatcgccattataaaaagtgtggcggtcatcaaaatacctggggcgtctttaaagaattcacttcgttgtttgtcaatatgttttatctcatcctcgcttaaaggaatgttttcctgtaatacaacctggaaatagtctattgggaaatgggtcattaaaggcaatttaagtttgtctgtccaatataagcctgatatccttgttatatcacgaatacttcccgggtacctcatccatgggtataccatgggtaatccatgcactattaatactgttcccatgcacttccaatgcactactcatgcactccccatgcactatgaatacactttacttttcgtactcatactttattaaccggtattggaaaacagttttataaacatcgccaattttatattggtccaccagctccccttcttttaccaggccgctattaatcaaaatcttttctgatgcattgttttcgggaaaaacagtcgcgtaaattttatggaggtgtagcgtgtggaatccaaagttcaggacttcttttaccgcctcggtcatgaggcctttgccccagaatggttccccgatccaatagcccatttcagcatggttatgacgggtatcaatactcaatcctactgcaccaatgaattcattgtgctcttttaaattaatcgcgaaaacaacccgttccccggtcacgtatgcctttagcgcaaggtctatccaaaaggcagcgtcttcctctttataaggataggagatatttaatatgttttcggagatcctcttgttattggcatactttaacagggcgcccaggtcatccctttctacttttcgcagttttaatctactggtatacagttcaggaaatactttcatgttgaaactcagctattacagtatgtaaatataacagataggctcctatatttttttgtattttctaacagaaaaaatggcgacccggaaggattcctcagacccacttcacccgttttaaataaaatcacgtctctaacagatatcaaatgctacgttatgaagctaattccacccaaatggagtcctttcctgcaaggactggtgctcttcttttggcttaaccagccggttgtttttgcacagggacaaaaacaggtaaccctgaaaagcgggaatgccgccatcagcctggcagatatattcaaagccatccggcagcaaaccggctatactgttttttataataatcttatcctgaacgataaggaaaaaataaaagtagacttcaacaaaagcgatttaccggcagtacttaatacgctgctgaaagataaaaatattgagtggacgtttaacgatacctatatcatcctgaagagaaaggacaatgttgcggctccttcccccaaacaggaaaagctgcagggcagggtaacagacgacaccggccagcccctggccagggcatccgtgagaattaaaaatacgaccgcggcggcgcagacagatgataacggcagcttctccatcgtcatgccggaacctgccggcattttacagatcggctttgtcggttatgaaccgctggaagtaccgcttacagacatgcgtttccaggacataaaactaaagcctgccaacagcggtctcaatgaagtaattgtgatcgggtatggcaccaccacccgcagggacctcacgggctcagtgggcaaagccaatgtggaggatatgcagaaagcccccgtagcatcttttgaccaggcgctggccggtcgcattgccggcgtggaagtaagctccaacgacggacagccaggcgctgcttcccggattgtagtgagaggaagctccgtaagccaggacggatctcccctgtttgtgatagatggtttccccattgaaaatatggatatcaattccatcaatcccaatgatatcgcctccctggaagtattgaaagatgcttcttctattgctatttatggcgcaagaggcgccaacggcgtcatcatcatcaacaccaaaagaggaaaaccaggtcccccaagagtgacttacagctatgcgctgggcatacagcaaatcacgaagaaaatggagatgctgagtccttacgaatttgtaaaactacagctcgaactggacagcgcggccagtacgcccggcacacccgttaacaccaacgcacgcatttacctcgatcctgcaaaaggcattacgctcgactcttataaaaacaatcccgggtacgactggcaggacctcctcctgcaatcaggactcacccaaagccattcgctgaatatcagcgcaggcaccgcagacacgcggtattccatcagtggctcctactacgaccagaaaggaatcattatcaataccggcctgaaaagatatgacggcaaattcacgctcgatcaacggttgaataaaaatctccggatgggcatcaccgccgggtattccaattcttcttcctatggcaccatacccgctgcatctttcagtggcggcgtagtacagggcatgtggcaataccggcccgtttccggcgtaggtaaccaggacctgctcaacgctgtgatcgacagtcttgcgctggaagacttcaacaatggcacctccaatgccaccctgggaaacaacctggtgaacccgctgctacaggcgcagaatgaataccggaaaaacatcaacaacaccggtactattaatgcgttcctggaatatacttttctgaagaaattcagactgaagatatcaggcggctataatgccaccaacctgaaatcggaaaccttttataactcacaaacacaacagggaaatttattcaagaacaaagcaggcgcagtgcccaatgtgaatggtattaacggcactatcaacaatcagctgaacagtaattatctcagtgaaaatattctcaactacaaaactactatcgggaaaaaacatatgattgatgcgctggcaggtttcacttatcaatacgccacgaacaattataccggcttcaggtccattaatgtgccacagtcgaccgaatacctgggcattaaaagcattggcggcggcaccgccgcatctcccaatgccggcggctcgcgctggcagctgttttcttttttaggccggctgaactatgcttttgaagataaatacctgttcaccgccactgcgcggtccgatggttcttcaaagtttgcggcaggcaagcaatggggctacttcccttccggcgcttttgcctggaggtttacagaagagcccttcgcagcaggcttgcgatccatactgaatgatggtaagttcagggccagttatggcagcgtaggcaacaacaaggtgggagacttcagctacctggctaccctcgctggtggtacgcagttcgcctaccctttcaacaattcctatacgagaggcaccgtaccatttggaaacggcaatgccaacctcacctgggaaaccactacagaactggatctcgggttgaatttaagcttcttcaacgaccggatctccgtggatgcagattattacaaccggaaaacaaagaacttcctgctgctggtgcaaatcccttacttcgcgggttacagtatcacgtctttcaatacccaataccagaacaccggggaaattaccaacaaaggttttgaactaaccatcaacaccattaatgttaaaggaaaaaatttcaactggagcagtagcttcaatatcagttttaacaaaggaaagattgataaattttatgatggctttgaagtaatgcaaacaggttataacctgcccggcggcaacagcaccactgcctggattgcaaaagtggacgcccccatctcccagttctatggttataagtgggccggcgtttaccagtatgatgattttgttaaacaagggaatggcgcctacatcctgaaaaacggcgtacctggctatgccaccggtattcagccgggggatccaaaatacaaagatattaacggcgatggcgtagtagatgccaacgatcaaactacgttgggcagccctctccctgttcatacaggcgggttctccaataattttaactataaaaatttctacctgaatattttcctgcaatggagctacggcaatgaaatactgaacgccaacaggatggcctttgcttccaccggaggttatttcccgaacggcaaccagtttgcagaatatgctaaccggtggacacccgataatccaaccaacgatgtgcccagggcaaagtataacaacaggggcgacgcgggcagcactacgccaaaggtaacctcccgctacatagaagatggctccttcctgcggctcaaaacaatttcgctggggtacgacctgccacccgaattgatccgccgtgcgggcttcaaaggattgaaagcatatgtggcagcgcagaatattttcaccatcacccattactccggcattgatccggaggtttcctctttcagggttcaaaaccctgccaatgcaccgggaaacactcccggcgttaccgctaccagcggcaccggctatacgtttcttcaacccagcagtagttactccgccttatccggcggactcgattatacggcttatccacgcgcctttacactcagctttggtattacggctacattctgattccatgtttaaaatgttgttatgaaaacttttcagcaattactacttccactcatatgcatactggcagcttcctgtaagatggatgtaagcctggatcctgtcaccttccgccctatcacatttaccaccgaagcgcaactggatgaacaagtggcggggatgtacaacatcctccagcaagacccgatgtatggttttggtttatggggatatatcaatgccggtgcggatgaaagcttccgtaacaacgccagttacagcaccacgctcacggagttttatcatatcagtaacactgaacagaatgttttgctgttatggcggagcttatataagggtattgaagatgccaacgtgatcctcgatgtggccgacaaaccacaaatagatgaaacaaaacgctcgcagattaaaggacaggccaggttcctgcgggcatattatttctacctgctggtgacccatttcggggacgtgccgcttaaaacaatgctggctaccgacctgggcaccaattacaatctcccgcgtacgccatcaaaagatatttatgcttttatcgtgaaagaaatggtggcagccgacagcctggtgcccaaaatgtcccaggtaaacacgcccactattgttacacaatctgccgtggaagccattctcgcaagggtgtatctttctatggccggcaatcccatgaatgacgtggcgcgttataaagatgcgctgttctgggcgcagaagctgattaattcaaacgtacatagtttaatcagctcaccacatccgctttaccccgctacccctgcctatgcccgtattttcatcaacaagatgcagaataacatgaatgataacggcacttcggaaagcatctgggacgccgctttcttatccaaatccaatgttaccggcaactatgcaggcaccgggtatcttgttacgcagcagctgggcgcagtaatgggcgtatactgccccgatgcgggcatttcgggtgtgaacgggtactctcccggcacgtaccgggtattgccgggtttatacaatctttatggttccggcgatcagcggagggattgggccattgcgccttatgtgtataaaagcgctgctaccacccgttactacacgctcaccgtgaacatcaccggtggcgggggtaccggcgctgcggccactgcttacaccgatgcacagggcgccattacttccgtagtaatcgacaaccccggcaacggctatacgactcctcccaccatcagttttactgcttacggtaccaattcgtctaccaatccctctgttaccacgcccaatgaagcggtagccactgccaccgtgagtagtggaaaggtaacggctatcaatgtaatatccggcggtgcgggttatccaacaacatacgaccgctgtgtgggtaaatggagaagggaatacgaaattaacctgccacccagccgcctccaaaacaatacttcctgcaacttccccattgtgcgttatgcagatgtgctgctgatggcagcggaagctgaactgaaagccaatggcagcgcaggcgctacggccgtggaatattataaccaggtaaggagacgggcatacggatatccgtctaacacgcctgcgccaggctttgatgtaaccacattcaccatgcaggatattatggatgaacgctcccgtgaactctgctttgaaggcgttcgccggcaggacctggtacgctggggcaaaatgacgcaggccatgcaacaggtgcttgccaacaacgacaactacgctcctaccaattatgttacgcctgccggtgtggctgcgaccaatttcctggtcgatccgcaaaagtattcactgttaccaatccccggcaatgaaatagtgctggaccaggtattaacacaaaaccccggatggcaataaaaaccgattaaacaaaatagtatgagatctattatatattatttcctcgccgctgttatgtttgcaggttgccgcagaaacgaagcaatcatgccggacttcaacgtaaacaccggccagctggcctaccaggcgggcgacactgttactttctatctctccggcaatgccggcgccattgttttcttttccggcgaaaccggcaaagcatatgaaaaccgggacaggaagttgatgcccggcgtggaaaaactcgtgttccagacatccatgcagcaaggcccggtgccgccaaagccttgcccggattcactacagctgctgatctccaccaacctggaaggatatgatgccgcacatatcacaaaggccacctggacaaatattaccaatcgcaacagcaaatggccgaagtcattgtccaccggttttacaacttctgattctatcgatatatcagattttaataaggcagataaagtgaacatcgctttccgcgtgctgaacaaaaagaccggtgtgatgccgcaaagaaaatgggttatccaaagcttttccctctataatttattacccgacagcagtaccacgcccctgtttacaaattttgccaacaccggctgggtacaggccagtttgcttaacaacagcgaaccgggaacagcggagaataactacactggcttcaacgcctggaacgtgggcacctggaacgtttccgcggccgacagtgtccggaacagcaacggcattcctatcaggaccggttatcccattacgttcaatcccggtaccaatattgataatgaagacaacgacgactggctgattacttcatccatcgacttaaaaaccaccaaacccgatataggtatggtgatacagaatgaagttgcgttgaagtcggccaccttcaaatacgcttttaacaaagcaggcacttaccaggtcacctttgtggccactaataacagcctggaagacagcaaaagccaggttaaacagctgacattaaaaattctaccctgattaaatatgaaccgatctttccttccggccatggtggcgttattgctcttttcgcaaatcctctttgcacaggtgatggcggtcggtagctggtggctgcagaacgcttcaaaagtaccgcagccgggcgcagcagtagcacaacccggcttctccgctaatggctggtatcccgccgtggtaccaggaacagtgctcaccacgctggtacataacaacgtatacccggaaccgttatatggcgaaaataaccgccccgacaggattcctgattccctttgccgcaccaactggtggtatcgcacagaaataaccataccatcatcttacaaaaataaaaactgctggctgcacttcaacggtattaattacattgcgcaggtatgggtaaacgggaaatataccggggagatacgtggcgcctttgcaaggggcatctttgatatcacagcggccgtaaagcccggagcaaccgccgccatagctgtattggtatccccacaacccaatccgggtgtgccacacgagcataccattgcacaaggcatgggcagaaacggaggcatcaccgctatggatggtcctacgttcctctgctctatgggctgggactggatacccgctatccgcgaccggaacaccggcatctggcaatccgtatatctcgatgccaccggtcctgtgcttgtaaaagatccattggtaactaccgatcttccattacccgcattaaataccgctgatgttaaaatagccgctaccgtagaaaatataacagaccagccgcaggaaggcatactgaaaggcgcctttggcaatgtagtgttcagtaagccggtagcattgccgccacacagcagccagcggattacctttgatcccgccacactgccgcagttaaaaataaaacagccgaaactctggtggcccaatggttacggtccgcaaaatttatatacccttcaactacagtttaacatcaggggagaaatatccgatgaacaacaattggatttcggcatccgcgaaatcagttacaccacgccggcttcagaagatctcaccatttccgtgaatgacgtaaaggttttttgtaagggcggcaactggggtatggatgaagcgatgaaacgtattccaaaagagagactggaaacacagatccgcatgcatcagcaggcgcattacaatatcatccgcaactgggtgggccagagcaccagcgaagacctgtacgccctctgcgataaatacggcctcatggtatgggatgaatttttccagcccaacccctccgacggacctgatcccgcagatgtgaatttgtacctcgccaacgtacgggagaaaatgctgcgtttccgcaatcatccttctattatcctttggtgcgcccgcaatgaaggcaacccgcctaaagtaatagacgattcacttcgcagcctgatggctgaactggagcccttgcggctgtaccagcccagttctacctccgggcgcggcgtacactccggcgggccttactacacccgcaaaccggcggagtattatgtttttactgaatctttcaaaacggaaatcggcagtttctctattccaacaatggagtccgtgcagggcatgatgccgcagcaggactgggaagtgatcaacgacgactgggccgaacatgacctcgccacaaaatactaccggaacatgattgccaaacggtttggtgaagtagccaacctggccgactttgtaagaaaatcacaactcaccaattatgaatcgttccgcgctatgtatgagggccgcaatgcaaaaatgtttaaccctgctactggtgttatcacctggatgagcaatcctgcgcagcccagttttgtatggcagctttatcatcacgacctggagcctaattcagccttatttgccgttcaaaaggcctgtgaaccggtacatattcaactgaacgaaaaagaaggaaatatacaggtgatcaataacggaccggcggtgctgaaaaatgcgcgtgcacatctcagcctgttcaatgcagacggtaagccggtgctgcaacaggattataatgttacggcccttcccgccgtagcaacggatctcggacaggtgcaatggcccgctgatttgtcgcccgttcactttgtaaaactgactttacatgatgccaacggcgcgctgctttccgataacttctactggaacacgcttccgttgggatcagaccagctggcgggcctggaaaagataccagtggttacgctcacggcaacggttaaacgccgcagtgtgcatggcaactgtttgctggatgtaagcctgcataatccatctgctcatatcgcggtaatgacgcacctgcaacttcaccggcaaggtggcgacagggtgttacctgttttttattcagataattatgtttccctgtgccccaacgaaacaaaaacaattaccgtagaagccagtgaggccgcccttcagggcagcaagccaatgatactggtggatggctttaatgtaaatataaaagaaagcaacagtcccgatgcagccattgcgctgaatgaaaacgcgcaggtgaaccattggcccattacccatttgccgcggcccgacagtaccgcaccaaaaaaataaaagcatgtttacatcaagacgggaattcctgaaaataaccacgtttggcagtacaggtttgttattaccgcctatctctgcatgggcgggcgtttataaagatgaactggcaaccctgagtgaacagctcctgcaacaatggggtgaaagtttactggcgctacaggtaaaccaaccgcaggcaaaaggattgcatggcggcattctgtgccccgcctgcgccaccatacacggccgctgcggtgatgccattttcccgttattatatcttgccagtaaaagaaaagaacaacagtatgtagatgcagctatccgtttgtacaactggatggaacacatggtaagcacgcccgatggcgcgtgggtaaacgaagtaaatgtaagcgactggaaaggcattacggtgtttggcgctaccagtcttgcggaagcgctgattcattttgaacatttactggacaaacccacagcacagcaatggaaaaacaggttacaaaaagcaggtgactatctctataaaaactttactgtgaacaccggtaatatcaactaccctatcgccggcagttatgctttgtgcctgataggcacctatctccaacaaccccattttattaccaagggcaaaagcctggcaaaggattgcctcgcctactttactgccaatggcctgatatacggggaaggaaaaccggtgcccgagaaaagtggaaaaggctgttattcggtggacctcggttataacgtggaagagtcgcttccctcttttgtgctgtatgcaaaattggtgaatgacaccgccctgctggatcagttgacgcgctccttaaaagcacacctggaatttatgctgcccgacggcgcctgggacaacagctggggaaccaggaactttaaatggacctattggggcagcagaaccagcgatggctgtcagcctgcctatgccctgatggccggcagcgaccctgcattttacaaagcagccttgcaaaacacccggctgctggcgcaatgcacgcacaataaattattgcatggcgggccgcattatgtacaacacggggtattgccttgtgtaagccattcgctggcgcacagtaaagcattgaccaccgttttgatccaggcgtcttcaataaaaagtagtacagctccgctcccacgggaacgcatatacggggtgaagtcatttcctgaaatcaatacctggctgatctccacgcataaatggcgtggcaccattacggggtacgaccaggaatattctatgaagggcggtcatgccagcggcggtgctttgtctatgctctggcatgaggataccggtcccctgcttgtggccagtatgaaccggtatcaaatggtggagagctttaacatgcagcgggataatgatccgttgcctgcttgctttacgcctggctttaccataatggccggcgaacagctgtaccggcacaccaatgatctgaaagccgctgttgaatatcatgaaagcaccgggcagataaccttcaacacccgttcattactggtagatgaaaaccagttaccggctgcttcaccggaatgtacgatcagttatctttttgagaaagatgtgtttcatattcacgctactgcgaaaaatgaaaaggccgtttatagtttgcctgttatcagtacgcacgacgaacccgtcacacttctttcagaaaataagctggaaatacgcaaagcgggtagtattgtggagataaccgccagtgcgcccataaaaacaacccgcgcattaacagaccgcgctttcaattttgtacccgggctcgaagccgttccgttactctttgaaacgaataatatcgatataaaaatttccgtaagaccacacacatgaaaaaagcatgcttactgatcagcgctgccctgtattttgtgatgcccgcaatggcgcaagccaggttcgatatattcagggaacaggccatcactgatgttagcccgcagggatggctgaaagaattcctgctccggcagcggagcggtcttaccgggcatccggaagtattatcgtatcccttcaattcctccttatgggcgggcgttatagaacgggtgggcgaacagcacggcgccaactggtggcgatacgaacaaactgcctactacagcgatggtatactccggttgggttatttgctgcgtgatacagcgctggtgaataaagcccgcgccggtattaactacacgctggcacacgtacaatccaatggccgcctgggtccggagatgttcaccagccaatggcctatcgctgtatatttccgggtgttacaggccgaatacgcagctaccggcgatcagcggatcattgccgccctgcataaacattacctgagctatatgcccgaagaaataggcaatgccaaacgtgccattgtaaacattgaaggcatgttgtggacgtatggcaaaacaaatgattcccgactgctggcgcttgcggaagcggcttatgccaaaggcggttttgagctgaacatgcaaacggcttcttcgccggatacgctggtgctgcatggcgttacctatatggaaatggctaagctgcccgccatcctgtatacttacaccggtaaaaaagtatatctcgatgcagcgctgaatgccatgtacaaactggatcgcgatcatatgttacccgatggcatccccagctccaacgaattcctggcagggaaagatccgttacagagccacgaaacctgcgatatcaccgactatacctgggcagtgggttacctgctgatggccaccggcgacggccgctgggccgataaactggagaaggccatcttcaatgcaggtcctggtgcggtatccaaagattttagaaatcttcagtacttctccagcgttaaccaggtgatcgctacggggcagtccaaccacaataaatttgcgcacggctctacctggatggcttactggccctgtcatgaaacagaatgctgcgccggcaacgtacatcgctttatgcccaactacgccgcgcggatgtggatgcgtgataccacaggagccccggtggcagcactttacgggccttctgttgaaacgctccgctacaaagggcagccactcagcattaccgaaaacacgcaatatcctttctctgaccagttgcagttcaccttccggatgcaacaggacatcactatgccttttaccttccgcatacctggctggtgtcaatcagcgatggtgagcatcaacggaaaacgatacaacggcgcgttaaagcccggctcctttgtaaccctgcaccggaaatttcataacaacgaccggatcagcatacaattccctatggcgccgcaactggtacaatggggccagtggggcgttgccgtggaacgcggcccgttgttgtacgcttatcccgttcccgaaaaagtaaccacagataccgccacttacgctaaccttggcggcaaaaaatctgcagatcctggtttcccggcgctggacatccgtcctgcgggtgactggaactacgcactgctggcacgtcccggacaatggctggtaacagaaaaacaggacaatacttatccctttgacgccgccgctgttaccattaaggtaccggccaggaaaattaacgactggcatttatcagaaaaccgctacacgcccccattacccaaacccggttctttccactatgaaacaactaccgataccatcaccctggtgccctatggtattaccaggctacgcatgacggtattcccggtgatcccttaatacattaaacccttgtaactatgactatcacaaacatctcccttttagaaaccacagcgggtaccaccgccaatgaacattgcaatctgctcggctattatgcgcccggcgatggcggcggcggagacttttactggcaacctgccaacaccaccggtgataaccggggcaccatcatcgttgttgccggcaatggccggtggctgcgggcagacaccaatctctttaatgtaaaatggtttggtgcaaaaggcaacgcctccacggatgataccgccgccattcagaaatgtattgataccgccgccacgggcaggatcatttattttccaaaaggaaattataaaataaccgcgcagatcaatcttaaaacaggacaaacctacaccggcgaacaaggcgactatggcattgtagattctcctacgcctaccattcttgactttaccaccgccaccggtaacattcattgtcttagcttcgacgccaccatcggcgctaccggtcccactatcaggaatcttacgctcaattgcggcgaagcccttaccggcatccggtattacagtaccaactattccaactgctaccgccccactttgcaaaatgtagacatacggttaaaagaaattgcagatcctgcgcaaacatgcgtgtggtgggagccagtgtacctcggcaccatcgacaggtgcctgctccgcggtggcaggataggtataaagctgatcgggtgtttcatgaaccgcatcatcaatgtaaccacgcaacagggtatttacaacaatggcaatccgcctgtggcggccatttacacccggcaaaccagggcaggcagaacaggctcctatataggcggcaggaacttaatagaaacatccgaaccgctcatcatttcgcccgatgctaacagcgtaatgattgatacggatggcgggctgattatccgcgacactgctatggaggtgaacaacggcagcagcaccggcacagccgccaaagcattgatatggttgcataaagatggtacccagtcgcctttccggtcggacctcctgctggaaagaggcgctgtatttaatactgccgcggctaccggcgccaacaacggcagggcccaatacggcatccttgcggaagcaggcatgtttacccggattgtggccaggggtgtgtcttttaaagataacccgatcgtgatcacaaatgccggcaacacggggcttgccacctccggcaccgacttccagcgactggatgtgcaaggcaacgactacgctacggcgtattatacggagtatgccggatggaagcccgctacagcctatgctatggggcaaaccgtacaaaacgggttgtatgtttatatcgtaaccaccacaggtatctctgatgccgcgggaggcccaaccggaaccggcgccggtattactgacggaacggtggtatggagctttgtaaaagaaaacaccggtccgtttcctttaaaacgctaccgcgaaaccaacaacgacgtatacattgtgggcgatgccaggggcgtgaaagataaccagttcattaacgccaacggctctacggagcggttcggtgcggcctggggattctttaaggcaacggtggatcccggtagtatcagcgataaccagtcgtgcataaaactgcgatacgacaacgccccgccttataacacgcccatgaaagcaacagtgacattacgccggctggcagcaggcgcttccgcgggcaggttcagcatgcagtgttcttccagtggtggcactaacctactaggaagatgggatttcaataacatcccgctcaacgaagataaacagtacgtggtgaccggcttcgccattccctccacgatgccggtggcagacttctccgcctggttccgggacagtgccagtcagccgctatgggacaacatcgccgtaagatcggtgcgcgtggaaaaagctaccaccttttgcggcagcgttaccatcagtgatatggctacttctgcagatgtaaattcatccagcttccagagcagcgatattacgctggtcagcgttcctaactttttactgcccgacaccgcaattatctccctgggcctgcccgcggtaacagccggtatgccgttgctgctcatcaatactccttatatcagtaacagaaccaccagtggttttactattaacctgtttctcaaaccaggtgcaggcaatagtattaccataccatataccatcacctattaaaccattcaccaccctggtggtcatagtatccgttaaaccattcaccacaggcgggccctgcctgtggtggataattttccgggcgttcacccgttttaagaaagaatctgtctataacatttatataccagcgcgcaggaaaaaagaatacaaatggggaagcaatcaattatccggaatacgctgttagtcatgttttggtgcagcagtcatttatcggccagcagtcagggtacacaggcatacgaccctgaaaaaacctatgccgcgccaacagacgaccgggtgaaagctaaattatcacattggcaggacctgaagtttggcctgtttatgcattggggtacctacagccagtggggtatcgtagaatcatggtcgctttcaccggaagactatccctttaccaaacgtacaggcccctatgcagcaaactggtttcagtataaacaggcgtatgaaaacctgcaaaccactttcaaccccgtgcactttaatcctgataaatgggctgacgccgcaaaagcagccggtatgcgctatgtagtgtttactaccaagcatcacgatggcttctgcatgttcgacaccaggtacaccgactataaaattaccagcgccaaaacacctttttcatccaatccgcgcagcaatatttccctggaaatttttaatgccttccgtaaaaaagattttatggctggcgcttacttttcaaaacccgactggcactcggaagattactggtggtcgtattttccgcctaaagaccgccaccagagttacgataaaaaacaatatccggagcggtggcaacggttctgcgatttcacgtacaaccagatagaggagctgatgaccaactacggcgcattagacctcctctggctggatggcagctgggcgggcatcaatatggctcccattgtaacaatggcgcgcaaacaccagcccggcctgattgtagtagaccgccacggcgcggcggaatatgtaaactacctcacaccggaacaaaagatcccggaccactacatccctgttccgtgggaaacctgtatgacactgggccggtcctggtcgtacattgtaaaagaaaattacaaaccatcgcggcagctgatacaaatgctggtggacattgttgctaaaaacggtaacctcctgctcaacatcgggccgggtcctgatggcgactggcacacagaagcctatcagcggctggccgatatcggcaaatggatgaaaataaacagtgagtctatttacaataccaaacctgttgctccttaccgccaggataaatgggcttttacaaaaagtgaaaaagcccgttatctttcttatctcccggcggaaaaagaaaatatactaccggccactatcagtgcacctttgaaagatgtgagccgtaaaaccggtatcaccctgctgggtacagaaaaaaaactgacatgggagcaaacgggcgattccatcaccatcagcattccagaggccgtgcgtaagcagctggccggggaagccgtgtgggtatttaaaatgagttaacgatatagatatgtcgataagattgacaggtgtagtacttctttttttactatcgctatcactgcatgcacaaacggattcgcttaacgccatgcaggaataccgcctccgccagggtttacccaacttctttgcgaaattgaaatccggcggtccgcttaccattgcctattttggcggcagcattaccgccgcctccggcggctggcgcgatcaatcggtgaaatggtttcagcaacaatacccgcaggcacaaataaaacagatcaacgccggtgtaggcgggaccggctccgacctgggcgttttccggctccgccgcgatgtgctgtcgcagcaaccggatcttgtttttgtggaatttgcggtaaatgacggtggcccgtatgtacaccaaacaatggaaggtattgtgcggcagatatggaaagtcaatccgtcgacagacatttgctttgtatataccatgtcggggaatatgttaccggtgctgcaacagggacagctatggcccaccatgctcgccatggaacatattgcgcagcactatggcattccttccgtacaacttgggatgcaggcattggcactgttgaaagaaggcaaactggtgttccaggggaaaccggatcagtacccggacaaacttgttttttccggcgacaatgtacaccctaacaccacaacaggtcaccgcctgtacaccgaagcgctggtgcgcgccatgcagcagctaaggaccaacgaccatccgctgaaacacacgcttattgctccctataccaaagataactgggaagatgcacagctggtggctgtgaaagacctgccccgtaccgggcagtggtctgatctttccaacagtaacgacaccgtggcggttcaattccgccagcgctttccattgcttgttaaatcgacataccccgggtcatcactgcagataaatttcaacgggcgcctggcaggtttgtacgacctggtgggccccggatgcggtgaatatgaggtaacgatagacggacaagccgccaaaccgtatccccgcttcgaccgtcacgccgtgtactatcgcacgcattactttttcctgccgctgctcgaagcaggaccgcacaccatcaacctggaagtatccggtaaaaagttagataaaatgtccatcctgaaaacaggtgataaccagcccggcgacctggaaaaatataatgaaaatgcctgttacgcaggctggctgctgctattgggcagtatcaccaaccagcagcaataatgaagcgctccggcatccggaaataaaaaataaatgagggaaacttaacaaagagatattaactttaagtacacgttatagagatttttaccacgttaataagtatctcttcatggataataacgacgacgggcttttattgcatcaactccggcagggtgatataaaagcgtatgaacaattatttaagaaatactacaaatcactgaatgttgacgcttactacctgttaaaggatgaaacagaagcggaagatcaggtacaatcccttttcatcgaaatatgggataaacaactgtatcttaacattacctactccgttaagtcgtacctccacactgctatccgtaataaatgcctcagttttattgagaagggaaaaaatgagcataagagatttcatgcgtatgccaatacactggaagataagatcaatgaaaatattgtagagaataaagagactgcacaacagatggaccttctcctcaatgagcttcctaaccagcgcttacgggctttcagcctggtttacctggaagataaaaagtataaagaagcggcagaagaaatgggtattactattaactctgttaaaacgcatcttaagctggcactaaaaatcttacaaaaaaagtttgcgggctacaaataacgatcacccgtttttgcgcaaaaatcgtctttaagttacagatggaagtaaacagagaacatataagagcattactttttgaaaaagtaaccgggtctatcagcgaagaagacaaccggctggtgaccgctgccattgaaaatgatgcggcggtagccgatatgtggcataacatccgggaggaactggacaatgataaaagccggcgcttcatggccggtatcgatgaaacccggggctggaacaacatacaaccgcaactgcgatcgcattcaaaagtattcctgctacggaaatggcgtgtagccgcagccgttgtattgcttattatagctgccggcgggatctggtatttttccggcagaaatatttcttccgggccagcaactttaccactcgcccaaaacacgctgctgctccgcttgtcggacgggaaagatatcccgttgtctgcttccgccggcaacaccattacggcgggtgctataaaactggttaccagcggcaaccgtcttacttatactgcgccggaaaatgcagcagatgaatgggccacgctgatggtaccgggaaaactggattataaaatagttttgaaagacggaacggaagtctggttaaactcacagtccagcctccgcttcccctatgctttcaagagcggtaaccgggaggtatacctgtctggcgaagcctattttaaagtagcaaaaaatgagcagcaaccttttattgtgcatgccggtgaaacaagggtggaagtattgggtacctctttcaacatccatgcctacgaccctgcaaaggttaccacgtctcttgttgatggggcggtagtcagcagcaaagaagatatcaaagtaaaattatctcccggttatcagtcggtatatgaagacggaaaatttgttaccacctcttttgatacctacaataccctgtcgtggatggacggcaccacccacttccgtgatgaaaaattaagcagcattgccgtgatcatctctcgctggtttgaagtgcctgttatattcgacaacccggcactggccaacgaaacgctgtccggcgctatcgacaagcgtaagccattggatgtgttcctcactaatatcgctatttcctctggtgttcagtactattacaagggtaacgtgctgcacctgaaataattcatttttaccgttcacccatatccgtagaatttaagtcctaaagatgcgttgtatatgcagcacttaagttttactattttgaacaaccgtatcattgcttcttttaccgccctcctggtctcccttgcaggacatgcgcaggacacgcttcgactgagcggttcctggaaggtacagcccgcacaatcgcagaatattgctcccgatagcagcaaatggggcactgttgccgccaccgactggagaaggatcacctccggtaaaaacagcgcctgggccgacacgccgcaggataaggtaaacagtttgtggtatgagcagcaggtaaacatcccggctgactggcagcccaaaaatgtgatcgccgacttccggcggatagagggcgacgctgttgtatttgtgggccagcagcgtgtaggagaagtgctccggcccggtggtgaagtaaacctgggtccattcctgcattacggacaacccaacacgctccgtgtttttgttaccagggattataacggcatctcccggggctttacagaagatccgcttcgttatgtgtcgaggcacggtgcgggaaacatcattcccatggcggattggccaatgggcatcacggcgcctgttacaattattgccagggcacagcaggccatcatcgatgtattctgtattacttctttcaggaataaaatgctgacgcttgaagtagaggtggatgccaaaaatgtaagcggcgcctacgacttggaggcggagatcattgatcagcatagtaaacgggtactcactctttccaataaaacaatgcagctgataaatgggaaacacgtgtaccgcctaacggccgcatggcaaaacccagtgtgctgggaactggatagtccttacctctacaaggcaaaagtggcattggtgcagggcggtaaaacgctttgccgttacccggaagtgaccttcggtttcagggaaatatggactgccggcaaccagctgtttatgaacggtcatctctcgcgctggcgggttacagatgtgtatggcgcgaatcaatatggtttgtcgctttaccggctgattggctacaacgttggacagttccagccgcatcataaactgtggtggctgaacgatgcagaaacgccgctccttcatgaagacatgctcgaggagatggaccgtacgggcatgggctgtactgtgccaggcccttctgtttccgtgctgcgtgataaactgctgcatgatccggagttgcagaacgactatcaaaaagaagctgcttactttacccgtcattaccgcaatcaccccagtattctcgcctgggtgatagctatgaacagcgccaatccaaaatcaaatattgatccggccaggatggggaaacgcgattccgtttattccacgcaaggcaaggtgatagacctggcgtgcagcatcgtgaaaaaggaagatcccacgcggctggtgtttgcgcatgccgatggcagcgtaggcgacatgtcgtccgccaacgtgtacctgaattttgtacccctgcaggaaagggaagaatggccgatggcctgggccagggaaggtaatatgccttattccgccgttgaattcggacctccttactggaataacttctggaagggaaagcagttcctgctcacggaatatttatccatgtacctcggtgatgccgcctatgccactgagggagaaaaagggctgcggcaaacgatagaaaaaagcaatgctgccagcagcgctacctgggaacaaatggactttcaacagtatcccggtttctggcgcttccaggaattatttacgcgcaataccaaccgtgcatggcgcacgtggggcgtcaacggaggctggctgtactggctgctggaaggctatggcaatcccaacggggaaaaactgaaaagcttcacacaacgttacaaatcactcaccgctccacttaccggcaaaccttcatgggccaacccacgcttcgatattttcaaggaggccaatcagccattgctggtttacctggccggttcgccggcgcacaccgataaaacgcataccttctttagcggcgaaacttttgaaaaagcggtggccgtagtatgggatggtcctcataaaataacgccggaagcaaaatggatgcttaaacaaggcgataaagtgtttcagcagggatctgtatcattggcggtaaatggcggcgaaataaagcagtttccgctttcgctgaaagcgccgcccgtaactgtccgggcggacatgcaactggtgcttgccgttgccggggtgcctaacgatacgtttgccctcactgttttcccgcggcccgcacctgctgtggtgaaagcaccggtgttgctttatgatcctgcggggaaatcggcagcatcactgaagcaattgggcatacaatattctgcatgggagaaaggtcgccgtatctcctctgatgccatactggtgataggccgcgaggccctgcagccgggggacacgctgccgtataatgaaaaagatattgcgcgcggtttgcgtgtgattatactggaacagtcacctgccgtatgggaaggtatgggttttgaaacgatagaaaccatgccgcgttatacttttatccgtgaccgggaaagtgcgctcctggcgggattgcagccggcagatatgatcaactggcggggcagtcccgacctcttaccggaaggcaggcaggtaaaaagctacgacacgcagcatgcgccaaagtggaccaatcgccatgcggttgcttccgtagtactgaaaacccctgaagtggcgggcttcacgcctatcctgcaaactgaatttgatatggcgtacacgccgttgctggaatggcggtatggcaaaggcaaagtaactttttgttcactcgatcttaccggccgcgttggcactgatccagcagccacactgctggcaaaaaacctgtttacgtcgcaggcgccgtcgcttcccggtttacgcgaggtatattatagcggcgacagcaccggcaggaaactgctcaccgatgcgggcatcgccctgcgggaagtccccggcgccggcaatgccatatgggtatttggtgcaggcaaaacgaccataccgccccaggtcaaggcatttgttgccgccggtggcattgcattttatcttccacagcagccatcatttttatcacagcagggattaaatacgatcgctaaaactatcgtacatgcgcagcctggaaaagccggacagctactcagggccatcggccccaacctgttacggtggcgggataccatacaggtaaccgcgtttacttcatcctcattatgtgacgggcttctttcagtaataaacaccggtaagggcaaaagcatctatctgcaaataaccccggatcaactggcgcaacgttatgcaaatgctcctgagaaacaggaagccgtccggttaagtgtgatccgcctgcatcagttgacagcacaattgctcaccaatcttggcgctgctccttcccctgcaactgcccgcaggctctgtaaggtaaaccgcccgctttctttccaaacactcagctcctggaaagtgctgggaccttatactgccaatacatccagcggcgcgaaggtactggcgactacttttccggggcagcaggatgctattgccggcgcggagaatccgaaccttacttataaaacagcagagggcaaagtgctggattggcggcaaacggtgaatgccagtcagcatggctttgtagacctcagtaaagtcttcggcggcaaagacgataatgcggtagcgtatgtaaccaaaagtatgaacagcccggtggcacaaaaagccattcttcgtatgggcgttgactactggatggaagtatggctgaatggcaaatccatcctgcgtgtagacgctaaccaccagaaaagggaaaacgaatttatcctcccggtttctctttccgcaggtgaaaatattctcactatcaaagttgcctccggcaaaggcgggtttggtttctgggctaatatggcgtatccggaagccggcgaggcgcaaaccaatgcaacggaaggagacagtttttacccggtaggatatcgtttctttgatccttaccagtttgtgtactggtagcatcttttttgccggtataacgttcagccttaaccctgcttccggtttaagaaacaaaaagcctccaggttctataacctggaggctttttaaatgatctcaatgcactacttagcttaccattggcaaatacttcttccggttttcaatgattacccagatattaattgccagcatcacaagtgcgataggcagccctgaaggagcatataagatatttgttaaaacaattcctaccattaccgggagaataactattgcgccaagtgccctggttttattaggaatgaaaagcgcaccgcctatcacttcagctgctccaacaagcggcattaaccagcttatctgcataaaggcgcccattaacttcatcatgctttcaggcatgtctttgggtaccggcatgtagttaaagaatttgttcagtcccgcgttaataaacataagtccgaaaagaagacttacgacaaataggattttgtttttcatagtttttattttccgtaaatatacatttcatttttatctgctgtatatccgcaatatgagttgtggagaaattctatttttttaatgatggcaacagttcgtccaatccttccatagccattcccagaccttctttgaaacccatttggatggttgcttccagttgagcaagatcggcataagagatgtgcaattgcaccagtgttacggcccctttgtcaacaaaggtgacgttccattccgattgcggcatctctttattgatatttcctgctgcatctgcaaaagcatcaagccccgtgaattttttctggacctggatgtttttgtaggtggccaatgcccaatgttcctcgccttccgggcccaccatggcataatgccaatgtccgccttctctgaagtccattgtttttgttctggctttccagggttttggcgcccaccagaggtcaaggatttcgcttttcgtataggcgtcccaaaccaaaggaagttccgcggcaaattcccgtttaacggtgatggtgttgttctccttgtttacagaaaaatcaaatgataagttcttactcatttctttttgttttttatagttaacaatacttggtctagttcattaaatctcccctcccataattccctgaattgcccgagccatttgtcaatttcctgcattttattaccatttagctggtagaaaatttcccggccggattgttcctgtttcaccagttcacattccgtcaggatgcgcaggtgtttcgaaacagcctgccggcttatttcaaaatgttcagctatggcgttgggtgtcaatgcctgaaccgcaataagtaatatgatggcccgtctggtcgggtcggcaatagcctgaaaaacatctcttctcatttctccgtaatttattcatgcaaccgatcagttgcaaatataagcaactaatcggttgcgcaaaatatttggagaattttttttggcgggaaaagagaacaggtatcaggtgaaaaagtaaatatcgcttccaacaagttgattatcagcagaattcaatcttgataacgcgaattttatcgaataaaaaaagccggtctgatgaccagctttgggaaaccaaccgaatattttacttgctttttaaccttccatcatttttttcagaatccccagcgtaccattccaatagaaattcaaatgctggtatatagtctccgtggggaaattagtgagtgtaagcgacaacaaagtatgctcctcctctggcgccagtgcaaaccggataacggtatagttctccctggcatcgggcaaccgggacaatgaacttaaaaagtcgtaactcactgcatgttctggtgaatattccagcaccgttcccttgttctcaaactttgcatgatgaaagccgctgaccactaatggtgatcccacttcccaggtagttgcaacactgagatttagctctgcacctcccatccattgtgtcattaacttaacatctgtaatggttttccacacctttgccacgggagcattgatcattatttttctttctatcattttttccattctttgagatttataattccggaggaaatcaccgtataatcatttacgtcatatgcgtccttcgaggtaggtcagcgttcccacctatgaatttagctaaactttaaatgcagccattaaaaagtttgtgaggatacaaaaaattgaatagctttaaattcaccagcaactattcctgatgatggcagaagaagactacgaagacgaagaatcctgcacacggaaggaaaccttccggggaactatacgggccttaaaacaaagggcaaaggacaacagcattatagtaacccactcccagatcgctgaccggttaaatttgtctgtagagcagtttaatgcttactatgtgagtgatgaagcgcccgaagaactgtttccattacttcgctcacaatacccggattttatcggcaacgtaactgtcgagatcataagcttcaccaccatccattaccctccggatccgccaacccctgatgtagcataaggcattgatcagaacgcatgataacgcattcctccatcaacagtggcaacagcaccagtaacataccctgcacggggcgacaccaggaaaacagccatgttggccatgtcctgtggtgtgccaaaatcacccagcgggatttcgcgctccgcaaatttccggcgttcctcgcccggaaagtagggccgtatattttctgtatctattaagcctggctgcaggcagttgaccctgataccatatttccccagttgacccgaaagttgtttggaccacgctaccaccgcagctttggctatcgccgacacattgatggtgcgtaattcatacgtgctgatcaggttcaggatggccccctgcttgcgtgctataaaatggggcaacagctgttgcgttaattgccgctggcgatcaaagtccagtgtcatcgactctacccacggctcctccggcccaacaacatccaccggccggctacggcccgcattgttaataagaatatccacgtgccccaaaatggacaacgccgcggcggcaatcttttgtggcccgtccggcgcaaccaggtcctggacaaaaatgaccggctccatgccacctgcccctgccacttccgctttaaagctatccagcaacgcttcgtttcttccaacggccaggaccctgactccttcaatagccagttcttttgcaattgcccggccaattccctggctggcgcccgttactactgcggttttcccgcttaaatacagatccatatttttagattaatctttgtaaaactcattttcatacccaaaaacaacggctgaaaatttctttgtaaaagtagcgggtagcatctaaatttacaggctatacaaccaattgtacggtactaacaaacgtgtaagtaatggcaaccagaaagaaaaactcaacttatagccgcaatgaaaacatcattgtggaatgtgatcttacctatgccgtgaataaaatcgggggcaggtggaaaattcttatcctggataaattagcggagaagaaaatgaggtttagtgaattgaaacacgagttctactacattacggaacgcatgttaaccctgcagttacgggcaatggaacaggacggactggttaaacgaaccgtatatgcggaagtgcctccacgggtggaatatgaactcactgaaatggcattggagttcggtcctatctttaaacagctaagtgcctggggaggcaaacaccgggatttaacgaagaaagatattgtataatgggactggacagcattgacctattggtcgaaattgagaattatttcggcattcagattccggatattgaagcggcggaaatctttacggttcagaatatggtcgatgtggcagcgaagcatttgcatgttgctgatcatgctatggatcttaaagcgcaggtctttcaacaggtggctgatagtatctcatcaacaaatcatgagattaagctgaccgacaaaatctccacctacctctctcctggtgatcaaaaaagctggtcagctttaaaaaaccatctccggcttgaagtaccccaacctgatatttttgcccgcgcaccgaaatatgattggactaccattaccatcgatcaattcacaacctccatatgcgcccgcaacttcaaaacgctgattgataaaaatgagatcaaaagtaaatatgaagtatatgttatcgtaatgggtattaccgttgccaaaacaggcgttgactactatgagataactcctgataaatcttttacaagtgacctgggcatcgattaagatgccgcccactaacggcttccgggccctccgggaaatacattcatataattaatcatatttgataaaaacacctcaaacgaaaaataacagtttcttcacaagcaaaacctcatgattttttcgtttgctctcaaagttttattacttttggcccccaaatgagagtagctatatttttcgcatatctgtgtttcctcctgctccggggggaaggctatgcttttacagctacccatcataacgatatttccaactctttcgccaggaatgttgaacacaaacaccggattaaatttaccgacaccaaccaggataattctgttgtcagcaatttagacaatgaagaagaatgcctgataagtgatgacattgaagaggaagatgcgaataattttctggccagaaaatataaactgctggccaggtattacctgacactccccgacctcgacgttttaagttatctccataaatgctttaaagcccccacaccttatctggggcatctttccaatagatacattacgcaaagcgttttaagaatctgatcaatagtatacatcagttaccgagggtgtgattattcatgcctggcggatgtatattcattttacttcctccgggctcccgctccggcgactgatccttttgcgtccataggcatccctgccttacaagcatcccatcgcttaatatccatttaatattatgagtagaattgtcatgtttacgggcttgtttgtcatgttatgccatacaagctgtaaatcaaaaaaagaagtaaaagaagaggcgggcaagtttaccgttaccagcccggtaagaatcgacacttcatttaccaacgaatatgtttcgcagataaaatctgtcaggaacatcgagatcagggtccaggaacgggggtatctccagaacatctatgtagatgagggccagtttgtaaaagcaggtcagctgctgttcaggatcatgccgaaagtttatgaggcggaactccagaaagcagaggcagaagccaaagcagcagagatagaactgcagaataccaaaaccctggtcgataaaaatgtggtgtcaaaaaatgagcaggccatggcgcaggccaaacttgaccaggcaaaggccgaaatggcactggcgaaactccacctctcgttcacagaaatcagggcgccgttcgatggcaccattgaccgtattccattcaaactgggaagcgttatcgatgaaggtggcctgctgaccagcctttcagacaacagccagatgttcgcctatttcaatgtatctgagccggaatacctcgactatgccaccaatgcaaaaggccgcggaagcaacaaagtaagcctgctgctcgccaataaccagcccctccaatataaaggagatgtggaaaccattgaaagtgagtttaacaatgaaaccggaaatattgccttcagggcaagattcccaaatcctgacaagcttttaaggaatggagaaacaggcaaagtgctcatgaccattccgcttaaaaatgcattggtcataccgcaaaaggcaacttacgaaatccaggataaattatatgtttttgtggttgacaaaaacaacatggtaaaatccaggaacattgccatccgtgggcagatgcccgacatgtacgtagttgaaaacggcatttcagaaactgataagatactgctcgaaggtgttcagaaagtaaaagatgatgataagatcacctatgaataccggaaacccgaggaagttatttcccatctgcgattaaaagcggaatagttcaatctaatagtgtagatcaatgcttaataagtttatacagcgaccggttctgtccatagtaatatcgctcattatcgttttcctcggcgctttagccatatctcagctaccggtaacccagttcccttccatatcgccgccaaaggtgaatgtaaccgcggaatacccgggagcgaacggtgaattgatgatcaaatcagtgatcattccgctggaaagggccatcaacggcgttccgggaatgaaatacattgcctccgatgcgggtaatgatggagaggcttctatccaggtcgtattcaacctgggtaccgatccaaaccaggcatcgttgaatgttcaaaaccgcgtggcatccgtagtgaacaaactgccgccactggtcgtacgtgaaggtgtaaagatcacccgtgaggaatccaacatgctcatgtacatcaacctttacagtgatgatccgcaaacggaccagaaattccttttcaatttcgctgatatcaacatcttaccggaattaaaaagagtagatggcgttggcttcgctgacattctcggtaaccgggaatatgccatgaggatctggctgaaaccagaccgcatgctggcttacaaaatttccgccgacgaagtaatgaaggcactgggtgaacaaagcctggaagcatctcccggtaaaaccggcgaaagctccgggaaaagatcccagacctttgaatatgtgctgaaataccccggaaggtttacgaataaggaaggatatgaaaatgtgatcctccggtccagcccgaacggcgaaatactgcggctgaaagatgtagccgacgtggaatttggcagctctatgtacgatatctattccaacctgaacggcaaaccttcggcggccattgtgctcaagcaatcgtacggaagtaatgccagccaggtgatcaaggatgtaaaggccaaaatggcggagatcaaagccaattcgtttcccaaaggaatggattatgaaatcagctatgatgtatccaaattcctcgacgcctccattgaaaaggtaatccatactctgctggaagcctttgtgctggtaggtttggtggtattcctgtttctgggtgactggcgctcgaccctcattcctgctatggccgtaccggtgtcgctcatcggaacatttgtattcatgcagtttttgggtatcacgctcaacctcatcacgctgtttgcgctggtgctggccatcggcgtggtagtagatgatgcgatcgtggtaattgaagcggtgcatgcaaaaatggaagaagaacacctctcaccgctgaaggccaccaaaaaagccatgcatgaaatcgccggcgctatcgtggctatcacgtttctgatggcagcagtgtttatcccggttgcattcatgtcgggcccggtaggtatcttctaccggcagttttccatcaccatggccaccgccattatcctgtcgggggtggtagcgcttacgcttacaccagcgctttgcgccatgatcctgaagaatacacatggagaagccaaaaagaaaaatgcgctcagcaaattcctggacggctttaataattcattcaaccgcacctccggaaagtatcagaaaatactgggtgtcatcgttaacaggcgggcgctcacctttggtatactggtggctttctgtgccggaatatgggtcatgaataaaacggtcccttcgggctttattcccaacgaagatcagggaatgttctatgccatcatacaaacgccacccggatcatccctggaaagaaccaaccagattgctgaaaagctgcagaaaattgctgaaggcgtggaaggcgtacaatccgtttcttccctggcgggttatgaaattcttactgaaggaacgggttccaattcgggcacttgcctcattaacctgaagagctgggaagacaggaaacattctgtccaggaaatcatcagtgaactggaagaaaaatccaaagacatcacgggcgccactatcgaatttttccagccgcctgctgtgccgggctacggagccgccggtggcttcgaattacgtttgctggataaagccggatcaggtgattataagaagatggaaacagtgagccgcgactttgtgaaagaactgggcaaacgcccggaactgtcgtctgtattcagcttctacagtgccagcttcccgcagtatatgctgagaattgataatgatatcgcgcagcaaaaaggcgtcagcatcgacaatgccatgaatacgctgtccaccctggtgggcagtaactacgaaatcagctttatcaaattcgatcgccagtataaagtgatcgtacaggcatcgccacagtacagggcattacccgacgatatcctgaagctttacgtgaagaacgaccgtgatgagatggtgccgttttcggatttcatgaaaatggaaaaggtgtacggcttatcagagatcacccggcataatatgtacaacgcctcggaaatcagcggcgccgccgcaccggggtacagtagcggtgaggccatcaaggtaatcaatgaagtggcgcaaaagagcctcccgagagggtttggaatcgactgggccggtatttcaaaagacgaggtggcccagggcaaccaggccatctatatattcctgatctgtcttggtttcgtatacctgatcctggctgcacaatacgagagctttatcctgccgctggcagtaattctctccttacctcccggtatcttcggcgcattctttttattgaaatgcctgggactggagaataacatttatgcgcaggtagccatggtgatgctcatcggtttgctgggtaaaaatgcggtgctgatcgtggagtttgcggtgcagaaacaccgcgcgggggaaacggtgctgaaagcggccatggaaggatcaaaggtaaggttccggcctatcctcatgacctccttcgcgtttattgcagggctgatcccgctggtactggcctccggcccaggcagggttggtaaccgtaccattggtaccgccgctgccggaggtatgcttttcggaactattttcggcgtgctgatcatacccggactgtactacatcttcggcagacttgcagaaggacatgcacttgtgaaagacgaagaagaaaatcctttaacagaagaaattgataacaatgtataaattcaggatacatagcggcgttggcctggttggtatctgcctggccatcgccagttgcagggtgccggccagcctgccctcggctgagaacaggtccgttcccgggtcttataacggcaacggggatacgacaaatacggcagctattgaatggagaaactttttcaccgataaaaacctcgcggacctggtagacactgcgttgaaaaacaaccaggagttgatggtcaccctgcaggaagtggaaatagcgaggaatgatatccggttcagacagggtgcgttgctgccaacagtgaccgccagagcgggtgttggcgtggaaaaagtaggaagatataccagccagggcgccggtgacgcctctacggaaatcactcccggtaaagaaatgcccgatccgttaacggatttgtctatcggcgcttatgccaactgggaagtggatatctggaagaagttacataacgccaaaaaggccgcggtaaccaggtatttatctaccgtggagggcaaaaactttgtactgacaaacctcgttgcggaagtagctaattcttactatgaactcctggctctcgacaaccagctcctgattgttaaacaaaacattgagctgcaaaaaaatgcccttgagattgtaaaagtgcagaaagaagccaccagggtaacggagctggccgtgcagaaatttcaggccgaagtactgaagtcgcaaagcctggaattcgacattcttcaaaatataaaagaaacagaaaacaagatcaacttcctgctgggacgctatccgcaggagattacccgggacaagggtaacttcctgagcgcggtgcctccggcggtaagttccggtattccttcacaattattggctaaccggccggacattaagaaagcagaattggaattggctgctgcgaaactggatgtaaaaattgcgcgggcagaattctatccttccctgggcatttctgcaggagcaggattccaggcatttaagccgtcttacctgttcaagatgccggagtctttattgtactctcttgcaggagacctggcagggccgcttatcaaccggaatgccattaaagccgaattcagtaacgccaatgcacggcaattgcaggccatatataattatgagcgcaccattttaaatgcatacttcgaagtttccaatcagctttccagcatcagtaacctggaaaagagctatgatctgaaatcgaaacaggtggatgccctcacccgttccatcgatatttccaacgacctgttcaagtcggccagggccgattatctggaagtgctgatgacacaacgggatgccttggaatccaaactcgacctgattgaaacaaaaaaacaacagctcaatgctgtgattaatgtttatagggatcttggaggtggctggaaataaaatagtattctgcataaaaaagccggctgtaatagccggcttttttatgttataaagaatttttcatgccatttctgttgatagtttacctgggcaacataacatccaatgatgccagccgcttcaagtcataattaaacggttccggagccgtataactccaataaatactctgttgtgaaggccctgcgggagcaagaaagaactgtatcccgttgctatctgcatctaccataatatgcgtaacattatcaagattaacaaactgataggtctgttcctgggcacatttaaaaaggaaagccatattgatatttttgatacaaaatacaaaaaagttgcaaataatatcccttcataataccttcttcaccaaaactaactgtattttatcaaaagcttttctttgatggtatggtaagctattttaatcatactatattcaatcgttatggacagcagcctgctaaaatcaaagcaacattttgaggtactggatggtttgagaggactggcggctctttccattgtggtattccacctgtatgaattcatggttcccgattataccaaaagtccgattggccatggttacctggcggtggattttttcttttgcttatcaggttttgtgatcggttatgcctacgatgaacgggcgccgcaactcggcctgcggacttttttccgtaaccgcctgatacgcctgcatcctatggtgatatggggcagcgtaattggtttgcttggctttatcttcgatccctatatcggtgcggcttccgttgcagaagcgggcataggcaaaatagtccttgctttcgtatgttcgttgctgatgttaccttttccctggttcccgggaagaggcaatgggttatttccatacaataccccggcgtggtcgctgttgatggagtatatcatcaacatcgtttacgggctggtattgttacgcgttgctaagcgctggctgctggttttactgggcttgtcagccatatggattgcggctgtagccaggtaccggggctggatcattaccggttgggatgcacctacttttgcggatggttttgcgcgggtatccttctctttcctggccgggctttcggtatatcgttttaacctgatcatcaggaaccagctgaacttcctgctgttgggcggtttgctgattggcatatttatgtcgcctcaccgtaccaacgactggattacggagatgatactggtgatgtttgccttcccgttacttttatcgctgggcgccggcgccgcggcacatggctggatacgcagtttctgcacctttaccggccgcttgtcttatcctttgtacatgacgcatatatgggcggtatggatctttggcaactatcttaatgcaaagaagcctggtcagggagaaatgtacctggctgccactgccgtatttgcgggatctgttttactcgcgtacctggtgctgcggttttacgatgagccggtaaggaattggctgaagaaaggcaataaaaatagaaaagagaaacgtttacccgttgaaagtttggcagcttcaaaaagctgatgcacaacagatatttatgaccgactttgaactgcttagaaagaatgtcgaacagtacatccagattacagacgcggaatttgatcagtttactgttaattttcatcacaggaagataaagaaaaaagcatttcttctgcgggaaaacgacacctgcaaatatgaggcttttgtaaccaaaggctgtttccgtatttattattctgacgaaaaaggcgatgcccagatcctgtacttcgcggtagaaggctggtgggcaacagatatagacagttttattaaccagaagccctctatcctgaatattgaggcattggaagacagtgaagtactcctcatcaataagccggataaagacttcctgtacgaaacgctccccaaagtagaaaagatgttccggatcatgaaccagaaatcactggttacctttcaacgcagggtcatttcttcattaggcaaaactgccgataagcgttacctggaatttatagaaaaatacccggacctcgaacaacgcctcaatcagcaacagctggccgcctatctcggtatatcacacgaatttttaagtaaaatcaggaagaagctgtccggcaaatagtgcattttttgaactagttcaaattccaggaaatagaagcccgctacttttatggcctaaaaaacaaggatatgaaaaaagcactattgattattgatgtacagaatgattattttgatggcggaaaacatgccttggtaaatgctgcggaagctggcaaacaggcacagctggtattacaaactgcaagaaaacagcatatgccggttgttcatatacaacacttggccactaacgaaggcgcagtttttttccttcccaacaccaacggcgctgacatacatcactgtgtaagtcccaccccggatgaaaaagtaatcatcaaaaactatccgaatagcttccgggaaacagcactgctggcatatctgcagcaaaacggtatgaccagtctcgttatttgtggcatgatgacggatgtgtgcgtggatgccactgtacgggctgcaatggacctcggtttcacctgtattgttatcggtgatgcctgtgctacccggaaccgtgagctgtatggtaaaacaataaaggccgaagcaataaacagtgcttacctcgccggaatgaccgcccttaatggcctctatgcaaatgtaattacagcggcggagttcatggagctgtagtacatctccctgattccatccttttgactacaacaatgagtactttggctacatctgttttgtgattgctgcggacctttgcatcaacaacaaaacaattatatgaacatcgtacttacaggttcgttagggaacattggaaaaccgctcgcacaggatttagtgcaaaaaggacatatggttactgttatcagcagcaacgccgaaagacaaaaagacattgaggcattaggtgcaaaagcggctatcggcagcataaaagacgctgattttctgtcagtcgctttcaaaggagcagatatcgtgtatgttatggaaacactcgacgctgccggcggcttctttgatcaggacgttgacttcatcgctaccattaaccagattggccataattacaaacaagctatcctgcaatcgggcgtaaagcgtgtggtgcatctcagcagtgttggcgcgcatatggacaaagacaacggcatacttatctttcatcacaatgtagaaaacatattaaagcaactgccggatgatgtttctattaaatttatgcgccctgttggcttttacaccaatatgttttcgtttgtacgcaccataaaaacacaaggcgctatcatacaaaattacggaggcgccaacaaagaaccctgggtttcacctttagacatcgcagatgttattgctgaagaaatggagcaaccttttgaagggaggcaaatccgttatatcgcaagcgacgaattttcgccggatgaagctgcttattttcttggtcaggcaatcgggaagcctgatctgaaatggctggtcatccctgatgaacagttgctgggcggttggctgtcggcagggatgaacccgcaaattgcgaaaggatttgtagaaatgcaggccggtatgggtagaggtatgctgtatgaagactattaccggaataaaccagtactgggaaaagttaaacttactgattttgtaaaggagtttgcggcggtttataatcaatagcaaaatgactatctttaattattaaaaaataaaaccattaaggaattaaggaaatcctggttccttaatggtttaatatattatggcaggtacaaaaacataccggattaaaacaatcagcgaatttcatcaactccggaatttgccaaaacctgagcacccgctaatcagtgtgatagattatgctacgatgccgcatccagaaaacagcgggataaactggatttgcgacttctactctatctctgtaaaacggggcttgagcggcaaggtggtgtatggacaacaggaatatgatttcgatgaaggtgtcatgttttttatttcacccaaccaggttttcaggcttgaagttaatccgaacctaacggcaaaacgctcaggttggatgctgctgatccaccccgatttcttatggaatactcctttggccaaaaccattaagcaatatgaatattttgattattctgtaaacgaagcgttgctgctttccgaaaaagaagaaatagttatcaataacatctttcaaaacattcagcaggaatatcattccaatattgataatttcagccagcaaatcattatcccgcaaatagaaacgttattcaactacgctgaaaggttctatcatcgccagttcattacaagaaaaattaccaatcacaaaattctaaaccgtttggaagaattgctgacagattatttcagcagtgataacctgatggaaaaagggttacctactgttcaatatatagccggtacattaaacgtgtcacctaaatatttaagcagtttattaaaggtactgacagggcaaacggcacaacaacacattcatgaaaagctgattgaaaaagccaaagagaaattatccactaccgatttatcagtaagcgagattgcttatgaattaggctttgaacattcgcaatcattcagcaaattgtttaaaagcaaaaccaatctttcacctttggagttcaggcagtcattcggctgatggaattccccgttgctatcactccgcgcggaactttacttcattggcccaatgtgctttccaatcgggatgaaacgccctcgcattcagttttgatacgctcctctcctttgccagctccatgcagctgccgggcgcgccgttatcgtttaccctgaatgatagcttaattgcctgtcttttgtcaatggccgcctttacttccggcaactccgaccatggaatagcacactctgtgatcagcgtattgccctctctgcgcaccgctagcttcccatttcttaccggtccttccccttccgaccgtggctgtcgcggaaaaaagtgtttacggttcaagcccggcgccagcaaccgccatatttcagtgccaccgccatattccggcgacacctggttgagcgcatattcgtaatcagtacatttatacccggtgtaacgcggcatggtacccggcggataagccagcatcccgtcttttccttcaggcagtacattaaatgccagcaacacattatcgtaagcatatcccaggccggaattatccggtgttaccgggtttttacggtaggtataatgccgcactcccgaaggccaaatcagtggaaacttcacttctttattcaccagcgataacacaacaccagccggcaattgcggcggcacacctactatataataccctgccttgccatatacgtttctccagttgccacgggtatcgaaatcttcttttacaaaaaaaccggcagcagcagtaggtgcatcgaataacaacgctgccagtttgggtgtataccaccagcctttgctatgcaatacaattctcactttcccggaaagctgcaatacctcccaggcgccattccagaggttgttgatgttgcgttgcaacaaacggccgccgttactgtatacttccagtaccacgcccggcacacgcaatgcaggcaggtacaatgccacctgcgtgagtgaatccaattgcaggtctacaccgaatgaattggtattatcgctgctttccaggtaatgcaggatacggccattgccggcggggagctgcaatgccgcctcttcttctgcaggcgcactgccttctttgctgatcagcgcctcctgcatatccatggcataggcggtatcgggataaaagaactcatcgtccgggcgctgctcaaaacggtaagtgcccggatgcggcgtgctgtccgctgttttggcggcaaaataaaagtattgatcgtcgtatgcaaaatagccgttggcatagccattggcacgggtgtcaaaatttttgaaaggataccaggcagcttctgttaaactaacctctgcaacgccctggctgcttaccgtttgaggcaatgccgttttccagtcgtccagctggccatcaacgtgtatacttaaccgtgaaatcaggttcacatgcatatcttcatcatgcactgccatgccatctgcaccggcatcaaaatgaaccgacagcggataggtattgttcacggaagtctttccccctttgatctttacaggaactgtaatggtttcatgcggcgccagcttcaccgtagcaggagcttcaatatccagatcccccaaagttatttgcaaacgcccctgcaccggacggttcagcatattggtcacctggagcggcataagtggtgattgttcaatacgtgcagtcatatcttctgcgatgatttccaccggctcatacccttctatacgcgcggttttcagcgccgccagcatagcggcaaacgaacctttggatccgtttgtccggagatagtatccctggctgttcagcggaatttcaagtttaccacctaccggtaagatagggttaccataaaaatcgaataactgaaaggcagcaggcaggatcatcttcccccccgttaaaggttcataggtaaccggcttcccggatgcccgtaacttttcagtggcagcggtttgcgccagtccccgcacttcccggaagagcacccgttccggaccaaacgcctcgcctatatcgccacatatcactacggtgccatcgtcgggattttttttaagcccgtcaaacaccatcacccagggtaatcctttggtaaacaacagctgtttaaaatcccgttctcccaccaggtgctgcacggcgcccagcgccgcggcctgcgaccaggtatcgggaatacgcgtaatttctttcacaccgtcaggcgtattaattttacgggtgaaatgttcactgccccggccaccggtatacatatatcctgcgtaaatacccatagaacggtcgtagccagcagaacggctggtagctacggtgaggcctatacgatcatcggtattgcccacccagctttcggtatcccagatcttcacacgaccgtgcggcgatttacggttcacccattccggataaatagcgggcgactccaggccctggtagtggatcgagcagaaatcgaagataggcaggaacgtcattttaccatctgcaaaaagtttatcccaggcattggaattggaatcgccaccgcctaccagcacgtctgctccttttttacggccatccagtacggcctgggccattaccgtatatatttcccggtaacgcggaatatccgattgccagccggaaatagacaagccttcccagggttcgttccacagggatacagctgttaccggtcctttaggccagccatattgcacgcaaagccggtgtacaaattcctggaaatccttatcggacgaaggcatccacaccatgtcctgttttgtttttttcatcacagcagcagtgtcaagaaatgaacggggtctgcccagtggctggtctgccgatcccgctccaaacatcagcaacacggtgatattcttctccctgtactcttttaatttgcggtcaatcgcttccatttttgccgtatagtctttggcggtagtgggcgtatagtccacccccatgcgaatggcctgcacgcctacccgctgcaggaaatcagcgcccatatcatcaagcgattgctttggatactgtatccgctgcggatttgcggcaaaggtgcgtaccaggctggtaataaacctgcggccatatttgccgagatccatcaccagcgcataaccaccaaaacgcggaggaattaccggaagatgctcaatgttgacatatcccttcggggaaatatttaccttcaccggcgtaacgctgacagtggcaaatttcaccatctccggctgccacacgtcacccggacggcctttggtgccatagctgatcagttctatcttcccctcagtagttatgggttcatcgagctggtttaccacctgtatcgtataggcaggctgttctccgggccacaacacattggtggtgttggaagccttcaccagcattacatcatagctataatggcgttggttatttcgtacgcccattaccgtttcataattcacccattcttccggcgctttcatctgggccatgccactcaccgcgctgagtatcagcaccggcatccatatatatttcatctgttattgctttataaatttacgctgaccgatcatctgaccagtaccggcgtctgaaatcaccagtatgtaggcactctgcggtaaactgcttacatctatcttccacggtccgctactttttcctggtattgttttcaccatttttccggagagatcgtaaatactgaccatacatgttttgggctttgttagccggatgtctacattcaaaacattcactaccgggttaggatatacgtttaatcccgaagacagtgttaccagtttaccggtggccagggagctgctgctatccatggttgccggcggcgtccagagatataacactaccttgttggcgttgtaatcatctttggtgatcatgtactcgccggtagaccggtgataggctttgatgccatattgtgaatccacatcgttgcctacatatacgttggggttgctgctgttcatggtaagcgccaatgcgccggtggtaagatcaaaaacatcgatatcgggaattgcatagtagccgacaaaaagataatttcctgcggccgacatcgacttagcctgcgcgcggctcagcgtaataacggtgtcgggcgtacgatttccggctacccatccgtgatatacttctatgcggttgccgatcagcgtccagtcggtgctgccgccggccagcaccatcacatcactggcagggatgtattgcagctggtttaaccgggcgatggtagcgggtgtaggtgtggatatcaccggtccccagataggcttgccgttgctggcaaaacccgttaacgggtaatgctggatcgcatttgttttatcctgggagatccagatatcacctaaagaatcaagacaaaatccattcctcaccttggagatggtatcgccgggtatagcgatgtatccatctgtagcaggattgaaatagtatgtgtaaaacacgtctgcgttctggttgttggccaccaggatccggtggccgcctacattggccaggtggccaaaatgttcgcccctgccacggtcgctcatctgtatccgcgcatcccagggatagcggtacggatccacggtattagccacatacgcaccgccatctgtaccggtataggagtaaatgatattgccgctgtaaagcaattcgccgtcagtgccggcatcagcggcggcacagccttcaaagttcagcgcctgtaaagtccataacagtgaatccgccgtgctgtagcaatgaatatcagtagccccgttcctgcccaggtcccatgtacctccccagggattgttgagcacatacaacttaccggaagcatcgcggccgatgcctactatccgcgtaaaacgcttgtcgcccgcagctccgcggatactgcccgtttcattgaggtaaccgcctaacgcaccaaaagttccactcagtacgggcgttcccgttaggttagtataaattttgatattcatatccggtccctgatcgcctaccagtaattgtcccctggcactatccgcatatagagcagacggacgcgcagtgacgccaacattcaacaccgtgcctgccacaccggtggagtcgaaacggcgtatggtaccgccacccagctgcaccacccaaacagcgccggcactgtcgaccgcaataggccccggcgaggtaacggcccattgtcttattaaaacgccaccggtggtaaataccgccacgcggttgccgctggaatcgctgacatatacacgtccaccggaaacggctataccgcgaacggcatcaccggtacctgtgctggcagtaaacaacaggtcgcgcagcttagtgctgcgattgtaacgtcctattttaccgctgttgggcgcctgttgtgcggtaaagatataagtggcattaccaccaatagcgctgccctgtgattctttagtgccgcccataccgccaatggtagccccattctgatagatgccgatattgcgtcccttttcatcccataatgaggcagtatacaccactccttccggcgacacccacatggaacgggcgcaattgcctacataagtggttacattggaaaaagtattgcctacccaggtggtggtatactgtgcatagcagaaggcagctgttaacaacagccataacgtggaaataattcttttcatctttataaatttaagatgttagtagccatgattctgtaccagccgcgggttacggcctatctccctcagcggaacaggccacaatgcctgatctgcgttaatgcccaatactgcttctgccctgcccgtacgcaccaaatcgtaaaaccggtgaccttcaaaagcgagttctttgaaccgctcgttttctatcgcgagagcaagattagtctccccgccatagggaaagtcatgtgcacccggtgcggttaatggctctgcaaaagccctgcggcggatgatgttcagcgcctctgttgcttcggccgttttgcccaggttgttcagcgcttctgccctgaccaggatgatatcggccagtcgcaacgcaataatatccggctctgtaccactggttaaacgggtatatttatttacatacggcaccgcagggctggaagtagtcaggcccaacgccgcattcttccggatatcgccggtttcataagtgccaatgatctttgccgtaggagttatctggtaactaccgggctgtatgcccgcaggaatgccattcaccggcacatataaactgaataagccgttggcctgtgaagaagaacttacaaactgtatttcgaatatcgcttctgtactgtttttgccgccggtggagaacatgttgctgtaggccgcagcgccgcttaccagcgtatataccgggctattcattacttcgagcgctttggcagccgcggagtcgtaatttttcacgctcaggtatgcctttgccagcaaggctttggcggcaccctgactggcccgtcccctggtagatgcggccgcggcaaacgtagcaggcaaagcagcttcagctgctttcaaatctgaaatgatcagctgaaaaacactgtcgacaggcgaccgtgcaatagtaaaatccgcattaaaagaagtatagggctccagtaccattggcacagcgccataagcttttaccaggttgaaataaaaatatgcccgcagaaaatgtgcttcccccaataactgttccttccgcccgcctgtaaacaggctgtctttcatggcaggcacatgtttcagcaaatcattggcgcgaccaataccggtgtaattattctgccagtagcttgccacaatggcgttatctaccgggataccgtgattggtgaacggactgtaattgatcagtaaagcggtggtggcgtcggaggcggcatcgaaagccaccgggaactgcatcgacatactttgtatggccgggtaaatgcctaccgccgcgctttccgcatcgctggcagtttgccagaagttttcatctgcaatggtatactccggcacctggtccagtactttggtacaggaagcaaatgcgaagagaagatatataagtcgtaattttttcatagcggctgcttttaaaagttcacatttaatccgagcaggaaggtgcgcggctgcggttgtacggcccagtcgataccaagctgcgagttcttcaccgactggttctgcgattcaggatccaggccggaatagctggtgatcaggaagaggttttgcgcactggcatacacccgggcgctgctgatccttatctttttgagcagctctgtccggaaagtatatcccagcgtaatatttttcatcctgataaatgatccgtcttccacgaagcgctgcgatacttccccgttggttaaactattgggcgtggcagggtcgttgaacacggccttcggcacatcggtattggggttttccggcgtccagcggttcagcgttcgtacgtcgccgttattgtagccgctcatgcgttccagcatgttgcgcgtttggttgtataccttattgccgtacgaccagtacaggaagaagctcaggtcaattcccttgtaaccaaaagtattggtaaggccaccggtataatccggtaatgcgttgccgaggatcacccggtcggctgccgttatccttccgtcggcattaatatcatcatagatcatgttcccggttttaggatctactcctttgctgcgatagccaaagaaggaaccaacgggctggcctacacgaaaaatactggtgggcaaactggtaccgaacgatccgggcaggctttctgtaaagtcggagctggaagggtcaccagctactgtttcaggcagactggtaattttattcctgttgaaatacaagttaaagttagtgctccaggtaaatttgccacggatattgtctgtattaatgcctatctccaatcctttatttaccatttgcccgatattagcgccattggtgcggttaaacccggaggtatagggaagatccagtttaaagatcaaacggttggtgagtttgcggtaggcatctaccgtaacactgatcctgctgtcccagaaactcaggtccagcccgaggttggtggcggtagtcgcctcccagctaagatccacatttgacaaagaggtagcggcaatgccggcttccgaaccataattatagccggtggaataagtggcgagtgcgggaaagtcacttccaagtccttcattgttacccgtaacgccaatgctggcacgcagtttcagctcattaataaaacgctgctgtttcataaaggcttcattggttacccgccagccggcagccacagagggaaagaatccatattttttattttcaccgaagcgtgaggaaccatccgtgcgcagtactccttccagcagataccggtcgtcgtaattataactgaggcggccgaaataagataccagtccccattgcgagcggtaatccagcggcgcagaaagggacgtaaaaccggtaactgcctcgatgatatcggttgaattggtattgccggaaacactgatccttctcacattggcttcctgcgcgctttgaccgaggagggctgttaatttgtgtttgccttttaacaccggcgtgtaggataatgtattttcattgacccataagaactgtgtgaatacagacacaaagccactcgcggcagaaccgttgttcaccagtttcgactggtaccggtcgtcggttacctgctggttatcgaagccaaaactggttttaaatttcagtcccgggaggatggtgtactcgccatatacattaccgatatagctgttcacgatcgactggaaccggaggttattagcgatcatcacgggattggtccagcggcggttcctatcggcatagtaagtgccattaggattgtagatgggatcgttgggattttctatcaatgccagcgccagtactgattgtccggagaagctgttgtccatgcggttgttggtagatcttacccctgttaaatttacaccgatctttaacttgtcggtagcggcaaaatcaaagttcacgcggccgttgaaacgtttatagtgttgcagacctacaatagtgcctgtttgatccaggtaaccgagggatacatagtgtgatgtttttcctgtgcccccggagatagataaattatagttagataccggcgccgatctgaaaatagcatcctgccagtcggtgttacggtcggtgttcactaccgcagaatctaccggtaatcctgcattaacacgcgattcccggaacagttctacaaactgttcgccgttcagcagcggcaaacgtttggggatgtctgcaacaccggtatacatgttgaaattaaaacgcgacttaccttccgcgcctcttttggtggtgatgaggataacgccgttggcgcccctggagccatagatagctgtggcggcggcatccttcagtatttccaccgactgtatatcgttggggttaatgttgttggtagttgcgatcctttgtccatcaccggaaacgccgtattgggcggcaggaagattgctcatgggcacaccatctattacatatagcgggcggttttcaccaaacaaagaaccgttaccacggatacggatatacgtttcatcgccgggagcgccggaattctgcactacctgtatgcctgctgcctttccctgcaaagcggcgtccaggctggttactgcaacgccggtaagctcactgcctttgatggaactcacggaagaagtcaggttctttttttgctgggtgccatagccaattaccaccaggtcgttcagcgaagcgctttgcagcttcagcacaatgttgatgagcgactgccccttaacgtttacctctttggattcaaaccctacatacgaacaaaccaggatgctgttatcatctggcacggcaagggtgaagctaccatggctgtcggtagtaatacccagcgacgtgccttttacccggatgctcacgcctggcagcggtgatcctttctcgtctgatatgttcccggataccgtgatccggtccagctcctttccggcaggaagtgaggttgtttttttagtgatcactactatcttatccgttatttcatattggagggaaagcttacccaggaaggatttcaacacctgttccaggggctggtccctgcattcgagcgatacgttgttaagtgctgccggctgatcgcgccagataaaagaatagcctgtttgttgctttaacagcaccagcactttttccagtggcacattttttacggaaattgttacctgttgtgcagcagcgttcaaatgcagcagcaggatggtcataaagatccatagcggtttggcgggccatttctttacggccgggagagtgcctgtggcaaggaatatcatatttttcagtcgtggattttaaacattagcaatcataaacgtggaaatttagtcaggtacgcacatagcttaccacgccgggggcccccggcaattggttttcagcagatgtgcttactacggatgatccgtgcagcaatcaggtcatgacatatctgttttaaaagagtgatttaattggcctcctggtaaggcatcacggtaatagttcttccctgtgtcttaaaacgtacgattttggttagttcaagtgcttttagtaactgtgatatctttgctgtccgggaaacgatgccggagagctcaatgccggacatatccccttcatactttatctctatatcataccatcgcgctatctgccgcatgatggtgctgatgtctgtattcctgaaataaaactccccgtttttccaaccgagtatttcttccatgtctggtttgttcacgctcagctcaccggaagcgtggtgcagtaccgcctgttcaccgggatgtaatattctgtccgcgtttatttttactgctccctgtaccagcgtggttttcacggcagcttcatcggcataggccattacgttaaacgacgttcccaatacctgcacgtccatgcctttggcggttacgataaatggtttcctgtcatcctttgcgatgtcgaagtatgcttctccagaaacttccaccattcttttatcctccgggaaagcggtgggataacggatagaagaagccgcattgagccagacatgtgagccgtcgggtaaaataagctggtacaggcagccggtgggtgtttgcatgatattgtataccaggccggtgttcttctgtgaaaattgtttataggccaactgcccgttggccagcttaattacctgtgcggagccctgttgggcgatggcgccgttagcggcgctgtcgagcgctatgcgggtgccatctcccaggatcagcataggccgcgctgttccccgcggcgattgcgacgcctgcgctatagtaccagtccctgtttttttacggttattccactcccagcttacagccagcagcaataaaaagatagctgctgcggcggcatatttaaaccaggggcgtgcaacaatggatggttttgtacgatgtaaaaccggtatggcttcactttgccgcgctttcatcatcacttccagcgccatttctccggcgtcaaaatctgcgctttcagcataagcaggatcattaaaagcctcctgcaacaattgggagagcaacgccttattttccggctgcagggccatgcttctgaacaaccggatctctccggcgttcagcgttccgctcatgtatcttttaaacagaccttcaaaagtaatttcagacatatgctgatacagatttaatatctcccgttataaggacggaaaacaaagaaggggtaagacagtaaaactgaaaaattcatgaaaaatgattggaagccaggaacaacaaggcgaaaacactttcggaatgccggcttaaatactcccggatgctgcgcagcgcccgtacaatataggtttgggagcttaccacagaaatattcagtttccgggagatctgcacatgacttagcccgttaaaacgatgcaacacaaacacggtctttactttctccgggagatgttcgatggcctgcagcaggatcttttccagctccttgtattccataccggactgggcatcgctgaatggagcttcggaaagatgatcggccaggaattcaatattatcagtatgcagcacctttttctccaggtggtccatgataagattgcgggcacatacatatataaacgtacccactttttccacgccgggaagctttgcccggttgttccataatttgagaaagatatcctgtgagaggtctttcgcctgttcgggagaacgtgtcaggcgtaacgccgtgccatatacctgtggccagtattgtttaacgagaacctggaagctccgctcatctccttttgcaacggagagcaacaattcctgttcattagcgtggatcacggatggtatcagtgttaattataacgggtagtgatgcatgaaaataatacaacctgttctaatttacaaaacaatacttccggcttttgaaaagtggcggctttagggtaagcgatcgctgttttaattatcctgaaatgactgcttaaacgctaccggggttaaattcgttttccgcttgaatagtttattaaaagactgaggatactcaaatcccagctggtaagcaatttcagccaccgacagctgggtagacatcaggtattcctttgctttttcaatcagtttttcgtggatatgctgctgggcattttgcccggtgagcgaacgtagcatatcactcaggtatcgtggtgaaacgtttagccgctctgctaaaaattcaaccgagggaagacctttctgcaatccttcttctttatcaaaataactattgagcagctcttctatgccggtaagcagatcgtgattcacagatttgcgggtaataaactggcgtttatagaaacgattgctatagttaagcaatacctcaatgtaggacacgatgaggtcctggctaaaggcatcaatagcattattaagttcttcttttatactctcgacaacagtaaaaatctgctgtttttctttgtcggataaatgcagggcctcattggtatcataagaaaagaatccgtactgtttaattttttgcccaatgggatagttcctgataaagtcgggatgaaaaagcaatgaaaacccttcatataccgcttcattcggaacggtgatcagttgattgggagcggtaaacaccattccgccttcatcgaaatcataatatccctgcccatatcccattttgcctttctgattgagtttatatgatatcttgtaaaaattcagcaacaaagcttccggaagctgactggtatcaactttgatactggtgttgtcgaaaaaaccaatcaaaggatgcacgggttttggtacccccaataatctgttaagttcagaaatggaatctatttttgcagggatattatttgacttcttcatttaccaaatttaagacttaatttcctaacacacttttaccaagctcgatgcgggccgcttccttaccaatttccaggcgtctgttatataacgcatttgcatactcaccacccacataggtaattttgttttgcccgtcggtagccgcttcatatactaatcccgctatttcgtctgctgttgaaaaagcttcaggatcgaataacgcaaacactttctgcatcatgtcctcgtaagccgggtgactgcccatttccagcgacctgcctgcaaaatcggtaacaataccacccggtgcaacggttttgatgccgatattatgcaggctcagttcataagataaagattcactccagccttccagtgcccatttggtggcatgataggtggaacccagcgggaagcccaccaagcctccgatggaagtgatcgtaataaataagccttgtttcttttccctgaaaaaaggaataaatgcttttgtaactcttataacgccgagtaaattggtgttcagctgttttacaatctgctcatcgctcaatgcgtccaacgcgcccatcagtccatatcccgcgttattgagtaccacatccacatcgtattttgcggtaacgttttttacgcaatcgttgatttgttccggattggtaacgtcgagcggcagcaggatcacattttctaattgtgaaagctccgtttcgttttccggcttacgcatggtggcgatcacctgccatcccttgctttgaaataacctggcagttgctttgcccagacctgttgatgctcctgtaatgaagatcgttttcatttgtcgatgtatttaattttacatctcaaaggtctgatactatggaaagctatatgttgccaaattgagttttgatgtagccgaaatgacgggcgccgttatgcctactatttaaaagtaacctttatcatttccgggatgcctggcaaggtggtaaatgaattgggattgggcaccaccgcaatcggcttgctttccgtgagcggcgttcctgctaaattgaactgtgtaacacctgctcccgggaactgatcaaccgcagttccattgttatataaggcaataccggtggaagcatcgccttttttaaagggatcaatgccatctgcaccggtggcgaagaaccagtcgttagagaacccatacatggtagctatcgccactctgtcgccttttgtaacggtaatttcccgggaaacatttcccccggcctgctcccctatctttggaagtaataccgtggtgttgggcgcaggaagcacatacaccgatttaatgccactttttgtttttaatgaagcggcgagtatattcgcattcccttgctgggccagttctttcaatccttcgttccggtcattctctcccactttaaacaacggatcttctattccgttatacaccactaccagcaccggagacaacggtgtaaatataccggtgatgctgcttatatacgttttcagcggcatgttatttcccgcttctgcgatggaggttaaaccattggcagaggacattcctttaacatacagcggggacggattgagtaaattgccgcctgcgatataggatatggcccatacaccaggacttaaaggcgtttcgttagccgttcctgccgaagtattccggagggtcagggtaaactgtgagttcccgttgtatttcagggttgcttttaccagtttggaagcagggagataggtatttccctgggcatcggtaccactgacttccgagatgtttttattttcaacagttcccggatggactacaccagcacctggcgcctggtttacacgggtgccattatcccatagctttacctgtgaagaaacgtcgccttcaataggttttccgtcctggtcatataccagtatccctggattttccggtgcaaaaaacaaatcgttggatgcgccatacatcgttgcaaaggtgatggcctcacctttggcggcagaaaatgtgatggcagcggattggctcggtaaaatcagcgccggtgttccggttccctggaaggcgcccgattctaccaggggccgggaatctaaaacgttttcaatggtgatggttgttttatcactcgcaccatccggaccatctgaatgatctttcttacaggcaggcaatgccaggggtatcagcgcagcagccacccagggggcaattctttttatgtgtttcatgttgtatggtctttcctgctttgtcggaaagccggtttattccttacagtcttttctatctttttaaagcaattctttttgtaaggaccagcgggttcatacgactaaagcaaaaaatctacaaatcatatgaaatcaaacgttaaaaaacacaagtacttccgcgtagccagctggaagaatgcctgcgttgtgttcgccgtgatgggtcttttaagttcaggtgatactgcgatggcgggcaccacaactgtaaaagacacggtagaaatggtggcaggtgttcctgtaaaaccggaagacatcagtcccctgctgataggcgaacccatacccatgctgcaactgcccacctcttcagggaaacgttttgacttgaataagtcggtggcagaaaagccggccatcctcgttttttatcgtgggggttggtgcccctactgcttaaaacaactgtcggggttgcaggaaattgagcaggaccttgtaaatatggggtaccaggtgattgctgtcagcacggacagcccggaaaatcttaataaaacattaaacaaacaaaaactgacttatacgcttttatcagatgcagacctggacgctgccaaaaaattcgggattgcttttaaaggcccccgggactatgattcatttttgggggaaacttccggaggtaaaaacgtgaacaaattattgccggtaccatccgtttttattatcagcaggaaaggcaccattctttttgaatatatcaacccggatattacccaacgggtaagcgcttccttgttaaaagcggctgcgggagccctgcgtgaggagatataaatgctatctcagtttatcatctatgctcttttgcagttcctgtttgaatttatcatccagcttccgttcagcctggccagctgaatggaagaaattgtgtaccatttgattgatgatgatgctttgctgctggaatgttttgcagatggaacaacctgccaggtggattttcagttccagtttctcacggagcgtaatgcggcctatctgctgcttctcaatcaggaaagtggctttccggcagttataggcgatcttttttaattcattcatagcggttgattaaatccagtttttttgaagacaggcgcgaagatttacttttgcccggtgtatgatcacccaaaaatttgatgcagatacttttaaggtattgcagatggtttcggtagattcatcatccatatgcttcatcgtaaaaaccgaaagccataacaccggcagcttcttcatgcatagctgcagtatccgctgaaactctttattttccagcgcatcaggccgttcaatccctaattctcttggccggtgctgatcattccagtgcccgtcgatggcatcgaaaaaatcctggtgttcccgttcagcatcgctgaggttagcgcgtttggcgaaggcggaggagtttttgcgataaacatctatcaccttgaattttaaaatggcggtaagccaggtccgctctgtgcttctgccttcaaatgtatcaaccttttccagggcagccaggaaggtttcctgtaccaggtctctcgcttgctcttcatcattaatgcgtgtaacggcatacgtatacaggtaatccgcatacttattcacccacgaatgcggatcgagtgtgttgccgccggcaatgatacctttgttctgatctctttgcatatatgaatttacgaatatattttttcccggtttcccggtagcgggtattagtcggagaagacggaaaaaccttacaggattttttcttttattttagaacctcctctataaattacactaaccattactttcttatcattttttgccctagtttgcgaaataatccagccttaaaaaataattgtcgtctaaccaaacatatactgaaaaggagctgcttttgcgcattgctgagggggacgaaactgcttttgcagctttatttaacctttactccacaccattggctttactcgccttacgcatgctccacagtgagccggccaaacaggaggtgttacaggaagtttttattaagatatggctgaacagggaccggctaagagacgtacagctcccggggccctggctgagaaaaatcaccattcatgaatgtttgcaatacctccgcaaaacatccttgtataataccaagctgggcgaccttcaccaggaagacgccagcttcaaccacgcattgagtagcatttcggtgaaagaaatacaatatgcggtgaaacgcgcgctccaggtaatgtccccacagcgcagaaccatttatgagctgagccgggaaaaagggctgagcacaaaagaaatcgccgctcatctcggcctttcagacggatatgtacgcaatgccatcagcgctgcccttcaaaccatccgcagttttctgccagactccgcccggttacccgccattattatttttttactttttttcagaaagtgatagtgacaagtctttctttcccgcatcttatatatagcgcatggaaaatacacgcatatattacctggcaggtcaatacctggataaaagcctgagcgacgccgagcaggtggagtttcagcagctgttacaggcccctgatcaccaggaggcattacaggcagcctttgatgagctggcaggcgagctggatatgaacgccacgcaggacgaggcactgttgcctttattgcagcgggccttaaacagcgataagcccgcacgccgcatgcacttcctgcctcgccggagctgggcagcggcttccatcatcctgctggtactggccgcaggcgcctatttctggcttgcccataaaaaaaatacgtcgccagctgctatggctgctaagcccacagacattgcccccggcagggagggcgccatccttaccctggccgatggctcccgggtagcgctggatagtctccacaacggcgtgatcgcgaaacagaacggcacgcagctggtactggcaaacgggcaactggcctacgatcccgcaggagcgtccaacggggaaatcgtattcaatacgatgtctactccaaaaggccggcaattccgggtcactttaccggatggcacgcaggtatggctgaatgcagccagttcaatacggtaccccacgctgttttccggtcaagaaagaaaagtagcggttaccggcgaagcctattttgaagtagcgagaaatgcggacatgcccttccgggtgagcgtgaacaataaagccgaaatagaagtgctgggcacacattttaacgtgaatgcttacgaaaatgaacaaacgattgccactaccctgctggaaggatcggtacgtgtggcgggcttcgccaacgggcgccaaccgggcaacataatgctccggccaggtcagcaggcgcaaatcggaaacgccgcgaaaacgggcatccgggtgattgaaaatgccaacaccgataaagtgatggcctggaaaaatggcatcttctattttgatggagtgagcttcgcggaaatcatgcgccagatggagcgatggtatgatatcgaagtcgtgtatgaaaaaggcattccggatattgagtttgaaggggaaatgaccaaagacgtttcgttaaacggcctgctggtgatgcttggcagagctggtatacatttccgcctggaaggcaggaagctgattgtgcaataatacttttattataaaaaccgtcacagcgctaactgtgacggtggatgaatttaattagtcaaaaaaacggtctaccaaccacttttattaacaaccaaatctgctgcaaatctatgcaaaaaaaatgctattgccctcctgttcgtgcggggcagcacccgggcattgcgcaatccgtcaatgaaggattcagcaagccctttagaaaaagaaccaaaatcctgagggctatgaaattaacgaccttcttattaactgctgcttttattcatgcccacgccgccagcatggcgcagcatgtcaccatctccggccggaacctgacgttgaagcaggtgttcaccgctattaaaaagcaaacgggctatgtactgctaaatcagaaaggcgtgctggccgatgccaaaccggtgtctctttctgctgataacctgccattgcgggagctgctgaatgatgtctttaaaaaccaacctttagaatatgtgatcgaaggcaagacaattcttgtttcccgaaaacttccggctgcgccttcgggccagctggcttctccttccgccccccctgctgccacattcattcctgttaaaggttttatccgttctgtcgacggacaacctttagcgggagtgaatattgtgattacaggaaccaataagggaactacttctgttgccaatggctctttttcttttgatgtgaatacgggagatgttattaaagtatctgctgtcggcttcgctccactcctcctgcgtttcaccggcagtaatttccaggtagtgtcatctgaactgcctatcaaacacaagtcttccggagttgaaggaacttctgccggcgcttcaaaactggtttcgggcaatccttctgcgctccttatccagctggcattaagcacttcacccatagatgaagtgcagataacggcctatggtacaaccaccaaaagatttaatgccggtaacattactacggttacatcaaaagagatagaaaaaaatcccgtaaataatgtgctggaagcgttgcagggaaaggtgccgggattatttatccagcaggtaaccggtcagccggggggcgcatttaccgtgaggatgcgcggctccgccaacctcaccaccggggccacacaaccgatgatcatcgtggacggtgtacgttacccgggcggcacattacctctttccaataatacctcctacggcacgcaaacttttctgcagggaggcagtggcctgaattatatcaatccaaacgatattgaaagcatcgatgtgctcaaagatgtggatgccactgctatttacggttcctccggcgcctatggtgtgatcctgattaccacaaagaaatccaggtctacccaacagtcgttcaatgccaatatctacaccggcgtatcagtgaacgggcaaacacccacattgctcaacaccgatcaatacctgatgctccgccgcgaagcgctggcaaatgataaactggaaataccggccagcgataatgatctgaatggtgtctggcctgccgaccgatacaccaactggcggaaagaattcatgggaaaatcggctgcaacttctaatgtcaatctttcttacagcggaggtgcacaaaacaccacgtacctgatcagcggaagtctccgtgatatgggtaacatacaacgccaccgcggatcaaacagggatggctctctccggtttgcgttaaacaccggcagtaccaacaataaattcagtttagccctaggcggtacttatctctcttcaaaaaatgatatggtgccctacgatttttcagtcagcgcgctgactcctcccaatgcaccaccagcttataacgaagacgggagtatcaactgggcgtcgatcggaagcgacctaaacagcagcggcaccgccagcaacgccaacaggctgtataaaaacgtaacgaataatctcctggccaatgcaacgctcacttaccggccggtcaaaaaagtgaccctccgcagtatttttggctacaataccattaacggaaaggaactgatcggctatcccacaacagtatttaatcccactaacacccaggcccctacgcaaacggtaggcatacttcatcagtataatacgcgctccatcactatttcaccatatggcgaatacaatactttaatcagtaagaagggtgatttaagcattaaactgggcggcgaggtcaacaaccaggtgacgtattttgacgacatcaccggaaccggatttccttctgatgccttgctgaataacccttctgcgggatctacggtaactactaattacaatcttacggagtaccggtccattggtatgtatggaattataaaatttgtatgggacgataaatatattatcgatatcaatacacggcgcgatggttctaccaagtttggccctggccgccgtatcgggaactttggttctgcagcgctggcctggattttcagccaggaaaagctgatcactgatcacctgccgtggctcagctttggtaagataaggatcagcagcggcgtggtaggcggcgatgccattggtgatttccggtacctggaaacatatagcgtcatcggcggatcgtatgatggaaaagttggattaacacccaactcgcttcccaatcccctgctgaactgggaacgtaattttaactcggaagccggtctggagctgggattttttcacgaccggattatgaccgactttagctattactccaatcgtgccggcaatcagctgctggggcagcccctatcaactgttaccggctatcccagctataccttaaactccgatgcgctgatacgtaccagtggtatggaaatcagcctgagttccaccaatatcaaaaacaggcattttacctggtcaacaaggttcaatatttccatacctaaaagcaaactgctgagattaccatcgagtactcaaaatgccaactatgtgctgaacaaacccgttaccggtaaactactctataaatacaacggggtaaacccggaaaccggcaactatagttttaccgatgcgaaaggaaatgtggctgattactcgggaggattaacacaggccgataaaaccgagtttgttgacctggcgccgaaatactttggcggactgcagaattcctttacttataaagggctgacactcgacttcaccttcaatttcaccagccgcaccggacaaaactttcttggtcaaaccgcctttcctttcgggctctatggcttaaatggttctactatctggttgcgccgctggcaacaacctggcgacataaccgatattccaaagttaagttcccagttcaccagcatcttccggcaaggcctcctgcaaagcagtaccggcggctacagcgacgccacttacgcacggttacagaatgtaagcatccgctatagtttcagcccggaagtaaacaaaatgctgcatctcaaaaatctatcggtgtacctgcagggacaaaacctccttaccatttccaaattcgatggcctcgatccggaaaacctgaatgcaggcgtaatcccgccactgcgcgtatttacaaccggaattaatgttacactttaatgcaatgaaaatgaagatgatctttcctgtcaattatagtttttcgaaacacctgctggccattacggcttcactgagcattacgctgaccagctgcgaaaaatacctggatggtacccagctaccggccaataccattgctgcggtggatgtatattccaccgataacatggcatcaacagtggttaccggcatttacctcaccatgaacaataccggtccttttaccggttccgcgaatgccaacattggctataccatgggtttgtataccgatgaactcagcagtttgctgaccggtaattttgcagatgtgttctacaagaatgctatacaaagcgggcaaagcggcaactggaccgacctgtataaaaaacttttcaccgttaacacggctatccagggcatcaatgccagcaagggtaacctcgtttataaaaatcaatggctgggtgaatgctatttcctgcgcgcctatttttattattacctggtcaatatttatggcccggtaccgctggcgctgacgaatgattacacggtaaacaaccggttgttccgcgtaccggaagctgatgtgtaccagcaaattattgccgatctcaaaatggctcaatcccttttagacaatgagtataaaaatggttacggggttactaccactaaccgtttccgccccaacaaagccgtggctaccgctatgctggccagggtgtacctctatgcaaaagactgggccaatgccgaagcgcaggcgggtgaactgatcagcaacaccaattatgcgatgctgccgatcaaccaggtgtttgttgccaacagcagggaaaccatctgggcattggcgaccaacagcccgaaattcaccaatgaatatgccttctacaacaatggtatgccggaaacgattgtgccgccgcaaagtcctgcttcctccagtgtattcgttaagctgagcaacctcttgaaggacacttttgaacccggcgatgcacgcttcaccaactgggtgcgtacctccacagtggcagcctcttctgccgccccggcaacggtgtactatttcccggccaaatataaatccgcgtccaccaatgcggagtaccaggtactgctgcggctttcagagcaatacctgatccgggcggaagccagggccatgcaaaataaaagtaatgccatggaagatttgaatgtagtgcgtttacgcgcgggcctcggagcgctgccggcaggtacacaggccagtttgctcaaggctattgccaaagaaaggcaaaccgaactgtttacagaatgtggccatcgttttttcgatctgaaacgcaccggcgccatcgatgccgtaatggccaccgtagcgccaaccaaacccactacctggatgagctatatgtcttactggccgataccgcccgctgacctcctccaaaatccgaatttaacgcccaacccgggatatcttcaataacctgattaacggacaggataatgataaaacaaaccatcctgtccgttctcaacacatcaatttttcatgaagaaaatttttatactggcagccatactggcgccgggatcggtgcttgcccagtccggcaaatacacgctaaccatcaaactacctgcgcttaccacccccgcaaaggcttacctgataacaaactatggctggagcaaccagcaggtcctcgactcagcgatgctgaataaaggtgctttccggtttagcgggcaggtgaaagatcctgcgatggtgcatgtactcattgatcataccggaaaagatttcgcaaaatggaagaagactgctgatgttaatgattgctacctggaaaaaggggctattcaaattaccggcaccgattctgtaatccatgcagcaattacaggaggtcctgtgaacaatgattacaagcggtacaaacacacggtgctgttccgcagggaacagctgggcaaagccgtggactccatgtttcacactgcaacacaacagcaaaaaaaagatccccactttatagatacggtgatgaaacaataccagatcgtttcaaaagaaacagactccctgaaatatgttttcatccgtcaaaatcctgcatcatacatcagcctcgctaccttgattgaggtggcaggcaaggatgtggatgtaccacgtattgcgccttttttcaaaagactttcccctgcattacgcaacaccggaaccggtaaacaattcgcgaaaaagctgtataacctggggcggctttcaattggtgtattggcgccggacttcacgcagaacgacgtgaacggtaaaccggttaagctttctgatttcaaaggaaaatatacgctggtcgacttctgggcatcctggtgcgggccctgtagggcagaaaatcccaacgtactgaaagcatacctggcattcaagcagaaaaactttacgatcgttggcgtatcactggataccaacaaagacgcatggcttggtgcagtgaagaaagacgacctgccgtggcaacagttatccgatctgaaaggatggaaaaacgaagcaggtaaactgtatgaagtaagcgccattccgcaaaacttcctccttgatccgcagggacgtatcatcgccaaaaacctgcgcggcgaggccttgatggaaaaactgcaggaactgatgccgtaatacttttatactgcgtgatcggccagtttacggctgatcacgcgggtataaccgttaattaatactaaccactgttaaacagtgttaagcccccatctcgggcaaaaaccgccaaatacaatactgtaaagctatacagcttaccggcatactgaaccattcccggcgtgaccatccgggtactttaaacttcgcaactccacggctatcttagatatatgctgaactaattcctttccaccccgtactgtggttactggatgttttcagtatgcaccaaaaaattaaatcttttaaaaaactcaaaacgcacaattatgatgaagcatttttttgtagcaggtttgttaatggcaacactggcgtctgtaaaaacctacgcacaacaaccgcagcaacaggatcgtgaaggattctttaaaaagatcgataccgatggggatggtaaactcagcaaagctgaggtagattcagcagcaaaggacaacaagcggctttccaggttaagcgaaaatttcgccgccatagacaccaataaagattctttccttgataaagatgaactgaaggcatatagaaaaagtcagggtccccgtaaaaaagaagagggcaatcaataacactaaaacgacaggcatccggataaccaggtgcctgtcgctttttatgcactaatccagtaaagcattataccgttgcaatgcttctaaaaaataataatccgcgtacaccagcggcacatcaatttctgcattatgcgggatacttcccacgctgtgcatcaatataaaattgccgttcttttcttccggcgcccggtacgcagtacctgcgagtgaatgcagtatggtgatcgctgcctggcggtattgctcccccttacccttgccggcataaccactcagctcaaatagtgctgatgccacaatagcggcggcagacacatcgcggtattttgttttcaccttgttggcattggaacgcacacctggaacatatccattctcctgtacattaaaatcccaatagggtactttatcttccggaagatttttattatccaggaaccagtcggccataccggtagcagttttgaggaaacgcgggtcatgtgtttcccggtagatcatggtaaaaccatagatgccccatgcctggccacgcgaccaggtagaattatcggcgtacccctgcgcagtttcgcgtgccagcaccttaccattggtggtatcataacataccacatggtaggaactgtaatccggccgtatctggttgtacatggcggtttccgcgtggctcactgcaatgtggcggaagctggtatcgccggtttctttagctgcaaaaaacaacagctccaggttcatcaggttgtcgatgatcacgggatagtagtatagctgctgactatgccacgatttaaaggcattccacgatttaatgctccgtgttaccgggttaaaacgggtgctgagcgagcgggcgccctggataaggatatcccggtacgctttgttgccggtaatacggtaagcgttgccatagctgcaatacatcataaaaccaagatcatggtgttgtgtaaaatccttcagcggctttaacttctccgtccacttaacagcttcctgtttcagcgcgggatctttggtttgttcatatgcataccagagtgagcccggaaaaaaaccgggtgtccagtcgtacatcgatgtagtgatcatcttcccctctttgttgatcgtcctgggaaaggccaggctgtcgcgggattccgtgtccttcagcatatgcttaagctgctgccgggcaaagcctgcattactgctgataaagtccttctccccgcccaccgtgtaggcagtgatgccggcggctaaaataaaataaagcaatggtttcatattcttatggtgtcactttaatgatcagttcccgtataaccttcttttcttcatccagtgtgtggttaaaagccacgaaggtggccttgtatacgcccggcgccggataagcataagcatattcttctttatccggttcattgatactcttgatgccggtacttacatctcccggaacacggcccgcgtataatggtttggtgacaatccagctggtatttgtagctgcgctgccaccaccaccggtaattttaagatccgtggcagaagctgtccaccggccgttggaagggctccatacattgccgtagcgtgtccagtaagccacatcggccgacaaagaactgatcaaaaccgttttctccggtaacacattgttcacggtaaattcggtgatcgtccaggtacgctgtgtggaacctgttacgccgctgtatttgaaagcaatgaagagtgaatcattttcgttagccacaaggtctgtcagatcagccgtaccaaaaggcactacggtggcgctggtagccagtgccccgcgatcattgatattcgtccatgcggcatttaccacagaagcggaatcaagaccgggtagtttattggtagccagtacctgcagggtatttgtttgcgtaccaaattccgattttgaggaaaaactcagcgtgatctttcccagtttgtttgcagacgtgcggccatcgtagcgcttgcctggttccccggaatagaaggtcacattgcctgcactgccgctgaacctgaagcgggtagtgtctcccaggcgataggtaaacgtgtctgataccagccttgcaggatcaagggctacattaaaatccggcgtatctatttccagtgttttagaacaagccaccgcaaggaaagacaacagtatgatgaatgattttttcatgtggatgtttttaagaattaccagcctgcgttttgtgtcagtaagcggtttagattgagttcgtaagttggcttcggcagcatcacgtgcctggcgcttatattgcgtactccttgcaaaccgttaggattacctgtggaggttacgcccgcaccgttagcggtagcccaggatgcgaagttctgcatgtctgatacaaaactgccccaccggatcaggtccgcttttctcacggcttcaaaacacagctcccgcattctttcatcgcggatggccagttgaaatgcatctttactaagacccggtgtaagatctgattcactaccggtagtgatggtggcagtagccgtagctgcggtacctgcataggtgaatacagcgccggtcaccgcaggatcagaagcgccggaggtatgagtgggtggcgtattagtagcagtgcctgccgttgttaccgtgtacagcataccgccattggtgacttgtgtgcctgtggtatagctggcgcccggcgtccagaaggtgcctatcactaccacaggcgaagtagtatagtaggagcctaccgtcaatgcaccagggctgttcaggtaaatacccgttatcttgccgccggtaaggatcgctgttcctgtagcgccgttaccgccaccgccagtaatcgttaccgcgggcgttttcgtatagccatcaccggtactcaccatcgtaatggattttactacgttgccattcatcagtccatatcctcttttgcgcacctggttcacatagttataagcattcgtagggccgttcacgtaattctctgcttccgcgcgcatcagcaatacatctgagtagcggatcatgggccagttgatattgtacgtgccgcctacaccattggtgttacggatcgcctgcggtacatattctcttctgaatttgccggcgcacatctgccagggattaggacgggctgcttttacgcggggatttgttccgctgtaaatatagttggcgcagttccagtcgcggcgcatatccagcgagggtttgtttggtaaaagggtactattgggatctgtttcataagcatcgaacagctttttagtggcccatacccatgcggcggaattataggaggtagagtccagggcagtcagcgtagactggatccccacaaagttaccgatatcattccccgatttgttcaccacaccggcagcggcgcccagtgagcccagctcccagatattttctcttacatcatattgatctgtagccaggttgatgaacacctggcggtaatcggggttcaatgcatgaaggccggagaggatcactttatctgtataggtgatcacatcctggtatttggcggtattgttttgcggataaccagcccaataaagatatacacgtgccagcatcgcctgcacggcggagagtgttactacctcgttgaatttcgcctgggtgatggtataatctttcagcagcacttctgcttctttcatatccttctcaatttgtacatacacgtctgcctgctttacctgcggaatgttcacatcattgatagcgggtgtgtgaagtactacaggtacatctccataattactggtaagaatgaagtacaggaacccgcggaggaacaatgcctgccctttgatgatattccggcgggatgcgtccatcgttggtttgtcgatgttatccagtaacgaattgagattattgatgcctacgtatgcataacgccagatgttggcaatatgcacaagggaggcgtcgtaattgtaacggagaccgcgtgcatcgccgtctgccgtgcggttagacattacctcatctgtggtggatacaaagttgaagcccatcacctgcgcatacagctctgggcgcatcaggtcgccgtacacaccgttcagcgcctgctggagctgtgcttccgttccgtaataatttgtggtggtataaaaatccgttggttgcgtatcaaggaattttttgcaggaagtaagccctgctattactatacatgccaggatgcaaatacgtttcatgttcatcattttagaaggttacatttaaaccggtcacataagacaatgagtgcgggtaaacggcgtaatcgaagccgggggtaaggttaccaggcctgccgttcacctcgggatccataccggagtacttcgtccatgtataaatgttttgggcagcaccgtagatacgcacattctttatcttcgcacgtttcagcaatgcgcccggcacattgtaccccagggaaaccgttctcagtttcaggtatgagccgtcttcaatcacgcgggaagaataagctgcattgcccataccgcctgcgcggaacatgctgttgctggggttggtgggcgtccagcgtttggcataactggcaaactggttcaggttcggattatttacaataccgccttcaaatacgtaccggttggcattgataatatcattgccataagaccactgcaataatacgttcagatcaaaattacggtaacggaaatcattgctgaaaccaccggtatgttttggtaaaccactgccaataatggtgtagtcctggttgttcacctggagatcgccgttcaggtctttatacttaatatcgcccggacggatagcgttgcgcgccgcgccattggtgggtacatccggcttcagcagatacgtattatttggcattacatcgaaatcggaatactggtatactccatcgaatacaaggccgtacatctcacccagcggccttccgattacagagatataagggaacagacccgaataagtagtattgaaaaaagttccggaaccagagagaatagattgctgtccttctgccagtgattgtattttattattattaaagctgatgttaaaactgctgttccagctgaactccctggtatccgcaattacacctgccactgtgatctccaggcctttgttctgtaactgacccacatttttaaatccctgcgcgctctctataccatgtgcataaggcaatgcggcattcagcagcagatcctttgtagtacgcagataggcatctacggtgagtgtgagcctgtttttcaggaaggccatatccaggccgatattggtttgttcgttggtttcccagcgcaggtccgcgttaccggaagaaatcatcaccgagccaatactcagcggtccatttcccacggaataccagtattgattgctggtgagttgtaactgggacaggtaagcaaagtcgcccacccggttgttcccggatgcgccatagcccagcctgatcttcgcatcagaaatgaaacttacatttttcataaactcttcgctgctgaagcgccatgcagcagaagcggaaggaaagtatccccatttgttgccggctgcgaatttagaggagccgtcggcacggacagacgcagagaaaagatattttgaattgtaatcgtagttcacgcgcagtgcgccggaggccattgtccaaccggagctaagtgaaagcagtgaagtattggccggcgcggccagatcgattccgtccagtccaaggtcttcattgggaatttgatttgccgaaaacctgcgttgcgaatttttatatccctgcgcttccagtacgccgagcacggtgaggttgtgtaacttattccagcttttgcggtaggtcagcgagttttccgaacgccagagtgaagtgggtttggtttccacgctgccattcacgccgttggcgttccatttactgccggattgcgttttggagttgttgaaaatattgatctcggtatttaccgtgttgataccaccggctatacgaagtgtgagaccattggtgatggcgtattccgcatacgcattagcgaacaggttgttcaccttgttcatggtatactggttctggatattttgcaacgggttcacgcgatagtcctggttatttgccagctcattgcccggatcataaaattcatccacgaggttcacactgctgtcgcggccggcgatactggtcgttggccggaagccccacacagaatacaacgtagtggcagacgcataaaaattggtggcggaaaccggtatcccgtaggtttcattgtaagcgtaattggcattaatacccactttcagcttgctgttcactgtttgatccagtgaaaaccggccctggtatcttttaaaaccgccattaataatgatccctttctggttattgaaattaccggaaagcgaatacctggttttatcatttcctccccgcacggcaatgtcgtggttctggttctgacctacgcggtacacaaaatcctgcatatctatggattccttgttgcggtaatcttccagtttagcgccgccggccaggtatacggaatcatagatagatgggttcacatcgcccacatattgtacaaactcgtaggcattcattaacgggattttgttcggcacctgctgccagccatagtacccgttataagttacctgcggcgcgccggttttaccttttttggtggtaataagaataacgccgttagatccgcgagcgccgtaaatggcggtggcagatgcgtctttcaatacgtcgatcgactcaatatcaccggggctgatcgcattggcgttggaactttcggtagggaaaccgtcgataacgtagagcggggaattatcctgtgtgatagaccctgcaccgcggataacgatattggagatagaacccggctgaccatcattgctcgctaccgcgacccctgctaccctgccggccagcgcttcgtcgaacgactttaccggcgccttcgcaaaatctttcatgttcacactacccactgccccggtcaggtctttccgttgctgggtagcatatcccactactaccacatcgttgagtgtgccggcctgctcactcatctgcacattatactctgtcctgttatctaccggctgctctatttttccgaaaccgacaaaggagaacactaaagtagcaccaggatttacgggaatagtaaaacgtccattgccatctgtatgcgcgccggtcttttcattttttaccattactgtcacacctggcaacggtgtaccatctttggcctttacagtgccggacactgttttcttttgttgagcaaaaaggaaaagcggaaaaagtaagatccacatgactcccgtaaaaaaataattgaaggcgaagctgcactctctccccctgctggttgattggcatgtctttttcataataattgtggaattgagcggaaataacggttgatacacaaatatgtggtaaccagttcaaatcacagggggataatcataaatgattggggtgaattttataaatcccccttcaacctgctgattatcagaataataaaagaatgatatttataaaaaacacccatttgccccgatacaattcttatattagagcatgatttcgaggtgcttcccgttcttatgcctgctgctcctcgctgcttttataaaaagcagcgggcaaaacgttacgttcaatcacctcaccgtagaagatggattatcgcacaacgcggtattgtctgttggagaagatgcccagggattcatctggtatggtacacactatggcctcaaccggtacgacggacatcgattcaaaatttatcgccagcaggcaggcgatagcacctcccttcccggtaaccagatcatgagcctgtaccgcgaccggaaaaatgtactctggataggcacctccgcagggctggctaaatatgatcctgagcaggaccgttttcaacgcatccaactggatcccgggcggccaacaaacattaattgtatttatgaagatagtaaaggccgccgctggatcggcgccaacaacgggctttatctccaggacggtaaccggcaggagtttctcatacccgggaaaattgccggttatgtagtgcgttgtgtgtatgaagacaagaaaggcaatatctggattggcaccagcaacggcctcaccaaaatgagcggcaatgattttgaaacattccgccatgaagacggacaaccggccagtctggcgatgaactttatcaccgccatcactgaggataaactgggcaggttatgggtggctacacaaaccggtggtattaatatatatgatcctgctaccggccgtttttcgttactggcgcaaccagcgatcattaataatatagtaagacgggtacttcgcgataaagccggcaacatgtgggtgggcacccaggaaggactcagcatcattgacccggtgacgatgaccagccggcactatcagcaggagcccggcaacagcaccagtcttagccagaattctgttcatagcatctaccaggataataacggtgtaatctggatgggtacctacttcggtggcgtgaacatggtgcatccctatggcacggcctttaccgcctggcagcagcatcccccgctcaatgggatcagcaacaatgtgatcagcagcatccttgaagatgcgcagcacaattactggatcggtacagaaggcggcggactgaattattataatcgcgctacccaacgttttaccagctataaacatgatgcaaataatcctgccagccttgggtccaacctggtgaaagtagtgtatgaagataaagaccacaacatctggacggccacgcatggcggcggactaaacctcctgcggcagggtgggtttaaacgcttcttctacgataccaaagatcccggcaccttttccagggaagtaacagccatactggaagacagccggaaccggttctgggtgggcaccaacaacgcgctccacctgctccaccggaatggccacgagctggagaaacgggccgattctattttaacgggtattgccgcccgccagtcgatccggtatatcctggaagattcccgtcaccggatcctgatcggttctatcagcaacctgtatgtgtttgaggcagacaccatgcggcttatccagccgggttatgtgaactccatacaggaagattcaaagcacaacatctgggtgagcatgtatttcgggggcctggttagatatgatccggagctgaagaagcaaacgcgttatacagaaaaagatggtttgccgaacgataacgtgattgggttactggaagatgatcagcataatttatggattagtacctataacggcctggcacgttttgatcccggccgcaactctttccagacctatactgtaagcgatggcctggcgggaaacgtatttaattacaactcctttttgcgggacagccgcggcgaatttctcttcggcggctataatggcatcaccagttttttcccggatcagatcattaccaattcccatccatccgtcatccggtttaccggtttgcggctgtttaacaaaccggtagttatcggccaggacaacggactgctgaaacaggatatcagctttacgaaggcgctgcgttttcatcacgaccaggaagtatttacgctcgaatttgcgctgctcaactatgtaaaaagcagcaaaaaccgttatgcataccggcttgaaggtgcggaccgcgactggattgaaaccaataatccggcggtaacctataccaatctctcttccggtcattatacattttgggtaaaaggcgccaacaacgacggcatctggagcgcgcccgcaaagatggagatcaccatcctgccgccattctggcgaacctggtgggcatatggcatttacgcattggggcttatcctgctgttcttcttcgtgacccgattctttttcctgtgggccttgctgcgcaaagaagaagaactgcaccaggtgaagctgaacttctttacacatgtttcccatgaaatccgtacccaccttacgtttctgctggtgccggtagaaaagatgatggatatgctgaagaaagacgatccgctgcaatccaccctgctgcagttacggaacaatgccgaccggttgctgaagctcgtgaatgaactgatggatttccgcaaagcggaaaccaatcacctcaaactgcatgtacaggaacaggacctgattccttttcttgatcatatatacaccagcttccgcgagctttcgctcgaccggaacatcagcatggtattcggtcatgatatggagcacgcctgggtttatttcgaccgggagcagctggagaaagtgttcttcaacctgctcagcaatgcttttaaattcacaccggatgggggacgcatccagttgcacattactcattcgcggcaaaacacggtggtcactatcactgataatggccgcggtattgcacccgaatacctcgacaagctattcaccaattttttccaggtacaggatcatggcttgcagaacaccggttacggcatcgggctggcattatccaaaaacattgtggaacaacataaaggaacgctgaccgtggaaagcgaaccttctactgcggaaaaggaaggccgtacctgttttacggttgccctgcctaccggcgccaaacattttgaaggtacccaacacaccgtaggccgggcgcctgccatgcccacggcgccggtaaaagcgacgctggcgccggcaaccccggatactattatcacagctgcaccgcaacccttcaccattcttatagtggaagacaacccggaactacgcgcccttatcagtcaaactttccgggatcaatacctggtactggaaagtgtgaacggggcagacggattggcaacagccaccgcacaaatccccgacattgtgatcagcgatgtgatgatgcccgaaatggatggcctgcagctttgccaggcgcttaaaacagatgagcgcaccagtcatattcctgtagtgctgctcactgccaaaagttcccaggccgatcatgtaagcggtcttgaaaccggggcagatctctatcttaccaaacctttcagtacccgtgtgctggcgctcaacgtccgcaacctggttgcttcccgcgaaaaaatgcgcgaacgctacagccgccagctgcaaacagaaacggaagtaccggatgcgttgcccagcagcctggataacgctttcctcgaaaaagtgatcgcattggtggaagagcatatggacaaccccgacttcggcgtggatatgctggcccggaaggtagccatgagccagcccgtgctgtacaaaaaactgaaggccgtcaccaatatgtcggtgaacgacttcgtaaaatcgctgcggttgaaaaaagcggcctccctgatacgcacccgtgagcataccgtataccaggtagcatacatggtggggtacaacgaccggaaatattttagccgcgaattcaagaaacagttcggtaaaacgccttccgagtttgcggaagcccctgatttgtgaaaattccccccatttactcggaataatcaccccacctaacaggcagggatcattagatttgttacaaatccactgttatgaaaatcagcatgctgcttatcctgggcttcctgtgtaatatgtcccatgcatggggccaaacggcgtacaccactattatggaccgtatccgtgccgaactgctctcgcaatccggcagtacttccacgctggacaataacgtaaccagcacattggccacgttgcaaagcaatggctcctggccggacgtcaactatgcctacagcgccaccacctatacggcggacgtacacatcaaccgggtaaaaaccttcgcgctggcctatacgaaatcagccagttcgtattacaaaagcaccacacttttcacagccattgtaaacagccttacttactggaacactaccgatccgcaaagctggaactggtaccataaccatatctccaatccgcagcgcatcggcgaaatcctgatccttttagacaccgcgcagcaaagcctgggcagtctccgcaatgccctgcttacgcaaatgagccgcggcaatccttccggtcaggccggcgccaacaagctggatgaggctatacactttatataccggtcctgcctcactgccaacgactccctgatgcagtacagcgtggaccaggcattttactccctcgtactcaccgccaatgagggcatccagcatgatctgtcatatcaccagcatggtccgcaattgtatttctttggttatggttccgtgttcgtgagcggcgaaaccaatgttgcctattatctgcgtggcacaccttatgcgctgtcaggctcccgcttatcggtgttcagtaattttgtgcggaacggtttcctcaaagctatgcggacccgttatatcgactacggcaccaacggccgcagcatcagccgggaaaatcaattagccattggcgttaccaaccacctggaaaagctcaaagtgctggacaccgctcatgcgactgaatacaatgagaacatcgcgcggctgaacggcagccagtcgccgggatacctcctgccctccctgcatacccacttctggcgttcggactataccgtacatcatcgtaccggctacctttttggggtacatatgacctccacccgcaccgccaaacaggaaaacggtaatggagaaaacctgaagggttattacctgtcggacgggtccacgcacatcgccgccagcggcaacgagtattataatattccggcggtgtgggactggagcaggatacctggtaccaccgtgccgtacattaccactattccgctgcgtacagcctggggcgtgaactttggcactaccgcattcgcaggtggcgtgtcggactcgctgtatggtgtttccgcgcttcaattctccgattacaatacgcaggcacgtaaagcctggttctttttcgacaacgaggttatttgtttgggcgccggtatcagctccacggccacacagcccatcaataccaccgtgaaccaatgcctgctgaacggcgcagtatctgccaatgtaaacggctccgtgagcactattgccaatggcacttacagctacaacaataccctgaaatggatcacgcataatggcattagctattacttcccttccggtggccagttgcaactgagcatgcaatcacaatccggtacctggagaagcattaataacggtggcagcaccactgtacagaacatgaacgtgttccagctgtggttcaaccacggcactgcgccggccaacggcacttatgcatattatgtattgccgggtcaaaatatgagcacttatgataccacggccgtacgtattgagcagaatacggcgaacatgcaggtagtatatcacaggggattaaatatctggcagatggtattttaccaggccggtaccttccataaggattcactcacggttaccgttgaccgtccatgtgcgctgatgctgcgcaatgcaggcactcccgacgtcacgttgtccgttgctgatccggcgcaatccgcttcgcctgttaatatccagttgaacctgccggggattccacaaacacgggagctgattgctaccctgccttcagggccttatgcaggctcctctgccacgtatcatgtgaacagtcaaacgcctgtttatggtgcatccgttatcacggctattgcggatgcctatgtaagaggaggttctgcttacggtagtgtaaactatggcaccgagtcgcttgtgctgaagcaggagaccaccacaagctatacacgggaaatatttctccgcttcaatgtgggtgcattacccgcgggtaccagccaggtaaaactgcggatgtatgtgagctatgcaaacaccagcgtcaccactgtaccgtggattgtgcgatatgtaagcaacgacagctggaccgaatcaggcatcacctacaacaacatgcctgccgcgaccagcgctgtggatacgatcatgggacgcactgccggcaattatgccgaatgggatgtaacagatattgcgctctcccagcaatctgccgatggcatgcttactttaaaactggtatccggactggcaggcgccaccaccgatgccacctttacttcccgcgagagcagcgacagcacccggcggccggtactcgtttgcagtacaggcagcaccctgcggaaaatgatgccagcgatggagcagaaaacggatggcgtgagcatctatcccaatccggcaagtgcattcatttatgtaaataccgccgaacgttggctgagagcggaattacatgataccgccggcaaagtggtgaaaatggaaaaactggatggccgtcagcagttcgatatccagatgagtgatatacaaccggggatgtatttactggtgttaaaagcaccaggtaaacaactggtaaaaaagatagtgaagatgtaagctgattttaatactgagctattgctgcacgcacctgctgccgcaatagctcatatgtttttacagtggttactttgtccaggaacagttgtacaataccagcagttctggtattcccgtattgctgtacaaaggagagatattcctctttattttccgggatcagtgaacggagattacttatattttcaaacgaaggcgtattgtctgtgccaaacaggtaatcctcacaatagccgttatattgttcccgggcggtttccacaaagatgctgtttggataagcgtccaggaacttttcccagttgagtgcgcgctttcctatcatgctgaaaggaatcagcaatcccgcatcggcgctgtataatacggtatcttcatctgcccgcagttgcaggaaagcattgtaatcagcgggcagggaagctttgaataaacttgtatagaatgcaggaaccgtgcgaagatcggtatacccctcgcctatttcccagggttcaatacccgcggtggccagtaaatgaatgcgttgttgtacctgcgcaggcagtacgatcatcccttttgtttcatcgtagtagtttacatactcattcagccatgcctgctcattggcggtaataccagccagtgctgtatccatataattcgccagggaactgtaaagccgggcagctgtggccgcattgatacctggcaattgtttttcgatggcttgtttcctgttgatgataccggaaacatatgcttctgtaggcaacgccggaatgtcaacttttttatgcgccggggaatctattctgacggcactaacaacaggttgcttgctttgggattctttgctgccaccattacaggcggccagcattatcacatgcatacaaaaaacaggtatccggatagggaggtgcataaacttgtgcttcatggtataagtcgccggttaattacgaagatgcaagataattattgctgttgcattgacaaattttaatcaggcaccaaatatggcttccctggggctggttaaaccacatttttcattgcccatatttgtatttccatcaacaccggcttcagtgaagtacctttttcggtcagtgaatattccactgttggcggcattgttgcaaaggctttccggttaatgatcttcctgttttcaagttgctttaattcttttaccagcattcttgtattgatgcctgtcacacttctttcgagctccttaaaccgcattttccccgccatcaggttattgatgatggacatcgtccacttgcccgaaatcaggtccatcgcttcctggaagggacatgtttcagatttatttatctttttttcatctttcaaagccatactatacctgttactttactttatgttactacctgccagaatggtaactacttgtaaatgtactggaacaggacgaaatttgcaacgaacacaaaacacctgttatgtcattacaagccatcgaacaatatataacggaacaacttcccaacgttaccaaacttgatagctttggatacaaattcttcttttatgaaacggaccaggtgctcccgtttgtaaccattgccgcatccgataatgagcatgataacaagtccaacctggatcgcaacggtattttccgggtaaatattggtatctcaaaagatgcttacaacaaactgttttcaggtactgaatccgggtgggattatacggcattaaaccgcttcatgcctcatccggattatgccgcgcagcactacatctgcatcctgaatcccggagaagacctgttgcctcaaacgatccggtttattgaggaagcccatcttattgcaaagaaccggttcgataaaaagcaatcggctaaaatgagaaagtcagggtaagccaactacgaagaaattgcaataatgactggtttttgctatcttcatattaccaggaaaaaataacctcatgatcaaacatgctgaagaccctcacagcggaaaacgccaggctgccacacctgtcacccccgcggctgtacatactgcgggcacaggcccacaggcagtgcagctacgtccttttcagcaactggcagacaacagcgacaaaataacgcagcaaaaggccctgcaaacactggcagacaaccgcccacggcctgcgcaactgaaggcagacacctatcaatctcccatacagaaaaaagaaaacaaaaccggcttgccggataatcttaaaagtggaatagagaatatgtccgggcaaagcatggacgatgtccgtgtacactacaattccgcagaacccgcccaactgcaggcccttgcctatgcaaagggaagtgacatccacctcggccccggacaggagaaacacctgccacatgaagcatggcatgtagtgcagcaaaaacagggacgggtacaggctaccacacaattaaaacagggtacacctgttaacgacgataaaggtctggagcatgaggccgatataatgggtcagaaggcgctgcagctgtacaacgcttcgccggtgcgcccgctggctactacccaattgaagcaggaagttgtacagcgcatcagtattgatgtgagcaagctgaatatggtgggtgaagaacacggagagtcgcaaaagcgccggcaaacagaagttgcgtacagtaaccatttattcggtcagactggtctttattggcaggaagctgcgttcaaacccattgaaatacatcaaacacgcggcgatgaagccgggttacgattaaaattcttctaccatctctattcaaaagatatcgtaaacgtaataaaaaccaccaatgatggggatatgcccttcctgatggccgtacgcggtatctggaaaacgatgaataccgtaaaaaccctgtacgacgaggaagtggaaacgctgagcgaagatgaaggactcgccctccatcaaatgataactaaccaggtatggaccggctgccaggctaaaatggacggattggtaacgcctcaaaacgccaacaacctcgaatacaggagagacctggtgactgatatcataaacctgaaaaaatactgggaaaccaagcctgctatttatgaacccagcaagcaagttgccagggccgaccgtaatgatcacatgcataacagcgccaccacagccgccttccagggacgtaaaggaatctggaaagttggagaaaaccacattatcggcatctcacaaatgttccccgcaggaagacactacaacctggtacacctggccgattttaataacgatattaatgcatatattcagagcactaccagtactaccagcgtgacgaaagagaaaaagtgatgctttgaatcacagacataattacaattatatatactgtttatggaaaggcaatggaaccagattaacgaaggtaaattcgtgtttttagtcaatggcgaagaaattggaacatatcaaagaggagacgactggcttaaagaacctacaactttcaatatccgtcaaaatgaatatagtattgagcattcctccggtcttttcagccgtaacagcttcaaaatagtagcgtcaggcgaacctgttttgaagctgaaaagtattccgttttcattaaacttcaatttcgaatatcaaaaccggcaatttaaacttgtctttaatgatacgccgctttggcaatggtcaattatggaaaaggatcaattagtcctttcttataaaacagacttcaccaaaggaacaacaggattatctattgtatctcaaaaagatgctgatgaccattacctgtttgattttttattgggacatctgattttaggtaaaggaaagaaagatgttcaggagtaattccaaatggtgtcagctaatgaattatccgcttgaacgaacttgcacaaacttgatcctgccttgaacaaccgcgctaacggggaaatagtacctttcatatgaaccaagaacttatatgaatctaactccggcgaccatgtacaaacttatcattactttatgtttcctatgcgtcattcagctaaacgcatcaacaggccaaacagtattcgttgaccctgcaaaaggaagggacaacgcaacaggaacaataggagatccactggcaagccttgacaaagcaattgccctggccaatagtttcaccggaaaggaggcggttaccatcaagcttgctcccggcctgtatactctcacgcaacagttggtgctacagtcttctaacccaacagatacggggaaatacaccatagaggcatccatcttgcccgatgacaccggttggctgccctccaaaatgccggttatacaatctgtttctcccaacaataaaaactacgggagctttgatcattgcatcggcttccaggttgaacgcaataacacctgcttcaggggattgaaattcctgggtaacacccatccttctgttgtttactattatgcaatcgagcgccaccggcctgaactaaaagacatggaaatttcgcaatgctattttgtaggcagtaagaattcagcgccaatacagggcgccattttcgcgcaaggcagtggtatcaaagtaagccattgtgtattttatgaatgcaggaacgcacttttgttattcttatctgtaacagggttttccctgaccaattctattatatatggggcttacgaaggggccatatggttcggaaaatattcagattttgttttcagagataatattatagcaaataataattgcttctggataagtatgaaagactacaaagcccaatataccttcaccaactctttaattacagggaatgctattgaaatgggtctgaataacaatggtatcatcgaaaaagatgaagtgaatcacccggttatgaagaatattcagcgctcaggaaaagtgctgcttaccgaaacagataaagacacgataccggtaaactatcttaacctatctcctgcctcagcaggaaaagacattccagccgggatattcaggttaatgagaaatcgttgaaaatgacagatatcttttcctactcttcaatatcctccctgcctaagaaatattctccagataattaagtacttcctccttcttccggctggaaactggtacctgttcattgttttgcatttttaaatatccctccctatagtacttttccacatagtggaaattaaccaggtaagactggtggcacctcaggaagccggcgggcaacagtaaaccctcatagtccttcaggcccttcgacacaaggatttcgcgcttgttcttcaggtagaaggtcgtatatcccttgtcgctcttgcagtacataatatcttctatcgaaacaatttctatatattcaatgcttttcaatgcaagccgcctgggcactgttccgccctgtgccaaataatgctgccgggctatttccagctgctgctggtcaataagttcctgcttccgctggtggaaacattttttcagcatttccgttaaagcggcttcgtctatcggtttcaacaggtatccgaaagcacccatattgagcgcctgtatggcatactgatcataagccgtaagaaaaataacctggaaaccttcattccctatttcatgaaatagccggaagctgtcgccgtctttcagccggatatcagctaaaataatgtctggtttcaaggcgggtatttccctcaccgcctgggccacctcgggtgaattccctatgacctctacaaagggaatgccttgaacgacctgtaaaaggtgcttcaatatgagcgcttcatcttcaagaatataaagcttcatgtatgattattttctggtttagtctttaatttccggtattacaatacgcacggtaacaccatgtgttccgttattgtctttattttcaatattgaagttcgcttcctgtccgttggatttgaaaagcgcctccagtctttctttaaggataattccggcaagggaccttttcttttgcggattctcctccttactggtaaggcctttgccgttatcatccaccaggatgataacctggttgttttccgcgctgaatgataccctgagcatgcctttgtattgaatattcctgaacccgtgctctatggcgttttcaacaaatggttgcactaacataggaggaatcagtatatcttcaggataaagatccgctgctaccgttacctggtaatcgaagatccctgcgaaacgcatctgctgcagctgaagataatttttcagcgaggtgacttcttcttccaggttgataaaatccctcctgctttgttccagcacactgcgcaacagccctgaaaatgctgagaggtaacggacagattcttttgtatcgccggaagcgaccaggctttgcaggttggcgatggagttaaaaataaaatgcgggtttagctgtgcctgtagtaatttttgctcgatgttcaggcggctgttctctaattggagcattttatttttttctttcaaccggtattgccggtgtataatgtagaagaataaaagtatgccaatgaacaccagcgatgccaatgccagcgtccatctctgctggcggatcaccttttcattcaacgcattccggctgcttagctcagcgatattccggtcctttttctctgcttcatattttgtctgtatctccgctactttaactgcttctatctgtttaatatgatctatttctacggaaaaggcgtaatccgctgtctccatggctgctgcgtagtcgcctttctttttatacgcctcaataagtcccttgtaataattgggatcttctttcccattttccctctttttggcaagggcaatagcctctttatagtagtggatcgccgaatccagctggttattacggataaaactggtagctaaattattatacgcatatgcctgcaggttattggttttctttaaataattaaagaagatcctgctacattcaaggcccttttcagattgcccctggcgggcatatacctgtgataggttatcgtaagaccgtgcaattgccatgctgtcgccgatgcttttcgcaaggtcacgcgcctgtacattatacagcagcattttatcataatcatcccccctggaggccagcatgaaagaaatatcataataccgttgccggattacgggatgggatttgtaaggatggcttttataatagcgttcggtatattccagtgattctttttcgttgtggttctggtaataagctttggccatcaggtcgtaaaagcgataggtcagcctgctatgggcgccttccgcttttttcatggcggccagtatgtcgttcattaaagccccttccaccatagtgccgttggcggtgctgttgtccaggaggctgtaggttttcagcagctccacttccacatcgccctttggtccggccatcttcttgtactcggctattgcgctgtcacgttgtctttccaggttataatatcttcccctgaaataatgataaaacgggttcacattgctgtcagcggtgtgccgcagcaggctgtcttcccggtaagtcgcgcttttcattccggcagatgataatgtatccagggagatgatcagggacaggtaatctttccggggcgctgcaggaagggcatttccctgatccttccccggcttttctttatccttgcacgaggcaataaaaagcagggtcaaaaccgaaataaccgcaaaggcggctcttgcattcatcaatgatgtaaatttagctgcacaaaaaaacataaatataaacggttcttctttttcttccccggttttataatgattattctctaaatatataatttaaaacgttcaataaccggcctggtaaatatccagtagctttcatcccatatccgtagcgcctgatccaatatttgcacctgcttccttttcagataagggataagatattttctattatctgtatttttaccggaagaaaacttagcatcaaaccataatggccaggaacgcaattttattacaccaggagcaactagcgccggcaggcgttgaaatagagctgatgaaaagtttggaccagaccgtgcaaatcccgcatagggacgaccattatatgttcatcattcaactgaagggacgctttttatgggagctggattttacggaagtcatcatgaaaggaccctccataagctttgttgcccccggtcaggtgcatagatatatcagctataaaaactgcgagggctggttagtatttgtggacaacgggcaaatatccacacagatccggggaatattcgacacttatcttaatgcccgtcagtcggtggcggttcgaaaggaggatgcggtttttaaaataatgcctttgtttgaagatctccttcatcagccatcattaccacttcaaaaaaacttaataagctccctgacagcaacgctggcgggaatgatcgcttcaaaaataatacagtcacaaaatgccctgagcctggttggcgggcaaaagtacaataccgttctccgtttcaaacaattggtcaatacaaaatgtaaagaactaaaacaggtgaaggcctacgcgtcattgctcaacatcactcccctttacctgaacgaaattgtaaaagaagtcaccggattcgccgccagtcattggattcaccaggaaatcctgctggaagccaagcgtttgctgttctattcctctttagatataaaacaggtcgcttacgaattagggtatgaagaccatgcatatttctcccgcttttttaagaagaacacgggaatgaccgccaccgggttccggatcaaaaaccattaattgtccaatcatagccattagatggctaccagccgttgcttcgatgccgtttaattttgtatccgtaaaatttaaattaataatacgatacaaaatgacagagaaaaaaccaatagctaccctgataacccctattatcatatcagtattcgctatttatcttaccatcggaatgactttgggaatacttcccggttttgtaaaaaacgatttaaaattcagtaacctggttgttggcctggtcataggattgcaatcactggctaccttgctgacaagggcatattcagggaaaaccacggatacaaaaggcgcaaaaacgagcacccatagcggtatattgcttgtaatgttctccggtgttttatatagcatagctgcagccagcagccggaacgccgcattggcattaggacttttaatggtatcgcggattgttcacggcatatcagaaagcatgtcggtgacgggcgcattaacctggggaataggtttggtgggcctggaaaggtccggtaaggtaatgacctggaatggtattgccatgtacgccggcattgctataggtgcgccggtggccatctggatgcaaaggtcctttggaacagggtatgtttttgccgtcatcatattgctgccggttgttgcctggctccccaccatcaagctgccggctttacctgtagatgcctcacatatcaggacacctttctacaaagtaataaacctgattggcaaacagggtttgggattggcattttcatccataggattcgcctgcatttcttccttcatttccttgctgttcactgaaaaacattggggcgatccctctatggctttcatggccttcggggcgtgctatgtacttacccgggtatttttttcttccttccctgataagtatggcggatataaagttgcgctggtttctttaatggtgcaggccacaggacagcttttgattggatttgcctcgtcaaaagtgatggcaatagcgggatgcagcctgaccggcattggcttttccctgatatttcctgcattaggtgtgctggtgatcaaaaaggtagcaccgcaaatacggggaacagcattaggtgcttatgccgcattctttgatctttctttgggactgtcgggccctattgccggtatcattgcaggttggtatgattataaaaccgtttacctgtttggtgcgttcagttgcctgctggccattttcatattgttctttaacaggaataatgcgcccagacaggtatagcacagttatacgcccccatcaaggggcgtgtaacttttattcaaaccgcagcagctttctcatctggtaaaagaatctttctatcagccgcaggtcctgcgtaactatttcggcgttgccttttaattctttatcaaagggaagggttttatggaaagatgtttgaagccctttcggcaaaatgacattcacataataattgccatctttatccggtgcattggcgatatttttcacccggccttccaccataccaaattcctggtaaggatagttgtccagtttcagcagcactttctgtcccacctttaccttgcctgaattggtggctggcacccgtaatccgccgatgagcatatctttatcatccggcatcacggacaacaggatgtctcctgttttcacaaactggttctttcccaggaactgctggaagcccactacaccggccactgaagaggtaagcaggtagttctgttcccaggcgttgagtgattttctcagttgctcaaatagttgtccggtctgcgctgttaaattgatcttatctttttgtgcattgatggttgccccgctccgtgtcctttcaatacccagtataccttcctgcagctgggatatcgcaaggctgatgttttccaggctctgttctgcctgcagaaatttcattttttccaggttcatttctgatgcagaaacaaccctttctttaaacagttcctggtaccggtcgaattcccttttagacagctcatacttcgtttgctccagacttttttgctgctgcagcgtacgtatcctgctccgtgattccgccaggctcttgttggctgctgcataatccggggaataaggctgcaaagtggtataaagttgtgcgtcggtcaacgcgcgggcaaaggcattgtagtccgcctggatctctcccagtttgaaccccgctacttcaccaagtgggaagtgctccactcccgcgttacccagcgaatcaacaatagccctcaaccggatcacgtcgcggtagtcggcagtggattgcagcaccatcagtatctgcccacgggaaaccggctgatggtcggttacaaatatttcctctactttggtattgatcctggcttccagcttctccggcggattccgggaggaaatgatgacggcagaaggaacaaattccgggtactttatcacgcagctcatcgctaaaatgagcagcagtataaaaaatatggtggtattcccccagcggaccatccaatgcggtggctgtgtaagaatgtcctgcaccccttctgagtgcagttgaatagtgtctaagatatcttttctagtttccaagttccagttgattttttacgagccggtaatactctttcctgagcgataccagttcatcatgacttccttcttccactacttttcctttatccagtacaatgatcttatcggcatttttcacggtcgacaaccggtgcgcaatgatcaccgccgtttttccttttaagaactgttccaggttgcccatgatcgctttttctgtattggcatccagcgcactggtggcctcatcaaaaaatatatattccggcgatttgtatacagccctggctataaagagccgctgcttctgcccgccgctgatgccaatgccttcattaccgatcttcgaattataacttaatggcaggctttccacaaaatcgcggatacatgccacatccacggccttgcggagctgttgccggtttatatcatctatccctatggcaatattttttgcgatggtatcattgaatacgtacccttcctgcatgaccacgccacattgatcgcgccagtaccgcgcagaaatattctgcaactgtacattcccgattttaatttcaccctcgcccggctcgtagaacttcatcagcagtttcagcagggtggtcttaccgctgccgctggcgcctacaatggcagtggttttgcggtatggtatacgcaggctcaagtgctcgaacaccggcgcaccggcacctacataccggaaagacacattattcaatgcaatatcctgctccggtatttctatcatcgtttgtacatcagtacgttcttcatcctccttatcgtggatctctcccagcctttccaacgatatttttgcgtcctgcatttgtttgacaaagtccatcagctgcatcagcgggccattcagctggccaatgatgtattgcaccgccagcatcattcccagggtaaggttaccatcgagtaccagttttgccgcaagaaaactgacaaagatgtctttcatctggttgataaaattggagcccaccgtttgccattgttccagcgacaatgacctgatctggatcttaaacagtttcacctgcataaattcccagccccagcgcatctgccgctctgcattatgcatcttgatttcctgcatgccattcaccagttcaatcactttactctgctcctgtgatacctgcgagaaacgtttatagtccagctcctttctcttcctgagaaaaaaagatatccatcctactgataagatagcgcccaacaggtagatcaggaataagcggtaatcatacagcaacagcaccacgctgaaaataaccaggttcaccaacgagaacaaggtatttagcgaagaattggtcaacagttgttctatccggtggtgatcattgatacgctgcataatatcgccggtcatacgggtatcaaaatagctgataggcagtttcatcagttttatgaagaagtcggacacaatggaaatattaatccggctggagagatgtaacaaaatccaaccccggattacttctattcccattctcccgataaacaacatcacctgtgccagtaataccaggtaaataaagttcaggtcgtggttctggatgcctatgtctacaatgctttgcgtcagaaaggggaagataagcgacagcaggctgcccgcaaagagacctattgccagctgggcgatcagctttttgtacctgaagaaataaccgaagaggaaagagaaatccttcctgctccgcggtgttgctgcatctgcttcataaaatgcaggacccggatccagcagcaggacgatcccctcctcgtcgcgctcctgcttcccttttcctatccagccatctataaactcctgttgcgtatattttatcaatccataagcaggatcggaaacatacacgaatgtatccggtcctgacttttttattttgtaaacaacaataaagtgttgctgtccccaatgacaaatacagggcagtggcgcctcttccaacagcgtaataaaatctatctttaccgccagggacttaaaacccagcccctccgctgcggcagacaatcccagcaaagaactcccctcccgcgtggtttccgccagcgaccggatagtctgaatatcggtcagccggccgtaatgcttgctgatgatctttatacaggtaggaccgcaatccttcctgtccggctgcatataaaaagggaatgctttcagtttcatattagtttattgtctctcccagcccgtaccaggcaatggcagcatgcttcaacggattctccgtccagtcctcccaggtgttgctgtacggatcgtacccgcatttaagcggcctggaataaatatcctgtggatcttccacgtaagcccggcaatcggtgcatacatgtctgaactcacaatctttacaaaccgctatttcatctttacggatttttccataccggtgaaatgcctgattgtccaatacttcctgcagcggtgtgtttgttatatgtccgaagttatccggcagtgaaggacaattcctgatatatccgttcagatctatactcagttttctgttcaggcaggtattgtgatgctggctctcggtgaacagttccatgtttgaaacgaagtagctggagcggatttcgccgcaggccaggcaggaattgatatgactgctgaagaaaattacgggcaccgaaccttcgaatattttctccggcttatcaaccggtgctgaatgaatcagcagcgacttcacgcgcggatatttttttaccagtttatccagcgttggcaggtccagcgtatcgtcatacggcagcaccagtttgatgaactttagcgttgtgccgttgaacacttccagtaattcgcggatcttatccaacgctattttcccgtaacacctgatctccagtgcctgtacatgcaggtcgaacagctcgcggaaaaaagggccggaataatcgatagcttcattatactcaataattacgttggtgattgctgagtacctgtcccagctgagatccagcggtatcagttccggtagcagccggtcgtccgtaaatcccagttctttgctcagcacaaaattaatgtaacccataatggttttacgattatcttccccgtaatgggccatgcactcgtcgatggaatgctgttgcaggaagaggaacacatcggcggtatcgttcgggatatggtaaaacctgcgcatttgcagatcgcagagcagcgacatacgggctcccttcacgagccggcagtttgcgtatagatttaaatattccattatcagaatttggagatcactttataaaaattgaaaagctcaaatcctccggaatttattttcggggccttttcaaatttgaggatggtataggtttgctgctggttatcctggtccaggaaatacagcgacagcggcaatcccttcttctctttcagtttactggtgaatttctttttcatgagcgctatttttatgcagcaacaatgctaacttcttttccaggtaatagttgcaagggtaagacaccatgccgaactggccctcggggttaatttcgaggaagtggtagtttccctgcatatctaccatcaggtcaatagaacctgtgcggaagcgcagtgctttcatcagctgctccagcttaagttccagatctgctggtagtttatagggcactgtcctgtttggccgctggttatcgtagttgcggaaatcatcttttgttttccggttgttttgcgaaaaaatagccatcgaatggcactcgccatccaggtaaaacgtgcgtatctcaaacttcttgataatcttctcctgtaccagcgagggaaaaaatttctctggtaccaggtgaagattggctttgttgatggttttggtgagcatcttgtacttttcgccatcagcgtcttctacaaaaatacattcgctgacaggctttacgattagctcgttgcacttatccagcaaatgtataattgcagctttggtggtcaccacttccgtaaaagggatgttaatcccgcattgacgggcaaggctcaatacgtgcagtttattcaggttatcttcggagatggggtcattgagccacttatggcggtcaatggtaaaaaacaagagggaatgaaggccgttgaattcatctaccaggaatcgtttaagggtgtactccgtattaaagtctgcttgtttaagacggtattttacaggaaagctgctgatctttctccggtaccagacagcagccatttcattgttgcctggcagatcatccaggttttgaatatcgaagaagtcctccccattaacccgcaggtagggtatccgcaaatggtccatccactggcaaacatgatccgtggtgccttccaggtgcgattgacttaatataaggatctgttgagacatggtgtacagttgattactggtagtaagaactgccggcaatcaccggcagttctgtagtttccggacataacaatggcggaaggagatgtttattactagtcgcgtttgtggtcgcagatgtaaacatccggtcctgaataatgggtaggcgagtgaatggtggtacctgcgccatcgccggaatcagccagctcgctcacgagggctagttttccgcccttaatcgtttccagggattcaattttctttgcattcagttttttcaacttttccatagtttttaatttttagaggttttacgtttggggttacttgttaggatcattccgggtatcagttacatagtgctgaccgttccacgaagcatggttttccgtggttctttcctggtcttcgaggaagaattcaagggcgagtgctctgccgcctttcaccgtttccggagatgctacctttttggtaaccaatttttctaactgtttcatgttattagattttaaatctgccttaaaattaggcggcaggagcaattccgcggagaggcaaggcatatttgactggttacgatccatattcgtagtacttggggaaataattgcagcattggccaggcagataccggattcaagttggcaccctgtcttgattttcttaattttgtaagatgaaaaaaggccaggcacgttcggtatccgcattcaataacgatctcaaactaaaaggctttaatgccttccagattgaggatgatagtcaggctacccgcttttacagccggaaggacttttataagatttgcctgaccacgggcaaaagcattattcattatgccgaccggagcttccatgcggaaggtacggtgctgttctttggcaacccgcacattccctattcctgggaaaccctgtcgaccacctacgtaggctatacctgtttattttcagaagaattcctgaatgtttcagaacgcgcggatatcctgcagcagtcgccatttttcaagataggtggcacccctatcctgaccatcaccgacgcgcagcggatttttctcaataccattttccagaagatgatcgaggaacagcagagcagttatatctttaaagatgacctgatccgcaattatatcaacctgatcgcgcatgaagccatgaaaatgcagccttctgaaaactttgatcagcataagaacgccgccaaccggatcaccgctgttttccttgagttattggaacgacagttccccattgaaagcccggataagccgcttcaattgaaaacggcacaggactatgcgcaaaatctcgccctgcacattaattaccttaaccgcgcggtaaaaacagtgactggtaagcccaccactgcacatattgctgaacggatcatcagcgaggcgaaggcgctgctacagcataccgactggaacattgctgatattgcctatgcattgggcttcgaatatcccagctattttaataattactttaaaaggatgaccggtaccaacccaacctcattgcgcagcctggaagtttgaaattcttaactattggtttgatagtcataaacagcaaagggacggcccatcctacctttgcgtgatgaaagatattttcgagagactacaagccggggagcccgtcgcgctggatgacccggaatttttcaaagtggatgcagtggttaaccgaacactggccctgtcgccggcactcaatgctgctgccagcgtagaggagataagagcaaaactcagcgaaattattggtactgcgctggatgaaagcaccgccatattcgcacccttctataccaacttcggccgttttatcaaaattggcaaaaatgtgtttataaatcatgcctgttctttcctggatatgggcggcattaccctggaagaccatgtactcatcgggccaaaagtgaatctcattacggaaaatcacccgctcaacccggcagaccgccggagcatgttgtgtaaacccattttaataaaaaagaacgcctggatcggcgcgggcgccaccattctgcccggtgttaccatcggtgaaaacgcagtggtggcagcaggcgcggtagtcagcagggatgttcctgacaacacggtggcaggcggggtgccggccaggttgatcaaaacaatttcctaataaggcatgtccgccttctttactaaaatctgaagcagtcattaatttcaaataaaaattatgcgtaccacatcagtaaaagcatatggcacaccggcagcggaagcgcctttgaacatgcttgacatcaggcgaagaacaacgactccgcacgacgtggagatcgatattctttattgcggggtttgccactccgatctgcacacggcgcgtaatgaatggcatttcaccgtgtatccttgtgttccgggtcatgagatcgtaggcaggattgttcgtgtaggcgatcatgtgaccaaattcaaggtcggagatgtagtgggtgtaggttgcctggttgactcctgccgggaatgccagtactgccgggaaggcctggaacagttctgtgagccgggccccacccaaacctataattcgcccgataaatatctggatacgcctacttttggcggttactcagaaagtgttgtggtagatgagaactatgtattgcgcataccagaaaaccttgacctggccgcaacagcgccattactatgcgccggcatcaccacctattctcccctgcgtcactggaacataggccccggaaaaaaagtgggtattgtgggtatcggcggcctgggtcatatgggcataaagatagccaaagccatgggcgcacatgtggtagcctttaccacttccgcatcaaagttcgcagaagcccaacggttgggcgccgacgaggtggtgctgtccaaagatgaagagcagatggccgcctacaggggcaaactgcactttatcctggacgccgtatctgcggagcatgatatcaatgcttacctgaacctgctgcgggtagacggttcgctggcattagtaggcgcccctgagcatccgctgccggttgccgccttcagtgtgatcatgggccgcaaaagtttttccggttcaatgatcggcggcattgctgaaacgcaggaaatgttggatttttgtggagcacataatattaccgcggatattgaaatgatcaatatccagcaaatcaacgaagcctatgaacgtttgctgaaaggtgatgtgaaataccgctttgtgatcgacatgaactctttgaaaaatgcctcgtaatggaaataacaagaatagcgtccaagccctctgccaaaggaccagccgactggttcaccggggctgtacgcattgatcctttatttgacgcgaacaatgcccgccgggccgccgcggccacagtcacttttgagccgggtgcaagaacggcctggcatacgcaccccctgggtcagaccatcatcattacagccggccttggctgggtgcaacgtgaaggcggccctgtggaagaagtacgcccgggtgatgtagtatggtttgaacctggcgagaaacactggcatggtgcttcggcttccaacggtatgacccatatagccatacaggaaaccctggacggcaaagtggtagattggctggaacatgtaacggacggggaatataagcgaccctgatttccgttagctaacataccataagggcgcccttatggtatgttaactaacgttaccggctatgcgaacaatatttctctttagaaaaagcagtaccggcatcctatagctgtaccaattttggcgtatgcccggtagaaggaataaattcgtttatcacccaggctgtacccagtttgaggtaactggtggtagtgccatcgctgcaaccataccactcttctgccagtatatcattatcgatcaccagctgtacctccattttctcatccagcatcagcccgaatatggtggttgcacctatatctgttcccagcattgatctcagtaattcaacaggcgcaaaggacaggcgggaaatcgccaacgctgcgctcaggtcttttgttttaaaaggcttcccggcggtagtaaccactaaataaaaatttgtttgctgccggttgcagagaaaaagcgtttttaccgttttcatgttcagccgctcatctatcctgatacagtcttccatcgtaatagcaggatcattgtcgacccgctcatacttcacccctctctcctccaacatttcatataccagttgctgtaacggtgttttaaacaccggtggcctggtttgttttatctcactgacaaaaaacatatcaatactcattattatttctttccaaagaaaaatcactggtggtcaaagataaccgataggcgttaaaaaataacctgcgacataaacgggtcgcaaaccaccctttaaattgtcgtatatagcctgcctctgaatctggttttcttaccatctttgttatgtcaacgataaataccagtggagcagcaaccactctaaaaacgggcgaaaccgaaaagccagatgagtaggaacaaaattatttcatatgtcaaacaatactgtttcactccaccgggttcttaaagcatctcccgaaaaggtataccgcgcatttactgaatccactgcaatcgcctcctggctgcctccttacggatttctttgtaccgttcatgagcagcaggcaaaagtaggtggtgctttcaaaatgtcgttccagaatttcaccaccggcaacagccattcattcggtggaacatacctggaacttaaacccaatgagtttttaaaatacactgataaatttgacgaccccaacctgccgggagaaatgaccacttctgtgtggctccggaaaacgatcgcgggaacagaaataaaaattacccaggaaggaatccccgctgtgataccggtggaaatgtgctacctgggctggcaggaatcactggaaaaacttgcgaagctggtagagccggaaataccggatgcctgaggcagcgagcaatatactttcagggaccaccgggtatataatgcctgatgatccctgaaagtatgtcactattggttattttcaagcaaaatgtcaattttgctttttagtattgccgatcgtcccggcgccggggcattgtcatccgacaccgctccttttttatcgataagcacatagcggggtatgcccgaaaaattaaatttcgcttccagcagcactgattcattcttatctgcataataatgctccccgccatcaaacattcttttcacagtcgtgtcccataagttttgatcacactccactccaacgtatagaaaaactatatctttcccttttagttcttttgccattgctatagaggctggcatttcacccatacagggcccgcaccagggagcccagaagtcgatgtatatcacctttccactgtaacgggtaaccagtttctgatagagctgttcctgttgcaacttaaatctaccctgattcccttcatgcgaaaatgtacccgcaagttcctgcttaagctgttcattatcctgttttaccaatgcacaaacaggttgattaccgatatgccgggtcataagctgcatgttctgcggcagaagtggttgccggaattgatttaaataattgctgattaccctcgccaacagaatatctgttccgataccaggaggcaactcccgcgccagccaggtctggatatttaaattgttcctgaaatttttgtaattaacttcatacagggaataaagctgcgacaccaatgcctcctgcgacgggttccggctggctttgggcattttaagcgcccgtttatcttcctgcgaaaccggaccggcattcgtttcaagaaaggcatacaattgcgcgtctgttacatcaatgggtataaattgccatcgtcccatccacatttcgaaatattcccttaaaaaagcagcgtactttccggttaccagggctttggtgttattaatgggaatttcctttaaaaaatcaaaatattctttggtcagcggctcccgtttcccttgccggtgcagccaaccataccttaccagatcctccgcagcccagtaatgtatgtgctgggacatcgcctgccgaaaatcattgctggtacattggttccggttgaacacatccagggtatccagcattcttttcatcacggcaaggcgccaggacttataagcggattgctccagcgagtcaatcattctcttttggttgtcgtaaggaatgatggctggcagctttggccagaaagcatttaagtattggttaaagtgcgacaacccaccagagaaacgaagggataaaaatgtggtgccggtttccccggcagacagttttttacctgccttgaatgctgccagatcgaagtatacattttcagtttgaccaggcaccgcatacatcatagagtagctaccatctatcagcagcataatttcctgtggtgataccagggggaaagtaacactggattttccgccgctgtctaattcgcatggtatcgttgtggtaataccattatagacagagaaatagttcaacttcagatatctgaaagcatctgtctttgggttataaccttcaacaaaaatattgacggtaacattcccgggattaagggaggcaggaacgttggataaagtacgggcctggcctgttaatatcaccggataaataatcaggaagagaataacgaattttttcatagctgcagatcattgacccagtcaggcatcatatctgaaagctacataatataagtgtcattttaacataaaataaataccccggttccggatacttgtctttgcccccttttattttttttgtaccttttgcctgaattacttcacacctttttgcaaacaaagattcagacacccggttgggctgcccccatatgaaaaaaaccatcaaaaacgagtcagtgcttcatccgccgacgaaagcaatacttgagcaggaaagaaagatattgctggatctcggcaacgatattaccaaagtaagagagaaaaatgacctgatcacactttttaaaaacaacattaagggattattttacttcacgcatacgattattactttaatagactataaagacgaaacctattatccatttctgctggataatgaaggatctcccatcagaacccatctgaaatataaggaactggtaaccggccggttttccctgaacgatcccttcattcaggctgtactgacagcagaagcacctgtttcttttctgctggaagaaataatggacaagccccagagcccacctttccttcatgtcaattatgaaggaggggtaagggaaatactgatgacaaggctgatgaaagaaggaaagccaatgggttttattcatttgtactcggaccggacggacagctttaatcatgaattcagaagtgtaatgaatggtatcgcaccacagctgtcgggtgcagtttccaatattattaaaaacgaagaattactgaataaagaaaaagagaaatctttcctcctcgattttagcagtgctatagccaccgtaagaacaaaggaagacctcacccgggcagttcgcacggcgctgcgtaaacttgatcagcaaagcggcttcgtcatccggcgcatcaatgaagataaagcgacgatgagcgcatatgtgtatgatctgggaccagcaggcgatgagaagtcgctcgccgtactggtaaaagcccaatatcctgttaacgatggcttgcaaaaccgcgtgctcaatagtgctattcctttactatttaatgtagaaagagaaatacagagagggatcacatcagcctatctgcaatactggaaaaagatgggcttcgaaaatttcgtgggtatacggttgcgcaacggggaaaccgatctcggaattctgctgctcgacattgaagagatcaagatagacctgctgcagggtatttgtgcacagatatccatagccatggccaatattatggctaatgagcaggtgagcaaaaaacaggaagaacaagcctttctgctgggcttcagcagcgccatcaccaaagtacgcacaaaagatgagctgcaggccgccatcttcgaggtgttggataaaaccatgaatacacagcttgccatgatccgcgtattggaagatgatggcgtccatttgggcgtatttatgtttgaccgcaggctattcggaaacgcccaggcagattttgataaattatcttccagtaaaattaaaattgatgaaacctatactgcacaggtgctcgcaagtaaggaaggaataatattcaatatagatgaagaattaagaagcggtaatgactatgcgaaactttggaaatccaccggcctgaaaaatatgtatggcttaccgttacgtatgggggacaagattatcggcaccatctggctgctggcagattccctggggcccttactcctgaaaggtatctgttcccagattactgttgccgtggcaaatatattagcaaatgaaaaattgctggcttataaaaagcaactggaaatagaaaatgattacctgaaagaacagatcaaaaccatatacaatttttctgaaatcattggcagcggcgacgcgatgcaggaggtgtaccgcctgatgggacttgttgcagcgtccaatactacggtgttgatactgggagaaacaggtaccggtaaagaacttatcgcaagagctattcacaatgcctcgccacgaaaagaaaacctcatggtgaaagtaaattgtgcggcgcttccttccaacctcatcgaaagtgaattatttggccatgaacgcggcgcctttaccggagcaacagaccgccgcatcgggaaattcgagatggcagataacagtaccctattcctggatgaaatcggggagctgccactggaggcacaggctaagctgctgcgtgtaatccaggagcgcgaactggagcgtgtgggcggtaaacatgtcattaaaatcaatgtccgccttgtagccgctaccaaccgcaacctggaagaagaggtaaaagccggccgcttccgcgccgatctgtatttcaggttaaatgtatttcccatcaacctccccccgctgcgcgaccggctggaggatattgaagcgctcacgcagttcttcgtaaagaaatatagcaggaacacaggccgcactatcaggaaaatagcgcccagggtaatacagcaattacgtagctatacctggcctggcaatgtaagggaactggaacatcttattgaaagaagcgtactgctggctaccgacagcaccctgagcgatgtttttattccgcgcagtgcagatgccgataaacacgaacaggctttcctgcagaaccggtcgctggaagaagtggagcgcgactatattattgaaacgctgaaacgctgtaaaggcaagatttccggtgccggcagtgcagcagaagtattacaaattcccggtaacacattacactctaaaataaaaaaactgggcatcaccaagagcgactacttctcctgataaaatcccttaataaagtgaaaggcctggtggtttcattaaatacagtgaaaaacagatgctccagctcttgctatttgattgatttttaatgatttactaaagatggcatttggttggcctgataggtagcatcattaaaaacaaaaatcaaattatatgaaagtcgtagtaatcggaggcactggtctcattggaaccaaagtggtaaatcaacttcgtcaggctggtcaccaggtgatcgctgcatcccccgcaactggtatcaacacgctcaccggcgagggactggcggaagccatgaaggaaaccgatattgttattgatctcgccaactccccttcctttgaagataaagcagtaatggaatttttccagacagcaggccgtaacctgttagccgcagaaattaatgcaggcgtaaaacatcacatagcattgtctattgttggcgtggatatcatgcaaaacattggctacatgcgtgcaaaaaaagtgcaggaagaactgattgagcaatcaggcgtgccttacaccattgttcgcagcacacaattcattgagtttattgccggtatcgccaatcaggctacagaaggcaatgaagtgcatctttcagatgtattgttccagcctatcgcctcagatgatgtagcaaagttcgtggcgaaatatgcactggctgccccgttgaatggcagggtagaaattgcaggacctgagcgttttgaaatgtacaaaattgtggagcgttacctgcaactggccaacgacccgcgtaaagtaatccctaacggtaagcctgcgtacttcggtggtgaagttacacacagcgcactggtgcctgctggcgaagcgcaaaagggtgcggttactttcgagaactggtgggccacacaggcggtgaaagcataataacagggagctgcgatctgttgaaacaaggtgcggtcaacagatcgcagctccctttctaacaatagatgcttacattgaatgtgccgccagtttgcccagcagctttaatttgttccgtacttcttccgaccagggtaaaccgatggaaagcctcatgcagttttcaaactgatcctgcagggtgaatatccttcccggcgcaatgctgatcttccgttttatggcgctgtcatacagttcggcggtattaatttttttattgaactccacccataaagtaagtccgccctgcggccggctggttttggtaccctccggaaaatattccgctatcgtatttacatagtgctggtaattgccctgtaaggtttgacgcaaccggcgaagatgattttcataccggccacttttcaggaaacccgccaccgcttcgtgtgtaacagcagacgatgatatggcatgcaccagcttcaatttcaatatttgctccttgtacctgccgggtgcaatccagcccacccggtaacccggcgccagcgttttggaaacagcgctgcaatacaacaccatcccctcttcatcaaatgacttgcaacatttcgggcgttgagatccgaagtacagatcgccatatatatcatcctcaatgagcgggatacgatgcctggccagcagcgacaccacttcttttttatgctcatcgggcatacagctacccaaaggcgtattaaaattcggcaccaacaggcaaaggttgatctttgaaatcaccttctttaaagcagctatttcaatacccgtggtaggatgtgtaggaagctcaagtacttttagtcctatactcctggctaattgcaggataccggagtaacaggggctttccatcgcaatggtatctcccggcttcgctaaagccatcatacaaaaagataacgcattcatccctccgctggcagtaaccaggtcattttcatgcaggtttcctccccatgccagcgagcggatggcaatcatccggcgcaatgctgcattgccctgcaaaggctcatatgcggtaccacatccctccaattcacgcgttgccttaacgatctctttgttcagcttcgccaaaggcagcaaacttccggaaggaacgccaatcgaaaaaggcatcaggtcatctctccccatattttcatatactttcctgatcagttcttccggctctttgttattacgggtcggagaaggcttgcttacttcaggaagcggaagtttcaggtaaggcaggcggcttacaaaatagccggattgtggttttgattcaatcagcgattgcgcttccaactccaggaataccctcttagcagtgttcatgctaatgctgtgttgccggcataatatcctgacggaaggcagccggtctcctgctctcaaaactccgctcctgatctggccggcaatgccattggtgatttcagtatacagaaactccttactcatttgtcaaagataactgtgtccattaaaataatcaaaactgagactgtgctaatcgagtggctgcagctatttttgcataaaacaattatgccagcagtaattattaaaaccggtaaagagcacatggatgtacaggcgatacatcgtttcttaagtgaagattcctactgggccaaagggatttcgtatgaactggtagataactcgctgcaacattcgttttgtacaggcgcctttacaggtggtcagcaaatcgggtttggaagggtgatcaccgactactccacctttggatggttcgcggatttttatgtattggaagaatacaggagacagggaatttctaaaaaaatactgacacacatattagcacaaccatgggctaagcgtttaaggagaataatgcttaataccaaagatgcacacggattatatcgccagtttcaattcagggatttggccaatccggcatttgtacaggaaatttaccggcctgatattcacctgcagttgcctgaatagtgcgccagggaaacgtcatttccgatttgaaataacggcctgttgtccccgtaccagcgcctcatctgcatctattactgttgctacgggaatattcaatagctggcaggccagtgtgtaaagcggagcatgctgcggccctgccaccaggtatacaggtgtaccaggtggcacagccttcagttctacaccaatgagcaggccgcttaaataaaaacggttatgggcggcagggatcttttttagcaactggttggtgcgtaccataaaggcggcatgcagcaggttgtccaaccttccggcctgtaccccttctgtgaagcaggcgagcgatgccgggtcatccagcgttgcgccgttttctacagacgcggcgaggatactgtgggtagagagcaggtcaaaaaattcgcctgtcatgaaggtttgaaaacgaatggcctggtgacggtttactaccacatgttttggatgcgtgcctggtatgagcagccattggtcctgcgttgtatgcggtaacaatgacccgcagcctgctattttcgtttcttcgccacgcatcacatcatgtccattggtggcgccggaaataatgatgaaccttttgaaagtatgtaccgccagatctgctccgctcatgttaaagggcagctccttgtaaggcaactctaccatgccaatgctggaagatgccatgccggacagcactaccggcgtatcctgcagcggaatgcctgttctctccgccagtgtatcgatctggcgattgataaccgatgcgaaaaaatcttcccgggccagcgatgtttgctgccattgctggtaagtgccggaaataccagcacctgatttttcttctgctatgatgttcaggttacttgtttccaccaatcgtaaccggaaggaactggtgccccagtcacaacttaaaaaataattcatctgctgctgtttaatattcatcatctcctctttttatccgttctacattccccaccaggaaaatatacgagcatgcacccagcagtccgagtactgccacaaaaaccaacgccggcgcaaagttgcctcctcttgccaggaaacctattacaatgggtacaacaataccggccagctggccaatgaagttaaacacaccgcctgtaagattgatgaggtgtttgggcgccaacgtagatacaaatatccaggtgatggaagcaaagcccactccgaaaaatgacagggacataaaaaagataatgagccccggtaggtttacataattagcgcccagtataaaagcagatagcaataagcctatgatgatgggcagcttgcgtgcttttgcagtagacactccttttttcaccaggtaatcagataaaaaaccggaacacaaaatgcctgtaaacgctgctacataaggcacggacacccaataacctgatttaatgaaatcaagaccccggtagtctgccaggtactttggaaaccaagtgaggaagaaccatagtgtggagttcaccgcaaattggccgatataaataccccagagcttacgataagaaagcaccgctttcaggtcggtccagcggaaagccgttttcttttcggccgcttgcttgtccagcaggccgccaccgttttcaatatgctgcaactccgcggcgttaacccttttgtgcctgagcgggtcccggtaaaacaggtaccatactattccccagatgatgccaatgatgccagtcacgaggaatagccctctccagcccacctccagctggatcatagatagtaccggcatcaggaaggccaggccaaggaactggccggaggtatacacagcaatagcagaagcccgctcattgtcagggaaccaattactcaccacccggttgttgatggaaaacgccggtgcttcaaacacgccggtggccatgcggaggccaaagagagaggcaaagccttttgcaaatccctgcataaccgtggtaaacgaccagctaataagacagatggcatacaggatatgcggactgaaacggttcaccaatatgccaccgggtatctggaaaagcaggtaggtccaactgaaggctgaaaagaccagccccagttgcaccggagtcaatttaaattccttatctatttcagaagcggctaccgccaggttgcttctgtccatgtagttgatcactacattcacaaatatcaggaacagtacctggtagcgtatttttgaaggcttcgcattaggattgagtgctttcatgtagtttttacaggtctgtgtttaccattccgccacactgccatcggtatgccgccacacggggttgcgccagttgtggccgtcagcggccattttccttacatgcgcttcgttgatctctataccaagacctggtttggaaggaatttccacatagccatccttgtattggaatactgttttatccgccaggtaatccagcaggtcgctgccctggttgtaatgaataccgaggctttgttcctggataaaagcgttgtggcaggtagcgtctacctgcaggcaggccgccagcgcaataggtcccagcggacaatgcggcgctgctgccacgtcaaacgcttctgccatggagatgatctttttgcattcggtgatgcccccggcatgggaaacatccggctggataatatccacgtaaccttccttcagcagtgttttgaactgccatttggaaaacatgcgctcaccggtggcaatggggatggctacgtgttgcgcaatctcgcgcaggtcttcattgttttccggcagtaccggctcttcaataaacatgggccggaacggctccatttctttggccagtattttagccatgggcttgtgcacgcggccgtgaaagtcgatgccgataccgatgcccggtccaacggcttcgcgcacggaagcgatgcgttcaatggcggcatctatcttttcataactatcaatgtactgcagttcctccgtagcattcatctttacggccaggaagccctgttctgccattttacgggcagccgctcctacttcagcgggacggtcgccgccaatccaggagtagaccttcattttgtcgcgcgctttgccgcccagtagctggtagacgggcgcgttgtaatacttccctttaatgtcccacaacgcctgatcgatgcctgcaatggcgctcatcaggatgggaccgccgcggtaaaagccggcacggtacatcacgttccagtggtcttcaatatgcataggatctttgcccaggaggtattccattaactcgtccaccgcagttttaaccgtggcggctttcccttctatcaccggttcgccccagccaataatgccttcgtccgtttctattttcaggaacagccagcgtggcggcacctggaacagttcatagctttttatcttcataacgatgtattactttttcaggattgaatggcgcggacgaactgttgtgcctttatggcgagttgctgcaaatattccggtgtaacggcaacaccggcactcaccagggcgctgccaatgccaaagccggcagcaccggctttctggaaatctttgatgttctcgggtgtgatgccacctgtaggtagcaggtgcattttaggcagtggtgcggaaatatctttgatataagcagcggaggtagccgggaaaaccttgatcatgtctgccccctgtttgtaggctgcataaacttcagtggccgtataggcgccgggaatgctcaccacacccagttcccgggctgttttgatcacttccggttccagtatgggagaaagtatgaagcgagctcccgccgccgctgcttccctggcagtagcggcgtccagcacagtgccggcgccgatgatcattttatcgcccattttagcggacacttctttgataacggccagcggctcgcttgaattcattgttatttcaagcaggcggatgccgccggcataaatggcctctgccacccgcagcacatctgccggctgtaccccgcggatgatggcaatgatcttatgttcgagtatctgagagagtgtagacatggaatttacgcgtataattgtctaccggaaagataaaaataattaagtgtattttcaacatttcttacactccgggcacgggaacgcccaaacgtaatattaataataccagtaagctacatgaagaactcctctgaaataattttaccatctttcacatgatatacgcaaagctcactcatcttcatacggtccctgccaatcatcttgagatccatggtgagcacgaatgcaataacattgccggcaatcaatggttccgaaacctccgtgccatacctggtttccaccatagcactgaactttttgtctttctcagttaaagcctcccgtcctttggtttctatttcaaagccaggcgtggcatagggttctatgctaactgcatcatcggcatacagttctttttgtgccacatcaaatttttcctgccggcaaagttccgttaaacgtgcagcaatttgttctactgtcataatatgggtttttattgatgaaaataaaaatacacattttatattacaggcggatttaaaagaatcgctatgcggacgatctataccacggagattttccgggtacctgaatttttcaggatcatgtgttatgttacgagtgtgcttatgctggtaatcatgtcccggcttttacactattcaaaaaaataatcactcgatgatattaccgaaacaaagggatccaagatttataacgataagacgtggtggcacattgacagatacccatcatcatttgctggcattatgggccgccagttgcgcggaacatgtgctccacctgtttgagcaggcctctgacgacgaccggccacaacaagcaatagcattgacacgggcatgggtaaacggagaaatcactatgaaagaagcgcacaaaacagcttttgctacaaatgctgctgcaaaaggattgcctgatgtcgccaggtttgcggcactggcagccgggcaagcggtagcagtggcccacgttgcagcacatgaacttggtgcagcagcctacgccatcagagcagcgatggaatccgttcctgaaaatgaaaaagatgaaatgcggcgcaaagaatgtcaatggcagcgggaacaacttccggatgccatccgtgaacttgttcttgacgatcagcaattaagaaataatatatgctggtttgtattcagcttgtaaggagtaagcgacaagtatccaatacttatcaccttatttacttttaagccaactgacatatttttccagttcatcgcctgtttcgcctgccgccaacgcgaggtattcgttaagcagtaccgggtcttttatatattcatcaatggcctgcaggcagccaatcttatgatactgctcatcaacggtgtcccacgattgtttcaatatcgtcctgatatccggatacttgagttttgccagcgccagcagggataaccgtttggtgtattcatcattgctatggtaaaggtttaaaaggatgtgcgctattccgggcgttagtgtatcgaactttttttcaaagcaggcagcaaactgatattttgcatcatcgtattcagttccggataatttggacacggccctggcaagtatcataaaatcttcgactgaaagatcgccgaggttcgataatacaggcgcccgggataaccatgcaatcattcttccaatatcccaatgccgcgcaatgaggtaaagcaaatgagccagatcctcctcatccagctgattgatttgtccggcggccagcagggctgaaaaataatcttctattggttgccactccggataactggcgtcattaacttgcaggtcctgtatctcttgcagggaatagtttgccgacagccattctttaaatgagtttacaaaaatttttagtgtggttttatggtctgtcatagttgcatcttacggtacaaaataaaatagccgtgtgaattatccaacatttttatacatcgaaaaagatttttatgcgcagtaaatcttaaattacataaaaccctgatcatgtctaaagctggactcgcacatcctggtcaaccggttaacaccacgtctctggaaaacttcttccctggttattttgcgctgataatggctacaggaatcgtttccataggaatgttcctctggtcgcatccccgcatggccggtatctttctcggtttaaatatatttttttacctgctgttatggatcattcttattctacggattataaaattcccggtagtggtttggaatgatctccatcatccggccaggggcgtaaccttcctcacactggtagccggtaacaatgtgctgggcagccaggtggcgcttatcaccggtcgcatggatattgcgctggcattatggatagcggggtttgtactctggatactgctgttatatactttcttccttgtaaatattatgaaggagcccaaaccttcgctggagcagagtatcaatggcgcctggctgttaatcgttgtatctacagagtcggtggctgttttgggggccatcatcgccaacagcagcgcacttcactggctgattgcatttatttccctgtgcacttatatgataggtggcatgttttactttgtacttatcgggctaatcctttaccggtggttgtttttcagcatgaaagcagaaaccctcacaccaccctactggattaatatgggcgcagtagcgattattacattggcaggttcccgtcttgtcatgtatgcccgggcacatgaaacactcggtgagtgggccggcttcgtacaggctttcacgatgtttttctgggcgtttgccagctggtggctccctttgttattcatcatgtttttctaccggcactttattgccggcgtgcagttgaagtacgatccacagtattggtcgatggttttcccactgggcatgtacggtgtatgtacgtatacatatgcggccatcaccggtttcagtttcctgaaacctatttccgctttatttgttatattagctttaggcacgtgggtgatcgtgatgattggtttgttcattgatcttttttcagcaaaaaaaatacaagagaaataaccccgttgtcttattcagctatccaaaaatgtacccatgcagcattctctcaataagaaagcggccattatttcgattattgctaccctcgtttgcgtagtgatttcattttatggctccaggaaactgcaaaattttgaccctgctttaattgcctatttattcggaaccctgtttgcgctgttcggaggcatttaccgttattgcgtatggctgcaaaggcctcctacctggatgtattttaaacgcacctggcaactggtcttctccggaaaaatcttcgctcatattttttccctggtagcagactccgtaaagaacctcctgttccagtcttttatctaccccaggggcaaaaaacggtggatagcgcactttatgctggcgtccggctgcctggcggcattcgccattaccattccgctcactcttggctggatcaatttcaccctggaccctgcatccgcattggatccgggagctactaaattatatgctgccaacttcttcggttttaaagtaatgaactttaaactgggatcggttatggcgtttttaatttttcatgctttaacctggtgctcctggtttgttatagcaggcgcggtaatttttttagtaagaagattaaccaatgcgggcctgatcgcatcccagacctttgaaggcgatctgctccccttgattctcctgatcattatttcggtaacggggctgggactgaatttcagctatgcttttatgaaaggcatcgcctatgattttatgtcggtaacacatgccatctccgttatccttttcctggtgtggattccctttggcaagttctttcatattatccagcgtcctgcgcagataggtgcgcatatttataggcgggaaggagaaaagagaggcatggcgatttgtccgcatacgggcaaagcatttacctcccagctacacgtagacgatctgaagaccgtcaccaaacaattaggtttcgatttcaccctggaagacggcacctctcacctggattacagcccggaaggaaaacgctccctgctggccaaggcacatctgaaggcccggcaggaaggcggtacgctgtttggataaacgcaaagaagcattacccgaaaataaaatacgatcagcatggccaaattacccgtttccaccgataaactgattgcccatttcggccctcatctcaactttgctccccaggagggatacaccggcagggatgaacctgatgccaccgttaaaactcattgctgcttctgtggtatgcagtgcggcattcagctactggtaaaaaacaacaaagtggttgggttcgaaccgtggatggaattccccttcaacgaaggacggctttgccccaaaggcgtacagcggtacctgcaggataatcaccccgaccggttaatggaaccactggagagggtggaaggagaaggctttaagccggtttcctgggatcatgcactcagcagggttactgccgctatcaggcagatacaggccgatcatgggaaagatgctttcgcggttttatcaggagtgtcactcaccaacgaaaaaagctacctgatgggaaaatttgcgcgggtagctataaaaaccgccaacctggattataatggcagattgtgtatggtgagtgccggcgccgggaataaaaaggcgttcgggctggatcgtgcctccaacagctacgccgacctggaacatgcggaggtgatcattgtcaccggcgctaatgtgagcgaaaccttccctaccctcacccattggctttggcgggcaagagacaacggcgcaaaactgattgtcatagacccaagggttattccactggccagaacggcagacatacacctcgcgataaaaccaggaacagattctgccctgtatggcgccatgcttaaatacctggcggaccatgatatgctggatcatgattttattgatcagcataccaccgggttccaggaaactattgaagcggtacaggactatacccttgaatgggcggaaaccattaccggtatcgaaaaggaaaaaatacaaatggcagcggaactatggggcaaagccagcaccagttttctcctccatgcacgcggtattgaacatcactccaaaggagtagacaatgtactgggctgtatcaacctggtattggctaccggccgcattggccggccctactgcggttacggcaccatcaccggtcagggtaacgggcaagggggccgggaacatggacataaatgcgaccagctgccgggcaaccgcgacatcaccaatccggaacaccggaaatatattgccggcgtatggaatatcccggaacaggaactgcctggaaaaggactcaccgcctgggagctgatagaagccatacatcgcggcgaggtaaaaggattgctgtctatctgcttcaacccgctggtatctttgcctaataataactatgtgagggaagccctcgagaaactggaattctatgtttgcatcgatttctttttaaacgaaaccgccaggcatgcagatatcgtactggcaggctccctgcacgaagaagaagaaggtaccgttactactgcagaaggccgggtaattcgtatacgccaggccgttacccctccgggaaatgcccgcacagatacttccattatcctggaactggcagccaggctgggagaagcagagcgatttaactacgccagctcagaagccatttttaatgaactgcgcatcgcctccaaaggtggcacggccgattactatggcatcacttataaaaaagtggaagataatatgggcatcttctggccctgcccttccgaagatcatccgggcacaccacgactgtgggaagataaaaaatttgccaccccggatggtaaggctcattttaacccggcaccgttccggcaaccatcagaggtaactgacagcgaatacccggtagtacttaccaccggacgggtagtatcacagtacctcagtggcacacaaaccaggcggatcggcaaactggtggggctgatacccgagccgctgctcgaaatacatcctgaactggcacaacgatacaatatccggcaacgcgaaaccgtacgggttaccaccaggcgcggcacggccgatttcccggcaaatattgtggaaacaatacgaaaagacaccgtattcatcccctatcactggcctggcaaaaaatcagccaaccagctgaccatcggcacactggacccggtgtcaaagatcccggaattcaaagtatgcgcgtgccagctggagccgttgggagttttcacccagccgggcgaagtacctgcatttgacagtatctgatttacacaaaacataataacctgatggaagttaccgcctacaaaaccgatatggagttcttcgtggacatgcagcgctgcattggctgcaaagcatgtgaaatggcctgtgcggaatgcgaaaccaatggccacgaaagtatgatccacgtaaattacgtggaacgcgctgttactatccaaaccacggtgcaggtatgcatgcactgcgacgatcccgtatgcgcgaaagtgtgtcctgctgacgctatttccaaagatgactttggcgttgtacacagcgccaataccgcgcggtgcataggctgctccaactgcgtgatggcttgtccttttggcgtacccatcaaagaagagaaatacgacatgatgatgaaatgcaacatgtgctacgaccggaccagcgccggcaaaaaaccgatgtgcgccactgtttgccccagccaggccttgttttacggcaccagggaagaaattaaccggatgcgccctaacagtacccccgtaaataaattcattttcggggaacaggaagtgacaacgaaagtaaatatcatgatgcccaaaggaagcacctttctgaaaatccattaaactgaacagtatgtctgataaaactgcaaaagcacctcattggaaagaggattttccgatagaaagaaccgaagccaccaaggtaagccggcgggatttcgcccgcttcctttgcctggtttccggcggtcttgcagcgggcagcgcctacgtagctgttaaagcgaatttctttccgccagaagaagtaacaggagaacactttgtttgtaaagcagccagcgttcctgtaggaggtacccgttcctttgttattgaaggaagcactatcccatatattctcatacgactggaaaacggtaactggaaggcatatgaacaaaaatgcacccatctttcctgtgcagtatattataagccaggctccgggcagattgtatgcccctgtcatgaaggtttctttgacgccatgacaggtgaagtgctcgcagggccgccgcccaggccattacctgccctggaagtattgctgaaaggggatgatgtgtatgtgaaagccgggaatcagaatgctgctaaaaacgcagctgccatttaaaaatctatctaacaatattaaaaatgagcaattttaaagatgcacaaaataaagcgcacccaaataaaacaaacacgctcatatctgcgctgatcattattcttatcctgaatatcggcatccagatatggctgctttataccagtcttaataacgccctcggcgaaaacagggatattgccctgccggcatttctggcctcactgtttttattcctgataggtttcttctggctgcatttcctgcctatgggataccggaaaaatgaccgggaataaagggaaatacatcaggaagtctatacaaaagctgcatttaaaaaatcattgagcggcttcagggatctataaatttcagccaacttctttggggcatctttttccaaaagcgctttatcagcaataggacagacggctacgaaatttttcagtttcaggtactcccctaccggatcatctttatcaaagccggaaggaacacgttttagctttccttcctcgctcaaaccgccgaaataatgccggaaactttcttcgcccacaattttctcaaactcccgtacattgccggaaatctctttccggagcgctttcaggttgtccttttccagcatataaataccacctgccagaaaggattgcccaggctggatatgcagatagtagccggcttttcctaccgctatgcttgccccgaaattggttttataaggggctttgttatgagaaaacctcgtgtcgcgatatatccggaaaagtgatttgccggcatctgctttcgctatattcttatcaaatttggtcatttgccctatcagttcttcaacaaaagaaataacatcttcgcgggcatccgtataaatatttttatgctcattgaaccattcccggctgttgttcgcgtctaatttttccagaaatttcagggtagatactttcatgttttagttgattgaatagagcaccattagatgctccattgtcatgtgaggcagcaaagttatggtgtgcctcaaacataaaattgtaaaaatgggacaatgctaatctttcctgtcaaagatcagggacatctttaagtggtcgccataaaattctttgggtgtcagtcctgtaaattccttgaaatccttaataaaatgcgcctgatcgtaatattcggcctggtaagctagtgcaataagactggcaggttcctcattcagcaatactttcagcgaggcttgcaacctgatggtttttgagagttgtttcggactcaaaccaatagctgatgaaaatttacgtactaattgcctgcgattggtattggtttgtttggaaagttcttcaacggaaagttgcctgctggctgttagaatagtttcaacagttgattttacaatgtggtcaatggtggcagtatccgttaaccggctcaataaaaaggcttctatcaattttattctctccgatgttgaatcagcgcttaaaatctcctgcccgatttcctttccgtcctctccaaacagctgttccaatgaaacggctgtattctccatttcttttattggtatggttgtaaagggcaaaaatccgtatggacgaaaacggacaaaaaaagtacctgtttctcccgtcggttctacttcaaggggacgtgtcagttgcccgattacaaagcatttcggcaggacaacacaacttccgtcttccaggtattgtttatacaaatcgccataatgaaaaatcattttcatactaccatcaggaactatggtgtttttcccaggtgttttttctttcgggctttccaaggtccaataacattcgacaagtgacgataagtcctggtggggtttataaatttgatggttcatttattggacggtatttgttagtgctgcgatacgtggcttcatttttagcaacgatcactttccattgtcaaaaataatagtggccacttctcattacaagcgccaatatataaaaataaaatagaacttcttcagaagcagataaccgggtttgtttgaaacgtttgcaactacatttttgttcaaatcaaaacaatcatctgtattagtgggttatatactttaccaggcactttgaagatgacgattttatttccctcattcattaactgttaaaaaatgaaaaataaccgatatctgttaagacagcccatatgtgtatgggcaaggaatatatgctacatcatacctgtttgcattctctgctcattccaactccaggcacaatcgcaacacaccaaacctggcccgccctggtatgtggagcgattcaaagtttctgccggcgccttctttcccatcaacaacaccgacgtttctgttggctctacggatagtagaataggcaccgatattgattttgaagacgacctgggttttaataaaaataccggcaccttcctgcttgatctccaatggagagccagcaggagatcaagatttgacctgagctattacagggtagccaggaactctgattacaggctgcagaaggacattactttcggtgaaaatacctataacatcaatacgagtataaacgcatttttcaatactgatatctacaggttctcctatggatatgcttttttcataaaccctaaatttgaagcaggattattagtgggcgcgcatattgttggtttggacgccggcataaatgtagtgggcgctaatgtgggtgcttctttaaaagataattttggtatcacagcaccactccccgactttggcatatggggcggctacagtttcgcaaagaaatggtatatcaatgccgaggttgattacttcgcgctgacggtaaacgactataaaggaagaatacttgcttataccgcagcagtaaactaccgggccgtgaaaggactggatgtagctgttgggtatactggtttgaatgcccgtatcgacgcggaaaaagacaggctgctcggttactttaaatggggatataatggtccgtctgttacggttagttatacatttggaagaagcaagtggtagttgcgaaacaagaagttctggcgaattaacaataactataatgagatatcccattgcaacctgaaccgccattgatcagcaggcatgccgcctgttttgtcataattgaaataacttacctcagctgttactttatttttatgcccgttaaaaaaccagttggcagcaacagaagtctcccgcttctttgtttgatcggcttccctgttaggcatatagccggcgttacgggccgctacttccaatggttccggccaccagttcaccaattgatgaaagaaaaaacccgcctccacataatatccatgaaggttatcagttttgttattagcgtccctgtcgatgatttgcttccagtgaaattctgattgccagctaaaacctttgtacttaaatgctgtttctatgttggcttgatttacacggtattgcccgggaagtccattctcatatccttcaagagatcctccccctgcctgggaaaaacgtgtatatggacttctgtttgtgattccggatatggctatttctgcagcaggatgctgatggatctccaggtcactgccttcaaaatctaaatagggtcctaagaaattccattgtattcttccgaaatacatcaggtgattatcatcattctccctgctgccacggcctgttcccgtagcaacagccacccaataattaaaatttaccagtcctttaccttcaatatggccatggattgatgctccctgttgcctgtcgaccgtaaaggcccggtttattaccgagcggtccaccatttgctgctcgccgctgctgatccttctttccctggtgtattcaactttccattgacccacctggaatttcagccactcccatttatctatagtaatagtaaaattaagaagatttgcctggctcaattcatactcccagtaatacttcaaccagggtttaaacgcatgtccccctactttcaaacgcgccctgtttatactgaatgtcgcagcccttttaccgttgaagtcatcgaatgtaaccgggtcctggtcttccggcgcggcaaatctgaattgaagcctgctttgtatttgtaacaggaacttattgtccctggtcctgaattcaaatcccttttcaccatactttacggggatataattattagaagtgtctatgttgttctcctgtcccaaactatccaggcttaggaaaaataatatcatggcgataagaaatctgttaggggcgatgaaatacatatgctgctctttagatcccaatccaatggaactacctattcacccttcttccctgggaaaacagttttccagtcaattttcatatctgccaccagccattttctttgtgtggcctcatccagtcccttatccaatttaccaatagacgactgccggtcgtatgcccattcccgctctgcatcggtatgatgtacatacagttcaaggttagggtacttgtttgatgccgtccactgaagcatttgcaggtcgccatccgaattcccacaggccaaaacgggtttacgtcctatgaatttgtggatgcccaccggcttaccatcatgatcgtctataaaatccagctccgccagcttcacaatcaccgggttgccgttattattatcaaatttggctttgatgctgcttccaacaatctgatctttagggataccataaactttctccgcccatgccctcataaaatctatacctccaccggatacaataaaagttttaaactggtgatcctgcagatactttatcagttccagcattggctgataaaccatccgcgtataatgtactttctttaccgggtgcaaagcggtatccatccattgctgcacagatgaatcaaacgcagtggtattcatacctgcatgggtggcggccataatctgaagaatacctttttccccctgcttcataatccctgccatatcattgtttaacacagatttgaaaggctctttggttttccagtcaggatgagccggcgccatagatttcgctttatccaacgcgtaaaaaagctggaaatacataggctgttccgcccatagggtaccatcattgtcaaaggtggcaattctgtctgctacgggaataaaatcggcgccagcagcattggtaacattactcacataactaatgatcctctttttaacctctccatcgttccacgatggcaatggatcttccgtactcaaagagtctattttcccattgctattgccgctggtaccggcagttttgcttttacatgataccagcactgacagggaaattacgattgctgcaaatgaaattatcttgactaaaagagcccataacattaacttcttacccatggtttctattttaaattagttcattgaaaaccttaattgcgaagatgctaaaccatgaatatgcttaagtaggtgggatgaatgctaaaggttgtgtatgcctgggaatagcgttgctatgagatagcagttctatttaaacattcataatcactttttgtttaaaacttaataaatgtgggaatgggtagaaaaacagttattaagagaagtataccagtggttaggtgcttagcatacgaaattctctcagtaccggattataaaagtttttgttaaaacactttgaattacaaagtacttttagttactttgtaattcaaagcatttctctcacttaaaaaggcgggatcatgaaaatttcaagaaaaagatttgttgtcctcttcctcattggtggatttgcctttctttctatatacaacgtaatttttcggtcagtcgtccggctcattcctgaaaacggagcgtcttttatgagcacggaatcacttactggctggaagagcatagtatccacaatgttgtatcctgttaaaattgttctggcgggtcccattcttccacttatgaatctgccggatcctccacccccattcctggttattggatttgctctctactggactatattggcgctcgcaattcattattttattggaaagattaagcgctcccgactaaaggcatgatgattctttttcgtatattaggtttgataatcaaaattgtatcccaataaaaaccggtccctcaaatgtttgataatcataaccgtactgatgttgcacaacccccttcccgtgcagcagcaaaccatcatagttcatctggcatttcgcggccatccatccacccctttcagcgtaaattagcacatgaagcaccgttatctcattcaatagatcaaaacaacgctattactcaggcaaaaacagccggcaatgtcgtgcaatttacgaacaggaacaaggaaatggcaaaaggagctggcataggggcattggcaggggccggagctgccggagtaagtgcttatttaggcgtttcggctttaacaggccccgttggtctgggtttggtagggatgggagctttggctggaggcgcatacaagtattatcagcaatcctatgccaataaagaaatggagcgcattgaaaacgggcagaaaggcttatacaagcgtgttcaggacgcatttgataacggggatattgacaacagcgctttggatgcactagatcacttacaacaggagcatttaaatcttgtcgattatgttcatcgtatgaatttagatctccccctgcccaaagatgctaaatttacgcctgaacaaactaaaacggtccagcaaaattggaacgccctgcgtaatgaaacaggtatcataaaaacaaataaggatgccacacctgaatttaagaaggaattaagggcgatgcatgccaaacttctttctcagcccaatggagctgaattgctaaaaaggttgctcgaaacaaaacaaacgcttgaaataaaacaaaacaaagcgcccaatctgtccaggaaggaaaaacaggaaagggtatatcgtaagcatgagataaatagggaactaaagcaatatggacccgaattggaagagataataaagcaaaacaaggagaatgttgagcgcgctgaaaaagaggagactttagatgcctattttgattcagaaatatatactaagcttatgtccaggaaaagagaacttgaggagcaggttggcagccgtgaagtagaaaaggataaatataattcttccgttgctaacgcagatcctgccggaaaagatgttgagctaagagaacggataaaagatagtgaaatggtgaatgaagataaggatcatcatcctatccctgctcccggatttattgtttatggacatgaactgatccatattttaaattcacgggtcacaggcaaggatcttaaatctcaaactcttggcgacaattggcacaataaagacgaaaagcatacgattgaaggaataccggaagaagctaccgtgcataatattaccgagaataaattgagagacgaccatggcctgcgcaaaagggaatggcatactggaaaatcccgggaagaattggaatatgaacgggacaagaagaataaataaaagctttcaattctcactcagtcttttaagcgctcgaagatggccatatgccccgtgaagaaatctgttttaaatattgcttcttttggggctgccgtttccgccttttcttcgccaaagcttttacctgttacaatttccagcatcctggtaatacccgaaacagattttttattgatccgtgccctttctaaacttaacttttcccaggctggtacgtgtttggcaaagtgattggtttgctgttgctgatccaggtacaacaatgcttccatgaccgtctgctgatcaaaatacagggaaggtgtggtcaggtaatgatcaagatactgatgcaggtatccgatacttttctccgtattaaaataagtaagggtaagggcgtagatatgtcctacgcagcacacttcacttttcagcaaatgaatacctatgatatcgatgaattccgtataacctttaatggcagcaaagtaggcccctaccagtcttgtacgccagttgaagtcgcccaacagttctttggttatctcccgggtgatctttccttttattttctccagggcgacgatccagctttgatcatttttcaagttaatttcgagataatatggcgttacccaatcctggaggaagctggcagagagttcctttgaatttttatgatcaggcagttcatcgaaggggtgagtatgcctgatggtagcaccagcaatgtgcagccggatcattttatcctggtcgttcatagtatagggaatgagattatgtggcgtaaatgtacagaatcatattcaataattattcaatacagcatcattctctaaacaagtccctaataacatgaacatgttattgaaccttaatgctattgctactttctttgctccttcaatgaaaccatggatttagcctaagccgctatcaaaatctgttgcttccaatcaaaatcttcaaaccttattatgctataaccattacttttaacaatatccaaaattacttcttcattcagcgcctttcgatacctggccttatccctggtaacataaattttgtcgttggcaattggaacgctcagcctggataaaataaaacgctgcatttcctgcatcaccttatcattcgtgtacccggttaaacaggtatgggtgacaatcgacagatgctttgccttgacaagctcccgctcttgtataaattcaattccagccgggtttaagtcgaaaaactccaaactcgccaggccaatatctctaatgtatgctacatcaggaagcaataaaatataatcttttaccaattccctaatcgaaaacaggcgggggattacgtcgcagaaccaatgataatgtgaatgggaccattcatcaaaagccaaaagatattttccgttgcccagggttcgtttttccctgtttacaggcatttccctgtgaatcacatagctatctaaaatgtgttttatctggtcctctttcaatggtaatataattatcgggaataattacgaagataaagcttagccgttattactacattacaaattatttcttctgatatctggattgtgtatttcggtaatataaaaaattcatgccgatctttttatcaaagtactatacattcccaataatcttcttccagtgtgacaattgagccggcgctttggaagccacttctttcaaaaactgctcggcaactttctggaattctttcttcagatcagaaagtggaaaggttttgttgcgccattttttactgccgctgccgccgccacctgagatagctgattcaacaatggaaaaggctacctcgttcggtttaaccagcacaaatcgaaaggcgggttgcccctgctccccctcatcataggtgtattcggtatcttttcctgattcgaagttgcggacgactgtgcccaacacattgagccaggcattcaggcatacatctccctctccaaaatagcccagggcgggtaccaccttctcatcgattatgatctgtaagcgaccgtgtacgtgcgaaaaatgatcggtgtttgcgcttggaatgggcctacagctgcccagtcctattcttaattgtcccataccggtaaaaataaatatttatcctgattcccaaaacaagaaaagcgatcacggttagtgctggatgacaaattgtataagaaagaatcaccatgatgctaattggagaagaagtgactttgtttcaacgtttttagtatcgcagttgtcagccggtaaaggtcgccgcctgcctggtcgtctttttcgttagtaagcaggataatggctgcctgctcatttggatatagcgaacaaaagctccggaatccattagtacctccatctatcctgatataataatcccaattccttgtcctgccaattgcccattgaaagccgacagcgtcttcctccacgttaccataaataacccggtgggtgagttttaccgcagcatctttttcagcgagttggtagtcagcatatttcaacatatcatctatgcaggaatgaagccctcctgcgcctggaaaagaaacctgtaccggctgtgctttttcaccactggcagtataaccgtcaagttttgcagcagcacgatttacaaatgtatttgtcatgcgtagcgggccggttatatagcggttgatcaacgtttcaaagtccacctggtaaatatgttccaatgcatagcccaataactggtaacctacgttggaataggcatattttaacgtcttcaaactatccagtttgatttgctgcaggtgatccaggaaataagcttccgtcattggaaccgatatgtcaccatccgtaaaactatttggaaacatcgcggtatgactcagcaagtatcccacgcgtaccggttcccccgatggatattgaagtgtggggaaatttccaggcaagtacttccggatatcttcatccagtttcattttgccttcgccgattgcatgtgccaccagcaggcccgtaaatgttttagtgatagatcctatctcataaattgagttggaccgtgtcagctcttttgattctggagccgtttgcccgtagttatagcgataatgacgctgatgatatattaccccgatggatatacccaccctccctgttttacttaaatataattttgccgaacgatccaccgtagaatccagttgggtttttaagggattgttgttcaacacctgagctgaacagttgaggtatactccaaaaaaggcgataatgatcccgattcttttcatggctattattatactttctttcctgttttcttaaacgctgtaggacttactcctttataccttttaaaaatacggtttaaatgactttcgtctgtaaagctaagctcataggcaatttcactcatgcgcatatcactatgtaatagcctggtttccactaacctgattttgtaatgcgtaatatagctctgaagtgtttcaccggtttgctttttgaaatacctgcccaggtaatttgtcgaaatattaaaatgacggcttaaattctccgttctgagtttctccgattcaaaaatgtttacttgtatataattcaatatttccaaaattggctcacctgtattttcctttatattcttgggcaattttaacgcaatatttcttgctacaaccgtaatgatggtactgataacctgttctgaaatacgggtatagtagatctgttgcctggtgtgctcatcaaggatcgcatttaccagtgaaaaaataaaaggtttatccgttttattttttaagatacacccgggcctgtgactggcattttgtaaaatgtatgttacatgcgtcaccgtatcctggtccttacccgatttttccctgatatatgattcattaaatcttagaaaaaagaaactggtcttttggtcaatatcaaaagagtaactatcctttggcgttaataaaaataaatttcctttccggtatttaaactggtggttattgacaaactgtacgccggtaccttccataatatagatgagctcaaagaaattattgcgctttacaggtttttcgaagcgctgtaactccttccattcgatttcatattgttgatgtaaggttcctcccggcatgttgtaaaaatacaaaattagcgtaataatgtacaaccagcatgacaatctccttgtatacatttgctcatataaattctaataagatgaaaattctaataattggtgcgggcggcactattggtaagaaggttactgcggcgctgaaagcgcatgaagtcatcaccgtggggagaaacaccggggatattatggctgatatctcttctccaactgccatggaaagcttatttaaacaagtgtcagatattgatgcgatcatttgtactgccggcgatagcgttacgggtcccttgccggagatgaataaagcgcaattcatggttggcattgagcagaagttatggccacagattaacttagtgctttccggcatgaagtatctgaaggataatggttcgatcacgcttatatccggcaaaatgggtgaacttcctgctaaaggttcgtcgggaaaagcatttgtaaatggagcgatcaacagctttgtaatggctgcggcgcaggaaatgcccaggggaatcagactgaatgctatcagcccgtctaaagtttcagatactggcggggatgaattaatagcggcttatgtaagatgtcttgaaacagcaataaatggggaaattataagagtaggttattataaacagtaattaaaatgaagcatattctatatctcgtttttacgatgtctgtctcttttgtacagggccaagataataaaggactatcggaccagcaccaattctggggcacctggtcgcttatctccgttgaaaatataatcgccgatggcagtaaaattgctccttatggcgaacatcctgtaggaatgctcgtttttacaaaagaaggaaaatacgccatccagatattaaaagctcaccggagtaaagttttagccaatgataaagataaagctaccacagaagaaaatgcggcgttagtacggggaaataactctcatttcggaacctatactattgatgaaaacaaacaggtaattgtattcaatatccaacatgctttttatccaaattgggagggaattacgcaagtacgtacttattcattgaaagatagtattcttacatataccgtgactacacctacaagcggaggcgctgcggtggcgaaggttgtatggaggaaaaattaacaaataatcatatcttaccggggtatttacagcggaaatatgcatataaactatatggatttaaatagcggagtggcaggtttttcacaaaaggattaccaattaaagcgtcatgcccatttccctatcgaagtagctttcagcttatcagggcagttaactattgaaaccgatacccacaaatatgctaatattcaatctgccattattaattcaaatgtgccgcatactttcagttgcctgaacagtgaatgccagctgtattttataaaccccgtgtcttataccgggaagaatatcctgaaatcttaccttagccataacgaagacattttaattgatcctgttgaaattgaacctttcagggaaaactatatactcgcttctgaaaatcaacatccggctttaaatgacatggacagcagggtgcagctaatcctggactggataaaagcgaattatgcaaccgaccggataaatattgtcaggcttgctgaagttgcttttttatcagaaagcaggttatcacatctatttaagaaggaagtaggcacctctattaatcagtatatcttatggaaaaagattgaaatggctataaaacatgcactggaaggctcctccctcaccaggtgcgcctactcttccggttttgcggactcttctcattttattaaaacatttcagaaaatgtttggcatctatccatcttttgccaccaaaaaatagcaggattatacaatttatcttgtcggcgtcgtcccaactttgcttctaaacagcacaaagatgaccgacacaataacagccattaacaaggcaatcgttcaacgactgtacaaggaagtactggtgaactggaatatgtcactggtggaggagtttgttgcacctcattttatatctcacgactggccggaaggcagcccatcaggtccggaagcattccggacttactattcaaccgtcatacgctccgtattaccggacgcccgctatgaagtggacgacctcattgcagaagggaaccgggtagtagtgcgatggaggcttttggggacccatcaaggcaacttccttgacatcgctcccacaggcaggtttatcacacttgagggtattgccatctaccgcctggaaaacaataaattggcagaacgctgggtggtcaccaatctgcacgggctacttgaaaaagcaaaagacacttcatcagccaacgtaaaacaacactaaaacacaagatatcatgttatataaaattgcgctattcttacacattataggggctttaatggtatgtgccgccattgctattgagtggctttgcatcatccatttcaggaaaacagctagtatggaccgcattaaggaatcgcttttctattattccaggataggtatcatcggcgatataggagcgctcctgattcttgttcctggcatatatatgatggtctccgtttggggtgatgccaggtgggctatatttggttttttggggttgatactcataggcttaattggcggtatcataacagggagaaaaatgaaaaaaatcaggaaaataatgaaagagaataatgcgcattcgcaggagttagaaaaacttataaacgataattcactgtggttttctatcaaaatgcgaacagcaattttcctgggggttatttttttaatgactataaaacctgaactggagggttccatcataacgatatccgtatccatcatacttggagcgcttcccttgcggatgaaatatgagccatctgctgccgggtaatacgctccaacctcatattttgttacaactaaagcagatccggttaggtctggcacccgcctattccggaattttgtcatctcaaacaagagatttcaatcaaacattgtatgaaaaaattaatctttattttaagcatgatcctctcttccttcgcgtacggacagccacaccatccccgtacttttctcttcgttcccggtgcatgggacggtggctgggactacgcaaaggtggattccattttaagcgcacatggcgacatcgtttaccgcccaacacttacaggccttggagaaaaggtgcatctctccaaccctgatatcaacctgaccacctacatccatgatatactgaatgtgatcaggttcgagaacctgcacaatgtcatcctggtgggtcatagctatggcggcatggtcatttcaggcgtggcggagcaggcgcctgaccgcatccaacagctgatttacctggatgcaatggtacctgacaacggagaaagtgcaaaagacgtgtgtggcgacctctgggagccaatgaccaaaggcaatatcaaagacagcatggtgctttatccttttggtcccacaaagcttactccgccgatggatgtgccacaaccattgaatacctttactgaaccgctgcagatcagcaaccccatggttaaaaagattccaaccgcctttctccagatgacgaaagacggtaagggaagtccggcacacgataaaatgggaatattgaaagccagggcaagaaaatggaaaatctatacactggagggcggacactactccatgcgtgagcaaccggaaaacctggtaaaaaagctggaagagatcgtacggtaatagctcccggggaaaaggacgggtatatgcctgaggcaatcttaaaccatttatcagtaacttaggatatggaaaacagggtgatacaccggataaaaacgatcagtgaataccataaggtaatgggccttcccaagccggaacatccgctgatcagtattgtggattacgggtctatacagctaccctgtaaagcgagtatgggtttcatgttcgacttttataccatccttatcgacagggattttaaaggcaacatgaaatacgggcagcagtcgggtgacttcgaggaaggcgtacttttttttatggcgccaggccaggtatttgaagtgagtgttgaagaagcggaaagcatcaaccgctcaggctgggtattactcatccatcccgatttcctatggaaaactacgctggcaaagaaaatcaggcaatacgactttttcaactatactgtgaatgaggcgctgttcctatcggataaggaagagaagtcgatccttgccatcatggaaggcatggcgcaggagtaccggaataacatcgacaaattcagcgaccccgtgatcattgcgcagctggaactgcttctgacatatgcggagcgattttaccagcggcagttcattacccgcaaaaaatacagccatacgatcctcgaccgcttagaatccttactgaatgaatatttcaacagcgaccggctatccacagaaggaatacccaccgttaaatatgtggcctcctcattgaatgtttctgcaggatacctcagcaacttactgaaagtgctgaccggcaaaagcacacaacactacctccaggacaggctcattgaaaacgcaaaggcgcaactatctactacgaatcagtcggtgagtgaaattgcctatggattgggttttgaacacccgcaatcattcagccggctgttcaagttaaggactaatttgtcgcctttggcgttcagggcaagcttcaactggaatgcggacgctgaaggatcaacagttcatactaaaaatgaggtactaaactgatccggaaataacatcatcggaatataggcattttgaaccgtttgcattccggtgcagacggttcaaaatgcctatatttatataacgcgtcaattgaatcatcccaaaacatacgcattgctatgaaaagaaagcatcatggcacaaaggtgctgcatatggttaacgccacgtccccggaagttcagcattattttgagatcatgttcaaagatttaaaagtacatctcccctttttctcagacgcattaaaaaacgctattatcgatagctgtgaagtatgctcttttaagaggaatgctatcctgctggactatggcgaaacctgccggtactgttatttttgcattaaaggactggttacgggaagatatataaaagatggggctgaaaaggcgaagtggttctttgcagaacatgatatgattatttcggtaaagagtttctttaaccaggtagttagtttggataagctggttgccaaggagcctactatatgcctggctatatcttgggaaaaactggaaaatatttatgccgaataccccgagttcaataagataggcaggaaactaacggagcactactatgagcttgcagaggaaagggccatgtggatcaattacactgcagaagagcgttaccacctgctttttaaagaatatcccaaactggaaaaccggataacggatacagatctggcctcctatcttggcatctcccggcagtatttaagtgctatcaaaaagcgctgtataaggagtcccaggcagcggatacccggataaaaaattgtcatatatcttaacaatcttctcaaatcagcctcctaattttgaaaatgataaaataaccctgctgtcttcagcatctccttatgagtattcagcgtttttcacctcaaaataagatatccatgattactcaaacaaaacaagcgccccaccgattacaattattagccgtagtaagctgttaaaaaagcccccgcatgcctgcgggggactcttaaaactgttctgaattgttgcaactttcctcagaacaggtagcagagggtgttcctgctactcatttttaacagcggcctgacttacacctgtcatgatgctgcctgctactgctactacctgggctacttcccctactatagacgggagttgtaccggtaaccctatcactgctgctgcgagcgcagtgagaatgagccctatgttgcgcaccttcacaaagaaaggtggtgtgggggcaattaatcgttgtactaattccatacagcatttgttttaaagagtgaaaaattacgcatccttaaacgctggcggataccgccatcaccttcatggaattgtatgtaccattggacagcttgtaaggctttccgttcactacctgtacaaactcaatgctgagtgccaggaacatcgggaacgtgctgttgggagaaacggtggcagtgagcttcagcggagcggtattattgctatccagtaccaatacttcgctggcagctatggcactttcatacttaccgcctgcaaagtcgatagcacaaacgccacaggtgataatgaagtgcgatgcccctgggggtgattgaatgccttccgccgggttgaagggcggcagctctattgttccggtaccggccacgcgatcaatgttagccgttaagggagcaaagagtgaggtatccatcaaactattcatattaaactcaaagctttcaatgaacccaacttctccgtcaattacattccgtaagccgcgatcgctggtagcatcggcctttaccacttttacgaattctttcgtgaggcggggggtagcccctttgtccgccgcgttctttatcatatcacgaaaagctgtacgtagcagtttactggctttgcctgcgcggccaaactcgaggccgttttcgcgggtgcgtttgaaggccgggtcggtggagatccgggctcctgatacgccagatcttttcctgactgcgtatccacgctttgttttataaaacgataggttttcgattgcgccgtcaaattgtagcaatccgtcttgtttactcataattaaaatgttttttcttaaagaataggcagtttctatagctatgcctgttaagcttttccatctgatcagacagggttgtacttcgaaatacgatacgaaattattcactggcagaagtgtggaaaaacaaacccgccgcttttgccgctttttgccggattatgccgaaaaacgttcgcaataggatggtgatctacaccaaagacattcaaaacatcatgggcaagagcgaccgctctgccagggagctaatgcaaaagctgcggcagatgtttggaaagcaggactggcagtacatttcagtggctgaattttgtgaatactccgggttggatgaggaggaggtcagggagttcctggacggataattcggggtcctaagtgtattgggagtgtatgcggagagtattgtgagtgtattacgagagtatggagactataaggggacagtataaggactgtatggggaatacgacacatagacgactcctaagtaaccgggaagtatgtgacatgtatgctacatgtatgggagaagtattctgatgaacggtattttaaaaataatcctgatattttaaacaattatgcttctgcctggttattgtacctgtatcctttcattcatttaaaacaccacaatgttatgggaaaatttgttatcaaaacagctaaaaacggccaaaactattttgctttgaaagccggtaatggcgaaactattttatccagcgaaatgtacaccactaaagccgcctgcaacaacggcatcgagtctgttaaaaccaacgcgccgaatgatagccgttatgaaaagcaaaccgctaagaacggtgagttctatttcacgctcaaagcggccaatttccaggttatcggcaccagcgaaatgtacaccacctcctccagcagggataacggtattgaatccgttaaaagcaatgctccgggagcgagtgttacagaggaataaaacacgaagggctgccgcggcagccctttttcacttttggtcgcttccggcaacagcgttgatcaaaccattaacaagctcctctcctatgctgcggatccttttcatttccgccttgcttaacgccggcaccaccttgccttcattgccccgcatcttcctgtaaaacgttggcgcgctatagttacattcttcgcaaacgcgctccctgaaaagaacgggcagtttggagaactccgtatgcaactccagcaatatattcttcttttggatttcaatactcataaagtaaatttgaatagtgatggtctattttagcaatactgatccgctcttctatctccagggaatgaagcgtcaggaaaaaggtgcggaagtaattgccggtaatagcggcaatggttccatctatccccttgtcgccgtcaaccagtatttcaatgtactgatcaagcgcagctgccaactcatccagctcaatacccgcctgaaaacttgacaactcatacagatcgctttccagctccgttaccagctccctggtaaggtcctccgcattggttcttttcagcgcatccctgaggttaaaagcagctttagtggtggttctgaacaaggtgtagaaggtcataaaatcggcccgctggcctggggaccagttattggcggaggtactgccgataacattgcatagttcgtgttcgcatagctcgacgaagcctgcggaggtgccacaggcggtaatgcgggttaagatggttaacagattttccataacagatatttaaagtgaataaatacagttttgaataggcaatacgattccggatcagctgtgaaggctgactaaccggtcgttgtaatatgcgtttatggaattggaatgagggtaccggagataaaaaagcgcggtccccacctttcacttttgaggccctgagaaaccgatgaaggtcgaccgcgaataaacgcgagtcatcaacttcatctgttcattaagattctcaggttttaaaagcgaatgtttatgatatctaatgttgaaagaattgaaaaactattatttttactttataagtaaaaggtgttttatcaatgttttaaatcagattttcgtctttttaattgacaatacaaaaatacttaaaataatgacatattcgtcattattttaaaaaatatttcaccccatcttgtacacatggcagaacaaataagaaataataatctgttgaaaggaatagcaacgattcttaaagaattacgtgaggctaaatctttaagccaagaagaagtttataacgatactaatatacacgttgggcgtatagaaactgctaaggcgaattctacagtcagcacagtagccgcactctgtaaatattttgacattacactttcagacttttacaaaagagtagaagagctttaaaatcgttgtattaacctaaaatatttatgccagatttttcccttaagaaaactgagtaacgatattacggtgcctcatgggaatatgatttactagttattagtaaacttaataaaatatcctagtatatatagtacccattttgaaataaaagtgtattaagaataatgatgcaatttctgcaagttggtacatattgtaaaagtgagcggtagtcgcaaaaagaaaaataaatgaaatcgattaaaataaaatcattcgatcatctaatcaaaacgttacaaaatccagagtattgctgtggacatgtagtatttagaggcgttacggacaaagtcaatcataaacttattccatcagccggtaggaagatacaataccactcagcgaaattgaatgaacttgtggatcatgagcaactcatcttgaaactttttcggcacagggcatatggagagctaaaaaagttacctcaaaatgattggacatggcttgcccttgctcaacatcacggattaccaacaagattattggattggacgtatagccctttaattgcagcttattttgcgacagaaccagaaataaaacacgatggtaccttgttggatttgccgaaaggttgtggtgcgatttacgtattacacgcctgcaattttatagatgcatatgacgatactcgtagcccatttgatattaaaaatgcctcattggtttacgctccagtggtaaccaatcgaatcgcaggccaaggtggactatttactatccatccggatcccagaaaagagttacaggatgtttttgaggacaaagagccaaacggcgcacagtggattcataagttggagttcgattataacgtagctattgatattcagaagactttatacttcctcggtgtccgaaagggtggtatttacccggatttggatggcttttcgggcgacatcaaaaacaggtttgtatttggtgaatgccacctgccaggttaaataatttgtctcatttaaaggtcttttgacagatccactccatgtacgtcgatttttctgtatacttgcgtatgcgcaaaaaattgattctgccccattctcgtaactttaaacatatagagccatccctgaaagtgctacaaaagctgaacaaaggtggcatgataaccctccaaaagccaggatcttccctacatcaattagcagtgaacctggtcaagaatacagggaaaggttttttgttgacatttcctgatgataaaagggagtatcatagcctattggatattgaaaatgttggtttccaaagcaatatcggcgattttaagtgcggtaaaataattccagttgaaacagattttaacactgtaacggcagaagttagcacgttctattccctagattttagtttgctaacagcctcttattttcggctaatgatcccatttgaaagtaatcttcattttcattatttcgtagataggaaatcgtttaaaaccaaaaacaaaagatcaggtgaatgcgtagggattaattatgaagaactacaattggatatgtacatatatcgtgctaaggatgcaaagcagtatatggtattagatacgacagaaaaagtgcagtttaaggcatttatggattattgttttgatgccttagtagccctgggttatgtcagcggccactttattcagaatgagggttacttcttccaatatccaaacatggaaatggaccatcccacagcgtatcactatagtgaattccgaaaatcctgccaaaccagttttaccccgatatatgctaatgcgtatagctatatccgcgacacgtcaatggccgaacaagtacataaagaactgcagccgctttctattaaagaattttctctcttgtgtcaaaagatcaatcaatcgatagaattttctgctgctatattattaatcattgaagcctgttccgcttcccaagtaatgatgcctgctgccttcatggtagcacttgaagcactcacaaatgagtgggtaaatggacccgtatccaaggttaagcccatccatgatactaacaaagctaaagcaataaaaaaagaattaatggctgttttgcaatcgcatacggttgaattggatctcaaatctgtagccatattgagaaataaaatcaatgatatcaatcgacctgttaatgcagatcaactatcgaagccttttgcagaattaggattcacacttagccctgatgatctggaggtaattatctctcgtaatgattttttgcatggccgtattacgctgattgatatagacaaaggccgcctacccgctcagtatacagacgaacttagtcggcatgtctatcactgctgcttacgaatatacacattgctaaccatattgatcctgcgccaatgtggttatgagggtaaaatggtcaactatcctaaaatacatgaacatattaccggtaaaaagttagatgaaccctacttccgggatgtatgttatgtgagccctattgtgctccattagtataggtatgggaacgaagatgcgtttaaataatctataatatccttttttacgtgatatgcgaatatataacctatttcttataatcatacaaaaataaatatttgtactcatgggagcaaacaccagttaccattctttacaatatgcacgatgttaaaaaggttatcaccagtgctccctgatcaaatatagctttacctaaaattactttatgtaaagtgcttgaaaattggtaaattcattagcataaattgaagattggcaacagcactgtccgagaaaacactataccgatggagaagattaccgactttttctatgatctgcgtgacagaaccagtaaccctttgtttgtttcatttataattgcctggctagtttacaattggaaaataccagttgtcttgacattatatcatttgggtgacctacagctggaagggtataaatcgtatgtccaatatatcagtggaaatctggaaccatggcgctctttcttcactcctttttgttatgctgttggatacactttattcttccctcctatccggatgttcattatggcctttatgacgttgataaaaacaaaaagtaattcatggaatctcgaaatatcaaaaactggaaagatttcatcagcccattttatcaagttgaggcaaaaatatatcgatcagacaaaattagtgagtgacgttattgagaatgaaagttcagcaatccagaaacttgcggaaataaatgataaggttaatgtccttcaacacgacctttctgttcaaaagcaaatacatactgaactctccggaaagattgaagcaattgatcaatatactactccttctattcttaatggctattggaaatataaatatcgctcacatcctggatccattaatttgtcatttgagtattactttattgatggtgaaatatttcatatatccgatgatatagatcgaataaaagtcaaagcatttgatatacaccatttttgttttaacattaagacaaatgaatttgttttcatccgcaatcctataggtggtggaactcccgaaattcagttcttgaaatttgctcaggcaatgaatgtgatggaagggaatgatcagcttggtgctgcgattagttatagcaggcttggggagtcggcaatattaacaacatgaatattcattgctattaataatttgtatacatactctattaattgagtaactccgattaagacaagctaaatggttatggtttttcagcgaaaaaattctatatactatggaaataattttaaaatacactggtatcgctgggttagcgttaacgattttatttcttgtatttaaaggcataataaaaaaagagattttcccttcattaactaagcgacaaggctataatattttaaggttaattattctttgcgtatttatactttccttattaagtcttgctgcttattttatgttaagctacaactctagtgtactttcagctgatttaatcaaagctgatacttctccaaatattgtagcagataaagttgttttcaacaaagggcagattggaacagtaatacaaggtaacttaatacaaggcccaaacgaatataccaacattgatgatggggagttcgaaatatttgcggatgaaaatgatgggaaggagatttttgtcaataccgtcataaatgatcggaaatttgattcgtcgtccctggattccaataaaatgttttataattatcccacttatataaatgaactcaaaacgaaatttaaaaccattactgacggtggggattatgtttcaagttcaattacagcattaaaatttacggttttgcacatcaccgatcctaagatagccaatgaaattgataaagatggacaagcaatctcttattattattctgaaccaatgcaaggtaatgctcttgtaacagttataattaatgagaagaatatgggattaataaattggaacaggaggcaaatacatatcaaagggaagtttttggtaaattttcaaattggagggcagggatttaacttcataacattatccccagtctaaaagatcatgccactttcattcaagaaggttttatgttctttagagatacaagtatttcaagatatggactttttccatttcatattattatcaactacattaatgagagctttgtttattgctttagttgtgacacttaaatctacgtatttgattgcgcaggtagaatcctccagtaataaaaatactcctgcccatcctctgctgataaaaagccataataatgaacaggccacaacaattgatgccaaagttgtatataggtccaatgccggttatgccaaaatttataaaataacagattcattatatgagtttaaggcgtgggaaaacaggatttatttaaatcgtactaacgttgaagagttaaaagaagcagcaaggatgctggaaaaagcggacaaggatgataaggtttcattaactacgtttcggtgtgaaatcaccaaggggaaaatgcttggagctgatgtttattgggttgaactattcaaacaaaaaagtatggtcgatttatcgaatctaagtcctgccgaaataaatgctgtacttaaatcaagcgatgttagtaccgtaaaagatgaaaaaggcgaaatagtggcaacaaaggcaaaaattgttcagtatgaagaaatgattaagagatttggaattacaaataaagacctgagaaatatcattagtattgagtagtagattttacaggagacgtatatcgaaccactaaagtaaacaaggtcgactatctatttatcacatttacaaggagatagaaggcataaaaaagggacgagtttagagacttctaacttaaatcgtcctaaaatactcataggtttctatcatctacgcaggcagcctttttcccagactcttcgtatagccgccaagcttgggtaagatccaaacctctctcatgcctcgcattcaagattcattgctcaggcaattccattgtttttcattttcctgtaaaaacatcatatcttcctatatcggtaaatttaaactaaactgagttaaaacatgctactaaaaacgtagcccattttgaaagaatatattacgcatgacaaaattacaagagatagaaaaaagcttggtttctatcaacgaggctgtctttcagaacgtttgtgattcaatattatatcacactgaagagaactgccaaaatattgttagaacaggcactacaatcggaaaacaaaagacctgcaaaggaacgccagatacttactttattcttcccaacgggcgttatgttttagtcgaatataccacgaaggacaaatctgaaagtaagaaggcattcttaaaaaaagctaaggatgatattgccaaatgcctagatgaaggcaaaaccggcttgaagactgatgagattgaaaaaataattttttgtttcaatagtaggcttactacaaaagaggtacaagccttaagagatttttgtacacatcaaggtatcttattggaactcagagggattgacacaattgcttttaatcttattggaccatgcaaacacacggcgaaggaatatttaggtattacaatcgacacagggcagatcttaccccccaaaatctttattgaagaatatgagcactctgattttgcaacgcctttatctaataagttgtatgggcgagaaaaggaattattgagcctgaccaacagtataaaaaacaatcaaattacaataatatccggagcaccaggagtaggtaaatcaagattggtcctcgaagcattatcagaattacaaatctctaataaggagttaaccgtactttgcctttcaaataaaactgccccaattcatgatgacctaagagtctatctggcagaagataaaccgtatgccatatttattgatgatggcaatcggcagtcaaataatctaaaaacgttacttggtctacttaaagaaaagcgtacaaataaaattcaagttgtaataactgtcagggattatgcactaacaggaattaaatcagagtgcattgattataaggtggcggacttcgagttattaaagcttgactatgctcaaatagagcaaattttgcaaggagaagattttcaaatatcgaaattccgttacttgcaacgtatagccgaaatatcaaaaggaaatccaagattagctatcatggcagcaagggtagctattgataatcaagatttaacatcattaaacaatgtttatagtttgtatgagcaatatttcgaacgaacgacaatagataggccagtgttatcggataaaatattgcttaaatcgataggattgctctcctttttttattcgattaatttagaaaatgtcgactttgtcagaaggatatgtcaagacttttcaatcgattatcatgagtttaaagaagcaatgctaaatatcgcaatatgggaactagccgaactttcgcctgatggaaatataattagaatttctgagcaaacactcgcaacatattttttctacaaaacctttttaaaggaaaggagtttggattttaatactattttgactaactatttccaagatcatgttcaccgatttaatgatactgtgttgggtgccaatagtgcttttggtcacactaacgttttaggaactatcgacccatatttatctaaatactggcagtcaataaataccgatactattatagcacttaaatttctaaaacttttctggctatataggcacgaagacatttacgaatatacagagcttgttataaataacctgccagaaataacatgtgttaattatatctatatcgaggatctaaaaaatagaggttatccccataatgatgaaatcatagagcttctttcaaattgctttccgtacgaagaatttagctacctcgatgcagttgatctatctttccaatatgtaaaacgtaaacctgaatgctttcaacaattattagatttattgattaaaaacttttctattgatattgaagatttatacaatggatgtaaaaggcaaaaggccctactcatgtttttaacagaaaaggtaaattatgatttgatttataaccaatcactattttatctgctaccaagctttttaagctatagatcatacaatagttccagaactgataaaatcaatgcaacaacaattgttacgaagaagattaaaatcattgatgcaattgcaagtttcagaagcggcatatggtcgtttgttattgacaattatccgacttataaatcaaggcttgatgatattttgctttcatttatctcagatggacggcagtttgcaaaagtcgctcatgaatttgactatcaatattggataaaactgtttaatgatcattttaagaaaaattcattacaagacgttttccttattcaaagtttgatatataactataaatggcttaatattcgtccgaaggacataagcaatctcaagtctcgttttctgacagaagactataagacatacctgatactcagttttaatagacttcgcgataaggaagacgtggatttcaccaactacgaacaatatcaattgctaaaggaaaaagaaattagaagcagcttcaacttcaaaaacgttgcagaattcaaaaaattctaccacaaatatgttgaaatgtccaaattaaaagataagggttacactcaaatttctgtgtctttagacatactcattcatgaacattcactgcgtgatcccaatttagcatattcgttcttaaggcaaatcatttccacaagtaacgaaactaatttctatccaatcagagtactaagtgtcttttttacatcacaagataaaatcttcttagactattatgaattgttgataaattcttcttttaaaggaaaagattggtggttatggtctttctattaccgattaccagacgaaagtgtaacattacaatatgcaaatgacctcctccagcttctatcaacgacaagagatggaatatatatcgaatttacaatctttgagaaatttacaaaagttaagaagcaattttttgtggacgctttaaatcgtgttattgcaacaaaatcggaaaataaaagaaatatacaattagatcactctttttttgaaaagtattctgaaatttacatagaacatgtcgatttgctgaagcagatttacttacttttcgataatgacagagatcatttcgattatgactgcaaacatttattggcattgataaaattggacaatagttttttcttcgaatacttcacgctaataacaacaacgcaccttcccttgcattccagggagtttgatcatttgtcaattatctggaatttaactaatgccgagacacttgttgaaaatgtattagatcactttttactacgtgataagcgtcatttcatggaggagattatcgtctcactttttaaaaatattgaatcaatccacatgacgcgaggaattcaatttttgaaaaactatttaaaatccaatataaatgatagcaaagcgtgcaattttgtatttgattgcgttcgcaattcatttagcgatcactggcacgtctttatcttatactatctatcccttgaagcagattttgaaaaatttaggcggatagagctgctaaataattctttttccagcaatggtgataaaatatggtccgacattagagccaatgacttagaaagcattctggaaacgatcaataagatccaaataaagaagtatcggtatagtaagcacaaaagttacattaaagaatggattttagctgaaaggcggcaggcagaccatgaacgcaaaatgcgtttccaacataagcattggcactagaattctagaagttaattttcgatattgtaacctttaaaggaggttagcaacgagaatcactcgttcttatcgtcgagcttcttactatggtcaaggttggtgttttagctgtgttctagcgcttttggtttgtagcagaactaaatgctccatttttacattagcacccaatgcttcgacctgtggaataaatgttgatgaagaaaaggcaaatagataaaacggtacactatcccataatatatgcccccgtcatgcctaatacagatatgcaaactaaatttaagtatgcgttaaatgactaataataagtagtacaaggttgaataataacagaaaatgataaagcaaatacctataataacgaccaatagagcacagccgccgcttgttattttcgaattttgagtaattgcagcaaattatatattaattgggagatgaaaagaactcctaatgctgtagtttttttttatagcacaaatcctttttataaattaccgaaatgacttcaaatacattaaatataataatttaaatatgacctatactccaccagaattctacaaatcggctttcaattgcccctcatgtgctgcatacgctaaacaaatttggactgaagttcatttaacaaatagatctgaaaactactcagctggaattggcgatatattatttgcagtttgtgaccattgtaattcttactctatttggcgcataaattccaatgaccgccgaatgatctatccctattctggaaatgcaccactacccaactcagacatgcctgatgatgttaaggcggattacattgaagcaagaagtatcgtaaatatatcacccagaggagctgccgcactgctaagattagcaattcaaaaactttgcagaatactcggagcatctggagaaaatataaatcaagatatagccttcttggttgcaaatggattaccagaaaaactacaaagagccttagataatattagagtcgttggcaataacgcggtacatccagggcaaatagatttttctgacggccccgatatcgccaataaactatttgtcttcataaatattatctgtgacaatcaaataacacagccaaatcttattaatgaattttatgatgaagtaattccagaaacttccagagaccagataaccaggagagacaatagacccaattaggccacgggtaatactaaaatataaaatttatttcaagaataattcccattattattaaaaaaataaatacatgaaagttctaggaaagaagattacatcccttacccgtgaggatataaaaatacttattgacgacaaaattgcggaatcaaaaactctggattataaagaggtttttaatgtcgctgatgataaaaaaaaatgaagagttcttaaaagatatatcggccttttataataccgagggaggaacaattattttcggtctatcagaaagaagagaggggaagaaaaaattgggtatccccattttaccggatactgataaactaaccattgacgattatgaaaaggaaaaatcaagaatatcacagatagttctttcaggtacaaatcctaaaattgttaatctccaatttagtgatctattggatatagatggttgtagggtttttgcaattggaatccccaaaaacatttcaattccaacaatggttatctacaatgggtctaatacatttcataaaagaaactatactgacaaatatatgccagatacccatgagctatttagggcctttttgagtcatcatagccttaaagaagaagtagctgcttttataaagtccaggacagagagaatttacgaaccattctctgaaggtttgagaaatttaccggtagtaataacacatatggtgccctcaaacttccaagatataattgccttggattcgttcagcactaaagaatttaaagaatttgcaagtaaaatattccagccgactggttttgctcaaaaacaacagcacggctactcattcgaaggactattccttctgcaaaaagatgatccgatgaatcctcaatatatgctcagggataagcaaagaggccatacattgttgttaagaaacggatgcgtagagtccatcaacaatatattttttaatgagatagaagaaggcgcaaaatattgtactctgtacattagggttcttgcggagttcttaaataatgcggtcagcaatgcctttttatattatcaaaattaaatatctctccagacttttatatttctataagcctatataatttaacagaattcacatcattagttgataaccttacaattggacacataaaatgtccatctttaaatcttccaataatgcatatttcagaaatcgaacaacgaaaagaaacactaggccttttgtttgatatactatggcagtgtgccggcgaatctcagtgtcctgatgaatttaaagacacgtgcttctcccccagctaaattgcatcgcaggatatatttgcgtataccacttcattatagatgacagatatacttcttaaaagttattaattaataaaggaatactttgaaaatgggcttatatagaactatttcatgctgaaaggagtttattaatctggaaacatattgtatagcatattgattacttaaagatatctagaatttatactcatttattcaattggctgctcaaacgatttatattattatcgttgcaccaactttaataggtggttaatggttatattcgatttttccctatctcacaactagtacctaatggcattttaatgcctatttcatacatcaaacgaccaaactataaatgcaatgccctaaagccttaataaacttaacgatatcaaccgtatcttgatgagatatactctgaacaattcctgttgaaatatctatatcagattcatgaacgatctgatttctcctaactataatattctttaattttacttttacatcatcttccgtcatcttcatacatttagcaacttcctgccatttatgagtctcgggccaaatcaaacttaatgcggaagttactttgtcaggatcttgaaatgctaaataactatgtgctgttataacgaattgagaaaatatcgcttccttcggaagaaatgtgctgccaaaattgtcatactgctccaaagaaatttgaaatttctgatagcctttagtagcagctctcgttttagtgaaaatttcgaccattcctattcgaaccaattcatgaactaacttgtcaaatgcagataccgcatacacaatctcacttcttagactatcttctatatcaccgggatttagcttgaggctatttattaggtgaagataaacagtatctatattggcaattcttatgaagttctcatcaaactgttttattgaattaagcattggctttaataagttctattttcttttcaaagtcattaaaaatcttattgaaagattttcttttgtctttcatttgggccaaaacagtaccggtacgaccgatttcgccatcttttagcgcataaacaggcagcccatatttatgagattgaggaagaagactttgaaaatcgggtatttcagcaatgcaataggtgtcagatatatctatactggtatagatagaatcactcaataacataccattagtccttaaacttggtaccagctcagaaactacagttgcatttatttcatccatattattcctaaatggagtagcaggaaggccattacggatattaaatcgttgaattactgtaccaccaaacttcggcttcttatctggaaatggataagatgcatctttaaacgcctctttcatctgatttgcgacattataccaccgcggtaatattcgcgataaggtctggatcgccattaatgaaaatggatctggatttgtcggaacaataaataaatcggagatgctaaataaattctggttaattgcggacaatcctgggtttaaatcaattaaaacatagtcaatttcgtaatggctacttgttttctctattaaggcattaaaggcccccggcaaattttgcatcgtagcaaatgcactcggtgccgtttgaacaaaacttagttgcggctcaagctcagtcaaattaggatgccccggcagtaaaaacagatttttgtttcttttgatgttaaaacactctacatgggtaattggagatggctggcttttgaaagcagaattcacacctgacattaggttgttctccttcgtagcagtatcaatgtagtactgatcaaatgaatcctgcataatcaaccccgtaagattacattgaggatcagcatcaacaagcaataccttattccctttttctgccaatttccatcctagatggaatgtcgtagttgttttacttactcctcctttatgattaaaaaaaacgattctcatagattttatttaacataaagttataatatatttacaataggcaggaataatctttttaaggtgtatatgataaaggatttttcgaaaataaagcaaattttggatcgctccaaccagccaataattagtccagggaaacttaagccaatacgagctttgacgctgtacgaaaaagcgaggtgagtacaaagtgaagctcctcttttttataaccaacattaagtagacatcatcaccatactactaatgtggacagcaagttaggaatgaatttattttctttattaaaacaataataacacttagaatggaagtcgtaaattcgcaaagatagtttcgctctttgtaaagccacgtaaactcaatagccaaatacaatctttatagagtaaataatagagtaaaaaacaaaaccccacgctaagcgtgaggtttgtaatcttccagtgatccccttgggactcgaacccaagacccatacattaaaagtgtattgctctaccaactgagctagggaatcttccttttttgtttaacggagtgcaaagataggaatttctaatttacttccaaactcattttgaataatttatccacatcaattgaaatgaatatataaaacgccctttctgcacaacgcagaaagggcgcaaagcaaatcacctggaagaaacagacgaaggattaaacttcgcatccagcatcttcataaaataccctcctactacactcctcgcctggaaccccaccatcttcccatcagtagtttcatgccagtcactcagcggtacccgtgtagtcgtgcccgttacataggtgtataaaggcgctaccagggcctcaaagtcggaagagttatcggtgagtacagccgtccacataatccagtcggatttggtgtaggttttacggctgtccagtggcagtccaaatttctgttgtttggtgaggtaaaagcttgtttcctttttgtataccgccgcaggaaataagttaaagttgagcactttgtcccataccatgttgtacttctggctccaggtgtttttgctttcgaaagcaagactgaaatgatcgccatcatcagcgagcttcacccagttggcggccatttctttggcggcgttttcgtatttggtggctacgtcggtaagcccttgctgtttagccagcatggcgtaggaacggataccggcaattgctttcagggaaagattggtattgcgggcaaggtggcctgcaaagtcgtcggtacataactggttagcggggtcaaagccttctttcagcaggtattccgcccaggtggtgagggttttccagtgttttttggcgtagtccgcattaccttctgcgcgggcaatggcgcctgccagcaccagcatgttaccggattcttctaccggcatgccttcgccgtaggcttgtccgttggcgagtggataggtgcccaggtcgtgtgcagcgtaaggttgtgtgtacttgccgctttcggagaaatagaagatgccgttcatcatgcctttcagcaggtccgggttgtagagcaggaacagcggggccgatggataggtaacatctaccgtattgatacaaccgttgctgaagttttctttggaaagaaacaggatatctccctgcggactcttagccagtttatgcgcggaaatcgcttgtctgtaggccagttcgcagagtttggcgtacgtttccccgccggcgcttacggcatctttatacagctgcgcattgaatttcgcgcatttgtcgaggatggaagcgtaatccgtgtaagcagcattcagttgtttgtcgatggtttgggtagcatcatttttccaccatgctttcaggttggtattgaaatactgtaaagcgtaaagatcatcgtagccgagcaggaacagttgttctttcggcgtggcgtttaccgtgcccaggtccacagcggtgctaagcaccagttgcttatcctgtttggtgctggcggtggtgccgttggcaaatgcggccatggcatcccctgcgttgctgatatattgtaccgggcgtgtggcggtgggtgtggctacatacatataaccccaatctatccgcaggtcgtcgcctttctttttcagtattggctgttctttagtgccggctttcagaatagaaagctggccgttggtatatttagtagcagtaactgcctgtgcgggcacgtttacgctgatgttggtagaggcgccaaagtatacctgcacattatgggcagcgttgtcgttggaggttactttataagagatgtaagaaacgggcctcgacagcagcatcaggtcgtccatcagcaagggcgaggtaaaggtgagggttacatctgctttgccgcaggtgaactggtagctggtttgggtggcgttgatgttcaccgctgtctgaatccctttctctatgtctttgttgcccggcggtggtaccaaacgcgcaatgccggcatccaggaaggcgccgccggcggtattcaggatgtgtacggccagtacattgcctttgggctttaacttgctttttacggcatccggtattggtttgtagatgtactgattcagccagcctttatgcccgtaaatttcctccccgttgaggtatacggtaatattatcatcatgagagattttcaggaataactccgcggcgctcaggtcgcccgcgtcaaaggttctcctggtccacagctccttgctttcccagcgggtaccgccggaggccacgttatcgccgaatggcgcttttcctgatttccaggctttgtcgtcaaaggaggccgccatccagccgtccgcaggggcggtttcggtatacttcacctggtatggcgcttcatcgctggtagcggctatggcctggtagctctgttcgttttgtcccagcaccctgtaagtaacgccatctaccttcaccaatccggtcagcgattgagccgcgccagtccagtgtttggtggtgctgccattcaattcgtcggtagccgaccagatactgaaataaggatcatgcgtaatcaaaggataagacggagccttttgttgtgccacagcgctgccgccgatgcccagcagggccaaaaatgcgagtgttttcaccataacgtgatttgataaatcgattaagcgtataaagtacagttaataaaagtattacattttccgggggattcataaccgttcataaaaaaacctccccgttactggtatatcgtccatcaacgtggttagtactagctgtcgaaaaaaatatctccggagaaaaaaaggaaaaggggaaacacaaaaaaaacgcaaaccctactcccgccttggaggccctgagaagccttgtcagtacgttttcggatctgcgcgtatcttaaattaattaaatgcggtgcctataaggagcgcaaaaatacacttttacattaaattcttcgctaaatcttggggaataacgcaaaccattccggccgcgaacggatcaatgtggcaatgccccatatcagcaacgccatacccagcgcgccccacgccttcttatccttccagctccaacccagcactaccggcagctcccagtacttgatcagcaaatacaccagcaacccgcccatgcctatccaggtaagtaacagcatgcccagctgcgatcccgttaccactaccccaaaaagaaagcccagcgtaaccacctgcagccagatataatttttacccccgctgtggatcacgtctgcaatggaaataaacaacaaggcgcctgtgaggaaaatggtcagcatcagcaaggcttccctcagcactaccggcagcaataacaatacgccccataccaccagggatatgagcacataagtggctgcacgctgatctttgggccgtaaccgctcgtaggtaaacggaaacagcaaacggctcaatgccttttccatgctccgcaacggcggcaacgtaaatatcccgatcatcgctggcacaatcacctcatacggataccacacatccgcgcatacctgcattacccacaacacggcgcccgaagtaaggatcgccggtacggatacatataaaaatgcctgcaacggcgtgttataatgatcaaaactctgcaggatgatatgcgtatactgcttcgcaaaataacggcgtgtaaggatagccgttagttgtgtccacaacagcaccaacgccacgtgaatcacaatggtacggatgatcagctccgggatcagcggcccccagtaaatgcccgccagcgctactatcagcaactcccagctaagcatctgcggcgaaaataaccgccggtaaaagggatacagatgccgcaccagccattgccaggcgcccggcaggtacctgccaatcaactgcacggccgcaaaagcccctaccagcgccgccagtcccagcaacagcctcgaagcggtaaacacacccctgagcgcctgcaaacgcgaaggcttcttaatggtataggtcaattcagtattcgttagcaactccgttgccagcaacttaccctgttcaggcgaaatagctcccaacgccggctgatgcacgcgccagaaactgtctgcctccgcaggactcgcccaggtattcaaggtgccatattgatacaataacgttctttgctcagaactaagagaggccaggatcttcgccaacgcagcatctgttgcaaatgccgcctgactgaaggttaacaggaacaggaatatttttatgatacgcatagatagtatcaaaaataataaaaaaattcactttgcaaaaaagaagaagcggatagctgaacagccacccgcttcctttatcttaaaaacatttttttataaccccgctcccagccagctgtctggtaccggttgcagcttactgccgttcacgctgtattccagcttcagcgtgtatccgcctcccccttctacaaacgccactttaataggatgccatcctttctccagcgctacctgcccgcttttctgcaacggcgcatgccagccatcgttgttcaccacttcctggtcatcgatatataatacggcgccatcatctgccgtcaggtaaaaactgtagatgccggtagccggcacattgatataaccatacacccgcgcaccaaacggaccgccgcccttacccattccttcgggaataatggcattgctcacacgcatggagctatcggcctgctccttgatcttggtagcgcttttgtaggcgccctcaacataatccagcttcaaacccggccgcgcatcttttaccacggtagctttgcggtaggcctctttgcggtaacgaagggtataaatatcgccccggttgcccgcaggactgaaagccgccagcctgatcgtttgcggctcacggatcacgtagttgtccggtaacacggcggcctgcccaccgggaatagtaccatccgttgtatagcggatagtcatgtccgttagtggcttcttcacatggagcgtcacttcgtctacaaacacattatcttctgtaaaaccatccaggtcaggtaaacggtagtgcacacccagcaaatccaggcgtttgtattgttcgttgaggcgttgcaggtagtgatcgtactcattccggttggtccataatacttctgccagcgcagtcatacgcggcataaacatatagtcggcgcgtttctcggaaggaatgtattctgtccacatattcgcctgcgcacccatgatgtgcgtagcctcatcggccgttaagccttttggcaccggctgaaaatgatatacattataaatggaattacgatccggaaccgcatcaaaatacagcgggttgcccggtgtcatgatcacggagttgccatgccgtgccgctttcacaggggcatccggcacccaggagcgccagtacatcagcaccgcagtaggactgatacctccttccagaatttcatcccagccaatcagcacttttccttttgagtggaaaaacttttccatgcgcttcacaaaataactctgcagctcttctaccgttttcaggttattggccttcattacttcggcacacagcggagaagcagcccagctggttttctctacttcatcggcgccgaggtgaatatattttgaaggaaacaacgcggcgatttctgtaaacacatcttctgcaaaagcaaaagtagattcgttacacgggcaaataggcgtggaaaaattcttgccccagcctatttcaccactgcaggcaagaaaaggatacgccctgatagcggccatcatatgaccaggcatatcaatttcaggaataatttccacctgcctgtcggccgcatagcggattatatccttcatctgctcctgcgtataaaagccgccatacagcgttttaccatctttatgaataatatgctgcgtatcaatagccatgtccggattggtagcggccatcttcatacaaacagaatcctggttattaaattccctccaggcgccctgtgtagtaagcaacgggtacttttttatttctatgcgccagccctgatcatcggtcaggtgcaggtgcagcttattcattttatataacgccagcaggttgatatattttttgagataatcaacagagaagaaatgacgcgatacatccaggtgcatcccacgccagccgtaggccgggtgatctttcaccagcatagccgggatggcgatgctttttaacgccgccgcatgcgctccttcaatggaagcaggcatcagctgtcttaatgtttgaatggcacggaaaaatcccgccggtgtgcgggcggtgatcagcaactgctgctcactcacgtccatcgtataatcttcctcgccggcaagcgcagcattctgctgcatcacaatagcgccttttacgggcttctttgttacccgcaaggatgctcccaatgcctgcgcaaataaagattgcagctgcgccgcttcggtagaaaattgcgcccggttggccggcaacaccagtttggtagcaggtgtaatgacaaatgagccggtcctggcctccagttgttgcggataaggaattaagggatagcgctcagattgcgcaaaagtagcctgcatcagtaaacacaaagcccctgcaagcaaaaaaatcttcttcataaaaaatctcattaaagcatgatgtccaaagggcaaacctaataagaaacaaggccccaaactaatgggatcttcacttatcatgcagctatattcatctctgacagatgttaatctttataatctgtgatcttcagcagttcaaaaaactcggcttcccgcagttcccttacttcgccgggttgcatgtctcccagcaacaggttttcgatagacacgcggatcagccgctggcagcggtgatgcaccgctcctaccattttacgcacctggtgaaatttcccttcggttaacgtgatcagcagccaggtatgcggtactttaataggcaactcccgtgggtgatcgaacagtccctccgggcgcgttactatttccacgcggcacggcgtggtaatgtactcctcgccttcccccacgcaaataggcaccccttctttcaaacgttgcagggtggcctcgttcatctcgccttttacttttacgagatacgttctttcatgcggtaccttcccctggaacaataaccgcgtcacctttttattggtggtcaatatcagcaacccttcggagtgattgtccagccggccaatggcatgggtgccctccgggaaatcaaacggcagctcccccagcaacctcacatcgtgagagctgacaaactgcgacaccatatcaaaaggcttgttaataatgaagtatctgtgcataagaggctgcaaagtaagttatatcagcaggatatcgatccggtgcgcctgtaccagctgctgctgattggaccaggagaatatcgtaaagtatccatcctgcgaggctaccagcgcctgtgaatcgtgctggtcgtgtacaaactgtgcagcggacaaatgccgcgttcccccgatggcagacggatgtatcagcgtaggcacgccgccttctatcggctcggccagcaatactttatcaaccggccaggcatctttggcccgggtaatcttagccccgaaggccagtaactcctgctggtcgtttacaatagtggcgccgtctacagcggtaagtccggtgatattctccacttcgcggcgaagtgcattctgccagaaaatttcggtcacgctttttccgtcatagcgcagcaaatcggccacccctgaaaaggcagggctgatgggatattgaagcgggtgaatgatagattcgcgccaggcgtcgctgttggaaggcgttaccagcaaaataccaccccgcttgtgcgcgcgcatcgacacggcaatttgtatcaatacattcacgctgttgttccataaacaggaaggcgttaagcccagcagggacttcaggatcggcggactgtcgggcagcaacccgctgtcttcgttcaccaccttcacctggtcgccacggagcatggccacattggtaaacttgcccaatccggccgcacggcggtgtttcaccaccagcaggcccggctccgatacatccaatacaaaacagaggttgggtaattttatggtagtgccccatacgtgcagctcatcgcccaccggccatacgccaatatgaatgccagggcgttccacgcccggcgccagtttcgtgagcaactgcggcgtaagcagcaggggtttctcaaaaagcaggggcttgccggcctgtgaaggcggcaaaaacgccagggaaatccggatggcgttcccttcttccttgcgcaagctggcccaaaaggccacgtcaatgatcttttccacctgccaggctgccggcacagtagccagatcatcttctccattctccttcgcagcgcaaagatgtttcttaaaatgtgcttctatcgttccggccacctttgcagcggcctggtatgttgcgtcgtttgctatttccataaatcctggtcacatttaatcgtccttatataatattaaaccgctaatttaaatcatttcggaatagcaggaagcatgtgaacttttctgtccctgctgttgtttctctacctaacgaccattttccttcctggcgtgaacaccatcagcaatcttcatcgttcccaattcactacacccaaaactccatttgtatgaagagtagaatgcttatgctgttaggtatgctcctgaccggatggctgtcatccgccactgcacaaaagaaaccaaacattattatcctcatgtccgacgataccggctggggcgatcttggcccctatggcggcggcgaaggccggggagcgcccaccccttcattcgaccagatggcccgggaagggatgctgttctgggacttttacggtcagcccagttgcacacccggcagggcggcagccattacaggccgcattcccaacaggagcggtatgaccactgtagccttccccggcgatggcggcgggctcccaaaagaagaatggacccttgcctccgtactgaaaacagcgggatatgccaccttctttgccggcaaatggcacctcggcgaagcagattatgctatgcctattgcccacgggtttgatgtaatgaaaaatgtaaccctctaccatctcaacgcatatacttatgcagatccgaaatggaacgcggatatgcccgctgcgctgcgcgaccgctgggccaaaggcacgaaaggcgcgctggaaggcgaagctggtaaaggtttccgtgaagtaaagaaaatcgacggctccgtgattccttatctcgacgaaaccaccgaaaatgaatccattaaatggctggaacaggcggccaaaggcgacaaaccattctttatggagatttgtttcgctaaaaaccaccagcccaaccttccacaccccgactttgtaaataaatctaccggaaaaaataaatatgccgattgcgtagtggaactggatacccgcgtaggccagatcatggagaagatccgcagcctcggcattgcagaaaataccctggtggtgtacactgttgataacggtacctggcaggatgtgtatcccgattgcggctacacgccgttccgtggtaccaagggaactgttagagaaggcggtaaccgcatccccactatcatgtggtggcccggtactatcaaagccggcagccagaatcatgacatcctcggctccctcgactttatggccaccttcgcatcattggcaggtgtcagtcttcctcaaaacgaccgcggcggaaaacccatcatcttcgatagctacgatatgtcgatggtattgaaaggtaccggtaaatcaaaacgcactacctggatgtacttcacagaaaatgaactttctcccggcgccatacgcatcagtcagttcaaagcagtatttaatttaaggggagatggcggccaggctaccggcggtctcgcagtagacgctaacctcggatggaaaggcgaagaaaaatatgtggctaccgcctcgcaaatcttcgacctgtggcaggatccccaggaaaggtatgatctcttcatgaacaacttcacagaaaaaacctggtttcttccaaacatacaggacgaaatcacggagtttatgaaaacatacgcaaaatatcctccccgcaaactgcaaagtaatatttataccggcccgattacgatcacggattatgaaagactggaaatcataaaagaaaagatcaaaaattataaagtaggtaccggcggcggcatgtaactttttaaatcttttaataaacgcggtggacgaagctccgccgcgtttattaaaagctaaaataatattaatagcggcgaatttacggctaacaagctatctggaaatcaagtaatttgagattacttgtaaccacgtatggaaataaatacttacaatgagagggaacttttgttgagcctcgctcagggcaacgatcatgcctttgcgggtgtattccatcactaccgtcatcgcatatacgcaattgccttccgcctgctcaattctacttcacaagctgaggatattgtacaggatgtttttctgaagatgtggctcaagcggtatgaactccatgaaatcagtcacttcaaagcatatctctttactactacccgtaatcatattttcacatccatgaagctgctggcccgtgaacagctcatggaatccgagctgtcggccgccatggtaccggatgtaagagacgttcatgtcatccataaagaatatgaacagatcctgcaacatgccatcgcccagcttccaccccaacaggaactgatctataaactcagcaaggaagaaggcctgaaaagaaatgaaatcgccgaccgcctccagctaagccctgaaaccattaaagtacacctggccaatgccatgcgctctatccgcgcattttgcctcacccgcatggacctcaacaccttccttctcctggtttggatttacagttaaatatttttttttaaaagcactaacccatgtgcttctttttatagtctccttattcaaatcgctattcatgacagtatcccgattcagatacctgtttgatcgttactatagccggcaatatacaccggaagaaaaaaaggagtttatgctcctgatggagcagtcaacacatgacgaagaacttaaagaactactcgatgaactgctccggcaggcagatgaggacagcagcgccatgccggacgataccgccgccaacatgctgcaacagatcatgcaaaccagcaacagcgagccacagccggcccctgtgcacaggatagcagtatggaaacgcgcagctatagccgcctgcgtgctcggcgtacttgcactggcgggctataaactgtatgtaaaaagcagcactgttaacacagcggttgccagcaaccatgctcctgcccgtaaagaggaacacgcccgcctggtacgtggcgatggcgcggtgatagacctggaacaacataaagatgaagcagtagatgtgcaatccggcgtatccgttgcccgcaaaggcaacacccttgcctataacagtagcgccaccatcacgcctaccatcaataccctctatactaataaaggaggtacctaccagctaatattacccgatggcaccaaagcatggctcaacgccgcctcttccatccgtttccccaccgcattcaccgacagcacccgcgaagtaactatccagggagaagtatattttgaaatagcgcatcaggccagtcagccttttattgtgaaagccaacaacatgaaaatagcggtactgggtacccactttaatgtgatggcatatgaagaagaacaaaacatctgcacctccctgctggaaggcgccgtaaacatcatcagcggaaacacggtaaggcaaataaaacccggccagcaggcgctcgtaaaccgcgatcatcgtggtatcagcatcagcaacgccgatgtagatgcagcaatcgcctggaaagaaggccgcttcgaattcaatggtaacatcaaaagtattatgcgcgaactggcccgctggtacgatgtgcagtttatctatgaaggcgagctgacaaataaagcgttcgccggcaccttctcccgccacgacagcctgaaagatattttgcaacaactggaattaaccggcagtattcatttcaacatcaacgataaaacaattacagtaagtccttaacaccacgcgcatttttagttatgaaaaaagaaataagtcagccaaaatcaacgacagcttaacatttaaagctatttaccggcagtgaataattaccagcggcctgctcgcactggcgtagctatgcccttatgttcctgttacgttatcaaccttaataacatgctaaatcgcagtaaaaaatgatgcaaacttctctgaaagtccgccataactggtggcatgtttcatcgaaccaaaaactattatgctttatgaaactaacctttctgctgctgctcgccgccgttctccaggcccacgccaccggctatgcgcagcccgttacgctgcacgtaaaagcagcccccctcacggaagtgattaaatctatcaggaagcaaaccgggtatgtatttgtatttgacctgcaaatggtggaaaatgccaaaccggttaactgctcacaggacaacgtacccctggagcgcctgctggacgacatcttccgggaccagcctctcacctggactatcgttaaaaaaacaattatccttaaaaagaaacccctcatcgtctccaccgttcccaccggcacggtgcgtataaaaataaaaggacaggtaacggaaaacagcggcacccccatggtaggcgtgtccgttgttaataaaacatcccgcaccaacgccctcaccgacgaactgggtatcttcaccatagaagccaatgtgggcgacagcctcctctttaccatgatcggtatgcagccgcaaacagtacaggtgaagaacgacaaactcctgaaaataacgatgcagcaaaaagtatcggatgtaggtgaagtggtggtggtagcctatggcacccagaaaaaaaccagcatggtgagcgcggtaaccagcatcaatccaaaagaactgaaaggccctaccagcaatcttaccaccatgctcgcaggccgcctgtctggtgtaatatcctaccagcgcagcggagaacccggcagggacaacgccagcttctttatacgcggtatcaccacttttggaaccggtaaagtggatccgctcatcctcatagatggaatggaatccagcaccaacgacctcgcccgcctgcagccggatgatatagccgggttttctattctgaaagatgccaccgcatcctccctctatggcgccaggggcgctaacggcgtagtattggtaacgaccaaatccggcgtggaagcaaaaacatcttttaatgtacgcttcgaaaactccatctccagcaatacccgcaacttccagtttgcagacaacatcacctatatgaaactggccaatgaagccgtgcttacccggtttccactgcaggatgttcaatactcccaatctaaaatagaccatactgccgccggcgatgatccgttgctgtatccgaataataactggatcgaacaactgatcaaagactacaccgtcaaccaacgcactaacttcaacctgaaaggcggcggaaaagtagcccagttctatattgcaggtacttataacgtcgacaatggcgtgctaaacgtggatcagcggaataatttcaacagcaacatcaaactaaaaaactattcgctccgctccaacgtaaacattaacctcacccccacttcgcaggcaattgtacgtacctacggccagttcgatgattataacggaccagtaggcggcggcgcaggactcttttcacaaactatatgggccaaccccgtaatgttccccgccgtttatcccgccagctatgcaccgcaattaaaacatccattgtttggtaacgccatcaaaccaggctcccccagcctgcccggcaacggaagtaacctctataataacccttacgccaactccgtttccggttaccagcaatacaacacctctacactgctggtacaactggaactgaaacaggacttaaaattcctgctccccggcctcaccgcgcgcatgatgggttatacagaacgttactcctacttcgatgtaacacgcaggtacaccccttacttttataccatgaggtatgatcagttcacaaaagaaccggtgctcacttcactcaacaccaatggtaccgaatacctgggctatgagcccggcaataaagtgctgaacactaccgcatacatggaagcggcggttaactacaaccagcagttcaataaagtacataacgtgtccggtatgctcatcggcctggtacgcaactacctcaccgccaacgccggtacactgcaaacatccctgccacaccgcaaccagggcgtgtctggcaggtttacctacgactacgacagccgctatcttgcagaatttaactttggatacaatggctccgaaagattcgccagcaaccaccgctttggattcttcccctccgccggtatcgcctggaaccttcaaaacgaagcgttctttaaaccattctccaaaacaatcgataaactgaaactccgcgccacctacggactggttggtaacgaccagatcggaaatgaagatgaccgcttcttctacctgtcggatgtaaatatgaacgacaattccaaaggcgcctccttcggagaaagaagaagctactaccgcaatggcgtatccgtgaaccgttatgagaaccgcgacatcacctgggaaaaatcatacaaaacaaacctcggtatggaggtcggcctcttcaacgccatgaacatcaccctggacgtataccaggaaaaccggaaaaatatcctcatgacacggagcaccattcccagcaccatggggctcaatgccgccacacaggctaatgttggcgaggcctccggtaaaggcgtggatctctcggtcgactatacgaaaagtttcaacaacaactccttcgtacagttccgcggtaacttcacctacgctaccagcaagctgctcgtaaatgaggaacccatttacccggaagaataccgctcacgggtaggacatcccctttcccaaagctggggttatattgcagaacggttatttgtagatgaacaggaagtagccaattcggcctaccagaactggggacaggcagtaatgggcggagatatcaaataccatgatgtaaacggcgacgggcaaatcaacagctccgatgcggtgcccatcgggttacctaccacaccggaaattacttatggcttcgggttttcttttggttacaaacaactggaccttagctttttcttccagggatctgcccgttcttccttctttatcagctcttaccaaatttcaccgtttgtgctgaacgaaggcggccagcatggcctgttacaagccattgcggatgatcactggagcgaaagtaaccgcaacctctacgccatgtggccacgcctcagcgactactttgtgaacaacaacaatcaaacgtctacctggtggatgcgcagcggcgattttctccggttaaaatccctcgaaatgggatacaccttttccaaacgcctgctggaccgcgtacacatgaccaacgcacgcatctacgccaacgcctccaatctttttgcgatcagcaaatttaaaacctgggatcccgaaatgggaggcaacggacttggctacccggtacaaagggttattaatatgggaataaccctgggactttgattcaccgcttaactgtgcaaatatgaaacataccaatacgctcaatatacgccggtacctgcaatggtgcggattatgcatactccttttctctgccgcttcctgtaaaaaattcctcgatgtagtacccgataacgtggctactatcgacaacgcttttaccatgcgcgcagaagcagaaaaatacctctttacctgttactcctatcttcccaacagtgcggacctctccacgaatcctgccctcgtggccggcgacgaattctggatggtacgcccatacagcaccagcgaaacaccctggcaggtggcacagggcttccagagcgccaacaacgtgtatatgtccacctggggatggtattacaaggcgctgcgcgactgtaacatcttcctggaaaatatccataaagtggtagacatgcgccagagtgaagtagaccgctggagtgcagaagtgatgttcctcaaagcatattaccactggctgctggtccgccaatatggccccgttcccgtgatccggtacaacctgcccatttccagcaccgctgaagaaactaaagtgccacgcgaacacgtggacaccgtattcaactacatctcgcacctgctggacaccgccgcagccgggttgccggaaatcatcgccgacaggtctacagaactgggacgcatcaccaaaccgattgcactcgccatcaaagcacgcatattggtgaccgctgccagtcccctgtacaacggcaacatcgattacaccgctttcaaaaattccgacggtgcgccgctgttcaataccgccttcgatgccaacaaatggaaagtggccgccgatgcttgtaaagcagccatcgacgtatgcgaacgcaccagcatgctgctctataccttcagcgagctgggggtaacgttgtcggatacactcacccggcaaatgtctatccgcaacagcacctgcgaacaatggaacccggaaatcatctgggccaatcccagtgtaagcacctatgaaatacaacggcaggctatgccccgccttgatcctgcccgcataggcaatgaatcggtactcggcagcctggcgcccaccatgaaaatagcagagcaattttataccgacaaaggcgtgcccatgaacgaagataaaaccttcgactatgccggtcgcctgaaactcagaacagccgtaaaagcagaaggagaactcatacaggaaggatataccaccgcggccatgcacttcaaccgcgagccgcgcttctacgcagatctcgcattcgacggagccatatggatgatgcaaaagaaaatgttccatatagaatccaaagcaggtcaatggcaaacacggaaaaatatttacgataataacactaccggctacttcgccaaaaaactggtgaactggaaaaatgaaatcctcgaaggacagggcctctttgtagaaacccacccctggccggaaatgcgactcgccgacctgtacctgctgtacgcagaagcactgaatgaagcagaaggcccgcaacccgcagcttttacctacatcgataaagtacgggcccgcgcaggattaccaggcgtacaagccgcatggacggcctactccaggcaacccggaaaataccagaccaaggaaggcttccgccagatcgtgcagcaggaaagactaatagaactcgccatggaaggcgcccgcttctgggacctccgccgctggaaaaaaagtatggaagaactgaacaaaccggttaccggctgggacgtagaccagtcagatcccgtgttctactaccgcgtaagaaccctgtaccggcaaacattccagacccgcaattacctgtggccgctggaaaactgggacctgctcaacaatccaaaactggtgcagggctttggatggtaatctttcatttactaaaaacgcacaacatgaacatcaataaatatatcctgccgcttgcctgcttactgctggcagccgcctgcaaaaaagaaacacatgagccggtaaatacctccggtgaaaaacctggcgtcattacaaatctcagcgttaccaatatgccaggcgccgcaaaaattacctacagcctgcccgacaacaaggatatcctgtatgtaaaggccctgtatgatatcaggccgggagagaaacgcgaaataagatcatcttactataataacttcctagtggtagatggctttggcgactccgccagccacgaaatagccctgtacgtggtaagccgtaatgaaaccgcctcggatgcagtaaagacaaccatcaagccgttgtcgccgcccatgctgattgtacgcaaatcactggagataaaagcagacttcggcggtatcaacatcagctttaaaaatgataccaaagcagatatcgccatcgttgcactcaccaccgattccctgggcgcattcagctcttcggatgttcattacaccaaactggaaggtggtaactattccatcaggggcttcgcagcagaaaagagaaagtttggattttttgtgagagaccgatggggcaaccaatcggatacccttatgcaggaattgacgcccatctttgaaaaactattggataaagcaaatttcagggaagtgaaattaccgggagatgtggactacggctggggcctgcctatctccaacctatggaacggaacattatggcactcggcagataaactcgacggcatgcccatgtctatcacgttcgatctcggcgtaacggcgcaactgagtcgtatcaccctgtggcaacgccctaatgaatggatttacctgcagaacaatgtccgcaagtttgaaatatggggctccaccaatcccgcctccgatggcagctgggacagctggacccgcctcgtggaacatactgtaatcaagccttccggcttgcccgtaggacaaaaaacacaggacgacatagacgccagcatcgccggcgaacaaatgaccgtacccctggatgcaccacgcgtaaggtatatccgcgtgaaaatactccgtacctggaccgacggcggatacgccgccaacatccaggaaatgaagttctggggtaacgacaaatgatgatcatctacctaaaacaaaatttatgcgcatccttcattctatcatattatatagtgtactgctgacagccatcagcgcctgcaccaaacaaagcgactataaaaaatacctgggcaacggtgaaatcctttacaccggtaaagcagattccttgctggtacattcaggccgcaaccgcgtacagctgtcgtggctcctgatctccgatccaaagatcagccgcgcaaaaatctactggaacaaccacaaagactccgctatgctcgatattaaacgcaccagcggcgtagacaccatccgctacgttatcaataatctcgaggaacgggcctatacgtttgaagtgtataacttcgaccgggacggcaacacctccgtaagatcagaagccaccggttttgtatatggtagtttttatgaagatgccctgctgaccagagccttcagcaacgcggaaatgaaagacggcaacgcggaaataagctgggccaacatcgacaccaccggcggtatcatcggtatgcaactgcaatacaccaccgccgacaatgtagcacatgacaccgttattgccgcagaagcggaaggccaggtaaccgttcttaacaactatctttccatgagcaccttccgttaccgtaccttgtacatgccggataagctttcggtagatacctttcacaccccttatgaaacaaaaggcgtaaaagagaatatcacagcaacgtatatacgtaacccgggcaaccctttcgtactggacgatactaaaccgtttagcggccgcttcggacaggtgaaagactggcaatacaacgcggaagcatccaggaacggtacctatgataatatcgacggcaccggcaggctcaccatgtggatctggggcaacggccctatcaccaacggcaaaatttaccagaccattaccctgccggcaggtgaataccgcttcgaagcagccgtctccaatatagataacaccctggaaaacacctggctgttagtagcccaaggcaacgtcttaccggatgtagaccaggtaaatacggcgttgggcgcagcaaggattgtagacaacaacaacaaatacgcctctgttgccttcacgctaacagccaccaccaccgtcaccttaggattcaccggcaccttttccaatcccgcggaacaaaccatccggataagcaacgtattactgatcagagataaatagcaattgcatcatgaacaaacaacttaggaaattagggatcatcctgctgttatgcagcccgctcatcaccctgcaggcgcaggagaaaaaatggatcggacatgaaacacccgccgaaaaagaaaaacgcatggcctggtggacacacgatcgcttcggtatgttcatccactggggactgtacgccatgcccgcccggcacgaatgggtgaaacataacgaaagacttaccaacgaacaataccagaattatttcgacttatttaaccccaaccagtttgatccgaaatcctgggcaaagcaggcaaaggccgcgggcatgaagtacgccgtactcaccaccaaacaccatgaaggcttttgtctgtttgactccaggtacaccgattataaagccaccaataccaaagcccaccgcgacctggtacgggaatttgtaaatgccttccgcgcagaaggcatcaaagtagggttctattactcgctgatcgactggcaccatcccgatttcaccatcgatggcgtacatccgcaacgggtggataacggcgccgacagcacctacgcacgcctcaacaaaggcaaagacatgaacaaataccgccagtatctccgcaaccagatcacggagctgcttacccaatacggtaaagtggatatcctctggctcgacttctcctatcccggcaaaaacggcaaaggcaaagacgactgggacgcggtaaacctcctgaaaatgatccgcaaactgcaacccggcatcatcgtagacaaccgcctcaacctcgaggaatatgaagatggcgccgacttcctcacccccgaacaggtaaaggtggaagaactggcacaataccgcggcaaaacatgggaaacctgtcaaaccttctccggctcatggggctattaccgcgatgaaaactcctggaaaagcacccaccagctgctggaacttctcatcggctccgtaagcaaaggtggtaacctcatcctcaacgtagggcccaccgcccgcggcctgttcgactaccgcgcacaaagcgccctcggcaacatcggcgactgggtgaaaggcaacagcgaatccatctacggctgcacctacgcaccggagactttcgaaacgcccaaaaacaccatgctcacctacaatcccaccaccaaaagattgtacgtacacctgctggaatacaataaccgcctccagctaccacaatacaaaggcaaaattaaatatgcccagctgctgcacgacaactcagaagtaaaattcaccactgatggcaacaacgtcacactgaccctgccggacaaacaacccaacgtggaaatccccgtggtcgagttggttcttaattagcagggtgcagcgaaggttgtcttactcaggattacgctgattttattgatttaggggatttgaacactttggattttaaaagatttggggagataaaagcggagatgcggattttgtctttcccgctgattacgctgattatactgatttttagattttgtttttttgatttaaaatgattggggagatataagcgaaaatatccgcttatatctccccaaatctgttaaaatccaaagtgatcaaatcagcgtaatcagtgaaataagtttaatcctgagtaagacaaccttcgcttggaatttattatatttagttcatgaagaagtatattttccctgttctcacgaccgctgcattgctggctggcatggctaacgcgaatgcacaaacgcgcagcctctttaactttaaggatctcagtgggtggcatattgatgttcctgccatggataaagatccgaacgtgaaaagcccgttcattgtaagggacggcgttttcgtaagcctggctaacccacaggggcacattattaccgatgccagttacgaaaatttccggctggaggtgcaataccgcttcccggctaaaccaggcaactgcggtgtactggtgttcgcttctacgccacgggtattatatgatatgttcccgaagtccatcgaagtacaattgcaaaaccaggatgccggtgacttctggtgtataggtgaagatatcaccgtaccggatatggaaaaacgcaggggaccgaaaagcgaatggggagctgtagatggtaaaaagcgccgcatcatcaacctcaccgatggctccgaaaaaccattgaaggaatggaacacgatgattgtggaatgcgtaggcaacgccattaaagtatgggtaaacggcgacctggtgaactatggcaccaatgctactgccagcaaaggacaaattgccctgcaggcggaaggttctgaagtggagttccggaaagtggatctcacgcctattactgccttctcccaaaaaggacattgatatgaaatcagtggaagtgggcgtagttatttctgcgcctggcgctccgccttttctttttctttctgtgcttttctttcccgctttgcctgtttccggaaataaccgcggaacaggaagttgttccgtaaggccagcatattggtatccagtttctgggtactgctttcgaggttatagatcgtttctttaaaggcgtccgccagcagggtgtcctttaaaagcatgcccaccggcgcttccggatcatccaggttggcccgcactcctgcactggcctgccgtagctcctgcacggtttgattggcgttgagcgctgcgctgttcatttcggtaacggctgcacgaagttgcgcaaataccaccgtatccgttaccaggtcgttggacaatacgcccttggtttgcagcttggccgcatataaagataaagccccggtgagccggcgggtatttaccaccgcggcattcaagccggccatggtggcattcagatctttgtaaacagtatcgtcggtaatcaatttccctaaagtgcctttcccgtctacaatgcctttggtgatcactttcaggttgtcggtgatttccaccaggcttttattgtttacctgcagggtactcataatttcttcggtgcttaaaccgctgaccacatgcagctgatcgccgttttctattaccggcatgttgggcgtaccgccagtcagcatcacgatcttattacccatcaggccctcagagctgatacgggcctctacatctttatggataaactcctgcgagctttcatcgatattcatcaacaccaggatctggttggttctcacaaaactgatctttttcaccgtaccgatctttacaccggagtacaggatattgcggcctacggacaacccgttcacatctttaaaataagccttcacctggatggacttgctgaatagtttctgttgcttgcccagcatcatcacggcggttacaaaaatggccagccccacaaatacaaagatgcctacaatgacagcgcgtttttttcctgcttccataacttactgtataaaattatagtcgtaaaaacttttaataagtccgtccttctcgttaaatacttcttcaaaacttccctgccgtataaatttcccttcatccatcactgctacccggtcgcccacttccttggcacaggtaagatcgtgggtaataataatagaactggtattgaatctttcctgtacagcgatgatcagtttattcagctccatgctggtaatagggtccaaaccagcagtgggttcatcatacagcataatttccggccgcaggatgagggtacggccaatgcctattcttttcttctggccacccgacagctccgacggcatctggttaatggtttccggtagcccgatggcttccagtacaatgtcgatcgttttccggatctgctctttggtcatatcgcgctgattacgtttcagcggaaaggccaggttttcccctaccgtcatgctatcatacagggcgctgctctgaaaagagaaccccaccttcagccgcaatgcacgcagctcggcttctttcagctgatccacctcttcccccaatacattcacagtacctgcgtctggtcgcagcagccctatgataatttttatcagcaccgatttaccggtaccggaacgacccagcaccaccacattttcgcctttatgaagatccaggtcgattccctgtagtacatgcttctctccaaaagacttataaaggttccggatactgatcacggtttcattcatatctatctggtgaccatttgttttcatgactagcggatggtattaaacacgtgaacaataattacttcctctataaatatcaggaacatggatacaataacggatacattcgctgccttacccacgcccgtggtgccctggcttgcattaaaaccctggtaacaactcacaatgccaatggtaaacccgtacaggatagctttggtaagtgcggtggtataatccaggaaagtgatctgcgcaaaggcattatcaaaaaacgataccaggctggtttgttcgtgcgcatgtacatcaaagtaagaacccaaacaacctatgagggcgttataaaacatgagcagaggcaaacaaaccgtcatggcaatgacgcgggtaaccaccaggtaacggaaagggttaatggcagatacctccatcgcatcaatctgttctgttaccttcatcgatcccagctctgcgccgatgctcgagcccaccttacctgcgcagatcagggccgcgatcagcggcgccagcgctctcaccaccgcaatagccaccagcgacggcaaccacgcagtaaccccgaactccgataaagtaggacgggactgctccgtaaacaccacgccggtgataaaccccgttaccgtaacaagggccagcgacttataccccacctggtaacattgccgcacaaactcgccccactcaataggaggccggaatgcctccctgaaaaagcgacctataaaggcggcgatatgataaaactggagaaaaaagccatcaatttttgcggttatgaccggcttatccgattttccgttggtagaattcatcttcttgttaatgcttactcacttattacaattctatgccgcttttgttaaatacacagatgttaacgtcaggccccgctgtgataggattttttgacgccacggcgcggaagctgctgcacaggagtaatctcccgtgaggatgtcccttcacactacggtcattatcttccccaaccggacaaaaaaaatgcagcggaatgttgttccgctgcattatctgtggttgtagacatatcattactataactgcatactgatgccgccgaaataattcctgcccggcgcaggattgtaataacggccgccaaaggcgttaagatcgttgcccaggctgtagtttacgttcagcaggttatcggcgcctgcacgcaagcggatgctgcaacgcgaacgcagcggcagtttccagctcacattggcctgcagcaaatgataaccgccggcatacacgctgttggcgtcgtttagcggtatgctgctggtaaaagtatgctgcgcatataacgacactgccgcagggaactgccacaacaaactgctcaccagcacatgctgcggcacaccggtgagtgcattccccgaatagtctttcccatcagcacttacatagtggttaaaccggaagtcactcagcgtatacccttcctgccaccggatgccgcgtaacacaccgccgttacgtggcttcatcagccaccacatgccctgtacctctatccctttctgctgaacgccgccggcattggtgaaaaactcctcgccattgtcgtgctgccggagcacaatggcattttgcattttgtaataaaagaaggccgcatcgattgttgccgtgtggttacgggaagccgcgcgtacaccggcttcatagttccagccggtttccggttgcagcgccgtgttgatcacgttgtcggatgcacgaacttctgccgtagccggtggggaatagcccctgctaaccgtaatacggcccgttacctgtggcgtaaacaggtacgacagcgagaagcgcggcatcagctgcggcgtgaagttgattttcgtgtgcccgttgctgttgtagcggtaaccataataatttaaactggccgctgcctcaaaggtaaatgcgctcacattggcctggaagcgggtaaagaaaaagtactgatccgcttttagcttatcggcagccatcaccgtatcgcgcttaccttgcttgttaccgtaattgatcacgtcggtggtggtttgctgccactcggcgccgttcagccatttccattggaacggcgagctgcgctgcggatcgttggtccattgcaggtaggtgcggaagccggcggtattttcatcccgcgcttcatagttggtgataaaaggattttcaaaatgagtattggccccaaacaccgagagcaggtgctgtagccgtggggtgaactgcgcttcgtggaccagtccgccctggaaagtacggttatagatgcctgccttttgcgctaccgcgcctggtgtagcgggcgtgccgggcctggcggcacggggattggcttcactctgcgccagggttaatcctcccggcgtgaggtacgacagatccgagtaaaacgccagcagcttcagtgcgtagcccggtttgtattcccagcgttgagccgtttgggtataagagcgtttcatggcggtattttcccggtagccatctgcccgctggtatccctggaatacctgtacctggtaatttttccattgctgctgccaggccgcactgccgtgaaacaggccatagctgccgccttgcaggttcacctgcaggtggtgcgtgtcggccggcggggggaaaaggtccagtcgcaccacccctcctgagttggcgccaaacaagctgccgtccggtcctttcagtatttccgcccggcttatcgcatcagcgtctataagattgagataggtattgcccccggcatccgtcagcgggatatcatctgcataaattttaatattccggataccaaagggagaacggagcaaactacccctgatggataaacgataactgcccggcgaccgctcctccattcgtatacccggcaccgtatttatggcgggcaacagggaagtgccctgctgaagctgcatgtcggcgggcgacaggatactcacggcggtgggtacacgctgcagcgaggcttttgaataataggattgcaccaccacctccggcaactgctgcagggtgtcctgctgggcctttagccccggcgaaaaggatagcatggttaataaaatgcctgccggcaaaacgctcattcgcatgtcagtaattctttatccgccgcggaagacggtcatctttcggcttaagatataaatatttctgcgaatgcaaccgctatttgtgtggaactgttatacgcctgttttggtggtaatccgcacctggtgtgtattgaacacctgcgaatatggcggaacacttttcgtgataaaaacgctgccgccaataatactgccctgcccgatcacggtattaccgcccaggatggtactgcgcgcataaatgatcacgttgtcctctaccgtaggatgcctttttacatccgacaactcctttgttacatgcaatgcacccagcgttacgccctggtatatcactacgttggagccgatgatactggtggccccaatcacgatgcccgtaccgtgatctataatgaagggcacactgatggtggcgttaggatgaatatcgatccccgttttgccatgtgcaaactcactgatgatccgcggcaataccggtatatccagttgcgttagccggttggcaatgcgatatactgtgatggcataaaatcctgggtacgatacaattacctcgttcacactggtggcggcggggtcgtattcgtgtattttagcagcatcctggcgaaggtgctgataaatggttcccaatgagttataaaaggcgtttacaatttcttctataggtacctcgcgggggtccaggtaactgagcaggatattctccaggtctatctggttcttttttaagatgccctcataggaggtttgtttagggagatgatttcccgggaataaaaaaccaaccaggtcgttcagccaggtaatggcatcctgggcagacggcgtagcttcccactccgcatgatgcgttttcctgagtaaactgattaacgtttgggtatgcttgttatccatacgggtgtgggatttaccggtaagatatgaataatctactaaattagtagggtaatgttttaaaagaagaaaataagcaacaggccgggataatatgtaattttgcggctcatcctgttttttatgagacgagtttttgcttttatctgcgccctgctgacggcaggcgccacatctgcccaggacagcagcaggttccggattaacatcgcccatctcaccggtaacctgtacgtatatacgtcttatggagaattcaagaatgtggtctaccctaccaatggcgtgtatgcggtaacaaaaaagggcgtggtagtaatggacacgccctggagcgtagatcaaacccggcagctggcagacagcatcctgaaaaagcaccaccgcaaaattacttactgcatcgttacgcattttcatgaagacagaaccgccggtctcgacctcttcaaaaaactgggtgtaaaaacctacagcagtaccgccacactggaattgtgcatggccaaaggagaaaaacaggcgcagtatgtatttaccaaagacaccacttttaatataggcggtgtgaaaatacaaacttactatcccggtgaaggacatacgaaagataatatcgttgcctggttccctgccacaaaagtattgtacggcggctgctttataaaaagcagcaaagcaaaagatattggttataccggcgatggcaacgtaaaagcatggcctgccagcgtagcaagagtgaaacaacaatttcccaacccggcttatgttattcccggtcatgatgcgtggcgcgacagcccagccgccatgttctcccgcacattagaactgctttctttgtaaacgcacacttaaagtaaaactttaagcagagatgaaaattgattaaaattctcattaatcatcctttctaaaacatatgaaaaccaacacaatatgaaatacatgtggttcaaagctttaacgcctcacctgggcgcattgatcctttttgtgaccctggcgtttgtgttttgcagccctgtattggatggcaaacaactattgcaatcggacatgatgcattacaaaggcatgcaaaaagaagcggctgattactatgaagctaccggcgatattcctctttggaccaacagcatgtttggtggtatgcccacctatgtcatctacaccgggccctccaccaacaaagtaggaatactgaaccgcgcgtttgccttataccttcccaacccggtagatatgttttttgtgctgatgatgggcatgtatgtgctgctgtgtgtactgggatttaaatactggatacggataaccggggccatcgcctatggctttgccaccttcaccattaccagcatcgacgcggggcatatcaccaaggtaatgagcatggcctacatggcgccggtgctgggcggcattatcctggcctaccgcaaacaatacctcgccggcggaagccttactgccctggcggcagcggtgatgatctacaacaaccacccgcaaatcacttattacaccggcatcatcgccttatgcgcagctgtagccgccggcatacatgccttccgcgaaaagcagctgcccgcgtttttcaaagcttccctggtattactggcagcgggtatcatggcaatcctgccctccatggataacctgcttatcatgaaagagtatacgaattatactatccggggcagccagtcggagttaacacaaccggataaagccgccaaaaaatccggcggtctcgatatcgcctatgcatttcaatggagctacggcaaaggagaaacctttaccatgctgttgcctcacctggtaggcggatctacttcggagaaattgtcgaccagctcccacgtttaccaaaccctcaccgatatcggcgtaccgccggcgaaagcagcggaagccgtggaacgcccgtcgtggcagctatactggggcggccagcccttcaccggtggccccgtttacatcggcgtagtcatctgcttcctgtttgtgcttggcctgttcatcgttcacagctggcataaatggtggctgatagccgccaccgttatcggcatactcctcagttggggcgccaacttcccggaactgaacaacttcctcttttatcatcttccgttatacagcaagttccgcgcacctacaatggcgctggtgatcccgcaggtaaccatggtgatcctcgcatgctgggctttgcaggagttattatatggtaagcagacaaaagcctggctggaacaacacctcaaaatgacgctgtatgtaaccggcggcctggtattactgctggccattggcggcagtgtggtatatgccttcaatggccctaacgacagtaacatccttgcgcggtatacacaaatgctgggaggcgaaattcccgccgccaggttattgaatgccctcaaacaggaccgcagcagcatcctgcgggccgatggcatccgcgcactggtgtttatgctgatcgcctttgccgccctctggttctccctgaaagaaaaattaaaaccagtatacgcaacaggcatcatcgcctttgcagtactcttcgatctcttccaggtggataaaagttatcttaatgaagacagcttcatggaagtatcccgcctggaaaactatattgccccttccccggcagatgaaatgatcctgcgcgacaaagatccgtattaccgcgtgctcaacgctaccactaatcctttcctcgatgccaacaccagctactttcataaatccatcggcggccagagtccggcgaagctctggatctatgaagacctgatccaacatcagctcaccaaaaacaatatggccgtgttcaatatgctgaacacccgctactttattgtgcccgatcagcggagcggtcagccagtagcccaacgcaaccccggcgccctgggcaacgcctggtttgtaaaagccatccagtgggtgcccaacgccaacgcagaaatgaaagcactcgatcattttaacccggcagataccgtgatcattgaccagcgctttcagcaaatcaccggcgccttcacacccgtggccgacagtaatgcgcgcatcgtactggataagtatagcctcaacgaactgaaatatactgctgtgaataccagggcgggcctcggcgtgttctccgatatttattaccctgccggttggaaagcttttatcgatggtaaggaaacacctatcctccgtgtaaactatgccctgcgcggcctggtagtaccggcgggaaaacatgaaattgtattccggtttgagccggccaccttcttcctcggaagaaagatctccacgatatcttctatcctgttactggtggcggtagcagcagggtttatcctggcatggaggaagcagggcaccacataacgcaacaccattttcatcacagcaaacaagacttctgtcacattgtaaattaaggatccgtgcgggcagttatttttagggaacaaaggagaaccctgttctccacccaaaactatccgctatgttcaaaaattattgcaggcacggctggagaaatctccttaaaaacaaactctccacccttattaatataggaggcctctcccttggtttggctaccggtatcatcatcctgttgtggatccatggggaagtcagctacgattccttccaccagcataatacggacattcatctgctgatgaacaatcagtaccacgaaggccggtggtttaccggcgacgttacaccggcgccactggcagagaaaataaaacgggagttccccgaaataaaatataccacgcgccaggtttatggcggacaacaattgctcagcaccggtaagaaaagtatttatcagcaaagcctgtacgcagatcctgactacttcaacatctttactttcccggctatatccggtaacccggttgtcgcccttcaggaccccggcgccattatactttcggaaagtgctgcccacaggctgtttggcgacaaagaccctattggcagtattgttaaacacaataaccagcatcacctccgggtagcagcggtaatccgcgatgcaccggaaaacagttccattcaattcgacgtagtactccccttccgcctttatgaactggagaatgccgactggatcaaccgctgggacaattaccgtgttggcagctttgcgctgttgcaaccgggaagcagcgtggatggctttaacaaaaagctgaagaaagcaaagctcactggtaccacggatagtaccagctacctgtttgcctacccgttcaccgcgctgcacctgcacggtggtttcagaaatggtgagcccagcggcggccgcatagagatcatgatgctgctgggcaccatcggcctttttattttactgattgcgtgtattaattttatgaacctttccactgcgcgtgcagaacgccgcgccagggaagtaggcgtaaggaaagcgcttggcgcctcccgcatcaccatcatctttcaatttctcatagaagcgctaatcatcacctttggcgccttgctcctgggaatattgctggtgaaactggcgctgccggggcttaacagcgtatccggcaaaaatatccacctcgattttacgaactggcaggtatggacagggatattattactgctcctgttcaccggcctcattgcgggtagttatccggcctttttcctcagcagcttccggcctgtaaaagtattgaagggcgtgatatccaccaatcgtggcggcgggctattccggaaaagcctggtcaccttccagtttatcatctccatttttctcattatctctaccatcgtgatataccggcagctgcagtacggggaaaaccggccagtgggttacaaccaggacaatcttctggaaatacccgcccgcggcgaaatggctaacaagtacaacctgctgcaggaagatctgctgcgtattcctgaaattgaaaacgtgtctgccggtacagacgacctgctgaggtttggcggcgccaccgatggtattgcctggccggggaaaacagcggatcagaatttccctattaatattacctgggtgaaatacgactgggtaaaaaccgccgggctgcagctggctgcaggacgcgatttcagcacggaatatggcagcgattccaccgggtgcctggtgaatgaagccgcagtaaagaaaatgggattgaaagaaccggtggtgggcacattactcggcactaatccgatcatcggggtagtgaaagactttgtaattaataacccttaccaggccgcgccaccgctggttatctatttaggcaacgggcctgtaagtcatatttttgtgcggctccgtaaaacggatcacccggaaacagcccttgccaagatagaagcggctctcaaaaaaagtaatcctgaatttccttttgaattcagcttcatcaaagaagcctatcaaaaaatgtttaacggcgtgcgttcgtcgggcttcatgttcaactggaccagcggtctcgctatcctgatctcctgcctgggattatttggtttatctacctacctcgcagaacggcgcagtaaagaaatcggcatccgtaaaattatgggcgccagcgtaggccggatttggtatatgctcgccaaagaattcctgaaacccgtattcattgcctttgtgattacggtgccgctggcggtgctggccatgcaggccgccctgcacaatatagattaccgcatatcactgcaatggtggatgtttgcggcagcaggcatacttacagcggtcattgcattactgaccatcagctatcagggtacgaaagctgcgatggccaatcctgtaaaggcattgcaatcggaataaaataaatcaggagtgggtaagcagatgttccggcgcttccagcaacgactgggtttgcagtaacatttctttcatcttcatcttaaagcgggtggcagcagaggtttcatccggtataacggtttcctgcagctcactctggaagagcacctggagatttcctttcagtctatacagatcgctctgtttagccaaaccggcagcaaatcctgcttctctgatagcctgttgctgatcgggttcaaaagaagcggcataccagataaccggcacctgtttcaggcgtttgatctttctcagctcacgcaaaaaatgaggcgtttcatctgaaggtaacaggctatccaggaaaatgtaatccgggacaaggccggggtgcttcttaaaatagtccagcgctttgctggtgttatcctgcgcaatgcaggccttgctcacattcaggaggtccagcgccaggtaaaactggttacgccggtcgcggtccgggtcaattagtaagctgattaatttctctctcattgcagggcagttttaatggcaggataaatcggtaacaattcgtactatgaaaaacaaagaggaaaaagaaaagttgtaactgctgcaaaagtacagcaggaaatgttcctgaaaaaatcagcgaccggcaatagccctcctttcttcagaaaagaaacacaattaacaaaaacacaacagatcgggcacctttacattggcaggatcactttaaaatcagcgcccttatccggtacaccgttcgcataaattcctcctttatgattcagtacaattttattacacagggccagccctattcctgttccttcataggtagtacggtcgtttaaccgttgaaagatctggaagattttatcggcataaatctggtcgaacccgataccattatccgaaactgtaatggtgcagtaggttctgcccgggtccagatccggtaatgccactgcgtcggcagcactgagtggctccgcgtaaatgttgatcaccggctttcttccgggcgacaaaaacttaatagcattaccgatgaggttatgaaacagctggttcatctgcagcgggcttacggtaagccggggcagttcttttgcgtcaatggtaacgtcatgctgaccgatcaccacttcgaaatccgtcagtacatttttcagtatttcgttgagatctgtttccacaaacggatcttttacgtgtaccagccgggaataatccagcagttcactgatcaggagcgacatccgtttggcgctttgcattactttctcaatatacatccgcgatgtttccgaaaggatgtctttgttcacgttatacagcatgcctgcaaacgtgtggatcttccggaggggttcctgcaaatcgtggctggttacataggcaaactgttcgagttcgcggtttgatttttcgagatagaagttcgcttccagcagttctttggttcgcagttccaccatagcctccagcttaatggccagctgcatatactgggcttcactttcctggagcgcctcgaataatctcttttgctgtgtaatatccctggctattttggatgcgccgattacatttccccgcaggtcttttatcggggagatcgtcagggaaatatccagcagttgcccgtctttggtgacgcgctttgtttcaaaatgatctaccctgttgcccgatctgagctgctcaatgatccgggtttcttcatccagtctgtcttccgggataatgcgggtgatgagttcccctttcatttctgcggcagtatacccgaacaacctttctgcgccggggttccagctggtaataacaccctccagcgttttactgataatagcatcatctgaattttccacgatggcggccagcctggatacatattcttccgcggttttctgatcagtaatatcaaccagcatattcactgcaccttgcagattgccggcgctgtcaaaaatcgggtcggggtatggctggatgatgcgcctggagccatcgggtctttctatcataatcaacttccctctcaccggcacggcgcctttgatggcctctgccatcgggcagctatccaggtcaatgggagtaacgccgtcggggtcgtatattttccaggaaccgcaccacatgtctactcctgcaacgggcgcccggccccacagtgtaacggcagctgtattataaaggagtacgcggccttccttatcacaggtatatacagcggcgggcaatgcctccagcaattgccggtaatgcactcccgcgccttgctgctggagcttttcccggcagagccgcatctctgcagccatgtacggcaggtaaccatgatatgccttgtgtaccggggtagcgctgcgaaccacctgcgcagcaggtaagtgcgcataacccaccggaacagacacggtaaacgtgcttccctcgccgggaatgctgctgatctgcaactccccgccgtgcagaaggatgccttcattggctacggtcaggccccggcggttccggggcggcccctgcaatgcagcgttgatttcagacaacaggccgggcgtaatgccgatacccgtatctgctatggaaagcaatacctggttgccctcctggcttagcctcacggccactccgcccttcaacgtatagctgatcgcgttagtgagcaacgacaacaggatctgttcccagatgtccctgtctatataaatatcttccggaacaatatccaggttaataactagggttaatcctccttcccggatcaccggttctacctgctccaggagtgtcctggtgaaattgcccagatctgttttaacaaacgtaggcgccttgccgttatgcagggcagcccccatgaacaggaggccggtatcgccggaatcgtctcttacaggcataccattaaactggtagcaactgccatccggccgcatcagctgcagctgcggagctgttaccgccgcatcagtggccgaccacaaggcgggccataccgttgctgccggttgtcccatggacaatggatgctggctgccaagtaattcgcggcaggcatcattataaataaaaatgctttcgttaccccagcataacagcatgggttgcacggaggagagtaaaatctggatacaggtctttaaactttgcgaccaatgatctgccggcccaaggggagtatctgtccagttaaaagaacggatcagctcacccgtttcacctccaccggagggaaacttatctgacgccgcagccggttcacctaaagttgcctttgtcggggcatttatcattgtacaaaatatataatcctaaaatatatactggttgattcgtaagatggggatgccattaaaattccacaatcaactataaaaccgtgtaataaaatgcacaatcatcatctattccggcttcattataaaactgatccttccgttcgtttccatatatgcctgctctatttcagcaagcgaggccttcagtgtttccagtctcaggctctccatgagatcggatttactcaaacaggccttattcatattctcccatttaatttctcctgcatcatatagcagcagcggctttccttttaccaggcggttgatcatatcgcttttcaaagagatccaggccaggctccggttgatagccaccatcacagcggcggcggctacggtacctaaaaacggcgaggcgcccacaatcaccctggccagcactgctcccatcataattacaataatcgtgtcgaaagcagatttcttcccaaaaatgcgcatccctcccaaccggatgagggtcagggtaacaaaatacatggctaccgccctgacagacatctgcagcacatttaactgatcgccttgtccccacaggttagccgcggcattcatttttcaggaaattttatttgctcataagcaggagctgcttcgatatatccaagtggcgtaaactgttttccttcctgctcattataggtaataaagaaaagctctatttcccggatggtttgcgccgacaccgcatccactcctttatataacttggataccaccggcactgctatgtaacggtcgttccggacaatggcgccatccctttccttttgctccgctttgatagcgcccagcaaacggcatttgatcatgcagccgggaaagcttttaaactcagagatcaccatcacgtccagtggatctccgtcagcccctttggttcccaggataaaaccaaaatcatatgggaaaaccataccggcgggtaatattttactgagtacaaaaaaccgcgatgcagggtcgaaatcgtatttttcactactccctctcggagtttcaatgacaacaggtaactctttaatgatcatacgcacattttgttggtctggttaaataggataaagaggactcagctgcgaagaaacaaaaaaaggaccaaccaacccacataaggcataatgattgtaccgcaaaagataaactttgcgacatggatacctttaacatacaactcggcaatcacgaaaccggggttacgcgccgcgacgaagatgtgtttatcgttcgtcttcctgaaaaaactatttacgtggaaaaaaggcaggacaatgaaggagctaaccactggtttgaacagggcaaggataatgaaacttccctcaccgctaatattggggccgccattgagaactggctggcgaaacataattcctgaactttattttaaaaaaaatactgcctgcttatcttgcaggcagtatttttacagagatgctgatcactggtttcctttattataaaagatgaacaatccatctttgccggctacgatcacatcttttttgccggatcccgtaagatcatgcgtcacaaaatataaccccgctccttttgatccatagctgatcacctgtttggtgaaagaggtgccgttccatttaaaataatagataccgcagggatcatcggaacccggatcatgatcattgtgcgcacggtaacgctttccggtgatcagttccggctccccatcaccatcgatatcttcccacagcatggtatgatattgcgaattgaaaggatcaatagcatgtttgatccatagccgcttatttgttttgctgtccttcttttgctcgtaccagtcgagcccataatcatgcccctgccctgctataagatcaggcaacccatccttatttacatcggctactattaccggtacgctggccgtgccgaggttaaactccgggtggaaggtccatgcagcactgtaaggcgatgccggcgcttctacccagccttccggcaccaccaggtccgtacgtccgtcgccgttaatatcaccgctgcccaggccatgtcccgatttacggtccagtattgtatgcgccgtaaatgaagcactgcctttggtataatgatataccaccagcggatcattcggcgtattgggaattatttcgggaatgccgtcgccatccaggtcccaggcgcgggtggtttcaatattgccgggagtggcgatcacgtgttctttccattcattatcgttccccgggttctctttccataccagcgtttttccaaaccagccgccggtcacgtaatctatacggccatcgccgtttacatcaaaaggaatggtggagaagtcatcccagtattcgccaaactgctttaccggtccaatataatgacgcttgaagtaagccggtccttcataccagaaagcaccggataccaggtcggggatcttgtcgttgtttacatccatcacggcgaccgattcatagctttctgcagcgatctgccgcttttcaaatttcaggggcgcaggacctttggcagattgggcggaaaccgctgcagtcaataacaataatcccgcaacaggaagaaggcgttttttcatatcgaacagttaaacgtggaatagaacaagataatgaatacctgtaataaactatcctgtagtgtcctgatgggtcaggaggtatccccgctggtaaccgatccgcatgcaggaagccctgcaataatgtattaattgaaagctgcctcgtcttccggggaaaaatcccctttagcaaaatgcagggtaaagctggtgccgctttcgggcaaacttgctactttaatagtgccaccattctgcgccgcaaactccccgcagagcaataagccgaggcctgtgccacgttccccatctgtaccatacttcggatgctggtgggaagtgaacagggtgctgagttgctgcggcgacatgcccacaccgtgatcggtaatagtaatcaccacatcctctgctatcaccgccattacttctatctgcccgccggtataactgaacttcagcgcattgctgaagagattccggaggatcaccgacacctggtcgcggtccgcatacaaagcagtagttacgggtatctgcaattctactgtaatctgtttttgctgtatgatcagttcaaaaaaatgaagcacttctgttaccacgggcgccagtaaaaaatgccggggccgggtttggatccccttcatgctgcgggtactccagcgtagtacgttgtcgagcgtaacacccagctgcgatacttttttgtgcagcacatctgccgcttcctccatgtcctcgcggggatactgtcctttccggaacatgtcgagcaggctttccagcgtagccagcggactgcggatatcatgcgccacaatagaaaaaagtttttccttgtccttgttcatcgacactaatgcctgtcgctgctgctcaatttcctgctggtagtccgcctggatatacttaaaaaagctaagcgccaccactacaaataataatgccactgccacattccaccataccctttccaccggcaccggtggcgccaggtaccatgaccgtggcataaatataatcagcataaaagccgtgatcaccaggaggctcaggctccccactatccatttattatcgtaaatcaggattacgataaaaaggatgttcagtaaaaaatattccgccccgttatgaaaataaacaccggtaaacgtatagatcaggatactgatacagatcaacactatccttgcactaagatacatccggtacttatggaatatcagtaccaacacggaagtagtggtggtaatggcattcaggcccgccagtatatacctgccctggatcgtatttaagatgcaataaaaaaacatgaaaggaatacagggcaatgacaataaattcaataattttgtgcgcctggattctatatagggcatagcaggatgcacaccaacattcacgatgttgttccagtgatattcggctgaacggtatagaaattgcttgactccctgcagcatagatgccgtaaagatactttataacgtttgtcggcggaatatttttttacccccctccccacttcctttaatccaattatttatttttttaatttattaagatgaacaaaaaagtaagagatcacttttttatcgtcacgggtgggcccggcatgggcaaaaccgctatcatagcggcgctgcgtgaacagggacatatcaccgttccggaaacgggccgggaaattatccggcagcaggtagctgccggcgggcaggcactgccctgggtcaaccggcaggcatttgcccggctgatgtttgagcagtctctgcaggattacctggaacagccagccaccggccgccccgtatttttcgaccggggcattgccgataccatcggttatcttgaactatgcagactgcccgttccggaagaaatggagcacgccgccgccttatacaggtaccatcaaaccgtattcctctcccctccgtggaaagccatttatgaacacgataaggaacgtaaacaatcttttgaggaagccgtgcaaacttatgaaagcatgataaaagtatacagccggctggaatataagctggttcagctccccgaaaccaccgaggcggaaagggcggcatttatactggatagcaccctgcatcttcctttataaacaaccataaaaatattatcttcctgtatgctctttaactatttgaaaatagcccttcgtcaccaccggaaaaacaagctgtatgcaggcatcaatatcattggcctggccattggtatcagctgtgttttgctggcatttttatatttgaaagatgaaaacagcttcgaccggtttcatcatcagaatccacatctttaccgtatcaccactgctgtaacccaaccaggtggcagtccgcagtggacgggcagcaccggtcagttacacggcccggctttcaaagcgcaggtaccggaaataaccgcctacaccagggtgatgggcggggatatttacggggacatcatcgccggtaacaaagtactcaaacaacagctcctgtttgtagaccccggcttcttccaggtcttttcttttcccctggtaaaaggcgattccgccactgcgctcaacgacattggatcggccgttattaccgaaagtacggccctgaaatattttaaccgcaccgacgtagtaggtgagctgctccggatggacgccgacccttctgcccgccgcctgggaaaaccactggtgatcagcggcgtggtgaaagatcctcccatacattcttctatccggtttgatgtgttacttcccttccggtttatgcagttgtcgtttaacgacaccgactggaacaatgtataccttagcacgtttgtggttacccggcccgatgccaccataaatacagttacgcagcaactaaaccgggtgaatgcaacctatgcaaaggatcataacgccaccgccctcagttttggccttcaacggatcaccaacattcaccttcatcccctctactcacccgatggcaaccgcgaaggtggtgtgatcaatggcagcaacccggtatttgcctggatctttataggcatcgccgtatttatcctggtaatggcgggtattaattttatcaatattacactcgccggctccctgagaagaagcaaagaggtaggtgtccgcaaaattaatggaagtagcaatatacaaatcatcaatcagttcctgacagaatccgcgctgctttgcgccatcgcgctgctgctggcctttctgatggccgccgccgcgctgccggtatttaatgaactatccggaaaagccattgctctccaggcaatattgcagccgctaacagcactggccgccgccggattgctgttgttcatcattgcattaaccggcgcgtacccggcatatgtgctggcaaagttcagcgccaaaaaagccttttccgggcaccagccgctcaccggcaggaatatacccggacgcatattgatcgtcacgcaattttcactggccgtatttttcctcattgttaccgccctgttttaccggcagatggactacgtgcaaacgaaagacctgggctatcgccccgaacaggtagtggtaacgcatatcagcggcgaccgcaacctcaaacaggtacaggatatcctgaaaaatgaactggccagtgaacccggcatcaccggcctttcctttggaggagaacgcggcggcgcgagcgcagtacatcttcatgataaagaaatcgcagccgtccaccgggtgatcgataaaaactacctggctgcattgggcattacactcaaagaaggccggaacttcacaaacaactggtccaatggcgtaatcgtaaacgaagcctttgtaaaagctgccgggctccaaaatcccattggaacacccattcgcacggatgaatattttgataaggaaatgaggaccatcaccggcgtggtgaaagattttcatgccggctccctgcgcgaacgcattgcgccgatggtgatgatcatgagcccctggtacggcggcgacatatggataaaactcgaccctcgcaggcaacaggccgcattagccgcagtggcggccgcatataaaaaggcattgccggaaaccgcctttacctacagtttcctcaacaacctgaatgcacaggaatatgcgcaggaccaacgctggaaagtaattatccgttgggcggcattactgtccgtgctcatctgctgctccgggttattcgggctcgcgcatattgctacccatcaacggatgaaagaaatcggtatccggaaaatattgggcgccggtgtgaccagcatcatcacccttttttcaaaagagttcctgcaactggtagctattgcctttataacagccgctcccctggcctggatagtgatccatcgctggctacagggctttgcctaccacaccggtatcagcgcatggatctttgtggctacaggcagttttacgttactcattgcactggctacggttagcttccaggtaatccgcgctgttggcgctaatccgttgaaacacctgaatgccggctgataatataaaggaacaacgccggacatttcagcaggaaaaaactatatttatgcccggcgcccctccgctatctggggctaaaagtgaacaattatcctgatgacaaagactactttctttcaaaaaatcagtaccggattgttatgcggtttactctcgctaacggtatctgcgcagcaaaaacctaacatcgttattatttatgcagatgatctcggatatggagatgtaagctgctacggtatgaaaaggatccaaacaccgcacatcgaccggctggcgcagcagggcgtccggtttagcaatgcatatgctacctctgctacgtgtaccccttcccgtttcggcatcttaacaggcaagtatccgtggcggcaaaagaataccggcatcgctcccggcgatgcttcgctgatccttcctaccgaccgccgtacccttcccggcatgttgaaagacgccggctaccagaccgctgttattggtaagtggcacctgggtcttggcgacggtaccgggatcgactggaacaaatccatcagtcccggtcccctggaagcaggatttacctattcctttattatgcccgctaccctcgatcgtgtgccttgtgtatttgtggaagatcatcatgtagtaaatgcagatcccaatgatcctattgaagtaaactataaacataaaataggcaatgatcccaccggcctggaaaatccggaaaagctacgcatgcatccggatccgcaccagggacataaccaaaccatcgtagacagcatcagcaggatcggctggatgagcggtggcaacagcgcccgctggaaagatgaaaacattgccgggatcatcacccgcaaagccatcgacttcatcagcaaaaataaacaacaaccattctttctctatttcgccagcggcgatatccatgtaccccgttaccctaacagcttgttccggggtaaaagcggcatgggcctgagaggagatgctatattacagctcgactggaccgtaggcgaaattgtaaaagcgctggacagccttggactcacaaaaaacacgatgatcattttttccagcgacaatggccccgtactcaacgacggatacctggaccaagcggcagaactggccggcaaccaccaccccgcaggacctttgagaggtggcaaatacagcgcctttgaagccggcgccagggtacctttcatcgttaaatggcctgccggcatcaaagcaaaacaaacttccaacacactgatcagtcaactggacctctttgcttccttcgcccgtttaaccggccagtccatccagcccggtgaagcgccggacagcttcgacatgctgcaacaactgctgggcaaatcccgtcaaaaccgcccctacctcgttacacacgcgggcaccctcgccattatctccggcgactggaaatatatttcaccctccaaaggcgccaaactcgaccgcgatgtcaacatcgaactgggcaacgacaccgccccacaactctaccacctgaccaccgacgccggcgaacaacagaacgtagccgcacaatatcctgccaaagcatccgcactggctgcggaactccaggcaatacgcgataagccataagttaaataggggctcaccgcgaaggttgtctttctcaggattacgctgattttgctgatttactggattttactcttttggattttaaaggattttgggagatataagcggatatcttcgcttatatctcccaaaatcctttaaaatccaaaatgatcaatcaaaaaaatcagcaaaatcagcgtaatcctgagaaagacaacatccgctgcattatttcgcatgggcggacctgtaatgttccagcagcaggtcgccgccgaaatcgtttttcaggtcccgtacgatagtgtgaatgtggttggcgttattttgggtattgtcgtattcgataatgaggccggggccctggatgcggtagtagcaaggattacccaatgcatgtactgtgctcccggcccatgtaaaccacaggttatccaaaccatcttgttggatatccttcagcattttatcggcaaacagtttggtgaagcgatgcacatatacgttaatgagctggagtaacaattgctgatgtgcggggctcaactccttaaaacggatgccttccgggtgtgcaatcatggcgttgcggctgttgcccgtaatgatttcagcaggcgctttggcggttaccagcgccttctgcaactccgctggcgacagggcatgcacaaggtcaaaggccagtgttgtttcttctttcagtacttccttatctttttgtggtccgtccagtacaatagcaggattagcgcccaggaaagccggggtgcctgctaccagctcttttttatctgccgaaaaattaaatgccacatgatgcccctcaaaccgccagccccagatagtattggcggcaggcaccccaaaaatggtgacgaagtatttgccggggtcacggtaatgatcgttctcttcccggtgttccagctgtttcaatacctggtcgagctgcatgatatcattcacctttttcacggtggtttcactcagcgccgtattcaataaatccatgagcgcttttcgttgcgccgggttcagctcatttacagaaatacccttccggtcgtcccggggaacataagcaaaatgatagcgttcaccggtatcgaaaggaaagagtgtttgtgcctgctgcgctttactgagcaaccggataaaccggtttgccttttcagacatctcctgcgcccggagaggcccggtgaatacgcaacaaccaataatgaataacaggaccaaccggtgcataaggagcatttgaataacgtggaaaaataataacagataaatatagtcgatcagcaacgattctgcaaccttatgccggaatgaaaaaaatcaaaaaaatgattaatttagaaggataccccttatacataacattatgccgccgaaagaccctgttaaattaaccgtatccgattttattcaccaccacgaagtgattgcggagctggaaagtttaaagcaaacctttgatcctgctgccagtggtggcaggcccctcatcgtttctgacgtgctggatgccgatggtcatcaatatgtgaacctggtacagaaaggcggcggcgtatttggcattgccctcgtaggatatacctatatcctggaagaaatgggtatccgtttcctccggctggccggtaccagcgctggagccattaacacggcgctgattacagtgattaaaaataaatctgataaaaaatcagcggaagtattacaggccatctgcgacctggatttcttttccctggtagatggacatcccgcggcacgcacgctgatcaaaaattttattacccggaaaaactatatcgataaagccaaaaataagctgttggtggtactggcggcatttgcattgctgatagtgggtgacgtggtgctggtgggattgagcaacaaatatcccgcgctgtatgtatggaccggcatctgttttattctcagcggatttttatcgctggtgattggcattggtgtttcttatctgattgatctttttaaaagactgaagaattcagggtatggaataaatccgggagatgttttttatgactggatcaaacggttgctgctggaaaaccaggtggctacggtgagcgatctgaataggaaagcggccatttgcccggcactgcaactgcgcgtacctaatcaaagcggactcgaagaactgaaaggagatgtcacctttattgcctccgaactggttacgcaaaataagatccagttccctgccatgtgctcactgttccgcacggatgtggatacactctcccctgctggcttcatccgcgcgtccatgtctattcccctcttctttgaatcttatatgatcaatgatattccggcaaacgacatccagatcaaagacgcgtggaaaaagtttttcggtatcacgcagccgccttccactgcccgctttgtagatgggggcatcctgtctaatttcccgatcagcattttttttaatcccaacgtaacggtgccaagactgccctcctttggtatcgacctggacgacagcaagcccgccgacaaacaggaaaatgccttcagctggtcgctcaccgggtacttcgggcgtatgtttaatactatccgcaactattacgataaagacttcctgcttaaaaatgaagtgtatcagcgcggtgtgggaaaagtggacctgtcgtccgatcagtacaactggctcaacttcttcctgtctgataaagataaaatcgacatgtttgtgcttggcgccaaagcggcctgtgaatttctaagaaacttcgactgggaaacctataaaaacgaccgcacagatcttcaaatccaactcaaaaaataaatatggaacttattatttcaaatgcctggtgttggttatgtttctctgcggccctgctgctgcttaccgcttttattatgctccggcaggcgcgccagttctacctcctggatgttgtggtacgcaagttcagtatcatcgatctgcagttccctgcttcttccaaagaaattcccgagctgatcaaagggatctacgcattgcctgccccccagcaatcacgtacgctttcagccctccgcggacagctgtgggtcgacttcctttttatgccagccttttatggcagcatctttttgttatgcatacaggtggcaaataaaatgacgcctgccggcgaaatattttttgaatgcctggcatggcttcagctcatcgcgtggttgtttgatgtaatggaaaactgctacctgctcaataaaataaaaccaggcgtaacgccctccactcccgaagtacacaaggcatatcagcaaatggtgtttgccaaatggatcctgttattaaccggcatcgtatgtgcattctccgcattgttgtttttctgggtgtcagggaaatatgaaaccagttcgctgcactacctgttaatactgacaggtgaaggagttgtatttgttacagcgcaggtaatagccggcaggcgcaaagccccggaagatgcagcaatggtcgtataacagctgttagtaagatgtaaatttatttaatcattccacgtttcacgctaatttccatgaacacgatgcaatccagaagacattttattaaaaacgcgggccttggtcttgcagggatcgggtttcttcctgtgctgggtcctgttggtcagctatggcgcccctccgtattgctaccgcacgcccttcccgaatcgcagggagtatcttcccgcggcatcctttcttttatcgaagccgccaatgcttccggcatcagctggcatagcttcgtattattaaggcatgggcatattgtggccgagggctggtggaatccttactcagccgaatttacacactcgttgtactccttgtcgaaaagctttaccagcaccgcaatcggcatgctggtaaaagaaggcaaactggatatccaaagcactgtggtgtcgttttttccaaaagacataccggctaacccgtcgcctaacctgcagaaaatgacggtcaaacacctgctcaccatgaacaccggcaacggcgcagacaccctgccacccatgcttaaatcaactaaaacctgggtgcaaactttcctggaacaaccagtggaatttgaacccggtactcatttcctgtataacaccggcgctacctatatgctgggtgcaatcctccacgccatcaccgggcaaaccctggaacagtacctggcaccccgcctgtttgagccgctggatattaccgggtacgattgggaaacctcgccacaaggactgaataccgcagggtatggcctccgcgttaaaacaacagatatcgccaaactgggacagctatatctgcagaaaggaaaatggaatggcaaaatacttctctctgaaagctgggtaaaagatgccaccggctaccaaacctcctcccaggaaggtaatggcgactgggcgcagggctatggctaccagttctggcaatgcaggcacggcgcctaccgcggcgacggcgccttcggacagtattgcatcgtaatgcctgataaagatgcggtgctggctgtgaccagtcaaaccgccgatatgcagcaatccctcaacatcatctgggaacacctgctccccgcactgcacgacaccgtgctgccggacaatccatcagagcaggcggcactcaaaacagcgctgggtcgtttagccttgcccgtggtaaccggcaacatggctaaagacactgcttcccggtaccagcgcaaaacctggacactggataaaaacgattttaacgccaccaccatgcagttcgatttctcaccagccggttgcacctggactacccaaacaaccgaaggcgtagccagtatccgtttaggttgggaaaaatgggtactgagcaaagaacggcagcactataaatttccggaagtgggattaaatcatcagcccaccaaagtagccggcaccgccacctggatcaatgataatacgttgcaactgaacctgcgctttgtggaaacactgcacggcgacaggattcaatgtgtttttgaaggagataaactgaccgttacattcctggatagcttaaccgccatgtctgccggaaaggccgatagccggaaaccgttgagtggagtgatgaagggttaagccgggtatgcaaacgcgttgcatattttagtaactgttgctcatggttggtaaagagctggtcccgcttagtgagcgggacttttttcttattgatccatttgatcatgttgcctttttgaaaataagcccggtcttcttctatcctgatatttttactgctaaaagagctgtcgtacatcggaatgttataatggtagtcccgtgtataaataaataccggcgtcccttgatcgtagtagatttcggtccgcttttttcccatctccccatacacatcctctacaatgagcacaatgctatctccggaaaaatagcccgtcaccgctccgccctctgtacttcgttcctctgtatctatcactacctggcgatacgttctgataccggcattgatttcccggtaacgctccatgatgtgccgggtgtcagtcccggactgataaaaaacaagtaagaggcaacaaaccttcaggtaagacatgtagaattgtatatttaactgccacaaattaaacatttgatttcctattttcacaattgtcgcatatcgccctcaagaatgtcgttttaacccaccctcgcatcacggtaacagcgctacctttatcttacaaaatcatattcacatggcaactgtaaaagaaaaacccgcaaaaggcaagctgaacaagcagtttagcgcaacactactgaaaagccccaatgccggtggctggacttacgtaatatggccggattcggtggcatttttcggcacccgtggcctggtaaaggtaaaaggcaccatcgacaaccacccttttcaaagctcgtttatggctttgggcgacggcacacataagctgccggtaaaagtggaactgagaaagctattgggaaaagaagccggggataccgtaacggtgaagcttacggagcggctttaaggggagatagtgcattcatagtgcatggggagtgcatcagaagtgcatggggagtgcatggggagtgcatgctaacagtattgatagcgcatggatactccagggtatacgcaaggctgaggcatgggagaagtaaccttgaggtagctgttactcctgtccgttatatcgccaatcaacaccaaacctacctaaacatctcccaaatcacctccccgatattcccactgggcacctggatattcagcaatgccgccacggtaggcgctatatctgtcataccggtggtacggtaggtgctacccggctttatcccccagcccatccatacaagcgggatatgcgcatcataaggataccataagccgtgtgtggcgccgctccggccgccatctttccagccggcctgcatcagcaggatcacatcaccgccgcgctgcttattgtaaccatttatcagcatggtgcgtaaaggctcatgcaatgcagccgtaccaagatcatgcaaactaacggcatcggctataccgggagttgcctttagtttttctatgactaatgcgataacctgttgcaacggaatgttccgcgccgcaaaggcggaccggtcgaggtataactggtaggccgataaagctacgacgccttttgctacgccaaattgctcagcgatagcggtattaatatccttcaatacaatgtctgcatccagcaggccggtgggcagccggtgctcttcgaggaagccaggcgactgtgacacgccgtgatctgcggtgataaaatagaggtagttgcctttaccgaatcttttatcaagataggtgaagaatgcttcgaggtctttatcaagacgcaggtatagatcttcttcctcgatggaattaggtccaaactgatgccctacggcatcgggagaagaaaagcttacggcaagaaaatctgtttccgtaccggcgccaaggccatagccttctatggctgctttggcaaacgcaaaagtaagcgtgttgccataaggggtggtgcgtatggaattcttttccctgccggtgaaagtatgtggaaacaccggcgccgtttcatgaccaaatgatttttcatagtctttattgtccgcatcactttgtgtataggtggtaatgggatatagtgtttcccagccttttgccaggtatttcacgggcaactgttgttcattgaaacgttgcgcccattccggcaatgctttcatataataactgctggaaataaagttacccgacctgccatcataccagaaagccgcattggccgtatgacccgcaggaagaatagaggccctgtctttcaatgcaacgcctaccaccttacttttgaaattggtcgccagccgcagctcatctgtaacagtagacaccagcagattgcggggcgacatattccctgctttcccttctgctcctaccgtggtttcggtgctatcttccgtgcaatacacggatcgctgcaacgcgcggctgcaccagtcgttgtccacgatgccatgcaccgccgggctgctgccggtatacaccgacgtgtgcccgcaggccgttaccgtgggcgcgtaattgatatacgtttgctcacatttaaaaccctcgcgcaacaggcgcttaaagccaccattcccataccttgcggcataccggtacaggtagtcccaacgcatctggtctaccatcatgcccactacaatccttggtttggatgcgggcgcctgcgctgctgcggtaaccgccagcaacaccaggatgcccgctgcataaagttgttgtatctgtttcatattttaaatcagtccagtattttcaggtaacgcgccatccaataaggcagcaaatattcatctcccgccagctcggattcaccattgccgccaccatccagggtaaaggcattggcattatgacgatgcaccggctgttcatccagtggcagcagtacttccgtgtactgatgccggaaattaggcggaagcagtgtaatgtctttacggtttgaattggtaaccttccaggtgatcaaatccatcgggaaagtttgcagccaccaggtagtagccggggcgtcgtaatcgcccgaggtagccagcgcaaccagattccatacggcattcttttccggttgctccacttcccagtgattgcggatagcgcctttatactgtgccctcagctcatccgtgaaggcgtatttatacagcacccaataagtaagaaaggccatctcatcatcagaatgattccagtcgcccatgcccatatcaattccctggtgcaggtatcccggtgttggtttgatagtgcggtagtcgatctgtatatttttcagatagccgtgcctgttaagcagcttataggcttctgttttatatttttctttgccggtcaactgatacgccagctgcaaacccgcaatgatagtggtgctgcccagtcgccggtcgccaatagtagtcgggtaccagttgatgtattccgggttccagcgcgcccacagtgtgggcttgttgtcgatgtccaccatcgtatacttatgatccacaatgtgtgtcatgatcttatcaataaaagcagcgacccgctttttttcgtccggcgtttccgccaccatttcatgtaatatcgccgtgatccagatataggctacatattcatcgctgctggtatggcctttccactcccattcgggatcgggtgagtcgcgccatctttcaggatcagaatttttatatccttttctttcaaatgtccgggaaggaaaacctgttaactggttgatcgataaaattctttcaaaggcttcaaaagcttcccaggcatatcttttagccattggatcatgggtaaccgcataccggaaagcctggctgccgagataaaagctgctccacaaaccatcattatccgtatccgccatttcagctgatcctacatctcccggcgggttcaggtgaaggttggcaatgaagccatagcggatgtgccgctcgcgtatcttacgctcaaagtaggccgctttctgcgccagtgtttgttgtataaaagcaattttattaagaccggtaccggtgagtacatacacatccccatggctgtcggcagccatactttttaccatatcctgatccagccagcgtttggaggcgaagtagcgataagtgccggaatcagtgcgcataaaagcgccggcgccggtaccagcccagatatgtccattcgacaccagcagttcattaataacgggaacgggcacacgtgtttgcaacggcatactcgtatcacctgtattgcggttaatactgtagtagccattcgccgtaccaagcaggatatcatttcctttgaaagccatggcagtagcatctttcaccgtatgcaccaccacaaaacgctgatctttcagcgcatacaccgctttattggttaagataaagaaagtacctccgttggcttccatccgttgcaccccctccgggatcagcggcagctcctgcagccttccattgttgccaatggctaatgcatccttgccggacaacagcatacgaccggcagcatctaccgccacccggttaaatttcccctgcgggagattaatatacgggatacctgcatatccgttggtcaggcatttatctgcgtagagataatacaaatggccgcttccctcctgcgtggtaacatccacggggatcttctgtgccagtgggcggaagcgcagatcgcgcaccaggtcgtttccgctgaggcgataaaagccttgcttcgtaagcacctgcacgttatcgttatagtcggtgattactttaatcagctccagtccctgcggaatgctgtacttaacggaaaccgcctgtataaaaggctggtcagacgcggcacgggcggagcacgacagtagcacagctgctgcaaggaaagctattttcttcatcccaataataattttataatttaatgagccacacttctgcaacccttgaatgttgtcgccagtttaaatgttcttcgttgatatcatcccatgttagcagcagtgtgccgcttttgctgatatcagcaggtacgggaaattcttttatctctcctgttcctttgttataaagagatggtttcagcaatacgccattcgcccgcagcaggctttcgccataacctgttattcttactacgtaatgcgcagtagtatccaggtgatcataacgcatggcagcaggccagcgcaggctcaccatccacgacaaccgcttacggctgtaaccactttcccaccagtcgaaacccggcgtatcgctgcggcgcatcagcggatccgtgtgcaggtcttccttccggactacatgcggcgatttcgatacattgccaatatcatcatagaaactgcctggccgccccgggttttcccatctccccaaagtgtccagcgccttacgctgctcagctaaaggaagcgttttaatataacggaacttatcttccagccaccagcggttattcaacggccggtccaggaaatccagtattgccccgcgttccggcccggcggctttatactttgccacactggtttgcagggataccgatttatacaggtcgtcgcacaatgctataatacgattccgccattgcggcttcactttttgatctgcctgttgtaatatcctttcggcgttggcgatctcattgcccttatgttccagcaaggtgcggttgacctccgcttccagcgtggcctcccggatggcacgttcacgggtatacgcatcgtaatacgccctcagcaaacacatttgccagcgccagttgccagccaactctgcgtgtagccgttcctgttgttgccacagtgtaagcgtggctgttataccgccgttatccgttaccggtccttcccagttcttttccagcgccaggatcccgtctgctattaattccggtgaggcagaagggaaaaagtaattggcatactggatcatcatctcccgcacatcggccttgctattccacccaagcatgctccagagcatcttattaatatcgtcatgcgcgccgtcggagtagctgataaagccatccatatcaggcgcaataaaacggtaaatgtttgcataatataccggctgcgggttcaccggctcacggccaagggtaaacgcaaatgcggggtcccaccatactacgggatagtcgcagcgaacagtatgcgtaatatccgggtaatgacggatcttgtactgtggcggcaaagctgccctggtattttccagcgaaggactggacggccctactacaatgcctcccagccacaatggtttacgttgatggatatacgaataaacgaaagcgcactccgtggaatcgtagccttgcagcgataaccagatggaggcttccggatgatactgctttaacggaaccgccaactcctccagcagcggcagcaccagctgcggtgcgttgttgccgggatccccgccaggaaaaaatacggcattcagccgcactgtctcgcggaacagcgtatcaaactgcatcaggaattgatgcttcttgatagtatccttcaggtcaaacgttgcgggtgtccacaccgaaaaatccaggtcgtattttttacagtacccgctgatccggtgggtcatctcgttggaagaaacggtgaaatgcggcgacgccggcataaacggaatcgcttctatactgttggccccgaagatggcgaggtcacggatatactgttcatattgctccggcgtccatccgtcgtaggagttggccaggttgcggtatccgatctggtgaccgcggattcctttctctggtgtggcgtctgcatgtatctcctccggcaacatcgccgccttctggcggtactgcataatacgcagcaaatagcccgccccatataacaatccgcgggagccatctccctctacgagaataatgcggcctgttctatggatatgatacgattccggtgcacatggctttgtctgaaagatgattaccacgccattatccggcgcctgcgctgtgatgggccatacaaggccggtacggcgtttcacttcttcctgtaatacctgcgtggcaacctgtttatcttttgacacaatggttacgggtggcaatacagacccggcacaaagttgcggaatgaaaaataatatgatcaggaatcctctcattatttcataaactgatgattgtaaaaaaaggaatagcaggacggttatttcattgtattcttcaggagattttctccgttggcttgtttttccaggtcaaaagcatcatacaattcgccggtagccgtataggcgcggaaagaaaccaccgcgggcttaacatccaccacctggaacagctgcgtataagagccggtgcgggtcatccacggctgcggatctatctccgacattttgggtccgcttacagacactacgtataccggtcccttgttgccgtcgcgtccacgggcataggtatgatcatgtccctggagtaccaggtctactttataccggtcgaacaacggcttaaagttttcacgcagccgctcgttgttgcggcttttcttggtcgacagtaccgggtgatggaacgtgatggccgtccaccggttgggattatttttcagcagctgttccagccataccttttgacggaccagcaacgtatcggatatttccacttcctgtgaattcagcgaaataaaacgcatgccctgcacatcggtatagtagcaggtttcctccaaaccggccgggccgttttccggtaaggtaaactgcggccgccagaaagcagaaggcacatcctggcctgcggcgttttcatagtattcgtggttaccggtcgtcatcatacccggaactgtgctgtgaataaaaccccctgcttcaaaccattgctgccattcattgttgttattgcccctgttcaccaggtcgcccgcatgaatgatgaggcgcgcatccggcgccacggaccaggctttccggatggtccttgaccacatggaaagaatatttgcctgggcatctcccaggtaaataaacgaaaagggttcaccgggcaatcctgccgtacggaaagaaaaccattcgctccagtcgttctcctgccctacgcggtacacgtaattggtattgggttggaggtgatcgaaagtaaagtgatgataccgcaccggtaaggaatctgcgaaaggcggcgtagtaacagcagtataccgtgtagccgttgccgtgaaacgtggatcggcagttgccggcgctagttctgcatagctaaccgctgccgcctcacccgttctccaggtaacagccgctgagcgggaagggtcggctgttacatttaatacaatcctgtcgggccgcaaacgctgggcatatacttgttgtaaaaagcaggtggccagcagccacccgcttatcaatattttcttcatagcttttacttcaggtaccacatcagcgtggtttgtttatctgctccaaatacggtgagtgctttctggtactgttcttcattggtatctctttcgccggtgggataaatataccgtttaggcagcaccgtagtggatgccattgggccgagtacaaacttaggcaggcccgtgcggcggttatcaaaccatgcttccgcgcctttcaggaaaccggcgatccacttctggccaatgagctgttccagcgtaccattgtattttacagaggcctggttaaagtagccggcatcaatagccgcctggtcaactccataaaatttcatattggcatggatgccatcataatacaggctttccgctgttttgcccggcaccgttactttgcctgcctgcacacattctgcgaggataaagcaaacttctgcataggtaagcatgctgcccctcagcatagcaccactagggctgctgaacaaagaagaaaggcgggaaatatgatacttaccaccattgtagtcgtaaggtgcaggaatcgcattaggtacgcctacataaggattcgggttggttgtccctcctgtcagcgaatccacccgcgcgatccaaactttcaggcggggatcattgcgctgtactaaagcatctacaatttctttgctgggtttgcgcttatcaaattcatcaaaggaacttcccagcgggctacccggccagctattggcgctcacagtaccctggtatataatttccgcgttatctgcgttgctttcaaaaatggggtacttactcttatcgttcaggatctcctgcatttctgtaaaggcagtgggatattttttggaaatgcgtaacagcatccgcaaacggagcgaattggcaaacttgcgccagttcaacggttctcccttgtacatcacatctgctaatgtatctatcttgttggtaacggaagacagctcatcatttgcttctttcaacgtttgcaataaggcagggtataccgtttgctgcggatcatacttcggatgggccagcgtttgagtcttcagcaacaacgcttcactgtaagggacatcgccaaacagatccgtgacatacgcaaaattaaaagcttccagcaccttgcctacagatacatactgcggtacattcagtttcttcgccaggtccatcatctcccggttggccgacagctttgaatagtagctatcccaactttgaggaccccagtcgaacttatcattgccctcattacgcaccatggtgatataacggccggcagaagcaggtttatcgaagtaagcctccttctggtaatcataggcggtgttaatcaacacggaggataacaggaattcaggattgatcacttccgattcattcggattcacattgatatcttccagtcctttttcgcaggaaacaaagaggacgccgaagattagtatcaggtatttaaaaggcatgcgttgcataaccatataattattggtttagaaattgaaacctaccttagcgccataagaacgggtgtaaggcaatccccagctggctactcccggggagaaactaccgttggaaatcgtcatcgccgtttccggatcgtacccctgttccgcagcagtccaggtaaacaggttgcgtgcaatcagtgatacgctcaggttacccagtggtagcttgccgagtgttttctttgaaaaggtataggtaagtgatgcttccctgagctttacatagctggcgtcgaaagtagaccggccggcatagtcccagtaatattcaccataatagttctcgggatctgtaacattatcattgagcttgtacttgccattcccgtcatctatataaccgaaaaggatcatgccatctgtacggttgttgccatccgcatctttccaggccagaccaccggttttcggatcgcggccggggatagtggtttgtgtgcggccatcgctcaacaggttctttgccacataagagaagaagttaccgccctggcgccagtcaatcaatacattcagggtaaaacctttgtaggtaaatgtgttattaatacccagcataaagtcaggattatagttccctatcttcacatactcatttaactgctggtaaccaccttcactactcaataaaggctgtcccttaaattcaccatctggtacagtggcccaggtttgtgcatacatgtctcccatttcagcaccttcttctaccaggaaccggataccttctgcactgcctaactggtagctgttcaagccatctatcagcttcagcactttattgcggttacgggtatagtttaattgcaggtcccagcggaacggtcctgctaccggcgttgcattcaacccgatctcaatacctttgttcctgatcctaccggcgttggtcaccatgttggaatacccggtggccattgttaccggtattttgatgatctgattacggtttacggtattataataagtaaagtcgatgccgattcttcctttcaggaaacgaacgtctgcaccgaattcatgcgaggtagcaatcagtggcttcagccggttatttttcaacacgttgctgatattcgccagttttgttttgtcccagtcctggccaaagctaaaggtgttatacaaattatagggatctgtatcgccacccacctgtgcccagttagcacggatcttagcaaaagacaacacgtccgattttatacccagcatatcggatacaatcaaactcagtgaagctgaggggtagaaataggaattgttgccggcgggcagggtgcttgaccagtcgttacgcgccgtcagatccaggaatgcataattgcggaagctcacctgccccatgccatacacgctgttgatacgtttggtatacctgccggaagtatttactaccgaaccggctttggcgttggcaatattgtacaggccaggtatcaccaatgcttccgatttctgactggagcctttagtgatttgattcatacggttggcgcctgcggaaacagatacaaagaaatctgagttgatattcttcttatagcttaacaggaagtcggtattctgttccctgaaaaattctgtttcaaaagcataggcgccggttggatttttcaccgcactgaaaggccgtttactttcgcgggtttcagagtaaagatccatacccgtgcggcccatgagcgacaggtctttcgtgatctggatattcaattccacgttaccggtcatacggtcacggtcaaacccgttgataaattcatatgccaccaggtaagggttatccgtagatcccggcacatgtgaaaactgctgcaatccttcctttccgggcagccagtagttgcgcagctgcctgatgtccacgttgggtgtggtggtatatacaatgttgctcacgcttccccggttaaaagtaggccggttgccgctgctgtttttcgtatagccgatattggtactcaccttgatgttgggattcagattatatcctgccgcaaggttgagcgtatttcttttcagatcagtattgggtatgataccttcatttttcaggttggtaaacgacaaccggaagttaccatccttgttattaccggtgatggcaatgttgttggtgaaggtagatccggtgcggaagaaatccttatgccggtcgggataagatacccagtcggtaggaatcggctgtccgttcgcatccaaaggactattccactgtacgtgtttggtgcctacatccagtcgtggtccccaggaagcgtcagaaatagtttcatcagaaccttcacggtcgccggaaccaaattcattctggaatttcgggaacagccagggttgatcaaacatcgcgctggagttaacggaaacgcctaaaccttttgtagtacctgagccggatttggtagtgatgagaatcacaccgttgatagcgcgggagccgtataaagcggaagcgctggcgcctttcagcaccgagatgctggcgatatcgtcgggattgatatccgagatggtgctgccataatccactactacctgtcctacgggctgtttcggattacgcaccgccggtgcaatgggaataccatctactacatacaacggctgattatagccttccaggctgctctggccgcggatggtaaccagcgaggtgccgcccgggtcggagctggtgcttcttacgtttacaccggttactttaccggctaaagcgttggcaatgtttacttcttttacggtgctcacctggtcgcctttcagcgtggcgatggagtaaccgagtgctttctcctggcgtttaataccaagcgcggtaactaccacatcatccaaactgcgtatggtagccaccagctgtacctgcagcattccgttgccagccaccgtttcttttgactggtagcctacagaacggaataccagaacggcattgctgccggctactttgatggtaaactgtccgtctacgttagtggccgtaccattagaggtgcctttttcatgcacgcttacaccgggaagggctacaccgctttcatcggttactatgccttttacggttacttcctgcatttttgtggcgcctgcttctccgccggcagggcggattgcataatcatgatcgcttaattttaccgcctgcaaacccagtggtgtaagcactttcgttaactgtgcttccaggttgctgccggtaacacggagttgtttccccgctacaaatttatccgccacttgtgtgggcgaataattaaagctgatgttaaaccttgtttcgaggttggtcagcatttgccggagtgggatggttcctgcttcccccggagtatctccgcttcttaccattaattgctgtgcgctggtttcggtgttcagcagcagcaacaacaacagcatcgctctccagggagcataaagcttcgtaaagctcttttgcataactgtaaattttaaaaaccttattcaaaaatgatgactgaattatcttgtttgattttcagctgatgcacggtggctatcgctttcaacaacatcgggggatcatcagcaggcacagagccggtgaataacaggctttccattttcttattcctgaactggatcttataaccatatatgtcttccagttgctgcgcaacgcttatcagcggcgtatccctgaacaggagccggcgttgcttccaggcggtgagttgcacaggatctgcctgcagccggtgatgttctcccggcgaaaaagacatcatatcgccgggtttcatatccaggctgtcgttcaccacaatcttcccttcttccagcaataccttcacctgatcatgacggtgatatacattaaaggcagttccttttacttcaatagttacctgtggcatcaatacccggaatttaggatgcagcccggcgggagatttggatacattaaaataggcctcgccattgagcgtaactgaccttacgttttcctttgtccatttacggggataagaaacagatgaattggcattcagctgtacaatagagccatcgggcagttgcagggttttggtttcaccaaagccagtctggacaaaaatgttttcaacggatggctcacttccctgtgcataccatatgccggcaaacagcagcacagcagcagcggtagccagtgcgtagtaccacggcctgcggacaactacgttattttttttaataacgggttcgtccagcaacaggtctatctgcgctttcacagcctccatttcttccatgcttacttcgttggtacggaaccgtagtgccagcaccaatgcgcgggcatcctgcaataccgcctccttctccgggtgtaccgctatccagctttcccagaaggccgcagcagtatcctccagcacccaggcacggaataagtcatccgcagcaaaatctgctgcctcaaattcactataattcataaaaaaacaccttgtacaataacaagagacgcggatgcggaaaataccctcacggaaatggatcttttttcgcgaatgttgtctttctcaggattacactgattttacggattaatttgattttactttttggattttttttggattttttgatttaatagcaaagggagatataagcggctatatacgcttatatctccctttctcctttacaaaatcaaaaaatccaaaaagtaaaatcaaattaatccgtaaaatcagtgtaatcctgagaaagacaacattcgcagcgcggcttcatcctgtgcgagcagctcttttaattcagcgatggcccggtagatgagggtgcgggcatactttacttctttcaataccataatgtcggcgatttcctcgtaggaaaggccctcgtagaagcgcaggtatacggcttccttttggcggagggtaagggcgtttagtttttgttgcagtagccgggtggtgttttcactgtgctgccggttgatgaggatactttccggggaaagctccagggcgaaggtggaggcggcgccttcgtcgagacttgcggggccgtgggccgacttgtcgaggtacctgaacagctttctcctggcggataccatcaggtagcttttcaggctgacaggaagcgaaaggccggccctttgcgcaaataactgcgagaagaagtcctgcaacatgtcctttaccagcgcccggtctgttgtaaaccggatacagtaccggaacagcaacgggaagtagcgccggtatatttctccgaaggcgtcccggtctccgctacagagccggacccacaggagctgttcattttgctgaggattgtatgggctgcttgacatctattgtgtgaattagcataaggatctttctctaaactacacattggccggttgccgtcataacttcctgtcagaaataacatcgatttaatgtgagggcaaaggcgccgacaccacttcccggatctgtaaacgctcgcaccagcctttaaaatcacggtaaatctgttgcaaggtttccttctgttccggcgtcagctccagcgcatgcgcgcggctgatggtgcgcaccggaatgccccttaactgcagaaaatattttgcgctcagcgggtaagctatgtggatcagcgggtctactctttgtaactccgattgtatccaatgcacatcttcctgccggctttcatcatttacatgattacagagccataccagtatttcaggataaaaatttccggagatagacgacatgccagctgcgcccatttgcatagaggctaccgcattaggcgtatgggcgtcgtagaactccagccggcttcccgctgtcacggccagtttggcgcgcacgttttccaccttgcaggaagtatccttgtgataaatgaggcggttggtagccagtaaggtttgcaggatctccggcgtaatcacccgtttataaggcgccgggcattcgtataatcctaagggtatattgccggtaagagaaaacaattcttcgaatctttgcagcagtacggaatccggttcgtctacattggcaaagtgcccggtgatcataatcacggaatccacgccggtgtcatagatcttttgtgtaaacagggccttgtctttgatcgtaagaccaaaggacccggtagccactaccggcacgcggccatttacatactgcactacgtggcgggtgagctccagtcgctcatcctcgctgatgctgtacatttcggacgacaggcaattggcgaaaaaaccttttacgccggcatccagataaaaatctaccaggtgctccaccatgtcatggtcaatctgtgctttcagattaaaaggggtgatcatcaccggtacaaatttcttttgcataacaaacgggtttaaataatcaggaagttttaaggcgttgcagccgcgatagcagcatacccgccaggaatattgataacgttcccaccacgatgatcatatgcgcatgcaacgggctgcgcaggctgactaacccggcggggagatactttgataacgacatccacaggatgactacaataccaatgatggtagcggtaacggccgtggcattttttgttttggagataatgcccagcaaaaacaatcccagcatgcctcccgcaaatatgccggacaactcccaccacatgtccaggatactcttcactccaatcatcgaaataccaaaaccgatagccagcaaacccgacaaggtagtggcgatatacaacacccgcatctcctttgcaggcgtgatttccggatcaacataccgctgataaatatctttcagaaaaacagtagccgtgctgttcataccactgctgacggtactcatcgccgcagaaaggatggctgctacgatcaatcccatgagccctttcggcactttggtaaccataaaccagggcaataccttatcgccgtaatcggctggctgtaacgatgcaaccggcacctgcctttccgccgctacctgctgtttcagcgccagcagcagttccgggtgctgttgcgcatacgcatacaaagcagtgccaataaaaaagaacaccatgctcaccggcacgtaccaatacacacaaagccatatactgcgcgacgcttctttttctgaacgggcagtatggtagcgctgcacatagttctggtccataccaaagttattcaggttaataaaaaatccatacaggaacaccacccagaaagtagaagtactgaaatcccgcagggaaaaactacccagtgaaaattttccatctgccattcctatcttccagatatccttcaccccatcgttcatacctgtaatcaccagccagaggatcactatagcgccggcagttttcacaataccctgcagcacttctgtccatatcaccgcttccataccacccaacaccgtatatataatgatgcatactcccgtaacggtcatgatagtacgcatttccaaccccgtaagtgcctgcagtgccagcgccacaccaaaaaagatggagcccatccgcgccagctgcatcaggataaaacaaaccatcgcataggttcttgcccatgggccaaaccggtgttccaggtgtgtgtatgcgctcacttccccgctgcggcggtaaaatggcacaaaatattttgccgcaataaaagcagccagcggcatagataaactgaacacaaaagcattccagttactgccaaatgattttcccggcacgccgagaaaagtattactgcttaaaaacgtggcatacaaagaaagccccaaagcccagcccggtatagttccggacgccgtggtaaattgtgccgcattcccgtttttccgtgaaaaccatacccccactccaatcatacatagcaggtaaatggcgattacagccagatcaattattggcagttggtgcataatgaatctccgattggtcgataaaaccagttcaatacgtggataaaaaaaattacagtcgttacacgaagattactaatttttatggatcaaacaatgttgaatgttatgaaaagaatagcttaaattactattgagatgaacaacctggccgccaacacaccgaccacctggaacttaccggaccacctgaaacgcaagctggaaaagcatccgcttggcagaaacctttttattaccactattggcctctatcctgaaaatgctgccctggaaatcagtgaaccaaagggcgcaccggtgtataccttattatatgtaacacatggaaaaggatggctggaaaccgggaaaaagaaagtgactatcaaacctaatcaatacctgctgttcccgaaaggcgccgcattccgctccggccctgctgaaggggagccgtggcggatctatgccgtgcaattttccggcaagctggcagacgacatatacagctacctgggcaccggcctgaaaccgcataccataccgcccctcgtaggacgcaatgcacagttcgatgatatcctccatcatctcgacctcatgaataatatagagaacctgctgtacgccaatttccggttctatagtttccttggcaccttccggctcacggttttcaactatatgaagaagggcgcagataatattattgaacaatgtatccagctcatgaaacaaaagctggaccagcacctcaccctggccgacctctccagggaaacctgtatttccgcttcatacctgtcggccctcttcaaagaaaaaacacgctactctcccatccagctgtttacctccctgcggatgcagaaggccagccagctgctgaaagatacccgtttgaccgtaaaagaaattgcacaggaaatgggctacccggatcaatacacgttttccaggtcgtttaaactgatcatgggggtatcgcccaaaaaattcagggataagggctgaatgatattaaccaattgttaagcagtaagaagcagtgagggatatggcgtttcaaaacgaatatatagaaggaacgaaactccttccatcatttaataccaaacactcatgcgcttttttatcccccgttatctgtttcttgtactgcctgtatactgcctgtttacaggcgcatgtaaaaaagataagcctgcaacaccccaaaaatcgcctaagtatgaactggtgacgggtacctggaaacaacaggacatcgtgctggcagtagccgttaaattgaataaacagaacattcccgctggcaccagcatcattgcattggcgcccctgctcggacccggcggcgccctgttcacctgcaccgtgaataacacctaccagtttaacggcgacggctcctttgccattgatggctgtaccacgctgatcctgcccgttgccggcaacagcggcacctgggacctggacgtacacgattcggtgttaaaactcatttctgccaaaggagaaaacgatccgcactggattgaaaatatcagcagtaccaacctggatctttccctcacggtaacgatccccggtgtggcgactatccccttaatactaaaattgaagaaataaacgaaccgcggagatatcgcatgctattgttgaaaataacaataatataatcggtaattccttgtatcttgtttagactgatcagatatttgctggcaattatggaaagtattgtacaggatattatcaatgggaatatcggaagttttaagatggtataccaacagtaccacacaaaactttacttctacgttctgaaatgtacacactccgtttacatagcggaagaaactgtgcaacttactttcatactcctctgggaaaagcgggagcgattgtctaccagcttcaatatctccacacagatttttcgtataggcaaaagcgtaatgaccgacctcctgcgcaaacaacaggtgcgtgaccgtcatacgcaaacactggtaagggataacaccaactggcatgtggaaacagatatctccgtaaaagaagaactgaagcgcgtgtataacagtatagaacagctatcccccatccggaaaaatgtttttaaactcagccgctttgaaggtctcccgcataaagaaattgccaggcagttatccatctcccctaaaacagttgaaaaccacattgtacgggctatccgccagttaaagaattccctgctgctactgcttctattgctgatctgttaactaaatgtgacgcagtgagggatttaccgttttcaaacgaatacatactatgaagcattcagtaacacttattgaaaagtttctccgggatgaatgcaatgaagccgagaagcaatgggtaaaagaatacattgcacagcatccggaggctttacaaccttacttaacggaagaaagctggcattccttccagccaggcgagctattgccggaggcggtttccggtaaaatgatgacagtgatcgaagggcatacttttcagaagaagcaggtaaacaggcgctggtatgcagcggcagcagccgttgtgctgattatttccggcggactgttatggacgatattacgcccgttgcccatcaataaaacaatggcggtaaaacccgtgcaaacaaataccgcccctgcagcaacattacgtaccgtaatgaacaacacccgtaaaacaatgccgctgcaactaagcgacggcagtatggtagaactggcccctgaaagcgaggtgaaataccaggagccgttcaccggcaaccgcagggatgtttatttaaaaggacaggccctgttccgtgtaaccggtaacaaagagcagccattcaccgtatatgcaggccagcttggcaccaccgcattgggtacggtattcaaaataacagcgtgggaccggaaagcgatcacacaggtacaactgatcagcggcaaggtagtagtgaaaccggatcatgcagcaggcgtttaccttcgtcccggtcaggcactgcgctacgaccgccagaaaatgctggtaacggtgaatgacgttatcaaaaaagataaaataccttcacgcataaacgaaattattactttcagcaatgaaccgctgaccggcgttttcaggcagatgtctgaaaaataccacgtcagcatccaatatacagccagcagccttacaggcatgaatttcaccggaacattcgacagtagcaaagaaacactaaaagaattcctgacaactattggtacgttaaataatcttactattaatcagaaagatgatgttatctacatagtacaataatcccggaaactaatttcccatacttacaacacaggcaacctctatgaggctgcacggacttccttttgcctaaaacgaacaatattatgtgtgtaaaaatcaaacaatcacgccccaccaccatcatctggctgttgctgttgctctggcaactgatggccggaaacgcgctggcgcaaaacccgcgccctgccgctatcggcctgatcaaaaatgaaagcaatgaaagcctgcccggtgtaatggtgaaaatggagaatgcagaccataaagtattagccaccaccgtcaccaatgaaaaaggcatctttacatttgcaaaactgcctgctggcggcccttatcatttcgtgttatcacaaatgggttataccaccgatacactgcgcggatatatgatcaacgattccagcaaattgtctttatcggtggtcctgaaaaaaaaagtagaagagttaagccaggtgctggtaacggcactgggcattaaaagagaaaagaaagccctcgggtattctgtggaagaactgggcggcaaggaatttaaccgcgtaacacaggaaaacctgctcaactccatgtcgggaaaagtggccggcgttaccatcaactccaccggcaccaccgggtcgtctgtaagcatgatcatacgcggcgctacctccctcagcagcgataaccagccgctgtttgtagtagacggcgtacccgtagccaacacggtgaacaacatcagccagattggtaaagataacatggtggattatggcaatgccatttccgatatcaaccccgataatattgaaagcgttaccatcctgaaaggccccagcgccgccgcattgtatggctcccgcgcggccaacggcgtagtgctcatcactaccaaaacaggcagaaaagttaataaggtaaccgttgatgcatatgtaaactccgtattcgatattccctataaatacctgaactggcaaacgaaattcggctccggtcaattggcaggcattcctttttcccgcagcggcaacctgctcaccaatcccttcggcactatcatccaggaaaatgtggatggcaccttcggcgccgaactggatatgggttatgaagaagtgcagtggaacagtcctctcgatgcaaacggcaaaaaaatacccatgccgctggtgtcgcacaaagataacgtgaagaatttcgtcaacaccggcatcactaccattgccggtgcttctgttgccaacaacaacgataagatctcctatcgcatttcgtatgcgaacatgtcgaacaaaggaattatccctaataccgatctctataaaaatacgctgagcctgaactccggcctgcaggtgaactcaaagctgagcttaagtaccaacattgatttcagccgcaacaactccaacaaccgcgcagccggcgaccgtggcgccaacccgctacaggcggtatacagcgtttccccgcacattgatatacgcgacctggcagactactggatgcccggacaggaaggattacaacaacgcacccaatataacggcgtgttcaataatccttacttcctcgcgtatgaagtaaagaacggatttgtgagagaccggttgtttggtaatatccgggccgactggaaaatactgccgtcccttacttttatggcgcggtatgcactggatacctacggcgaaaaaagagaaaccaaaatttccaacagctacctgaataatcccggtggcgcctacggcatcatcaacctcgataactacgagcggaacatggatgtattgcttacctataaaaaagccattcatcatttcgatgtttccgtttctgccggtggtaatatgcgctaccagacaggcagcaacgttaccacctctacgaaagacggtaccggtcttaatacgcccggcgtatataccattcagaatatttctcctgccaacctcaacttctacagtagcacctttgaaaaaggtgtgaacagtctttatggtatgctgaacataggatacaaaggaatggcgtacctggatgtaaccggccgtaccgattggtccagcaccctccctgatgccgcttcctacttttatccgtcggcctcactgagtgtgctcctgaatgaaatggcgcacatcacctccaccaatatcaatatgatcaaattaagaggcggtgcagcgcaggtaggtaacgacgcttctccttaccagctggtagctactttgggcagtgtaggcgcctgggggaatattccgcagctcaccacgttcggcaccctgctgaatcctttcctgaagccggaaatcgctacgtcgtacgaaggcggtgttgacatcaacctgtttcagaaccgcctgcatttttcaggcacctattatatcgttgaaaacaaaaaccagatcttcagccctaaaacacctccttcttcgggctactcttcccgcagcatcaacgcgggtttgctcaggagcaggggcattgaattaacgctcggcggcacgccggtacaaaccaggaactggagatgggatgtggactttaacttcacccgcaacagaacccgcatcatttccctgccggatgatatgccttactataccctttgggaagaaggaaaaggcggcgcctggacctatgtgggagaagatatcggcgacatctacgatgcgcagctggtaacagttacagacaaatcgtccccatactacggctaccctatattagataacaccggtaaatggcaaagtatagatgccatcaatacaaaaaataagatcggcaattttaacccggattttatcatgggttttcagacgtccatctcctataaaagttttacactgaacatgacgttcgactggcggaatggcggtgactttgtatcgcaaacttaccgttacggagaagaacatggtaactcccagttgttcctcgacaagctcacggatcccggcacgatgaaaggccaggaactgcgcgattacctggttagtcaccaggatcagctggtaatccccaccggcaataacttcccgctggtaggcggtcctacgccggaatacaatagttttccttttacgtatggtccgtatgtgttgccttatggcggcgtatttattccgggcgtaagggcgaagggatacgacagcaacggtaaccctaccggctatcttgaaaatcttggtaacgatggcaccctcacgcttccttatgccggcagtaccgcctggtcgtttacaagggcgtttttattccctgcgtcttacctgaagctgagagaagtgtcgctgacttatgcgctgccgcagcgactgatcagtaccgcgaaattgcaacgtgccagcttctctgtatacagcaggaatattatcctgtggactgccgccaaaatcggcattgatcctgaaaatgcctatcagccttctaccgctgtacagggctcgggtatgcagttcaagcagggtattgaaagatacaatgttactccctgggctatcccggtgggcgcaaaactgaacgtcaccttttaagtgttcctttaattctgatatatgaaaacagtgcgtaaatctattatactcagtatcgggttcctttgtttatctgttacatcctgtaaaaaggacctgatcagcatgaacgaaaatcccaacggcgccaatccggctaccattaatcccaacctggtgttgtctaccgtgctcaccaccacagggtttcagctggtattcctgggctaccaggatatggccggggtgatgcagcacacgcaaaaagatggctggactaccacccacaacgaatacgactggtccgggtccaacagctggacaggatactacgatatgctgcggaacaaccagctggtgtataaccgcggcgtggaactgaacagtgaactgcaccagggcgtggcactggtgatgaagtcgctgctcttcggcctgatcacggacctatggggcgatgcgccttacacctatgccctgcagggagaaaagggcacacccgaaaccacgctcccggtattcgatccgcagcaaactatttacaccgggatactcgctgatcttgaaaaagcaaacactctgctttcaaagcctaaaagcgcctattccaaccctattgatgccgtggatgtgtattaccagggcgacccggcgaaatggcgtaaaatggccaattccctcgcattacggtattatatgcggctgtctgagaagctgccggccatcgcaaaagccggtattgaaaaaatggtagccgatcccgcgcaatatcctcttatcctcagcattgatggcgcagaagatgcgaccatgtcgttccccggcaacagcaatgcggattcctggcctatgaatgtagcctacgacaccgacagcagcaactaccgcaggttgaagatgtgcagcacatttgtgaatgccctgcaatccaggcacgatcccaggttgggcgtatgggccaataaagtgcagtgttttttattggtagatgataccaaaccagccggcaccggcaacgtttataaagccaccgacaccgtgatagcaggagaaccgcggaaggtaagatacatttcacccgacgtgctggcctccaaaggacttactgcgaatgatattaaccaggacgaaaattacgtggggcttcccccggccatttccggcccggcagtatataaccttagtcctgatgccagccaggcatccaggaacccgcatgtttcctggctcaacgacatatacaaacaaccgaaaggaccactgctaaaggcaaggattatctcggcatcagaagttcattttattctggcagaagctgctgccataaaaggatgggcggccggtgacgcggaagcgcattacaacgccggcattcaggcatcgctcaatgtttggggagtagccggcagcactgccgcttatctcgcgcagccttccgtaaaattcaatcatacgcaggaacagatcatcatacagaaatggatcgccagctggaccgccgccaccgaagcctgggcggattataaaagaacaggctacccggtattgcaggccggcccttatgcaaaaggccccgtagtgccggtacgactgtactatatgctggaagaacgcaacctgaataaagcaaatatggaagcagctgccggccggctggaagtaaccacttactcgtcctttggcgccaatggcaccaaaaacagtccgtggtcgaaaccctggatcatccagggtaccggaaaaccctggtaatttcttatatttcatcaacccataaaaaacaattctatctggatatgaagcaactctttttaaatgccgccactgcatttgtactcctgctaagccaggcgaatacttttgcacaacaaaccgtaacacctgccaacgcgctgaaaagctacctggacaacggagatacttcgttcaaatgggaactgaaggattctttcaacgttactaacggcaaaggctataacgtactccttacttcgcagaaatggcgggaatacacctggacgcaccagctcactatttttgtgcccgacgaaattaaatacgacggtgcattgctgtttatcaccggcggctccgtaaaagatggcttgcctaactggaacggccctacggatgaactgtaccagcaaatgggaaaagtagccgccgtgaatcacgcggtaacagccgtattacggcaaacccccaatcagccgctctttggtaaactaacagaagatgcgctgatctcatacacccttcaccagtttaaaaaagatggcgactacaactggccactgctgttcccgatggtaaaaagcgcggtaagggctatggatgtaatccaggaatttgcagataaacaactgaaccgcaaagtgaatggctttgtagtatccggggcgtccaaacgcggctggactacctggcttaccggcgccaacgacaaacgcgtggtagctattgcaccaatggtgattgatgtgctgaatatgccggtgagcctggattaccagatcaaaacctggaaagaatatagtgtgcagatagaagactacgtgaaactgggcatcccccaaacggcgcataccaccgaaggcatggccatcaacaccatgattgacccctactcctaccgcagcagcctgtctattcccaaaatgatattcatgggtaccaatgatgaatactgggtagtagataatatcaaaaattacatagacagtatccctggtaaaaatcttattaactatgtaccaaatgccggtcataacctgggtgataaacagcaggccttccagggactcagcgccttcttcggaatgacgctgagcaaacagccgtaccctgattgcagctggactacccgcacgcacagcggtaaagtacagcttaccgccaaggctacctccgatcgtttactggatgtaatcctgtggtcggccaactcttcagacctggatttccgcaacgacaaatgggaatccaagagcctggggatggcgcatcagtcgaaagtaaaagtaaccaccaccctgccgccaaatggctaccgcgccttttacgtagacctgaaataccagaatgccaccggcggtacctacaccgttagtacacgtgtattcgttaccgatactaaagccattctttgatgaaatcaatgatattactggcagctgcctgctgcctcgccattaactcctttggtcaaacgctgccggctacacgaaataaatttgtggtggtagcgcatcgcggcaaccatgtgagcgtgccggaaaataccgtggcagccatcgaagaaacgatccgctgcggggccgactacgccgagctggatctccgcaccaccaaagacgggcagttgatcctcctgcacaaccccaccgtggataaaatgacgaatggcaccggcaatgtaacggaccttacgctggcggagatccaaaaactgcaggtacgcagtgccgatggaaaagtataccgggtgcctactttcgcagaagcattacaggcatgtaagggcaaactgaacatctacctcgactttaaagccgccgatgttcccgaaacctggagacaactgcaagccgccggcatggaaaaacaggtggtagtatatctcaatgaaaaaaaacaatacaaagcgtggagggaaactgcgccggaagtaccgctgatggccagtttacctgaagaaataaaaacaccggaacagctggaagccttcctgaaaaaaattcgtatagccgtactggataatatcaccgaccctgcgatgctggcggttaccggcaaatacaacaccgcggtgtggctggatgtacagtcgcccgatgaaggccctgccagctggcaggcagctatgggcaaaggaatacagggcgtgcaaacggatcatccggaagcgctgatcacctggctgaagcagtatcaacctacaaaataaaaaagcaggggcgccattcaagcgcccctgtaattatttagtactccgcttccgcgaacgccggttctcccattactttcataaacaactcttcattcagtaaatcctttacggatttaataataaaatcaggcgaataaccaaaatgcgcgaggtcgtcttcatgtgttacgcctgataaggtgagtacggtagtaaagcccatagaacccgcacccaggatatctgttcccatggtatcgcctatcatcaccgtttcatccgtagtgagctgtagtgctttgcgcgccatgcgcatcatcacggggctgggtttccccacactaaaggctttgatgccgctggcaaattccagcatagctaccagtgcgccgcaacctgcgcggtatttaccatcgcccatggggcagttaggatcaagattagtggcgattaatttggcgcccttcatgatcatgttgatcgctttatcaacggattccagcatgatcgttctgccttctcctataatcacataatcaggctgatcatctacaatagaataaccggcattgtaaagttccgtcagtaacccgccttcaccgattacatacgcagtaccgttttcttttttagaagccaggtatcttgcggtagccatggcacaggtaaaaatatctgtgtcatttaccttaaagcccatcttattcagcttgtaacatacatccctgctggttctttggctattgttggtgaggaacaggaaaggaaggcctttatctctgagaccattaataaattctactgcaccgggaataggttcgctgcctttgtagattacgccatccatgtcgattaaaaatcccttttttttcatagcaatcagatgttaatgaactggtttgtgattcaataaatttcatggaatgaataaaggcgggaaacggtatagccgcagcgaagcatccgtagagttggatagcttccccctaaagataataaaataaattaaaaacttttttctttttgtgagaagaacaacggatctattgaataccctgtaaaaataattccaggtgatgattgaaaatctctggttgttccatattgggcatatgcgaagcgtcctttattacaacgagttgcgcatttttgatacgcgcctgcattcctttcgccacctccacgggagtaaacccatcttcttctcccactacaattaataccgggcaatggatatctggcaacatcacggtatggtcccttcgctctgccctgccccgctgcaccagggaggcgcccaacgggtttgtgttcaccatcatatcgcgcaaatgtgctaccacaggcggctttcctgccatcgttgctttaccgaggaattgatgcaggtgctgatctgtataaaactgcattcctttcgccaacagatcctgtgataactgcaaccgcgcctggtaactttgcgcactctcggcctttgcatctgtatctgccagcaccagggcatggcacaaatgcggcgctaaccggtacaattcaaaaagcacctgtccacccatcgatagccccacaaacgtggccttccttatttgcagcgcctccagcaaatgaatgatatccagcgccagttcatccagcaacgtcatcccggaaggcatatcactctccccatatcccctgagatcaggcacaatcaggcgatagccggttttgaatacgccgatctgctgatcccacatgctgcggttaaatggctgcccgtggataaacacgatcgtttccccgctgccgtaatcatcgtatactatattgattccccttacctttaggtgctgcttcataattaatgagaatttagtctcacgaaagtagtacctttatagctgaaatcaaattttaaaactacgcatgggcaaattatcattggacggaggcaggattgcgcaaaaattaaaaacacgggaagccctgatagcagtggccaacacactcctgttacaagggaaagacatcagcgtggaactggtagcaaaagaagccggtatctccaaagctacggcctaccgctatttcaccggaacagaagtattaagaagagaagcctccttacagctgaaagcccaaacaagcgacgacctctttgccaacatccctgaaaaagatctggaagcgcgggtgaataaactgatcgattaccacttcgaactctttacaaaaaatgaaacagaattcaggttattcctcagctctgtgatatcagaatccattcatcccaaaagtggttattccagggccggccggcgtattgtactgatagaagaagcgctcaaaccattgcggaaaacaatggatcccatggccttcaggcacatggtaaatgcgttgagtatatttttcggaatagaatctgttacgatcctgaaagacctgtgtaaactggataatgaagcgatattggaaacctggcgctggtcggtgcaccggattgtttttggatgagattaaacatccccctccggccgcttctctgcggcaattaccagcaaagctacaataagtataaaactatattcgcatcctcccgtgccgtgctcccctacaaaccatcccagggaagcatgtatcaatacaattcccaccagcaacagcacgataaaacccgctgcgagcaatcgtgtatacctgcccagcagcagcaacagtccgcccgcaatttcataggccgtaatagcccatacccatgctacaccaacaggcagccccttactttccatgaactcaccaaaacggggaatggtaccattacagatccgcacaattgcatgtgccaggaatataacggccacagatatacgcagtaggagtaacgattgcttcagggtcaggaaagggaatttttgcatcaggagtggttattatacaaatatagaaaagcggcggccggaaacaatacctgtaaaccggtatttctattgctttgccggagacgccgccgccggccgtttacggataaaaagaaagcccatcaatccgcccataaagcccagccctgccgacaaccgcataatagttccataagcagcaataaaaccatctttataaactttacggatggcctgctgatgcgcaggatcaatatccgcaggcacggatgcattacccaggttcaccgtttgcgcgatcaccgcctgctggtgcgcaccacttagtggcaacgcatggatttcccgctgcaccgctcccgaaaaaaacaatacggccagcgcaccaaaaatagcattggcaaaaacaccggcaatacgggtaacggcattgtttacaccagaggcagtgccggataaatgatcgctcaccgatcccattaccgcagcggttaacggcgccactgtgatagacatgccaagacctaatcccacaatgcccggaaaaaaagtagtccagtaatcggccgctccctgtgtttgttttacaaaagacaacaagagtaacccaccgccggcaatacatggaccagccaccaggaataaacggggaccgtatttatcggccaggctccccgcgaaacgtgcaataatgatcattaatacagtaaagggcaaaaaggtgagccccgactggagttggctgtacccctgcacctgcaccatgttcagcgaaaggaacaacatacccgcaccaagacccgcatacaaaaagaacgtaagcaggttggtaccggtaaaggttaaattcttaaacagctgaaccggtagcataggatgagggcttttgttttccaccacgataaaaacaatcagcaatatgacgccacctgcaatagtgccatatacttccgcgtgacgaaaacccagcaccggcatccgcaggaacccaaaagtgagcagtgccggtcctgccgccgtaagcaccgcgccgggataatcgagccgctgatccccttccgtttccctgctctcgcttaccttcaatgccaggaataccagggccgccacgccaataggcacattgatgaaaaagatataccgccacaaccctgcatctgccagggcgccaccgagtataggtccgcccatagtcaccagcgtggtgatggccgaccaggttccaatagctttccccctttcattttcattaatggaagaagtgatcagggacaggcttccgggaatcatcaatgcaccgccaataccctgtatcatccggaaaatgatgagcagcgtggcagtaccggcaaacccgcacgcggcagatcccaagataaaaataaagatgccggccataaaaactttcttgcggccaagccggtcgcccaacgtgccgcctatcaatatgagagaagccagcatgagcatataggcgtttaatacccagaacagctctgccgcggaggcattcagattgtgttgcagcgcaggcaacactacattcaatgcagtaccatctataaaagccatggcagaagcgagaatcgtggttaccattacccatctgccttcggaactcctgagtgctacggttgtcatgataatcattaacgttcaactgcttaaaatgtttccttcctcatcgatgttcgtttccggacacgccggttacgcaagcggacattttacatgataacaaggatcataacgttatcaatatcaatactcctgatgattggcatatttttcacgctttgactgtcaatcccacacttcctgttatgtttaaaagttacataaaaatagcctggagaaacatgctccgcaacaaggtatatgctgccatcaacgtaattggccttgggcttggcatcagcgcctgcctggtgatatttctcagtgttcactttgaactgagttatgaaaactttcaccccggcaaagaaaatatttaccggattgtatcgcagctcaattcccctgaacgcggcgcccgtaaaatgtcgcgtgtgccggattcagccccggaggctttaaccaacaaatttacaggcgttgaaacgctcgcggctattcatcccatttaccccaaggtagctgtttatggaagcaacggcgtggtgaagaaatttgaaaacggcggcaagcccgacgtgttgattgcttctcctgaatacttcagcatatttcaatatacctggctggccggcaatcctgccaccgctttacaggaaccctttaaggtagtattaaccgccagcaaagcagctaaatacttcggcgagctgcctgttgaaaaatacatggggaaaactgttcactacaacgattctatccctttaacagtagcgggtattgtgaaagacctgccacggaacagtgatttcctcttcaacgattttatttcctttgcttcggtaaagaacagtccgttcgaaaatgaatttgggtttggtcaatggggcatgttcggtggcacacaggcttatgtaaaactaaaccccggcgctgatacagcactgctgaacaggcagctggccgccttcgccagcgaacgggtattagccgaaacaggagaaagcaaagccttccggctgcagccgttggcagatatccatttcaacggcgactatacggatgaattcgggcacaaggcacatctgcctacgatgtacggactcatggccattgcattatttatactgatcattgccgccatcaacttcatcaatctgtctaccgcccaatcagtggagcggtccaaggaaatagggatcaggaaagtactgggcagcaacaaacgaagcctggtggtttatttccttacggaaacattcctccttacggtagctgctgtactgctgtcgcttttagcagtaaaacctttactggatattttcagttcgtttatgcctgatggtgtatcgctgtatttattcagctggcctaccgttgtgttcctgttgctgattacactgttcaccacgctgctatccgggttctatcccgcaaaaatattgtcgtcgttcaagccggtgcaaagtctcaaaggaagcaccggggtaaagggaaaccaacggggatatcttcgtataggcctggtagttttccagtttaccatctccctggtatttattattggttcactggtggtgaataaccagatcaggtatatgctgaacaaggatcttggatttacgaaagatgcgatcatcacctttaacaccaaccgcgcatatgccaaaacccttccacgggtattggcggagaagatccggttactgccgcaggtggaaatggtgagcttaagccagggccctcctgccgacaaaggccattggggcaccgatcttaaatacacgggcaaaaccgagctgcaggcaaattgtcacctggaattcggcgatgaaaactacttgcccctttaccagctgaagctggtagccggcaggaacctgcagccttcagataccatgaaggaagtgctgatcaatgaaacctgcgccaaagcattaggatttaaaaacccggcagatgcggttggtaaatttgtagagcctggcatgagggacgggccatccccgaaaatcatacccgttgttggcgtactggccgattttcataccgttgcactccgtgaccagatcaagcctgttttcgtcacttcttccctggatatctgccggtttgtaaatgtgaagttgtcgctggccggttataccggcgcacaactgcaacacaccattgctgatatacagaaagcatatgcctctgtatatcccaacgagaaattcgattaccatttctttgacgataccatccgcaaattttacgaacgggaacggcagatggaacaactgatgaacaccggtatgaccattgccatcgttatttcctgtcttggtttatttggcctcgccgcctttactgcccgccagcgcaccaaagaaatcggtatccgcaaggtgctgggcgccagtgtggcgaatattgcagcactgctgagcagggacttcctccggtatgttttcattgccgccgtgctggccgctcccattgcctggtatgccatgcacaagtggctgcagggctttgcctacagcgctcctatttcctggtggatatttgtgctggccggcatcattgccatgttcgttgcactggtaacggttagtttccaatcggtaaaagcagcgcttgccaatccggtgaaaagcttaaaagcagaatagtcaaatgatcatttaattatgccggcagatcgaccatctttatttatcttcattgtacgattttcgcaaagatgtcaggcgctagatgaaaaagacgattctaacagtattaatttactgcggcataataggcacaccctggaatgatctgagagcacaggcttccactgaaaatacgcggttgttccgcttttacgaagacaatgacttcattaacctcaatggtaatggaacggaccaggcatataccaatggtacgcggttcgatttgttttataccaggccgcagcctccacgctcctttcccgaccggtggatgcccaaagctggcaaagaaagcatcaatacatatggctggggatttatgcaggtgatgtttacgcccagagacctccggaaggtggtgccggtgccgggcgactttgcctatgccggcggattgtttattacgcatactatccactccactaacccggtccgcaaattcaacctgcaaacggaatggtttgccggtgtaatgggtccctgggcattggcaaaagaaacccaaaccatcgcccatcgcattctcggctttaccaggccacggggatggcgtaaccagatcggtaacaaagtgctcctgaatctcaatctcacggcagagaaacaggtagctgcctataaaaaaatagccgaggtaacagcaggcggtcagctatacgccggtaccatgctgaatggtttcgctgcctactccctgatcaggatcggcaaaatgcttccttactataacgggtatatcacccaatacgccaacaccaagcactggcagctctatgctatcatccggcccggtgtggagctgatgttcaccaacgcgctcgtgaaaggcgtagcgcccgtagaaaacccgggccagccgccgcttccgggtaaccgccctacctatgcgaataataaactgttagccgggatagactgcggactggtagccgtatttggaaaggcgggcttctctctcacccagaaaaccatgtcgccggtgatcaatggaatatcacatcacgaagtaggtaatatttctttctatcttgcctggtaatatttacttcccgctgaaaagcatatctgtgggaagggggacatcttcctgtccttctgttttaatataaatgggctgaagatctacttcattctttttatgaaaaaaattaatccgcaatggataaaaccctttctccaggggtaccataaagctctcgccttctcctgttttgaaatgcccgccaagaatcagccggttatttaaatacaacctggtatggtcattaccggttcccatctcaaaaatataataccccggctcactgattttaatatatccttcctgtaccaatgcgtaattattcttttttgaaactttattaagattaaaatcttttccggcaatacctgtttctaccggcgtcaactttctgaaatcatgtatggtatcccagttgccttcataatatttataccttagtccgcccggcagggctcctgccggcatcatcatcgcagggaacacttcttccacctgaaaaaaaccatttgctgatttgtcgtactcccttcgtttgcctaaagatttaacggtcacttttgaatccctgttgatggtaatggcggtttcttcgcctgttatccggggagaataaataccgggtgtggtaccatcagtagtataacggagatatgcatctgccaccaggttatagcatattaatttaaacggcttgttgcgcaatacgatcccattatccggcttgatggcaattttccgggatgtagggtaacctcctgcagaggcgtagaaaccaccataggaaaatttcagtccctcccaaaagcctttgaagtttgtggaataatgcgtttcattgctatactgcacacatttccaatcgaggccgggaggagcgtttgctttgagaatggaatccatgcccgccacgcccatgaattgataggcagcgccttcgcggcctgccataaaaagcgtattattcatggtgtcgcgccgggcaaatttttccgctgccagttgatgtaaataaaaatgatcccaccacaaactcggatcaatggctacaaaggaagtaaacagatcaggtgcagttaaaaacgtatacattacaaacagtccgcccattgaaccgccatacaaggtatgtccgcctggttttgcgtgataccgcttgccgatatagggcatcagctcattccggaaaaacaacaggaaccggccggcctcccctgaattcgcagacgtttttgtgggtgcaagatccctttcccgcatattcacgccatgttgttcaaagtccgggatacccaccaggatcgtgttcttaggaataaagccttcccattgcaaaaggctccattccacgttcaaaaagtccgggatatcgcccaggcaatatattacctcgtattcaccggaagcagcgggatcgtaatttttcggaagcacgacattcagcggacgcatttctttcaacgtggctgaaaaaagggaatcttttattgtggaaatatgctgcgacctggctttgatgctaaccaggagcaggataaacagcggaattttgacgatggtagataggttcattttacaaggtatcctataaaaataaggtttttctgtcggtgatgaagcccctcctccatccgttaattaaatttgtctttatgtaaagtatactttacatttatatcagaaaaacaagtctccctatgttcacagccacgaaatatttcggcatcgcactggtactcgcaggcatcccttttttctggatgaaccatgcgcaaaccggttctgaactgccgctcatcaccgggttattcctgatctttttcacccgcgaaaaaacagaagatgaaagggcgcaaagcctccgtgccaatgcgctcatgatcagctttgcattgggatacatcattgaagtggcaacaacctatcttcacagcaaaggtgtactcaccttccagctgtctactccccgctactttatcatgctggtactcaccctgggtatcctgatattctacatcaggttgcttttcactggcagctacagcaagtaaggcgatatgaaaaacacaattaaagtgcagcgggccaaacaaaatatcacgcaggcagaactggcggagaaagcaaaagtgtcgaggcaaactattaacgccatagaactgggtaagtttattccatctaccttactggcattgaaaatagcacgcatctttggtactacggtggagcagctgtttatactggaaccgcatgatgaataaagaagcttaaccttccggtaacaatgagtagctattttgtgcattatttattttgccttccactactttatatatcgcgtaccccaatgcgggtgatgaacagcaaatgttcacagacctgttccgtaagcacggggcgaagattttcttctattttaaaaaatatgtaaaacgggaagagatcgccgaagatcttttgcaggaagtatttgccagcctgtggagtaaaagggatcgcctgcaacaggaaaaaaatatcaccgcctatttatttgtaagcgcgcggaaccagctgtacaatcacctcaaactggctgtggccactgctaccactacccttccggaagatacgctgccactgtcatatgaacatgtggaggaagctatccgttacaaagaaacaaaagctacctattacgaagccctttccacccttcccccgcaacgccgcaaagcctttatcctcagccgtgaaaagggattgtcataccaggaaattgccacagaaatgggtatttctccccgcaccgttgaaaaacatgtttcggccacgctccacttattaagagataaaatgaacgatccgtatgtcctctgccttttgttcataatttggtaacactgcggcatacgggtagcggaacaaaattttgtacttgttggtataaagtattgtcaacgtgaatttacaacaagcaaaacacctcgcgcataaagtcctggccaacgaggccaacccggaagagaaggctgctttacagcaatatattcaagacaacgccctcctccccggtttggaagagcagctgtttccattacaggaactcatgtctgcaccggatagcgcattacctgctggtatggaagaaaggatcctgaccccgttaaccggtggaaacgctcccgcaattcccgcacgccggcctgtacttcgccaactgctgcgcatcagcgcagccgctgctgttgtgctcatagtatgcctgggcgcctatcgtctcctccatactgatcgcacaccggatacaacgctccaaacgctggttacgcccaatggcagccagggtaatattacactggcagatggtacacagatccggctcaatggcggaaccacactgcgttacccatcttcctttaccggtaaaacccgggaaatatacctcgatggcgaagccttctttgaagtaagcaaagattccagtcacccgtttattatccacgcacctgcttttacaactaccgtactgggtacctcttttaatatcaaatcggctgccgggcagcaattatccgaagtagccgtggccaccggtaaagttcgtgtagccgccaccgttgcaggaacggcagattcggtcgcttacctcacaccgggcgaagttgtttattaccaccccaatgatccggcagggatacataaaggcagcatagcacttaatacgatcggagcctggaaagaccggcgcttccattacgatcaaacaccgctgcacagcatccttcacgacatggaaagtgcgtacggactgcatttccgggtagtaaaccccgctgtattgtcctgtaccttcagcgccacttttaataacatgacggcaacggaaatcctccagacactggcactcatgagccaggtgaaattccagataaaagacagcctgaccgaagtctctggtcagtcctgcaactaataaaaaaaccgccctgtttgcggcagggcggcgagtccatcataaaattatcatgaacatcaaaatcaatttcaaaagtatgtattttatcagagagtttttgtcacttctaaaaaacaggatactactgcaaaaagcaggcgcagtatggttgctatgctttatctgtttttccggttacagccagcaacctattaaaacacctgttaccattattgccagcaacaaaacattaaaggagatctttaaagaattagaacaaaaaacaggatacaccattaacttccaggacaatgtgatcaatgccctgcaaaaagtatcgattgaagcccgccagaaaccactggacgtagttttacaacaattattacagggctccggagcaaacttccggcaacagggtaatatgatcctcctgtttaaacaaccggcagaaagcagtccgcaaaaaaaaatacccggcaaattaaccggcaaaatcatcgatgaggaaaatggtcagcctgttgttggcgctactatccgggtaggcaacacgggcaccaccagtaatgccgagggtgctttcagccttacgttgccccccgggaattatgttgccacagtaagtttcatcggatacggaacaaaagaaatcaataaaattgaactgaaagataatcaaccctttcttttaaatctcaccttaaaaagagcaaaaggtcagctggcgggtattgtggtaaaatcaagcgccggtaaggaaagtactgcctccttttataccaggcagaaaaatgccgcgaccgtaacagacggaatctcttttgaacaactcaacaaactcccggataacaatgtgggcgcagccctgaaaaggatcagcggcgtatcggtggttgacaataagtatgtagtggtgcgcggcatgacagaacggtacaaccaggccatgctcgacggtatgatactccccagcactgatgccaataaaaggaactttgccttcgaccttatccctaatgaaatggtaggcgaaatactggttaacaaaaccgctacgcctgatgccagcgccgaatttgtaggtggccaggtgatggtgaaaacactggacataccttcccggaatttcaccgtcatcagcattggcgaaagcatcaatacccaaacaaccggtaaagatttttatagcctgggcaaaaggcaaacaggcgactatttcgcagtggaaaacggccagcgtaccatccccggcaataccgtttcctggtcgctctacaatcaacaggaagatccaacaaaaatagttaccgacgccaacgggtataaatatggatttgaaggcgccatagaccaaagtaaacggtttaaccccgatggcttccggctctatcaaaccaccgcctatccgaatctcaatttcaaatacattatgggcagggtatatcaactggataccgcggccaacaggaagatcgggttcaccggcggtatcacttaccgtaaccggaatcaaacagatgaattcagcactacccgcggactcgatctttcacgcgactacttcgttacagacaccgcaggaaaagggaaaatatatagtttcagtacaattgccactgccttattgaatgttggctatagcacccggaaaaacaaaatcacattgcggaacctccatagccggagttttgcggaagactattaccgctcgctggagttcacggatgattttagtcacggccggcaacggacttccctggtgatgccggtgtccacctccatacaacaacataaactggaaggcgaacaccgtatcacccgcggtgggctcaccctcaactggatggctggctatgccgccatgaaccaggtgtataatgatgtgcgcagcttccagtatggccctgccaataaaacctttggtgatatctaccaggccagcaatccctccagcaatgcggctacacaggcaagctggtcgtggccttaccggctgtggtccaatgtggaacaaaaagattatacctggggtatggatatcagtcagcctttccaattcctccgtggtaccagcatcgtgaaagccgggtacaatggctgggacaaaaaacgccgccagtcgatggatatctttaaaatatataccgcctatcgcggcctggacgttgaattcctgccttatcatatccagatggacgcagatcatgtaggcgtgggaaaaggacagacctattattggggagatctggaaaatggcgaccaggcagcgtcaggctcccaataccacgcgatatacgctatgctggatcagcgcatgtttcaaaaactgcgattggtgtatggtctgagagcagaaaatttcggactggcaaatcagcaacttgctgaactcagaaggatagcacaatttaaaaaagagcatcccgatcttgcctataacggcacactgcccgtgctcaccggcgaaaaaaactggaacttccttcccgctgccaatctcacttacagcattaccagtaaaataaacctgagagcagcttacagcaaaacaatgattcgccccaccttccgcgaaacatccgttacgtctttccccgacccggctatgaacgcgcttatcagcgggggtaatatcagcagcaccaaaatagataataaagacctgcgcttcgaatggtatccgaaacccggtgatatgttgtctgtttctgccttccataaaaaactggataaacccgtggaactggtggtgaattcactcaacagcacccccatcggcatggcttatcaaaaccagcattcagccaccagcaaagggctggaaatggaattcagaaagaacctggcctttatttccgggctgctgaaaaacatgaccatctatggtaacggcgcctggtttgcctcgaaagtaaatacgatcaaccgggtaaatgatccggccactcccggaaaaaaaatagagctactgaaggaactcgaccggccactgatgggccaatccccctatctggtaaatcttggattactatatgaagaagacggctttagcggtaacatcgtttttaaccgcactggctaccgtcccaactttgcggtagatgggcagccaggcgcttcagaattccgcgccgcctatagccagctggatttgcaattctccaaaaaattattccacaacaaagcggagttcaaactaaacattaccaacctgctcaaccaggaagaattttactatcgtaatatcaaaggttatgaaacaggttttatcaatggtaaataccagatcattaaattgaagtactatgttccggccgacagctacttcccgccagccaacggaaatcccgactatcgctatagtgattttgtaaagttaaaagacaactacagcgcaaaacaaggcgatcagaaaacttacagcatcaaaagagggatcaacatgaacctgtctttctcttataatttttaatatcatctgccatgaaacaattccttcattttactttagtgatgatcattttattgaccagcaacacttcctgcaaaaaggaaacagcggcagatgattttatcgtattcggacagctgaagataaataacgctacctcctatagcgcactccgcttcggactggaaggctaccccaaacaaatacaatcaactgacttcatgaagctggaaccaggcgccaataagctgcagatatggggaattacagaagacccggcggataaacctgtttttcttttcgatagcctcctgcaggtagaagccacacaaacctacgagttcaccctgtttcagccggatgaagttaccactcccattgcgttagtcaatacccaggcagctgaatccaaacctcctgcaggttttatgaaaataaaagccgccaattttgctacccattgctttccccgtgaagtagacctgcaactgttaatgatggacttcagcctgggcgacataacaaatgtagacaccatcccgcagttaaaagctgcatttgactcctatgggttatatcaaacactggatgccgtcaatactgatggatatacgatcttctatattctggaccccgttacgcatgaacggttacatcctgatttcattttcggtattgatctcatgaattacactaccggcaaactttatgaggtagttactctttttatctatgaaaaacagaacaacgcgggatctttcaccggcacagacggcaataaatatgacgtcgctgtaaaggccctgtacctcgactaatcaccgttgctgcgaagccctgcccgtaccgggcagggcttcaatatcattttattaaccttccttaacattaatgcaaggcttgttaacctgcttttgccacacccggacctactttcggtaacaaagtaaacgtccgctatgcaaaaatattacctgtggcttcttatctcctgtttatcccttgccgccaacgcacaaaggaatggtgttatcaaaggcactgtgtctgataccagtgccggccgtccagtggcatcagccactatcaccctgctgcagaaaaaagactcctcactggtttcctttaccatgactaacgacaaaggatattttgaaatcaacggcatacacgccggcgaataccggctgctcatcacgcatgtaaaataccactctctccagcgcatggtaacgatcagcaacgcaacgcccgtgatgaacttccctgctcttgtgcttcacgacctcagtatccagctcaatgaagtagccgtaaccggagaagcgccaccggtaacactcgtaggcgacactatccagtataatgcgggctcttttaaaacaccgcccaattccagcgtagaacaattgctgaaaaaactgccgggcgtagaggtggcaaaagacggcaccgtaaaagcacagggccagaaagtaaaccgcgtgatggttgacgggaaagagttttttggcaaagaccccaaaatggcaactaaaaatctccctgccgatgcagtcgacaaagtacaggtatacgaccgcctcagcgatgcggcacaactcaccggctttgatgatggcaacagcgaaaaaaccattaacctgaaactcaaacaggataaaaagaaaggcatgtttggaaaagccatggccggtgccggtaccagcgaccggtacgaagggcgctttaacctcaacgcctttaaaggagcacgacaactttccgttatcggcatggccaacaacaccaatgcagaaggcttctcctttatggatatgatgagcttcagcggagaactgaaccgcatgcggcaaagcggcagcggcaacgccagtttcaccatgagcgccgacgaccccgccgccgcattcatgggcggcagcagcggcaacggcattaaaaccgtatggggcggcgggatcaattataataacatcatcggaaaaaaaacagaatttaccagcagctacttttataaccgctataatccttaccaggaaagcgaaatacaacgccagtatttcctgccggactcctcttatttctacaaccagcacgctgccagcaacaacatcaataatacccaccgcctcgacctgggcgccgatatccagatcgactccctgcactcggttaaaatatcatcgtcttttggttaccaggaaaaccgcagcaaaagctacagcaaatatgaaaccctttcggaagaccagcagctggccaatgaaggcttcagcaataactactccgcaggtcatggctccaatttcagcaatgatgtattgttccgtaaaaaattcctgcgcaaaggccgcacattttcactcaatctgcaaaacagtaccaataacagcgaaagcaacggcagcctgctttccgtaaatcatttttataaccgccccgcctcgcagcccggttacgattccatccaccagcgcaataccatatccggagatatgaacagctataacgcccgcgccgtatatacggaaccgttattcaaacactcactggtggagttcagtatcggcaacagctatacgaaaactacttccgataaaatcacttatgattacaacggcgataacgggaagttcgaccagccaaatcccgcgctgacaaacaacttcgaaaatgcctatagctataccaatgcaggtatccgtctgcgtacaaaacaaaaaaaatacagtctcgctgcgggcctcaactggcagtatgcttcgctgaaaggcaccattatcgccggcaccaaagactccgtgatccgccaaacgttttataacctgttaccatcgctgcgtttccaatacgactttacccgttaccggaacctcagcatcaactacgcagccattaccaaccagcccgatatgtcgcagctgcaaccggtgccggacatcagcgatcccctcaatatccgcgaaggcaaccccgatctgaagccggagttaacgcacaccgtacagctcaacttcatttcggtaaaccccttcaaaaataaaaacctgttcgctttcttcaacatccaggaaacgcagaacaagattgtgaatgatgatgtggtggatagtcttggtattaaatacagccggccagtgaatgtaaacggtgttttcaacatgaccggcagcatcaacctgggcctgcccctgcgggccctgaaaggcacggttaacttcagcagcaacgtgggttacagcaaaacaaaacagtttatcaacaaggtatccaacggtatcagtacggttacgctggggccttctgtacgttttgacctgaacccttcggataagctgaacctcacgtttggcgggggtattaattactacaaaacagcttactccctgcagcctgccctcaacaccggctattttctgcaacaatatgacggagaagtaaactggcagctgcctgcaaatttttacgtgagtaccagttttaactatactattaacagccgccgcacagatggatttaatgcaaaggtgccgttatggaatgcgtctgtcagccgccagttccttcgctttaaccgcggggagctgaagctgagtgtatttgatatcctgaatgaaaatgtgggtattaaccgcagcaccaaccagaattatattgaagacagccgcacgaaaaacctgcaacgctttttcctgttgagcttcacttacagtcttagtaagaatggcattttcaatgctgcagcgccggggatcaggatgatccggcgttaaaaagtaaggggcataagaaaggggccggatgatatcatccggcccctttcttatggcagttatttactgtgctatcctgatactgcgtgtggcgccgccgccattgcgctgcatttcgttcatcagcttctcccgtgctttattaaactcctcttccgttacctttttccctttggaaggctcccggatggcggcaagatctgcctgcggcgatacttccagcgcctggtaaacggtagcgccgttgttgatgtcaacagccaggataagcccgggaagctgtccctggaagtccggcccggcaggcaccgggatagccaatgtaaaccaggcggtgatattggccgtatcggccacctctttggttttcatctgcccgttttccatggaggtcatggaacgcttgccgatacgctgcgttacagcctgctggcagggataattaagtatagtacgggtttcgcccgtgatcttccagttgagccgttggatactgtccgtaataaggtagttctttgcagcaaactcacgttgttctactacgcggtcgttggagaaactggtataggtcacgtcgttgtcgccggccaccatcatgcggatatgcataccaccttccccggcgaattcttcgggagcatcttcctccacggcgcggcgcagcgactgcccattgccaaacaatacttcgagcttatctttcctggaatgcggcagtatgttatcaggttccggccctgcgtctgcaccagcagccattcccatcatccgcatctgcatctgtacggtgcgctcgtagagcacgcgcccctgctgttgctggccgctggcggttaacaggcatccactgatggctaacgtaaaaattatcttcttcatgttacatacatttaagaaaataaagctatttccttcccgccggaacagaggttaacatcacttgatttaatgttaatttaggttaatgtttccgcgttgggaagcaggaaatgatacatttgcggtagtattgttatttcttaccattcaatcaacatagtgcgatataaactttccataccggctaccatttccctgattgcgctgaccatcctgctgatcaccgctttccaggcatactggctgagcaataactaccgggaggaaaaaagattgtttaccgcccgcaccaatattcttttccgggaaaccatttttcgcctgcaggccgtaaagctcaacctggattccaatatcagcctgcgggtacatgaccgtgcgggtatgacgggtgtcaccaatgtgttgcaggaaagaatgagagattctaccatgagcgctcctgccatgcccatcagaaagcggacgatgtttgtggcggtagatcctgcatcgatgccggaagatgattccgtgaatgtacaatacggcgttaccaaaggagttcccgctacaacggtattccagttcctggccggtgtagattccctcagggattctattaccgtaaaagaagtggtggaccggtaccaacgggcgctggaacgggaaaagattaacgtttcctttactgttaataccattcccgtagatactactaccaatcatatgttcaataccttcccggatgacctggaaggtaatacggtgaccatcggttttaccaaacccatgagctaccaggttttatttgaaaacaatacctggtacctgctgaaacgcatcagtcaaccgatactgatatccttctttctcctggctgttaccatcttctctttcctgctgctttaccgcaacctgaaacaacaacaacggctggcacaactcaaaaatgattttatcagcaacatgacgcatgagctgaaaacgcctatcgccactgttagtgtggccattgaagcgctgagaaattttgatgcactggaagatctgcaaacaacactcgaatacctcgatatatcggccaatgaaatgaaccgcctggcgctgctggtagataaagtgctgaaactctcgatgtttgaaaacagggaaattcctttgaacaaagaacccttcgatcttacagatctcacccggagcgtaatgatttccatgaagctgcagtttgaaaaacaacgcgcagttaccacgctgaaaagaacaggtcataactttaccatcacggccgataaactgcatatgaccagcgtattgtacaacctgctggataatgcattaaagtacagtagccaggaccctaatatcctgatccatatcattgatcacaaacaatacctggaactacgtgtaaccgacaacggtataggcattgcgcgtgaatataaaaacaagatctttgagaaatttttccgcgtacccagtggcaaccggcataatataaaaggatatggactgggcctcagttatgtatctcacattgtacaatcgcacatgggctttattgaagtggaaagtgaactgcataaaggcagtacgttttccatcaagcttcccttcgcagaagcgccggtcattcattacgacaaaaaccgccgggtgataaagcttaaaacaggatgaaatgagtattaaaattttatatatcgaagatgaactgtcgctgggcaaaatagtgaaagaaagtttacagcgacggggatacgaagtaatactggaaagcgatggcgcccatgtaatgcaattgttcaaacaggtaaaccctgctgtatgcgtgctggatatcatgttgcccaataaagacggatttgaaattgccgccgaaatacgcgctatcaaccaggaagtacccatcctgttcctcaccgccaaaacacaaaccaacgacctcgtaaaaggatttacgctgggaggcaacgattatatccgcaagcctttcagtatggaagaactgattgtacgcattgaaaacgtattgcgtaaatcagataaaacacctgctcctgctgccaatcacatcaaaatcggcaagttccggttttatactaaccgccaggtactggccaacgacgtagaagaaaaaaagctgtcgtacaaggaaagcgaactactcaaactactatacgaaaaccgcgacggcatcatcgaccggaaaaatatccttgacctgctctggggacatgattcctttttcaacagccgcaacctggatgtatatattacccggctgcgcgtacacctgaaagaggatgacaacctgcagatcctcaccattaaaggtgtaggataccggtttgtgctgggttgatttttttattgcagatgatcgtcgtgtgcttctttaaaaatatccgcataaaaaagcccgcaggcattgcaccggcgggcttcttcattaattaatcttatgaatgctcaggttatcatagtaaatataacctacggtagatgattcccagtaagactggctgccaccgcggaacgtatgaaaagttacgcccctgatcagccgtttgctgtcgttggtggtccaccggatatcccggtcgagcagcacggtgccgttgatcacgatctgaacgtgaccatcggtattactgccggtgttgctttttatgtacaggtgtacgtgataagtagtgcctttctggatgctgccgctggcagggtaagtgagcccgaagtcgtcgccgtactggcccggctggtccctgtaatacaggtagggctggaagtacaccctgttggcgtcgttacggtaccacatgagccggagggtgccgccattaccatcccaggcgggatcgccgccggtgttgccatcaccaatagaaaagccgaagcctattttaccgccacggctccagtcgaactggctgtgaaaacggatatcataatccatttcataagcggcgccgtcagatacatcgatgttggccactaccccgccggctgcggagagtgcgttgggatccagctggatgcggaggttgccattggaaatgtagccgcggttgttgttccagccggttacattgccaaaatcactggcagcattggtagatgtgtaggtagtgccattggcgtaattatcccagttaacagaccaggtgctgttaatggcgttaattcctatagcagcatcggcggcagccagggttgtgttgtggggcaggtttgattgcgccagttccttcttacaggaaataaaactgacactgaataacagcagtccggctgctgcaacattacgtgagaaaacagtggaattcatgaatgtgtaattgtgggtgagaaaataggtttatcatcaggagggtttactgtataatgattttcttcacgagccgttgattgtcgtgcatcacttccaggatatacgtgccgccggcgatggcgccggtatttacattgaaggtcttagcattgggttgctgtactgccacgggctgcatgcccgcgctgatcagggtagcctttacaggcgcttttgggttgtagtgttgcagggtaacggtgaatgcactgcccgaacggatgggattgggatatacatggatagcagcagcggcagcttcttccgggatggccccatgcgtggcagcaacggcagcggtggtgctgctgatggctgccagtccgctcaccgctccataattgaacgattcccacgtaccaaccgtagttctccaggagctcattgcctgcgtgccattttccgagcagatatagccgccattgttgcacaacagtgaaatggtgccgttgctgttattgatccaggtgaatttttcccagtcctggatactggtacggttacacgtaatggcctgcgtgccgttttcggatgatacatacttgccctggctgcgtaaagcaattttgccgccgccggcatccactacggtaaactgttcccagccctgtgcgctggtacggttgcagttcattgcctgggtgccattctcgccgctcacatacaggttgttgttgccgcgcagccatatcgtttgcccaacaggcgcattgccgcccgggttgccggtacggctaagtactacctcatgaatggccgacagcaacgaattggctcctgtggcgtcctgcgacaactcccagatcatcacaccgctgccctggtcaaaagccaggttcgttttttgtttgatggtagtaatgccgttgtagccaacattatcaaatacatcggcataaggattggcgccacgcgccaccagctgggcgtacgactcccaggttggccttccgtaaaaaggcacgccaagcacggttttggaagctgggagtccgcggccgcgccagtagttcaccgactgggtagcataactgtaagtagagtggtcgaagttattgtagtcgtaagccatgaggttataaaaatctaccaacgcaaaagcgctgtttaagatactggccccgccggtacccacaatagcgccggtaaggagtttacccctgttatgcatctctgtgctgagctgcgtcatcagcgtaatatagttattggccgatgcgccggcatcgggatactcccagtcgatatccacgccatcaagaccatactggttcacgaaattgatcatgttggtcacgaaattattgcggtaggtactgttggcggcgagcgattcaaagccgctgtcgttcccatcattccagccgcccacagatatcagcacctttacattattggcatgcgcagtgctcaccaggctctgtaacttcgcggggttatcgattgcctgcaaaccgccggtactggtaggcaacaggaatgcgtaattgatatgagtaagcttactatactgcacctggtttacattacctgcccaggaaggcatatatccaataacgcggaaaggggtttgagcaatggtattaaacgcacaaacaaggaggatagctaacagctttagaaatggtttcatacgggtagttttttggttgaaaagaaatgtggattaatcctttcaaaagtaggggttcgcataaaaaaaccatcatccggcactacggcattactacgtcacagggatatttttttatatttcgcgggtaatcagtaacggaagaagaagttgcttatcttttcattctaaataatacccgtgataagccatataaagaaagcgctgcttcccctgttcatcctgcccgccttcctctgccaggcacaggacaaccgcatccctgccctgcctccggcgcttgaaatacaagtacaccacgttcccaaaccggtagtaaccggcggacatcctgtactcttctacgaaattcatcttaccaacttctctccctggcccctgctgctcacaaaagtggaagcacaggatgcgaagaataccactgctttgacgctgataaaagacaccagcctgttgcaacggctggctgcaccgggacaaaaatcccccaccgccaccataccgcccggtaatgtggcggtgctgtttgtggaatattccgctgccgccgctcaattccctgctgaaattattcaccaggtatctttcaaaaatacccttcgtgatacggccacggaatataccatcacgggcgcggccatacaactggtaaccagtccggcaattgtattgggcgccccgctgaaaggaggcccgtggaccgccgtttacagcccggtatgggcacaggggcaccgtcgcgtaatatttgtaaaggatggggtagcacgtatccccggaagatttgccgtcgactttgtaaagctcgacagcaccggtaaattcgccggcggcgatgacgacaggatcaccaactggtacggctatggcgccggcatactggcagtggcagatggcgtggttagttccaccagaaccgatttcccggaaagcaccgcattatctaatcacccggattatgccgcccacctggccacgggcaattatatctctttaaaaatagcagaaaatacctacgtgttttatgaacacctgcagccggaaagtatcgtggtaaaagcaggccagcgggtaaagaaaggagacgtgatcgcccggctgggattcacaggtcagtccaccgggccgcaccttcacctgcatgtggcgaacgccgatgcgccactgggcgcagaaggacttccctttgtatttgaaaaatttacgctgacgggtactatccccgacttcaacaaatttggcagcgcgccgtatattccgcaatcacaacccgtacgccgtgagctgcccgtttccaatagcgtcatcacatttccgtgatactatttacggtattccctgggcgtaattccctctgcccgtttaaacaatttaataaagtaattcaggttattaaaccccgattggtaacacacatccgtgatactcaatgcaggatccgccatgatctgctttgcgcgccggatgcgctcctgcaaaatatactccagcggtgaaataccatattgctctttaaatgcctggaaaaaaacggaacggctcatgcaggatacttttgccaacgcatcaatagtaatcttttgggtaagatgctccctgatatattgcaacaccggtgtaaaccggtgattacctactcctgcatcattaatggccaccaggttttgtgtttgtataatacgcagtaataaaaatttcagcgagagatctgccagtgcatcctttgcaggatcactctccatgctgatcccgatcagtttattcatactggccgccagctctttgttatttaaaaagtgataccggctgaaattcagctgccattcaaacggcgccgccttattgggatactgctcattcagaaaagccaggttcttattcaccatatcccagtcgagcgccagggtggcgcactgcaccggatgcctttcatccgcctccggaaaatctactttcatagacacgccttccggcaggatcacactttctcccggcaaaaaaaagaactcttccgatccggacaacgacatgatctttttaccccgcatcatactggatactaccagcccgttataagagagtgccacattactgcagcggtgaaaagtttcaaagatgttcagctcacagtgccgcaggttaaacacccggcggtgctctaccatcgtatccagcgaagtggcatcactcaggttaataggagaaagatggcatatctggttcatggtggaatttttatcgtaacgcaggttttccgccttataaatttatcgataaattcccgttggatcatcaaagaaataaaaaaatagcatcgttctatcaatcaggataatcgttcaattcccccatctccaatatgcttaatattggttattccttcacattaaaatcctgttatgaatatcacgttaaaacaggcggaagctgttattgctgccgctaaagccaaagccaccgaaattaaaacactgatgaacattgcagtcgtggatgcaggtaccaaccttatcgcctttgttcacatggacgacgcctggctggggtctatagatatttcgcagaaaaaagcccgcacggcacgatacttcaatatgcccaccggcgaaatcggcaagctgtcgcaaccaggcggctccttgtataatattgaacattccaatggtggcctcatcaccttccccggcggcgtggtcatccgcaatgaaaaaaatgagatcatcggcgccgtaggcgtatccggcgactccgtggaaaacgatcatatagtggcgcaggcaggcgcagatgcgattaaataacttctaaaaagatatggtatgtgtaaaaatcatggtgttgcttatatagaacccggtgtggtggaagtaagggaaattgattatcccaaactggctttgggcgaccgtaaatgtgaacatggggtgatcctgaaaattgtgtccaccaatatctgcggaagcgatcagcacatggtgcggggacgtaccaccgctcctgccggactggtactgggacatgaaattaccggcctcgtcattgaagctggcagggatgtggaatttatcaaagtaggcgacctcgtttcggtgcctttcaatattgcctgcggacgttgccgcaactgcaaagcagggcaaacaggcatctgcctgaatgtaaatcctgcccgccccggcgcagcctatggctacgtggatatgggcggctgggtaggcggacaggcagaatacgtaatggtgccgtacgccgattttaacctgcttaaattccccgacagcgaccaggccatggaaaagatccgggacctcacgctgctcacggatattttccccactggttttcatggcgcggtgaccgcaggcgtaggaccaggcagtatcgtttatatcgctggtgcaggtcccgtaggactggcatgcgccgcctcctgccacctgcttggagcggcggtagtaattgtgggagatatgatcgatgaacggctggcacaagccaggagctttggctgcgaaaccatcgacctgaaacaggaggcctccctcgccgaccagattgccgccatcaccggcacgccggaagtggattcagctgtggactgcgtaggctttgaagccaagggacatgggcacaacagcaacgtggaacaaccggccaccgtgctgaattcaattatggaaattacccgtgcaggcgggcaactgggcatacctggcctgtatgttaccggcgatcccggcgcggtagacgaggccgccaagaaaggaagcctgagcatccgcatcggcctcggctgggcaaaatcgcactccattcataccggtcagtgccccgtcatgaaataccaccgtcagctgatgaacgccatcctgtacgataaaataaaaatagccgatgccgtaaatgtagaagtgatcacccttaacgactcggtaagaggctaccacgattttgataaaggcgcagcgaaaaaatttgtgattgatccgcatggcatgataagggcataataaacgggaactaaaacaacaatggctgccagtaatggcggccattgttgttttagttcccaaccgccaacgatttgtatattcacggaaacctgtttatattcatctcctttaccaaaacccagcccggtatgcgtttccgccttttgtttttcctgctgatgtattgcgctgtatcgcaaagccaacctactcaacccgccgattatggattgcaggctttcaccattcacgataactcccttggaaccattcgtttttatgtgagcagtaaagatattggcaaaaagaaaccggttttactggcgctggatggctccggtcagtacccgatggcgttattcgtgcagctccggaaaggctccttcgtcgctaattcatttgatcaagggttgctggaactggcagataaatttcacgtggtaatgatcagcaaacccggcatcaatttctgtgatacaatcaatatagataaggacagcgccagtgtggcagatgcggttgcactattgcccccttcaacggaataccggcagcgggccggctttcaatggcgcatagcagcggcttccagggtgctcgactatgtatacagtcacttccccgtgaataaatcaaaagtggtagcttatggctactccgaaggtgcacaggtagtaccgggactgtcggtggcgaataaaaaaattacgcattgcgcctgcatcgccggatcaggtcttaaccagttctatgattttataaccgctgtgcgcatgaaagccgcccagggggccatttccccacaggaagcacagcaacaggtggattcgctgtttgcgcaattcgctgccatttacgccgctcctcatgatacccaacgcgaatgggaaggtcattcctatcagcgctgggccagcttctgttcagacattccaatggacaacctcacaaaactgaacattcccatttttatgacggcaggtaccaatgatgccagctcgcccatttacggattggaatatgtaaagctggagttcctgcggctgggcaaaaagaaccttacattccgggtgtatcccaccgatcactctttccaggaaatgaaacgggttaacggaaaagacaccgtcatttcccacaagcaggaaatgacggcagatatgatgaaatggctgaaaatgtaatgacttagtgcatcggtgtgctgctcaggtctttgctgttgatcacgtccagcagctccggatgttctttcttttccctgctcagcaccttatggataataacgatactgattaatatacaaacagcgccgatcaggaaatgtacgcccggcaaatggaacggcgctttcgaggaggtgaaataagcaaaggtgctgttcatgatcagcggaccaatgatagtggtaaggctcatcaaactggtaagcgctccttgcagttctccctgctggttagccggcacatgacccgatatcaccgactgcagcgacggtccgcagatcccacccaaacaataagggatcaggaatacaaacatcatccatccctgtgtggcaaagccaaacaataccaatcccactgcataaagcgccagcccgagataaatacttttttcattaccgatttttgggttcaccaccctggttaatccgccctgtaccgctcctaccaatactcccactactgcgagggaaatacccaccattttctcactccagttaaaattataaatggtaaagaaattccagttgctctgcactgcctgggcgcccaggtaaataagaaagaagccgaatgccagtccgccgatttccggatgcctggttaaaaatttcagcgacccgaacggattagcccttttccattcaaaagaccggcggttttccttacttaaagattccggcaggaaaaagtatccccatatacagttaaccaaacacaatacagcagcggcataaaaaggcgcacggatgccccagttggccagcaatgcgcccagcgccggaccaagcacaaatcccagtccgaaagccgcaccaatcagcccgaagtttttagccctcgaagtttcatccgtgcttacatctgcaatgtaagcagcagcggtagtaaagctggcgcctgtaatacctgcaataacgcgtcctgcaaataaccatccatatgcaggcgccaatgccaggataatataatcgatcccaaaacctaacagggaaagtaataataccggccggcggccgtatttatcactcaggttcccgatcaccggggaaaataaaaactgcgtgatcgcaaaaacggataacagcaacgcgccataagtactggcttcgttaacggggatgtgttttaactgcgcaatgagatctgccatcacgggaataatcaatccccaccccattacgtcaattaatagtgtaacaaaaataaagctgatagctgcctttctggatgtgtgcatattggtgtttttgtaaagtatctttcagatctttggcggatgttttctccttctcacaacgggtatccctgattcggtttcaaatataggatgcactgtttttttatggaaaacctttccggtcaggatcatcgttccaccggtaaaacgcctggttttaccggtgaaaacctcagggcacaaagatatttacttcattgtcaaatgagcgggcaaaataagacaataaaagggcagtttgcgacagatataaatgttaccacgttagttggagcaacgatacaccttgtccgggtaaatcatttggcagcactatttcaccgttctccggctgcatccatgcgggcgacgacagcaactgtaactgcccggcactttccagctgcgctatttgcgaagcatcaggatgctgaggtgatcccatatttttccaagcttcgtaggcgttgctatgcgcagtatcaatccggtaatgcttcagtaatacacgggtagccggcagtccttttatttttatttttacgggagatgattgtgccggaataatgttgtcgtcatgatagttccacaccattacgctcacgctgcgctcatcaccggatgctaatgcattaatatcacgcctggctccccgcacgctgctgtcgaggatctgctggtagttatagttcgtggacccacttacctccagcctgttgccctgcatcaggccaaacatccggaatacatttaaaacgggtttgtccaccccgttggtggccaggtcgcggaaacccgcaaaccagggctggtcctcaaactcaaaggcccaggtcactgcgcctgccaggtttacaccacgggcagccgccaggtcgtacttccgcgcaaacgatgcggcggtataactcgaatacatggtgccgttacggtaagcattggcaggatgaaatgcttctgaacatgcggcacatccttcaggatctgattcaccgataatgatgggcagcttcttcagtgacggataggaagctactatttcaaagcctttatcaatatcacgcagctgtgcggccatgttcatctgtaccacgccgttcaccactttgggcgcacctttggcgtgaaaggtgatcacatccagcggcgcgccggttttgccggtggcgtagtttttaccactcaccacatgatccaggaaggttttaaaaaacttggcagatacatcccagttggggcctgttacttcagggccgccgatcctggcagtgggcaatgcgcgtttcacggcgtcggcagtgtaatcatacagcttgatgtattcttctgtagtacctttccaatagccgatattaggctcgttccataattcccagtaccagctttccacttccgcttttccataacgcgctacagaatgctttacccattcatataccagcgccgcaaatttctggtagtctttcggaggatacgcccagccggtaaatatatcgccatacttattatccggctgccagtgatggcggtaaggcgagggctttaccgacagcgcctccggcataaacccgatctgcgcaatcggcttcatgccccgttctataaaagtatcaaagatcttgtcgatgatcgtccagctgtacacaggattcccggcggcatcttcggtgtatgcattggtggaaccccatttcagcgcagccgtgccatcgccggttaccagcaggctatgtacccgtacgtataccggcactttactcaatgcagcaatttccgtcagcaatttcttaccatctttcatataggtgtagttgggctcatcgtagccaaaccaggcccatatgggtttcagcggccctttgcttttccgggcatctacgcctatcaacagcgtgtcttgttgcgcatgcgccggcaatgccgttaagagcagcaggagtgtaaaaaattgtaacaggtatttctgcatggtcaattattttctggttatataaaaatcacggtacaaccggaacacccggtacatcaccaacccactcgtcataatcagcaggatatagctaaaagacaggtgtttcccatcttccgcaggcaacacatatatcaacccgtaactcagcatggaaacaattacattgcataagccgcccgtcagcccgccggcaatccccgcattcctgggaaatatctgcaaacaaaaagtaaagtaattattgtgggtaaacccggagccgatatgcaccaggaaagcaaacaccagtatcgtccataacccgccatacaccgaaaacaacagcagcagcagcaaagccatcaccagctgcagtgcgaggttgatgctgatcttcttcacaaaaggtttgcggatcattcctttgctcaaaaagccgcccaacatccaggcaatgcccagtaacaacgaacaataaccggtgatcacagacgacaggttaaaataatgctcaatgataaaaggaccggacatgttatataccatcaccatcgaataggccagtccgagcatcacaatacccagtgtaaaactgccggtacggatcatcccataataaatagacaggatcttcgccgggtgaaacggcgtggtatgctggatggtttccccgctgaaaattatttccagcaggaataatattgcggcaaaaccacccaggaaataaaaattagattcccacccaaaggtgatttcaagatatccaccgataaaaggggccacaataggcccggtagaccagataatcgtaaacaggctcaggtaatgtttcagctgctcccccttgtagaggtctacaataaaggcgcgcttactcaccaccatcatcgctatggtaataccatgcagcacccgcatggcataaatgacgtaaatattatgcgtattggcaatgatcacacacgatgcacaaaagataagcatcgctaccaatgcaatccggtaccggccaaagctgtccagcaagcctcctataaaaagctgcgatacgccgtagctgatcaggaaaaggctcaccgtgagctgggcctggctgctggaaataccgagggcgttggccatacccggcagtgacgggatgtaaatatctgtggcaaaacccgacatcgggatcatggcaaaagccagcagggtggctattcttatattgctatcctttattcttttgtccgtaacagggctggttatcattacaatagctgttgattcgcttacccaaaatacggtatctaatcaactttatttgcctgttttaatcagttccatcgtataggtaatttccgggtccttacccgcctggatatacgtcataaacttcgtcaacggaatttccctgtcggggataataccgcggccattgtcggcgctggcattgaagaaatataactccgacagcggcacggttaacacgcaccttgttttgggcaacaggtatttcataaaccacgctgccgtagtagcagccacaccgctgccggtttccttcccgataatctctccccgcttatttttctggacaagcgaagcaaaataagtagcagcagaaacagtgcccccgcccgtcagcacatatacattcccgtgaaacgcatctttatccggcggaaaattttccagcaacccttcttttaaacgggcatttccaacataaaacccggaagaatctttatcaaaacgctggtaaaggaagttcttatgcccctggatatcttcgtcagataatcttctgccgttatccgccaccgcgtattcgggataggccagatctatggtgcgggtgcggtaattataaacattccggaaaggcgcctctaccaggaaggaataaagcaatgcggaaatagccgggttaccgcccccgttactacggatatctataatcacctgcttgtatctccgcttgtttacttcccggaaaaattcgctgaattctttataggcatccgcttcatttaacccaaaagtgtttactgtcaacagccccgtttgtgtatcatcaaaataatcattgtagatataatacgcccgctgcaaaaggtttaccgggaaaaccgacaaccgcccggcgtgatacgcctgggtaggatcggcagcggaaagcgtagtgcgcctcacctccctgctcccgggcgcaagaaaagttacttcgtaacttttaagccttggattcaacaggctgaaaactacctggaaattcggatacagcctgtccatcccggtagtaatgtagccatcgctgtaagcgggggccgacaaagcagccaggatatcttttaccggcatactgttaatgctcaccacctctgcgccaaaaggaatactaccacctttaatgttaacgaatatcttctcccgttctatcacaacagggaacgggaaaaaattgatcatgctgtacaactccttcccgttatcattagagaagcccaggttggtatgtacatcctttaacaggtaaacaggcgaatactgcaggccagacaatacatccggctcctgcgctactttgtttaacaacgaatccactttgcgcgcaaaggtgacggagtctataaacttatacggattgggatgctgtttcctcaagatatctaccgccagtttaaaatctgaaataacatcttcccttgtcaggttcgataactttttctcctgggcagctgtgtttaaacaataacatgcctgtatggcggtaacgccaagtatcaacagttttttcatatactttttgattttctgtgttaagaaccgatcaattccaggatgccttcattccggatgatcatcatcccttgccggtcttctgtaataccttcctccagtttgtaggtataacgcggacggttgccatccataatagttggtaaataaacgaattgaacattgctgctgtcctttaatgcctcgcccacttcaataatatgcgtggacacaataaagaggcagtcgcggtactcggcaaaagcggccgtcaccgccaaagtcccgtcgtacgcgtcttttacgttggtacctttgaacagctcgtcgaacatcagcagcaaccgctgaccgctggcggcggcttctgcggcgtgtttcacacgtacaacttctgcgtaaaaatggctgtaaccaagactgatattatccgccacattgatagacgaataaatgccttcccgcaccgaaaactgcatatgtgcagctgccaccgggaaacccatatgcgccaggtacatcccgatccctacagatttcatcagggtggatttaccggccatattggcgccggttaaaaacagcacattgctgtggtcattcatctgcacaatatttcccaccgcgccctctatacagggatggcccagctcctccgcggccagcatattttctgccggcggcaacgcttcagcgtaggtgaagcccctggcgcgcgccacatcgctcacggcaatgtttacatccagttcgtaaataaacaacagcactgcttccatctctttccggaacctgctcttcagcaggtgatcataaaaggcaagggttttcaccggcaacgcctggtagatatccatattcagcaaccgctccagcaatttatcggagaggatagtttttacggcctgtaaacggacggtaaaaggccccatatccggcggcgccatttcgagaaaggaataacatcttttcaacgttacaatagttgcctgcaacccctgcacttttttcttgtaccgttcatcgcgggtaagaccggaaagccattttttgagaagggtatcggccagtgtcagcagcccgttagccagcatgccggcatccaggtattccctcattaaattcagctgcgatatatcaaatggaaagcccagtttcgcccgctgaaaactccggaaaatacggctgcggttattgatagcatcggcatgctccatcgggtgacggaacatatcgtcgagcaactgttcccctcctcttgtttttacgtggttgaacaagtgatatactgatccctgccggtatttgcccagcaggttcagttcatccatcgtttgcctgtctgtattaaaacccatgatgatgattatttttttatttcacaagatgtacaacgctgcgcttcttcccgttcttcaacgtttcaaggatcccttcgttccggataatgatcataccatgacgatcatctgtgatcccccgctccagcgtataagtatactccggcgtgtggccgttcatgcgcgtgggcaaatacaggaacccgatattgccccgttgctttaatgcttcgccggcctccacgatgtgcgaggaaataatgaacatacttttctgcttccctgcaaatgccttagtaatagccactgtagcctcatgtgcatctttcacattggtaccacggaacaactcatcaaatattaccagcaatgattttccgccgcttaattccgtagctattttttttacgcgcagcacctccgcataaaagtgactggcgccaatacccaggttatccggcaggttgatggtggtgtaaataccatccatcaccgaaaactccatgaaccccgcggccaccgggaagcccatatgtgctacgtataccgctgtacttaaggaacgtaaaaaagtagacttccccgccatattggccccggttaaaaagatcaggttctgactggcattcatcaccaggttgttgccaatgggttgtttcagccccggatgatataccccttccagtttcaactcagtagcgcctttgtccagcgcttttggaaaaacaaattgcctgtccaccgccacttttgctacggagagatacacatccaggtaatagatataccccatcagtttttctatcttataacgctcccgggtgcggaaaaggagatcatacgcggttaccgccgcataagacaacttccctttcccgctttctttcagtgccggttcaaaggcagcgtcggtgagtaataccgcaatgcgttcccgctcccgtgcataggcaacaatgccggtcacttcttctctctctataaaaaattttataagatgaataagtgatatcaccgcgcttaccccgttagagatatccttttcactcagcacggtttgttttgcattggcgccggtattcattaaatacttttcagccatatcaaacagggccgcatcaaaggggaaggccagtttcaggcgggcaaaatgcgcaatcacgctgctccgcctgttgatctcctcgcggtccgacaacgggttacggaacatttcttccagtaccgtttcacccccacgggtgtgggtatgattgtacaggtcgtagatgccgctcacatcacgtttaccaaatatccggaggtcatctatcgtttgatcatctgtttgtaaaaacatagttgttgttttattttcttttacgccggatcaataatatgatggcgaatagcagtaccgcgcccggcaatatccacacgtataaaattttcaacacagctgccccggcagatgaaatggtgaacaggctatccagtggttttggacggggtgtataaataggataatggttgtagtcgagccagctgtaaaaacctttgccgaggaagccgccgccctgccgcaggttgctcatcatatcagcgtctgcgcctaaaacaatacgttgatccttgttgttgactttcctttccagggagatgtagttggcatatgctttcgcctggctatctccttccccggggttaaattcaggaggcgttgaatctgttaccagggtgccggctttcagccataccctgttttccagtgtttgcagtaaaggctttatctcaaaagcgccggtatccgtataagcaaaagcagtagttccgggagccatcatgaacatgctgtcgccgtgttccttatacgcttccttcagtatgagaagaaaaggttcgtcggccaggttagcagcgtcgcgcgtaataaatggtaccaccatatgaggcatttcatctttggagagctgcaccagtgtgccatccattaactgcacgcccaggtgtgccagcaaggggttcagcatttgttgcttgcctggttctcccaatatgaacatattgccgcctttgtcgatgtactgcttcaatttgcccatggtagcagcgctcagttccgttttaggatcggccagtatcagcgtggtgatgttagcagggatatccgcgttatccagtgaaagcgtatccgactcaaaacccaggttgatcagggcattacggttacctttttcaatggtatggaagcggaattcccgttctcctcttttaataatgctacgctccaggttgcccgtgagataaaggttctttggcaaatcagcttttaaaagccgtttgaaagccggcgccacctgttgttcttcgggccagaatagattatcttcaaaagtccgcaggaaggtagtttcgcctttgtacttcaactgcattaccagccggtaactttcaggtcccaggtcgatcttcttacggatctcttcccgcggcataaacatagatggatttaaatcatacccatctgctacctgctcttcaatctctttcaaacttttacctggccagttcttataaatggaactgtcgttgtcgtcgttatcatagtagtatacgtacttaaaagtaatatccggtttaaagcgctggtagcgctcccagagggttgttaaataatcattccggttttccgggaagccgcggcccgcccctcctcccaacaggttggtataaagggtaacctccaatggttctttgcccagttcctttatgatcttctgtgtattcggatgcagggtgttgatgtcgccaacagtggtatcccaataccctgttagtgccgggcgtgaggatatatagccgatcgtcagcaccaccagcgcaactgctacatatctcacggcgctcacaaaccagggtttcgattcccgtcctcctttcagtttgatcattgtaaacgatacaaacatataaacgatcagcacaaaataaatgacatccttcgtggtaatgagcccctgcaacattttcccggtacggcccgagatggaaagaaaataggtcaggtctctcacaaaatcatacttctgccataagccaccgatacggctcaggataaaaacagccaggaagctgccaatggcggatacgatctggtaggtagtaagactggacataaacaacccgatggccgtatagcagcacatcagcaggtaaaagcccagcatagcggataacaacatgccataatctaccgaccggatagtgaataaacctgttacaataaaaatccctacaatgcctaccagcaacaggttgtataacataatagccaggtacttcccaaaaacaatttcacgcaacttcaccggggacgaatagagtaacttgatggtgccattgttaatttccctgctgatcaggcccatggtgagcaatggaacaaacaggtacaggttttgcagcacattaacgaaaataccattgggatctaaatacatccccgccgtcagcgaaagattaaagtctttgaacttcggattattttttgccaatatttcctgccactttgtaagcggatacaatgcgtaagtataaaaaaccgcgcactgcaccataaacgcaatcgtcagaaaccaggctaccggcgaataaaagagattccgaagctctgttttcgcaactttaaatatcatcttcatgtcgtaagtttattggtgggattgaatagttaattgcttgaaaatgtcgtcgagcagacctttatcaagactgatctcctggaggcgccattcgtgttgtacggcagcggcgatgatcctttctgtgatatctttctccccgtcaaaataaatacgcgcctgtttttctgtcagcaactccactttggaaacccctctgatcctcatcagctcgggagccggcggcatgttttccattcccaccaacagggtatgcggctgtacataattgttgaatgcgtccatactgtcggagaaaatgatccttcctccttccatcatgatcacttctttacagagcaggtgtatttcagataaaatgtgagaagacaacaacacggtatgatccagggcaatttccctgatcagtttacgggcttcaatcagctggttaggatcgagcccattggtgggctcgtccatgactaccagtttgggtttatggataatggcctgcgcaatgcccacccgttgacggtatccgccggacaggttgcggatcagtcttgtgctgaagtgggcaataccgcagcgttctttggcttcgttcaccgctgctttgatccggtgtttttctatcaaccgcagctctgcacaataggtaaggaattcatctaccgtaaggtctgtatacaaaggaggattttgcggtaagaaaccgatctctttttttgccagttccggttgctccctgatatcgattccgttgacataaacacggccctccgtttgattcagcacaccgcacataatattcatggtggtggacttcccggccccattggaccccagcagtcctactaccccggtttgttctatttcaaggttaatatcccgtatagcccaggaagtgctgtacctgtgtgagagcccctcaattttcagtatagtgctcatagtgcgtttttagtaaataaaatattgatgaattaattcagtacctgatctgcattaccgcggttgcattggtgccggtacctcccggcagtcccaccagggccagggtaaaattcttatacatccagggatgcgcccaaacagtggtttgatgatagatgcccactgtgataaagcttcccagcaacgcgccgctggcggcatcccggaactcaaactcgtagtcgggcacttcaaacccggcactgtatttcttaaaaacagtactgcctttataaggcaggcgtgctacttccggcgcccctgtttgccctttgatgttgatgctgacatccttgctgccgggagaaagattgacaaacctgatactcattgaactgtcggcagtgacatgataaggcaggtcatccttaataaacagtgtatccggtgaggcaacagtacccgttaaaaacaacgtatgaatagagccaatgggcaaatccagcaccaggttaaaaagaggaacgcttttctccgtggtgtcgggatactgatacagggccagcggttgggtaccgctaaactgtgtatagcggttattataatcactgtatgctttgtagtatatccggttggcgtgataatattcaaacggatttcctcctttgaaattagttaccattgagctgttgcccactaccgcattgatcagggtaagtgatgcgctaccgggcgctgttgtttgtttggcgcaggaacccagtatgagcatgagcagcggggcggctataagcgcgctgcggagcggctgccatacggtttctgatctggaaaatatctgctgcatattaatagccgggattttgggtgaggaaatgattaaccgtaatttccgataccggaataggataaagcaattggtaatcgcctaaccagggctgtttcaccggcatagccgacagcacatcatgcgccatgccggtgcgtttcagatccagccaacgatgtccccattctgcaaaaagctctgtttgccgctcctttgctacggcagcctttacctgcacgacggtgaggttagccggcaggcttgccaaccctgccctgtggcggattacattcaggtcggcaatcgcagcggcgatacctccgggccctccattggcggcggcttccgcacgtaccaggtacatttcagccaaacggaacactacataatactcttctgcatctgcaccataaacagcgttgccggagccgatcttatacttactgggataatgggtaatgcctggaaatgtacctgttccataggaattatcagtactgtccgtccatgcaacataacgttgatccccttcttcaaaaactttcaacaattgaccggataacatgaagctcgtcttgccggtaacaaaaatgcctggcaggaactggtatccttccggtgtggcattctttagtgaaacatctgtggtagttggctttaactgccagatggcctcccggctatcttttaagaaaacgtgtgtcagatcagtttccaggccatacaccgccgtgttgttgatcagcgttgtagcagcggcaacagcgttggcatactcacccaggtagaggtatacccgtgccagcaaagcggtggcagtggctttgttggggcgtaccctttcgccgttgccggtaggatagctctccggcatattggcttccgcatccttcaggtctgctactatttgctggtacacctgttgctgcgccgttctggacatgctgcgcgtctggttaaaatctaccgtgagcgcaaggggaacatcgccaaataaattggtgagatagaagtaattaaaagcgcgcacaaactttgcttccccggtaagcgctttgcgcgtgctgtctctcagcgctaccgcagtagatgccgcaatgccctctatcaccgagttggcagcataaattgttttataggccgtttcccaggccattccggctttatcggcctggtaaacggtaagtttgttggtactgagcagatttagtgccggttcattgctacctgaatagttatccatctcgccggatgatagcccgcccatgatggttaacagtccggcgctaagaaaactttgcccggccgacaccacactctgcaccttatctccattgatcatgacactgtatatgccggccatagcagcgttggcctttgtttctgagctaaacacctgtgtagtggtaatggtgttgataggtgcaggaatagcgatcagttttctgcaggatgaatgtatcatactccagaaaaggctgctgataacgatgagtgttgttctttgatagatccgcatcactggtattttaaagcgtaattgataaggcgccggaaaaactccggccagccggaacagctgaataatcctgcacttcaggatctatacccgggtagttggagatcgtgaaaatattctgcaaccggaacgacagcgtacatccttttaatccagccttctttgataatttatcggagaaagaatagctaatggccacagacctcaaacgaaagtaggaggcgtctgtcatccccgcatcagaactggatacttcccccctgctggtattggaatagcggacataccgggcgttatcaccaggcttttgccagcggtcattgagtatgcttgcgggaaagttagacatctgcccttgtacgttggtaataaacggatcccgtcccaactgctttttgaaatcaaataaaagattagcggaaagtcccttatagtttacggtggtgcctataccgccaaaatatttcggcgttctgtctatgacgatataccggtcgtcgtccatagtaccggcaggaacgttataatttgcctttgcgaggccatctttattatgatcagcaaaactgtatccacccgtttgcggatctacccccaggtaatgcaatacatattgtgcattcaacgactgccccactttatactgggtgtagtaaggagataattcaaaatccggataagacaccagcaggttgcggttagcggccatgttaaaactgacagaccatatcaaatcttttttcttaatcaaagtggcagagatcatcccttcccagccactgttttccaccagtgcagaccagttgctcgtcacagttttgaagccagtataagcaggggtaggcagaccggtaatctgatccccggaacggttctgataccgggatacatctatcgtaatgcgctcttccaggaagctggcgctgaagcctgcttcgaatttcttatttgtctcccagtgatagtcctggttaacggcatgtatgggtacaaaaggctgcacaccgttataggcgtaaagcggcataaaatcaccggctgctattactgcccattgcgacaggtactggtaatccgttggtgtattccctcctacaagtccatagctggcccttagcttcataaagttcacccaggacggcaggaaacgctttatccatttttcttctgagaagttccatgcagcagctgccgatccgaaattaccaaactgcctgcctggggcaaagcgtgaagatccatccctcctggcagtcatatttaaaatatacttgtgctcccagtcataattgatacgcgccagaaaaccgacgtatttatacttactatatccctcactggtttgcgaaaaaggcgcgctgccaacactgcggatcagatcatcatccccatagcccgcagcgtaggtggtgatgccattcgtcatcgtggattgataagtacctcctaccagcaagctcagatctccacggcctataaaacggttgtacgtgagttgcggctcaacggtcaggttggcatttttcgacgtacccaaaacagctgaccctgtcggattactaatcgggttgtacgatgcgatgggcatgaaatagttacttgcacccgtcataaaagagtagccaccgctggtaacaaactttagtcctctcgccagctcatagctcatcctgatgctactgctgaactggttggtttgtgtattattcgacctgaggaggtcagcaaaagggaatcgatcacctacgcccgctgcattccagtcggcatagttcaggtcacccttgctgtcgtataccggtggagcgttgggaggcagcgttaagatagaaatactggcaaaatgcgcatctacgtttgtataactgtaaccaagcaccaggccgagtgagaatttctgattaacactgcgcacatctatgctggatgtcacagacgcctgctgattcagaccgctgttcttcatcagatcttcctgttgcgcgtaattcgcgctgatgcgatacatcgccaggttatcgccgcccgttaaactggttaccactccactttgcttaccggttcccagcaatactttttgccagtcggtataccgcgtgctgtcccacaatacaacatccggcgcagtgcttattgttggaaacataccatcatttttcagcgcctctctccgcacccgcaaatactgtgaggtattcagcatctggtaacgtttgggcacatcaatgatcccctggttaacttccatgttgaaagtggtcctccccggcttgccctttttggtggtaatcaataccaccccattcgctgcgcgggagccataaatagcagtggcatctgcatctttcaatacctctatgctggcaatatccctggggttcatactaaacaacggactttgcccgccggtaactgaaagcccaccctgcgtgtatcccggcgaaaccccggaattataacggatagagccgcttacatccagtactgttagtggtaccccgtctattacatacaatggttcagataacatatccggattcagcgaatttcttccccttatttctaccttcacaggcgcagcagcataaccactggtttgtgtgatcagcaaacctggcactctcccctgcaatgccagtaaaggattcatcaccggttgcctttctatttcttccgccgttaccctgctgatattcccggtagccaaacgcttgctggtaataccatacgcctgcaccacggcctggtctaatacactggtagccgttttcatagtcacgtatacgagcgacattcccattggaacttttaccattaccttttcgtacccgatacaggtaatcgtaagttgctcatcctcctttaactttctcaaaacaaaagatcccttttcatctgtttgcgttcctttagcagaacctcttacaatgatactggcgcctatcaccggagcgctggtcttctcatcatacaccaagccggttacatcatgcacaaccggatccaggtttatttttatcgaatccgaaccgttgtcaaccctgggaaaaacaacaatggtggtacctacaatcgtgtaacttaaaggctgtttagccaatatcaatttcataaatacttccagcggctgcttctttgcatttaccgaaatagccacgtttacattgatcagctcgggattaaatatcaccgcataatcagcctgcttttttatttcatcaaaagcctgctgcaacggtacctgtttgccgctgaaggtgatggtttgggataatacatgaactggcaaacccagtgcagcagtgatgaggaataatacaatcagcctgctgaacacccggtccccccggcacaaccgcttgtaaaatctggatcttagcataacaatctttttggttgatttaaataactaattctttcctgtggagcataccactcccggaggagtcactttactgtgatcactccccgtttcaaatgcgtttaattcttcagtttggataaagctccgcctgtagccttacagcttttcttttaaacataccggatggtggtgattccggactggcatacccattaattgatgttgattgatactacgaaccttagctatggcattactattattttctttccttcgatcctgtaatgaacacccatcttttccagcacaagaagtgcctgtgataaattcagatctctttttatttccccgctgaatataatatccggtacgccgttttcataaacaacgcctacatcataccaccgcgacatttgccgcaacacttcgtcgagatgcgcatggttaaaccggaacagtccatttttccaggctactaccatctccacatccgcgttgtgaatgatattcatcttcaactcattgttgatctgcgcctgctgccccggccgaagcatcgcagtttgctgatcatggatcatcataatacttccttccagtaaagtggtccggattacttgttcatccgtataggcgcttacgttaaaactggtacctaaaactgctacggtggctttgctattaatatccaccataaacggctgctccttgttttgggccacttcaaaataaacttccccggtcacttttactttgcggtagttatctgtaaaaacagtaggataagtgatgctggattccgcgttaagccatacagcggtaccatccggcaactgcagccggtactggccaccacggggcgtggaaagtgtgtgatattccaccttgccggccttcccttcgtaatccagtttgccgctgtcattattcacattaaaatttccattccgcacaatactgccttgcgtgctgtccagcaatatttcatcgccatcgcccagcttcagcaccgcgcggttggaccctgacataatttccccggaagaagatacattccccgccagtaatggcacgccttttttatggtggttgataaaccataccgctgttgtagctaccgccatgatcaatactgctgctgccgcataacgccaccaggaagagatacggcgaaccggcacgttcctgtcttctactgctgcctgtaaccgctgcaggatccgctggctggcttcgccggaaagcacgggtggctcagcgaatgactgatcataaacccgctgcaataacgtttccagtgcttcattgtcttcaatggcattctccttcaacaattcaaacaacgctgcgctttcggactccgtaatggtgccgtccaggtacttttgaagcaagtcagtttcggaaaatttattcggctccatattaataagactaatgaataaaacaaatgggtggatgcgggggaaaaaattatttcagcgataccaacagtatcagcaatgaaatatcgccgtgttccattagatactccttaattgactttaccgccagcgacaggtgctgtttaaatgtattacgggagatgtgcatcagtgcagcggcttcttcgtatgttttgccctgctgccggcaaagcataaatgcctcgcgacgttgtggtggcaggctggcaaccgctttctgaagcagctcttcatactgcttcgcctccatggcattcattaaggtttgatcgttgatacccagggaaacccggtgcagtacttcatcccggatcgtatcgtacagcgagatccggttcaattgcgttaatgccgtattcctggccagccggtacaggtaagcctggaacgatgatttaatatccaattgcccccttacctcccatatcttcaggaaaacatcatgtaccaggtcttcagtaagtatgggattcttggtaaatttcagcaggtaattatatataccaccgtggtattttaaataaatagctgtaaacgcctcctggttgccaagagcaagttggtttagtaattcctgttcattcattatggtgtgataatatcgttcaatcgggagaccgttcacatgacgacaggtaaattaaacattaattaccagattttataacaggacaggcgatctattgtttcacccgttttgaacttagccagatacccgccaacaccaatacgccgccggccatctgccagggagtaaaggtatctttcaggaagatcatggcaatcacggcgccgatcacggggtttaagttcaggaaattacccacctgggcagcgggtaaactttccaatgctttattataaagaaaataggccagcgcagaagcaaacacccccaggtaaataattccggcccaggctctccccgatatttcaggcatgccgtgctggtataattcaaccgccgatatgggtatcaggaaagccgagccaataaaagtactgatcgcagtagctaagatcgtatctgtatctttcaggctcctcgacaacaacgtatatgcgctccagcagcaaactgccagcagcatcagtatacttccccgcaatgtatgcgttccctgcgggcttcccacaaaacctaccagcaccactccggttacacataatataataccggcaatacttctgccactgatatgctctttcagcaaccaggctgcagggatggcaatagccaccggtatcaggccctccaccagcgcaccggtagatgccgggatataaagcatggcaaaattgaacaggccatagtataccgtaattcccaggatgcccattaccgccagccttttataaggcagctgctgttttacttttttacgctgatgaagataaaatggtaacagcaatgcgcaggcaacgatatggcgcagcgtggcaaacaggtacggggatacttcctgcaccactgttttggtaaccgcaaatgaactgccccaaatgagcataacaaacacgatgctgattatccctttcgtccggtcagctacagcatttttttccacaagtcagtttttcatttttaacatcatctgcctggaggcccagagccaggcaattactacacacagggttatcactaaagccgcccctgcaagtgcctggtaaaataacggatcaaatccattatgcatcacgtaaataaccgatatatagaggaccattatgccggaaacgcgcaggctatacttaattcccgttaccaggtagcggcggggatcagcaaaaatcgccatgccggctttgcctccccaaaaccaggtagcaccaaaaaggaacacaaaaaacaacagcatatcgatgttgatttgcgcatcaataaaaaagatcagtccgttcgcaaggtcggaccctgcttctccaaaaaaccatatcaactccagtataatcattgccaccagttgagcggcgattgcctgctttctaccaatttgtcttgctatgtctaacgtcattctatctgtaatgtaaaattatattgtaccaaattaacgaaaaagctgcttatgcggcatttcctgggtttgccccttaaaataagatagtgttttttcaggatgggacagggtgatgtttgcttattcacatccgggcgtggttatagtccttattcgcggatatacatttcatatgtatacgtgaatgatttttttgcgccggcatttacggccagttcaaaatccagttgccgtccttggttgatatcgtttttgtattcaaggttcagtgactggctatatttggtactggccgaagtaaccgcgccgcttattgttttctgtacctgtatatcggccaaccggcccttgctgttaacaacagtaatggtgccttttacggtagctaacgtatatttatacccgttatacgttttggcctcttttttcaccgaaacaagcgcttctttttcctgtaccaggatatccggcgaagtggtaataaatatgggcgtagaggcgcctttggcggtaaacttaagcacatcctgtgcaatgggctttagtgtatttttttgtaagattaaaacagcgcccgatgtaaatggattgtcggtattattgtagatttctacaaagtggttcactttgttgggcgatgcactacgcgctgcatgactcgcggcttccatctcttctgatgccgcatcatcatcgccgtttgtccggtaggtactcatcacagatgcgggcaataccgttttataaaaatggcggatcttcaccgtttttttaaacaccggatattgcgccctttctcctttgcggaggctaatgtttttgagtgtataaaaatagaggtcttcgttttccactgccacattattttccgatggcgcctcttcaggcattacaacggattccaccatcctgtccctggcgtaatccgacctcaattgtgtggcgttgctgtatatattggcgttctcaacaccaccggtagcgctaaagttaagcagggtagccagtgtggtagcctgcgaaaaattgggtacccccatcacaaaatcaacatccgtattcttaatatcttctacattattatttacttctgcctgcaggttgagcgttgcttctgtttcagacgctaattgcaattggtaaacaggggtccagctcaatccgttttgcaggtacatcatggtaaaggactgctgcccgctttgcgcaaaatgtatggtaactacaggtttttgaacagcaatacgcgcggttgtagtgcgactgggtttatcttcaaatgtaattgtcttgatggtggcaggctctataccgatccatttaccattcattttcagtaaaagaacggggttggccggggcatacagccggtcaaactggtattgcccgcggtattcattcgacaattgcatttgctgcaactgcagcctgctgttaatttcttcgggcaggtcaaagtcttccacactgcctttgtaagtattattatctgtggcaacaattgtaatgttcttgcctttgttggcatgcagcagttctaaaaagctgttggcttttctttcctgtatttcatttatctgctctacccggctgctcacgcggcttacaggattagtagtgccggcaaaccaataagtgccaaataacgccaccggaaggctgttgagccggaagccactgtcgggtacctgggcggttatttcttttaccacaaaggattgcccgtttttaaacacagacaatgatttgataactgcattatcctgtgcaacaagcgttatgcctgtagccagtaacaatgccactaaaataaatttcatacgcataattgctgttttaaaccctgaggctgtaatgatacacaataataaacacaattgcttcctgataatatccctggaaacaggtataataacctgtgtatattctctttaatttcagggccatatgcaggcaggaatcaaacaagaaaagaatatgatgataaattccagcggtcaggcgcttagtccggacgatgaaaaactggtacgctggtggcagaaaaagtatggcaggaaagcctggcagtgggccggcttgctcgtactccccttcctgctgtcagccttgttttttattttattcggccgggaagaaaggctgtgggcttatatatttatacttccctttatgccatttgctgcattttttgtttataagctggtgaatgtttttggaaagatgaggccaacccggaccgctctgcgcaggggattgaaacaggtgaccacaggtacgctgcaggaggtgacagcagataaacatctgctcacttatacgatagaccataacaccataaaggtagctgcaccgggacctttagaacatgtttccggcagcttttttttgccgggggcattaatcgtattggaatggcttcccgtcaccgtacaagataatatactactgaacgtacattataaagatgtgccggaagcgaccagcatcgccggacctgcaggcacagcagaaaaagcgaccctgatgatgcgctggaacagccgcaccatcaaaatactattcttcacactcgcaattccatctggcatctgcctgatggtttctgaaagggcacgtgaacccgcaataatgttaggcatgctgcttttcgttgcagcgattgctattttcctggcagggttcaccctggttttcaatcgccgtgtacaaaacgctgaacaaagaatagtccttaccggtatcattacagaagtttttgtttcccgttatgataacgatggcagtgaagataccagggtatattggtaccgtattggagagcaaattgtatcaggatatcatgatgatgaccgcttcctgcccggtgataaagtttgctgcgtttacctggccgataaaaaaggagtgcagcatggactgttcagcatggcattgctatagttaagacaaaaaataagctattcttttttcaggtcaatagtgatgaactccgaatccggcaaaatgatgtttagctgctcataatcccttttgtatgtcaccttcgcacctttgggtaactggcggccccccgccaaatgatcttcagacagtgttccggaaacaaacgtactatcggttgcgatgaccgctttgccggtgcagggccagccaaacaccagctgatcatacgcaagtgtaacgttccacgtatcggggcaattgataacaacccctatgtaatctttcacctgcaaattgaaaaagcgggtaggctttgataaatgaaccgaatcaacatccgtcagttgggcctgtttcctgtagttcatatcaaaatcagtttgataataaaccgtatcgtttgttgaaagagcaataccggctacggtttcaggctgttttaatatgaaagtgtgaagcgccttctgctgcctgaattccctcctgctttccccatcactgatccatccgctcactattacccacattgctaccagcagcggaaacagtaacacggcggcgccaatgccggaaaaccatcttacccagctgctgtttttccggcgaagacaggcccatagcaacagacaacctgctggcagggtaacataccaaaagtaaaatgtgtatatcaaatactcgccaaaagggccgaagtgaaagtccatccgtttattttaatcagtattgttctatcagctacaaagatagccctctcatgatggttgtatatacctggaaacgggggtttttaaaagatggtcctataatataacatacccccttccaacccctctgttcatttcattcattttaacattgtcatatccatttcatcctttatccgtgttaagcttctagctatcagtattataattaaattactactgtcgaaatgaatctggatatcgtctattgatcatattgctatcgaaaactccctaatgacttcaaatcaaagtcctcctcagcatttttacgccctcgacgctatcagaggcatcgccgctatgatagtggtcctataccactggcaatttttttactacgcaaacgacgtttatgtacagggagggtttgagaaaacggcacttccgtggtataaatacctgtctattttctatactgatgggatggtggcggtcgacctgttcttcctcctgtcggggttcatcttcttctggctgtatgcagagaggattgccaaccggcagataaacttccgcaagttcatcatttacagggtcagcaggctctatcctattcactttgttaccctggtgctggtgggagtgcttcaatggctgatgctgaaaaatatagggcactattttatcattcaatataatgatggttatcatttcctgctgaacctcgtcttcatgcaaaactggggatttgagaaaggtccttcctttaacggtccttcctggtctgtttccgtagaagtattcctgtatttcctgttttttattatctgttacctcaaactggaaaagaacaaactgctgctcttcctgctgattcctcttggcgcatttatacaatatcattattctctgattgggaaaggcatgtttacctttttcctgggggcgtttgtatactacctgtacgtttggatgatgaaagaaaacagggcaaaaaaatacctgccgtccctcatcaccatcacgctcctgctatggatagccatgttcgcagaataccaattctctattttacagggcatatggataaaactgcttcaccaggtgatgcccggtacaagtaccgaaaccgcgatgagcctgtttggccagctccggaacttctttttccgccttgctgtatctccctgcactatccttaccctggcaatgtgggaaacaaccaaaggtatgctgaacaagaaatgggcgctgctgggcaactgtagctacgccatgtacctgatccattacccgttacagataatattcgttctcgtagttgactggtttcatatgagccgccttgtattaagatcgccagttacattaatgctgtttttccttttactgatcccgttaagcatggtcacttattactatttcgagctgcccgcccaggacaagctcagagccagattttccaaaaagaataaaacccgtgtaacgattgctgatgtaaacgtaacgacttaaaagttccgtaatgaaggaggcccatcacctcctgtttgatgaaaaacctttagcgaataattaccggagaaaatcctgtattcacacgtcattttatacaataccgcattgataaattaatcactatatatgggattaaaatttagcttaccactgatcctggcgttagttatcattaccggatgcgcgggcacccaaaaactaacttactttaatgacattgccacagcggcgggagccgattccctcaaccgcctgcagcagctcaaaatacaaccgggtgatatcctgcaaatcaccatcaccacgctcgacaaagaagtatcacagatctttaatcccaacgtggcggtttccggccccgcagcaggaaccggcatagaacagggatacctggtagacagcaccggtaatatttccctgccggtcatcgggaagataaatgtaaaagacaaaacaactgctgccatcaacgacctggtatcgcaggagctggagaaaacagtccgtaatgcttatgtagctacccgcctggtaaatttcaggatctccgtactgggcgatgtagcccgtcccggctctttcaggatcggcgcagaaagggcctccctcctggatgcattaagtatggcaggcgacctcaacgtaacggctaaacgcgatgatatcatgatcatccgggaagtgaatggcataaaaacatatgcttccattaacctgaacgacagcaaaaccctctcgtcgccgtactattatctcagcaataacgatgttatatatgtaaagcccggaccagaccgcaagttcgccacatccaaaacaatacagctgctgccggctatcatcggcgtgatatcactcattaccacgattgtcattttaagtaaatgatccgtaatatgaatcaaccaaaaacgacaaacaacaggaactccgttatagatctcaatgatcttttccagaaaatagtttttcactggccactatatctcctggtgcttatggccatggtgaccagcgccatgctgtacctcaagtacaaaaaaccgatatacatgtcgagcgccaaactgtacctgaaagatgaaaaaaaaggcggcggagaagaaatggatgccctcaaatcactgtcgctttttaacaacggtaaaaatattgaaaatgagatggaggtactgaaatctcctatcctggtggaaaaagtaatcgccggcaacagctttaatatccggtattatataaaaggaaccgtaaagaatgaagagatctataaccaaccgccgctccacctccgagtactgggcgacagctcaaaagtagggaactacgtttttgatgtaacccgggaaaaggacctgctgaaaataaaactggtgaactataacaccgacaccagcctgcagttaacagcaaagcccggcgaaccatttaccgtggcgaaagataaattcgtgattaccttctccccgctcgccggcagcactcctgctaataccttccgcatccgggtggattccgtaccggaatacgcctacgaaaagatagaggaaataggtactgcgctcgttaacagggacgccactgtgatactggtgagttacaaagaccccgttccggaaagaactgccgacttcctcaactccttgctggaagcctacaacgaatataccctcgatgataaaaataaagtggcattcaaaaccattcatttcctgtcggtgagagtggattccttaaaagaagaactgggactgctggaaaaacaggaggaaaatttcaagatccagcgaggcatcaccgatattgacgccagttccaaactggcactggaacaggtaaaggaggcggatatccggctcagtgaagccaacctgcaactgtcggtatttgaccaggtggacagctacatcagcaaccccgccagcgattaccccttcgcccccgtgcttggcaacatcgaccaaacacttacttctatgatcaaccggtacgaagaagcgctccgggaaaagaaacggctctccctttcgctgaaacctaccagcgacatcctgaaaaatgtggagtcgcaaattaccgatacccggaaaaccattaaggactatatctccggttacaggcgaaatgccggcgtggtgcaaagaaaaacacaggacaaggtaaaccagatacaaggcaaaatagcgaatatacctacctacgcaaaagaatacattaacatcaaaagacaacaaggcgtgaaggagaacctgtatctctatctcctgaaaaagaaggaagaagcatcggtcgcctatgcgagtaacgtggtagacaataaagtgatagcgccggcatttgttcccgacaaacccattacccctaaaaaatcactggtattcattggctttattgcagcaggactggtacttaccagcgcctatatctatcttaaatatttcttaaacccaagtgtactcagtaaaaaagaaatagaacaggtgttcgacctgccggtgatcgcagaaatttaccagcaggaagaaggcgcacgcgatatgtcgctccagaacagatctgtactggtggagcaggtgtttaatatgcgtaccaatctgaagtttctgctcaccggggtatccggtacgcccaccatcctgcttacctccagcatatcaggcgaaggaaaaacgttcctgtcggcccacctgggcaactccttaacagtaagcaataaaaaagtagtgctactggaactggatctccggaaaccaaagctctcgcagttcctcgggctggatcataacgtgggcgttacgaattatatcatcggtaataaaaccattgaagagatcatcaaaaaagtacccggtaccgacggcctctacctggtttcctccggacccattccgcctaatcccattgagctgattgaaggagaccgcatggctgatctgctggcgcagctgaaagacctgtttgactatgtggtgattgatatgtcgcccatcggtatcgtgtctgatgcgaaaagcatttcacaccaggtagactgcgccctgtttgtagtacggtacaatttcacgctcaaatccaaactgataccggtatcggaaaatatccggaaaggattcttcaaaaaaaccgggatcatctttaacggtatagagcaggatactttctacccttattattactacgatcattattcatacacagaaaataaacaacataatcatacgtggtcgtcactggttaaaaaaataaaacaacgcattgcataaactatttgaaaatagcggttggcttctggttgataagctcagcaaactttttccgggcattatcatcatggcgcttattgccaggcacctgggtcccgaagaattcgggatctggaactatgcgctggcgctcaccactattatcggcagtgtggccatattgggcatggataaactcgccgtgaaagagttgatcaacaatgaacataagcagggaactattgtagccactgtgatcctgatgcggatcattgccggcgtggtgtgcatggcggtaagcgttggcattgtgctgctgaccggaaagcatcagcagctttatctttactgtaccattttctctgccctcatcatcctcttgcagtcttttgatgtactggattatttctaccaggcaaaaaataatgtcaaaaaggtgatcatccccaaagtagtggtatttatcattttctgcgggataaaagtgctcatcgtatacctggatggcgcgctgattgcattcctgtggacttccataatagaattagtggttacgtacctgatcatcattgcggtatatctatcccgtcatgctgcggcttttacctggcgtattgatacggcattggcacaaacgctgctggtacaaagctggccgctgatgctctccaacctcgtggtggtgttgtttatgaagatcgacctggtgctgctggatgcattggctaaccctgctgaactagggaaatatgtaggcgccgccaggatttctgaactctggtacgctattcctacggtgatatccgtggcgatgctgcccagcctcctgcaaacgaaaaagatcagtcacaaggcttacctggcaacactggaaaaatggctgcggctgtcgttctggctgagcgttgtcattgccgtaatggttacattaaccgcgcatatcatcattccgtttctctatggccctggttacgcggcggcatcatggatgctgatgatccatatctgggcagggatccctgtattcctgagcattgtgatggtgcaatacctgttcgtggaaggggaatataaaatatacctgtacggtaatctttccggcctgatcgtaaatgcaggcattaattttttcctgatcccgctatatggcggcataggcgctgccattgccacagtagcggcctacagcaccgtttatggcatgttgctcctgctcgataaaagcggccagggatacttgcttaccataagaatgtttcatcccttactggcattttctgatataaggcaagtatacaacagcctgcggatttttaccatcaacctggttaccgtacaacaaaaaaactatacgaaatgagcagcatcaaagatatcgctgtaaaattagtcaccaccttattcccccgcctcagttacggtgtgcgggcctacagttcggagggagaagacctgatcctgaaaaggattttcgaccagaaaaagaaaggcgtttatatagatgtgggcgcgcatcatcccttccgggtatccaatacctacctgctttacaagagaaactggacgggcatcaacatagatccgttgccgggttcaaaggcattatttaacaggcaccggcccaaagatattaacctggaaataggcgtctcggtagtaaaacaacaactcacgtatttcatttttaatgaaccggctttaagtactttttctcctgaaaaagtaaaagaatatacacagttaaccaaataccgggtgatcggtgaaagaaaggtagatacctggccactggcggatattcttgataaatacctgccggaaaatgttgccatagattttatcaccatcgacgccgaaggccttgatatggaagtactgagatctaataactggaataaatacagacccgcatatgtactggcagaatcatcaccatttgaggtacttcaaacagaccgcagtgagttatgccagtttatgcaccaggtaggatatagcatgtttgccaaaacctattacacttacttctttaaaaacatgaacgcgtaagatgtcaggaagcaggttatatgtacaatatggttgcgggcctttttcggcgcccgccggctggaaaaattacgattcctcgcccaccctcaggatccagcagatgcccgtgatcggtaaactgctgaaacccctgatgcatgtttcctttcataaggatgtgttgctgggcgatatcctcagaggcttgcccggtataaaagaaagttcctgtgacggtatttattgctcgcatgtactggaacacctttcttataacgactgcctcctggcgctcaggaatacctttcacatcctgaagccaggcgggtacttccgctgcgtgctgcccgacctggaaggcgccgccaggagatatattgaccagctaaagaataacgatccaaaagccaacaccagcttcatggaagaaaccctgctgggaaaagacgacaggatacgtggcatgaagcaactggtacagctggccctgggtaaccgtgaacacctgtacatgtgggatcacctgtcgttatcgcaccagctggctgcagcaggatttaaaaacatacggcactgcgggtttaacgacagcagcgatgccatgtttaaactggtagaagaagaaataagatttaataacgccgttgcattggaggcaactaaataatgttacagacgccggtcttattactggtatttaaccgccctgaacaaacgctgtttgtattcagccagatccggctgcagcagccggaacagctgtttattgccgccgatggtccacggccggacagacccggggaagctgcgctgtgcgaagccacgcggacagccgttttacagggcatcgactggccatgtaaaataacaacgctgttccgggaacataacctgggctgcggcaaggcggtaagttcggcgatcgactggttctttagccaggtagaagaagggattatactggaagatgattgtgtaccggatcccaccttcttttctttctgtacagcgatgctggagagataccggttaaacaacaccgtcatgcatatcaacgggagtaattaccagtcgggcgttacaaggggaatggcttcctattacttttcccgctacgcacatgtgtgggggtgggctacctggcgccgcgcgtggcagcattacgatttctcccttcaccgctaccagcataattcccggagcgggctcaatacttttttacgggccgaactgcaatccatatacgacgcccaaacagatacctgggatatccaatggttcatgacagtatggttttgcaagggatgggtaattacgccgaatattagtcttgtcagaaacattggctacggcaaagaagccacccatacccgctccaccccacggtggttcaggaaaatacactacggcgccataacggatatcattcaccccggtgaaaacaatattgatgaggcagcagaccggtataccatcaacacactatataacagcggcaggctatctatcaggcttaaaaaaatagtaaagaacaacaggttgctgtacagtttatacaaacgcatcccttgatcagtaaaaaataatatggaaacaggatataccagtcttcaaagcagtaattttttcgtggaatgtttcagggaaagcatgcccctggtcattgccgcgatactgctgtacctgtattataaaaagcggatctctattatagacacgctgctgtatgcctttgcgtcggaggcgtatactatgcttgttatagggcctacttttactgctaccttttttgttggcatcttcattttcattgaacaggcgcatcaattgtttaccggcaaacagtacatccggaaagaatatcttttcctgctgttgcttccgctcctgtccaatattgccgtgttcctgatcacacagttgtacaaagatccctttaattaccctggtggtaaaatgttggctttttataccaagcccatttatttttatgtaaaaacgtacttaccattatttgcgatcggcgccaagatagtgcaggaaagggagcagctttcgtttgagaagtttacagttaccatgaaaaaaattgcggtgatatcctgtgtgattgccgctatacaaatcgccgtgcagcttattttcagaagcgtggaactgagtgaactcctcgggttacagagccggtatatgctgcaggaaatcaacgggccgctggggttacgcgtacaggcattatttgcagaacccaaaatattcagcgccttcctgtctttagcgattcctttatttatgagggacaggaattacaaagcggccattgtaatggtcattgtaggcatcctcacttcttcccaaactttctggataaatatcctggccggcggcctcctgtttttatgtctccctaaactgatgccagtaagatggaagatcatcagtaccctgggtatgatcgttggtattttcctttcgatcgctgcctcaaaagaatacttcctgaaacattacatggctaaccgcaaccagccggtataccagctcctcttcgaaagatctgcttaccggtatgataatgagatctggggtaagaataatattatactcgggattccgctgcaaagggatatggaactgccggtggtcgacttcctgcgggatgaaccctatttggttatatcgggatatggtgcgggaaacagcacctttattccggcgagctatttctttggacagctgagttaccagaaccgggtagcaggcattggcgggcataatctcaatatgcggtggttttttatcctggcagaatttggggctgtttccctgttcttcttcttcctgatactcactaaaacagggcagcatattatgccctttcagcgcagctacctggcgtatgtagccgtttgtttctttttcagccagatagacctgttcctgataatagtggcattactgtgtgcatatgataacgaatccataaatgatacaggatatgaacaaagcacgtagtatactatggggtatccggttccggctgtcgttgctgtatcattaccttttcaacagcaaggtaagacggcggacaacttggcgcgaaatgaagtaccatctcttttcgccgcgcatgtatgccattgccaatgaaaaagctaccctggtaaataaagatgacaaatacaattactaccggataaaaggttacgaggagttgtttatttaccccgcgtccgccccgcattacagctttgcgatgatcctggcagaagcaaggccggagcactggcattactatgagatcccgcaaacagccatcgccccgggggatgtggtggttgactgtggcagcgcggaaggcttctttgcattcaaacaccagcacaccgccagccgcatttttgtactggaacccttacccctgttcgtggattcccttcaacaactgttccggcaaaaaagcaaagtggtgattctgccggtagcagcgggagatacctgccagaaggcgtacatcaacatggcctccaacgacacggtattgaatggcaccatcggccagcacaacagcaacgggaatgcggtggaagtggaagtagtaacgctcgacagcctctttgcagaaaagggtatccgcatagattacctgaaggcagacattgaaggattcgaggaaaacatgatccgcggcgcattggaaactatcagggccagcaaacccaaaatagccatcactacttatcatgaaggacaaaattatgaaacgctgatagccctgataaaaggggtggtaccggagtacaaccacctcgtaaaagggattcattacatctccggcaacccggtgatgttacacatgtggatttaatcatacaatgatgcaggtatttttggacaatattgtattctctattcagaaagcaggtggcgtatctgcctactggtacgagctgttgtccggtatgtgcaacagcgggttatcggttggctttttaaatgcacgcccgggatcagacaacatctttgaacggaaaatagattatcaccggtttaattgtatccgggaaagctggattcccagcaagtacctccgctatctcccggtacgctacccgcttcctgcggcggcggtttttcatggaggatacctgcgggtttccccacagaaaaatatcctcaacatccttacggtacacgactttgcacacgaacggaagctggcgtcgaagtttccgcggggccttgccaataccctgcaaaaagcatacggtatcaggcgggccgatgggattatctgtatttcagacagtaccaggaaagagctgttccacttttatcccggcatcgatcctgcaaaggtgaaagtaatctatcacggcattgcgggcgacttctaccccatcaacaaacgcctgccggtaaactgttcgctggagatggatcttcaaaaaaaattcattctctatgtaggtgcgcgcaggaattataaaaactttttcatggcggtaaaaaccatggagctgctgcctgctgactttcacctggtagtaataggtggtgagccctggaaaaaagaagagatcaatatgatgaaagaaaaactggccggccgttatcatatcttcccgaccgttagccaggcagacctcaatattttatacaaccatgcattttgcttgctctatacctccgcttatgaaggcttcggatttccgccgggagaagccatgaaagcgggctgccccgtggtcaccaccagtatgacctccatgcccgaagtagtaggaaccgccgggctgatggccggcaaggcagatccactgctgtttgcagaaaaaataagatccctggaaaatgacgcattcaagcaacagctgataacacaaggacttcaacaggtacaacagttcacatgggataaaagcgtacaggaaacaattggtttttacaaagattgctggaactacaaattctcgacatgagtattattttcaaaattgcagacacggtaaaagtattcctgacatccggcaggggtttcacttcgttgctggaaaaaggtgcgtctgtagcctctacgcagatactacacaactgccggcactatatcccctcgttaggcgtaattatagacgcaggcgccaaccagggacagtttgccatggctgccagtcacttttacccgcaggcgcgtatccattcctttgaacccctgcccggcgtgttttccctgttgcaacgcaatacccgcaggctcaccaacatcaacacgtataacatggcgctgggcaactccacagggacactggaattttacagcaatgcgtattcccacgccagttcagccctgcatgtatctgacctgcaaaaaaacatgcttcccaaaacagctaactccaaccgcatacaggtaccggtacaacgcctggacgacctacggcataaagtgccttttatcccgccggtattattgaaaatggatgtgcaaggatttgagaaagaagtactgaaaggagcgctgcagagtctccggcaaattgactacctcctgtttgaaacctcttttgttcaaatgtatgatggcgagccactgtttgatgaaatgcaccattttgttaaagaactgggattcgattttatagcgcctgttggcttcctgcaatcggaaaaattgcagatcctgcaaatggaccttttatataaaagaaagaaaggatgaaaattgttgtgaacgaccattccggccatgcctttaccttacagcttagccggcaatttgcggaaagcgggcatgaagtattgcatgcctactctgtttctttccagtcgcccaaaggaaactttgaagaccttcccctgtcagggtccgggcttaccgtgctgcctattatgatcaaaggaaaattcgacaaatactctcttttaaaaagaaggaaacaggaaattgaatacgcgcgtcagctgactaacaaactggatacattccggcccaacgtagtactgagcggcacaacgccgttatttgtacagcaacatgtacagcaatactgcctccagaaagggatcaaatttgtgtactggtgccaggacatttacaccatcgccatccggcagattgcccgccagaagttaggcatgatcagctttcccatctggtactattttaaaagcctggaaacaaaactgctgaagagaagtgcgcatgtgatcagtattacacaggacttcaatgatctttttgacaagtggaaattgcatccggagcaggtaacctgtattcccaactgggcgccgctccgggaaataacgctcaccggtaaaaataacgattgggcgcagcggcacaacgtagcagataaaacctgtattgtttattcgggcacattgggattaaaacacaacccggcgatgctgtcggcagcggcggcctatttccgtacgcataaagatgtggtgtttattgttatctccgaaggattgggagcagccttcctgcaaaaagaaaaagaggaacggcagctggacaacctgctgctccttcccttccaggatttcagggatatgagccaggtgctgggcgcagcggatatcctgctggccatactggaaaatgatgcgggcgcctattccgtgccgtcgaaagtactcacttacctgtgcgctaaaaagcctattgtgctggcgatgccaccggataacctgagcgcggccattgtactggataacaaagccggctattgcatttccccggataatcagcagggcttctgccagcacatagaaaagctgctcagggatacgacattaagacaggaaatgggacacaacggacgggcatatgcagaaaagcatttcgacataaaacatattgaaaacaaatttcttcaggtatttaataccatcctgaactgataaagatgctcattcataaccggcgccacccatactatccatcatcttttaattatgaaccttatgatacccggtaaccatattaatttcctgctgagactcctgatcgattatgtagtgctgatactggcttttctgggcacccgtgaatatattgcgggtttgggagatgtattcttctccggctttaacctgctattgctctgcatcagcattacggcctggaccatcatcggcatgtcgcttcatttatacgacgaattcagaacgaggtcgttttcctacgagtttattgccattcttaaaacagcattgttgcatgcctgtttcttcaccttcctgttcttctactgctttaaatattatccctatccgagaacgttcaccttgctgtatgctttcctcaattttgtaagtattaccgtggttaagtttatggtcaaacaatctttgctccggttgcggtcaaacggttacaacataaaaaatatactcatagtaggtaccggcgataccggcatgaaattctataaaaccattttatccaacgatcatttcggttaccggtgcgttggctttgtggatgaacaaaccaatccttacctgaacgggcagtacctgggcaaaatatcggacctcacgaggatcctggaaagtcatgagatagacgatgtgattgtagccctgccggaccctaatacggagatggaaaaaattattatcaccagtgagaaggaagccaaacgggtaaggatcattgcagactgccaccgcttctgcacctctaccgccagtatgaatttctttggtaaattcccgctgctgacgatccgtacttctccgctggatgacctggcgaagcagcggttcaagcgcctttttgagctttgctttactaccatcctctttattacggtatttagctggttgtttccgctcatcagtatactggtcaagctatcgtcgcccgggccggtgctgttcaaacaggaacggtggggactgaagaacaaaaaaatcacctgttataagttccggtccatgaccatgaacagcgatgtagtggatgcaaacgggcgatacctccaggctacccggaacgactcccggattactgcagtcggccggtttctccgcaaaaccaatctcgatgagctgccgcagttttttaatgtgttgatgggaaatatgtcgctggtgggaccccgcccccatcccattcctttacaccaggaatctaaaaacacgatacaaaattatatgctgcggcatgtggtaaagccgggtattacaggctgggcgcaggtgaatggctgcaggggggaaacgaggatatcagggcagatgcagaaacgggttgactttgacctgtggtatattgaaaactatagcttctggctcgactgccagatcattttccagacattgatgaatatgatcaagggagataaaaatgcgtattaacgctggggcttcctcagggccacaatattctggaaggaaaagatttcatagctggtgctgttgtatgctcccagggctttgagtccgtcgggtaataagcggtaaaattcatagcccggcaatatatctacaatatccttaaaaaaggttctggagataatattcatttcgttgaactccacctgtatcacatctgccagtccgcgggcaatagtttggcgggcgcctttcagcacactcagttcatgtccttctgtatctatcttcagtaaggctatcctggatatttcttgctgtgctacaaattcgtcgatggtagtgagatcaatggacacttcttccgcggtgcccttatgaagatgttctatcacccctttatacatgctggcatgctctgagccgccatcgccctggtagtcgtaaatagtagccatgctactctcctcgccggcgccctgtggaacagcggtgaaatggtgggttgctgccgccgcgcttagcttgcggaacgccacagggtgtggctcaaaagcaaagatcgggagggtgatgccgttctttctcagcatcactgaatagttgcccatgttggcgccaacgtccatgatcacgccggtatccagcttgcggcgggccttcaggaatttaataaacgccttctctccggacacggtatcattttcatgattcctgattcccaacccgaacatactgagcttatacaagaagagattcacgggataaaaaaccttccgggcgaataagagtacatacactcttttaacagactttccgagcgcattcatagtttggttattggttgccggcagtgaatactgcactctactaaattacggctatttatgcagcggggcctgttcactttattcatttccggatttacgcacctgtccttatctgtacaatttggtatcttgcgcccttatccaatttgatcgcttaaatgaaacgcagatctgtatcgcttacttttaatattttcctggggattggcttgctgatggtggtcattgccgttatgatatgctataatgttaaaacgttcaatgcctccgcggtaaaaaccagcggaacagtggtggacatgatcgccaggggaaaacggtcgtacgccccggtgataacgtatttcgatgatgcaggcgtgaagcaccgttatatttccagcgtttcttccaatcctcccgggtacgaaatcggggaacgcgtcgacatttattacgaccccaaaaaaccggacgatgcgaaaatagccggctggatggaatactttggcgctatcgtcgttggcggcatggggttgctattcagcttctttggcctggggtattatttaaagagaaaggtgagccgctcgcgcagggaccagctgaaacaatcggggttgctggtccgggccgactttgactcggttgacaccaacaggtatattcgggttaaccgtcgtaatcccttctttatacgctgcaactggaaagatccgctcaccggcgtaaactaccgtttcaagagtgggttcatgtggtccgaccctacttcactgattggggttcatcaaaaaatagacgtatacatggacaaaaataatccacgtaagtattacgtggatatttctgcctttgagcaataatacagttacggcgggctgtgaaagtaacagcccgccgtcgttatcaataagcatacttcggatctaccttacgctcatccacactgatgccttccttcatccatcttggcatgggtttatctttgagatagtgatcaaagaactgtcccattcgcagtgtccagtcctgttgcgggatctcctcctccaatgtgtggttcagtcctttgtagttaagcagccaggcgggcttgcgcagcctgcgcatagccaggaacaggtccagcccctgggtaaaggccaccgcaccgtctttgtcgttatgaaaaatcagcagcgggctggtgatcttgtcggcattaaagatgggcgaattggcgatgtaggcttctttatcttcccacagcgttttccctaaacgatactgctccacttcacatttaaacatacccggcgccccattggagcgcactgccgtgtagttgtaggtaacgttaacggcgccggcgccgatgttaacgcatttaaaaaggttactacgggtagctatatacgctacttcaaaaccggcaaagctgtgcccttgcagacccatatgcgccttgtctgcaataccccggctaatcaggtccattacgccgcttaccaccgcattgtaagcgctttcaccgggttttccggtagtgtagtgtatgtccgggcggaataccacgtagccgttacttacataagtaggaatatcgatagtagacgtgctgtaacccggcactaaatactcatgcagatcatgggaatgcgtttcataaaaatcaacgatcatcgggtaagtccgggtggtatcaaagttttcagggagatataagagtccctggttttgtttcccttcgtaatttttccattccaccacttttgctgaaccccagccgtactgcgcctgttgagggttcctgttggtgaggcgtttaactgccgtaagaccggcattgccccaccagatgtcgggatactgccggtaactctgccgggcgaaaacgaaggcattaccattgcctgcaacactaattacttttacggtgtaagccggattatcggccagcgctactgctttcccgccggggtttaagcgatacagtccgcccgactttgtttgctcattgaagctgcgcagcaggagtgcttttttcaggtccagcatgccgccataatccgccccctgcaaccggaaacttacgtgatgctgccggccatagccgccggtaatgcaacgggcaggttgtttgccggtcaggtctattgcccacatatcgtaccggtcgtatacaattacggtattgccttcgtctgtccatccagccataccataggatggtggcgctttgggcaggtcgaaatcttcttcatacaccgggtagccaatggcagcagaaatcgttacaaactttgcctcctccggtttcaatacctgccattgtttttcattgccgttatatatcactgcaaaccggccgttggggctccattgcgggttatcggtacaatcttccgccaccagtttgcgctcgcccgtgcgcacatttaccaggtaaatgtcagcattcagcgagtacttccagtcgagcatatattcatagcgcgactgatccgtgagcaatgcataattgtaactcccgctttgaggtgtaaaaagcatccctgcatattcaggcgccacctgcaccagctgcttcgtatccaggtggtagatgaattttgcatcgtccatcatcgttctgtcgtatacccctctccgttgccgccgttgggatacgggttcattccaggtccacagctccaggtctgctgcgttgggattgggcttgggtggggttttgcgcgctgtattgaagcttacttccagcagcaattgtgtggtaccaggtgtaatttcgtatgccttttgcgtaatacggtaacccggcggagcggtaatatcgttgaaatccatgagcagctgaggcgtacttttcttcagcgaaaaagcatacagctttgtgcccgacaacagcgtgccttcttctttaccaggattaaaactgtagtcggttaccggaccactaaacagcgcagtgtgcctgcctttcagcgggccggccatgagccggtcgccacggagataaaccacctggcccttgccggaaagagaatacctgtctgcctgttcgaggatggtactgtcgttggtatccgtattccagatcacccaccggctaccggctgccgttttatagttataggaaatatagggagatgtttgactgttgctgataaacgaggtagtcgtccaccggatctttttcccatctttcaaacgcatgagcattagtgaatcattcacattatacttcagccatttgcctttattaaaaaaatcggcccccgaagtgttgtccaacaggatctccttgctggtttgtgtattgaccagatgtttttgcggattatcgtcatcgggcaaatcatacattacccaatcgccataataactgataacgggaatacctatacgtttccattctttataggcggcggtatccagcgctttctgctgcgctgcagcgggcagtatgccggtacctgtcagtgcggcatataagagcaaagacctttttctcattgttctgcttttaaaatctcaataacctggcttaattcatcggcaagtgcgcttggactgccgccgtatccttctgccgtatatcttattattccgtttttcaatactacttttcttggaatagcggaagactggaaaacgggcaacatacttttaaatacgcggtcgtttcctttcgtatccgggttctcatcatcgtacaacactttaaaactataacccgacgaccttatatatttagagatatcttccttgtaagttttagcgcgttccatggtggcgatgaaataaaaatcaaccgacggatcagcggcatacttgctcactgccatctgcatgccggggaaggccattttacaggggaaacaccaggtagcccagtagtccagcacaatgatcttgttgttccagctatcggagctaacggtgctgccattcatatccttcaaccggaaaggcgtgatcttttcgcggataagtttagccttgatttcattgctgtccacagcaggtttaagacccgccacgtatgcatcaaatcctgctgttttgccgtatatccttttcagtttttccatcataacaggcgtagcggcgccggctttaacacctgcttccaatacagttttcaccttcttttcgccaccggtatgttccagtatgtttacccaggcttcattcagattggcattgttgtagcggcctttcccggagcgctgcgccccgtaaggaagtgcttctttatacttacccattttattcagcatgctgatatggatagccaggcgggcatccatttgtgtgcgggcattttcgcgggcttgcagcggggtgtagcgggtatcttccatgtatgatccatcatcgctttttttgatgatgtcgtcgatcagcatttttgagaacggataaatttttgctaatggtgttttcccgataataaatgctttatcgagattagcccggtatatttcattcagcgtaacaaaatccatatcgcggagatgttttttcaggctgtcggtacgacccgtggcaatgtacacctggcccagcaaacggtatatattgtggtaaataaattgctgcgaggcgatagtgtccctgcggtattccgccaccgggaaatcacggaggaaagtttccatggcagcaaactgcgcttcgcccatttgtcccatataagctttgctgtatgcatcgaaccgggcggcacggcctttgggaaaccgttgcagttggagctttctcacggaatcagctttctgttggtctttcagctggaacctgtaggtttcatacacgatgttatagccttgttcatcgagtccgggtatccttaaaaacttttccaggttgcgcggcgctctctgtggaaattcatcgccgagttttagtttgagcatagccaggtagctgtcgaaaaattttggcatgctatcgggataggcttccatttccttacgcacccacatttccagtgcttcgttgctgatatcgtagttattaaaataaaatggcgctttggcgacagaaggcttacggaaaataccccatgccagctggccgccgggtaaacggttaccgtttttatcggtggtaaccgacataaatccatgatcattattattgtcggaggcggccaccataccgttttcagtggtcacaaatttaatggccacaaatgcgcagtttgcaggaaccgcgtactggccgttccaggtggcgccgcgttgttgcagtacaatatcatccacataccagcggtaattccggtagagataaatcatggcgcctatatctgccttaccggccaatggcccgccggcgggattatacaggaggcggagcgtatctcctgccacgggtttttccagccccgttaagcggctgctgtcctgcgtgtacgcggttgtggaaaacgccagcagcaacgccagcatacttatccatcttttcatgttgtttccgttttttaatggcatgccctgagcggctgcctggtggcagccgctctaccggacatcccgggttatgatggttggttaaatattatcttgggctttgcgctatttccggattcagcaggatgtattttgtaccaattggaaagatataccggttgctgtttggctccagtgtatagtttacgcctttgaaagtgcgggtaaccgttttggcaaaagcggcgtctttgttcaggcgtttctggtcgaaccatcttaatcctattccaaaaaattcgcgctttctttcatccactaccctgctgagcgcttccgccggggtgccgggtgtatacgccgtatagtctgctgtgaggaatcgtttttcgcgcaggctgttcaatacgttggtggcggttaccgcatccccggagcgggcagcgcattctgctttaatcagcatcatttccggtacgccaggaccttgtgtgatggcattgccctcgcggctgtagcgatagcgccagtagccataacctgtaaacgccggaaaaaagttgccgcccggttttacaaacaaggcatagcgcatatcttttgtgccgagcagcgacaacaacgccgtgtccagttggatacctccctggtagaaaccagcgttaatctttgaaaagatcacttccggatctttcagccggtagggaaaagtggctacactcgtggcgtagtcacggaggtccagcacgccgttttgcagtgtcagggcctgttctgcataactccgcgcggtagtgaaatcgcgggtcatcaggtaagtacgtgccaacatggcgtaggcggctgctttagaagggcgcgtattataatcaggcaaagccggcagtgcgtccactgcctgtttcaggtcgccggtaatctggttgtacaccgtagctacagctactctttgcagcgatgcaaacaggtcgggcgttaataataaaggaacacccaggtcggtggcggcggtggcggcatcgtactgcgcactgtaaatattcaccaggcaccagtaagcatatgcccggtgtgtgagcgcttctgcgaacagctgtttcttgtctgcatcagtaccattttcgctggccattacaccggccagcacttcgttgcaggtgtaaattgttttgtacagtttgtcccagtctccatccgactgtgtatcactccagtactgcggctgccacgtataggcattcccgttaatatcggtcatggtagcctgtttcgaggaatccaggaaacgggtatcatcaccggaataaatagtgaggctgaaacctgcttccaactgggagttattatccagcaaagcgcggtagtctttggtgtaggtaggcgtacgttttcctatctgatctatttccacgtatttacggcatcctgtggccagcgccattaccgctacgaaatatattagtcttttcattttcttcgctgttagaatgatgcattgatgttaaacatatagctggttaccggtggcatgctgtaatagtttgcatttgaattcaggtactccggatcaatcccatctttattagctctccataaaataccgaggttacgcgcactgccactaacattaagacttttaatcacccgttgcggcaataattctttcgggaagctataggtgagcgatatttgttgcaggcggatgttgtcggcctttcttaccagcttatccgaattccggtaacggacaatactgttgttattcacgttttcaagacccggcacgtcggtaaaggcttcatcacctggttccttccagcggttagcaagatccttttgccttccgggcaaaccaaaataataccccgcagatgtaggatagttggtgatcgcaggtttcataaaaacatgccccatgtaataggtcatctgcaccctcatttcaaatcttttatagcggaaggtattaaagaacccgccgtggtaaggcgctactctcacgcccgcatatttcaggtcgtttatatcaaatgccgacgtaaggttggtggtattgctgatgattttattgttgcggtcatagatctgggtttgacctttattgtccagtcctgcggagcgatatacaaacgtagcgccaatgggatagccgtttaccggggagccgccgctgataaggttggaggcctgtgtaatgttatagcggttatcagttacttcgttggtaccatatgcaaaattgaaaacagaagtaatgccccagtcccttgtttccagcaatttacctgcaatgccgaactccataccatgacttttcagcgtaccagtattaaactgcagggtagaccagccataggtggagttatacggcagcgtggtgatgatgccttcgctccttttggtgtaggcatctgcggttagcgttaagcggttattaaaggccctgaggtcaactccgaaattgagtgttttggtcagctcccatccaagttgctggttgcccggcgattcaataacaccgatgggcagttgtgtgctgggatctgtggcagccagattgataaggggtacattgcttcctgctaatggcaccgaaccgccggtaccgtaggtaacgcggaggtctaacccattcagccaatgaatattctgcataaatgattcctggcccatactccatttcgcgccggcggaccagaaaggttttgcgcgtttgctgcgttcaagacccaacagcgtatagtcgtcgaagcgcgcgctggcggataaattgtattttgctttataggtataattgccattaccgaaataactgaggtagcggttcttttgttctgttaccggggtggttaccgggccgatattctgcgtccagccatacatggtcatgagctgtgcattgggatccacggtagcaaaggtgttgccatccgcattatatccatagcgggtagacgcatatgacctgctataggtttccctgatttcccctcctgcaagtgcaatcagctggtgatccggattaaaattacggtggatgttcagcataccacgcaggttgtaatcgtaggcattggcatccgacaaataataacggccaccataaggcagattgtaagttggtttgccgctggaaggattggtcaccgtgtaagtgttcatcaatgtgcgtccggcgtaactttgcacatcatccacgctttgaagactattcgcattacgctggtacataccggtcacgtccaggttggcccagtttgtaagtttgaaattgagtcctgcgttgagccggacctgttgcatactatttttagtggtagaataccccaattcatcgatcgcattataagtagcgggcaaaaagcctttggccaccaggctgtcgtttacttccgggcggaagcctacatttcgctgtatgtggttgccatttgcgtctaccagcatatcgtagggacgcaatgcagtagcgttttgtcccaatgcgtcggcagcggcattattaaagtaagtagtgccgctctggtagctgaaaccggtagacagcttaacacggcggttaaacagatcgttggtgaggttaccggtgaggaacacgttttgtgcgctgttgctcctgaaaataggttggtctttattaaagttaccggagagatagtagctgttgttatcgccgccgccggatacggacaggttgtattgctggttcacggcggtgcgcagcaggtacttttctatttgcccgtagttgttgcgggaggaaatttccgcgatggcggcatctgcctgcgcctgtgtggctgttcctcttttcactttgtaaaaccattcctgtacttcgctgggattggatgcctgcaatgggttataatagccgagcgaaagtgcatctgtaaaaaatcctttattcagcatttccatttcaagatctacatattccgcggtagacatccagttgagatccgaaatggaaggcgctttggataccccgaatgtggcggaaaggcttactgcgggtgctccccgctttcctttctttgtttctatcacaataacgccattggcgcctcttgctccccagatggaagtcgccaccgcatctttcagaaaggtgatctgttcaatatcgttcggattaaaagacgacagcaccgaaccattggccatgaccgagccaccgagtgtcgtcagtttttgagcatccccggtggggatcatgggaaagccatccactacgatgagcggcgcggtagtgttgccataagtattggtagtacggatctgtatggtgttgcccctgatatcgaattttacgccaggcactttaccttccagtctttccataatgttattggaaggcacttcagccaggtctttcgcagtaataatactgtaagaaccggtagctctttcttttgaaatcgtctggtaaccggtggatacagatacattgatggcgctgatatcgatggtggcgcgttcgagtacgattaccaggtcggtgttgttgctgatcttcacttcctgggatttgaagcctacgtagctgatcaccagtacatcgcctacattcacgctcagatcgaagcgcccgttttcatcgttgatcactgaccgcccggttccttttaccttgatggtagcgccaaagaggatgttaccccgggcatctttcacgatgccctgcacgggaatcgttaccaaaggagtggtggtattggcataaggcagcggaagaggcattgtttttttgctgacgaaaatggtttgctcctgcagcatatactgcaattcctggcctttgaaaataatgtcgaggaactgccctaacggcatatccacggcagccaggttcactttctgcgtgcctttcagcaggtctaagtcacaaaatatgtgatagcccgtttgcgaccggatggtttgaaaagccttttccagcgtgatatttttgccggataaggtaaccgattgggagactcctttggcgcttactcccatcagtgcggccgttaataatagcgtggttagtttcatcactaacagaatttttttgcagagactataccctttggttgtctcattgattccccgagatttggttgagaaccggggcccttcctgcctgcatctgtgcatagcatggccactccggttacaagacgcatttttttgcataacttgcaattggttaggttgattgaaaacagttgacgcgaattaattgtctatcgttcaccctggctataggccgctctgaatcctacctcagagcggttttttagtatagggaaaaatacttacggtaatactaccagccggttgccggcttctatccggaaattcaccccggatgcttttaatccttccaggacctgcgacaggctaaggttccggcctatttcaccgtagaacttcctggtgggaatggcgccctcgtatacgacttctatattgtaccaccgggataattgccgcatgacttcggcgattcccagctggtcgaaattaaaggtgccttctttccaggcaactacctgggcggtattcacctggttgtttatttttatgttgctgtttacttccgcttgctgccccggctgcaatatagccgcctcggtccggagacttattttcacgctgccctccaggagtgtagccctgatgttggtttcatcgtcataggcattgatattaaagtgcgtgcccagcacttccagcgttgcctggttattgatttgtacccggaagggtttggcagcatctttcgctacttcaaaatacgcctctccttttacctccacctttcgttcatttcctgtgaaggccgtggggtaacggatagcgctggcggcgttgagccatacctgggagccgtccggcaatgtaagccggaactgccttgcccggggtgtgcttacggtattatacgctatgcccgaagctttgccggcatcgtaactgagtcctccgttttgcatgatcacggtggtgccgttctggttggcgaggatgccgttgcccatactgtcgagcgtaatttgcttaccatctgccagggtgagcatggccccgctgtgacccggcgctacatctgcttttccggccagttcttttttgggtgttccggggcgtaatgtaaataccagtatggcggccagtactgcggccgcggcggcgggccaccatatccgcatcctgcggacctttgcccggtcctgctcctgcaaccggcgccggagctgttccaggaaagccggggaggcttcttcgtacaacactggtcctgatgccgcttgtaattgctgatgaaattcttccgcagacacggtttcgtaccaggaaaaaaattccatttcttcctgttccgtcagcgtaccgctccggtatttatttaaaagcgctattttattcccgttgttcatagatggcactatatactacagacgaacacgtgttgtattcgtatacgccaaaaaggaatttttttttatttcccgttaagccaaagcaggaaaaggatagcaacaggtccgccgtgctgttccagcacggactttaaggtatggaaggcggcatagtaatgttttttcaccgttaccacggcgatgccgaaccgggcggcaatttcctcaaagctcagtccttcttcggtgcgcagcaggaaaatgtcgcgcttttgtttgtcgaggccattaatggcccgcagggccgtatcatgtaattccttatactccagtgcatccggcatatcggctgccgaggcgcgctgttccagtgcttccattgcccggagatgtacttttttccgtcttaacagatcaaataccaggttgcgggcaatccggaaagcataattttcgaaggacttcaccagcaacagtttttcccggatcttccagatccggagaaatgtttcctgtaaaacctcgtcggtttcatggcggtcctgtgtaataaagttaacggctacctgcagattggggtaataccaggtgtacaattgcgcataggcatcctggtcgccatcggcggctgcctgtaccagtaaatgttcgttggagagcggtacccggtgatattgcgaaaaatgtgaactagccaatccgtttgcaagatacggaaaataaaaaaccatccctgaacgggatggttcgctttatcattgcacccgctgctgttgcttcagcagcttagccctgttgatgtctttctgtgcctctttaatattgatctcattgcccagctgcgttttgaggtgtcccctgttctcaaaaaattcagcgcggttattattaatctttattgcctcattgaaatcttccaaagcagacatctgttggtttaacttcagttttatcagtcccctattattaaacatcatcggtagctggttgctgctaaccctatcaaacaacttgtcgatctgatccagcgcctcctggaatttctgctgctgatacagctggttagtccggttaagcaactgttctattccttgtgctttcaccaggctatcgatgtttaaaaagctgttcagggaagcatccggctgattgacgaaattatagccttttgctattgccaggagccgtttggctttggtagggtgactgcatcctgcttcgagttcagggggcggatgtttatccaccgcctgaatgcccgactctgcattctttaaagttcccttcagcttcttaataatatacccggagaaaaaatctgcctctaattccctttgcctggaaagggcgtatgttaacgcctggttccggagggaatgccccagaaaatggtgccctacttcatgcgcaaagatggcaaaggccacccagtctgtattctgggctactaatttattgaggtattgacggttgtataaaatataccgggtactgtcgccacgggtcattacggctttaaacacaggccccggaaaggcgcattcatacaggatgaaatttgccgccacctggttgtccgtttccatgcctaataactgctggatcttgagaattaccatagccggggtaaaaccatctgcacttaatgatggctgcatatccgggatacaatcatcttccagctgactactcacaaacccgcaggaaaaaaggaaattactatcttccgggatggtatcgctaagcggctgtaaaaccggggcggtctggctgtatgcccggtattgccccggcagcagcataacggctgcgcatagcaacatacatacgatatactttgccattatctggtgaggttataggtgatcgccaggaaatgtccccatttgtaaaaagactccgtttccactgttgttccaatcgttgcctttggaacgatctggccttcctggtatttcgaagaaagcaatgttgcctgggtgagtgtccatccaaagctagcgataaaccgctgttcacggcctaaggccgcagaaacgcccaggtggtaattgaactttgtggtagaccctgtggacaagctcacccctacagccaacgctggctgaaagtcccaccctgttctgtagtaggcgtgcatcagtgcgccgagagagggtactactttattgcggttatcatttctccctattttcacattatccggatcgccgctgatgctatccagccggtaagactggtcaaagaaattgtcgcttccaaaattcataaagaagccggtgctgaagtcgagtttaaacccgccatacgttctgacgataatcggggcttgtaagccaggatccgcacaagtggtgttatcttttggttctattttgatgtcaaatttcagttcatctttatctgcaatagctgcctgcctgatgatataattgatggggttgatcaccttatagctattcactatcaaattcttctgatcaagcagtttataattatcaatgatttcaatcccttttttaacggccgcctcattggattgtttcgtttccactctttcattggtaaccctgatggccttatcgaggataaggttatcgttggcaaactcttctgctttagctgtcttctttacggttaccaactttgccatcagcttgtcagcatcttctttaaaaggttttgcggcctcattaatgtccttctccaattgctccagcgttgccttttcagtggtagccacctgcgtatagtgatcgaggatattaatcacctgggcgagcaacagttcttttgaggccgctgctgtttccgttccgattttattattgttgacaaaagcggtggtggctgccaggaggtttgtctccgcctgcgggtaggcgccatcacaggcctcttttatggctatcagttcatttttataatagaggctatgttgcagtactgctactgcttttttaaatttctccaggctctcccagtaattatccagtttatcatttaactttttatagcttgctttaaacggcgttaactccgcctggtacgaggttttcaatttcaacacaccatcgttaaatgaaaatgcggcgccacctgcgggtttaggatcatctgcggtaccaagatcaacggttgatccgtcgagttttgagaggatagccggttgttgcacgaagaaattggtactggtattatttacctggatgttgtagcggcttttattgatattaatgatttccagtaccaccaggtttccatgctttacgcggtgctttatccttgatttgggtaaatgctggtagtcgatcaggatggtatcgggcgactgggcgtacaggtctgctataggtaacaggaataataatgaaaggaactttttcatgtgtaactattagggataaggaataattgtcgggggctacgaagtactaatctgctctaagataagaaatattacataaaaaaagcatggcatctttcttccggatgataccatgcttttatcatatcgttgttaaactaaactttcaggaacaccttctgtttatacataaaatacaggaataaccattttagaaataccagggagatgctgagggccaccgcgccgaacgggtctcctaccaactgcccaagccatttaaaaaacacctcattgctatagttccagtcgataaagtggcccgaaatatagatgagaatagagttcattccaatcacgcggaaaaagaaagcccattttttataccctgcaatatcgataacataatagaaaagcgcgagcaacaacaggctgataccgcctacctgcaacacaaatgaactggtccacagatttttattaatgggaaaatcaaggttccacaactgtgccagcactaaaaaaacgagtcctgtaagggccattacgcctactttctttaccggggccatcgtgctgttccgtaataaattaccggtgagaatccccaacatcgcggtgctgatagccgggaaggtggaggtaaatccttccggatcatgaataccgagatacaatttaccaggaacaacgagacggtccacgtacgatgcgaaattcccttccatggtaagatcaccgggcgaaaatccgggcgccgctgtaaacttcagcagcagccagtacgcgaccaggatacctacgaaccagatcatttgcgcccgttcctttgtatacaggtaaatgatgttggcaaacatataagccaggccgatacgacctaaaacgctgcaaaatcttatctgcgataccggctgcaattgcaggccgttattataaataacacccagcaacaccagtaccagtcctctttttattacacgcaacagcagctgggtgcggcttttacctttttccagttccctgcctaccgaatacggcgtggaaacaccggccatgaacaggaaaagcgggaatatcagatcatagaaatgaaatccgttccacgcaggatgttcaagctgtacggcgatggcaccccagaaaggagatcctgttgcctttgctatttcatgaaagatggagccgccgcccataatccagaacatatcaaatccccggagggcatctaatgagtaaagccggccttttttttcattgtcacggtttattgctgccggggtcccggtttccaccggcaatgctgttaatgtgctcattgttgaagagatcaaacgattagtgtataatttcaaacgattttggcagcatacaagctaataaaaatggcgctaactttttctaaaattaatctgcaggaaaatcagcccattatatcagcaactaaaagattgattatcaacattgttattcctaacatttaattaccggcgccgctttcttcccgtaaatcttactacagcgccttttccaatatgacattgcccttcacttaaaaggatttcttcttcctccagtgtcagtatatcatagttctcaaagtctgctgctatctctgttttggaaagcagcatattcatatctgttggcccacctacagcaggattgagcttcttcagctctacatgctttttactgaaggcctctaaaataatgatcccgccaggtttaaggtagctgcttaattgttggtgaaatatagattttttagcggcggcgaagtgcgcatacaccagcccgatagcatcaaatgattccttttcaaacgttagctgctccaggtcgccgacaatatattccaggctaacatggtttgctgcggccagttgcaatgcctttgatttccctgctgcactcagatcaaatgaagttaccttccatccaagctgtgcagcgaatacaccattgcgaccttctccgtctgccggcatcagtatggcgcccggctcaaattgctgcagccattcgctgaaaaaatcattcggggctttcccataggcgtactcgttgtttttataccggtcgtcccacatatttttgtattgctcatcccaggattgattcatatacgttgatttataattaaaaaatgagagggtttccgcaaaggtaatgggagcggcacacagaggagtaggacaaaaatgtagtagtataggatttatctgtaatcgcgtctgaacgtttcgggtgaatagcctgtatgttttttgaagaacctgatgaaataggaaacatcttcgtagccaagatgatctgctatctggtttacctgcccggatgttgccagtagctgtcttttggcttccagtataatatattcattaataagtgctgaacaggttttacctatcgttgccttggtgatggcattcagctgatagctggaaagattcagcatcccggcatattgggatacctccttacactttaaaacatgcgtctccaaaagactgaacaacgcatccagttgctcctgcctgtaaatgtttgcgttgcggtgagcatcattaccggactgtcttatcagctgaataaacaacacatccaggtgggctttaataacatgccggtagttttcctgtttgccggtatattcccggaagatatcagttaatatcgcctgcaattgttgaaacccggcagcattaagctgatagtggttgatatttcctgccctgcgtaacaactggctggatactttgtgatgagagaaacagaatccgtcattgaaatgcatcatgtaccctgtgctgcctgctttcaatactaaccggtgtacctggcccgggcgaagaaaaaaaacagtatggtcgccgatcacgtagcgggtgaagtcaatatcatgactaccgcttcccttctccaaaacaagcatataaaagaagtcgtgccggtgatactcctgcaccatgtcatccccatccagtaaggtctgaagatcccggatgccgaagccttcagcagcatccgtacctttttccgctgtagtaatatgtctgacaggtatcttttccatttaactgcactccagtaaaattattattgctgcaatgtgagtcaaatgtaattacattttcataagcccggggtagatccttaaatatacctggagcgccagcggatttttgccatacaaatcatgcagggatttatcatcaaagaaaacactcagctgcccacccaatgcaagccgcgtttttgcaatattcagcaggtcgtaacttacccctgcggtaagtgcgttaaccggaaacagggcatcaccgtacttcgcaggatcaagatccaattcttccactgatttctgtacccattcgtagcgggtataaaccgctgctttcttcatctgccatgctccttccagcaggaacgcgttctctccttcatgaccgggcgttttattcaggccccacagcgttgttacattcatccggttatcgttgcgcattggcaggctgaatatggcagaagcggtagtccggttaacatcttcaccgggatgaagcgcttcggggcttttaacgtagccgtgtgacacctggaatgcccagttgcgggaagggttaaaggaaagcctgccactccaggaatcaaatcgcattttatcgaagttgtacctgttctcgtcgggctcccttcctgtaaagagtgacccttccaatttaaacttatccacgcgcacaccgagggtggccactccgaaagtgatatgcgttccgtcgttccagtgatgactgacaggcgcatccgggtttgctaacgcagacgggcgatgcataaaggcaacagatcccaatgccggttcacccggatagccgaaataagcaaaggcgtctactttttttgaaaaagcataactgtaactgacggataattcagaaaacaggtcatgcggatgctggcggtcgaccagtggctgtcccttccagctttcgccagatcccacgagtattatgccactttagcctatctctaccgtcacatcatccgtaagtggaaagctctggcaaagcagcaccattccctcatccagctcctgttgcctgagcgcataattaccgcgcatttttactttcccggcagtgagtttcgccgcacaaataccgcaggtgcctcctttgcaggaatatggcaatggtatcctgtcttccagcgccgcttcgagaatcgttttgccggcggccacgtccagcaggttgctctgttcgtaaaagtggagcaatacttcctgcgcggcaccgggcaatacttcctcttctttgctactatccggggaaaaccattccatgaaaatacgatctgccggcacttgcagcgcttccagcacttcctgctgcattttcatcaagcctgatggaccgcagagaaaatagtgaaccccctcaccggaatcggtcactgcctgttgaataagcttacgggtaaccagtttgcccagtctgccgctgataaattcgggggcagctgctccttcataaactgatatcgcgtgataaacgttgatccgttcccggtagtgttccttccactgtgcaatgtcatctctgaatataatttcatccggtgtacgactggcgtagacgagtgtaacatgtgtgtccggagcggtatcgatcactgacctggcaatggcatacaaaggtgtgatcccgcttccgccggccagcagcacaacgtgctttgcctgatagctaccgggtaccggcgtaaatgagccatagggaccggatactgtccaatgttcaatggcggaggccttatcggcaatatagttgctcatgatgccaccggctactctttttacggtaatggctggttgtttatccctgctacagactgtgcttaaagaataagacctggtaacagtggcgccgttgatcgttaatgttagattgataaactggccgggttgatatataaaaggctggccgccggtatcaaactttatggtgactgtggaggcagtttcccggatgatacccgcggtgcgccagatctgtacattgttcatgctttctgatgatttattttaaagacgtgcggcttttaaacgcaaactattgctgaccacacttactgagctgagggccatcgcagcaccggcaatcataggatctaataaaaatccgttgacagggaataaaacaccggcggcaatgggaataccaataatgttgtagatgaatgcccaaaagaggttctgtttaatggtgctaaccgttttccgcgacagcttcagcgcttttggaatgctattgagatctgaggtaatcaacgtcattttggccacatccatggcgatatccgatcctttgcccatggcaatacttacatccgcctgggccagtgcctgtgagtcgttgataccatcgcccaccatcgccaccacttttccggattgctgcaattcttttacaaatgcagctttatgggaagggagtacttctgctttatagtgcttcaatccaactttcctggctaccgctgcggcggtgtgggtgttatcaccggtaagcatatatacctcaatgccttgtttttgcaaggatgcaatcgcttccctggaggtttcctttattttatcggcgatggcgatgaccgccagcagttgtttgcctgcggcaaaatagatcactgttttggcatcttcctgcaaggcagcggcttgtgttgcctgttgcggatcgatggtgacattgttctcctccatcagtttgcggttacccaccaggtaaacagtttgttcaaaagtgccttgtatccccttaccggtaaggctttcaaaggcagacaacttagcgaatgctgcgccgttgtctttcaggtaagatactacggcctccgccagcgggtgttccgactgttgttcaagtgcatacaatactgattgggctgcggagtgggtatgagcaggtgcatgccaaaccaggtcagttaccaccggtttaccttccgtaatggtaccggttttgtcgaggatgatggcattcactttatgcgccagctccaggctttcggcatctttaataaggatattattttcggcgcccttccctactcctaccatgatggcggtgggtgttgccagtcctaatgcacacggacaagcgatcaccaataccgttaccgaggtaagcagtgcatgggtgaaagcattattgccaccaaacaccatccaggaaacgaatgtaaggatagcaatgcctattaccaccggtacaaagatccctgcaatcctgtctaccagcttctgaacaggcgctttactgccctgtgcttcctgcaccattttgataatctgggccaggagtgtatctgcgcctactttttctgcacggaaacggaaactgcctttctggttgatggtaccggcaaatactgtatcaccggcatgtttagccaccggcaccggttcgccggtgatcatactttcatccacgtaggaagttccgtctgccagctttccgtctaccgggatcttttctcccggctttaccagcagcaggtcctggacttttacagcggagacaggaatttcgcgggtttcgccggattcatctaccagcaatactgttttgggttgcagaccgataagtttttttatggcagatgaggtattggatttggctttttcttccaggagtttaccgagtgatataaatgcaatgaccacagcggccgcttcaaaatacacatgtgcatgtaatccgcgctggtgccagaacccgggatatattgtattgaaggcactgaacaaccaggcgataccggtactcagcgccaccagtgtatccatattggctttcctgtgcctggcctgcttccaggcattgatgaagaagttgcggcccaggaagaacaccaccggggtagcaagcgccatcatgatccagttgccgtatggcatattcataaagaacatcccgatgataacaatgggaagcgataataccgatgcccagatagtacgttgttttacctcgcgatagtgacgctgctgtgcttcttcctttacttcatcctggttttctttgtctatcaccaggtcgtaccccactgaacggacgctgctttgcagcatttcaggggtgacggcggcatgatcgtattgtacccaggcggtttgattggcgaagttaacgccggcgtcctgtacgccgggcaccgatttcaacatggactccacgctaacggcgcatgccgcgcaggtcatttccaacacgggaaaggtttcttttgtggtaccggcagcgtgcttcctgttggtggttggttcctgtaatgatatagctgatgacatatattgctgattttctacaaaactacgctgctgccggggcacgtatgttacactattcagggggaattgtatataattttaagaccggttgtcagggtgatgggtcagggcctgctttgatttcctgatttctttaaagtgagaggtattgaggccggtttgatctttaaactgccgggacagatgggcgccgctgctataacccagtttaaaggcaatgtctgaaagggtttcatcggtataaaccagtaattcctttactttctctacacggtattctttgatatatttctccagggtaacgccttctgcttctgaaaatatattgctgatcatactataatctttattcagcgcgctggatactacctctgaaaacctgaagttatccgggaagtcataggatcccgaatacacctggtcgatcaggttcttcacctctcttaccagcttcgtctttttatcttccagcagggtgaatcccagcagcgctaatttctcccggagagtatccatatccggttctgataatgccgttatggtggttacctgccccagcacaatgccggctaccggtatccgcagctcgtgcagcgcttctttcaccgcaaggatacacctgtcgcaaaccattcccttaataaatatcttatagttacttagcatataaacagtatttgagctatgcaaagttcaactattccaccggcaggggtattataaaattcaggggaatatttatataattataatttactgtttatagatatactccagtgcttcatctttgttattaataaaattgagggaacggtaggtaattgctttatcgggcattaatgctccttttttacctttccagttttcccaatacctggttgaatagccgatcacgatcttcgtgttcggaagccggaatccgcgtacttctccatagtggtttatgttgccgctggtcatttgtcccaccaaaatggcattggtatatcttttaaattcaacggcattcatcagggcagaagaaaaagtttgcttcccgataagtacataaaaatgcgctttcttatttaaataactgtgtttaatactgtcgataaaaggtctcagtacgccggaatttcctccgctgttaaaccggaggtcaacaataattttaccgggatgtaagctgtttatttttgaaaacagttcctcattaaactgcgcgaatgggtgttgttcatcatcgttgcaccgaatgaaattgaaatagattgtttttctggcggagtcatattcataccaatagtctctattttgctccctgtaaggtaacatggcgtcgtattgggcggacagggctatgttcaggctgtctttatgaacggctggaagtgttacctggtacacttctccatcgcggctttgcagcgtgaatgccgcgctttcatccgagcttagaatgcccagtcctttaagaaaagagggattattcagcaattgttgttcatagacttcaaaataggattgattatccgccttaattacttctttaaatttcctgttgatttcatcgatggaatgcccgttaatcgctgttagtttagataaaagcgcagttgattgctgcggagcaataccagtaacaaaaatgccgtcgtcgaacacggtaaactttacaggcaaaacagttttgaactgcggctcaatcctggtatgctcatcgccgatcaatacgtttaacctgaaaagttccaccatgaaggtttcatcattcagggtgtcaattttccccgctacaccggcaactttattttcaaattcctgtttgctgattttattaaagagatttttgtgctttaccggaagggtatcgcggtagtacattaagtcttccagcagttgttttttttccaggtgctgcgaaaaggaatgattggaaattaatatcaacaggcaggatatcaaagcacagtgtcttttcatttggttcagttttttgttgtctcctgcatagctgttgcaggtatccaacaatatacgtccaaccggttgagtttcgtatacgcggactggtttaaatatggatatcttgtcttgttccttaattcctacatttgtattttaaatttaccgggaatggaagaaaataaagcgcactgggagaatgtttaccatacaaaaaaaccttcggaggtaagctggacacaagatgtaccgcaaacatccctcgatttcattctttcctgtaatattccaaaaacggcaggcattattgatatcggcggcggcgacagtaaactggccggcttcctgctggatgcaggtttcaccaatattaccgtactggatatttcggccagggcattggagagggcgcgacagcgcctcggtgaaaaagctgacctggtgaaatggatagtgcaggatattactacttttcagccggatgcctcctacgaggtgtggcatgacagggctacttttcatttcctgacggcagcagaacaggttgaccggtatttaaatattgcccgtcaaagtatcaatgccggtggctatgctgttataggtactttttctaccaacggtccggaaaaatgtagtggtctccctataaaacaatataacgagggtacgctgacggatcagttaagcaacggtttcaagaaagtaaaatgtatcacagaaaaccatgtaacgcctttcaatacaacgcaacatttcctgttttgctcgtttaggcgaactttgtaacatgtttacgcttttaatacctgccgctctgaaagcttgccgtatttaaggtgatattctttcgggctcatgtctacctggcggcggaaaaccttccggaagaagctgatatcttcataaccgcattgcaatgctacgctctcaacgctttcccgggtattttccagcagctttttcgcggcttcaatacgcacgcgctgcaggtattcaatgggggtattgccggttgcctgtctgaagcggcggatgaagttcctcacgctcatatgatggtcgctggccagtttttccaggatgatggcttccccgtagtttgcttcgatgaagtgttgtattttcttaaccggatcatccgcatgatcatgctggaagcggaatacggagaaagccagctgtgagtcaccgtgtgtgttgatcattagtatttttgatgccatcacggcttcttcgtgacctactaatttttctatcaggtagatcataaaggaggtgaagctaaacgcgcctccacaggagcataccggtccttcgtccacgatgatcttatcgtcctgcacaccgatagccggatagcgctgctggaaccggccggcaaacagccaattggtggtagcctttttgccgttcagcaagcctgtttcggcaagcaggaaagcacccacgcagatgctggccaggtcggcgcctttctggcgttgttgtttcagccatgttaccagcctgccttcccgggcaatcacctcgtcgatcttatcatagcgcatggcgggaatgataattaaccggtaccggtcgcgcggactgagcttttcggccttattgcttccttgtggacgcctggtaagctggccatccgcttcggcaataaaatcgatctcaatgttctcctttaagggtataccggttgccaacggatacatcctgctgaggcctccccatatgtcagcagggcctgtcacgcacgttggaaccgcatctttataatccagaatagcaatacgcaaggcagttcttttacgtccaaagatatggcaatatcgccttcttttttgtcattactgccacttatttcattccgggaggagggctacttttatggtgttaaaagtaactggcaatagccgggtatacatcactcaataaatctgaattttatgtcaacagtaactaataccatcatgacgacccacgaagtggccgcgcgattcaacgaactggctcaacaggaattgtggtttgaaatccaggatgagttttttgcagatcatgtaaaaagcatagacccaccccattctctctactttggctatgcggagggcatagcggatgtccgcaaaaaaggtaaagactttgtttcaaaaatccgggacgttcacggcgctcataccaccgagcctgttgtggcgggtaattatttttctgtaggccggaatatggatgttacggtagaaggatttggaagaatacagatcgatgagatcatgttatacgaagtaaaagacgggcagattatatcggagcaattcttctattaagctgctgctagtccagtatccgcatccggtaggcattcatagccgtagcgccgagctttgtgacaaggcggtaatttaccactacgcccacagccgcacccactacgggcagcaactgtcccattttagccagatcaatatgatcacggtattcgatctggaattgctgccaatcgaagctgtgaatgtcttccggtaaccggctgcttttctctttccagtccacaatacactcatacacgttttgccggtgttcctggctgctgaaggccagctggaaaatataaaggatatacaaccgttccttataatcttttacatcaaagccataaaaggtggcgatgtcaaaaagcagtttcaatttcatcccgagcagtatcgggaaatcagcaaggccccataaaaacccgccggcgccggtaagcccaccttcagcggcagccgttttccggtaaaagtccacccggcgaagcaccgcttcttccaaatcatacaacgaagcaaaaacaggctggttgggtacggtgtacatagaaccgaacagtaccccccgcaccatttgtttaatggttacagtaatagcatcatgcactttttgcgggattatgcggttgatgcgtgactgcaccgaccgggataaccggtctgccagagaaggccggccctgcattttatgctgccagatctccaattctactttcatccgctgttcatataacataaccgaaattacaaaaaagaagacagccggcagcacccggtgtttaaccagttcgattttaaaaaggaccagcaggaagatataaaaagtgtggaaagaagcgctgtgaaataactttatcaggacaccccgctgccgggttgaataccgcagccctggcggtcctcattaaaaaacattttcatttttccggtcatcatcccgttccatccggcctggctgaggtatacctcattgcctgccatgttcctgaacacggaagtagtcgtgatcatcttctgctgatgaccacctattacaaaatcaatatgcgtagacctggtagccatatcagcgttatctgctgtttcgccgggttgcttaaagccgaggtgggaaaggcagatcactacgtggcagccatgctcttttttaagtttagcggccacttcgtcggcggttgctaccggcggcaggaaggtgacaccgggaacatccggcagttgcggccccacaccggtgatacctatttttaacgagcccgcatatacgattttatgacgtaccacctggcgtgcgagtgatggatcggtaaaacggtagttgcaatttacaagggcaaattgcatatgcgggatcagtgcggccaatgcagcctggccgttagccagttcacgattaccgatagtggctgcatgataaccggctttattcatggcctgtatcatttccatacaggcgttcacgttatccgttccactggtaaaatcacctgcgtccaggaatacaccctgatctcctgccgggcggtgaccggccagctggccatgcaggtcgttggtatgccagatcaggagttcccggttatcgccgggaagataagtcgcattttctgaagtggaagtcagcgctctgagaggattctgcaacagcaataaacctgttacaagagatgtattccgtagaaaggaacggcgttctttattcataatatagggatctggaaaaaagtgatgtgaagataaacacttccgttgatttcttgttaaagcaaataaatattactttgaaaaaaaaataaaatatacttttatggcagtttttcatagataacacgactaatatcccttgcaataccagatacaacgattatgaatgactctactccctacctgtcagagatctttttagtggcttttaattttgcgccgagagactacgcgttatgtaatgggcaattacttcccattaaccggaatcaggctttattttccctgttgggtactgcgttcggcggcgatggccgggttaattttgcattacccaacctgagagggcgcataccaatgcaccaggacgcggcccatatgctgggaacagtaaccggcaaggttactactaccgtcaccgttgccaatcttccggtacatgaacacggcgttacggccgtacttaaactgcctgtgggagctgcggcaaatactgattcttctgccaatgcttatcctgcacccgttgccgccagcgccaggtacagcgacaccgcggatgaacaaatggccacggtacagggcggcgaccttgcagcagacacggcgaatggtgcgttagctacggagaccaatccctctccgaatacacctgttaacaacatgatgccttacctcaccatgaattatatcatagccctgacaggcatatttccttcaaccacctgatttttaaatatatgtcggcactcgatccattcgttggtgaaatcattatggtccctttcaattttgcgccaaaaaatttcgcgttttgtgacggacaactgctccctatttctcagaatatctcgcttttctccatcctgggcacttactacggaggggatggcaagagcacttttgccctgccggacatgcagggaagagttcccatcggggccggccagggacctgatctgacacagcgggagcttggcgaaatggggggcgccaatgaaaaccagctcaccatcaatcaaatgccggtgcatacgcatctgatcaagcggcgaccgttatctttaccggcaggcgaaaataataataccaacaatcctatcaacaattatcctggcatagcgccttcgggacttccctatggtaaaacagccggcaccgcaacaatggcagatctgaggtcaaggatgcgggcagcaggagcaggcggcaatacaccagtgaataattgtcaaccaaccctcactattatgtttgctatatcgatggcaggagtattccctccccgtcaataataaatgatcacactcaaacactgatacgaatgccttttgtaggagaaataagaatatttgccggaaattttgcaccacttggatgggccttttgcgatgggcaattacttcccatttcagaaaacgatgtactgtttcaacttattggtactacctatggtggggatggtcagtctgtttttgcgttgccggatctgcgtggcagggtgccgctgcatatgggtagcgattcttccagcggcttaacttatcaaattggcgaaaagggaggagaagaaactgtcaccttggcttccgataatcttccgccgcatatgcattttatttccggaccggtatttttacctgccctgggagaaaatcacgcaaatgccatcaaccctcagaatcgttcttttgccatcaccccatcagaaaaaatttacagtactgttaaaagcactaccaaaaggttggcgcctttacaggttgcacatacaggcatgtcgccagccggtgattctttaataatgacggtacagccaaccggcggtacagcccccaccgacaatatgcaatcatacctggtggtaaattttattatttccctgtttggcgtatttcctacaccttaagaaccagccatatgaaaataggagcactcctacccagatctacctttcatccgctgctgcagcacgacttcctccagggtgtggaggcttatctgcaataccggggcgtacctgttacatggtttaccgccaatatcgggtttggcaccaacgccgaaatggtaatggaacaggcagaaaaaatgatgctggaacaccatgccgatgtactggtgttatatgcagatcaaccggcagtaagcaatatagccgcactggcaaagtcgttgaaccgcctcgtactactggtacacaacggcgcaaaatatatgcatgaatgggaacctcatccaacagtactgtcgcacacacttaacaacaccattcaatgccgactgaccgggatctacgctgccaccctcgcaaaggatgccgctgtatgtacttcgttttatgacggcggctattctcataatcatgcgctggtacaatcgttcgccgataacggcggcagtgttgcctataacttcgtaagccagtataaagtgaaggaatttgattccacgccactgcatcacttcctgcgtactaacgcacacgtacaaacgttgctggcggtttataacggggacctggcgcattgttttcttcagcagttgcaggcatcggatgtaacggagggcctgcaggtattcgccagccccatgttgctggatgaaaccctgtcagcagtgcatggtcacctggaaataccgttccaggtgagcgggtatgttccgtggatttcatctctcaaaaatagcgctaacgaattactgaaaacacagtttactgcttataccggccgcgaagctaatttacctggtatgcacggctggagtaccggtattatccttgaacatatttataatacggcagatacacatcgattccgggcacgggagatcctgctgacgctccacgacgtaacactggatagtccccgcggccccctgcatatggatgcagccactcaccacatgatggcacctgcatggctggtgaaaacaaatgaagcgtttgagccggaaataattggcggaacagataacaccgcgcagatctggcaggaaattgtgaatacggagatacaaggtgtgtcttccggctggatcaacacttacctctgcgcctgataaagatcaggtgaggtactttcaagcaatttaacatcctgaacaacagggtgcatgtctatatatttcttatacctaaggctcgcctttttatgaagttaattttacgcagaaccctgatatccctattattactcacaggcattgctacctgcgcgcaggcgcaggcctttggccccggcgatctcgtttttaccggcgtgaatatttatgacgacgacaataacggcagcatacagaacgatgcgttttcgtttgtgctgctccgtgagtgcccggctaatacgatcatttattttacagatctggggtggacaggtgccggctttcagtctatttccagcgacatttccaccggctccaaaacagatggtattcttcaatggtcgcccggcaccagcaaaatggcggtgggaacacgggtaactatttactgtaaatatagtcctactgcctcttccggcgtacttaacctgaccagctctacccctactgccaacagcgccgcactgaccaataaagaatatatcagtcttggtattgcaggtgatcagttgtttgctttcaccggtagttcaggtaatccgaatatcattgccggtatcaatgtgaaccgcaacacctgggaagcatctcttgctgcggatgaatttacttcttccaaatcaacccagccagctactaccagcgttctcaattttcccagcgtaaacgcagtgaacgcgcggtataattgttcgttaactatcggtacttcggcccgcctgcgagcctttatacaggacaccaccaactggacgaaggactataccttgtcagcgccagcccctgccgcattaaaccttgccgtcacaccaacgtgttccctgacggtagtgaaccccgatgtcaacggcattgtatatgtaaacaaaatatttcccataaacggcgacggcagcagctgggccaggccggtggttgaattgtcgactgcactcaaagccgccgcagagccgctgaatggtattacaaaaatatgggtagccgcaggtacttataaacctgactactcggggaacaccctggctacatttactataccttccggcgtagccgtttacggtggttttataggtaatgaaactaaattggccgaccggaatattccggtcaacccggtaatcctgagcggggatgtggatggaaatgaccggcttaccaataacgttgtcctgagtacagcgaatatccggggcgccaacagccgtcgcgtgataacggtgggctttctcagcgcagaaagcatactggatggcgtcatcattaccggaggccaggccagtaatgccggtggtggtatagacgccacgaatgccacactgacaataaagaattgtcaattttacgggaactacagcgcccaatatggcggcgctgttaaccaatccggcggcttactgcaactggtcaactgcgtgttctttggcaacaatgccgtgcttgacggagccgctataagaagctccggcaataccactcttaccaatgttaccgtgggaggcaatacctccggagggtccgctatatccagcagcggcaccttcacttcgtataacagtgtggtagctaaaaatacttcttccggtagtgggggcgattattccggtcccactccaaacatccgttacagcatttttggtaacctgtattatgccagcacaggtacttcacaggctactcctgatgtggtgttcaacaaccttagcaccggggacctgcggttaacgcccgtcaactatggtatcaacaaaggcgatccgcaaaccaacgacgcaggctatcccgcacaggcagatacattggatcttgacaggaaaatacgtatcagcaatactgttattgacctgggcgcatatgaaatacaggcaataccacaaacgatcactttcccggccttccctgctactccggttattacctacggtgatatagatattgatccgaaggcaactactaccggagatggtgtcattacttatacttccggcaatacggccgtagcagacaccctgaacgggaaaataaaaactaccggtgcaggtacggcggtgatcaccgctcacgcagctgctaccaatatttatctgcctgcaacacctgtaacaagacctgttaccgtcgcgaaaaaagcgctgaccataaaagcagatgatgccagccggccgtataaaacggcgaaccccacccctacgtttacctacaccgggtttgcctacacagatgatgcgagtgcgatcaacggtacggtagctgccatctgggcagctgatataaacagcaacgtgggcaactatgctattacaacggatctgagcagcgccactgctgataattacaccttgtcaggagcaggtggtatattaaccattacgcaacagcagcaaaccatcaccttccctgcaccatccggtgtggtttatggtgcggcgccgattaccctgccacttaatacggatgcaggtttgcctatcatttacaatgtggtgtctggtccggctaccgtgagcggcaacacgctcaccattaccggcggaggcaatgtaaccgttaccgccgatcaaccgggaaataccaattacaccgcagcgctacaggtaacacaaacatttaacgtagccagagccattctcacgataacagcaaacaataagaacaggccgtataagcaggctaatcctgtattggattataccattaccggcttcgtgaacggcgacaacagcagcgtgataaacggtgatgcgagcatcagcactacagcggatattgatagtcataccggcgactaccctatcaccataagcgccggcactgctactgccaccaattaccagttcagcttcaaaccaggtacgcttacagttaccaaagcaccgcaggtaattacccttagtgccttaacggataaaacatatggcgacgctccttttgccctgaatgccaccagtacctccggtctcacggtggccttcagtgttgccggtccggctactatcagcggtaacatccttaccattacgggcacaggaaatgtaacggtggcggctacacaaagcggcgacacagattacgatccggcaaccattgtcacaggcgggtttaccgttttgaaaaaatcattatttgtaaatgcagataacaaacagcggttatatggagaaaataatcctgcattaacctatacctacaatgggctggtgaatggagatgataacagcgtagtaacaggcactccgctgcttagtaccacggcagatgccagcagtgcgccgggtggttacccgatccaggtgaccaacgccgcctcgctgagcgctgtcaactatagcatcattcctgtaaacggactgctgacggtaacaacggcgcctcaaaccattaccttcccggcaataggcaataaaacctatggcagtgcgccggttacgcttaacaccaacagcgatgcaggtttgcctatcacttataacgtagtaagcgggccggcaacactcagtggtaatgtcctcacattcaccggcgcgggcgatgtaactatcactgctgatcaggcaggtaatggcaattactcgccggcgacgcaggcatcacaaacattcagcattaccaaagccacactaacggtaacggctaatgataaaaacagggtatacaaacaaactaatccaacaccggattatactgttaccggttttgtaaacggcgaaaacagcagtgtagtaagtggtgatgc

(The sequence listing continues in the following parts.)